European Patent Specification EP 3 642 334 B1, published December 27, 2023. Title: NUCLEIC ACID-GUIDED NUCLEASES. Applicant: INSCRIPTA, INC. Application PCT/US2018/034779. The sequence listing filed with the application follows.

SEQUENCE LISTING (801 sequences)

SEQ ID NO: 1 - protein, 1358 aa, Artificial Sequence
  Description of Artificial Sequence: Synthetic polypeptide
MGKMYYLGLDIGTNSVGYAVTDPSYHLLKFKGEPMWGAHVFAAGNQSAERRSFRTSRRRLDRRQQRVKLVQEIFAPVISPIDPRFFIRLHESALWRDDVAETDKHIFFNDPTYTDKEYYSDYPTIHHLIVDLMESSEKHDPRLVYLAVAWLVAHRGHFLNEVDKDNIGDVLSFDAFYPEFLAFLSDNGVSPWVCESKALQATLLSRNSVNDKYKALKSLIFGSQKPEDNFDANISEDGLIQLLAGKKVKVNKLFPQESNDASFTLNDKEDAIEEILGTLTPDECEWIAHIRRLFDWAIMKHALKDGRTISESKVKLYEQHHHDLTQLKYFVKTYLAKEYDDIFRNVDSETTKNYVAYSYHVKEVKGTLPKNKATQEEFCKYVLGKVKNIECSEADKVDFDEMIQRLTDNSFMPKQVSGENRVIPYQLYYYELKTILNKAASYLPFLTQCGKDAISNQDKLLSIMTFRIPYFVGPLRKDNSEHAWLERKAGKIYPWNFNDKVDLDKSEEAFIRRMTNTCTYYPGEDVLPLDSLIYEKFMILNEINNIRIDGYPISVDVKQQVFGLFEKKRRVTVKDIQNLLLSLGALDKHGKLTGIDTTIHSNYNTYHHFKSLMERGVLTRDDVERIVERMTYSDDTKRVRLWLNNNYGTLTADDVKHISRLRKHDFGRLSKMFLTGLKGVHKETGERASILDFMWNTNDNLMQLLSECYTFSDEITKLQEAYYAKAQLSLNDFLDSMYISNAVKRPIYRTLAVVNDIRKACGTAPKRIFIEMARDGESKKKRSVTRREQIKNLYRSIRKDFQQEVDFLEKILENKSDGQLQSDALYLYFAQLGRDMYTGDPIKLEHIKDQSFYNIDHIYPQSMVKDDSLDNKVLVQSEINGEKSSRYPLDAAIRNKMKPLWDAYYNHGLISLKKYQRLTRSTPFTDDEKWDFINRQLVETRQSTKALAILLKRKFPDTEIVYSKAGLSSDFRHEFGLVKSRNINDLHHAKDAFLAIVTGNVYHERFNRRWFMVNQPYSVKTKTLFTHSIKNGNFVAWNGEEDLGRIVKMLKQNKNTIHFTRFSFDRKEGLFDIQPLKASTGLVPRKAGLDVVKYGGYDKSTAAYYLLVRFTLEDKKTQHKLMMIPVEGLYKARIDHDKEFLTDYAQTTISEILQKDKQKVINIMFPMGTRHIKLNSMISIDGFYLSIGGKSSKGKSVLCHAMVPLIVPHKIECYIKAMESFARKFKENNKLRIVEKFDKITVEDNLNLYELFLQKLQHNPYNKFFSTQFDVLTNGRSTFTKLSPEEQVQTLLNILSIFKTCRSSGCDLKSINGSAQAARIMISADLTGLSKKYSDIRLVEQSASGLFVSKSQNLLEYL

SEQ ID NO: 2 - protein, 1334 aa, Artificial Sequence
  Description of Artificial Sequence: Synthetic polypeptide
MSSLTKFTNKYSKQLTIKNELIPVGKTLENIKENGLIDGDEQLNENYQKAKIIVDDFLRDFINKALNNTQIGNWRELADALNKEDEDNIEKLQDKIRGIIVSKFETFDLFSSYSIKKDEKIIDDDNDVEEEELDLGKKTSSFKYIFKKNLFKLVLPSYLKTTNQDKLKIISSFDNFSTYFRGFFENRKNIFTKKPISTSIAYRIVHDNFPKFLDNIRCFNVWQTECPQLIVKADNYLKSKNVIAKDKSLANYFTVGAYDYFLSQNGIDFYNNIIGGLPAFAGHEKIQGLNEFINQECQKDSELKSKLKNRHAFKMAVLFKQILSDREKSFVIDEFESDAQVIDAVKNFYAEQCKDNNVIFNLLNLIKNIAFLSDDELDGIFIEGKYLSSVSQKLYSDWSKLRNDIEDSANSKQGNKELAKKIKTNKGDVEKAISKYEFSLSELNSIVHDNTKFSDLLSCTLHKVASEKLVKVNEGDWPKHLKNNEEKQKIKEPLDALLEIYNTLLIFNCKSFNKNGNFYVDYDRCINELSSVVYLYNKTRNYCTKKPYNTDKFKLNFNSPQLGEGFSKSKENDCLTLLFKKDDNYYVGIIRKGAKINFDDTQAIADNTDNCIFKMNYFLLKDAKKFIPKCSIQLKEVKAHFKKSEDDYILSDKEKFASPLVIKKSTFLLATAHVKGKKGNIKKFQKEYSKENPTEYRNSLNEWIAFCKEFLKTYKAATIFDITTLKKAEEYADIVEFYKDVDNLCYKLEFCPIKTSFIENLIDNGDLYLFRINNKDFSSKSTGTKNLHTLYLQAIFDERNLNNPTIMLNGGAELFYRKESIEQKNRITHKAGSILVNKVCKDGTSLDDKIRNEIYQYENKFIDTLSDEAKKVLPNVIKKEATHDITKDKRFTSDKFFFHCPLTINYKEGDTKQFNNEVLSFLRGNPDINIIGIDRGERNLIYVTVINQKGEILDSVSFNTVTNKSSKIEQTVDYEEKLAVREKERIEAKRSWDSISKIATLKEGYLSAIVHEICLLMIKHNAIVVLENLNAGFKRIRGGLSEKSVYQKFEKMLINKLNYFVSKKESDWNKPSGLLNGLQLSDQFESFEKLGIQSGFIFYVPAAYTSKIDPTTGFANVLNLSKVRNVDAIKSFFSNFNEISYSKKEALFKFSFDLDSLSKKGFSSFVKFSKSKWNVYTFGERIIKPKNKQGYREDKRINLTFEMKKLLNEYKVSFDLENNLIPNLTSANLKDTFWKELFFIFKTTLQLRNSVTNGKEDVLISPVKNAKGEFFVSGTHNKTLPQDCDANGAYHIALKGLMILERNNLVREEKDTKKIMAISNVDWFEYVQKRRGVL

SEQ ID NO: 3 - protein, 1238 aa, Artificial Sequence
  Description of Artificial Sequence: Synthetic polypeptide
MNNYDEFTKLYPIQKTIRFELKPQGRTMEHLETFNFFEEDRDRAEKYKILKEAIDEYHKKFIDEHLTNMSLDWNSLKQISEKYYKSREEKDKKVFLSEQKRMRQEIVSEFKKDDRFKDLFSKKLFSELLKEEIYKKGNHQEIDALKSFDKFSGYFIGLHENRKNMYSDGDEITAISNRIVNENFPKFLDNLQKYQEARKKYPEWIIKAESALVAHNIKMDEVFSLEYFNKVLNQEGIQRYNLALGGYVTKSGEKMMGLNDALNLAHQSEKSSKGRIHMTPLFKQILSEKESFSYIPDVFTEDSQLLPSIGGFFAQIENDKDGNIFDRALELISSYAEYDTERIYIRQADINRVSNVIFGEWGTLGGLMREYKADSINDINLERTCKKVDKWLDSKEFALSDVLEAIKRTGNNDAFNEYISKMRTAREKIDAARKEMKFISEKISGDEESIHIIKTLLDSVQQFLHFFNLFKARQDIPLDGAFYAEFDEVHSKLFAIVPLYNKVRNYLTKNNLNTKKIKLNFKNPTLANGWDQNKVYDYASLIFLRDGNYYLGIINPKRKKNIKFEQGSGNGPFYRKMVYKQIPGPNKNLPRVFLTSTKGKKEYKPSKEIIEGYEADKHIRGDKFDLDFCHKLIDFFKESIEKHKDWSKFNFYFSPTESYGDISEFYLDVEKQGYRMHFENISAETIDEYVEKGDLFLFQIYNKDFVKAATGKKDMHTIYWNAAFSPENLQDVVVKLNGEAELFYRDKSDIKEIVHREGEILVNRTYNGRTPVPDKIHKKLTDYHNGRTKDLGEAKEYLDKVRYFKAHYDITKDRRYLNDKIYFHVPLTLNFKANGKKNLNKMVIEKFLSDEKAHIIGIDRGERNLLYYSIIDRSGKIIDQQSLNVIDGFDYREKLNQREIEMKDARQSWNAIGKIKDLKEGYLSKAVHEITKMAIQYNAIVVMEELNYGFKRGRFKVEKQIYQKFENMLIDKMNYLVFKDAPDESPGGVLNAYQLTNPLESFAKLGKQTGILFYVPAAYTSKIDPTTGFVNLFNTSSKTNAQERKEFLQKFESISYSAKDGGIFAFAFDYRKFGTSKTDHKNVWTAYTNGERMRYIKEKKRNELFDPSKEIKEALTSSGIKYDGGQNILPDILRSNNNGLIYTMYSSFIAAIQMRVYDGKEDYIISPIKNSKGEFFRTDPKRRELPIDADANGAYNIALRGELTMRAIAEKFDPDSEKMAKLELKHKDWFEFMQTRGD

SEQ ID NO: 4 - protein, 1298 aa, Artificial Sequence
  Description of Artificial Sequence: Synthetic polypeptide
MTKTFDSEFFNLYSLQKTVRFELKPVGETASFVEDFKNEGLKRVVSEDERRAVDYQKVKEIIDDYHRDFIEESLNYFPEQVSKDALEQAFHLYQKLKAAKVEEREKALKEWEALQKKLREKVVKCFSDSNKARFSRIDKKELIKEDLINWLVAQNREDDIPTVETFNNFTTYFTGFHENRKNIYSKDDHATAISFRLIHENLPKFFDNVISFNKLKEGFPELKFDKVKEDLEVDYDLKHAFEIEYFVNFVTQAGIDQYNYLLGGKTLEDGTKKQGMNEQINLFKQQQTRDKARQIPKLIPLFKQILSERTESQSFIPKQFESDQELFDSLQKLHNNCQDKFTVLQQAILGLAEADLKKVFIKTSDLNALSNTIFGNYSVFSDALNLYKESLKTKKAQEAFEKLPAHSIHDLIQYLEQFNSSLDAEKQQSTDTVLNYFIKTDELYSRFIKSTSEAFTQVQPLFELEALSSKRRPPESEDEGAKGQEGFEQIKRIKAYLDTLMEAVHFAKPLYLVKGRKMIEGLDKDQSFYEAFEMAYQELESLIIPIYNKARSYLSRKPFKADKFKINFDNNTLLSGWDANKETANASILFKKDGLYYLGIMPKGKTFLFDYFVSSEDSEKLKQRRQKTAEEALAQDGESYFEKIRYKLLPGASKMLPKVFFSNKNIGFYNPSDDILRIRNTASHTKNGTPQKGHSKVEFNLNDCHKMIDFFKSSIQKHPEWGSFGFTFSDTSDFEDMSAFYREVENQGYVISFDKIKETYIQSQVEQGNLYLFQIYNKDFSPYSKGKPNLHTLYWKALFEEANLNNVVAKLNGEAEIFFRRHSIKASDKVVHPANQAIDNKNPHTEKTQSTFEYDLVKDKRYTQDKFFFHVPISLNFKAQGVSKFNDKVNGFLKGNPDVNIIGIDRGERHLLYFTVVNQKGEILVQESLNTLMSDKGHVNDYQQKLDKKEQERDAARKSWTTVENIKELKEGYLSHVVHKLAHLIIKYNAIVCLEDLNFGFKRGRFKVEKQVYQKFEKALIDKLNYLVFKEKELGEVGHYLTAYQLTAPFESFKKLGKQSGILFYVPADYTSKIDPTTGFVNFLDLRYQSVEKAKQLLSDFNAIRFNSVQNYFEFEIDYKKLTPKRKVGTQSKWVICTYGDVRYQNRRNQKGHWETEEVNVTEKLKALFASDSKTTTVIDYANDDNLIDVILEQDKASFFKELLWLLKLTMTLRHSKIKSEDDFILSPVKNEQGEFYDSRKAGEVWPKDADANGAYHIALKGLWNLQQINQWEKGKTLNLAIKNQDWFSFIQEKPYQE

SEQ ID NO: 5 - protein, 1235 aa, Artificial Sequence
  Description of Artificial Sequence: Synthetic polypeptide
MHTGGLLSMDAKEFTGQYPLSKTLRFELRPIGRTWDNLEASGYLAEDRHRAECYPRAKELLDDNHRAFLNRVLPQIDMDWHPIAEAFCKVHKNPGNKELAQDYNLQLSKRRKEISAYLQDADGYKGLFAKPALDEAMKIAKENGNESDIEVLEAFNGFSVYFTGYHESRENIYSDEDMVSVAYRITEDNFPRFVSNALIFDKLNESHPDIISEVSGNLGVDDIGKYFDVSNYNNFLSQAGIDDYNHIIGGHTTEDGLIQAFNVVLNLRHQKDPGFEKIQFKQLYKQILSVRTSKSYIPKQFDNSKEMVDCICDYVSKIEKSETVERALKLVRNISSFDLRGIFVNKKNLRILSNKLIGDWDAIETALMHSSSSENDKKSVYDSAEAFTLDDIFSSVKKFSDASAEDIGNRAEDICRVISETAPFINDLRAVDLDSLNDDGYEAAVSKIRESLEPYMDLFHELEIFSVGDEFPKCAAFYSELEEVSEQLIEIIPLFNKARSFCTRKRYSTDKIKVNLKFPTLADGWDLNKERDNKAAILRKDGKYYLAILDMKKDLSSIRTSDEDESSFEKMEYKLLPSPVKMLPKIFVKSKAAKEKYGLTDRMLECYDKGMHKSGSAFDLGFCHELIDYYKRCIAEYPGWDVFDFKFRETSDYGSMKEFNEDVAGAGYYMSLRKIPCSEVYRLLDEKSIYLFQIYNKDYSENAHGNKNMHTMYWEGLFSPQNLESPVFKLSGGAELFFRKSSIPNDAKTVHPKGSVLVPRNDVNGRRIPDSIYRELTRYFNRGDCRISDEAKSYLDKVKTKKADHDIVKDRRFTVDKMMFHVPIAMNFKAISKPNLNKKVIDGIIDDQDLKIIGIDRGERNLIYVTMVDRKGNILYQDSLNILNGYDYRKALDVREYDNKEARRNWTKVEGIRKMKEGYLSLAVSKLADMIIENNAIIVMEDLNHGFKAGRSKIEKQVYQKFESMLINKLGYMVLKDKSIDQSGGALHGYQLANHVTTLASVGKQCGVIFYIPAAFTSKIDPTTGFADLFALSNVKNVASMREFFSKMKSVIYDKAEGKFAFTFDYLDYNVKSECGRTLWTVYTVGERFTYSRVNREYVRKVPTDIIYDALQKAGISVEGDLRDRIAESDGDTLKSIFYAFKYALDMRVENREEDYIQSPVKNASGEFFCSKNAGKSLPQDSDANGAYNIALKGILQLRMLSEQYDPNAESIRLPLITNKAWLTFMQSGMKTWKN

SEQ ID NO: 6 - protein, 1260 aa, Artificial Sequence
  Description of Artificial Sequence: Synthetic polypeptide
MDSLKDFTNLYPVSKTLRFELKPVGKTLENIEKAGILKEDEHRAESYRRVKKIIDTYHKVFIDSSLENMAKMGIENEIKAMLQSFCELYKKDHRTEGEDKALDKIRAVLRGLIVGAFTGVCGRRENTVQNEKYESLFKEKLIKEILPDFVLSTEAESLPFSVEEATRSLKEFDSFTSYFAGFYENRKNIYSTKPQSTAIAYRLIHENLPKFIDNILVFQKIKEPIAKELEHIRADFSAGGYIKKDERLEDIFSLNYYIHVLSQAGIEKYNALIGKIVTEGDGEMKGLNEHINLYNQQRGREDRLPLFRPLYKQILSDREQLSYLPESFEKDEELLRALKEFYDHIAEDILGRTQQLMTSISEYDLSRIYVRNDSQLTDISKKMLGDWNAIYMARERAYDHEQAPKRITAKYERDRIKALKGEESISLANLNSCIAFLDNVRDCRVDTYLSTLGQKEGPHGLSNLVENVFASYHEAEQLLSFPYPEENNLIQDKDNVVLIKNLLDNISDLQRFLKPLWGMGDEPDKDERFYGEYNYIRGALDQVIPLYNKVRNYLTRKPYSTRKVKLNFGNSQLLSGWDRNKEKDNSCVILRKGQNFYLAIMNNRHKRSFENKVLPEYKEGEPYFEKMDYKFLPDPNKMLPKVFLSKKGIEIYKPSPKLLEQYGHGTHKKGDTFSMDDLHELIDFFKHSIEAHEDWKQFGFKFSDTATYENVSSFYREVEDQGYKLSFRKVSESYVYSLIDQGKLYLFQIYNKDFSPCSKGTPNLHTLYWRMLFDERNLADVIYKLDGKAEIFFREKSLKNDHPTHPAGKPIKKKSRQKKGEESLFEYDLVKDRHYTMDKFQFHVPITMNFKCSAGSKVNDMVNAHIREAKDMHVIGIDRGERNLLYICVIDSRGTILDQISLNTINDIDYHDLLESRDKDRQQERRNWQTIEGIKELKQGYLSQAVHRIAELMVAYKAVVALEDLNMGFKRGRQKVESSVYQQFEKQLIDKLNYLVDKKKRPEDIGGLLRAYQFTAPFKSFKEMGKQNGFLFYIPAWNTSNIDPTTGFVNLFHAQYENVDKAKSFFQKFDSISYNPKKDWFEFAFDYKNFTKKAEGSRSMWILCTHGSRIKNFRNSQKNGQWDSEEFALTEAFKSLFVRYEIDYTADLKTAIVDEKQKDFFVDLLKLFKLTVQMRNSWKEKDLDYLISPVAGADGRFFDTREGNKSLPKDADANGAYNIALKGLWALRQIRQTSEGGKLKLAISNKEWLQFVQERSYEKD

SEQ ID NO: 7 - protein, 1263 aa, Artificial Sequence
  Description of Artificial Sequence: Synthetic polypeptide
MNNGTNNFQNFIGISSLQKTLRNALIPTETTQQFIVKNGIIKEDELRGENRQILKDIMDDYYRGFISETLSSIDDIDWTSLFEKMEIQLKNGDNKDTLIKEQTEYRKAIHKKFANDDRFKNMFSAKLISDILPEFVIHNNNYSASEKEEKTQVIKLFSRFATSFKDYFKNRANCFSADDISSSSCHRIVNDNAEIFFSNALVYRRIVKSLSNDDINKISGDMKDSLKEMSLEEIYSYEKYGEFITQEGISFYNDICGKVNSFMNLYCQKNKENKNLYKLQKLHKQILCIADTSYEVPYKFESDEEVYQSVNGFLDNISSKHIVERLRKIGDNYNGYNLDKIYIVSKFYESVSQKTYRDWETINTALEIHYNNILPGNGKSKADKVKKAVKNDLQKSITEINELVSNYKLCSDDNIKAETYIHEISHILNNFEAQELKYNPEIHLVESELKASELKNVLDVIMNAFHWCSVFMTEELVDKDNNFYAELEEIYDEIYPVISLYNLVRNYVTQKPYSTKKIKLNFGIPTLADGWSKSKEYSNNAIILMRDNLYYLGIFNAKNKPDKKIIEGNTSENKGDYKKMIYNLLPGPNKMIPKVFLSSKTGVETYKPSAYILEGYKQNKHIKSSKDFDITFCHDLIDYFKNCIAIHPEWKNFGFDFSDTSTYEDISGFYREVELQGYKIDWTYISEKDIDLLQEKGQLYLFQIYNKDFSKKSTGNDNLHTMYLKNLFSEENLKDIVLKLNGEAEIFFRKSSIKNPIIHKKGSILVNRTYEAEEKDQFGNIQIVRKNIPENIYQELYKYFNDKSDKELSDEAAKLKNVVGHHEAATNIVKDYRYTYDKYFLHMPITINFKANKTGFINDRILQYIAKEKDLHVIGIDRGERNLIYVSVIDTCGNIVEQKSFNIVNGYDYQIKLKQQEGARQIARKEWKEIGKIKEIKEGYLSLVIHEISKMVIKYNAIIAMEDLSYGFKKGRFKVERQVYQKFETMLINKLNYLVFKDISITENGGLLKGYQLTYIPDKLKNVGHQCGCIFYVPAAYTSKIDPTTGFVNIFKFKDLTVDAKREFIKKFDSIRYDSEKNLFCFTFDYNNFITQNTVMSKSSWSVYTYGVRIKRRFVNGRFSNESDTIDITKDMEKTLEMTDINWRDGHDLRQDIIDYEIVQHIFEIFRLTVQMRNSLSELEDRDYDRLISPVLNENNIFYDSAKAGDALPKDADANGAYCIALKGLYEIKQITENWKEDGKFSRDKLKISNKDWFDFIQNKRYL

SEQ ID NO: 8 - protein, 1318 aa, Artificial Sequence
  Description of Artificial Sequence: Synthetic polypeptide
MTNKFTNQYSLSKTLRFELIPQGKTLEFIQEKGLLSQDKQRAESYQEMKKTIDKFHKYFIDLALSNAKLTHLETYLELYNKSAETKKEQKFKDDLKKVQDNLRKEIVKSFSDGDAKSIFAILDKKELITVELEKWFENNEQKDIYFDEKFKTFTTYFTGFHQNRKNMYSVEPNSTAIAYRLIHENLPKFLENAKAFEKIKQVESLQVNFRELMGEFGDEGLIFVNELEEMFQINYYNDVLSQNGITIYNSIISGFTKNDIKYKGLNEYINNYNQTKDKKDRLPKLKQLYKQILSDRISLSFLPDAFTDGKQVLKAIFDFYKINLLSYTIEGQEESQNLLLLIRQTIENLSSFDTQKIYLKNDTHLTTISQQVFGDFSVFSTALNYWYETKVNPKFETEYSKANEKKREILDKAKAVFTKQDYFSIAFLQEVLSEYILTLDHTSDIVKKHSSNCIADYFKNHFVAKKENETDKTFDFIANITAKYQCIQGILENADQYEDELKQDQKLIDNLKFFLDAILELLHFIKPLHLKSESITEKDTAFYDVFENYYEALSLLTPLYNMVRNYVTQKPYSTEKIKLNFENAQLLNGWDANKEGDYLTTILKKDGNYFLAIMDKKHNKAFQKFPEGKENYEKMVYKLLPGVNKMLPKVFFSNKNIAYFNPSKELLENYKKETHKKGDTFNLEHCHTLIDFFKDSLNKHEDWKYFDFQFSETKSYQDLSGFYREVEHQGYKINFKNIDSEYIDGLVNEGKLFLFQIYSKDFSPFSKGKPNMHTLYWKALFEEQNLQNVIYKLNGQAEIFFRKASIKPKNIILHKKKIKIAKKHFIDKKTKTSEIVPVQTIKNLNMYYQGKISEKELTQDDLRYIDNFSIFNEKNKTIDIIKDKRFTVDKFQFHVPITMNFKATGGSYINQTVLEYLQNNPEVKIIGLDRGERHLVYLTLIDQQGNILKQESLNTITDSKISTPYHKLLDNKENERDLARKNWGTVENIKELKEGYISQVVHKIATLMLEENAIVVMEDLNFGFKRGRFKVEKQIYQKLEKMLIDKLNYLVLKDKQPQELGGLYNALQLTNKFESFQKMGKQSGFLFYVPAWNTSKIDPTTGFVNYFYTKYENVDKAKAFFEKFEAIRFNAEKKYFEFEVKKYSDFNPKAEGTQQAWTICTYGERIETKRQKDQNNKFVSTPINLTEKIEDFLGKNQIVYGDGNCIKSQIASKDDKAFFETLLYWFKMTLQMRNSETRTDIDYLISPVMNDNGTFYNSRDYEKLENPTLPKDADANGAYHIAKKGLMLLNKIDQADLTKKVDLSISNRDWLQFVQKNK

SEQ ID NO: 9 - protein, 1339 aa, Artificial Sequence
  Description of Artificial Sequence: Synthetic polypeptide
MEQEYYLGLDMGTGSVGWAVTDSEYHVLRKHGKALWGVRLFESASTAEERRMFRTSRRRLDRRNWRIEILQEIFAEEISKKDPGFFLRMKESKYYPEDKRDINGNCPELPYALFVDDDFTDKDYHKKFPTIYHLRKMLMNTEETPDIRLVYLAIHHMMKHRGHFLLSGDINEIKEFGTTFSKLLENIKNEELDWNLELGKEEYAVVESILKDNMLNRSTKKTRLIKALKAKSICEKAVLNLLAGGTVKLSDIFGLEELNETERPKISFADNGYDDYIGEVENELGEQFYIIETAKAVYDWAVLVEILGKYTSISEAKVATYEKHKSDLQFLKKIVRKYLTKEEYKDIFVSTSDKLKNYSAYIGMTKINGKKVDLQSKRCSKEEFYDFIKKNVLKKLEGQPEYEYLKEELERETFLPKQVNRDNGVIPYQIHLYELKKILGNLRDKIDLIKENEDKLVQLFEFRIPYYVGPLNKIDDGKEGKFTWAVRKSNEKIYPWNFENVVDIEASAEKFIRRMTNKCTYLMGEDVLPKDSLLYSKYMVLNELNNVKLDGEKLSVELKQRLYTDVFCKYRKVTVKKIKNYLKCEGIISGNVEITGIDGDFKASLTAYHDFKEILTGTELAKKDKENIITNIVLFGDDKKLLKKRLNRLYPQITPNQLKKICALSYTGWGRFSKKFLEEITAPDPETGEVWNIITALWESNNNLMQLLSNEYRFMEEVETYNMGKQTKTLSYETVENMYVSPSVKRQIWQTLKIVKELEKVMKESPKRVFIEMAREKQESKRTESRKKQLIDLYKACKNEEKDWVKELGDQEEQKLRSDKLYLYYTQKGRCMYSGEVIELKDLWDNTKYDIDHIYPQSKTMDDSLNNRVLVKKKYNATKSDKYPLNENIRHERKGFWKSLLDGGFISKEKYERLIRNTELSPEELAGFIERQIVETRQSTKAVAEILKQVFPESEIVYVKAGTVSRFRKDFELLKVREVNDLHHAKDAYLNIVVGNSYYVKFTKNASWFIKENPGRTYNLKKMFTSGWNIERNGEVAWEVGKKGTIVTVKQIMNKNNILVTRQVHEAKGGLFDQQIMKKGKGQIAIKETDERLASIEKYGGYNKAAGAYFMLVESKDKKGKTIRTIEFIPLYLKNKIESDESIALNFLEKGRGLKEPKILLKKIKIDTLFDVDGFKMWLSGRTGDRLLFKCANQLILDEKIIVTMKKIVKFIQRRQENRELKLSDKDGIDNEVLMEIYNTFVDKLENTVYRIRLSEQAKTLIDKQKEFERLSLEDKSSTLFEILHIFQCQSSAANLKMIGGPGKAGILVMNNNISKCNKISIINQSPTGIFENEIDLLK

SEQ ID NO: 10 - protein, 1280 aa, Artificial Sequence
  Description of Artificial Sequence: Synthetic polypeptide
MNKFENFTGLYPISKTLRFELIPQGKTLEYIEKSEILENDNYRAEKYEEVKDIIDGYHKWFINETLHDLHINWSELKVALENNRIEKSDASKKELQRVQKIKREEIYNAFIEHEAFQYLFKENLLSDLLPIQIEQSEDLDAEKKKQAVETFNRFSTYFTGFHENRKNIYSKEGISTSVTYRIVHDNFPKFLENMKVFEILRNECPEVISDTANELAPFIDGVRIEDIFLIDFFNSTFSQNGIDYYNRILGGVTTETGEKYRGINEFTNLYRQQHPEFGKSKKATKMVVLFKQILSDRDTLSFIPEMFGNDKQVQNSIQLFYNREISQFENEGVKTDVCTALATLTSKIAEFDTEKIYIQQPELPNVSQRLFGSWNELNACLFKYAELKFGTAEKVANRKKIDKWLKSDLFSFTELNKALEFSGKDERIENYFSETGIFAQLVKTGFDEAQSILETEYTSEVHLKDQQTDIEKIKTFLDALQNLMHLLKSLCVSEEADRDAAFYNEFDMLYNQLKLVVPLYNKVRNYITQKLFRSDKIKIYFENKGQFLGGWVDSQTENSDNGTQAGGYIFRKENVINEYDYYLGICSDPKLFRRTTIVSENDRSSFERLDYYQLKTASVYGNSYCGKHPYTEDKNELVNSIDRFVHLSGNNILIEKIAKDKVKSNPTTNTPSGYLNFIHREAPNTYECLLQDENFVSLNQRVVSALKATLATLVRVPKALVYAKKDYHLFSEIINDIDELSYEKAFSYFPVSQTEFENSSNRTIKPLLLFKISNKDLSFAENFEKGNRQKIGKKNLHTLYFEALMKGNQDTIDIGTGMVFHRVKSLNYNEKTLKYGHHSTQLNEKFSYPIIKDKRFASDKFLFHLSTEINYKEKRKPLNNSIIEFLTNNPDINIIGLDRGERHLIYLTLINQKGEILRQKTFNIVGNTNYHEKLNQREKERDNARKSWATIGKIKELKEGFLSLVIHEIAKIMVENNAIVVLEDLNFGFKRGRFKVEKQIYQKFEKMLIDKLNYLVFKDKKANEAGGVLKGYQLAEKFESFQKMGKQSGFLFYVPAAYTSKIDPTTGFVNMLNLNYTNMKDAQTLLSGMDKISFNADANYFEFELDYEKFKTNQTDHTNKWTICTVGEKRFTYNSATKETTTVNVTEDLKKLLDKFEVKYSNGDNIKDEICRQTDAKFFEIILWLLKLTMQMRNSNTKTEEDFILSPVKNSNGEFFRSNDDANGIWPADADANGAYHIALKGLYLVKECFNKNEKSLKIEHKNWFKFAQTRFNGSLTKNG

SEQ ID NO: 11 - protein, 1154 aa, Artificial Sequence
  Description of Artificial Sequence: Synthetic polypeptide
MENFKNLYPINKTLRFELRPYGKTLENFKKSGLLEKDAFKANSRRSMQAIIDEKFKETIEERLKYTEFSECDLGNMTSKDKKITDKAATNLKKQVILSFDDEIFNNYLKPDKNIDALFKNDPSNPVISTFKGFTTYFVNFFEIRKHIFKGESSGSMAYRIIDENLTTYLNNIEKIKKLPEELKSQLEGIDQIDKLNNYNEFITQSGITHYNEIIGGISKSENVKIQGINEGINLYCQKNKVKLPRLTPLYKMILSDRVSNSFVLDTIENDTELIEMISDLINKTEISQDVIMSDIQNIFIKYKQLGNLPGISYSSIVNAICSDYDNNFGDGKRKKSYENDRKKHLETNVYSINYISELLTDTDVSSNIKMRYKELEQNYQVCKENFNATNWMNIKNIKQSEKTNLIKDLLDILKSIQRFYDLFDIVDEDKNPSAEFYTWLSKNAEKLDFEFNSVYNKSRNYLTRKQYSDKKIKLNFDSPTLAKGWDANKEIDNSTIIMRKFNNDRGDYDYFLGIWNKSTPANEKIIPLEDNGLFEKMQYKLYPDPSKMLPKQFLSKIWKAKHPTTPEFDKKYKEGRHKKGPDFEKEFLHELIDCFKHGLVNHDEKYQDVFGFNLRNTEDYNSYTEFLEDVERCNYNLSFNKIADTSNLINDGKLYVFQIWSKDFSIDSKGTKNLNTIYFESLFSEENMIEKMFKLSGEAEIFYRPASLNYCEDIIKKGHHHAELKDKFDYPIIKDKRYSQDKFFFHVPMVINYKSEKLNSKSLNNRTNENLGQFTHIIGIDRGERHLIYLTVVDVSTGEIVEQKHLDEIINTDTKGVEHKTHYLNKLEEKSKTRDNERKSWEAIETIKELKEGYISHVINEIQKLQEKYNALIVMENLNYGFKNSRIKVEKQVYQKFETALIKKFNYIIDKKDPETYIHGYQLTNPITTLDKIGNQSGIVLYIPAWNTSKIDPVTGFVNLLYADDLKYKNQEQAKSFIQKIDNIYFENGEFKFDIDFSKWNNRYSISKTKWTLTSYGTRIQTFRNPQKNNKWDSAEYDLTEEFKLILNIDGTLKSQDVETYKKFMSLFKLMLQLRNSVTGTDIDYMISPVTDKTGTHFDSRENIKNLPADADANGAYNIARKGIMAIENIMNGISDPLKISNEDYLKYIQNQQE

SEQ ID NO: 12 - protein, 1307 aa, Artificial Sequence
  Description of Artificial Sequence: Synthetic polypeptide
MTQFEGFTNLYQVSKTLRFELIPQGKTLKHIQEQGFIEEDKARNDHYKELKPIIDRIYKTYADQCLQLVQLDWENLSAAIDSYRKEKTEETRNALIEEQATYRNAIHDYFIGRTDNLTDAINKRHAEIYKGLFKAELFNGKVLKQLGTVTTTEHENALLRSFDKFTTYFSGFYENRKNVFSAEDISTAIPHRIVQDNFPKFKENCHIFTRLITAVPSLREHFENVKKAIGIFVSTSIEEVFSFPFYNQLLTQTQIDLYNQLLGGISREAGTEKIKGLNEVLNLAIQKNDETAHIIASLPHRFIPLFKQILSDRNTLSFILEEFKSDEEVIQSFCKYKTLLRNENVLETAEALFNELNSIDLTHIFISHKKLETISSALCDHWDTLRNALYERRISELTGKITKSAKEKVQRSLKHEDINLQEIISAAGKELSEAFKQKTSEILSHAHAALDQPLPTTLKKQEEKEILKSQLDSLLGLYHLLDWFAVDESNEVDPEFSARLTGIKLEMEPSLSFYNKARNYATKKPYSVEKFKLNFQMPTLASGWDVNKEKNNGAILFVKNGLYYLGIMPKQKGRYKALSFEPTEKTSEGFDKMYYDYFPDAAKMIPKCSTQLKAVTAHFQTHTTPILLSNNFIEPLEITKEIYDLNNPEKEPKKFQTAYAKKTGDQKGYREALCKWIDFTRDFLSKYTKTTSIDLSSLRPSSQYKDLGEYYAELNPLLYHISFQRIAEKEIMDAVETGKLYLFQIYNKDFAKGHHGKPNLHTLYWTGLFSPENLAKTSIKLNGQAELFYRPKSRMKRMAHRLGEKMLNKKLKDQKTPIPDTLYQELYDYVNHRLSHDLSDEARALLPNVITKEVSHEIIKDRRFTSDKFFFHVPITLNYQAANSPSKFNQRVNAYLKEHPETPIIGIDRGERNLIYITVIDSTGKILEQRSLNTIQQFDYQKKLDNREKERVAARQAWSVVGTIKDLKQGYLSQVIHEIVDLMIHYQAVVVLENLNFGFKSKRTGIAEKAVYQQFEKMLIDKLNCLVLKDYPAEKVGGVLNPYQLTDQFTSFAKMGTQSGFLFYVPAPYTSKIDPLTGFVDPFVWKTIKNHESRKHFLEGFDFLHYDVKTGDFILHFKMNRNLSFQRGLPGFMPAWDIVFEKNETQFDAKGTPFIAGKRIVPVIENHRFTGRYRDLYPANELIALLEEKGIVFRDGSNILPKLLENDDSHAIDTMVALIRSVLQMRNSNAATGEDYINSPVRDLNGVCFDSRFQNPEWPMDADANGAYHIALKGQLLLNHLKESKDLKLQNGISNQDWLAYIQELRN

SEQ ID NO: 13 - protein, 1129 aa, Artificial Sequence
  Description of Artificial Sequence: Synthetic polypeptide
MAVKSIKVKLRLDDMPEIRAGLWKLHKEVNAGVRYYTEWLSLLRQENLYRRSPNGDGEQECDKTAEECKAELLERLRARQVENGHRGPAGSDDELLQLARQLYELLVPQAIGAKGDAQQIARKFLSPLADKDAVGGLGIAKAGNKPRWVRMREAGEPGWEEEKEKAETRKSADRTADVLRALADFGLKPLMRVYTDSEMSSVEWKPLRKGQAVRTWDRDMFQQAIERMMSWESWNQRVGQEYAKLVEQKNRFEQKNFVGQEHLVHLVNQLQQDMKEASPGLESKEQTAHYVTGRALRGSDKVFEKWGKLAPDAPFDLYDAEIKNVQRRNTRRFGSHDLFAKLAEPEYQALWREDASFLTRYAVYNSILRKLNHAKMFATFTLPDATAHPIWTRFDKLGGNLHQYTFLFNEFGERRHAIRFHKLLKVENGVAREVDDVTVPISMSEQLDNLLPRDPNEPIALYFRDYGAEQHFTGEFGGAKIQCRRDQLAHMHRRRGARDVYLNVSVRVQSQSEARGERRPPYAAVFRLVGDNHRAFVHFDKLSDYLAEHPDDGKLGSEGLLSGLRVMSVDLGLRTSASISVFRVARKDELKPNSKGRVPFFFPIKGNDNLVAVHERSQLLKLPGETESKDLRAIREERQRTLRQLRTQLAYLRLLVRCGSEDVGRRERSWAKLIEQPVDAANHMTPDWREAFENELQKLKSLHGICSDKEWMDAVYESVRRVWRHMGKQVRDWRKDVRSGERPKIRGYAKDVVGGNSIEQIEYLERQYKFLKSWSFFGKVSGQVIRAEKGSRFAITLREHIDHAKEDRLKKLADRIIMEALGYVYALDERGKGKWVAKYPPCQLILLEELSEYQFNNDRPPSENNQLMQWSHRGVFQELINQAQVHDLLVGTMYAAFSSRFDARTGAPGIRCRRVPARCTQEHNPEPFPWWLNKFVVEHTLDACPLRADDLIPTGEGEIFVSPFSAEEGDFHQIHADLNAAQNLQQRLWSDFDISQIRLRCDWGEVDGELVLIPRLTGKRTADSYSNKVFYTNTGVTYYERERGKKRRKVFAQEKLSEEEAELLVEADEAREKSVVLMRDPSGIINRGNWTRQKEFWSMVNQRIEGYLVKQIRSRVPLQDSACENTGDI

SEQ ID NO: 14 - protein, 1108 aa, Artificial Sequence
  Description of Artificial Sequence: Synthetic polypeptide
MATRSFILKIEPNEEVKKGLWKTHEVLNHGIAYYMNILKLIRQEAIYEHHEQDPKNPKKVSKAEIQAELWDFVLKMQKCNSFTHEVDKDVVFNILRELYEELVPSSVEKKGEANQLSNKFLYPLVDPNSQSGKGTASSGRKPRWYNLKIAGDPSWEEEKKKWEEDKKKDPLAKILGKLAEYGLIPLFIPFTDSNEPIVKEIKWMEKSRNQSVRRLDKDMFIQALERFLSWESWNLKVKEEYEKVEKEHKTLEERIKEDIQAFKSLEQYEKERQEQLLRDTLNTNEYRLSKRGLRGWREIIQKWLKMDENEPSEKYLEVFKDYQRKHPREAGDYSVYEFLSKKENHFIWRNHPEYPYLYATFCEIDKKKKDAKQQATFTLADPINHPLWVRFEERSGSNLNKYRILTEQLHTEKLKKKLTVQLDRLIYPTESGGWEEKGKVDIVLLPSRQFYNQIFLDIEEKGKHAFTYKDESIKFPLKGTLGGARVQFDRDHLRRYPHKVESGNVGRIYFNMTVNIEPTESPVSKSLKIHRDDFPKFVNFKPKELTEWIKDSKGKKLKSGIESLEIGLRVMSIDLGQRQAAAASIFEVVDQKPDIEGKLFFPIKGTELYAVHRASFNIKLPGETLVKSREVLRKAREDNLKLMNQKLNFLRNVLHFQQFEDITEREKRVTKWISRQENSDVPLVYQDELIQIRELMYKPYKDWVAFLKQLHKRLEVEIGKEVKHWRKSLSDGRKGLYGISLKNIDEIDRTRKFLLRWSLRPTEPGEVRRLEPGQRFAIDQLNHLNALKEDRLKKMANTIIMHALGYCYDVRKKKWQAKNPACQIILFEDLSNYNPYEERSRFENSKLMKWSRREIPRQVALQGEIYGLQVGEVGAQFSSRFHAKTGSPGIRCSVVTKEKLQDNRFFKNLQREGRLTLDKIAVLKEGDLYPDKGGEKFISLSKDRKLVTTHADINAAQNLQKRFWTRTHGFYKVYCKAYQVDGQTVYIPESKDQKQKIIEEFGEGYFILKDGVYEWGNAGKLKIKKGSSKQSSSELVDSDILKDSFDLASELKGEKLMLYRDPSGNVFPSDKWMAAGVFFGKLERILISKLTNQYSISTIEDDSSKQSM

SEQ ID NO: 15 - protein, 1149 aa, Artificial Sequence
  Description of Artificial Sequence: Synthetic polypeptide
MPTRTINLKLVLGKNPENATLRRALFSTHRLVNQATKRIEEFLLLCRGEAYRTVDNEGKEAEIPRHAVQEEALAFAKAAQRHNGCISTYEDQEILDVLRQLYERLVPSVNENNEAGDAQAANAWVSPLMSAESEGGLSVYDKVLDPPPVWMKLKEEKAPGWEAASQIWIQSDEGQSLLNKPGSPPRWIRKLRSGQPWQDDFVSDQKKKQDELTKGNAPLIKQLKEMGLLPLVNPFFRHLLDPEGKGVSPWDRLAVRAAVAHFISWESWNHRTRAEYNSLKLRRDEFEAASDEFKDDFTLLRQYEAKRHSTLKSIALADDSNPYRIGVRSLRAWNRVREEWIDKGATEEQRVTILSKLQTQLRGKFGDPDLFNWLAQDRHVHLWSPRDSVTPLVRINAVDKVLRRRKPYALMTFAHPRFHPRWILYEAPGGSNLRQYALDCTENALHITLPLLVDDAHGTWIEKKIRVPLAPSGQIQDLTLEKLEKKKNRLYYRSGFQQFAGLAGGAEVLFHRPYMEHDERSEESLLERPGAVWFKLTLDVATQAPPNWLDGKGRVRTPPEVHHFKTALSNKSKHTRTLQPGLRVLSVDLGMRTFASCSVFELIEGKPETGRAFPVADERSMDSPNKLWAKHERSFKLTLPGETPSRKEEEERSIARAEIYALKRDIQRLKSLLRLGEEDNDNRRDALLEQFFKGWGEEDVVPGQAFPRSLFQGLGAAPFRSTPELWRQHCQTYYDKAEACLAKHISDWRKRTRPRPTSREMWYKTRSYHGGKSIWMLEYLDAVRKLLLSWSLRGRTYGAINRQDTARFGSLASRLLHHINSLKEDRIKTGADSIVQAARGYIPLPHGKGWEQRYEPCQLILFEDLARYRFRVDRPRRENSQLMQWNHRAIVAETTMQAELYGQIVENTAAGFSSRFHAATGAPGVRCRFLLERDFDNDLPKPYLLRELSWMLGNTKVESEEEKLRLLSEKIRPGSLVPWDGGEQFATLHPKRQTLCVIHADMNAAQNLQRRFFGRCGEAFRLVCQPHGDDVLRLASTPGARLLGALQQLENGQGAFELVRDMGSTSQMNRFVMKSLGKKKIKPLQDNNGDDELEDVLSVLPEEDDTGRITVFRDSSGIFFPCNVWIPAKQFWPAVRAMIWKVMASHSLG

SEQ ID NO: 16 - protein, 1252 aa, Artificial Sequence
  Description of Artificial Sequence: Synthetic polypeptide
MTKLRHRQKKLTHDWAGSKKREVLGSNGKLQNPLLMPVKKGQVTEFRKAFSAYARATKGEMTDGRKNMFTHSFEPFKTKPSLHQCELADKAYQSLHSYLPGSLAHFLLSAHALGFRIFSKSGEATAFQASSKIEAYESKLASELACVDLSIQNLTISTLFNALTTSVRGKGEETSADPLIARFYTLLTGKPLSRDTQGPERDLAEVISRKIASSFGTWKEMTANPLQSLQFFEEELHALDANVSLSPAFDVLIKMNDLQGDLKNRTIVFDPDAPVFEYNAEDPADIIIKLTARYAKEAVIKNQNVGNYVKNAITTTNANGLGWLLNKGLSLLPVSTDDELLEFIGVERSHPSCHALIELIAQLEAPELFEKNVFSDTRSEVQGMIDSAVSNHIARLSSSRNSLSMDSEELERLIKSFQIHTPHCSLFIGAQSLSQQLESLPEALQSGVNSADILLGSTQYMLTNSLVEESIATYQRTLNRINYLSGVAGQINGAIKRKAIDGEKIHLPAAWSELISLPFIGQPVIDVESDLAHLKNQYQTLSNEFDTLISALQKNFDLNFNKALLNRTQHFEAMCRSTKKNALSKPEIVSYRDLLARLTSCLYRGSLVLRRAGIEVLKKHKIFESNSELREHVHERKHFVFVSPLDRKAKKLLRLTDSRPDLLHVIDEILQHDNLENKDRESLWLVRSGYLLAGLPDQLSSSFINLPIITQKGDRRLIDLIQYDQINRDAFVMLVTSAFKSNLSGLQYRANKQSFVVTRTLSPYLGSKLVYVPKDKDWLVPSQMFEGRFADILQSDYMVWKDAGRLCVIDTAKHLSNIKKSVFSSEEVLAFLRELPHRTFIQTEVRGLGVNVDGIAFNNGDIPSLKTFSNCVQVKVSRTNTSLVQTLNRWFEGGKVSPPSIQFERAYYKKDDQIHEDAAKRKIRFQMPATELVHASDDAGWTPSYLLGIDPGEYGMGLSLVSINNGEVLDSGFIHINSLINFASKKSNHQTKVVPRQQYKSPYANYLEQSKDSAAGDIAHILDRLIYKLNALPVFEALSGNSQSAADQVWTKVLSFYTWGDNDAQNSIRKQHWFGASHWDIKGMLRQPPTEKKPKPYIAFPGSQVSSYGNSQRCSCCGRNPIEQLREMAKDTSIKELKIRNSEIQLFDGTIKLFNPDPSTVIERRRHNLGPSRIPVADRTFKNISPSSLEFKELITIVSRSIRHSPEFIAKKRGIGSEYFCAYSDCNSSLNSEANAAANVAQKFQKQLFFEL

SEQ ID NO: 17 - protein, 1287 aa, Artificial Sequence
  Description of Artificial Sequence: Synthetic polypeptide
MKRILNSLKVAALRLLFRGKGSELVKTVKYPLVSPVQGAVEELAEAIRHDNLHLFGQKEIVDLMEKDEGTQVYSVVDFWLDTLRLGMFFSPSANALKITLGKFNSDQVSPFRKVLEQSPFFLAGRLKVEPAERILSVEIRKIGKRENRVENYAADVETCFIGQLSSDEKQSIQKLANDIWDSKDHEEQRMLKADFFAIPLIKDPKAVTEEDPENETAGKQKPLELCVCLVPELYTRGFGSIADFLVQRLTLLRDKMSTDTAEDCLEYVGIEEEKGNGMNSLLGTFLKNLQGDGFEQIFQFMLGSYVGWQGKEDVLRERLDLLAEKVKRLPKPKFAGEWSGHRMFLHGQLKSWSSNFFRLFNETRELLESIKSDIQHATMLISYVEEKGGYHPQLLSQYRKLMEQLPALRTKVLDPEIEMTHMSEAVRSYIMIHKSVAGFLPDLLESLDRDKDREFLLSIFPRIPKIDKKTKEIVAWELPGEPEEGYLFTANNLFRNFLENPKHVPRFMAERIPEDWTRLRSAPVWFDGMVKQWQKVVNQLVESPGALYQFNESFLRQRLQAMLTVYKRDLQTEKFLKLLADVCRPLVDFFGLGGNDIIFKSCQDPRKQWQTVIPLSVPADVYTACEGLAIRLRETLGFEWKNLKGHEREDFLRLHQLLGNLLFWIRDAKLVVKLEDWMNNPCVQEYVEARKAIDLPLEIFGFEVPIFLNGYLFSELRQLELLLRRKSVMTSYSVKTTGSPNRLFQLVYLPLNPSDPEKKNSNNFQERLDTPTGLSRRFLDLTLDAFAGKLLTDPVTQELKTMAGFYDHLFGFKLPCKLAAMSNHPGSSSKMVVLAKPKKGVASNIGFEPIPDPAHPVFRVRSSWPELKYLEGLLYLPEDTPLTIELAETSVSCQSVSSVAFDLKNLTTILGRVGEFRVTADQPFKLTPIIPEKEESFIGKTYLGLDAGERSGVGFAIVTVDGDGYEVQRLGVHEDTQLMALQQVASKSLKEPVFQPLRKGTFRQQERIRKSLRGCYWNFYHALMIKYRAKVVHEESVGSSGLVGQWLRAFQKDLKKADVLPKKGGKNGVDKKKRESSAQDTLWGGAFSKKEEQQIAFEVQAAGSSQFCLKCGWWFQLGMREVNRVQESGVVLDWNRSIVTFLIESSGEKVYGFSPQQLEKGFRPDIETFKKMVRDFMRPPMFDRKGRPAAAYERFVLGRRHRRYRFDKVFEERFGRSALFICPRVGCGNFDHSSEQSAVVLALIGYIADKEGMSGKKLVYVRLAELMAEWKLKKLERSRVEEQSSAQ

SEQ ID NO: 18 - protein, 1192 aa, Artificial Sequence
  Description of Artificial Sequence: Synthetic polypeptide
MAESKQMQCRKCGASMKYEVIGLGKKSCRYMCPDCGNHTSARKIQNKKKRDKKYGSASKAQSQRIAVAGALYPDKKVQTIKTYKYPADLNGEVHDSGVAEKIAQAIQEDEIGLLGPSSEYACWIASQKQSEPYSVVDFWFDAVCAGGVFAYSGARLLSTVLQLSGEESVLRAALASSPFVDDINLAQAEKFLAVSRRTGQDKLGKRIGECFAEGRLEALGIKDRMREFVQAIDVAQTAGQRFAAKLKIFGISQMPEAKQWNNDSGLTVCILPDYYVPEENRADQLVVLLRRLREIAYCMGIEDEAGFEHLGIDPGALSNFSNGNPKRGFLGRLLNNDIIALANNMSAMTPYWEGRKGELIERLAWLKHRAEGLYLKEPHFGNSWADHRSRIFSRIAGWLSGCAGKLKIAKDQISGVRTDLFLLKRLLDAVPQSAPSPDFIASISALDRFLEAAESSQDPAEQVRALYAFHLNAPAVRSIANKAVQRSDSQEWLIKELDAVDHLEFNKAFPFFSDTGKKKKKGANSNGAPSEEEYTETESIQQPEDAEQEVNGQEGNGASKNQKKFQRIPRFFGEGSRSEYRILTEAPQYFDMFCNNMRAIFMQLESQPRKAPRDFKCFLQNRLQKLYKQTFLNARSNKCRALLESVLISWGEFYTYGANEKKFRLRHEASERSSDPDYVVQQALEIARRLFLFGFEWRDCSAGERVDLVEIHKKAISFLLAITQAEVSVGSYNWLGNSTVSRYLSVAGTDTLYGTQLEEFLNATVLSQMRGLAIRLSSQELKDGFDVQLESSCQDNLQHLLVYRASRDLAACKRATCPAELDPKILVLPVGAFIASVMKMIERGDEPLAGAYLRHRPHSFGWQIRVRGVAEVGMDQGTALAFQKPTESEPFKIKPFSAQYGPVLWLNSSSYSQSQYLDGFLSQPKNWSMRVLPQAGSVRVEQRVALIWNLQAGKMRLERSGARAFFMPVPFSFRPSGSGDEAVLAPNRYLGLFPHSGGIEYAVVDVLDSAGFKILERGTIAVNGFSQKRGERQEEAHREKQRRGISDIGRKKPVQAEVDAANELHRKYTDVATRLGCRIVVQWAPQPKPGTAPTAQTVYARAVRTEAPRSGNQEDHARMKSSWGYTWGTYWEKRKPEDILGISTQVYWTGGIGESCPAVAVALLGHIRATSTQTEWEKEEVVFGRLKKFFPS

SEQ ID NO: 19 - protein, 986 aa, Artificial Sequence
  Description of Artificial Sequence: Synthetic polypeptide
MEKRINKIRKKLSADNATKPVSRSGPMKTLLVRVMTDDLKKRLEKRRKKPEVMPQVISNNAANNLRMLLDDYTKMKEAILQVYWQEFKDDHVGLMCKFAQPASKKIDQNKLKPEMDEKGNLTTAGFACSQCGQPLFVYKLEQVSEKGKAYTNYFGRCNVAEHEKLILLAQLKPEKDSDEAVTYSLGKFGQRALDFYSIHVTKESTHPVKPLAQIAGNRYASGPVGKALSDACMGTIASFLSKYQDIIIEHQKVVKGNQKRLESLRELAGKENLEYPSVTLPPQPHTKEGVDAYNEVIARVRMWVNLNLWQKLKLSRDDAKPLLRLKGFPSFPVVERRENEVDWWNTINEVKKLIDAKRDMGRVFWSGVTAEKRNTILEGYNYLPNENDHKKREGSLENPKKPAKRQFGDLLLYLEKKYAGDWGKVFDEAWERIDKKIAGLTSHIEREEARNAEDAQSKAVLTDWLRAKASFVLERLKEMDEKEFYACEIQLQKWYGDLRGNPFAVEAENRVVDISGFSIGSDGHSIQYRNLLAWKYLENGKREFYLLMNYGKKGRIRFTDGTDIKKSGKWQGLLYGGGKAKVIDLTFDPDDEQLIILPLAFGTRQGREFIWNDLLSLETGLIKLANGRVIEKTIYNKKIGRDEPALFVALTFERREVVDPSNIKPVNLIGVDRGENIPAVIALTDPEGCPLPEFKDSSGGPTDILRIGEGYKEKQRAIQAAKEVEQRRAGGYSRKFASKSRNLADDMVRNSARDLFYHAVTHDAVLVFENLSRGFGRQGKRTFMTERQYTKMEDWLTAKLAYEGLTSKTYLSKTLAQYTSKTCSNCGFTITTADYDGMLVRLKKTSDGWATTLNNKELKAEGQITYYNRYKRQTVEKELSAELDRLSEESGNNDISKWTKGRRDEALFLLKKRFSHRPVQEQFVCLDCGHEVHADEQAALNIARSWLFLNSNSTEFKSYKSGKQPFVGAWQAFYKRRLKEVWKPNA

SEQ ID NO: 20 - protein, 973 aa, Artificial Sequence
  Description of Artificial Sequence: Synthetic polypeptide
MKRINKIRRRLVKDSNTKKAGKTGPMKTLLVRVMTPDLRERLENLRKKPENIPQPISNTSRANLNKLLTDYTEMKKAILHVYWEEFQKDPVGLMSRVAQPAPKNIDQRKLIPVKDGNERLTSSGFACSQCCQPLYVYKLEQVNDKGKPHTNYFGRCNVSEHERLILLSPHKPEANDELVTYSLGKFGQRALDFYSIHVTRESNHPVKPLEQIGGNSCASGPVGKALSDACMGAVASFLTKYQDIILEHQKVIKKNEKRLANLKDIASANGLAFPKITLPPQPHTKEGIEAYNNVVAQIVIWVNLNLWQKLKIGRDEAKPLQRLKGFPSFPLVERQANEVDWWDMVCNVKKLINEKKEDGKVFWQNLAGYKRQEALLPYLSSEEDRKKGKKFARYQFGDLLLHLEKKHGEDWGKVYDEAWERIDKKVEGLSKHIKLEEERRSEDAQSKAALTDWLRAKASFVIEGLKEADKDEFCRCELKLQKWYGDLRGKPFAIEAENSILDISGFSKQYNCAFIWQKDGVKKLNLYLIINYFKGGKLRFKKIKPEAFEANRFYTVINKKSGEIVPMEVNFNFDDPNLIILPLAFGKRQGREFIWNDLLSLETGSLKLANGRVIEKTLYNRRTRQDEPALFVALTFERREVLDSSNIKPMNLIGIDRGENIPAVIALTDPEGCPLSRFKDSLGNPTHILRIGESYKEKQRTIQAAKEVEQRRAGGYSRKYASKAKNLADDMVRNTARDLLYYAVTQDAMLIFENLSRGFGRQGKRTFMAERQYTRMEDWLTAKLAYEGLPSKTYLSKTLAQYTSKTCSNCGFTITSADYDRVLEKLKKTATGWMTTINGKELKVEGQITYYNRYKRQNVVKDLSVELDRLSEESVNNDISSWTKGRSGEALSLLKKRFSHRPVQEKFVCLNCGFETHADEQAALNIARSWLFLRSQEYKKYQTNKTTGNTDKRAFVETWQSFYRKKLKEVWKP

SEQ ID NO: 21 - DNA, 4077 bp, Artificial Sequence
  Description of Artificial Sequence: Synthetic polynucleotide
atgggaaaaatgtattatcttggtctggatataggaacaaattctgttggatatgccgtaaccgacccatcgtaccatttgctcaaatttaaaggcgaaccgatgtggggtgcccacgtgtttgctgcggggaatcaatcagctgaacggagaagctttcgtacgagccgcagacgccttgaccgcaggcaacagcgtgtcaaactggttcaagaaatctttgctcccgtgattagtcccattgatccacgtttttttatcagacttcatgagagcgctttatggcgggatgatgtggctgaaacggataaacatattttctttaatgacccgacctatacggataaggaatattattctgactatccaaccatccatcatctcattgtggaccttatggaaagcagtgaaaagcatgacccgcggcttgtttatttggctgttgcctggctggttgctcatcgtggtcatttcctcaatgaagtggataaggataatattggggatgtcctgagttttgacgccttttatcctgagtttctggcatttctttccgataatggggtgtcaccttgggtatgtgagtcaaaagcactccaagcgaccctgctttcacgaaactccgtcaacgataagtataaagccttgaagtctctgatctttggcagccaaaagccggaggataattttgatgccaatatcagtgaagatggacttatccaacttttagcaggaaaaaaggtcaaggtcaataaactttttcctcaagaaagtaatgatgcttcctttacactcaatgataaggaagatgcaattgaggaaatcttaggaacgcttacaccggatgagtgtgaatggattgcgcatattaggaggctgtttgattgggccatcatgaaacatgctctcaaagatggcagaacaatctccgaatcgaaagtaaagctctatgaacagcatcaccatgacttgacacagctcaagtattttgtgaagacctatctagcaaaggaatatgatgacatttttcgaaacgtagatagtgaaacaaccaaaaactatgtcgcatattcctatcatgtaaaagaagtcaagggtacattgcccaaaaataaggcaacccaagaagaattttgcaagtatgtccttggaaaggtaaagaacatcgaatgcagtgaagctgataaggttgattttgatgaaatgattcagcgtcttacagacaattcctttatgccgaaacaagtatcaggtgaaaacagggttatcccttaccagctttactattatgaactaaagactattttgaataaagccgcttcttatctgccttttttgacccaatgcggaaaagatgccatctccaatcaagataagctcctttccatcatgacctttcggattccgtatttcgttgggcccttgcgcaaggacaattcagagcatgcctggctggaacgaaaagcagggaaaatctatccgtggaattttaacgacaaagttgaccttgataaaagtgaagaagcgttcattcggagaatgacgaatacctgcacttattatcccggtgaagatgttttgccacttgactcccttatttatgaaaaattcatgatcctcaatgaaatcaataatatccgaattgatggttatcctatttctgtagatgtaaaacagcaggtttttggcctctttgaaaagaagagaagagtgaccgtaaaggatatccagaatctcctgctttccttgggtgccttggataagcatggtaaattgacgggaatcgatactaccatccatagcaattacaatacataccatcattttaaatcgctcatggagcgtggcgttcttactcgtgatgatgtggaacgcattgtggagcgtatgacctatagtgatgatacaaaacgcgtccgtctttggctgaacaataattatggaacgctcactgctgacgacgtaaagcatatttcaaggctccgaaagcatgattttggccggctttccaaaatgttcctcacaggcctaaagggagttcataaggaaacgggggaacgagcttccattttggattttatgtggaataccaatgataacttgatgcagcttttatctgaatgttatactttttcggatgaaattaccaagctgcaggaagcatactatgccaaggcgcagctttccctgaatgattttctggactccatgtatatttcaaatgctgtcaaacgtcctatctatcgaactcttgccgttgtaaatgacatacgcaaagcctgtgggacggcgccaaaacgcatttttatcgaaatggcaagagatggggaaagcaaaaagaaaaggagcgtaacaagaagagaacaaatcaagaatctttataggtccatccgcaaggattttcagcaggaggtagatttccttgaaaaaatccttgaaaacaaaagcgatggacagctgcaaagcgatgcgctctatctatactttgcgcagcttggaagggatatgtataccggggaccctatcaagttggagcatatcaaggaccagtccttctataatattgatcatatctatccccaaagcatggtcaaggacgatagtcttgataacaaggtgttggttcaatcggaaattaatggagagaagagcagtcgatatcctcttgatgctgctatccgtaataaaatgaagcctctttgggatgcttattataaccatggcctgatttccctcaagaagtatcagcgtttgacgcggagcactccctttacagatgatgaaaagtgggatttcatcaatcggcagcttgttgagacaagacaatccacgaaggccttggcaatcttactaaaaaggaagttccctgatacggagattgtctactccaaggcagggctttcttctgattttcggcatgagtttggtctcgtaaaatcgaggaatatcaatgacctgcaccatgcaaaggacgcatttcttgcgattgtaacaggaaatgtctatcatgaacgctttaatcgccggtggtttatggtgaaccagccctattccgtcaagaccaagacgttgtttacgcattctattaaaaatggtaattttgtagcttggaatggagaagaggatcttggccgcattgttaaaatgttaaagcaaaataagaacactattcatttcacgcggttctcttttgatcgaaaggaaggcctgtttgatattcagccactaaaagcgtcaaccggtcttgtaccaagaaaagccggactagacgtggtaaaatatggtggctatgacaaatcgacagcagcttattatctccttgttcgatttacactagaagataaaaagactcaacataaattgatgatgattcctgtagaaggcttgtataaagctcgaattgaccatgataaggaattcttaacggactatgcacaaactacaatcagtgaaatcctacaaaaagataaacaaaaggtgataaatataatgtttccaatgggaacaaggcacattaaactgaattccatgatttcaatcgatggtttttatctttccattggaggaaagtctagtaagggaaaatcggtgttgtgtcatgctatggtacctcttattgtacctcataagatagaatgttatattaaggcgatggagtcttttgcacgtaaatttaaagaaaataataaattaaggattgtggaaaagtttgataagattacggtggaagataacttgaacctatacgaactatttttacaaaaacttcaacataacccatataataagttcttctccacacaatttgatgtgctgactaatggaagaagtacatttactaaattatctccagaggaacaagttcaaacgttattgaatatcttatcaatttttaaaacttgtcggagctctggctgcgatttaaaatccattaacggttctgctcaagctgccagaattatgatcagcgcagatttaactggactctcaaaaaaatattccgatattcggcttgttgagcaatcagcatctggactttttgttagtaaatcacaaaatcttttggagtatttatga

SEQ ID NO: 22 - DNA, 4005 bp, Artificial Sequence
  Description of Artificial Sequence: Synthetic polynucleotide
atgtcttcattaacaaaatttacaaataaatacagtaagcagctaaccataaaaaatgaactcatcccagtaggaaagactctcgagaacattaaggaaaacggtctcatagatggagatgaacagctaaacgagaattatcaaaaagcaaagataatcgttgatgattttctacgagatttcataaataaagctttaaataatacccaaataggaaattggagagaattagcagatgctttaaataaagaagatgaagataacatagaaaagctccaagacaaaatcagaggaataattgtaagtaaattcgagacatttgatttgttttcttcttactcgataaagaaagacgaaaagataatagatgatgataatgatgttgaagaagaggagctagatctaggaaaaaaaacttcctcatttaaatatatttttaagaaaaacctttttaaattagtacttccttcttatttaaagacaacaaatcaggataaactgaaaataatctcttcttttgataatttttctacctatttcagaggattctttgagaacagaaaaaatattttcactaagaagcctatatctacgtcaattgcctacagaattgtccatgataactttccaaagtttctagataacatcagatgttttaatgtgtggcaaacagaatgcccacagttaattgtaaaggctgataattatttaaaatcaaagaacgtcatagctaaagataaatctttagcaaactattttactgtaggagcatatgattacttcttatcccagaatggcattgatttctacaacaacattatcggcggtctaccagcatttgctggtcatgagaaaatccaaggacttaatgaatttataaatcaagaatgccaaaaggacagcgaactaaaatctaaactgaaaaacagacatgctttcaaaatggctgttctatttaagcaaattctttcagatagagaaaaaagttttgttatagacgagttcgaatctgatgctcaggtcatagatgcggttaagaacttctatgcagaacaatgtaaggataataatgttatttttaaccttctaaatcttatcaagaatatagcgttcttatctgatgatgaattagatggaatttttatagaaggcaagtatttaagctctgtttcccaaaagctatattcagattggtcgaagcttcgaaatgatattgaagatagtgcaaacagtaaacaaggaaataaagagttagcaaagaaaattaaaacaaataaaggcgatgttgaaaaggccataagtaaatatgagttttctttatcagaacttaactcaattgtacatgataatacaaaattcagtgaccttctttcttgtacgttacataaagtggctagcgaaaaactagtgaaagttaatgaaggggactggccaaaacacctgaaaaataatgaagaaaaacaaaagataaaagagcctttagatgcattgttagaaatttataatacattgctgatattcaactgcaagtcatttaataagaacggtaatttctatgttgattatgacagatgcataaatgagctttctagtgttgtttatttatataacaaaacaagaaattactgtacaaagaaaccttataacacagacaaattcaaattaaactttaacagtcctcaattaggagagggctttagtaagtcgaaagaaaatgactgtctgacattattatttaaaaaagacgacaattactatgttggaattatcagaaaaggggcaaaaattaactttgatgatacacaagccattgcagacaatacagataactgtatatttaagatgaattatttcctattaaaagatgctaaaaagtttattcctaaatgttcaattcagttaaaagaagtaaaagcacattttaaaaaatcagaggatgattatatcctgagtgacaaagaaaaatttgcctctccccttgttattaagaaatcaacatttttattagcaacagcacatgtaaaaggaaagaaaggaaacataaaaaaattccaaaaggaatattctaaggaaaatccaacagaatatagaaattctctgaatgaatggattgcattttgtaaagaatttctaaaaacatataaggcggcaacaatctttgacattacaacgttaaaaaaagctgaagaatatgctgatattgttgagttttataaggatgtagataatctttgttataaactagagttttgccctattaaaacatctttcattgagaatcttattgataatggggacttatatttattcagaatcaataataaagatttcagttcaaaatctactggtacaaagaatcttcatacgctctatcttcaggcaatctttgatgaaagaaacctcaataatcctactattatgttaaatggcggagcagagttattttatcgaaaagaaagcattgaacagaaaaataggataactcataaggcaggatcaattcttgtaaacaaggtttgtaaggatggaacaagtctagatgacaaaatcagaaacgaaatatatcaatatgaaaacaagtttattgatacattgtctgatgaagctaaaaaagttttacctaatgtaataaaaaaagaagcaactcacgacataacaaaagataagcgatttacatcagataagttctttttccattgcccattaacaattaactataaggaaggagatacaaaacaatttaacaatgaggttttatctttccttagaggtaatccagacattaatatcatcggaattgacagaggagaaagaaaccttatatacgtaactgttattaatcagaaaggcgaaatacttgacagcgtttcgtttaacacagtaacaaacaagtcgagcaaaattgaacaaactgttgattatgaggaaaagcttgctgttagggaaaaagaaagaatagaagcaaaaagatcctgggattcaatatcaaagatagcaaccttaaaagaaggttatctatcagctattgttcatgagatatgcctactgatgatcaaacacaacgcaatcgttgtacttgagaatctaaatgcaggatttaagagaattagaggaggattatcagaaaagtctgtttatcagaaattcgagaagatgcttattaacaaactaaattactttgtatctaaaaaagaatcagactggaataaacctagtggacttttaaatggtttacaactttcagaccagttcgagtcatttgagaaattaggaattcaatctgggttcatcttctatgttcctgcagcatatacatctaagattgatcctacaacaggatttgcaaatgttcttaacttatccaaggtaagaaatgttgatgcaataaagagttttttcagtaatttcaatgaaatttcatatagcaaaaaagaagctctctttaaattctcttttgatttagattccttatcaaagaagggcttcagctcatttgtaaaattcagtaaatctaaatggaatgtatatacatttggagagagaataataaaaccaaagaataagcaagggtatcgtgaagataagagaattaatttaacatttgaaatgaaaaaacttctgaatgaatataaagtaagttttgatcttgaaaacaacttaattccaaatctaacctctgcaaatctgaaagataccttctggaaagaactattctttatttttaaaacaactctgcagcttagaaacagtgtaacaaatggcaaagaagatgtactgatttctccagtaaagaacgctaaaggagagttctttgtatcaggaactcataacaagacattacctcaagactgtgatgcaaatggagcatatcatatcgccctaaaaggtctgatgattcttgaacgtaacaatcttgttagagaagaaaaagacacaaagaagataatggcaatttctaatgttgactggtttgagtatgttcaaaaaaggagaggtgtcctgtaa

SEQ ID NO: 23 - DNA, 3717 bp, Artificial Sequence
  Description of Artificial Sequence: Synthetic polynucleotide
atgaacaactatgatgagtttaccaaactgtacccaatacagaaaacgataaggttcgaattgaagccgcagggaagaacgatggaacacctcgaaacattcaactttttcgaagaggacagggatagagcggagaaatataagattttaaaggaagcaatcgacgagtatcataagaagtttatagacgaacatctaacaaatatgtctcttgactggaattctttaaaacagatttcagagaaatactataagagtagagaggaaaaagacaagaaagtttttctgtcagaacagaaacgcatgaggcaagagatagtttctgagttcaaaaaagacgatcggtttaaagatcttttttcaaaaaaattgttttctgaacttctcaaggaagagatttacaaaaaaggaaaccatcaggaaattgacgcattgaaaagttttgataaattctcaggctattttattgggttgcatgagaaccgaaaaaatatgtattctgacggagacgagatcacggctatctctaaccgtattgtaaatgagaatttcccgaagttcctcgacaaccttcagaaatatcaggaagctcgtaaaaaatatccagagtggatcattaaggcagaatctgctttagttgcacataatatcaagatggatgaagtcttttccttagagtatttcaacaaagtcctgaatcaagaaggaatacagagatacaatctcgccctaggtggctatgtgaccaaaagtggtgagaaaatgatggggcttaatgatgcacttaatcttgcccatcaaagtgaaaaaagcagcaagggaaggatacacatgactccactcttcaaacagattctgagtgaaaaagagtccttttcttatataccagatgtttttacagaagactctcaacttttaccatccattggtgggttctttgcacaaatagaaaatgataaggacgggaatatttttgacagagcattagaattgatatcttcttatgcagaatacgatacagaaaggatatatatcaggcaagcggacataaacagagtttctaatgttattttcggggagtggggaacactgggggggttaatgagggaatacaaagcagactctatcaacgacatcaatttggagagaacatgcaagaaggtagacaagtggctcgactcaaaggagtttgcgttatcagatgtattagaggcaataaaaagaaccggcaataatgatgcttttaatgaatatatctcaaagatgcgcactgccagggaaaagattgacgctgcaagaaaggaaatgaaattcatttcggaaaaaatatctggagacgaagaatcgatccatattatcaaaaccttattggactcggtgcaacagtttttacattttttcaatttattcaaagcgcgtcaggacattcctcttgatggagcattctatgcggagttcgatgaagtccatagcaaactgtttgctattgttccgttgtataataaggttaggaactatcttacgaaaaataaccttaacacgaaaaagataaagctaaacttcaagaatccaactctggcaaacggatgggatcaaaacaaggtatatgactacgcctccttaatctttctccgcgatggtaattattatctcggaataataaatccaaaaaggaaaaagaatattaaattcgaacaagggtctggaaatggcccattctaccggaagatggtgtacaaacaaattccagggccgaacaagaacttaccaagagtcttcctcacatctacgaaaggcaaaaaagagtacaagccgtcaaaggagataatagaaggatatgaagcggacaaacacataagaggagataaattcgatctggatttctgtcataagctgatagacttcttcaaggaatccatcgagaagcacaaggactggagtaagttcaacttctatttctctccaactgaatcatatggagacatcagcgaattctatctggatgtagaaaaacagggataccggatgcattttgagaatatttctgccgagacgattgatgagtatgtcgaaaagggggacttattcctcttccagatatacaacaaagactttgtgaaagcggcaaccggaaaaaaagatatgcacaccatttattggaacgcggcattctcgcccgagaaccttcaggatgtggtagtgaaactgaacggtgaagcagaacttttctacagagacaagagcgacatcaaggagatagttcacagggagggagagatactggtcaatcgtacctacaacggcaggacacctgtgcctgacaagatccacaaaaaattaacagattatcataatggccgtaccaaagatctcggagaagcaaaagaatacctcgataaggtcagatatttcaaagcgcactacgacatcacaaaggatcgcagatacctgaatgataaaatatacttccatgtgcctctgacattgaatttcaaagcaaacgggaagaagaatctcaataagatggtaattgaaaagttcctctcggacgaaaaagcgcatattattgggattgatcgcggggaaaggaatcttctttactattctatcattgacaggtcaggtaaaataatcgatcaacagagcctcaacgtcatcgatggattcgattaccgagagaaactgaatcagagggagatcgagatgaaggatgccagacaaagctggaatgctatcgggaagataaaggacctcaaggaagggtatctttcaaaagcggtccacgaaattaccaagatggcgatacaatacaatgccattgttgtcatggaggaactcaattatgggttcaaacgcggacgtttcaaagttgagaagcagatatatcagaaattcgagaatatgctgattgacaagatgaattatctggtattcaaggatgctccggatgaaagtccgggaggagtcctcaatgcatatcagcttactaatccgcttgaaagtttcgctaaacttgggaaacagacaggaattcttttctatgttccggcagcctatacttcgaagatagatccgacgaccgggtttgtcaatcttttcaatacttcaagtaaaacgaacgcacaggaaagaaaagaattcttgcaaaaattcgagtcgatctcctattccgctaaagacggaggaatattcgcattcgcgttcgattatcggaagttcggaacgtcaaaaacagaccacaaaaatgtatggaccgcatacacgaacggggaaaggatgaggtacataaaagagaaaaaacgcaacgaactgttcgacccctcgaaggagatcaaagaggctctcacttcatcaggaatcaaatatgacggcggacagaacatattgccagatatcctgaggagcaacaataacggtctgatctacacaatgtattcctctttcatagcggccattcaaatgagggtctatgacgggaaagaagactatatcatctcgccgataaagaacagcaagggagagttcttcaggaccgatccgaaaagaagggaacttccgatagacgcggatgcgaacggcgcgtataacattgctctcaggggcgaattgacgatgcgtgcgatagcggagaagttcgatccggactcggaaaagatggcgaagctagaactgaaacataaggactggttcgaattcatgcagacaaggggggattga

SEQ ID NO: 24 - DNA, 3897 bp, Artificial Sequence
  Description of Artificial Sequence: Synthetic polynucleotide
atgacaaaaacatttgattcagaattttttaatttatattctcttcaaaaaacagttcgttttgaactcaagccggttggtgaaacagcctcgtttgttgaagattttaaaaacgaaggtttgaaacgagttgtttcagaggatgaacggcgtgcggttgattaccaaaaagtgaaagaaattattgatgactaccaccgagattttattgaagaatcgctgaactattttcctgagcaggtctcaaaagacgctttggaacaagcttttcacctttatcaaaaactaaaagccgctaaggttgaagagcgtgaaaaagcattgaaagaatgggaagcccttcagaaaaaactgcgcgaaaaagttgttaaatgtttttcagattcaaacaaagcacgcttttcccgcattgataaaaaagaactgattaaagaagatttaattaactggttggttgcacaaaatcgcgaagatgacattccaaccgttgaaacctttaacaactttacgacttattttacggggtttcatgaaaaccgaaaaaacatttattcaaaagacgatcatgccacagccatttcatttcgactcattcatgaaaacctgcctaagttttttgataatgtgatcagctttaataaattgaaggaaggatttccagagctgaaatttgataaggttaaggaagatttagaagttgattatgacttgaaacatgcctttgaaatcgaatactttgtcaattttgttacccaagccggaattgaccaatataactatcttttggggggtaaaaccttagaagacggcaccaaaaagcaaggcatgaatgaacaaatcaatctgttcaagcaacagcaaacccgagacaaagcccgacaaattcccaaactcataccattgtttaaacaaattctaagcgaacgaacggaaagccaatcgtttattccaaaacaatttgaatcagaccaagagctatttgactcactgcaaaaactgcataacaactgccaagataaatttaccgtactgcaacaagccattttaggcttagccgaagcagatctgaaaaaagtattcattaaaacatctgatcttaatgcgctatcaaataccatttttggaaattacagtgtgttttcggatgcgttgaatttatacaaagaatcgctcaaaacaaaaaaggcgcaagaagcgtttgaaaaactacccgctcacagcattcatgacttgattcaatatttggagcaatttaatagctctttggatgcagaaaaacagcaatcaactgacaccgtactgaattactttattaaaacagacgagctgtattctcggttcataaaatcaacgagcgaagccttcacacaagtacaaccactctttgaattggaagcattaagctcaaaacgtcgtccaccggaaagtgaagacgaaggcgcaaaaggtcaggaagggtttgagcaaattaaacgcataaaagcctatttggataccttgatggaggcggtgcattttgcaaaaccactttatctggtgaaggggcgcaaaatgattgaaggtctggacaaagaccaaagtttctatgaagcctttgaaatggcttaccaagaactagaaagtctgattattccaatctacaacaaagctcgtagttatttaagtcgtaaaccgtttaaagcggacaaattcaaaattaattttgataataatacattgctttccggttgggatgctaataaagaaacggctaacgcttcaattttgtttaagaaggatggtttgtattatttaggaatcatgcctaaaggaaaaacgtttttgttcgattacttcgtttcatcggaagattctgaaaagttaaaacaaagaagacaaaaaaccgccgaagaagcgcttgcgcaagatggcgaaagctactttgaaaaaattcgttacaagctgttacctggcgccagcaaaatgttgccgaaagtatttttttccaacaaaaacatagggttttacaacccaagtgatgacatacttcgtatcaggaatacagcctctcacactaaaaacggaacaccgcaaaaagggcactctaaagtagagtttaatttgaatgattgtcataagatgattgatttctttaaatcaagcattcaaaagcatccagagtggggaagttttggattcaccttttcagatacatcagattttgaagatatgagcgccttttatcgagaagtcgaaaaccaaggttatgtcattagtttcgataaaataaaagaaacttacattcagagtcaagttgaacaggggaacctatatttattccaaatctacaataaagacttctcgccctacagcaaaggcaaaccaaatttacacacgctttactggaaagcgttgtttgaggaagccaacctaaataatgtggtggcaaaactcaatggtgaagctgaaattttctttaggcgacactcaatcaaagcatctgataaagtggtgcacccagcgaatcaagccattgacaataaaaacccgcataccgaaaaaacgcaaagcacctttgaatatgatcttgtaaaagacaagcgctatacccaagacaaattcttcttccatgtaccgatttcattgaactttaaggcacaaggtgtttcaaaatttaacgataaagtgaatggatttttaaagggtaacccagatgtcaatattattggcattgaccgaggcgaacgacaccttctgtatttcactgtggtgaatcagaaaggtgaaattttggttcaagagtcgcttaataccctaatgagtgataaagggcatgtgaatgactaccagcaaaaactcgacaaaaaagaacaagaacgcgatgccgctcgcaaaagctggacgacggttgaaaatatcaaagaattaaaagaaggctatttatctcatgttgttcataagttggcacacctgattattaaatacaatgccattgtttgcttggaagacctgaattttggtttcaaacgcgggcgttttaaagtggaaaaacaagtttatcagaaatttgaaaaagcgcttattgataagcttaactacttggtatttaaagaaaaagagttaggcgaggtgggccattatctaaccgcctatcagttgaccgcaccgtttgaaagtttcaagaagttaggcaagcaaagtggcatattgttttatgttccggcggattacacctccaaaattgacccaaccaccgggtttgtcaactttcttgatctgcgttatcagagtgtcgaaaaagccaaacagctcttaagcgactttaatgccattcgttttaattcagtacaaaactattttgagttcgaaatagattacaaaaaactcacacccaaacgtaaagttggtactcagagtaaatgggtgatttgtacctatggagatgtccgctatcaaaatcggcgtaatcaaaaaggtcactgggaaacggaagaagtcaatgtgactgaaaaactaaaagcccttttcgccagtgattccaaaactacaaccgtaatcgattacgccaatgacgacaacctaattgacgtcattctggaacaggacaaagccagcttcttcaaagaactgttatggttattaaaactcaccatgacgctccgccacagcaaaatcaaaagtgaagacgactttattctttcacccgttaaaaacgaacaaggcgagttttacgatagtcgaaaagcgggcgaggtgtggcctaaagatgcagacgccaatggcgcttatcacatagcgttgaaaggcttgtggaatctgcaacagatcaatcagtgggaaaagggtaaaacacttaatctggcgattaaaaaccaggattggttcagttttattcaagaaaagccctatcaagaataa

SEQ ID NO: 25 - DNA, 3708 bp, Artificial Sequence
  Description of Artificial Sequence: Synthetic polynucleotide
atgcacacaggcggattacttagcatggatgccaaggagtttaccggacagtaccccctttcgaagactctgcgttttgaactgagaccgataggcagaacgtgggacaatctcgaagcatcggggtatcttgcggaggacagacaccgtgcagaatgctatcccagggcaaaagagctcttggacgacaaccatcgtgcattcctcaaccgtgtcctgcctcagatcgatatggattggcacccgatcgcagaggcattctgcaaagtccacaagaatccgggaaacaaggaattggctcaggattacaatcttcagctgtccaaacgcagaaaggagatttcggcctatctgcaggatgcggacggctataaaggtctgtttgccaaacctgcattggatgaagcaatgaagatcgcgaaagaaaacggaaatgaatcggacatagaggttcttgaggcattcaacggtttctccgtatacttcaccggatatcatgagagcagggagaacatctattcggacgaggatatggtgtcggtagcttatcgcatcaccgaagacaatttcccgagattcgtttccaatgcgcttatattcgataagctgaatgagtcgcaccccgatataatctcggaagtatccggaaatctgggcgtagacgacatcggaaaatattttgatgtgtctaactacaataatttcctgtcgcaggccggtatagatgactacaatcacatcatcggcggccatacgacggaggacggtctgatccaggcattcaatgttgttctgaatctcaggcatcagaaagaccccggattcgaaaaaatccaattcaaacagctgtacaaacagatactcagcgtccgtacatccaaatcctatatcccgaaacagttcgataattcgaaggagatggtggactgcatctgcgactatgtgtccaagatcgaaaaatccgaaacggtcgagagagcattgaagctggtaaggaacatatcttcttttgatttgcgcggaatattcgtaaacaagaagaatctccgcattctttccaacaaactgattggtgattgggacgcgatcgaaaccgcgctgatgcactcctcctcttcggaaaatgataagaaatccgtctacgacagcgccgaggcatttacgctggatgatatcttttcgtccgttaaaaaattctcagatgcatctgcagaggatatcggaaaccgggcggaggacatatgcagagtcatatctgagaccgctccgttcataaacgatctgagggctgtcgatttggacagtttgaatgacgacggttacgaggcggcggtttccaagataagggaatctctggaaccatatatggatctgtttcatgaactggagatattctccgtaggcgatgaattcccgaaatgtgcagctttctacagtgaacttgaagaagtctccgaacagctaatcgagattataccgttattcaacaaggcccgttcgttctgtacgcgcaagagatacagtacggacaagataaaggtcaatttgaaattcccgacactcgccgacggatgggatctcaacaaagaacgcgacaacaaagccgcaatactcaggaaagacggaaagtactacctggccatactggatatgaagaaagatctttcttcgatcagaacttcggatgaagacgaatccagttttgagaaaatggagtacaagcttcttccgagtccggtaaagatgctgccaaagatcttcgtaaaatcgaaggcggccaaggagaagtacggtctgaccgaccgtatgctggagtgctacgataaagggatgcacaagagcggcagtgcattcgatctcggattttgtcacgaattgatcgattactacaagaggtgcatcgcagaatatcccggctgggacgtcttcgatttcaagttcagggaaacatcggattatggcagcatgaaggagttcaatgaggatgttgcaggggccggatactatatgtccctcagaaagatcccttgttcggaggtctacaggcttcttgatgagaaatcgatatatcttttccagatctacaacaaagattattcggaaaacgctcatgggaataagaacatgcataccatgtattgggaagggctcttttccccccagaatctggaatcccctgtgtttaaactcagcggcggtgcggagcttttcttccgtaaatcctccatacccaatgacgccaaaacggtccatccgaagggaagcgtcctggttccgcgcaatgatgtaaacggccgcaggatacctgacagcatatatcgggagctcaccagatatttcaaccgcggagattgccgcataagcgacgaggcaaagagttatctggacaaggtgaaaaccaagaaagctgaccacgatatcgtgaaagacaggaggttcacggtggacaagatgatgttccacgtccctatcgccatgaatttcaaagcgatttcgaagccgaatctcaataaaaaggtgattgacggcataatcgacgaccaagatctgaagatcatcggcatagaccgcggagagcgcaacctcatctacgtaaccatggtggatcgcaaagggaacatcctctatcaggatagcctcaatattctgaacggatacgattaccgtaaggccctcgacgtccgcgaatatgacaataaagaggctcggaggaactggacgaaggtcgaaggcatccgtaagatgaaagaggggtatctgtcgcttgcagtcagcaaattggcagatatgatcatagagaacaatgcgattatcgtcatggaggatctcaatcacggattcaaggcagggcgttcgaagatagagaaacaggtctatcagaagttcgaatccatgctcataaacaaactcggttacatggtcctcaaggataagtctatcgatcagagcggcggagctctccacggataccagcttgccaaccatgtgacaacattggcatctgtaggtaaacaatgtggagtgatattctacatccctgctgcatttacatccaagatagatccgacaacaggatttgcagatctgttcgccctcagcaatgttaaaaacgtggcatctatgagagaatttttctccaagatgaagtctgtaatctatgataaggcggagggaaaattcgcatttaccttcgactatcttgattataatgtgaaatccgagtgcggaaggaccctttggaccgtgtatacggtcggagagagattcacatacagcagggtcaatagagaatatgtcagaaaagttccgacagacataatctacgacgcattgcaaaaggcaggaatatctgttgaaggggatctcagggacaggattgctgaatcggatggcgacactctgaagagcatattctatgcattcaagtatgcattggatatgagagtagagaaccgcgaagaggattacatacagtctcctgtcaaaaatgcctccggagaattcttctgttccaagaacgcaggcaaatcgctccctcaggattccgatgcgaacggtgcatacaatatcgcactcaaggggatcctgcagctacgtatgctttccgagcagtatgatccgaatgcagagagcatacggttgccactgataaccaacaaggcctggctgacctttatgcagtccggtatgaagacatggaagaactga

SEQ ID NO: 26 - DNA, 3783 bp, Artificial Sequence
  Description of Artificial Sequence: Synthetic polynucleotide
atggatagtttgaaagatttcaccaatctgtaccctgtcagtaagacattgagatttgaattaaagcccgttggaaagactttagaaaatatcgagaaagcaggtattttgaaagaggatgagcatcgtgcagaaagttatcggagggtgaagaaaataattgatacttatcataaggtatttatcgattcttctcttgaaaatatggctaaaatgggtattgagaatgaaataaaagcaatgctccaaagtttctgcgaattgtataaaaaagatcatcgcactgagggtgaagacaaggcattagataaaattcgagcagtacttcgtggcctgattgttggggctttcactggtgtttgcggaagacgggaaaatacagtccaaaacgagaagtacgagagtttgttcaaagaaaagttgataaaagaaattttacctgattttgtgctctctactgaggctgaaagcttgcctttctctgttgaagaagctacgaggtcactgaaggagtttgatagctttacatcctactttgctggtttttacgagaatagaaagaatatatactcgacgaaacctcaatccactgccattgcttatcgtcttattcatgagaacttgccgaagttcattgataatattcttgtttttcagaagatcaaagagcctatagccaaagagctggaacatattcgtgcggacttttctgccggggggtacataaaaaaggatgagagattggaggatattttttcgttgaactattatatccacgtgttatctcaggctgggatcgaaaaatataacgcattgattgggaagattgtgacagaaggagatggagagatgaaagggctcaatgaacacatcaacctttacaaccaacaaagaggcagagaggatcggctccctctttttaggcctctttataaacagatattgagtgacagagagcaattatcatacttgcctgagagttttgaaaaagatgaggagctcctcagggctctaaaagagttctatgatcatatcgcagaagacattctcggacgtactcaacagttgatgacttctatttcagaatatgatttatctcggatatacgtaaggaacgatagccaattgactgatatatcaaaaaaaatgttgggagattggaatgctatctacatggctagagaacgagcatatgaccacgagcaggctcccaaaagaatcacggcgaaatacgagagggacaggattaaagctcttaaaggagaagagagtataagtctggcaaatcttaatagttgtattgcctttctggacaatgttagagattgccgtgtagatacttatctttccacactgggccagaaggaaggaccacatggtctatctaatctcgttgagaacgtttttgcctcataccatgaagcagagcaattgttgagctttccataccccgaagagaataatctgattcaggacaaggacaatgtggtgttaattaagaatcttctcgacaatatcagtgatctgcagaggttcttgaaacctctttggggtatgggagacgaacccgataaagatgaaagattttatggagagtataattatatccgaggagctctagatcaggtgatccctctgtacaataaggtaaggaactacctcactcggaagccttattcgaccagaaaagtaaaactcaattttgggaattctcaattgcttagtggttgggatagaaataaggaaaaggataatagctgtgtgattttgcgtaaggggcagaacttctatttggctattatgaacaataggcacaaaagaagtttcgaaaacaaggtgttgcccgagtataaggagggagaaccttacttcgaaaagatggattataaatttttgcctgatcctaataaaatgcttcctaaggtttttctttcgaaaaaaggaatagagatatacaaaccaagtccgaagcttttagaacaatatggacatggaactcacaaaaagggagatacctttagtatggatgatttgcacgaactgatcgatttcttcaaacactcaatcgaggctcatgaagattggaagcaattcggattcaaattttctgatacggctacttatgagaatgtatctagtttctatagagaagttgaggatcaggggtataagctctctttccgaaaagtttcggaatcttatgtctattcattaatagatcaaggcaagttgtatttatttcagatatacaacaaggacttttctccctgcagcaaagggacacctaatctgcataccttgtattggagaatgctttttgacgagcgcaatttggcagatgtcatatacaaactggatgggaaggctgaaatctttttccgagagaagagtttgaaaaatgatcatcccacgcatccggctggtaagcctatcaaaaagaaaagtcgacaaaaaaaaggagaggagagtctgtttgagtatgatttagtcaaggataggcactatacgatggataagttccagtttcatgtgcctattactatgaattttaaatgttctgcaggaagcaaagtcaatgatatggttaatgctcatattcgagaggcaaaggatatgcatgtcattggaattgatcgtggagaacgcaatctgctgtatatatgcgtgatagatagtcgagggacgattttggatcaaatttctctgaatacgattaacgatatagactatcatgatttattggagagtcgagacaaagaccgtcagcaggagcgccgaaactggcaaactatcgaagggatcaaggagctaaaacaaggctaccttagtcaggcggttcatcggatagccgaactgatggtggcttataaggctgtagttgctttggaggatttgaatatggggttcaaacgtgggcggcagaaagtagaaagttctgtttatcagcagtttgagaaacagctgatagataagctcaactatcttgtggacaagaagaaaaggcctgaagatattggaggattgttgagagcctatcaatttacggccccatttaagagttttaaggaaatgggaaagcaaaacggcttcttgttttatatcccggcttggaacacgagcaacatagatccgactactggatttgttaatttatttcatgcccagtatgaaaatgtagataaagcgaagagcttctttcaaaagtttgattcaattagttacaacccgaagaaagactggtttgagtttgcattcgattataaaaactttactaaaaaggctgaaggaagtcgttctatgtggatattatgcacacatggttcccgaataaagaattttagaaattcccagaagaatggtcaatgggattccgaagaattcgccttgacggaggcttttaagtctctttttgtgcgatatgagatagattataccgctgatttgaaaacagctattgtggacgaaaagcaaaaagacttcttcgtggatcttctgaagctattcaaattgacagtacagatgcgcaacagctggaaagagaaggatttggattatctaatctctcctgtagcaggggctgatggccgtttcttcgatacaagagagggaaataaaagtctgcctaaggatgcagatgccaatggagcttataatattgccctaaaaggactttgggctctacgccagattcggcaaacttcagaaggcggtaaactcaaattggcgatttccaataaggaatggctacagtttgtgcaagagagatcttacgagaaagactga

SEQ ID NO: 27 - DNA, 3792 bp, Artificial Sequence
  Description of Artificial Sequence: Synthetic polynucleotide
atgaataatggaacaaataactttcagaattttatcggaatttcttctttgcagaagactcttaggaatgctctcattccaaccgaaacaacacagcaatttattgttaaaaacggaataattaaagaagatgagctaagaggagaaaatcgtcagatacttaaagatatcatggatgattattacagaggtttcatttcagaaactttatcgtcaattgatgatattgactggacttctttatttgagaaaatggaaattcagttaaaaaatggagataacaaagacactcttataaaagaacagactgaataccgtaaggcaattcataaaaaatttgcaaatgatgatagatttaaaaatatgttcagtgcaaaattaatctcagatattcttcctgaatttgtcattcataacaataattattctgcatcagaaaaggaagaaaaaacacaggtaattaaattattttccagatttgcaacgtcattcaaggactattttaaaaacagggctaattgtttttcggctgatgatatatcttcatcttcttgtcatagaatagttaatgataatgcagagatattttttagtaatgcattggtgtataggagaattgtaaaaagtctttcaaatgatgatataaataaaatatccggagatatgaaggattcattaaaggaaatgtctctggaagaaatttattcttatgaaaaatatggggaatttattacacaggaaggtatatctttttataatgatatatgtggtaaagtaaattcatttatgaatttatattgccagaaaaataaagaaaacaaaaatctctataagctgcaaaagcttcataaacagatactgtgcatagcagatacttcttatgaggtgccgtataaatttgaatcagatgaagaggtttatcaatcagtgaatggatttttggacaatattagttcgaaacatatcgttgaaagattgcgtaagattggagacaactataacggctacaatcttgataagatttatattgttagtaaattctatgaatcagtttcacaaaagacatatagagattgggaaacaataaatactgcattagaaattcattacaacaatatattacccggaaatggtaaatctaaagctgacaaggtaaaaaaagcggtaaagaatgatctgcaaaaaagcattactgaaatcaatgagcttgttagcaattataaattatgttcggatgataatattaaagctgagacatatatacatgaaatatcacatattttgaataattttgaagcacaggagcttaagtataatcctgaaattcatctggtggaaagtgaattgaaagcatctgaattaaaaaatgttctcgatgtaataatgaatgcttttcattggtgttcggttttcatgacagaggagctggtagataaagataataatttttatgccgagttagaagagatatatgacgaaatatatccggtaatttcattgtataatcttgtgcgtaattatgtaacgcagaagccatatagtacaaaaaaaattaaattgaattttggtattcctacactagcggatggatggagtaaaagtaaagaatatagtaataatgcaattattctcatgcgtgataatttgtactatttaggaatatttaatgcaaaaaataagcctgacaaaaagataattgaaggtaatacatcagaaaataaaggggattataagaagatgatttataatcttctgccaggaccaaataaaatgatccccaaggtattcctctcttcaaaaaccggagtggaaacatataagccgtctgcctatatattggagggctataaacaaaacaagcatattaaatcctctaaggattttgatataacattttgtcacgatttgattgattattttaagaactgtatagcaatacatcctgaatggaagaattttggctttgatttttctgacacctccacatatgaagatatcagcggattttacagagaagtcgaattacaaggttataaaatcgactggacatatatcagcgaaaaggatattgatttgttgcaggaaaaaggacagttatatttattccaaatatataacaaagatttttccaagaaaagtaccggaaatgataatcttcatactatgtatttgaagaatttgtttagtgaagagaatttaaaggatattgtactgaaattaaacggtgaggcggaaatcttctttagaaaatcaagcataaagaatccaataattcataaaaaaggctctattcttgttaatagaacatatgaagcagaggaaaaagatcaatttggaaatatccagatagtcagaaaaaacataccggaaaatatatatcaggagctttataaatatttcaatgataaaagtgataaagaactttcggatgaagcagctaagcttaagaatgtagtaggtcatcatgaggctgctacaaacatagtaaaagattatagatatacatatgataaatattttcttcatatgcctattacaatcaattttaaagccaataagacaggctttattaatgacagaatattacaatatattgctaaagaaaaggatttgcatgtaataggcattgatcgtggtgaaagaaacctgatatatgtttcagtaattgatacttgtggaaatattgttgaacaaaaatcgtttaacattgttaatggatatgattatcagattaagctcaagcagcaggagggggcgcgacaaatcgcacgaaaagaatggaaagaaatcggcaaaataaaagaaattaaagaaggctatttatctcttgtaattcatgaaatttcaaagatggttattaaatataatgccataattgcaatggaggatttaagctacggatttaaaaaaggtcgtttcaaggttgagcgacaggtttaccagaagtttgagacaatgcttatcaacaaactcaactatctggtatttaaagatatatccataacggaaaacggtggtcttctaaagggataccagcttacatatattccagataaactgaaaaatgtgggtcatcaatgtggctgtatattttatgtacctgctgcctatacatcaaaaatagatcctacaaccggatttgtaaatatattcaaatttaaagatttaacagttgatgcgaagagagaatttataaaaaaatttgacagtatcagatatgattcagaaaaaaatctgttttgttttacattcgattataataactttattacgcaaaatactgttatgtcaaagtcaagctggagtgtatatacgtacggagttaggataaaaagaagatttgtcaatggcaggttctcaaatgaatcggatacaattgatataacaaaagatatggaaaaaacactcgaaatgacagatataaattggagagatggtcatgatctgaggcaggatattattgattatgaaatcgtacaacacatatttgagatttttagattgactgtacaaatgagaaacagtttaagtgaattagaagacagggattatgaccgtttgatttctccggtgctcaatgaaaataatatattttatgattcagctaaagcaggagatgcgttacctaaagacgcagatgctaatggtgcatattgtatagctctaaaaggcttgtatgaaatcaaacaaattacagagaattggaaagaagacggtaagttttcaagagataaacttaaaatttccaataaggactggtttgactttattcaaaataaaaggtatttataa

SEQ ID NO: 28 - DNA, 3957 bp, Artificial Sequence
  Description of Artificial Sequence: Synthetic polynucleotide
atgacaaacaaatttacaaaccagtactcgctttccaaaacacttcgatttgagttgattccacaaggaaaaacattggaatttattcaagaaaaaggattgctctctcaagataaacaacgagcggagagttatcaagaaatgaaaaaaactattgataaatttcataaatactttatcgatttagctttaagcaatgctaaactaactcatttagaaacttacttggaattatacaataaaagtgctgaaacaaaaaaagaacaaaaatttaaagacgatttaaagaaagtacaagacaatttacgaaaagaaatcgttaaatctttttcagatggtgatgcaaaatcaatttttgcaattttggataaaaaagaactgattaccgtagaacttgaaaaatggtttgaaaacaacgaacaaaaagacatttattttgacgaaaaattcaaaacgtttactacttattttactggttttcatcaaaacagaaaaaacatgtattcggttgaacccaattctacagcaattgcttatcgattgattcatgaaaatttacctaaatttttagaaaatgctaaagcatttgaaaaaataaaacaagtagaaagtttgcaagttaattttagagaattaatgggggaatttggagatgaagggctaattttcgtaaatgaattagaagaaatgtttcaaatcaattattataatgatgtgctttcacaaaatggaattacaatttataatagtataatttcaggatttaccaaaaatgatataaaatataaaggtctaaatgaatacataaataattacaatcaaaccaaagacaaaaaagaccgtttgccaaaattaaaacaattgtataaacagattttgagtgataggatttcactttcgtttttgcccgatgcttttacggatgggaaacaagttttgaaagccatatttgacttttataaaatcaacttactttcttataccattgaaggacaggaagaaagccaaaatcttttactattaattcgtcagacaattgaaaacctttctagttttgatacccaaaaaatttatctaaaaaatgatacccatttaaccactatttcacaacaagtatttggcgatttttcggtgttttcaactgctttaaattattggtatgaaactaaagtaaatccaaaatttgaaacggaatatagcaaagccaacgaaaaaaaacgagaaattttagataaagccaaagcggtatttacaaaacaagattatttttcaattgcttttttacaagaagtactttcggaatacattcttaccttagatcacacttctgatattgtaaaaaagcattcctccaactgtattgcggattattttaaaaatcattttgtagccaaaaaagaaaatgaaaccgacaaaacctttgattttattgctaatattactgcaaaataccaatgtattcaaggtattttagaaaatgcagaccaatacgaagacgaactcaaacaagaccaaaaattaattgataatttgaaattctttttagatgctattttagaattgttgcattttattaaacctttgcatttaaaatcagaaagcattaccgaaaaagacactgctttttatgatgtgtttgaaaattattacgaagcattgagtttgttgaccccattatataatatggtgcgaaactatgtaacgcaaaagccgtacagcaccgaaaaaataaaattaaattttgaaaatgcacaattattgaatggttgggatgccaataaagaaggtgattacctaactaccattttgaaaaaagacggtaattattttttagccataatggataaaaagcataacaaagcgtttcaaaagtttccagaaggaaaagaaaattatgaaaaaatggtgtataaactattgcctggagtaaataagatgttgccaaaagtatttttttccaataaaaatattgcttacttcaacccatcaaaagagttattagaaaactataaaaaagagacgcacaaaaaaggagacacattcaatttagaacattgtcatacgttgatcgattttttcaaggactctttaaacaaacatgaagactggaaatactttgattttcaattttctgaaacaaaatcgtatcaagatttgagtggtttttatagagaagtagaacatcaaggctacaaaatcaattttaaaaatatcgattcagaatatattgatggtttggtgaacgaaggtaaattgtttctatttcaaatttacagcaaagatttttcgcctttttccaaagggaaaccgaacatgcacactttgtattggaaagccttatttgaagaacaaaatttgcaaaatgtaatctataaattgaatggacaagccgaaatattttttagaaaagcctctataaaacctaaaaatataatattgcacaaaaagaaaattaaaattgccaaaaagcattttattgataaaaaaacaaaaacatctgaaattgttcctgttcaaacaataaaaaacctcaatatgtactaccaaggaaaaataagtgaaaaagaattaacacaagatgatttaaggtatattgataattttagcattttcaatgaaaaaaataaaacaattgatattataaaagacaaacgatttacggttgataaatttcagtttcatgtgccgattaccatgaactttaaagcaacgggcggaagttatatcaatcaaaccgtattagaatatttgcaaaacaatcccgaagttaagattattggattggatagaggcgaacgccatttggtatatctgacactgatagaccagcaaggaaacatcttgaaacaagaaagtttgaatacaatcaccgattctaaaatctcgacaccttatcataagttgttggataacaaggaaaacgagcgtgacttggctcgaaaaaattggggaacggtggaaaacatcaaagaactcaaagaaggctacatcagtcaagtggtgcataaaattgctacgttgatgctggaagaaaatgccattgtggtaatggaagatttgaattttggatttaaacgtggacgttttaaagtggaaaaacaaatttatcaaaagctggaaaaaatgttgattgacaaattgaattatttggttttaaaagacaaacaacctcaggaattaggcggattgtacaacgcattacaactcaccaataaatttgaaagtttccaaaaaatgggtaaacaatcgggctttttgttttatgtacccgcttggaacacctccaaaatagacccaaccacagggtttgtcaattatttttataccaaatatgaaaatgttgacaaagccaaagccttttttgaaaaatttgaggcgattcgtttcaatgcagaaaagaagtattttgaatttgaagtaaaaaaatatagcgattttaacccaaaagccgaaggcactcaacaagcctggaccatttgcacgtatggcgaacgaatagaaaccaaacgacaaaaagaccaaaacaacaaatttgtaagcactccaattaatctaaccgaaaagatagaagactttttgggtaaaaaccaaattgtttatggtgatggtaattgcatcaaatctcaaattgctagcaaagacgacaaggctttttttgaaaccttattgtattggttcaaaatgactttacaaatgcgaaacagcgaaacaagaacagatatagattatctaatttcgcccgtgatgaatgacaacggaacattttacaacagccgagattatgaaaaattagaaaatccaactttgcccaaagatgccgatgccaacggagcgtatcatattgccaaaaaaggattgatgcttttgaataaaatagaccaagccgacttgacaaaaaaagtggatttatctattagtaacagagattggttgcaatttgtacaaaaaaataaataa

SEQ ID NO: 29 - DNA, 4019 bp, Artificial Sequence
  Description of Artificial Sequence: Synthetic polynucleotide
atggaacaggagtactatttaggactggatatgggaaccggatctgtaggatgggctgttacagattcggaatatcatgtcttgcgtaaacatggaaaagcactatggggagtccgattatttgaaagtgcatcgacagcagaagaacgaagaatgttccgaacatcaagaagaagactagatcgaagaaactggagaattgaaattttacaggaaatttttgcagaggaaataagtaagaaagatccaggatttttcttgcgaatgaaagaaagcaaatattatccagaagataagcgagatatcaatggaaattgtccggaactgccatatgcattatttgttgatgacgattttacagataaagattatcataaaaaatttccgacaatttatcatctcaggaaaatgttgatgaatacagaggagacaccggatatccggttggtgtatctggcaattcatcatatgatgaagcataggggccatttcttgttatctggtgacattaatgagattaaggagttcggaacgacattttcaaaattgttggagaatatcaaaaatgaggaattggattggaatcttgaactgggaaaagaagaatatgctgttgtagaaagtattttaaaagataacatgttaaaccgatccacaaagaaaaccagattaataaaagcattaaaagcaaaatcaatatgtgaaaaggctgtactgaatttattggctggtggaacggtgaaattgagtgatatatttggtcttgaagaattaaatgagacagaaagaccgaagatttcctttgctgataatggatacgatgattatatcggagaagttgaaaatgagctgggagaacaattctatattatagagacggcaaaagcagtgtatgactgggcggtattagttgaaatattgggaaaatatacgtcaatttcagaagcgaaagtagcaacgtatgaaaaacataaatcggatttacaatttttgaaaaagatagttcggaaatatctgacaaaggaggaatataaagatatttttgtaagtacgagtgacaaattgaaaaattactctgcttatataggaatgacgaaaataaatggaaaaaaggttgatttgcagagcaaacggtgcagtaaagaagaattctatgattttattaagaaaaacgtacttaaaaagctagaaggacaacctgaatatgaatatttgaaagaagagctagaaagagaaacatttctaccaaaacaggtgaacagggataatggtgtaataccgtatcagattcatttgtacgagttgaaaaagatattaggaaatttacgggataaaatagacctcattaaagagaacgaagataaactggttcaattatttgaattcagaattccgtattatgttggtccgctgaataagatagatgacggaaaagagggaaaatttacatgggctgtacggaaaagtaatgaaaagatatatccatggaattttgaaaatgtagttgatatagaagcaagtgcagaaaaatttatccggagaatgacaaataagtgtacatatctgatgggcgaagatgtattgccgaaggattcattgctttacagtaaatatatggttttaaatgaattaaataatgtaaagttggatggcgaaaaattatctgtagaattgaaacaacggttgtatacagatgtattttgtaagtatcggaaagtaactgtaaagaagataaaaaattacttgaaatgtgaaggtatcatatccggcaatgtcgaaataactggaattgatggtgattttaaggcatcgttaacggcatatcatgattttaaagaaatcttgacaggaacagaattggctaaaaaggacaaagaaaatattattaccaatatagtattgtttggagatgataaaaagctgctgaaaaagagactgaatcgattatatcctcagattacgccgaatcagttgaagaaaatatgtgcgctatcctatacaggctggggaagattttctaaaaagttcttagaagaaataacagctccagatccggaaacgggagaggtatggaatatcattacggcattgtgggaatcgaataataatctgatgcaattattaagtaatgaatatcggtttatggaagaagtcgaaacatacaatatgggaaaacagactaaaacattgtcgtacgaaacagtagagaatatgtatgtttctccatctgtgaaaagacagatatggcagacgctgaaaatcgtgaaagaattagaaaaagtaatgaaagaatctccgaaacgtgtatttattgagatggcgagagaaaagcaagaaagtaagagaaccgaatcgcgtaaaaaacaactaatagatttgtataaggcttgtaaaaatgaagaaaaagattgggtaaaagaactgggagatcaggaagaacagaaattacgaagcgataagttgtacctatattatacgcaaaagggtcgttgtatgtattctggcgaggtaatagaactgaaagacttatgggataatacaaaatatgatattgatcatatatatccacaatctaaaacgatggatgacagtcttaataatcgcgtattggtaaaaaagaaatataatgcaacaaaatcagataagtatccattaaatgaaaatatacgacatgagagaaaaggcttttggaagtcactgttagatggagggtttataagtaaagaaaaatatgaacgcttaataagaaatacagaattgagtccggaagaattagcaggatttattgaaaggcagattgttgaaacgaggcagagtacaaaagctgtagcggaaatattaaagcaagtgtttccggaaagtgaaattgtatatgtcaaagcaggtacggtttcaagattcagaaaagattttgaattactgaaagttcgagaagtgaatgatttgcatcacgcaaaggatgcgtatttaaatattgtagttggtaatagttattatgtgaaatttactaagaatgcatcatggtttataaaagaaaatccgggacgtacttacaacttaaaaaagatgtttacatcaggttggaatattgaacgaaatggagaagttgcatgggaagtcgggaaaaaaggaacaattgtaacggtaaaacaaataatgaataaaaataatatattggtgacaagacaggttcatgaagcgaaaggtgggctgtttgatcagcagattatgaaaaaaggaaaaggtcagattgctataaaggaaactgatgaacgtcttgcatcaatagaaaagtatggaggctataataaagctgccggggcatattttatgctggtagaatctaaagataaaaaaggaaaaacaattcgaacgatagaatttataccattatatttaaagaataaaatcgagtcggatgaatcaatagcattgaactttttagaaaaaggcagaggtttgaaagaaccaaagatactattgaaaaaaattaagattgatacattatttgatgtggacggattcaaaatgtggttgtctggaagaacaggggacagactactatttaaatgtgcaaatcaattgattttggatgagaaaataattgtaacaatgaaaaaaattgtaaagtttattcaaaggagacaagaaaatagagaattaaaattatctgataaagatggaattgataatgaagtacttatggaaatatataacacttttgtggataagttagaaaacacagtgtatagaatacgattatccgaacaggcaaaaacgcttatagataaacaaaaagaatttgaaaggttatcactagaggataaaagtagtactttgtttgaaattttacatatttttcagtgtcaaagtagtgcggccaatttaaaaatgataggcggacctggaaaagcaggaatattagttatgaataataatataagtaagtgtaacaaaatttctattataaatcagtctccaacaggaattttcgaaaatgagattgatttgttaaagat

SEQ ID NO: 30 - DNA, 3858 bp, Artificial Sequence
  Description of Artificial Sequence: Synthetic polynucleotide
atgaaatctttcgattcattcacaaatctttattctctttcaaaaaccttgaaatttgagatgagacctgtcggaaatacccaaaaaatgctcgacaatgcaggagtatttgaaaaagacaaactaattcaaaaaaagtacggaaaaacaaagccgtatttcgacagactccacagagaatttatagaagaagcgctcacgggggtagagctaataggactagatgagaactttaggacacttgttgactggcaaaaagataagaaaaataatgtcgcaatgaaagcgtatgaaaatagtttgcagcggctgagaacggaaataggtaaaatatttaacctaaaggctgaggattgggtaaagaacaaatatccaatattagggctgaaaaataaaaataccgatattttattcgaagaggctgtattcgggatattgaaagcccgatatggagaagaaaaagatacttttatagaagtagaggaaatagataaaaccggcaaatcaaagatcaatcaaatatcaattttcgatagttggaaaggatttacaggatatttcaaaaaattttttgaaaccagaaagaatttttacaaaaacgacggaacttctacagcaattgctacaaggatcattgatcaaaatctgaaaagattcatagataatctgtcaatagttgaaagtgtgagacaaaaggttgatctcgccgagacagaaaaatctttcagcatatctctatcgcaattcttctcaatagacttttataacaagtgtctccttcaagatggtattgattactacaacaagataatcggtggagaaactctcaaaaatggcgaaaaactaataggtctcaatgaactaataaatcaatataggcagaataataaggatcagaaaatcccatttttcaaacttcttgataaacaaattttgagtgaaaagatattatttttggatgaaataaaaaatgacacagaactgatcgaggcgctgagtcagttcgcaaaaacagccgaagaaaaaacaaaaattgtcaaaaagctttttgccgattttgtagaaaataattccaaatacgatcttgcacagatttatatttcccaagaagcattcaatactatatcaaacaagtggacaagcgaaactgagacgttcgctaaatatctattcgaagcaatgaagagtggaaaacttgcaaagtatgagaaaaaagataatagctataaatttcctgattttattgccctttcacagatgaagagtgctttattaagtatcagccttgagggacatttttggaaagagaaatactacaaaatttcaaaattccaagagaagaccaattgggagcagtttcttgcaatttttctatacgagtttaactctcttttcagcgacaaaataaatacaaaagatggagaaacaaagcaagttggatactatctatttgccaaagacctgcataatcttatcttaagtgagcagattgatattccaaaagattcaaaagtcacaataaaagattttgccgattctgtactcacaatctaccaaatggcaaaatattttgcggtagaaaaaaaacgagcgtggcttgccgagtatgaactagattcattttatacccagccagacacaggctatttacagttttatgataacgcctacgaggatattgtgcaggtatacaacaagcttcgaaactatctgaccaaaaagccatatagcgaggagaaatggaagttgaattttgaaaattctacgctggcaaatggatgggataagaacaaagaatctgataattcagcagttattctacaaaaaggtggaaaatattatttgggactgattactaaaggacacaacaaaatttttgatgaccgttttcaagaaaaatttattgtgggaattgaaggtggaaaatatgaaaaaatagtctataaatttttccccgaccaggcaaaaatgtttcccaaagtgtgcttttctgcaaaaggactcgaattttttagaccgtctgaagaaattttaagaatttataacaatgcagagtttaaaaaaggagaaacttattcaatagatagtatgcagaagttgattgatttttataaagattgcttgactaaatatgaaggctgggcatgttatacctttcggcatctaaaacccacagaagaataccaaaacaatattggagagttttttcgagatgttgcagaggacggatacaggattgattttcaaggcatttcagatcaatatattcatgaaaaaaacgagaaaggcgaacttcacctttttgaaatccacaataaagattggaatttggataaggcacgagacggaaagtcaaaaacaacacaaaaaaaccttcatacactctatttcgaatcgctcttttcaaacgataatgttgttcaaaactttccaataaaactcaatggtcaagctgaaattttttatagaccgaaaacggaaaaagacaaattagaatcaaaaaaagataagaaagggaataaagtgattgaccataaacgctatagtgagaataagattttttttcatgttcctctcacactaaaccgcactaaaaatgactcatatcgctttaatgctcaaatcaacaactttctcgcaaataataaagatatcaacatcatcggtgtagataggggagaaaagcatttagtctattattcggtgattacacaagctagtgacatcttagaaagtggctcactaaatgagctaaatggcgtgaattatgctgaaaaactgggaaaaaaggcagaaaatcgagaacaagcacgcagagactggcaagacgtacaagggatcaaagacctcaagaaaggatatatttcacaggtggtgcgaaagcttgctgatttagcaattaaacacaatgccattatcattcttgaagatttgaatatgagatttaaacaagttcggggcggtatcgaaaaatccatttatcaacagttagaaaaagcactgatagataaattaagctttcttgtagacaaaggtgaaaaaaatcccgagcaagcaggacatcttctgaaagcatatcagctttcggccccatttgagacatttcaaaaaatgggcaaacagacgggtataatcttttatacacaagcttcgtatacctcaaaaagtgaccctgtaacaggttggcgaccacacctgtatctcaaatatttcagtgccaaaaaagcaaaagacgatattgcaaagtttacaaaaatagaatttgtaaacgataggtttgagcttacctatgatataaaggactttcagcaagcaaaagaatatccaaataaaactgtttggaaagtttgctcaaatgtagagagattcaggtgggacaaaaacctcaatcaaaacaaaggcggatatactcactacacaaatataactgagaatatccaagagctttttacaaaatatggaattgatatcacaaaagatttgctcacacagatttctacaattgatgaaaaacaaaatacctcattttttagagattttattttttatttcaaccttatttgccaaatcagaaataccgatgattctgagattgctaaaaagaatgggaaagatgattttatactgtcacctgttgagccgtttttcgatagccgaaaagacaatggaaataaacttcctgagaatggagatgataacggcgcgtataacatagcaagaaaagggattgtcatactcaacaaaatctcacaatattcagagaaaaacgaaaattgcgagaaaatgaaatggggggatttgtatgtatcaaacattgactgggacaattttgtaacccaagctaatgcacggcattaa

SEQ ID NO: 31 - DNA, 3516 bp, Artificial Sequence
  Description of Artificial Sequence: Synthetic polynucleotide
atgattatcttatatattagtacctcgaatatgaacatggaaggagtatttatggaaaattttaaaaacttgtatccaataaacaaaacacttcgatttgaattaagaccctatggaaaaacattggaaaattttaaaaaatccggacttttagaaaaagatgcctttaaggcaaatagtagacgaagtatgcaagctataatcgatgaaaaattcaaagagactatcgaagaacgcttaaagtacactgaattcagtgaatgtgatcttggaaacatgacatcaaaagataaaaaaataactgataaagcagctacaaatttaaaaaagcaagttatcttatcttttgacgatgaaatatttaataattacctaaaacctgataaaaatattgacgcattatttaaaaatgatccttcaaatcctgtaatctctacatttaaaggttttacgacatattttgtgaatttttttgaaattcgaaaacatattttcaagggagaatcatcaggctcaatggcataccgaattatagatgaaaacctgacaacatacttgaataatattgaaaaaataaaaaaactgccagaagaattaaaatcacagctagaaggcattgatcagattgataaacttaataattataatgagttcattacacagtcaggtataacacactataatgaaatcatcggcggtatatcaaaatcagagaatgtcaaaatacagggaattaatgaaggaattaatctatactgtcagaagaacaaagttaaacttcctcgactgactccgctatacaaaatgatattatcagacagagtttccaactcttttgtattagacactattgaaaatgacacagaattaattgaaatgataagtgatttgattaataagactgagatttcgcaagatgttataatgtcagatattcaaaatattttcataaaatacaaacaacttggtaatttgccgggtatctcatattcttcaatagttaatgctatttgctcggattatgacaacaatttcggagatgggaagcgaaaaaaatcttacgaaaatgatcgcaaaaagcatttggagactaatgtatactccataaattatatttctgaattgcttacagataccgatgtttcatcaaatatcaagatgagatataaagagcttgagcaaaattatcaggtttgcaaagaaaattttaatgccacaaactggatgaatattaaaaatataaaacaatctgaaaaaacaaaccttattaaagatttgttagatatacttaaatcgattcaacgtttctatgatttgtttgatattgttgacgaagataaaaatccaagtgctgaattttatacctggttatcaaaaaatgctgaaaagcttgactttgaattcaattctgtatataacaagtcacgaaactatctcaccaggaaacaatactctgataaaaaaatcaagctgaattttgattctccaacattggccaaagggtgggatgctaacaaagaaatagataactccacgattataatgcgtaaatttaataatgacagaggcgattatgattacttccttggcatatggaataaatccacacctgcaaatgaaaaaataatcccactggaggataatggattattcgaaaaaatgcaatataagctgtatccagatcctagtaagatgttaccgaaacaatttctatcaaaaatatggaaggcaaagcatcctacgacacctgaatttgataaaaaatataaagagggaagacataaaaaaggtcctgatttcgaaaaagaattcctgcatgaattgattgattgcttcaaacatggtcttgttaatcacgatgaaaaatatcaggatgtttttggcttcaatctccgtaacactgaagattataattcatatacagagtttctcgaagatgtggaaagatgcaattacaatctttcatttaacaaaattgctgatacttcaaaccttattaatgatgggaaattgtatgtatttcagatatggtcaaaagacttttctattgattcaaaaggtactaaaaacttgaatacaatctattttgaatcactattttcagaagaaaacatgatagaaaaaatgttcaagctttctggagaggctgagatattctatcgaccagcatcgttgaattattgtgaagatatcataaaaaaaggtcatcaccatgcagaattaaaagataagtttgactatcctataataaaagataagcgatattcacaagataagtttttctttcatgtgccaatggttataaattataaatctgagaaactgaattccaaaagccttaacaaccgaacaaatgaaaacctgggacagtttacacatattataggtatagacaggggcgagcggcacttgatttatttaactgttgttgatgtttccactggtgaaatcgttgaacagaaacatctggacgaaattatcaatactgataccaagggagttgaacacaaaacccattatttgaataaattggaagaaaaatctaaaacaagagataacgagcgtaaatcatgggaagctattgaaactatcaaagaattaaaagaaggctatatttctcatgtaattaatgaaatacaaaagctgcaagaaaaatataatgccttaatcgtaatggaaaatcttaactatgggttcaaaaactcacgaatcaaagttgaaaaacaggtttatcaaaaattcgagacagcattgattaaaaagttcaattatattattgataaaaaagatccagaaacctatatacatggttaccagcttacaaatcctattaccactctggataagattggaaatcaatctggaatagtgctgtatattcctgcgtggaatacttctaagatagatcccgtcacaggatttgtaaaccttctgtacgcagatgatttgaagtataaaaatcaggagcaggccaaatcattcattcagaaaatagacaacatatattttgaaaatggagagtttaaatttgatattgatttttccaaatggaataatcgctactcaataagtaaaactaaatggacgttaacaagttatgggactcgcatccagacatttagaaatccccagaaaaacaataagtgggattctgctgaatatgatttgacagaagagtttaaattaattttaaatatagacggaacgttaaagtcacaggacgtagaaacatacaaaaaattcatgtctttatttaaactaatgctacagcttcgaaactctgttacaggaaccgacattgattatatgatctctcctgtcactgataaaacaggaacacatttcgattcaagagaaaatattaaaaatcttcctgccgatgcagatgccaatggtgcctacaacattgcgcgcaaaggaataatggctattgaaaatataatgaacggtataagcgatccactaaaaataagcaacgaagactatttaaagtatattcagaatcaacaggaataa

SEQ ID NO: 32 - DNA, 3924 bp, Artificial Sequence
  Description of Artificial Sequence: Synthetic polynucleotide
atgacccaatttgaaggttttaccaatttataccaagtttcgaagacccttcgttttgaactgattccccaaggaaaaacactcaaacatatccaggagcaagggttcattgaggaggataaagctcgcaatgaccattacaaagagttaaaaccaatcattgaccgcatctataagacttatgctgatcaatgtctccaactggtacagcttgactgggagaatctatctgcagccatagactcctatcgtaaggaaaaaaccgaagaaacacgaaatgcgctgattgaggagcaagcaacatatagaaatgcgattcatgactactttataggtcggacggataatctgacagatgccataaataagcgccatgctgaaatctataaaggactttttaaagctgaacttttcaatggaaaagttttaaagcaattagggaccgtaaccacgacagaacatgaaaatgctctactccgttcgtttgacaaatttacgacctatttttccggcttttatgaaaaccgaaaaaatgtctttagcgctgaagatatcagcacggcaattccccatcgaatcgtccaggacaatttccctaaatttaaggaaaactgccatatttttacaagattgataaccgcagttccttctttgcgggagcattttgaaaatgtcaaaaaggccattggaatctttgttagtacgtctattgaagaagtcttttcctttcccttttataatcaacttctaacccaaacgcaaattgatctttataatcaacttctcggcggcatatctagggaagcaggcacagaaaaaatcaagggacttaatgaagttctcaatctggctatccaaaaaaatgatgaaacagcccatataatcgcgtccctgccgcatcgttttattcctctttttaaacaaattctttccgatcgaaatacgttatcctttattttggaagaattcaaaagcgatgaggaagtcatccaatccttctgcaaatataaaaccctcttgagaaacgaaaatgtactggagactgcagaagcccttttcaatgaattaaattccattgatttgactcatatctttatttcccataaaaagttagaaaccatctcttcagcgctttgtgaccattgggataccttgcgcaatgcactttacgaaagacggatttctgaactcactggcaaaataacaaaaagtgccaaagaaaaagttcaaaggtcattaaaacatgaggatataaatctccaagaaattatttctgctgcaggaaaagaactatcagaagcattcaaacaaaaaacaagtgaaattctttcccatgcccatgctgcacttgaccagcctcttcccacaacattaaaaaaacaggaagaaaaagaaatcctcaaatcacagctcgattcgcttttaggcctttatcatcttcttgattggtttgctgtcgatgaaagcaatgaagtcgacccagaattctcagcacggctgacaggcattaaactagaaatggaaccaagcctttcgttttataataaagcaagaaattatgcgacaaaaaagccctattcggtggaaaaatttaaattgaattttcaaatgccaacccttgcctctggttgggatgtcaataaagaaaaaaataatggagctattttattcgtaaaaaatggtctctattaccttggtatcatgcctaaacagaaggggcgctataaagccctgtcttttgagccgacagaaaaaacatcagaaggattcgataagatgtactatgactacttcccagatgccgcaaaaatgattcctaagtgttccactcagctaaaggctgtaaccgctcattttcaaactcataccacccccattcttctctcaaataatttcattgaacctcttgaaatcacaaaagaaatttatgacctgaacaatcctgaaaaggagcctaaaaagtttcaaacggcttatgcaaagaagacaggcgatcaaaaaggctatagagaagcgctttgcaaatggattgactttacgcgggattttctctctaaatatacgaaaacaacttcaatcgatttatcttcactccgcccttcttcgcaatataaagatttaggggaatattacgccgaactgaatccgcttctctatcatatctccttccaacgaattgctgaaaaggaaatcatggatgctgtagaaacgggaaaattgtatctgttccaaatctacaataaggattttgcgaagggccatcacgggaaaccaaatctccacaccctgtattggacaggtctcttcagtcctgaaaaccttgcgaaaaccagcatcaaacttaatggtcaagcagaattgttctatcgacctaaaagccgcatgaagcggatggcccatcgtcttggggaaaaaatgctgaacaaaaaactaaaggaccagaagacaccgattccagataccctctaccaagaactgtacgattatgtcaaccaccggctaagccatgatctttccgatgaagcaagggccctgcttccaaatgttatcaccaaagaagtctcccatgaaattataaaggatcggcggtttacttccgataaatttttcttccatgttcccattacactgaattatcaagcagccaatagtcccagtaaattcaaccagcgtgtcaatgcctaccttaaggagcatccggaaacgcccatcattggtatcgatcgtggagaacgcaatctaatctatattaccgtcattgacagtactgggaaaattttggagcagcgttccctgaataccatccagcaatttgactaccaaaaaaaattggacaacagggaaaaagagcgtgttgccgcccgtcaagcctggtccgtcgtcggaacgatcaaagaccttaaacaaggctacttgtcacaggtcatccatgaaattgtagacctgatgattcattaccaagctgttgtcgtccttgaaaacctcaacttcggatttaaatcaaaacggacaggcattgccgaaaaagcagtctaccaacaatttgaaaagatgctaatagataaactcaactgtttggttctcaaagattatcctgctgagaaagtgggaggcgtcttaaacccgtatcaacttacagatcagttcacgagctttgcaaaaatgggcacgcaaagcggcttccttttctatgtaccggccccttatacctcaaagattgatcccctgactggttttgtcgatccctttgtatggaagaccattaaaaatcatgaaagtcggaagcatttcctagaaggatttgatttcctgcattatgatgtcaaaacaggtgattttatcctccattttaaaatgaatcggaatctctctttccagagagggcttcctggcttcatgccagcttgggatattgttttcgaaaagaatgaaacccaatttgatgcaaaagggacgcccttcattgcaggaaaacgaattgttcctgtaatcgaaaatcatcgttttacgggtcgttacagagacctctatcccgctaatgaactcattgcccttctggaagaaaaaggcattgtctttagagacggaagtaatatattacccaaacttttagaaaatgatgattctcatgcaattgatacgatggtcgccttgattcgcagtgtactccaaatgagaaacagcaatgccgcaacgggggaagactacatcaactctcccgttagggatctgaacggggtgtgtttcgacagtcgattccaaaatccagaatggccaatggatgcggatgccaacggagcttatcatattgccttaaaagggcagcttcttctgaaccacctcaaagaaagcaaagatctgaaattacaaaacggcatcagcaaccaagattggctggcctacattcaggaactgagaaactga

SEQ ID NO: 33 - DNA, 3390 bp, Artificial Sequence
  Description of Artificial Sequence: Synthetic polynucleotide
atggccgtcaaatccatcaaagtgaaacttcgtctcgacgatatgccggagattcgggccggtctatggaaacttcataaggaagtcaatgcgggggttcgatattacacggaatggctcagtcttctccgtcaagagaacttgtatcgaagaagtccgaatggggacggagagcaagaatgtgataagactgcagaagaatgcaaagccgaattgttggagcggctgcgcgcgcgtcaagtggagaatggacaccgtggtccggcgggatcggacgatgaattgctgcagttggcgcgtcaactctatgagttgttggttccgcaggcgataggtgcgaaaggcgacgcgcagcaaattgcccgcaaatttttgagccccttggccgacaaggacgcagttggtgggcttggaatcgcgaaggcggggaacaaaccgcggtgggttcgcatgcgcgaagcgggggaaccaggctgggaagaggagaaggagaaggctgagacgaggaaatctgcggatcggactgcggatgttttgcgcgcgctcgcggattttgggttaaagccactgatgcgcgtatacaccgattctgagatgtcatcggtggagtggaaaccgcttcggaagggacaagccgttcggacgtgggatagggacatgttccaacaagctatcgaacggatgatgtcgtgggagtcgtggaatcagcgcgttgggcaagagtacgcgaaactcgtagaacaaaaaaatcgatttgagcagaagaatttcgtcggccaggaacatctggtccatctcgtcaatcagttgcaacaagatatgaaagaagcatcgcccggactcgaatcgaaagagcaaaccgcgcactatgtgacgggacgggcattgcgcggatcggacaaggtatttgagaagtgggggaaactcgcccccgatgcacctttcgatttgtacgacgccgaaatcaagaatgtgcagagacgtaacacgagacgattcggatcacatgacttgttcgcaaaattggcagagccagagtatcaggccctgtggcgcgaagatgcttcgtttctcacgcgttacgcggtgtacaacagcatccttcgcaaactgaatcacgccaaaatgttcgcgacgtttactttgccggatgcaacggcgcacccgatttggactcgcttcgataaattgggtgggaatttgcaccagtacacctttttgttcaacgaatttggagaacgcaggcacgcgattcgttttcacaagctattgaaagtcgagaatggtgtcgcaagagaagttgatgatgtcaccgtgcccatttcaatgtcagagcaattggataatctgcttcccagagatcccaatgaaccgattgcgctatattttcgagattacggagccgaacagcatttcacaggtgaatttggtggcgcgaagatccagtgccgccgggatcagctggctcatatgcaccgacgcagaggggcgagggatgtttatctcaatgtcagcgtacgtgtgcagagtcagtctgaggcgcggggagaacgtcgcccgccgtatgcggcagtatttcgtctggtcggggacaaccatcgcgcgtttgtccatttcgataaactatcggattatcttgcggaacatccggatgatgggaagctcgggtcggaggggttgctttccgggctgcgggtgatgagtgtcgatctcggccttcgcacatctgcatcgatttccgtttttcgcgttgcccggaaggacgagttgaagccgaactcaaaaggtcgtgtaccgtttttctttccgataaaagggaatgacaatctcgtcgcggttcatgagcgatcacaactcttgaagctgcctggcgaaacggagtcgaaggacctgcgtgctatccgagaagaacgccaacggacattgcggcagttgcggacgcaactggcgtatttgcggctgctcgtgcggtgtgggtcggaagatgtggggcggcgtgaacggagttgggcaaagcttatcgagcagccggtggatgcggccaatcacatgacaccggattggcgcgaggcttttgaaaacgaacttcagaagcttaagtcactccatggtatctgtagcgacaaggaatggatggatgctgtctacgagagcgttcgccgcgtgtggcgtcacatgggcaaacaggttcgcgattggcgaaaggacgtacgaagcggagagcggcccaagattcgcggctatgcgaaagacgtggtcggtggaaactcgattgagcaaatcgagtatctggaacgtcagtacaagttcctcaagagttggagcttctttggtaaggtgtcgggacaagtgattcgtgcggagaagggatctcgttttgcgatcacgctgcgcgaacacattgatcacgcgaaggaagatcggctgaagaaattggcggatcgcatcattatggaggctctcggctatgtgtacgcgttggatgagcgcggcaaaggaaagtgggttgcgaagtatccgccgtgccagctcatcctgctggaggaattgagcgagtaccagttcaataacgacaggcctccgagcgaaaacaaccagttgatgcaatggagtcatcgcggcgtgttccaggagttgataaatcaggcccaagtccatgatttactcgttgggacgatgtatgcagcgttctcgtcgcgattcgacgcgcgaactggggcaccgggtatccgctgtcgccgggttccggcgcgttgcacccaggagcacaatccagaaccatttccttggtggctgaacaagtttgtggtggaacatacgttggatgcttgtcccctacgcgcagacgacctcatcccaacgggtgaaggagagatttttgtctcgccgttcagcgcggaggagggggactttcatcagattcacgccgacctgaatgcggcgcaaaatctgcagcagcgactctggtctgattttgatatcagtcaaattcggttgcggtgtgattggggtgaagtggacggtgaactcgttctgatcccaaggcttacaggaaaacgaacggcggattcatatagcaacaaggtgttttataccaatacaggtgtcacctattatgagcgagagcgggggaagaagcggagaaaggttttcgcgcaagagaaattgtcggaggaagaggcggagttgctcgtggaagcagacgaggcgagggagaaatcggtcgttttgatgcgtgatccgtctggcatcatcaatcggggaaattggaccaggcaaaaggaattttggtcgatggtgaaccagcggatcgaaggatacttggtcaagcagattcgctcgcgcgttccattacaagatagtgcgtgtgaaaacacgggggatatttaa

SEQ ID NO: 34 - DNA, 3327 bp, Artificial Sequence
  Description of Artificial Sequence: Synthetic polynucleotide
atggcgacacgcagttttattttaaaaattgaaccaaatgaagaagttaaaaagggattatggaagacgcatgaggtattgaatcatggaattgcctactacatgaatattctgaaactaattagacaggaagctatttatgaacatcatgaacaagatcctaaaaatccgaaaaaagtttcaaaagcagaaatacaagccgagttatgggattttgttttaaaaatgcaaaaatgtaatagttttacacatgaagttgacaaagatgttgtttttaacatcctgcgtgaactatatgaagagttggtccctagttcagtcgagaaaaagggtgaagccaatcaattatcgaataagtttctgtacccgctagttgatccgaacagtcaaagtgggaaagggacggcatcatccggacgtaaacctcggtggtataatttaaaaatagcaggcgacccatcgtgggaggaagaaaagaaaaaatgggaagaggataaaaagaaagatccccttgctaaaatcttaggtaagttagcagaatatgggcttattccgctatttattccatttactgacagcaacgaaccaattgtaaaagaaattaaatggatggaaaaaagtcgtaatcaaagtgtccggcgacttgataaggatatgtttatccaagcattagagcgttttctttcatgggaaagctggaaccttaaagtaaaggaagagtatgaaaaagttgaaaaggaacacaaaacactagaggaaaggataaaagaggacattcaagcatttaaatcccttgaacaatatgaaaaagaacggcaggagcaacttcttagagatacattgaatacaaatgaataccgattaagcaaaagaggattacgtggttggcgtgaaattatccaaaaatggctaaagatggatgaaaatgaaccatcagaaaaatatttagaagtatttaaagattatcaacggaaacatccacgagaagccggggactattctgtctatgaatttttaagcaagaaagaaaatcattttatttggcgaaatcatcctgaatatccttatttgtatgctacattttgtgaaattgacaaaaaaaagaaagacgctaagcaacaggcaacttttactttggctgacccgattaaccatccgttatgggtacgatttgaagaaagaagcggttcgaacttaaacaaatatcgaattttaacagagcaattacacactgaaaagttaaaaaagaaattaacagttcaacttgatcgtttaatttatccaactgaatccggcggttgggaggaaaaaggtaaagtagatatcgttttgttgccgtcaagacaattttataatcaaatcttccttgatatagaagaaaaggggaaacatgcttttacttataaggatgaaagtattaaattcccccttaaaggtacacttggtggtgcaagagtgcagtttgaccgtgaccatttgcggagatatccgcataaagtagaatcaggaaatgttggacggatttattttaacatgacagtaaatattgaaccaactgagagccctgttagtaagtctttgaaaatacatagggacgatttccccaagttcgttaattttaaaccgaaagagctcaccgaatggataaaagatagtaaagggaaaaaattaaaaagtggtatagaatcccttgaaattggtctacgggtgatgagtatcgacttaggtcaacgtcaagcggctgctgcatcgatttttgaagtagttgatcagaaaccggatattgaagggaagttattttttccaatcaaaggaactgagctttatgctgttcaccgggcaagttttaacattaaattaccgggtgaaacattagtaaaatcacgggaagtattgcggaaagctcgggaggacaacttaaaattaatgaatcaaaagttaaactttctaagaaatgttctacatttccaacagtttgaagatatcacagaaagagagaagcgtgtaactaaatggatttctagacaagaaaatagtgatgttcctcttgtatatcaagatgagctaattcaaattcgtgaattaatgtataaaccctataaagattgggttgcctttttaaaacaactccataaacggctagaagtcgagattggcaaagaggttaagcattggcgaaaatcattaagtgacgggagaaaaggtctttacggaatctccctaaaaaatattgatgaaattgatcgaacaaggaaattccttttaagatggagcttacgtccaacagaacctggggaagtaagacgcttggaaccaggacagcgttttgcgattgatcaattaaaccacctaaatgcattaaaagaagatcgattaaaaaagatggcaaatacgattatcatgcatgccttaggttactgttatgatgtaagaaagaaaaagtggcaggcaaaaaatccagcatgtcaaattattttatttgaagatttatctaactacaatccttacgaggaaaggtcccgttttgaaaactcaaaactgatgaagtggtcacggagagaaattccacgacaagtcgccttacaaggtgaaatttacggattacaagttggggaagtaggtgcccaattcagttcaagattccatgcgaaaaccgggtcgccgggaattcgttgcagtgttgtaacgaaagaaaaattgcaggataatcgcttttttaaaaatttacaaagagaaggacgacttactcttgataaaatcgcagttttaaaagaaggagacttatatccagataaaggtggagaaaagtttatttctttatcaaaggatcgaaagttggtaactacgcatgctgatattaacgcggcccaaaatttacagaagcgtttttggacaagaacacatggattttataaagtttactgcaaagcctatcaggttgatggacaaactgtttatattccggagagcaaggaccaaaaacaaaaaataattgaagaatttggggaaggctattttattttaaaagatggtgtatatgaatggggtaatgcggggaaactaaaaattaaaaaaggttcctctaaacaatcatcgagtgaattagtagattcggacatactgaaagattcatttgatttagcaagtgaacttaagggagagaaactcatgttatatcgagatccgagtggaaacgtatttccttccgacaagtggatggcagcaggagtattttttggcaaattagaaagaatattgatttctaagttaacaaatcaatactcaatatcaacaatagaagatgattcttcaaaacaatcaatgtaa

SEQ ID NO: 35 - DNA, 3450 bp, Artificial Sequence
  Description of Artificial Sequence: Synthetic polynucleotide
atgcccacccgcaccatcaatctgaaacttgttcttgggaaaaatcctgaaaacgcaacattgcgacgcgccctattttcgacacaccgtttggttaaccaagcgacgaaacgtattgaggaattcttgttgctgtgtcgtggagaagcctacagaacagtggataatgaggggaaggaagccgagattccacgtcatgcagtccaagaagaagctcttgcctttgccaaagctgctcaacgccacaacggctgtatatccacctatgaagaccaagagattcttgatgtactgcggcaactgtacgaacgtcttgttccttcggtcaacgaaaacaacgaggcaggcgatgctcaagctgctaacgcctgggtcagtccgctcatgtcggcagaaagcgaaggaggcttgtcggtctacgacaaggtgcttgatccaccgccggtttggatgaagcttaaagaagaaaaggctccaggatgggaagccgcttctcaaatttggattcagagtgatgagggacagtcgttacttaataagccaggtagccctccccgctggattcgaaaactgcgatctgggcaaccgtggcaagatgatttcgtcagtgaccaaaagaaaaagcaagatgagctgaccaaagggaacgcaccacttataaaacaactcaaagaaatggggttgttgcctcttgttaacccattttttagacatcttcttgaccctgaaggtaaaggcgtgagtccatgggaccgtcttgctgtacgcgctgcagtggctcactttatctcctgggaaagttggaatcatagaacacgtgcagaatacaattccttgaaactacggcgagacgagtttgaggcagcatccgacgaattcaaagacgattttactttgctccgacaatatgaagccaaacgccatagtacattgaaaagcatcgcgctggccgacgattcgaacccttaccggattggagtacgttctctgcgtgcctggaaccgcgttcgtgaagaatggatagacaagggtgcaacagaagaacaacgcgtgaccatattgtcaaagcttcaaacacaacttcggggaaaattcggcgatcccgatctgttcaactggctagctcaggataggcatgtccatttgtggtctcctcgggacagcgtgacaccattggttcgcatcaatgcggtagataaagttctgcgtcgacgaaaaccgtatgcattgatgacctttgcccatccccgcttccaccctcgatggatactgtacgaggctccaggaggaagcaatctccgtcaatatgcattggattgtacagaaaacgctctacacatcacgttgcctttgcttgtcgacgatgcgcacggaacctggattgaaaaaaagatcagggtgccgctggcaccatccggacaaattcaagatttaactctggaaaaacttgagaagaaaaaaaatcgtttatactaccgttccggttttcagcagtttgccggcttggctggcggagctgaggttcttttccacagaccctatatggaacacgacgaacgcagcgaggagtctcttttggaacgtccgggagccgtttggttcaaattgaccctggatgtggcaacacaggctcccccgaactggcttgatggtaagggccgtgtccgtacaccgccggaggtacatcattttaaaaccgcattgtcgaataaaagcaaacatacacgtacgctgcagccgggtctccgtgtcttgtcagtagacttgggcatgcgaacattcgcctcctgctcagtatttgaactcatcgagggaaagcctgagacaggccgtgccttccctgttgccgatgagagatcaatggacagcccgaataaactgtgggccaagcatgaacgtagttttaaactgacgctccccggcgaaaccccttctcgaaaggaagaggaagagcgtagcatagcaagagcggaaatttatgcactgaaacgcgacatacaacgcctcaaaagcctactccgcttaggtgaagaagataacgataaccgtcgtgatgcattgcttgaacagttctttaaaggatggggagaagaagacgttgtgcctggacaagcgtttccacgctctcttttccaagggttgggagctgccccgtttcgctcaactccagagttatggcgtcagcattgccaaacatattatgacaaagcggaagcctgtctggctaaacatatcagtgattggcgcaagcgaactcgtccccgtccgacatcgcgggagatgtggtacaaaacacgttcctatcatggcggcaagtccatttggatgttggaatatcttgatgccgttcgaaaactgcttctcagttggagcttacgtggtcgtacttacggtgccattaatcgccaggatacagcccggtttggttctttggcatcacggctgctccaccatatcaattccctaaaggaagaccgcatcaaaacaggagccgactctatcgttcaggctgctcgcgggtatattcctctccctcatggcaagggttgggaacaaagatatgagccttgtcagctcatattatttgaagacctcgcacgatatcgctttcgcgtggatcgacctcgtcgagagaacagccaactcatgcagtggaaccatcgagccatcgtggcagaaacaacgatgcaagccgaactctacggacaaattgtcgaaaatactgcagcggggttcagcagtcgttttcacgcggcgacaggtgcccccggtgtacgttgtcgttttcttctagaaagagactttgataacgatttgcccaaaccgtaccttctcagggaactttcttggatgctcggcaatacaaaagtcgagtctgaagaagaaaagcttcgattgctgtctgaaaaaatcaggccaggcagtcttgttccttgggatggaggcgaacagttcgctaccctgcatcccaaaagacaaacactttgcgtcattcatgccgatatgaatgctgcccaaaatttacaacgccggtttttcggtcgatgcggcgaggcctttcggcttgtttgtcaaccccacggtgacgacgtgttacgactcgcatccaccccaggagctcgtcttcttggagccctgcagcagcttgaaaatggacaaggagctttcgagttggttcgagacatggggtcaacaagtcaaatgaaccggttcgtcatgaagtctttgggaaaaaagaaaataaaaccccttcaggacaacaatggagacgacgagcttgaagacgtgttgtccgtactcccggaggaagacgacacaggacgtatcacagtcttccgcgattcatcaggaatcttttttccttgcaacgtctggataccggccaaacagttttggccagcagtacgcgccatgatttggaaggtcatggcttcccattctttggggtga

SEQ ID NO: 36 - DNA, 3759 bp, Artificial Sequence
  Description of Artificial Sequence: Synthetic polynucleotide
atgacaaagttaagacaccgacagaaaaaattaacacacgactgggctggctccaaaaagagggaagtattaggctcaaatggcaagcttcagaatccgttgttaatgccggttaaaaaaggtcaggttactgagttccggaaagcgttttctgcgtatgctcgcgcaacgaaaggagaaatgactgacggccgaaagaatatgtttacgcatagtttcgagccatttaagacaaagccctcgcttcatcagtgtgaattggcagataaagcatatcaatctttacattcgtatctgcctggttctcttgctcattttctattatctgctcacgcattaggttttcgtattttttcaaaatctggtgaagcaactgcattccaggcatcctctaaaattgaagcttacgaatcaaaattggcaagcgaattagcttgtgtagatttatctattcaaaacttgactatttcaacgctttttaatgcgcttacaacgtctgtaagagggaagggcgaagaaactagcgctgaccccttaattgcacgattttacaccttacttactggcaagcctctgtctcgagacactcaagggcctgaacgtgatttagcagaagttatctcgcgtaagatagctagttcttttggcacatggaaagaaatgacggcaaaccctcttcagtcattacaattttttgaagaggaactccatgcgctggatgccaatgtctcgctctcacccgccttcgacgttttaattaaaatgaatgatttgcagggcgatttaaaaaatcgaaccattgtttttgatcctgacgcccctgtttttgaatataacgcagaagaccctgccgacataattattaaacttacagctcgttacgctaaagaagctgtcatcaaaaatcaaaacgtaggaaattacgttaaaaacgctattactaccacaaatgccaatggtcttggttggcttttgaacaaaggtttgtcgttactccctgtctcgaccgatgacgaattgctagagtttattggcgttgaacgatctcatccctcatgccatgccttaattgaattgattgcacaattagaagcccccgagctctttgagaagaacgtattttcagatactcgttctgaagttcaaggtatgattgattcagctgtttctaatcatattgctcgtctttccagctctagaaatagcttgtcaatggatagtgaagaattagaacgtttaatcaaaagctttcagatacacacacctcattgctcactttttattggcgcccaatcactttcacagcagttagaatctttgcctgaagcccttcaatcgggcgttaattcagccgatattttactaggctctactcaatatatgctcaccaattctttggttgaagagtcaattgcaacttatcaaagaacacttaatcgcatcaattacttgtcaggtgttgcaggtcagattaacggcgcaataaagcgaaaagcgatagatggagaaaaaattcacttgcctgcagcttggtcagagttgatatctttaccatttataggccagcctgttatagatgttgaaagcgatttagctcatctaaaaaatcaataccaaacactttcaaatgagtttgatactcttatatctgctttgcaaaagaattttgatttgaactttaataaagcgctccttaatcgtactcagcattttgaagccatgtgtagaagcactaagaaaaacgctttatccaaaccagagatcgtttcctatcgcgacctgcttgctcgattaacttcttgtttgtatcgaggctctttagttttgcgtcgtgccggcattgaagtgttaaaaaaacataaaatatttgagtcaaacagcgaacttcgtgaacatgttcatgaaagaaagcatttcgtgtttgttagtcctctagatcgcaaagccaagaaactccttcgattaactgattcgcgtccagacttgttacatgttattgatgaaatattgcagcacgataatcttgaaaacaaagaccgcgagtcactttggctagttcgctctggttatttgcttgcaggacttccagatcaactttcttcatcttttattaacttgcctatcattactcaaaaaggagatagacgccttatagacctgattcagtatgatcaaattaatcgtgatgcttttgttatgttagtgacctctgcattcaagtctaatttgtctggtctgcagtatcgtgccaataagcaatcgttcgttgttactcgcacgctaagcccttatctcggctcaaaacttgtctacgtacccaaggataaagattggttagttccttctcaaatgtttgaaggacgatttgctgacattcttcaatcagattatatggtctggaaagatgccggtcgtctttgtgttattgatactgcaaaacacctttctaatataaagaagtctgtattttcatccgaagaagttctcgcttttttaagagaactccctcaccgcacatttatccagaccgaagttcgcggccttggcgttaatgtcgatggaattgcatttaataatggtgatattccgtcattaaaaaccttttcaaattgcgttcaggtaaaagtttctcggactaatacatccctagttcaaacacttaatcgttggtttgaaggaggaaaagtttctcctccgagcattcaatttgaacgggcgtattataaaaaagacgatcaaattcatgaagacgcagcgaaaagaaagatacgattccagatgcccgcaactgagttggttcatgcttctgacgatgcggggtggacaccaagttatttgctcggcattgatcctggcgagtatggaatgggtctttcattggtttcgattaataacggagaagtcttagattcaggctttattcatattaattctctgatcaattttgcctctaaaaagagcaaccatcaaactaaggttgttccgcgtcagcagtacaaatctccttatgcaaattatttagaacaatctaaagattctgctgctggtgatattgcgcatatactcgatcgacttatatacaaattaaatgcgttgcctgtttttgaggctctttcaggtaattctcagagtgctgctgatcaagtttggacgaaagtcttatcgttttacacttggggtgataatgacgctcagaattctattagaaagcagcattggtttggagccagtcattgggatatcaaaggtatgttaaggcaaccccctacggagaagaagcctaaaccgtatattgcttttcctggctctcaggtttcttcgtatggtaattcccaacgttgctcttgctgcggtcgcaatcctattgaacaacttcgagaaatggcaaaggatacctctattaaagagctaaaaattcgcaattctgagatacagctttttgacggaaccattaaattatttaatccagacccatccactgtgatagagagaaggcgacataatcttggtccatcaagaattcctgttgctgaccgtactttcaaaaacatcagtccatcaagtctagaatttaaagaattgattactatcgtgtctcgatctatccgtcattcacctgagtttatcgctaaaaaacgcggcatagggtctgagtatttttgcgcttattccgattgcaactcatccttaaattctgaagctaacgcagctgctaacgtagcgcaaaaatttcaaaaacagttattttttgagttataa

SEQ ID NO: 37 - DNA, 3864 bp, Artificial Sequence
  Description of Artificial Sequence: Synthetic polynucleotide
atgaagagaattctgaacagtctgaaagttgctgccttgagacttctgtttcgaggcaaaggttctgaattagtgaagacagtcaaatatccattggtttccccggttcaaggcgcggttgaagaacttgctgaagcaattcggcacgacaacctgcacctttttgggcagaaggaaatagtggatcttatggagaaagacgaaggaacccaggtgtattcggttgtggatttttggttggataccctgcgtttagggatgtttttctcaccatcagcgaatgcgttgaaaatcacgctgggaaaattcaattctgatcaggtttcaccttttcgtaaggttttggagcagtcacctttttttcttgcgggtcgcttgaaggttgaacctgcggaaaggatactttctgttgaaatcagaaagattggtaaaagagaaaacagagttgagaactatgccgccgatgtggagacatgcttcattggtcagctttcttcagatgagaaacagagtatccagaagctggcaaatgatatctgggatagcaaggatcatgaggaacagagaatgttgaaggcggatttttttgctatacctcttataaaagaccccaaagctgtcacagaagaagatcctgaaaatgaaacggcgggaaaacagaaaccgcttgaattatgtgtttgtcttgttcctgagttgtatacccgaggtttcggctccattgctgattttctggttcagcgacttaccttgctgcgtgacaaaatgagtaccgacacggcggaagattgcctcgagtatgttggcattgaggaagaaaaaggcaatggaatgaattccttgctcggcacttttttgaagaacctgcagggtgatggttttgaacagatttttcagtttatgcttgggtcttatgttggctggcaggggaaggaagatgtactgcgcgaacgattggatttgctggccgaaaaagtcaaaagattaccaaagccaaaatttgccggagaatggagtggtcatcgtatgtttctccatggtcagctgaaaagctggtcgtcgaatttcttccgtctttttaatgagacgcgggaacttctggaaagtatcaagagtgatattcaacatgccaccatgctcattagctatgtggaagagaaaggaggctatcatccacagctgttgagtcagtatcggaagttaatggaacaattaccggcgttgcggactaaggttttggatcctgagattgagatgacgcatatgtccgaggctgttcgaagttacattatgatacacaagtctgtagcgggatttctgccggatttactcgagtctttggatcgagataaggatagggaatttttgctttccatctttcctcgtattccaaagatagataagaagacgaaagagatcgttgcatgggagctaccgggcgagccagaggaaggctatttgttcacagcaaacaaccttttccggaattttcttgagaatccgaaacatgtgccacgatttatggcagagaggattcccgaggattggacgcgtttgcgctcggcccctgtgtggtttgatgggatggtgaagcaatggcagaaggtggtgaatcagttggttgaatctccaggcgccctttatcagttcaatgaaagttttttgcgtcaaagactgcaagcaatgcttacggtctataagcgggatctccagactgagaagtttctgaagctgctggctgatgtctgtcgtccactcgttgattttttcggacttggaggaaatgatattatcttcaagtcatgtcaggatccaagaaagcaatggcagactgttattccactcagtgtcccagcggatgtttatacagcatgtgaaggcttggctattcgtctccgcgaaactcttggattcgaatggaaaaatctgaaaggacacgagcgggaagattttttacggctgcatcagttgctgggaaatctgctgttctggatcagggatgcgaaacttgtcgtgaagctggaagactggatgaacaatccttgtgttcaggagtatgtggaagcacgaaaagccattgatcttcccttggagattttcggatttgaggtgccgatttttctcaatggctatctcttttcggaactgcgccagctggaattgttgctgaggcgtaagtcggtgatgacgtcttacagcgtcaaaacgacaggctcgccaaataggctcttccagttggtttacctacctctaaacccttcagatccggaaaagaaaaattccaacaactttcaggagcgcctcgatacacctaccggtttgtcgcgtcgttttctggatcttacgctggatgcatttgctggcaaactcttgacggatccggtaactcaggaactgaagacgatggccggtttttacgatcatctctttggcttcaagttgccgtgtaaactggcggcgatgagtaaccatccaggatcctcttccaaaatggtggttctggcaaaaccaaagaagggtgttgctagtaacatcggctttgaacctattcccgatcctgctcatcctgtgttccgggtgagaagttcctggccggagttgaagtacctggaggggttgttgtatcttcccgaagatacaccactgaccattgaactggcggaaacgtcggtcagttgtcagtctgtgagttcagtcgctttcgatttgaagaatctgacgactatcttgggtcgtgttggtgaattcagggtgacggcagatcaacctttcaagctgacgcccattattcctgagaaagaggaatccttcatcgggaagacctacctcggtcttgatgctggagagcgatctggcgttggtttcgcgattgtgacggttgacggcgatgggtatgaggtgcagaggttgggtgtgcatgaagatactcagcttatggcgcttcagcaagtcgccagcaagtctcttaaggagccggttttccagccactccgtaagggcacatttcgtcagcaggagcgcattcgcaaaagcctccgcggttgctactggaatttctatcatgcattgatgatcaagtaccgagctaaagttgtgcatgaggaatcggtgggttcatccggtctggtggggcagtggctgcgtgcatttcagaaggatctcaaaaaggctgatgttctgcccaagaagggtggaaaaaatggtgtagacaaaaaaaagagagaaagcagcgctcaggataccttatggggaggagctttctcgaagaaggaagagcagcagatagcctttgaggttcaggcagctggatcaagccagttttgtctgaagtgtggttggtggtttcagttggggatgcgggaagtaaatcgtgtgcaggagagtggcgtggtgctggactggaaccggtccattgtaaccttcctcatcgaatcctcaggagaaaaggtatatggtttcagtcctcagcaactggaaaaaggctttcgtcctgacatcgaaacgttcaaaaaaatggtaagggattttatgagaccccccatgtttgatcgcaaaggtcggccggccgcggcgtatgaaagattcgtactgggacgtcgtcaccgtcgttatcgctttgataaagtttttgaagagagatttggtcgcagtgctcttttcatctgcccgcgggtcgggtgtgggaatttcgatcactccagtgagcagtcagccgttgtccttgcccttattggttacattgctgataaggaagggatgagtggtaagaagcttgtttatgtgaggctggctgaacttatggctgagtggaagctgaagaaactggagagatcaagggtggaagaacagagctcggcacaataa

SEQ ID NO: 38 - DNA, 3579 bp, Artificial Sequence
  Description of Artificial Sequence: Synthetic polynucleotide
atggcagaaagcaagcagatgcaatgccgcaagtgcggcgcaagcatgaagtatgaagtaattggattgggcaagaagtcatgcagatatatgtgcccagattgcggcaatcacaccagcgcgcgcaagattcagaacaagaaaaagcgcgacaaaaagtatggatccgcaagcaaagcgcagagccagaggatagctgtggctggcgcgctttatccagacaaaaaagtgcagaccataaagacctacaaatacccagcggatcttaatggcgaagttcatgacagcggcgtcgcagagaagattgcgcaggcgattcaggaagatgagatcggcctgcttggcccgtccagcgaatacgcttgctggattgcttcacaaaaacagagcgagccgtattcagttgtagatttttggtttgacgcggtgtgcgcaggcggagtattcgcgtattctggcgcgcgcctgctttccacagtcctccagttgagtggcgaggaaagcgttttgcgcgctgctttagcatctagcccgtttgtagatgacattaatttggcgcaagcggaaaagttcctagccgttagccggcgcacaggccaagataagctaggcaagcgcattggagaatgttttgcggaaggccggcttgaagcgcttggcatcaaagatcgcatgcgcgaattcgtgcaagcgattgatgtggcccaaaccgcgggccagcggttcgcggccaagctaaagatattcggcatcagtcagatgcctgaagccaagcaatggaacaatgattccgggctcactgtatgtattttgccggattattatgtcccggaagaaaaccgcgcggaccagctggttgttttgcttcggcgcttacgcgagatcgcgtattgcatgggaattgaggatgaagcaggatttgagcatctaggcattgaccctggtgctctttccaatttttccaatggcaatccaaagcgaggatttctcggccgcctgctcaataatgacattatagcgctggcaaacaacatgtcagccatgacgccgtattgggaaggcagaaaaggcgagttgattgagcgccttgcatggcttaaacatcgcgctgaaggattgtatttgaaagagccacatttcggcaactcctgggcagaccaccgcagcaggattttcagtcgcattgcgggctggctttccggatgcgcgggcaagctcaagattgccaaggatcagatttcaggcgtgcgtacggatttgtttctgctcaagcgccttctggatgcggtaccgcaaagcgcgccgtcgccggactttattgcttccatcagcgcgctggatcggtttttggaagcggcagaaagcagccaggatccggcagaacaggtacgcgctttgtacgcgtttcatctgaacgcgcctgcggtccgatccatcgccaacaaggcggtacagaggtctgattcccaggagtggcttatcaaggaactggatgctgtagatcaccttgaattcaacaaagcatttccgtttttttcggatacaggaaagaaaaagaagaaaggagcgaatagcaacggagcgccttctgaagaagaatacacggaaacagaatccattcaacaaccagaagatgcagagcaggaagtgaatggtcaagaaggaaatggcgcttcaaagaaccagaaaaagtttcagcgcattcctcgatttttcggggaagggtcaaggagtgagtatcgaattttaacagaagcgccgcaatattttgacatgttctgcaataatatgcgcgcgatctttatgcagctagagagtcagccgcgcaaggcgcctcgtgatttcaaatgctttctgcagaatcgtttgcagaagctttacaagcaaacctttctcaatgctcgcagtaataaatgccgcgcgcttctggaatccgtccttatttcatggggagaattttatacttatggcgcgaatgaaaagaagtttcgtctgcgccatgaagcgagcgagcgcagctcggatccggactatgtggttcagcaggcattggaaatcgcgcgccggcttttcttgttcggatttgagtggcgcgattgctctgctggagagcgcgtggatttggttgaaatccacaaaaaagcaatctcatttttgcttgcaatcactcaggccgaggtttcagttggttcctataactggcttgggaatagcaccgtgagccggtatctttcggttgctggcacagacacattgtacggcactcaactggaggagtttttgaacgccacagtgctttcacagatgcgtgggctggcgattcggctttcatctcaggagttaaaagacggatttgatgttcagttggagagttcgtgccaggacaatctccagcatctgctggtgtatcgcgcttcgcgcgacttggctgcgtgcaaacgcgctacatgcccggctgaattggatccgaaaattcttgttctgccggttggtgcgtttatcgcgagcgtaatgaaaatgattgagcgtggcgatgaaccattagcaggcgcgtatttgcgtcatcggccgcattcattcggctggcagatacgggttcgtggagtggcggaagtaggcatggatcagggcacagcgctagcattccagaagccgactgaatcagagccgtttaaaataaagccgttttccgctcaatacggcccagtactttggcttaattcttcatcctatagccagagccagtatctggatggatttttaagccagccaaagaattggtctatgcgggtgctacctcaagccggatcagtgcgcgtggaacagcgcgttgctctgatatggaatttgcaggcaggcaagatgcggctggagcgctctggagcgcgcgcgtttttcatgccagtgccattcagcttcaggccgtctggttcaggagatgaagcagtattggcgccgaatcggtacttgggactttttccgcattccggaggaatagaatacgcggtggtggatgtattagattccgcgggtttcaaaattcttgagcgcggtacgattgcggtaaatggcttttcccagaagcgcggcgaacgccaagaggaggcacacagagaaaaacagagacgcggaatttctgatataggccgcaagaagccggtgcaagctgaagttgacgcagccaatgaattgcaccgcaaatacaccgatgttgccactcgtttagggtgcagaattgtggttcagtgggcgccccagccaaagccgggcacagcgccgaccgcgcaaacagtatacgcgcgcgcagtgcggaccgaagcgccgcgatctggaaatcaagaggatcatgctcgtatgaaatcctcttggggatatacctggggcacctattgggagaagcgcaaaccagaggatattttgggcatctcaacccaagtatactggaccggcggtataggcgagtcatgtcccgcagtcgcggttgcgcttttggggcacattagggcaacatccactcaaactgaatgggaaaaagaggaggttgtattcggtcgactgaagaagttctttccaagctag

SEQ ID NO: 39 - DNA, 2958 bp, Artificial Sequence
  Description of Artificial Sequence: Synthetic polynucleotide
atggaaaagagaataaacaagatacgaaagaaactatcggccgataatgccacaaagcctgtgagcaggagcggccccatgaaaacactccttgtccgggtcatgacggacgacttgaaaaaaagactggagaagcgtcggaaaaagccggaagttatgccgcaggttatttcaaataacgcagcaaacaatcttagaatgctccttgatgactatacaaagatgaaggaggcgatactacaagtttactggcaggaatttaaggacgaccatgtgggcttgatgtgcaaatttgcccagcctgcttccaaaaaaattgaccagaacaaactaaaaccggaaatggatgaaaaaggaaatctaacaactgccggttttgcatgttctcaatgcggtcagccgctatttgtttataagcttgaacaggtgagtgaaaaaggcaaggcttatacaaattacttcggccggtgtaatgtggccgagcatgagaaattgattcttcttgctcaattaaaacctgaaaaagacagtgacgaagcagtgacatactcccttggcaaattcggccagagggcattggacttttattcaatccacgtaacaaaagaatccacccatccagtaaagcccctggcacagattgcgggcaaccgctatgcaagcggacctgttggcaaggccctttccgatgcctgtatgggcactatagccagttttctttcgaaatatcaagacatcatcatagaacatcaaaaggttgtgaagggtaatcaaaagaggttagagagtctcagggaattggcagggaaagaaaatcttgagtacccatcggttacactgccgccgcagccgcatacgaaagaaggggttgacgcttataacgaagttattgcaagggtacgtatgtgggttaatcttaatctgtggcaaaagctgaagctcagccgtgatgacgcaaaaccgctactgcggctaaaaggattcccatctttccctgttgtggagcggcgtgaaaacgaagttgactggtggaatacgattaatgaagtaaaaaaactgattgacgctaaacgagatatgggacgggtattctggagcggcgttaccgcagaaaagagaaataccatccttgaaggatacaactatctgccaaatgagaatgaccataaaaagagagagggcagtttggaaaaccctaagaagcctgccaaacgccagtttggagacctcttgctgtatcttgaaaagaaatatgccggagactggggaaaggtcttcgatgaggcatgggagaggatagataagaaaatagccggactcacaagccatatagagcgcgaagaagcaagaaacgcggaagacgctcaatccaaagccgtacttacagactggctaagggcaaaggcatcatttgttcttgaaagactgaaggaaatggatgaaaaggaattctatgcgtgtgaaatccaacttcaaaaatggtatggcgatcttcgaggcaacccgtttgccgttgaagctgagaatagagttgttgatataagcgggttttctatcggaagcgatggccattcaatccaatacagaaatctccttgcctggaaatatctggagaacggcaagcgtgaattctatctgttaatgaattatggcaagaaagggcgcatcagatttacagatggaacagatattaaaaagagcggcaaatggcagggactattatatggcggtggcaaggcaaaggttattgatctgactttcgaccccgatgatgaacagttgataatcctgccgctggcctttggcacaaggcaaggccgcgagtttatctggaacgatttgctgagtcttgaaacaggcctgataaagctcgcaaacggaagagttatcgaaaaaacaatctataacaaaaaaatagggcgggatgaaccggctctattcgttgccttaacatttgagcgccgggaagttgttgatccatcaaatataaagcctgtaaaccttataggcgttgaccgcggcgaaaacatcccggcggttattgcattgacagaccctgaaggttgtcctttaccggaattcaaggattcatcagggggcccaacagacatcctgcgaataggagaaggatataaggaaaagcagagggctattcaggcagcaaaggaggtagagcaaaggcgggctggcggttattcacggaagtttgcatccaagtcgaggaacctggcggacgacatggtgagaaattcagcgcgagaccttttttaccatgccgttacccacgatgccgtccttgtctttgaaaacctgagcaggggttttggaaggcagggcaaaaggaccttcatgacggaaagacaatatacaaagatggaagactggctgacagcgaagctcgcatacgaaggtcttacgtcaaaaacctacctttcaaagacgctggcgcaatatacgtcaaaaacatgctccaactgcgggtttactataacgactgccgattatgacgggatgttggtaaggcttaaaaagacttctgatggatgggcaactaccctcaacaacaaagaattaaaagccgaaggccagataacgtattataaccggtataaaaggcaaaccgtggaaaaagaactctccgcagagcttgacaggctttcagaagagtcgggcaataatgatatttctaagtggaccaagggtcgccgggacgaggcattatttttgttaaagaaaagattcagccatcggcctgttcaggaacagtttgtttgcctcgattgcggccatgaagtccacgccgatgaacaggcagccttgaatattgcaaggtcatggctttttctaaactcaaattcaacagaattcaaaagttataaatcgggtaaacagcccttcgttggtgcttggcaggccttttacaaaaggaggcttaaagaggtatggaagcccaacgcc

SEQ ID NO: 40 - DNA, 2919 bp, Artificial Sequence
  Description of Artificial Sequence: Synthetic polynucleotide
atgaaaaggataaataaaatacgaaggagattggtaaaggatagcaacacgaaaaaagccggcaaaaccggccctatgaaaaccttgctcgttcgggttatgacacctgacctgagagaaaggttagagaatcttcgcaaaaagccggaaaacattcctcagcccatttcaaatacttcacgtgcaaatttaaataaactcctcactgactatacggaaatgaagaaagcaatcctgcatgtttattgggaagagttccaaaaagaccctgtcggattgatgagcagggttgcacaaccagcgcccaagaatattgatcagagaaaattgattccggtgaaggacggaaatgagagactaacaagttctggatttgcctgttctcagtgctgtcaacccctctatgtttataagcttgaacaagtgaatgacaagggtaagccccatacaaattactttggccgttgtaatgtctccgagcatgaacgtttgatattgctctcgccgcataaaccggaggcaaatgacgagctagtaacgtattcgttggggaagttcggtcaaagggcattggacttttattcaatccacgtaacaagagaatcgaaccatcctgtaaagccgctagaacagatcggtggcaatagctgcgcaagtggtcccgttggtaaggctttatctgatgcctgtatgggagcagtagccagtttccttacaaagtaccaggacatcatcctcgaacaccaaaaggttataaaaaaaaacgaaaagagattggcaaatctaaaggatatagcaagtgcaaacgggcttgcatttcctaaaatcactcttccaccgcaaccgcatacaaaagaagggattgaagcttataacaatgttgttgctcagatagtgatctgggtaaacctgaatctttggcagaaactcaaaattggcagggatgaggcaaagcccttacagcggcttaagggttttccgtccttccctcttgttgaacgccaggcgaatgaggttgattggtgggatatggtctgtaatgtcaaaaagttgattaacgaaaagaaagaggacgggaaggtcttctggcaaaatcttgctggatataaaaggcaggaagccttgcttccatatctttcgtctgaagaagaccgtaaaaaaggaaaaaagtttgcgcgttatcagtttggtgaccttttgcttcaccttgaaaagaaacacggtgaagattggggcaaagtttatgatgaggcatgggaaagaatagataaaaaagttgaaggtctgagtaagcacataaagttggaggaagaaagaaggtctgaagatgctcaatcaaaggctgccctcactgattggctcagggcaaaggcctcttttgttattgaagggctcaaagaagctgataaggatgagttttgcaggtgtgagttaaagcttcaaaagtggtatggagatttgagaggaaaaccatttgctatagaagcagagaacagcattttagatataagcggattttctaaacagtataattgtgcatttatatggcagaaagacggcgtaaagaagttaaatctttatttaataataaattacttcaaaggtggtaagctacgcttcaaaaaaatcaagccagaagcttttgaagcaaataggttttatacagtaattaataaaaaaagcggtgagattgtgcctatggaggtcaacttcaattttgatgacccgaatttgataattctgcctttggcctttggaaaaaggcaggggagggagtttatctggaacgacctattgagccttgagacgggttcattgaaactcgccaatggcagggttattgaaaaaacgctctataacagaaggacgagacaggatgaaccagcactttttgttgccctgacatttgaaagaagagaggtgcttgactcatcgaatataaaaccgatgaatctgataggaatagaccggggagaaaatatcccggcagtcatagcattaacagacccggaaggatgccccttgtcaagattcaaagattcattgggcaatccaacgcatattttgcgaataggagaaagttataaggaaaaacaacggactattcaggctgctaaagaagttgaacaaaggcgggcaggcggatattcgagaaaatatgcatcaaaggcgaagaatctggcggacgatatggtaagaaatacagctcgtgacctcttatattatgctgttactcaagatgcaatgctcatttttgaaaatctttcccgcggttttggtagacaaggcaagaggacttttatggcggaaaggcagtacacgaggatggaagactggctgactgcaaagcttgcctatgaaggtctgccatcaaaaacctatctttcaaagactctggcacagtatacctcaaagacatgttctaattgtggttttacaatcacaagtgcagattatgacagggtgctcgaaaagctcaagaagacggctactggatggatgactacaatcaatggaaaagagttaaaagttgaaggacagataacatactataaccggtataaaaggcagaatgtggtaaaagacctctctgtagagctggatagactttcggaagagtcggtaaataatgatatttctagttggacaaaaggccgcagtggtgaagctttatctctgctaaaaaagagatttagtcacaggccggtgcaggaaaagtttgtttgcctgaactgtggttttgaaacccatgcagacgaacaagcagcactgaatattgcaaggtcgtggctctttctccgttctcaagaatataagaagtatcaaaccaataaaacgaccggaaatactgacaaaagggcatttgttgaaacatggcaatccttttacagaaagaagctcaaagaagtatggaaacca

SEQ ID NO: 41 - DNA, 4077 bp, Artificial Sequence
  Description of Artificial Sequence: Synthetic polynucleotide
atgggtaaaatgtattaccttggtttagacattggcacgaattccgtgggctacgcggtgaccgacccctcataccacctgctgaagtttaagggggaaccaatgtggggtgcgcacgtatttgccgccggtaatcagagcgcggaacgacgctcgttccgcacatcgcgtcgtcgtttggaccgacgccaacagcgcgttaaactggtacaggagatttttgccccggtgattagtccgatcgacccacgcttcttcattcgtctgcatgaatccgccctgtggcgcgatgacgtcgcggagacggataaacatatctttttcaatgatcctacctataccgataaggaatattatagcgattacccgactatccatcacctgatcgttgatctgatggaaagctctgagaaacacgatccgcggctggtgtaccttgcagtggcgtggttagtggcacaccgtggtcattttctgaacgaggtggacaaggataatattggagatgtgttgtcgttcgacgcattttatccggagtttctcgcgttcctgtcggacaacggtgtatcaccgtgggtgtgcgaaagcaaagcgctgcaggcgaccttgctgagccgtaactcagtgaacgacaaatataaagcccttaagtctctgatcttcggatcccagaaacctgaagataacttcgatgccaatatttcggaagatggactcattcaactgctggccggcaaaaaggtaaaagttaacaaactgttccctcaggaatcgaacgatgcatccttcacattgaatgataaagaagacgcgatagaagaaatcctgggtacgcttacaccagatgaatgtgaatggattgcgcatatacgccgcctttttgactgggctatcatgaaacatgctctgaaagatggcaggactattagcgagtcaaaagtcaaactgtatgagcagcaccatcacgatctgacccaacttaaatacttcgtgaaaacctaccttgcaaaagaatacgacgatattttccgcaacgtggatagcgaaacaacgaaaaactatgtagcgtattcctatcatgtgaaagaggtgaaaggcactctgcctaaaaataaggcaacgcaagaagagttttgtaagtatgtcctgggcaaggttaaaaacattgaatgctctgaagcagacaaggttgactttgatgagatgattcagcgtcttaccgacaactcttttatgcctaagcaggtttcgggcgaaaaccgcgttattccttatcagttatattattatgaactgaagacaattctgaataaagcagcctcgtacctgcctttcctgacgcagtgtggaaaagatgcaatttcgaaccaggacaaactactgtcgatcatgacgttccgtattccttacttcgtcggacccttgcgaaaagataattcggaacatgcatggctcgaacgaaaggccggtaagatttatccgtggaactttaacgacaaagtggacttggataaatcagaagaagcgttcattcgccgaatgaccaatacctgtacctattatcccggcgaagatgttttaccgttggattcgctgatctatgagaaatttatgattttaaatgaaatcaataatattcgtattgacggctacccgattagtgttgacgttaaacagcaggtttttggcttgttcgaaaaaaaacgacgcgtaaccgtgaaagatattcagaacctgctgctgtctctcggagctctggacaaacacgggaagctgacaggcatcgataccactatccactcaaactataatacgtatcaccattttaaatctctcatggaacgcggcgtcctgacccgggatgacgtggaacgcatcgttgaaaggatgacctacagcgacgatactaagcgtgtgcgtctgtggctgaataacaactatggtactttaaccgccgacgatgtgaaacacatttcgcgtctgcgcaaacacgattttggccgtttatccaaaatgttcttaacaggtctgaagggtgtccataaggagaccggtgaacgtgcctccatactggatttcatgtggaacacgaacgataacctgatgcagctcctttccgaatgctacacgttcagtgatgaaatcacaaagctgcaagaggcgtattatgcaaaagcccagttgtctttaaacgattttttagactcgatgtacatctctaacgcggtgaaacgtccgatttacagaactctggcagtggtgaacgatattcgaaaagcatgtgggacggcccctaaacgcattttcatcgaaatggctcgtgatggtgaatcaaaaaaaaagagaagtgttacacgtcgcgagcagatcaaaaacctgtaccgctcgattcgtaaagatttccagcaggaagttgattttctggaaaagatcctggaaaataaatctgatggtcaacttcagtcagatgctttgtatctttactttgcacaattagggcgcgatatgtacacgggcgatccaataaagctggagcacatcaaagatcagagtttctataacatagaccatatttacccgcagtctatggtgaaagacgattccctagataacaaagtgctggtgcaaagcgaaattaacggcgagaaaagctcgcgataccctttggacgccgcgatccgcaataaaatgaagcccctttgggacgcttactataatcatggcctgatctccttaaagaaataccagcgtctaacgcgctcgaccccgtttaccgatgatgaaaaatgggactttattaatcgccagttagtggaaacccgtcaatctaccaaagcgctggccattttgttgaagcgtaagtttccagacaccgaaattgtgtattcgaaggcggggttatcgtccgacttcagacatgaattcggccttgtaaaaagtcgcaatattaatgatttgcaccacgctaaagacgcattcttggctatcgttaccggcaatgtgtaccatgaaagattcaatcgcagatggtttatggtgaaccagccgtactcagttaaaactaaaactctttttacccacagcataaagaatggcaacttcgttgcctggaacggcgaagaagatctcggtcgtattgtaaaaatgctgaagcaaaacaaaaataccattcacttcacgcgcttctccttcgatcgcaaagaaggattatttgatatccaacctctgaaagccagcaccggcttagtcccacgaaaagccggtctggatgtcgttaaatacggcggatatgacaaatctaccgcggcctattacctgctggtgaggttcacgctcgaggacaagaaaacccagcacaagctgatgatgattcctgtagaaggcctgtacaaggctcgcattgatcatgacaaggaatttcttaccgattatgcgcaaacgactataagcgaaatcctacagaaagataaacagaaagtgatcaatattatgtttccaatgggtacgaggcatataaaactcaattcaatgattagtatcgatggcttctatcttagtatcggcggaaagtcctctaaaggtaagtcagttctatgtcacgcaatggttccactgatcgtccctcacaaaatcgaatgttacattaaagcaatggaaagcttcgcccggaagtttaaagaaaacaacaagctgcgcatcgtagaaaaattcgataaaatcaccgttgaagacaacctgaatctctacgagctctttctccaaaaactgcagcataatccctataataagtttttttcgacacagtttgacgtactgacgaacggccgttctactttcacaaaactgtcgccggaggaacaggtacagacgctcttgaacattttaagtatctttaaaacatgccgcagttcgggttgcgacctgaaatccatcaacggcagtgcccaggcagcgcgcatcatgattagcgctgacttaactggactgtcgaaaaaatattcagatattaggttggttgaacagtcagcttctggtttgttcgtatccaaaagtcagaacttactggagtatctctaa

SEQ ID NO: 42 - DNA, 4005 bp, Artificial Sequence
  Description of Artificial Sequence: Synthetic polynucleotide
atgtcatcgctcacgaaattcactaacaaatactctaaacagctcaccattaagaatgaactcatcccagttggcaaaacactggagaacatcaaagagaatggtctgatagatggcgacgaacagctgaatgagaattatcagaaggcgaaaattattgtggatgattttctgcgggacttcattaataaagcactgaataatacgcagatcgggaactggcgcgaactggcggatgcccttaataaagaggatgaagataacatcgagaaattgcaggataaaattcggggaatcattgtatccaaatttgaaacgtttgatctgtttagcagctattctattaagaaagatgaaaagattattgacgacgacaatgatgttgaagaagaggaactggatctgggcaagaagaccagctcatttaaatacatatttaaaaaaaacctgtttaagttagtgttgccatcctacctgaaaaccacaaaccaggacaagctgaagattattagctcgtttgataatttttcaacgtacttccgcgggttctttgaaaaccggaaaaacatttttaccaagaaaccgatctccacaagtattgcgtatcgcattgttcatgataacttcccgaaattccttgataacattcgttgttttaatgtgtggcagacggaatgcccgcaactaatcgtgaaagcagataactatctgaaaagcaaaaatgttatagcgaaagataaaagtttggcaaactattttaccgtgggcgcgtatgactatttcctgtctcagaatggtatagatttttacaacaatattataggtggactgccagcgttcgccggccatgagaaaatccaaggtctcaatgaattcatcaatcaagagtgccaaaaagacagcgagctgaaaagtaagctgaaaaaccgtcacgcgttcaaaatggcggtactgttcaaacagatactcagcgatcgtgaaaaaagttttgtaattgatgagttcgagtcggatgctcaagttattgacgccgttaaaaacttttacgccgaacagtgcaaagataacaatgttatttttaacttattaaatcttatcaagaatatcgctttcttaagtgatgacgaactggacggcatattcattgaagggaaatacctgtcgagcgttagtcaaaaactctatagcgattggtcaaaattacgtaacgacattgaggattcggctaactctaaacaaggcaataaagagctggccaagaagatcaaaaccaacaaaggggatgtagaaaaagcgatctcgaaatatgagttctcgctgtcggaactgaactcgattgtacatgataacaccaagttttctgacctccttagttgtacactgcataaggtggcttctgagaaactggtgaaggtcaatgaaggcgactggccgaaacatctcaagaataatgaagagaaacaaaaaatcaaagagccgcttgatgctctgctggagatctataatacacttctgatttttaactgcaaaagcttcaataaaaacggcaacttctatgtcgactatgatcgttgcatcaatgaactgagttcggtcgtgtatctgtataataaaacacgtaactattgcactaaaaaaccctataacacggacaagttcaaactcaattttaacagtccgcagctcggtgaaggcttttccaagtcgaaagaaaatgactgtctgactcttttgtttaaaaaagacgacaactattatgtaggcattatccgcaaaggtgcaaaaatcaattttgatgatacacaagcaatcgccgataacaccgacaattgcatctttaaaatgaattatttcctacttaaagacgcaaaaaaatttatcccgaaatgtagcattcagctgaaagaagtcaaggcccattttaagaaatctgaagatgattacattttgtctgataaagagaaatttgctagcccgctggtcattaaaaagagcacatttttgctggcaactgcacatgtgaaagggaaaaaaggcaatatcaagaaatttcagaaagaatattcgaaagaaaaccccactgagtatcgcaattctttaaacgaatggattgctttttgtaaagagttcttaaaaacttataaagcggctaccatttttgatataaccacattgaaaaaggcagaggaatatgctgatattgtagaattctacaaggatgtcgataatctgtgctacaaactggagttctgcccgattaaaacctcgtttatagaaaacctgatagataacggcgacctgtatctgtttcgcatcaataacaaagacttcagcagtaaatcgaccggcaccaagaaccttcatacgttatatttacaagctatattcgatgaacgtaatctgaacaatccgacaattatgctgaatgggggagcagaactgttctatcgtaaagaaagtattgagcagaaaaaccgtatcacacacaaagccggttcaattctcgtgaataaggtgtgtaaagacggtacaagcctggatgataagatacgtaatgaaatttatcaatatgagaataaatttattgataccctgtctgatgaagctaaaaaggtgttaccgaatgtcattaaaaaggaagctacccatgacattacaaaagataaacgtttcactagtgacaaattcttctttcactgccccctgacaattaattataaggaaggcgataccaagcagttcaataacgaagtgctgagttttctgcgtggaaatcctgacatcaacattatcggcattgaccgcggagagcgtaatttaatctatgtaacggttataaaccagaaaggcgagattctggattcggtttcattcaataccgtgaccaacaagagttcaaaaatcgagcagacagtcgattatgaagagaaattggcagtccgcgagaaagagaggattgaagcaaaacgttcctgggactctatctcaaaaattgcgacactaaaggaaggttatctgagcgcaatagttcacgagatctgtctgttaatgattaaacacaacgcgatcgttgtcttagagaatcttaatgcaggctttaagcgtattcgtggcggtttatcagaaaaaagtgtttatcaaaaattcgaaaaaatgttgattaacaaactgaactattttgtcagcaagaaggaatccgactggaataaaccgtctggtctgctgaatggactgcagctttcggatcagtttgaaagcttcgaaaaactgggtattcagtctggttttattttttacgtgccggctgcatatacctcaaagattgatccgaccacgggcttcgccaatgttctgaatctgtcgaaggtacgcaatgttgatgcgatcaaaagctttttttctaacttcaacgaaattagttatagcaagaaagaagcccttttcaaattctcattcgatctggattcactgagtaagaaaggctttagtagctttgtgaaatttagtaagagtaaatggaacgtctacacctttggagaacgtatcataaagccaaagaataagcaaggttatcgggaggacaaaagaatcaacttgaccttcgagatgaagaagttacttaacgagtataaggtttcttttgatcttgaaaataacttgattccgaatctcacgagtgccaacctgaaggatactttttggaaagagctattctttatcttcaagactacgctgcagctccgtaacagcgttactaacggtaaagaagatgtgctcatctctccggtcaaaaatgcgaagggtgaattcttcgtttcgggaacgcataacaagactcttccgcaagattgcgatgcgaacggtgcataccatattgcgttgaaaggtctgatgatactcgaacgtaacaaccttgtacgtgaggagaaagatacgaaaaagattatggcgatttcaaacgtggattggttcgagtacgtgcagaaacgtagaggcgttctgtaa

SEQ ID NO: 43 - DNA, 3717 bp, Artificial Sequence
  Description of Artificial Sequence: Synthetic polynucleotide
atgaacaactacgacgaattcaccaaactgtacccgatccagaaaaccatccgtttcgaactgaaaccgcagggtcgtaccatggaacacctggaaaccttcaacttcttcgaagaagaccgtgaccgtgcggaaaaatacaaaatcctgaaagaagcgatcgacgaataccacaaaaaattcatcgacgaacacctgaccaacatgtctctggactggaactctctgaaacagatctctgaaaaatactacaaatctcgtgaagaaaaagacaaaaaagttttcctgtctgaacagaaacgtatgcgtcaggaaatcgtttctgaattcaaaaaagacgaccgtttcaaagacctgttctctaaaaaactgttctctgaactgctgaaagaagaaatctacaaaaaaggtaaccaccaggaaatcgacgcgctgaaatctttcgacaaattctctggttacttcatcggtctgcacgaaaaccgtaaaaacatgtactctgacggtgacgaaatcaccgcgatctctaaccgtatcgttaacgaaaacttcccgaaattcctggacaacctgcagaaataccaggaagcgcgtaaaaaatacccggaatggatcatcaaagcggaatctgcgctggttgcgcacaacatcaaaatggacgaagttttctctctggaatacttcaacaaagttctgaaccaggaaggtatccagcgttacaacctggcgctgggtggttacgttaccaaatctggtgaaaaaatgatgggtctgaacgacgcgctgaacctggcgcaccagtctgaaaaatcttctaaaggtcgtatccacatgaccccgctgttcaaacagatcctgtctgaaaaagaatctttctcttacatcccggacgttttcaccgaagactctcagctgctgccgtctatcggtggtttcttcgcgcagatcgaaaacgacaaagacggtaacatcttcgaccgtgcgctggaactgatctcttcttacgcggaatacgacaccgaacgtatctacatccgtcaggcggacatcaaccgtgtttctaacgttatcttcggtgaatggggtaccctgggtggtctgatgcgtgaatacaaagcggactctatcaacgacatcaacctggaacgtacctgcaaaaaagttgacaaatggctggactctaaagaattcgcgctgtctgacgttctggaagcgatcaaacgtaccggtaacaacgacgcgttcaacgaatacatctctaaaatgcgtaccgcgcgtgaaaaaatcgacgcggcgcgtaaagaaatgaaattcatctctgaaaaaatctctggtgacgaagaatctatccacatcatcaaaaccctgctggactctgttcagcagttcctgcacttcttcaacctgttcaaagcgcgtcaggacatcccgctggacggtgcgttctacgcggaattcgacgaagttcactctaaactgttcgcgatcgttccgctgtacaacaaagttcgtaactacctgaccaaaaacaacctgaacaccaaaaaaatcaaactgaacttcaaaaacccgaccctggcgaacggttgggaccagaacaaagtttacgactacgcgtctctgatcttcctgcgtgacggtaactactacctgggtatcatcaacccgaaacgtaaaaaaaacatcaaattcgaacagggttctggtaacggtccgttctaccgtaaaatggtttacaaacagatcccgggtccgaacaaaaacctgccgcgtgttttcctgacctctaccaaaggtaaaaaagaatacaaaccgtctaaagaaatcatcgaaggttacgaagcggacaaacacatccgtggtgacaaattcgacctggacttctgccacaaactgatcgacttcttcaaagaatctatcgaaaaacacaaagactggtctaaattcaacttctacttctctccgaccgaatcttacggtgacatctctgaattctacctggacgttgaaaaacagggttaccgtatgcacttcgaaaacatctctgcggaaaccatcgacgaatacgttgaaaaaggtgacctgttcctgttccagatctacaacaaagacttcgttaaagcggcgaccggtaaaaaagacatgcacaccatctactggaacgcggcgttctctccggaaaacctgcaggacgttgttgttaaactgaacggtgaagcggaactgttctaccgtgacaaatctgacatcaaagaaatcgttcaccgtgaaggtgaaatcctggttaaccgtacctacaacggtcgtaccccggttccggacaaaatccacaaaaaactgaccgactaccacaacggtcgtaccaaagacctgggtgaagcgaaagaatacctggacaaagttcgttacttcaaagcgcactacgacatcaccaaagaccgtcgttacctgaacgacaaaatctacttccacgttccgctgaccctgaacttcaaagcgaacggtaaaaaaaacctgaacaaaatggttatcgaaaaattcctgtctgacgaaaaagcgcacatcatcggtatcgaccgtggtgaacgtaacctgctgtactactctatcatcgaccgttctggtaaaatcatcgaccagcagtctctgaacgttatcgacggtttcgactaccgtgaaaaactgaaccagcgtgaaatcgaaatgaaagacgcgcgtcagtcttggaacgcgatcggtaaaatcaaagacctgaaagaaggttacctgtctaaagcggttcacgaaatcaccaaaatggcgatccagtacaacgcgatcgttgttatggaagaactgaactacggtttcaaacgtggtcgtttcaaagttgaaaaacagatctaccagaaattcgaaaacatgctgatcgacaaaatgaactacctggttttcaaagacgcgccggacgaatctccgggtggtgttctgaacgcgtaccagctgaccaacccgctggaatctttcgcgaaactgggtaaacagaccggtatcctgttctacgttccggcggcgtacacctctaaaatcgacccgaccaccggtttcgttaacctgttcaacacctcttctaaaaccaacgcgcaggaacgtaaagaattcctgcagaaattcgaatctatctcttactctgcgaaagacggtggtatcttcgcgttcgcgttcgactaccgtaaattcggtacctctaaaaccgaccacaaaaacgtttggaccgcgtacaccaacggtgaacgtatgcgttacatcaaagaaaaaaaacgtaacgaactgttcgacccgtctaaagaaatcaaagaagcgctgacctcttctggtatcaaatacgacggtggtcagaacatcctgccggacatcctgcgttctaacaacaacggtctgatctacaccatgtactcttctttcatcgcggcgatccagatgcgtgtttacgacggtaaagaagactacatcatctctccgatcaaaaactctaaaggtgaattcttccgtaccgacccgaaacgtcgtgaactgccgatcgacgcggacgcgaacggtgcgtacaacatcgcgctgcgtggtgaactgaccatgcgtgcgatcgcggaaaaattcgacccggactctgaaaaaatggcgaaactggaactgaaacacaaagactggttcgaattcatgcagacccgtggtgactaa

SEQ ID NO: 44 - DNA, 3897 bp, Artificial Sequence
  Description of Artificial Sequence: Synthetic polynucleotide
atgactaaaacatttgattcagagttttttaatttgtactcgctgcaaaaaacggtacgctttgagttaaaacccgtgggagaaaccgcgtcatttgtggaagactttaaaaacgagggcttgaaacgtgttgtgagcgaagatgaaaggcgagccgtcgattaccagaaagttaaggaaataattgacgattaccatcgggatttcattgaagaaagtttaaattattttccggaacaggtgagtaaagatgctcttgagcaggcgtttcatctttatcagaaactgaaggcagcaaaagttgaggaaagggaaaaagcgctgaaagaatgggaagcgctgcagaaaaagctacgtgaaaaagtggtgaaatgcttctcggactcgaataaagcccgcttctcaaggattgataaaaaggaactgattaaggaagacctgataaattggttggtcgcccagaatcgcgaggatgatatccctacggtcgaaacgtttaacaacttcaccacatattttaccggcttccatgagaatcgtaaaaatatttactccaaagatgatcacgccaccgctattagctttcgccttattcatgaaaatcttccaaagttttttgacaacgtgattagcttcaataagttgaaagagggtttccctgaattaaaatttgataaagtgaaagaggatttagaagtagattatgatctgaagcatgcgtttgaaatagaatatttcgttaacttcgtgacccaagcgggcatagatcagtataattatctgttaggagggaaaaccctggaggacgggacgaaaaaacaagggatgaatgagcaaattaatctgttcaaacaacagcaaacgcgagataaagcgcgtcagattcccaaactgatccccctgttcaaacagattcttagcgaaaggactgaaagccagtcctttattcctaaacaatttgaaagtgatcaggagttgttcgattcactgcagaagttacataataactgccaggataaattcaccgtgctgcaacaagccattctcggtctggcagaggcggatcttaagaaggtcttcatcaaaacctctgatttaaatgccttatctaacaccattttcgggaattacagcgtcttttccgatgcactgaacctgtataaagaaagcctgaaaacgaaaaaagcgcaggaggcttttgagaaactaccggcccattctattcacgacctcattcaatacttggaacagttcaattccagcctggacgcggaaaaacaacagagcaccgacaccgtcctgaactacttcatcaagaccgatgaattatattctcgcttcattaaatccactagcgaggctttcactcaggtgcagcctttgttcgaactggaagccctgtcatctaagcgccgcccaccggaatcggaagatgaaggggcaaaagggcaggaaggcttcgagcagatcaagcgtattaaagcttacctggatacgcttatggaagcggtacactttgcaaagccgttgtatcttgttaagggtcgtaaaatgatcgaagggctcgataaagaccagtccttttatgaagcgtttgaaatggcgtaccaagaacttgaatcgttaatcattcctatctataacaaagcgcggagctatctgtcgcggaaacctttcaaggccgataaattcaagattaattttgacaacaacacgctactgagcggatgggatgcgaacaaggaaactgctaacgcgtccattctgtttaagaaagacgggttatattaccttggaattatgccgaaaggtaagacctttctctttgactactttgtatcgagcgaggattcagagaaactgaaacagcgtcgccagaagaccgccgaagaagctctggcgcaggatggtgaaagttacttcgaaaaaattcgttataaactgttaccaggggcttcaaagatgttaccgaaagtcttttttagcaacaaaaatattggcttttacaacccgtcggatgacattttacgcattcgcaacacagcctctcacaccaaaaacgggacccctcagaaaggccactcaaaagttgagtttaacctgaatgattgtcataagatgattgatttcttcaaatcatcaattcagaaacacccggaatgggggtcttttggctttacgttttctgataccagtgattttgaagacatgagtgccttctaccgggaagtagaaaaccagggttacgtaattagctttgacaaaatcaaagagacctatatacagagccaggtggaacagggtaatctctacttattccagatttataacaaggatttctcgccctacagcaaaggcaaaccaaacctgcatactctgtactggaaagccctgtttgaagaagcgaacctgaataacgtagtggcgaagttgaacggtgaagcggaaatcttcttccgtcgtcactccattaaggcctctgataaagttgtccatccggcaaatcaggccattgataataagaatccacacacggaaaaaacgcagtcaacctttgaatatgacctcgttaaagacaaacgctacacgcaagataagttctttttccacgtcccaatcagcctcaactttaaagcacaaggggtttcaaagtttaatgataaagtcaatgggttcctcaagggcaacccggatgtcaacattataggtatagacaggggcgaacgccatctgctttactttaccgtagtgaatcagaaaggtgaaatactggttcaggaatcattaaataccttgatgtcggacaaagggcacgttaatgattaccagcagaaactggataaaaaagaacaggaacgtgatgctgcgcgtaaatcgtggaccacggttgagaacattaaagagctgaaagaggggtatctaagccatgtggtacacaaactggcgcacctcatcattaaatataacgcaatagtctgcctagaagacttgaattttggctttaaacgcggccgcttcaaagtggaaaaacaagtttatcaaaaatttgaaaaggcgcttatagataaactgaattatctggtttttaaagaaaaggaacttggtgaggtagggcactacttgacagcttatcaactgacggccccgttcgaatcattcaaaaaactgggcaaacagtctggcattctgttttacgtgccggcagattatacttcaaaaatcgatccaacaactggctttgtgaacttcctggacctgagatatcagtctgtagaaaaagctaaacaacttcttagcgattttaatgccattcgttttaacagcgttcagaattactttgaattcgaaattgactataaaaaacttactccgaaacgtaaagtcggaacccaaagtaaatgggtaatttgtacgtatggcgatgtcaggtatcagaaccgtcggaatcaaaaaggtcattgggagaccgaagaagtgaacgtgaccgaaaagctgaaggctctgttcgccagcgattcaaaaactacaactgtgatcgattacgcaaatgatgataacctgatagatgtgattttagagcaggataaagccagcttttttaaagaactgttgtggctcctgaaacttacgatgaccttacgacattccaagatcaaatcggaagatgattttattctgtcaccggtcaagaatgagcagggtgaattctatgatagtaggaaagccggcgaagtgtggccgaaagacgccgacgccaatggcgcctatcatatcgcgctcaaagggctttggaatttgcagcagattaaccagtgggaaaaaggtaaaaccctgaatctggctatcaaaaaccaggattggtttagctttatccaagagaaaccgtatcaggaatga

SEQ ID NO: 45 - DNA, 3708 bp, Artificial Sequence
  Description of Artificial Sequence: Synthetic polynucleotide
atgcatacaggcggtcttcttagtatggacgcgaaagagttcacaggtcagtatccgttgtcgaaaacattacgattcgaacttcggcccatcggccgcacgtgggataacctggaggcctcaggctacttagcggaagaccgccatcgtgccgaatgttatcctcgtgcgaaagagttattggatgacaaccatcgtgccttcctgaatcgtgtgttgccacaaatcgatatggattggcacccgattgcggaggccttttgtaaggtacataaaaaccctggtaataaagaacttgcccaggattacaaccttcagttgtcaaagcgccgtaaggagatcagcgcatatcttcaggatgcagatggctataaaggcctgttcgcgaagcccgccttagacgaagctatgaaaattgcgaaagaaaacgggaacgaaagtgatattgaggttctcgaagcgtttaacggttttagcgtatacttcaccggttatcatgagtcacgcgagaacatttatagcgatgaggatatggtgagcgtagcctaccgaattactgaggataatttcccgcgctttgtctcaaacgctttgatctttgataaattaaacgaaagccatccggatattatctctgaagtatcgggcaatcttggagttgatgacattggtaagtactttgacgtgtcgaactataacaattttctttcccaggccggtatagatgactacaatcacattattggcggccatacaaccgaagacggactgatacaagcgtttaatgtcgtattgaacttacgtcaccaaaaagaccctggctttgaaaaaattcagttcaaacagctctacaaacaaatcctgagcgtgcgtaccagcaaaagctacatcccgaaacagtttgacaactctaaggagatggttgactgcatttgcgattatgtcagcaaaatagagaaatccgaaacagtagaacgggccctgaaactagtccgtaatatcagttctttcgacttgcgcgggatctttgtcaataaaaagaacttgcgcatactgagcaacaaactgataggagattgggacgcgatcgaaaccgcattgatgcatagttcttcatcagaaaacgataagaaaagcgtatatgatagcgcggaggcttttacgttggatgacatcttttcaagcgtgaaaaaattttctgatgcctctgccgaagatattggcaacagggcggaagacatctgtagagtgataagtgagacggccccttttatcaacgatctgcgagcggtggacctggatagcctgaacgacgatggttatgaagcggccgtctcaaaaattcgggagtcgctggagccttatatggatcttttccatgaactggaaattttctcggttggcgatgagttcccaaaatgcgcagcattttacagcgaactggaggaagtcagcgaacagctgatcgaaattattccgttattcaacaaggcgcgttcgttctgcacccggaaacgctatagcaccgataagattaaagtgaacttaaaattcccgaccttggcggacgggtgggacctgaacaaagagagagacaacaaagccgcgattctgcggaaagacggtaagtattatctggcaattctggatatgaagaaagatctgtcaagcattaggaccagcgacgaagatgaatccagcttcgaaaagatggagtataaactgttaccgagtccagtaaaaatgctgccaaagatattcgtaaaatcgaaagccgctaaggaaaaatatggcctgacagatcgtatgcttgaatgctacgataaaggtatgcataagtcgggtagtgcgtttgatcttggcttttgccatgaactcattgattattacaagcgttgtatcgcggagtacccaggctgggatgtgttcgatttcaagtttcgcgaaacttccgattatgggtccatgaaagagttcaatgaagatgtggccggagccggttactatatgagtctgagaaaaattccgtgcagcgaagtgtaccgtctgttagacgagaaatcgatttatctatttcaaatttataacaaagattactctgaaaatgcacatggtaataagaacatgcataccatgtactgggagggtctcttttccccgcaaaacctggagtcgcccgttttcaagttgtcgggtggggcagaacttttctttcgaaaatcctcaatccctaacgatgccaaaacagtacacccgaaaggctcagtgctggttccacgtaatgatgttaacggtcggcgtattccagattcaatctaccgcgaactgacacgctattttaaccgtggcgattgccgaatcagtgacgaagccaaaagttatcttgacaaggttaagactaaaaaagcggaccatgacattgtgaaagatcgccgctttaccgtggataaaatgatgttccacgtcccgattgcgatgaactttaaggcgatcagtaaaccgaacttaaacaaaaaagtcattgatggcatcattgatgatcaggatctgaaaatcattggtattgatcgtggcgagcggaacttaatttacgtcacgatggttgacagaaaagggaatatcttatatcaggattctcttaacatcctcaatggctacgactatcgtaaagctctggatgtgcgcgaatatgacaacaaggaagcgcgtcgtaactggactaaagtggagggcattcgcaaaatgaaggaaggctatctgtcattagcggtctcgaaattagcggatatgattatcgaaaataacgccatcatcgttatggaggacctgaaccacggattcaaagcgggccgctcaaagattgaaaaacaagtttatcagaaatttgagagtatgctgattaacaaactgggctatatggtgttaaaagacaagtcaattgaccaatcaggtggcgcgctgcatggataccagctggcgaaccatgttaccaccttagcatcagttggaaagcagtgtggggttatcttttatataccggcagcgttcactagtaaaatagatccgaccactggtttcgccgatctctttgccctgagtaacgttaaaaacgtagcgagcatgcgtgaattcttttccaaaatgaaatctgtcatttatgataaagctgaaggcaaattcgcattcacctttgattacttggattacaacgtgaagagcgaatgtggtcgtacgctgtggaccgtttacaccgttggtgagcgcttcacctattcccgtgtgaaccgcgaatatgtacgtaaagtccccaccgatattatctatgatgccctccagaaagcaggcattagcgtcgaaggagacttaagggacagaattgccgaaagcgatggcgatacgctgaagtctattttttacgcattcaaatacgcgctagatatgcgcgttgagaatcgcgaggaagactacattcaatcacctgtgaaaaatgcctctggggaatttttttgttcaaaaaatgctggtaaaagcctcccacaagatagcgatgcaaacggtgcatataacattgccctgaaaggtattcttcaattacgcatgctgtctgagcagtacgaccccaacgcggaatctattagacttccgctgataaccaataaagcctggctgacattcatgcagtctggcatgaagacctggaaaaattag

SEQ ID NO: 46 - DNA, 3783 bp, Artificial Sequence
  Description of Artificial Sequence: Synthetic polynucleotide
atggatagtttaaaagattttacgaatctatatcccgtaagcaaaactcttcgttttgaactgaaacctgttggaaaaacgttggagaatatcgagaaagcgggcatcctgaaagaagacgagcaccgtgccgaaagctacaggcgtgtcaaaaagattatcgatacttatcacaaagtgttcattgatagcagtctggagaacatggcaaaaatgggcatagaaaatgaaatcaaagcaatgctgcagagcttttgcgagctctacaagaaagatcaccgaacggaaggtgaagataaagcactggacaaaattcgcgccgttcttcgcggtctgattgttggcgcgttcaccggcgtgtgcggccgccgtgaaaacaccgtgcagaacgaaaagtacgagtcgctgttcaaagaaaaactgataaaagaaattttgcctgactttgtgctttcgaccgaagcggaatccctgccattttctgtcgaagaagcgacccgcagcctgaaagaatttgactcattcacaagttactttgcaggcttctacgaaaaccgtaaaaacatctacagcacgaagccacagagcacggctattgcttatcgcctgattcatgagaacctgccgaagttcatcgataacatccttgtttttcaaaaaattaaagagccgattgcgaaagagttagaacatattcgagctgacttttctgcgggtgggtacattaaaaaagatgagcggctggaagacatcttcagtctaaactattatatccacgttctgtcgcaggcaggcattgagaaatataatgcgctgattggtaagattgtcacagaaggcgatggtgagatgaaaggtcttaatgaacatatcaatctgtataaccagcagcgtggtcgcgaagaccgtcttccactgttccgcccactgtataaacagatcctgtctgaccgggaacagctgtcctacctgccggaaagctttgaaaaggatgaagagctacttcgcgcattaaaggagttttacgaccatattgcggaagacattttgggtagaacgcagcaactgatgacgtcaatttctgaatacgatctgagtagaatctacgttaggaatgatagccagctgaccgatattagcaaaaaaatgctgggcgactggaacgctatctatatggcacgtgaacgtgcatatgatcatgaacaagcaccgaaacgtataaccgcgaaatatgagcgtgatcgcattaaggcgctaaagggagaagaaagcatctcactcgcaaacctgaactcctgtatcgctttcttagataacgtgcgcgattgtcgcgtcgacacgtatctgtcaacccttgggcagaaagagggtccacatggtctgtctaacctggtggaaaatgtctttgcgagttaccatgaagcggaacaactgctgtcttttccataccccgaagaaaacaatctaatacaggataaagataacgtggtgttaatcaaaaacctgctggacaacatcagcgatctgcaacgtttcctgaaacctttgtggggtatgggtgacgagccagacaaagacgaacgtttttatggtgagtataattatatacgtggcgcccttgaccaagttattccgctgtataacaaagtacggaactatctgacccgtaagccatattctacccgtaaagtgaaactgaactttggcaactcgcaactgctgtcgggttgggatcgtaacaaagaaaaagataatagttgtgttatcctgcgtaagggacaaaatttttacctcgcgattatgaacaacagacacaagcgttcatttgaaaataaggttctgccggagtataaagagggcgaaccgtacttcgagaaaatggattataagttcttaccagaccctaataagatgttaccgaaagtctttctttcgaaaaaaggcatagaaatctataagccgtccccgaaattactcgaacagtatgggcacgggacccacaagaaaggggatacttttagcatggacgatctgcacgaactgatcgatttttttaaacactccatcgaagcccatgaagactggaaacagtttgggttcaagttctctgatacagccacatacgagaatgtgtctagtttttatcgggaagtggaggatcagggctacaaacttagttttcgtaaagtttcagagagttatgtttatagtttaattgatcagggaaaactttacctgttccagatctacaacaaagatttctcgccatgtagtaagggtaccccgaatctgcatacactctattggagaatgttattcgatgagcgtaacttagcggatgtcatttataaattggacgggaaagcagagatcttttttcgtgaaaaatcactgaagaatgaccacccgactcatccggccgggaaaccgatcaaaaaaaaatcccgccagaaaaaaggagaagagtctctgtttgaatatgatctggtgaaagaccgtcattacactatggataaatttcaatttcatgttccaattacaatgaacttcaaatgttcggcgggttccaaagtaaatgatatggtaaacgcccatattcgcgaagcgaaagatatgcatgttattggcatcgatagaggcgaaagaaacctgctttatatttgcgtaattgacagccgtggtaccattctggaccagatctctttaaacaccatcaatgacatcgattatcacgacctgttggagtctcgggacaaggaccgccagcaggagcgccgtaattggcagacaattgaaggcataaaagaattaaaacagggttacctttcccaggccgtacaccgcatagcggaactgatggtggcctacaaagccgtagttgccctggaagacttgaatatggggtttaaacgtggccgtcaaaaagtcgagagcagcgtgtatcagcaatttgaaaaacagttgattgacaagttgaattatttggttgataaaaagaaacgtccagaagatattggtggcttactgcgtgcataccagtttacggcaccttttaagtccttcaaagaaatgggtaaacagaacgggtttctgttttacatcccggcctggaatacatccaacatcgatcctaccaccgggtttgtcaacctgtttcatgcacaatatgaaaacgtggataaagcgaagagttttttccaaaaattcgatagtatttcgtataacccaaaaaaagattggtttgagtttgcgttcgattataaaaattttactaaaaaggctgagggatcccgcagtatgtggatcctctgcacccatggcagtcgtattaaaaattttcgtaattcgcaaaagaatggccagtgggactcggaagagtttgccctgaccgaagcgttcaaatcgctgtttgtacgctacgaaattgactacacagcagatctgaaaacagccatcgtcgatgaaaaacagaaagatttttttgtagatctcctaaaactgttcaaactgactgttcagatgcgcaattcctggaaagagaaagacctggattatctgattagcccggtagccggtgctgatggacgatttttcgatactcgtgaaggtaacaaaagtctcccgaaagatgctgatgccaatggtgcatacaatattgcattaaaggggctatgggccttgcgacagatccgccagaccagcgaaggcggcaagctgaaattggccatatcgaataaggaatggttacaatttgttcaggaacgtagctatgaaaaagattga

SEQ ID NO: 47 - DNA, 3792 bp, Artificial Sequence
  Description of Artificial Sequence: Synthetic polynucleotide
atgaacaacggcacaaataattttcagaacttcatcgggatctcaagtttgcagaaaacgctgcgcaatgctctgatccccacggaaaccacgcaacagttcatcgtcaagaacggaataattaaagaagatgagttacgtggcgagaaccgccagattctgaaagatatcatggatgactactaccgcggattcatctctgagactctgagttctattgatgacatagattggactagcctgttcgaaaaaatggaaattcagctgaaaaatggtgataataaagataccttaattaaggaacagacagagtatcggaaagcaatccataaaaaatttgcgaacgacgatcggtttaagaacatgtttagcgccaaactgattagtgacatattacctgaatttgtcatccacaacaataattattcggcatcagagaaagaggaaaaaacccaggtgataaaattgttttcgcgctttgcgactagctttaaagattacttcaagaaccgtgcaaattgcttttcagcggacgatatttcatcaagcagctgccatcgcatcgtcaacgacaatgcagagatattcttttcaaatgcgctggtctaccgccggatcgtaaaatcgctgagcaatgacgatatcaacaaaatttcgggcgatatgaaagattcattaaaagaaatgagtctggaagaaatatattcttacgagaagtatggggaatttattacccaggaaggcattagcttctataatgatatctgtgggaaagtgaattcttttatgaacctgtattgtcagaaaaataaagaaaacaaaaatttatacaaacttcagaaacttcacaaacagattctatgcattgcggacactagctatgaggtcccgtataaatttgaaagtgacgaggaagtgtaccaatcagttaacggcttccttgataacattagcagcaaacatatagtcgaaagattacgcaaaatcggcgataactataacggctacaacctggataaaatttatatcgtgtccaaattttacgagagcgttagccaaaaaacctaccgcgactgggaaacaattaataccgccctcgaaattcattacaataatatcttgccgggtaacggtaaaagtaaagccgacaaagtaaaaaaagcggttaagaatgatttacagaaatccatcaccgaaataaatgaactagtgtcaaactataagctgtgcagtgacgacaacatcaaagcggagacttatatacatgagattagccatatcttgaataactttgaagcacaggaattgaaatacaatccggaaattcacctagttgaatccgagctcaaagcgagtgagcttaaaaacgtgctggacgtgatcatgaatgcgtttcattggtgttcggtttttatgactgaggaacttgttgataaagacaacaatttttatgcggaactggaggagatttacgatgaaatttatccagtaattagtctgtacaacctggttcgtaactacgttacccagaaaccgtacagcacgaaaaagattaaattgaactttggaataccgacgttagcagacggttggtcaaagtccaaagagtattctaataacgctatcatactgatgcgcgacaatctgtattatctgggcatctttaatgcgaagaataaaccggacaagaagattatcgagggtaatacgtcagaaaataagggtgactacaaaaagatgatttataatttgctcccgggtcccaacaaaatgatcccgaaagttttcttgagcagcaagacgggggtggaaacgtataaaccgagcgcctatatcctagaggggtataaacagaataaacatatcaagtcttcaaaagactttgatatcactttctgtcatgatctgatcgactacttcaaaaactgtattgcaattcatcccgagtggaaaaacttcggttttgattttagcgacaccagtacttatgaagacatttccgggttttatcgtgaggtagagttacaaggttacaagattgattggacatacattagcgaaaaagacattgatctgctgcaggaaaaaggtcaactgtatctgttccagatatataacaaagatttttcgaaaaaatcaaccgggaatgacaaccttcacaccatgtacctgaaaaatcttttctcagaagaaaatcttaaggatatcgtcctgaaacttaacggcgaagcggaaatcttcttcaggaagagcagcataaagaacccaatcattcataaaaaaggctcgattttagtcaaccgtacctacgaagcagaagaaaaagaccagtttggcaacattcaaattgtgcgtaaaaatattccggaaaacatttatcaggagctgtacaaatacttcaacgataaaagcgacaaagagctgtctgatgaagcagccaaactgaagaatgtagtgggacaccacgaggcagcgacgaatatagtcaaggactatcgctacacgtatgataaatacttccttcatatgcctattacgatcaatttcaaagccaataaaacgggttttattaatgataggatcttacagtatatcgctaaagaaaaagacttacatgtgatcggcattgatcggggcgagcgtaacctgatctacgtgtccgtgattgatacttgtggtaatatagttgaacagaaaagctttaacattgtaaacggctacgactatcagataaaactgaaacaacaggagggcgctagacagattgcgcggaaagaatggaaagaaattggtaaaattaaagagatcaaagagggctacctgagcttagtaatccacgagatctctaaaatggtaatcaaatacaatgcaattatagcgatggaggatttgtcttatggttttaaaaaagggcgctttaaggtcgaacggcaagtttaccagaaatttgaaaccatgctcatcaataaactcaactatctggtatttaaagatatttcgattaccgagaatggcggtctcctgaaaggttatcagctgacatacattcctgataaacttaaaaacgtgggtcatcagtgcggctgcattttttatgtgcctgctgcatacacgagcaaaattgatccgaccaccggctttgtgaatatctttaaatttaaagacctgacagtggacgcaaaacgtgaattcattaaaaaatttgactcaattcgttatgacagtgaaaaaaatctgttctgctttacatttgactacaataactttattacgcaaaacacggtcatgagcaaatcatcgtggagtgtgtatacatacggcgtgcgcatcaaacgtcgctttgtgaacggccgcttctcaaacgaaagtgataccattgacataaccaaagatatggagaaaacgttggaaatgacggacattaactggcgcgatggccacgatcttcgtcaagacattatagattatgaaattgttcagcacatattcgaaattttccgtttaacagtgcaaatgcgtaactccttgtctgaactggaggaccgtgattacgatcgtctcatttcacctgtactgaacgaaaataacattttttatgacagcgcgaaagcgggggatgcacttcctaaggatgccgatgcaaatggtgcgtattgtattgcattaaaagggttatatgaaattaaacaaattaccgaaaattggaaagaagatggtaaattttcgcgcgataaactcaaaatcagcaataaagattggttcgactttatccagaataagcgctatctctaa

SEQ ID NO: 48 - DNA, 3957 bp, Artificial Sequence
  Description of Artificial Sequence: Synthetic polynucleotide
atgaccaataaattcactaaccagtattctctctctaagaccctgcgctttgaactgattccgcaggggaaaaccttggagttcattcaagaaaaaggcctcttgtctcaggataaacagagggctgaatcttaccaagaaatgaagaaaactattgataagtttcataaatatttcattgatttagccttgtctaacgccaaattaactcacttggaaacgtatctggagttatacaacaaatctgccgaaactaagaaagaacagaaatttaaagacgatttgaaaaaagtacaggacaatctgcgtaaagaaattgtcaaatccttcagtgacggcgatgctaaaagcatttttgccattctggacaaaaaagagttgattactgtggaattagaaaagtggtttgaaaacaatgagcagaaagacatctacttcgatgagaaattcaaaactttcaccacctattttacaggatttcatcaaaaccggaagaacatgtactcagtagaaccgaactccacggccattgcgtatcgtttgatccatgagaatctgcctaaatttctggagaatgcgaaagcctttgaaaagattaagcaggtcgaatcgctgcaagtgaattttcgtgaactcatgggcgaatttggtgacgaaggtctaatcttcgttaacgaactggaagaaatgtttcagattaattactacaatgacgtgctatcgcagaacggtatcacaatctacaatagtattatctcagggttcacaaaaaacgatataaaatacaaaggcctgaacgagtatatcaataactacaaccaaacaaaggacaaaaaggataggcttccgaaactgaagcagttatacaaacagattttatctgacagaatctccctgagctttctgccggatgctttcactgatgggaagcaggttctgaaagcgattttcgatttttataagattaacttactgagctacacgattgaaggtcaagaagaatctcaaaacttactgctcttgatccgtcaaaccattgaaaatctatcatcgttcgatacgcagaaaatctacctcaaaaacgatactcacctgactacgatctctcagcaggttttcggggattttagtgtattttcaacagctctgaactactggtatgaaaccaaagtcaatccgaaattcgagacggaatattctaaggccaacgaaaaaaaacgtgagattcttgataaagctaaagccgtatttactaaacaggattacttttctattgctttcctgcaggaagttttatcggagtatatcctgaccctggatcatacatctgatatcgttaaaaaacacagcagcaattgcatcgctgactatttcaaaaaccactttgtcgccaaaaaagaaaacgaaacagacaagactttcgatttcattgctaacatcaccgcaaaataccagtgtattcagggtatcttggaaaacgccgaccaatacgaagacgaactgaaacaagatcagaagctgatcgataatttaaaattcttcttagatgcaatcctggagctgctgcacttcatcaaaccgcttcatttaaagagcgagtccattaccgaaaaggacaccgccttctatgacgtttttgaaaattattatgaagccctctccttgctgactccgctgtataatatggtacgcaattacgtaacccagaaaccatattctaccgaaaaaattaaactgaactttgaaaacgcacagctgctcaacggttgggacgcgaataaagaaggtgactacctcaccaccatcctgaaaaaagatggtaactattttctggcaattatggataagaaacataataaagcattccagaaatttcctgaagggaaagaaaattacgaaaagatggtgtacaaactcttacctggagttaacaaaatgttgccgaaagtattttttagtaataagaacatcgcgtactttaacccgtccaaagaactgctggaaaattataaaaaggagacgcataagaaaggggatacctttaacctggaacattgccataccttaatagacttcttcaaggattccctgaataaacacgaggattggaaatatttcgattttcagtttagtgagaccaagtcataccaggatcttagcggcttttatcgcgaagtagaacaccaaggctataaaattaacttcaaaaacatcgacagcgaatacatcgacggtttagttaacgagggcaaactgtttctgttccagatctattcaaaggattttagcccgttctctaaaggcaaaccaaatatgcatacgttgtactggaaagcactgtttgaagagcaaaacctgcagaatgtgatttataaactgaacggccaagctgagatttttttccgtaaagcctcgattaaaccgaaaaatatcatccttcataagaagaaaataaagatcgctaaaaaacacttcatagataaaaaaaccaaaacctccgaaatagtgcctgttcaaacaattaagaacttgaatatgtactaccagggcaagatatcggaaaaggagttgactcaagacgatcttcgctatatcgataacttttcgatttttaacgaaaaaaacaagacgatcgacatcatcaaagataaacgcttcactgtagataagttccagtttcatgtgccgattactatgaacttcaaagctaccgggggtagctatatcaaccaaacggtgttggaatacctgcagaataacccggaagtcaaaatcattgggctggaccgcggagaacgtcaccttgtgtacttgaccttaatcgatcagcaaggcaacatcttaaaacaagaatcgctgaataccattacggattcaaagattagcaccccgtatcataagctgctcgataacaaggagaatgagcgcgacctggcccgtaaaaactggggcacggtggaaaacattaaggagttaaaggagggttatatttcccaggtagtgcataagatcgccactctcatgctcgaggaaaatgcgatcgttgtcatggaagacttaaacttcggatttaaacgtgggcgatttaaagtagagaaacaaatctaccagaagttagaaaaaatgctgattgacaaattaaattacttggtcctaaaagacaaacagccgcaagaattgggtggattatacaacgccctccaacttaccaataaattcgaaagttttcagaaaatgggtaaacagtcaggctttcttttttatgttcctgcgtggaacacatccaaaatcgaccctacaaccggcttcgtcaattacttctatactaaatatgaaaacgtcgacaaagcaaaagcattctttgaaaagttcgaagcaatacgttttaacgctgagaaaaaatatttcgagttcgaagtcaagaaatactcagactttaaccccaaagctgagggcacacagcaagcgtggacaatctgcacctacggcgagcgcatcgaaacgaagcgtcaaaaagatcagaataacaaatttgtttcaacacctatcaacctgaccgagaagattgaagacttcttaggtaaaaatcagattgtttatggcgacggtaactgtataaaatctcaaatagcctcaaaggatgataaagcatttttcgaaacattattatattggttcaaaatgacactgcagatgcgcaatagtgagacgcgtacagatattgattatcttatcagcccggtcatgaacgacaacggtactttttacaactccagagactatgaaaaacttgagaatccaactctccccaaagatgctgatgcgaacggtgcttatcacatcgcgaaaaaaggtctgatgctgctgaacaaaatcgaccaagccgatctgactaagaaagttgacctaagcatttcaaatcgggactggttacagtttgttcaaaagaacaaatga

SEQ ID NO: 49 - DNA, 4023 bp, Artificial Sequence
  Description of Artificial Sequence: Synthetic polynucleotide
atggaacaggaatattatctgggcttggacatgggcaccggttccgtcggctgggctgttactgacagtgaatatcacgttctaagaaagcatggtaaggcattgtggggtgtaagacttttcgaatctgcttccactgctgaagagcgtagaatgtttagaacgagtcgacgtaggctagacaggcgcaattggagaatcgaaattttacaagaaatttttgcggaagagatatctaagaaagacccaggctttttcctgagaatgaaggaatctaagtattaccctgaggataaaagagatataaatggtaactgtcccgaattgccttacgcattatttgtggacgatgattttaccgataaggattaccataaaaagttcccaactatctaccatttacgcaaaatgttaatgaatacagaggaaaccccagacataagactagtttatctggcaatacaccatatgatgaaacatagaggccatttcttactttccggggatatcaacgaaatcaaagagtttggtaccacatttagtaagttactggaaaacataaagaatgaagaattggattggaacttagaactcggaaaagaagaatacgcggttgtcgaatctatcctgaaggataatatgctgaataggtcgaccaaaaaaactaggctgatcaaagcactgaaagccaaatctatctgcgaaaaagctgttttaaatttacttgctggtggcactgttaagttatcagacatttttggtttggaagaattgaacgaaaccgagcgtccaaaaattagtttcgctgataatggctacgatgattacattggtgaggtggaaaacgagttgggcgaacaattttatattatagagacagctaaggcagtctatgactgggctgttttagtagaaatccttggtaaatacacatctatctccgaagcgaaagttgctacttacgaaaagcacaagtccgatctccagtttttgaagaaaattgtcaggaaatatctgactaaggaagaatataaagatattttcgttagtacctctgacaaactgaaaaattactccgcttacatcgggatgaccaagattaatggcaaaaaagttgatctgcaaagcaaaaggtgttcgaaggaagaattttatgatttcattaaaaagaatgtcttaaaaaaattagaaggtcagccagaatacgaatatttgaaagaagaactggaaagagagacattcttaccaaaacaagtcaacagagataatggggtaattccatatcaaattcacctctacgaattaaaaaaaattttaggcaatttacgcgataaaattgaccttatcaaagaaaatgaggataagctggttcaactctttgaattcagaataccctattatgtgggcccactgaacaagattgatgacggcaaagaaggtaaattcacatgggccgtccgcaaatccaatgaaaaaatttacccatggaactttgaaaatgtagtagatattgaagcgtctgcggagaaatttattcgaagaatgactaataaatgcacttacttgatgggagaggatgttctgcctaaagacagcttattatacagcaagtacatggttctaaacgaacttaacaacgttaagttggacggtgagaaattaagtgtagaattgaaacaaagattgtatactgacgtcttctgcaagtacagaaaagtgacagttaaaaaaattaagaattacttgaagtgcgaaggtataatttctggaaacgtagagattactggtattgatggtgatttcaaagcatccctaacagcttaccacgatttcaaggaaatcctgacaggaactgaactcgcaaaaaaagataaagaaaacattattactaatattgttcttttcggtgatgacaagaaattgttgaagaaaagactgaatagactttacccccagattactcccaatcaacttaagaaaatttgtgctttgtcttacacaggatggggtcgtttttcaaaaaagttcttagaagagattaccgcacctgatccagaaacaggcgaagtatggaatataattaccgccttatgggaatcgaacaataatcttatgcaacttctgagcaatgaatatcgtttcatggaagaagttgagacttacaacatgggcaaacagacgaagactttatcctatgaaactgtggaaaatatgtatgtatcaccttctgtcaagagacaaatttggcaaaccttaaaaattgtcaaagaattagaaaaggtaatgaaggagtctcctaaacgtgtgtttattgaaatggctagagaaaaacaagagtcaaaaagaaccgagtcaagaaagaagcagttaatcgatttatataaggcttgtaaaaacgaagagaaagattgggttaaagaattgggggaccaagaggaacaaaaactacggtcggataagttgtatttatactatacgcaaaagggacgatgtatgtattccggcgaggtaatagaattgaaggatttatgggacaatacaaaatatgacatagaccatatatatccccaatcaaaaacgatggacgatagcttgaacaatagagtactcgtgaaaaaaaaatataatgcgaccaaatctgataagtatcctctgaatgaaaatatcagacatgaaagaaaggggttctggaagtccttgttagatggtgggtttataagcaaagaaaagtacgagcgtctaataagaaacacggagttatcgccagaagaactcgctggttttattgagaggcaaatcgtggaaacgagacaatctaccaaagccgttgctgagatcctaaagcaagttttcccagagtcggagattgtctatgtcaaagctggcacagtgagcaggtttaggaaagacttcgaactattaaaggtaagagaagtgaacgatttacatcacgcaaaggacgcttacctaaatatcgttgtaggtaactcatattatgttaaatttaccaagaacgcctcttggtttataaaggagaacccaggtagaacatataacctgaaaaagatgttcacctctggttggaatattgagagaaacggagaagtcgcatgggaagttggtaagaaagggactatagtgacagtaaagcaaattatgaacaaaaataatatcctcgttacaaggcaggttcatgaagcaaagggcggcctttttgaccaacaaattatgaagaaagggaaaggtcaaattgcaataaaagaaaccgatgagagactagcgtcaatagaaaagtatggtggctataataaagctgcgggtgcatactttatgcttgttgaatcaaaagacaagaaaggtaagactattagaactatagaatttatacccctgtaccttaaaaacaaaattgaatcggatgagtcaatcgcgttaaattttctagagaaaggaaggggtttaaaagaaccaaagatcctgttaaaaaagattaagattgacaccttgttcgatgtagatggatttaaaatgtggttatctggcagaacaggcgatagacttttgtttaagtgcgctaatcaattaattttggatgagaaaatcattgtcacaatgaaaaaaatagttaagtttattcagagaagacaagaaaacagggagttgaaattatctgataaagatggtatcgacaatgaagttttaatggaaatctacaatacattcgttgataaacttgaaaataccgtatatcgaatcaggttaagtgaacaagccaaaacattaattgataaacaaaaagaatttgaaaggctatcactggaagacaaatcctccaccctatttgaaattttgcatatattccagtgccaatcttcagcagctaatttaaaaatgattggcggacctgggaaagccggcatcctagtgatgaacaataatatctccaagtgtaacaaaatatcaattattaaccaatctccgacaggtatttttgaaaatgaaatagacttgcttaagatataa

SEQ ID NO: 50 - DNA, 3831 bp, Artificial Sequence
  Description of Artificial Sequence: Synthetic polynucleotide
atgtctttcgactctttcaccaacctgtactctctgtctaaaaccctgaaattcgaaatgcgtccggttggtaacacccagaaaatgctggacaacgcgggtgttttcgaaaaagacaaactgatccagaaaaaatacggtaaaaccaaaccgtacttcgaccgtctgcaccgtgaattcatcgaagaagcgctgaccggtgttgaactgatcggtctggacgaaaacttccgtaccctggttgactggcagaaagacaaaaaaaacaacgttgcgatgaaagcgtacgaaaactctctgcagcgtctgcgtaccgaaatcggtaaaatcttcaacctgaaagcggaagactgggttaaaaacaaatacccgatcctgggtctgaaaaacaaaaacaccgacatcctgttcgaagaagcggttttcggtatcctgaaagcgcgttacggtgaagaaaaagacaccttcatcgaagttgaagaaatcgacaaaaccggtaaatctaaaatcaaccagatctctatcttcgactcttggaaaggtttcaccggttacttcaaaaaattcttcgaaacccgtaaaaacttctacaaaaacgacggtacctctaccgcgatcgcgacccgtatcatcgaccagaacctgaaacgtttcatcgacaacctgtctatcgttgaatctgttcgtcagaaagttgacctggcggaaaccgaaaaatctttctctatctctctgtctcagttcttctctatcgacttctacaacaaatgcctgctgcaggacggtatcgactactacaacaaaatcatcggtggtgaaaccctgaaaaacggtgaaaaactgatcggtctgaacgaactgatcaaccagtaccgtcagaacaacaaagaccagaaaatcccgttcttcaaactgctggacaaacagatcctgtctgaaaaaatcctgttcctggacgaaatcaaaaacgacaccgaactgatcgaagcgctgtctcagttcgcgaaaaccgcggaagaaaaaaccaaaatcgttaaaaaactgttcgcggacttcgttgaaaacaactctaaatacgacctggcgcagatctacatctctcaggaagcgttcaacaccatctctaacaaatggacctctgaaaccgaaaccttcgcgaaatacctgttcgaagcgatgaaatctggtaaactggcgaaatacgaaaaaaaagacaactcttacaaattcccggacttcatcgcgctgtctcagatgaaatctgcgctgctgtctatctctctggaaggtcacttctggaaagaaaaatactacaaaatctctaaattccaggaaaaaaccaactgggaacagttcctggcgatcttcctgtacgaattcaactctctgttctctgacaaaatcaacaccaaagacggtgaaaccaaacaggttggttactacctgttcgcgaaagacctgcacaacctgatcctgtctgaacagatcgacatcccgaaagactctaaagttaccatcaaagacttcgcggactctgttctgaccatctaccagatggcgaaatacttcgcggttgaaaaaaaacgtgcgtggctggcggaatacgaactggactctttctacacccagccggacaccggttacctgcagttctacgacaacgcgtacgaagacatcgttcaggtttacaacaaactgcgtaactacctgaccaaaaaaccgtactctgaagaaaaatggaaactgaacttcgaaaactctaccctggcgaacggttgggacaaaaacaaagaatctgacaactctgcggttatcctgcagaaaggtggtaaatactacctgggtctgatcaccaaaggtcacaacaaaatcttcgacgaccgtttccaggaaaaattcatcgttggtatcgaaggtggtaaatacgaaaaaatcgtttacaaattcttcccggaccaggcgaaaatgttcccgaaagtttgcttctctgcgaaaggtctggaattcttccgtccgtctgaagaaatcctgcgtatctacaacaacgcggaattcaaaaaaggtgaaacctactctatcgactctatgcagaaactgatcgacttctacaaagactgcctgaccaaatacgaaggttgggcgtgctacaccttccgtcacctgaaaccgaccgaagaataccagaacaacatcggtgaattcttccgtgacgttgcggaagacggttaccgtatcgacttccagggtatctctgaccagtacatccacgaaaaaaacgaaaaaggtgaactgcacctgttcgaaatccacaacaaagactggaacctggacaaagcgcgtgacggtaaatctaaaaccacccagaaaaacctgcacaccctgtacttcgaatctctgttctctaacgacaacgttgttcagaacttcccgatcaaactgaacggtcaggcggaaatcttctaccgtccgaaaaccgaaaaagacaaactggaatctaaaaaagacaaaaaaggtaacaaagttatcgaccacaaacgttactctgaaaacaaaatcttcttccacgttccgctgaccctgaaccgtaccaaaaacgactcttaccgtttcaacgcgcagatcaacaacttcctggcgaacaacaaagacatcaacatcatcggtgttgaccgtggtgaaaaacacctggtttactactctgttatcacccaggcgtctgacatcctggaatctggttctctgaacgaactgaacggtgttaactacgcggaaaaactgggtaaaaaagcggaaaaccgtgaacaggcgcgtcgtgactggcaggacgttcagggtatcaaagacctgaaaaaaggttacatctctcaggttgttcgtaaactggcggacctggcgatcaaacacaacgcgatcatcatcctggaagacctgaacatgcgtttcaaacaggttcgtggtggtatcgaaaaatctatctaccagcagctggaaaaagcgctgatcgacaaactgtctttcctggttgacaaaggtgaaaaaaacccggaacaggcgggtcacctgctgaaagcgtaccagctgtctgcgccgttcgaaaccttccagaaaatgggtaaacagaccggtatcatcttctacacccaggcgtcttacacctctaaatctgacccggttaccggttggcgtccgcacctgtacctgaaatacttctctgcgaaaaaagcgaaagacgacatcgcgaaattcaccaaaatcgaattcgttaacgaccgtttcgaactgacctacgacatcaaagacttccagcaggcgaaagaatacccgaacaaaaccgtttggaaagtttgctctaacgttgaacgtttccgttgggacaaaaacctgaaccagaacaaaggtggttacacccactacaccaacatcaccgaaaacatccaggaactgttcaccaaatacggtatcgacatcaccaaagacctgctgacccagatctctaccatcgacgaaaaacagaacacctctttcttccgtgacttcatcttctacttcaacctgatctgccagatccgtaacaccgacgactctgaaatcgcgaaaaaaaacggtaaagacgacttcatcctgtctccggttgaaccgttcttcgactctcgtaaagacaacggtaacaaactgccggaaaacggtgacgacaacggtgcgtacaacatcgcgcgtaaaggtatcgttatcctgaacaaaatctctcagtactctgaaaaaaacgaaaactgcgaaaaaatgaaatggggtgacctgtacgtttctaacatcgactgggacaacttcgtt

SEQ ID NO: 51 - DNA, 3465 bp, Artificial Sequence
  Description of Artificial Sequence: Synthetic polynucleotide
atggaaaactttaaaaacttatacccaataaacaaaacgttacgttttgaactgcgtccatatggtaaaacactggaaaactttaaaaaaagcggtttgttggagaaggatgcatttaaagcgaactctcgcagatccatgcaggccatcattgatgaaaaatttaaagagacgatcgaagaacgtctgaaatacacggaatttagtgagtgtgacttaggtaatatgacttctaaagataagaaaatcaccgataaggcggcgaccaacctgaagaagcaagtcattttatcttttgatgatgaaatctttaacaactatttgaaaccggacaaaaacatcgatgccttatttaaaaatgacccttcgaacccggtgattagcacatttaagggcttcacaacgtattttgtcaatttttttgaaattcgtaaacatatcttcaaaggagaatcaagcggctctatggcttatcgcattattgatgaaaacctgacgacctatttgaataacattgaaaaaatcaaaaaactgccagaggaattaaagtctcagttagaaggcatcgaccagatcgacaaactcaacaactataacgaatttattacgcagtctggtatcacccactataatgaaattattggaggtatcagtaaatcagaaaatgtgaaaatccaagggattaatgaaggcattaacctctattgccagaaaaataaagtgaaactgccgaggctgactccactctacaaaatgatcctgtctgaccgcgtctcgaatagctttgtcctggacacaattgaaaacgatacggaattgattgagatgataagcgatctgattaacaaaaccgaaatttcacaggatgtaatcatgagtgatatacaaaacatctttattaaatataaacagcttggtaatctgcctggaattagctattcgtcaatagtgaacgcaatctgttctgattatgataacaattttggcgacggtaagcgtaaaaagagttatgaaaacgataggaaaaaacacctggaaactaacgtgtattctatcaactatatcagcgaactgcttacggacaccgatgtgagttcaaacattaagatgcggtataaggagcttgaacagaactaccaggtctgtaaggaaaacttcaacgcaaccaactggatgaacattaaaaatatcaaacaatccgagaagaccaacttaatcaaagatctgctggatattttgaagagcattcaacgtttttatgatctgttcgatatcgttgatgaagacaagaatcctagtgcggaattttatacatggctgtctaaaaatgcggagaaattggatttcgaattcaattctgtttataataaatcacgcaactatttgacccgcaaacaatacagcgacaaaaagataaaactaaacttcgacagtccgacattggcaaagggctgggacgcaaataaggaaatcgataactctacgataattatgcgtaagttcaataatgatcgaggtgattatgattatttcttaggcatttggaacaaaagcaccccggccaacgaaaagataattccactggaggataacggtctgttcgaaaaaatgcagtacaaattatatccggatccaagcaagatgcttccaaagcagtttctgtctaaaatttggaaagctaagcatccgaccaccccagaatttgacaagaaatataaggaaggccgccataagaaaggtcccgattttgaaaaagaattcttgcacgaactgattgattgctttaaacatggcttagtcaatcacgatgaaaagtatcaagatgtttttggattcaatttgagaaacacagaagactacaattcctacactgagtttctcgaagatgtggaacgatgtaattataatctgagctttaacaaaatcgcggacacctcgaatctgattaacgatggtaaactttatgttttccagatctggagcaaggatttctctattgacagcaaaggcaccaaaaacctgaacaccatttactttgaaagtctcttcagcgaagaaaatatgattgagaaaatgtttaaacttagcggtgaagctgaaatattctatcgcccggcaagcctgaactattgcgaagacattatcaaaaagggtcatcaccacgctgaactgaaagataaatttgattatcctatcataaaagataaacgctatagccaggataaatttttttttcatgttcctatggtcattaactacaaatcagaaaaactgaactctaaaagcctcaataatcgaaccaatgaaaaccttgggcagtttacccatataattggaattgatcgcggagagcgtcatttaatctacctgaccgtagtcgatgtatcgaccggcgagatcgtcgagcagaagcacttagacgagattatcaacactgataccaaaggtgttgagcataagacgcactatctaaacaagctggaggaaaaatcgaaaacccgtgataatgaacgtaagagttgggaggcaattgaaacgattaaagaactgaaggagggttatatcagccacgtaatcaatgaaattcaaaaactgcaggaaaaatacaacgccctgatcgttatggaaaatctgaattacggtttcaaaaattctcgcatcaaagtggaaaaacaggtatatcagaagttcgagacggcattaattaaaaagtttaattacatcattgacaaaaaagatccggaaacttatattcatggctatcagctgacgaacccgatcaccacactggataaaattggtaaccagtctggtatcgtgctttacatccctgcctggaataccagtaaaatcgatccggtaacgggattcgtcaaccttctatatgcagatgacctcaaatataagaatcaggaacaggccaagtcttttattcagaaaatcgataacatttactttgagaatggggaattcaaatttgatattgatttttctaaatggaacaatcgttatagtatatctaagacgaaatggacgctcacctcgtacggaacccgaatccagacattccgcaatccgcagaagaacaataaatgggacagcgccgagtatgatctcactgaagaattcaaattgattctgaacattgacggtaccctgaaaagccaggatgtcgaaacctataaaaaatttatgtctctgttcaagctgatgctgcaacttaggaactctgttaccggcactgatatcgattatatgatctcccctgtcactgataaaacaggtacgcatttcgattcgcgcgaaaatatcaaaaatctgcccgcagatgccgacgccaatggggcgtacaatattgcacgcaagggtatcatggcgatcgaaaacattatgaatggtatcagcgacccgctgaaaatctcaaacgaagattatttgaaatatatccaaaaccagcaggaataa

SEQ ID NO: 52 - DNA, 3923 bp, Artificial Sequence
  Description of Artificial Sequence: Synthetic polynucleotide
atgacccagttcgaaggtttcaccaacctgtaccaggtttctaaaaccctgcgtttcgaactgatcccgcagggtaaaaccctgaaacacatccaggaacagggtttcatcgaagaagacaaagcgcgtaacgaccactacaaagaactgaaaccgatcatcgaccgtatctacaaaacctacgcggaccagtgcctgcagctggttcagctggactgggaaaacctgtctgcggcgatcgactcttaccgtaaagaaaaaaccgaagaaacccgtaacgcgctgatcgaagaacaggcgacctaccgtaacgcgatccacgactacttcatcggtcgtaccgacaacctgaccgacgcgatcaacaaacgtcacgcggaaatctacaaaggtctgttcaaagcggaactgttcaacggtaaagttctgaaacagctgggtaccgttaccaccaccgaacacgaaaacgcgctgctgcgttctttcgacaaattcaccacctacttctctggtttctacgaaaaccgtaaaaacgttttctctgcggaagacatctctaccgcgatcccgcaccgtatcgttcaggacaacttcccgaaattcaaagaaaactgccacatcttcacccgtctgatcaccgcggttccgtctctgcgtgaacacttcgaaaacgttaaaaaagcgatcggtatcttcgtttctacctctatcgaagaagttttctctttcccgttctacaaccagctgctgacccagacccagatcgacctgtacaaccagctgctgggtggtatctctcgtgaagcgggtaccgaaaaaatcaaaggtctgaacgaagttctgaacctggcgatccagaaaaacgacgaaaccgcgcacatcatcgcgtctctgccgcaccgtttcatcccgctgttcaaacagatcctgtctgaccgtaacaccctgtctttcatcctggaagaattcaaatctgacgaagaagttatccagtctttctgcaaatacaaaaccctgctgcgtaacgaaaacgttctggaaaccgcggaagcgctgttcaacgaactgaactctatcgacctgacccacatcttcatctctcacaaaaaactggaaaccatctcttctgcgctgtgcgaccactgggacaccctgcgtaacgcgctgtacgaacgtcgtatctctgaactgaccggtaaaatcaccaaatctgcgaaagaaaaagttcagcgttctctgaaacacgaagacatcaacctgcaggaaatcatctctgcggcgggtaaagaactgtctgaagcgttcaaacagaaaacctctgaaatcctgtctcacgcgcacgcggcgctggaccagccgctgccgaccaccctgaaaaaacaggaagaaaaagaaatcctgaaatctcagctggactctctgctgggtctgtaccacctgctggactggttcgcggttgacgaatctaacgaagttgacccggaattctctgcgcgtctgaccggtatcaaactggaaatggaaccgtctctgtctttctacaacaaagcgcgtaactacgcgaccaaaaaaccgtactctgttgaaaaattcaaactgaacttccagatgccgaccctggcgtctggttgggacgttaacaaagaaaaaaacaacggtgcgatcctgttcgttaaaaacggtctgtactacctgggtatcatgccgaaacagaaaggtcgttacaaagcgctgtctttcgaaccgaccgaaaaaacctctgaaggtttcgacaaaatgtactacgactacttcccggacgcggcgaaaatgatcccgaaatgctctacccagctgaaagcggttaccgcgcacttccagacccacaccaccccgatcctgctgtctaacaacttcatcgaaccgctggaaatcaccaaagaaatctacgacctgaacaacccggaaaaagaaccgaaaaaattccagaccgcgtacgcgaaaaaaaccggtgaccagaaaggttaccgtgaagcgctgtgcaaatggatcgacttcacccgtgacttcctgtctaaatacaccaaaaccacctctatcgacctgtcttctctgcgtccgtcttctcagtacaaagacctgggtgaatactacgcggaactgaacccgctgctgtaccacatctctttccagcgtatcgcggaaaaagaaatcatggacgcggttgaaaccggtaaactgtacctgttccagatctacaacaaagacttcgcgaaaggtcaccacggtaaaccgaacctgcacaccctgtactggaccggtctgttctctccggaaaacctggcgaaaacctctatcaaactgaacggtcaggcggaactgttctaccgtccgaaatctcgtatgaaacgtatggcgcaccgtctgggtgaaaaaatgctgaacaaaaaactgaaagaccagaaaaccccgatcccggacaccctgtaccaggaactgtacgactacgttaaccaccgtctgtctcacgacctgtctgacgaagcgcgtgcgctgctgccgaacgttatcaccaaagaagtttctcacgaaatcatcaaagaccgtcgtttcacctctgacaaattcttcttccacgttccgatcaccctgaactaccaggcggcgaactctccgtctaaattcaaccagcgtgttaacgcgtacctgaaagaacacccggaaaccccgatcatcggtatcgaccgtggtgaacgtaacctgatctacatcaccgttatcgactctaccggtaaaatcctggaacagcgttctctgaacaccatccagcagttcgactaccagaaaaaactggacaaccgtgaaaaagaacgtgttgcggcgcgtcaggcgtggtctgttgttggtaccatcaaagacctgaaacagggttacctgtctcaggttatccacgaaatcgttgacctgatgatccactaccaggcggttgttgttctggaaaacctgaacttcggtttcaaatctaaacgtaccggtatcgcggaaaaagcggtttaccagcagttcgaaaaaatgctgatcgacaaactgaactgcctggttctgaaagactacccggcggaaaaagttggtggtgttctgaacccgtaccagctgaccgaccagttcacctctttcgcgaaaatgggtacccagtctggtttcctgttctacgttccggcgccgtacacctctaaaatcgacccgctgaccggtttcgttgacccgttcgtttggaaaaccatcaaaaaccacgaatctcgtaaacacttcctggaaggtttcgacttcctgcactacgacgttaaaaccggtgacttcatcctgcacttcaaaatgaaccgtaacctgtctttccagcgtggtctgccgggtttcatgccggcgtgggacatcgttttcgaaaaaaacgaaacccagttcgacgcgaaaggtaccccgttcatcgcgggtaaacgtatcgttccggttatcgaaaaccaccgtttcaccggtcgttaccgtgacctgtacccggcgaacgaactgatcgcgctgctggaagaaaaaggtatcgttttccgtgacggttctaacatcctgccgaaactgctggaaaacgacgactctcacgcgatcgacaccatggttgcgctgatccgttctgttctgcagatgcgtaactctaacgcggcgaccggtgaagactacatcaactctccggttcgtgacctgaacggtgtttgcttcgactctcgtttccagaacccggaatggccgatggacgcggacgcgaacggtgcgtaccacatcgcgctgaaaggtcagctgctgctgaaccacctgaaagaatctaaagacctgaaactgcagaacggtatctctaaccaggactggctggcgtacatccaggaactgcgtaacta

SEQ ID NO: 53 - DNA, 3390 bp, Artificial Sequence
  Description of Artificial Sequence: Synthetic polynucleotide
atggcggttaaatctatcaaagttaaactgcgtctggacgacatgccggaaatccgtgcgggtctgtggaaactgcacaaagaagttaacgcgggtgttcgttactacaccgaatggctgtctctgctgcgtcaggaaaacctgtaccgtcgttctccgaacggtgacggtgaacaggaatgcgacaaaaccgcggaagaatgcaaagcggaactgctggaacgtctgcgtgcgcgtcaggttgaaaacggtcaccgtggtccggcgggttctgacgacgaactgctgcagctggcgcgtcagctgtacgaactgctggttccgcaggcgatcggtgcgaaaggtgacgcgcagcagatcgcgcgtaaattcctgtctccgctggcggacaaagacgcggttggtggtctgggtatcgcgaaagcgggtaacaaaccgcgttgggttcgtatgcgtgaagcgggtgaaccgggttgggaagaagaaaaagaaaaagcggaaacccgtaaatctgcggaccgtaccgcggacgttctgcgtgcgctggcggacttcggtctgaaaccgctgatgcgtgtttacaccgactctgaaatgtcttctgttgaatggaaaccgctgcgtaaaggtcaggcggttcgtacctgggaccgtgacatgttccagcaggcgatcgaacgtatgatgtcttgggaatcttggaaccagcgtgttggtcaggaatacgcgaaactggttgaacagaaaaaccgtttcgaacagaaaaacttcgttggtcaggaacacctggttcacctggttaaccagctgcagcaggacatgaaagaagcgtctccgggtctggaatctaaagaacagaccgcgcactacgttaccggtcgtgcgctgcgtggttctgacaaagttttcgaaaaatggggtaaactggcgccggacgcgccgttcgacctgtacgacgcggaaatcaaaaacgttcagcgtcgtaacacccgtcgtttcggttctcacgacctgttcgcgaaactggcggaaccggaataccaggcgctgtggcgtgaagacgcgtctttcctgacccgttacgcggtttacaactctatcctgcgtaaactgaaccacgcgaaaatgttcgcgaccttcaccctgccggacgcgaccgcgcacccgatctggacccgtttcgacaaactgggtggtaacctgcaccagtacaccttcctgttcaacgaattcggtgaacgtcgtcacgcgatccgtttccacaaactgctgaaagttgaaaacggtgttgcgcgtgaagttgacgacgttaccgttccgatctctatgtctgaacagctggacaacctgctgccgcgtgacccgaacgaaccgatcgcgctgtacttccgtgactacggtgcggaacagcacttcaccggtgaattcggtggtgcgaaaatccagtgccgtcgtgaccagctggcgcacatgcaccgtcgtcgtggtgcgcgtgacgtttacctgaacgtttctgttcgtgttcagtctcagtctgaagcgcgtggtgaacgtcgtccgccgtacgcggcggttttccgtctggttggtgacaaccaccgtgcgttcgttcacttcgacaaactgtctgactacctggcggaacacccggacgacggtaaactgggttctgaaggtctgctgtctggtctgcgtgttatgtctgttgacctgggtctgcgtacctctgcgtctatctctgttttccgtgttgcgcgtaaagacgaactgaaaccgaactctaaaggtcgtgttccgttcttcttcccgatcaaaggtaacgacaacctggttgcggttcacgaacgttctcagctgctgaaactgccgggtgaaaccgaatctaaagacctgcgtgcgatccgtgaagaacgtcagcgtaccctgcgtcagctgcgtacccagctggcgtacctgcgtctgctggttcgttgcggttctgaagacgttggtcgtcgtgaacgttcttgggcgaaactgatcgaacagccggttgacgcggcgaaccacatgaccccggactggcgtgaagcgttcgaaaacgaactgcagaaactgaaatctctgcacggtatctgctctgacaaagaatggatggacgcggtttacgaatctgttcgtcgtgtttggcgtcacatgggtaaacaggttcgtgactggcgtaaagacgttcgttctggtgaacgtccgaaaatccgtggttacgcgaaagacgttgttggtggtaactctatcgaacagatcgaatacctggaacgtcagtacaaattcctgaaatcttggtctttcttcggtaaagtttctggtcaggttatccgtgcggaaaaaggttctcgtttcgcgatcaccctgcgtgaacacatcgaccacgcgaaagaagaccgtctgaaaaaactggcggaccgtatcatcatggaagcgctgggttacgtttacgcgctggacgaacgtggtaaaggtaaatgggttgcgaaatacccgccgtgccagctgatcctgctggaagaactgtctgaataccagttcaacaacgaccgtccgccgtctgaaaacaaccagctgatgcagtggtctcaccgtggtgttttccaggaactgatcaaccaggcgcaggttcacgacctgctggttggtaccatgtacgcggcgttctcttctcgtttcgacgcgcgtaccggtgcgccgggtatccgttgccgtcgtgttccggcgcgttgcacccaggaacacaacccggaaccgttcccgtggtggctgaacaaattcgttgttgaacacaccctggacgcgtgcccgctgcgtgcggacgacctgatcccgaccggtgaaggtgaaatcttcgtttctccgttctctgcggaagaaggtgacttccaccagatccacgcggacctgaacgcggcgcagaacctgcagcagcgtctgtggtctgacttcgacatctctcagatccgtctgcgttgcgactggggtgaagttgacggtgaactggttctgatcccgcgtctgaccggtaaacgtaccgcggactcttactctaacaaagttttctacaccaacaccggtgttacctactacgaacgtgaacgtggtaaaaaacgtcgtaaagttttcgcgcaggaaaaactgtctgaagaagaagcggaactgctggttgaagcggacgaagcgcgtgaaaaatctgttgttctgatgcgtgacccgtctggtatcatcaaccgtggtaactggacccgtcagaaagaattctggtctatggttaaccagcgtatcgaaggttacctggttaaacagatccgttctcgtgttccgctgcaggactctgcgtgcgaaaacaccggtgacatctaa

SEQ ID NO: 54 - DNA, 3327 bp, Artificial Sequence
  Description of Artificial Sequence: Synthetic polynucleotide
atggcgacccgttctttcatcctgaaaatcgaaccgaacgaagaagttaaaaaaggtctgtggaaaacccacgaagttctgaaccacggtatcgcgtactacatgaacatcctgaaactgatccgtcaggaagcgatctacgaacaccacgaacaggacccgaaaaacccgaaaaaagtttctaaagcggaaatccaggcggaactgtgggacttcgttctgaaaatgcagaaatgcaactctttcacccacgaagttgacaaagacgttgttttcaacatcctgcgtgaactgtacgaagaactggttccgtcttctgttgaaaaaaaaggtgaagcgaaccagctgtctaacaaattcctgtacccgctggttgacccgaactctcagtctggtaaaggtaccgcgtcttctggtcgtaaaccgcgttggtacaacctgaaaatcgcgggtgacccgtcttgggaagaagaaaaaaaaaaatgggaagaagacaaaaaaaaagacccgctggcgaaaatcctgggtaaactggcggaatacggtctgatcccgctgttcatcccgttcaccgactctaacgaaccgatcgttaaagaaatcaaatggatggaaaaatctcgtaaccagtctgttcgtcgtctggacaaagacatgttcatccaggcgctggaacgtttcctgtcttgggaatcttggaacctgaaagttaaagaagaatacgaaaaagttgaaaaagaacacaaaaccctggaagaacgtatcaaagaagacatccaggcgttcaaatctctggaacagtacgaaaaagaacgtcaggaacagctgctgcgtgacaccctgaacaccaacgaataccgtctgtctaaacgtggtctgcgtggttggcgtgaaatcatccagaaatggctgaaaatggacgaaaacgaaccgtctgaaaaatacctggaagttttcaaagactaccagcgtaaacacccgcgtgaagcgggtgactactctgtttacgaattcctgtctaaaaaagaaaaccacttcatctggcgtaaccacccggaatacccgtacctgtacgcgaccttctgcgaaatcgacaaaaaaaaaaaagacgcgaaacagcaggcgaccttcaccctggcggacccgatcaaccacccgctgtgggttcgtttcgaagaacgttctggttctaacctgaacaaataccgtatcctgaccgaacagctgcacaccgaaaaactgaaaaaaaaactgaccgttcagctggaccgtctgatctacccgaccgaatctggtggttgggaagaaaaaggtaaagttgacatcgttctgctgccgtctcgtcagttctacaaccagatcttcctggacatcgaagaaaaaggtaaacacgcgttcacctacaaagacgaatctatcaaattcccgctgaaaggtaccctgggtggtgcgcgtgttcagttcgaccgtgaccacctgcgtcgttacccgcacaaagttgaatctggtaacgttggtcgtatctacttcaacatgaccgttaacatcgaaccgaccgaatctccggtttctaaatctctgaaaatccaccgtgacgacttcccgaaattcgttaacttcaaaccgaaagaactgaccgaatggatcaaagactctaaaggtaaaaaactgaaatctggtatcgaatctctggaaatcggtctgcgtgttatgtctatcgacctgggtcagcgtcaggcggcggcggcgtctatcttcgaagttgttgaccagaaaccggacatcgaaggtaaactgttcttcccgatcaaaggtaccgaactgtacgcggttcaccgtgcgtctttcaacatcaaactgccgggtgaaaccctggttaaatctcgtgaagttctgcgtaaagcgcgtgaagacaacctgaaactgatgaaccagaaactgaacttcctgcgtaacgttctgcacttccagcagttcgaagacatcaccgaacgtgaaaaacgtgttaccaaatggatctctcgtcaggaaaactctgacgttccgctggtttaccaggacgaactgatccagatccgtgaactgatgtacaaaccgtacaaagactgggttgcgttcctgaaacagctgcacaaacgtctggaagttgaaatcggtaaagaagttaaacactggcgtaaatctctgtctgacggtcgtaaaggtctgtacggtatctctctgaaaaacatcgacgaaatcgaccgtacccgtaaattcctgctgcgttggtctctgcgtccgaccgaaccgggtgaagttcgtcgtctggaaccgggtcagcgtttcgcgatcgaccagctgaaccacctgaacgcgctgaaagaagaccgtctgaaaaaaatggcgaacaccatcatcatgcacgcgctgggttactgctacgacgttcgtaaaaaaaaatggcaggcgaaaaacccggcgtgccagatcatcctgttcgaagacctgtctaactacaacccgtacgaagaacgttctcgtttcgaaaactctaaactgatgaaatggtctcgtcgtgaaatcccgcgtcaggttgcgctgcagggtgaaatctacggtctgcaggttggtgaagttggtgcgcagttctcttctcgtttccacgcgaaaaccggttctccgggtatccgttgctctgttgttaccaaagaaaaactgcaggacaaccgtttcttcaaaaacctgcagcgtgaaggtcgtctgaccctggacaaaatcgcggttctgaaagaaggtgacctgtacccggacaaaggtggtgaaaaattcatctctctgtctaaagaccgtaaactggttaccacccacgcggacatcaacgcggcgcagaacctgcagaaacgtttctggacccgtacccacggtttctacaaagtttactgcaaagcgtaccaggttgacggtcagaccgtttacatcccggaatctaaagaccagaaacagaaaatcatcgaagaattcggtgaaggttacttcatcctgaaagacggtgtttacgaatggggtaacgcgggtaaactgaaaatcaaaaaaggttcttctaaacagtcttcttctgaactggttgactctgacatcctgaaagactctttcgacctggcgtctgaactgaaaggtgaaaaactgatgctgtaccgtgacccgtctggtaacgttttcccgtctgacaaatggatggcggcgggtgttttcttcggtaaactggaacgtatcctgatctctaaactgaccaaccagtactctatctctaccatcgaagacgactcttctaaacagtctatgtaa

SEQ ID NO: 55 - DNA, 3450 bp, Artificial Sequence
  Description of Artificial Sequence: Synthetic polynucleotide
atgccgacccgtaccatcaacctgaaactggttctgggtaaaaacccggaaaacgcgaccctgcgtcgtgcgctgttctctacccaccgtctggttaaccaggcgaccaaacgtatcgaagaattcctgctgctgtgccgtggtgaagcgtaccgtaccgttgacaacgaaggtaaagaagcggaaatcccgcgtcacgcggttcaggaagaagcgctggcgttcgcgaaagcggcgcagcgtcacaacggttgcatctctacctacgaagaccaggaaatcctggacgttctgcgtcagctgtacgaacgtctggttccgtctgttaacgaaaacaacgaagcgggtgacgcgcaggcggcgaacgcgtgggtttctccgctgatgtctgcggaatctgaaggtggtctgtctgtttacgacaaagttctggacccgccgccggtttggatgaaactgaaagaagaaaaagcgccgggttgggaagcggcgtctcagatctggatccagtctgacgaaggtcagtctctgctgaacaaaccgggttctccgccgcgttggatccgtaaactgcgttctggtcagccgtggcaggacgacttcgtttctgaccagaaaaaaaaacaggacgaactgaccaaaggtaacgcgccgctgatcaaacagctgaaagaaatgggtctgctgccgctggttaacccgttcttccgtcacctgctggacccggaaggtaaaggtgtttctccgtgggaccgtctggcggttcgtgcggcggttgcgcacttcatctcttgggaatcttggaaccaccgtacccgtgcggaatacaactctctgaaactgcgtcgtgacgaattcgaagcggcgtctgacgaattcaaagacgacttcaccctgctgcgtcagtacgaagcgaaacgtcactctaccctgaaatctatcgcgctggcggacgactctaacccgtaccgtatcggtgttcgttctctgcgtgcgtggaaccgtgttcgtgaagaatggatcgacaaaggtgcgaccgaagaacagcgtgttaccatcctgtctaaactgcagacccagctgcgtggtaaattcggtgacccggacctgttcaactggctggcgcaggaccgtcacgttcacctgtggtctccgcgtgactctgttaccccgctggttcgtatcaacgcggttgacaaagttctgcgtcgtcgtaaaccgtacgcgctgatgaccttcgcgcacccgcgtttccacccgcgttggatcctgtacgaagcgccgggtggttctaacctgcgtcagtacgcgctggactgcaccgaaaacgcgctgcacatcaccctgccgctgctggttgacgacgcgcacggtacctggatcgaaaaaaaaatccgtgttccgctggcgccgtctggtcagatccaggacctgaccctggaaaaactggaaaaaaaaaaaaaccgtctgtactaccgttctggtttccagcagttcgcgggtctggcgggtggtgcggaagttctgttccaccgtccgtacatggaacacgacgaacgttctgaagaatctctgctggaacgtccgggtgcggtttggttcaaactgaccctggacgttgcgacccaggcgccgccgaactggctggacggtaaaggtcgtgttcgtaccccgccggaagttcaccacttcaaaaccgcgctgtctaacaaatctaaacacacccgtaccctgcagccgggtctgcgtgttctgtctgttgacctgggtatgcgtaccttcgcgtcttgctctgttttcgaactgatcgaaggtaaaccggaaaccggtcgtgcgttcccggttgcggacgaacgttctatggactctccgaacaaactgtgggcgaaacacgaacgttctttcaaactgaccctgccgggtgaaaccccgtctcgtaaagaagaagaagaacgttctatcgcgcgtgcggaaatctacgcgctgaaacgtgacatccagcgtctgaaatctctgctgcgtctgggtgaagaagacaacgacaaccgtcgtgacgcgctgctggaacagttcttcaaaggttggggtgaagaagacgttgttccgggtcaggcgttcccgcgttctctgttccagggtctgggtgcggcgccgttccgttctaccccggaactgtggcgtcagcactgccagacctactacgacaaagcggaagcgtgcctggcgaaacacatctctgactggcgtaaacgtacccgtccgcgtccgacctctcgtgaaatgtggtacaaaacccgttcttaccacggtggtaaatctatctggatgctggaatacctggacgcggttcgtaaactgctgctgtcttggtctctgcgtggtcgtacctacggtgcgatcaaccgtcaggacaccgcgcgtttcggttctctggcgtctcgtctgctgcaccacatcaactctctgaaagaagaccgtatcaaaaccggtgcggactctatcgttcaggcggcgcgtggttacatcccgctgccgcacggtaaaggttgggaacagcgttacgaaccgtgccagctgatcctgttcgaagacctggcgcgttaccgtttccgtgttgaccgtccgcgtcgtgaaaactctcagctgatgcagtggaaccaccgtgcgatcgttgcggaaaccaccatgcaggcggaactgtacggtcagatcgttgaaaacaccgcggcgggtttctcttctcgtttccacgcggcgaccggtgcgccgggtgttcgttgccgtttcctgctggaacgtgacttcgacaacgacctgccgaaaccgtacctgctgcgtgaactgtcttggatgctgggtaacaccaaagttgaatctgaagaagaaaaactgcgtctgctgtctgaaaaaatccgtccgggttctctggttccgtgggacggtggtgaacagttcgcgaccctgcacccgaaacgtcagaccctgtgcgttatccacgcggacatgaacgcggcgcagaacctgcagcgtcgtttcttcggtcgttgcggtgaagcgttccgtctggtttgccagccgcacggtgacgacgttctgcgtctggcgtctaccccgggtgcgcgtctgctgggtgcgctgcagcagctggaaaacggtcagggtgcgttcgaactggttcgtgacatgggttctacctctcagatgaaccgtttcgttatgaaatctctgggtaaaaaaaaaatcaaaccgctgcaggacaacaacggtgacgacgaactggaagacgttctgtctgttctgccggaagaagacgacaccggtcgtatcaccgttttccgtgactcttctggtatcttcttcccgtgcaacgtttggatcccggcgaaacagttctggccggcggttcgtgcgatgatctggaaagttatggcgtctcactctctgggttaa

SEQ ID NO: 56 - DNA, 3759 bp, Artificial Sequence
  Description of Artificial Sequence: Synthetic polynucleotide
atgaccaaactgcgtcaccgtcagaaaaaactgacccacgactgggcgggttctaaaaaacgtgaagttctgggttctaacggtaaactgcagaacccgctgctgatgccggttaaaaaaggtcaggttaccgaattccgtaaagcgttctctgcgtacgcgcgtgcgaccaaaggtgaaatgaccgacggtcgtaaaaacatgttcacccactctttcgaaccgttcaaaaccaaaccgtctctgcaccagtgcgaactggcggacaaagcgtaccagtctctgcactcttacctgccgggttctctggcgcacttcctgctgtctgcgcacgcgctgggtttccgtatcttctctaaatctggtgaagcgaccgcgttccaggcgtcttctaaaatcgaagcgtacgaatctaaactggcgtctgaactggcgtgcgttgacctgtctatccagaacctgaccatctctaccctgttcaacgcgctgaccacctctgttcgtggtaaaggtgaagaaacctctgcggacccgctgatcgcgcgtttctacaccctgctgaccggtaaaccgctgtctcgtgacacccagggtccggaacgtgacctggcggaagttatctctcgtaaaatcgcgtcttctttcggtacctggaaagaaatgaccgcgaacccgctgcagtctctgcagttcttcgaagaagaactgcacgcgctggacgcgaacgtttctctgtctccggcgttcgacgttctgatcaaaatgaacgacctgcagggtgacctgaaaaaccgtaccatcgttttcgacccggacgcgccggttttcgaatacaacgcggaagacccggcggacatcatcatcaaactgaccgcgcgttacgcgaaagaagcggttatcaaaaaccagaacgttggtaactacgttaaaaacgcgatcaccaccaccaacgcgaacggtctgggttggctgctgaacaaaggtctgtctctgctgccggtttctaccgacgacgaactgctggaattcatcggtgttgaacgttctcacccgtcttgccacgcgctgatcgaactgatcgcgcagctggaagcgccggaactgttcgaaaaaaacgttttctctgacacccgttctgaagttcagggtatgatcgactctgcggtttctaaccacatcgcgcgtctgtcttcttctcgtaactctctgtctatggactctgaagaactggaacgtctgatcaaatctttccagatccacaccccgcactgctctctgttcatcggtgcgcagtctctgtctcagcagctggaatctctgccggaagcgctgcagtctggtgttaactctgcggacatcctgctgggttctacccagtacatgctgaccaactctctggttgaagaatctatcgcgacctaccagcgtaccctgaaccgtatcaactacctgtctggtgttgcgggtcagatcaacggtgcgatcaaacgtaaagcgatcgacggtgaaaaaatccacctgccggcggcgtggtctgaactgatctctctgccgttcatcggtcagccggttatcgacgttgaatctgacctggcgcacctgaaaaaccagtaccagaccctgtctaacgaattcgacaccctgatctctgcgctgcagaaaaacttcgacctgaacttcaacaaagcgctgctgaaccgtacccagcacttcgaagcgatgtgccgttctaccaaaaaaaacgcgctgtctaaaccggaaatcgtttcttaccgtgacctgctggcgcgtctgacctcttgcctgtaccgtggttctctggttctgcgtcgtgcgggtatcgaagttctgaaaaaacacaaaatcttcgaatctaactctgaactgcgtgaacacgttcacgaacgtaaacacttcgttttcgtttctccgctggaccgtaaagcgaaaaaactgctgcgtctgaccgactctcgtccggacctgctgcacgttatcgacgaaatcctgcagcacgacaacctggaaaacaaagaccgtgaatctctgtggctggttcgttctggttacctgctggcgggtctgccggaccagctgtcttcttctttcatcaacctgccgatcatcacccagaaaggtgaccgtcgtctgatcgacctgatccagtacgaccagatcaaccgtgacgcgttcgttatgctggttacctctgcgttcaaatctaacctgtctggtctgcagtaccgtgcgaacaaacagtctttcgttgttacccgtaccctgtctccgtacctgggttctaaactggtttacgttccgaaagacaaagactggctggttccgtctcagatgttcgaaggtcgtttcgcggacatcctgcagtctgactacatggtttggaaagacgcgggtcgtctgtgcgttatcgacaccgcgaaacacctgtctaacatcaaaaaatctgttttctcttctgaagaagttctggcgttcctgcgtgaactgccgcaccgtaccttcatccagaccgaagttcgtggtctgggtgttaacgttgacggtatcgcgttcaacaacggtgacatcccgtctctgaaaaccttctctaactgcgttcaggttaaagtttctcgtaccaacacctctctggttcagaccctgaaccgttggttcgaaggtggtaaagtttctccgccgtctatccagttcgaacgtgcgtactacaaaaaagacgaccagatccacgaagacgcggcgaaacgtaaaatccgtttccagatgccggcgaccgaactggttcacgcgtctgacgacgcgggttggaccccgtcttacctgctgggtatcgacccgggtgaatacggtatgggtctgtctctggtttctatcaacaacggtgaagttctggactctggtttcatccacatcaactctctgatcaacttcgcgtctaaaaaatctaaccaccagaccaaagttgttccgcgtcagcagtacaaatctccgtacgcgaactacctggaacagtctaaagactctgcggcgggtgacatcgcgcacatcctggaccgtctgatctacaaactgaacgcgctgccggttttcgaagcgctgtctggtaactctcagtctgcggcggaccaggtttggaccaaagttctgtctttctacacctggggtgacaacgacgcgcagaactctatccgtaaacagcactggttcggtgcgtctcactgggacatcaaaggtatgctgcgtcagccgccgaccgaaaaaaaaccgaaaccgtacatcgcgttcccgggttctcaggtttcttcttacggtaactctcagcgttgctcttgctgcggtcgtaacccgatcgaacagctgcgtgaaatggcgaaagacacctctatcaaagaactgaaaatccgtaactctgaaatccagctgttcgacggtaccatcaaactgttcaacccggacccgtctaccgttatcgaacgtcgtcgtcacaacctgggtccgtctcgtatcccggttgcggaccgtaccttcaaaaacatctctccgtcttctctggaattcaaagaactgatcaccatcgtttctcgttctatccgtcactctccggaattcatcgcgaaaaaacgtggtatcggttctgaatacttctgcgcgtactctgactgcaactcttctctgaactctgaagcgaacgcggcggcgaacgttgcgcagaaattccagaaacagctgttcttcgaactgtaa

SEQ ID NO: 57 - DNA, 3864 bp, Artificial Sequence
  Description of Artificial Sequence: Synthetic polynucleotide
atgaaacgtatcctgaactctctgaaagttgcggcgctgcgtctgctgttccgtggtaaaggttctgaactggttaaaaccgttaaatacccgctggtttctccggttcagggtgcggttgaagaactggcggaagcgatccgtcacgacaacctgcacctgttcggtcagaaagaaatcgttgacctgatggaaaaagacgaaggtacccaggtttactctgttgttgacttctggctggacaccctgcgtctgggtatgttcttctctccgtctgcgaacgcgctgaaaatcaccctgggtaaattcaactctgaccaggtttctccgttccgtaaagttctggaacagtctccgttcttcctggcgggtcgtctgaaagttgaaccggcggaacgtatcctgtctgttgaaatccgtaaaatcggtaaacgtgaaaaccgtgttgaaaactacgcggcggacgttgaaacctgcttcatcggtcagctgtcttctgacgaaaaacagtctatccagaaactggcgaacgacatctgggactctaaagaccacgaagaacagcgtatgctgaaagcggacttcttcgcgatcccgctgatcaaagacccgaaagcggttaccgaagaagacccggaaaacgaaaccgcgggtaaacagaaaccgctggaactgtgcgtttgcctggttccggaactgtacacccgtggtttcggttctatcgcggacttcctggttcagcgtctgaccctgctgcgtgacaaaatgtctaccgacaccgcggaagactgcctggaatacgttggtatcgaagaagaaaaaggtaacggtatgaactctctgctgggtaccttcctgaaaaacctgcagggtgacggtttcgaacagatcttccagttcatgctgggttcttacgttggttggcagggtaaagaagacgttctgcgtgaacgtctggacctgctggcggaaaaagttaaacgtctgccgaaaccgaaattcgcgggtgaatggtctggtcaccgtatgttcctgcacggtcagctgaaatcttggtcttctaacttcttccgtctgttcaacgaaacccgtgaactgctggaatctatcaaatctgacatccagcacgcgaccatgctgatctcttacgttgaagaaaaaggtggttaccacccgcagctgctgtctcagtaccgtaaactgatggaacagctgccggcgctgcgtaccaaagttctggacccggaaatcgaaatgacccacatgtctgaagcggttcgttcttacatcatgatccacaaatctgttgcgggtttcctgccggacctgctggaatctctggaccgtgacaaagaccgtgaattcctgctgtctatcttcccgcgtatcccgaaaatcgacaaaaaaaccaaagaaatcgttgcgtgggaactgccgggtgaaccggaagaaggttacctgttcaccgcgaacaacctgttccgtaacttcctggaaaacccgaaacacgttccgcgtttcatggcggaacgtatcccggaagactggacccgtctgcgttctgcgccggtttggttcgacggtatggttaaacagtggcagaaagttgttaaccagctggttgaatctccgggtgcgctgtaccagttcaacgaatctttcctgcgtcagcgtctgcaggcgatgctgaccgtttacaaacgtgacctgcagaccgaaaaattcctgaaactgctggcggacgtttgccgtccgctggttgacttcttcggtctgggtggtaacgacatcatcttcaaatcttgccaggacccgcgtaaacagtggcagaccgttatcccgctgtctgttccggcggacgtttacaccgcgtgcgaaggtctggcgatccgtctgcgtgaaaccctgggtttcgaatggaaaaacctgaaaggtcacgaacgtgaagacttcctgcgtctgcaccagctgctgggtaacctgctgttctggatccgtgacgcgaaactggttgttaaactggaagactggatgaacaacccgtgcgttcaggaatacgttgaagcgcgtaaagcgatcgacctgccgctggaaatcttcggtttcgaagttccgatcttcctgaacggttacctgttctctgaactgcgtcagctggaactgctgctgcgtcgtaaatctgttatgacctcttactctgttaaaaccaccggttctccgaaccgtctgttccagctggtttacctgccgctgaacccgtctgacccggaaaaaaaaaactctaacaacttccaggaacgtctggacaccccgaccggtctgtctcgtcgtttcctggacctgaccctggacgcgttcgcgggtaaactgctgaccgacccggttacccaggaactgaaaaccatggcgggtttctacgaccacctgttcggtttcaaactgccgtgcaaactggcggcgatgtctaaccacccgggttcttcttctaaaatggttgttctggcgaaaccgaaaaaaggtgttgcgtctaacatcggtttcgaaccgatcccggacccggcgcacccggttttccgtgttcgttcttcttggccggaactgaaatacctggaaggtctgctgtacctgccggaagacaccccgctgaccatcgaactggcggaaacctctgtttcttgccagtctgtttcttctgttgcgttcgacctgaaaaacctgaccaccatcctgggtcgtgttggtgaattccgtgttaccgcggaccagccgttcaaactgaccccgatcatcccggaaaaagaagaatctttcatcggtaaaacctacctgggtctggacgcgggtgaacgttctggtgttggtttcgcgatcgttaccgttgacggtgacggttacgaagttcagcgtctgggtgttcacgaagacacccagctgatggcgctgcagcaggttgcgtctaaatctctgaaagaaccggttttccagccgctgcgtaaaggtaccttccgtcagcaggaacgtatccgtaaatctctgcgtggttgctactggaacttctaccacgcgctgatgatcaaataccgtgcgaaagttgttcacgaagaatctgttggttcttctggtctggttggtcagtggctgcgtgcgttccagaaagacctgaaaaaagcggacgttctgccgaaaaaaggtggtaaaaacggtgttgacaaaaaaaaacgtgaatcttctgcgcaggacaccctgtggggtggtgcgttctctaaaaaagaagaacagcagatcgcgttcgaagttcaggcggcgggttcttctcagttctgcctgaaatgcggttggtggttccagctgggtatgcgtgaagttaaccgtgttcaggaatctggtgttgttctggactggaaccgttctatcgttaccttcctgatcgaatcttctggtgaaaaagtttacggtttctctccgcagcagctggaaaaaggtttccgtccggacatcgaaaccttcaaaaaaatggttcgtgacttcatgcgtccgccgatgttcgaccgtaaaggtcgtccggcggcggcgtacgaacgtttcgttctgggtcgtcgtcaccgtcgttaccgtttcgacaaagttttcgaagaacgtttcggtcgttctgcgctgttcatctgcccgcgtgttggttgcggtaacttcgaccactcttctgaacagtctgcggttgttctggcgctgatcggttacatcgcggacaaagaaggtatgtctggtaaaaaactggtttacgttcgtctggcggaactgatggcggaatggaaactgaaaaaactggaacgttctcgtgttgaagaacagtcttctgcgcagtaa

SEQ ID NO: 58 - DNA, 3579 bp, Artificial Sequence
  Description of Artificial Sequence: Synthetic polynucleotide
atggcggaatctaaacagatgcagtgccgtaaatgcggtgcgtctatgaaatacgaagttatcggtctgggtaaaaaatcttgccgttacatgtgcccggactgcggtaaccacacctctgcgcgtaaaatccagaacaaaaaaaaacgtgacaaaaaatacggttctgcgtctaaagcgcagtctcagcgtatcgcggttgcgggtgcgctgtacccggacaaaaaagttcagaccatcaaaacctacaaatacccggcggacctgaacggtgaagttcacgactctggtgttgcggaaaaaatcgcgcaggcgatccaggaagacgaaatcggtctgctgggtccgtcttctgaatacgcgtgctggatcgcgtctcagaaacagtctgaaccgtactctgttgttgacttctggttcgacgcggtttgcgcgggtggtgttttcgcgtactctggtgcgcgtctgctgtctaccgttctgcagctgtctggtgaagaatctgttctgcgtgcggcgctggcgtcttctccgttcgttgacgacatcaacctggcgcaggcggaaaaattcctggcggtttctcgtcgtaccggtcaggacaaactgggtaaacgtatcggtgaatgcttcgcggaaggtcgtctggaagcgctgggtatcaaagaccgtatgcgtgaattcgttcaggcgatcgacgttgcgcagaccgcgggtcagcgtttcgcggcgaaactgaaaatcttcggtatctctcagatgccggaagcgaaacagtggaacaacgactctggtctgaccgtttgcatcctgccggactactacgttccggaagaaaaccgtgcggaccagctggttgttctgctgcgtcgtctgcgtgaaatcgcgtactgcatgggtatcgaagacgaagcgggtttcgaacacctgggtatcgacccgggtgcgctgtctaacttctctaacggtaacccgaaacgtggtttcctgggtcgtctgctgaacaacgacatcatcgcgctggcgaacaacatgtctgcgatgaccccgtactgggaaggtcgtaaaggtgaactgatcgaacgtctggcgtggctgaaacaccgtgcggaaggtctgtacctgaaagaaccgcacttcggtaactcttgggcggaccaccgttctcgtatcttctctcgtatcgcgggttggctgtctggttgcgcgggtaaactgaaaatcgcgaaagaccagatctctggtgttcgtaccgacctgttcctgctgaaacgtctgctggacgcggttccgcagtctgcgccgtctccggacttcatcgcgtctatctctgcgctggaccgtttcctggaagcggcggaatcttctcaggacccggcggaacaggttcgtgcgctgtacgcgttccacctgaacgcgccggcggttcgttctatcgcgaacaaagcggttcagcgttctgactctcaggaatggctgatcaaagaactggacgcggttgaccacctggaattcaacaaagcgttcccgttcttctctgacaccggtaaaaaaaaaaaaaaaggtgcgaactctaacggtgcgccgtctgaagaagaatacaccgaaaccgaatctatccagcagccggaagacgcggaacaggaagttaacggtcaggaaggtaacggtgcgtctaaaaaccagaaaaaattccagcgtatcccgcgtttcttcggtgaaggttctcgttctgaataccgtatcctgaccgaagcgccgcagtacttcgacatgttctgcaacaacatgcgtgcgatcttcatgcagctggaatctcagccgcgtaaagcgccgcgtgacttcaaatgcttcctgcagaaccgtctgcagaaactgtacaaacagaccttcctgaacgcgcgttctaacaaatgccgtgcgctgctggaatctgttctgatctcttggggtgaattctacacctacggtgcgaacgaaaaaaaattccgtctgcgtcacgaagcgtctgaacgttcttctgacccggactacgttgttcagcaggcgctggaaatcgcgcgtcgtctgttcctgttcggtttcgaatggcgtgactgctctgcgggtgaacgtgttgacctggttgaaatccacaaaaaagcgatctctttcctgctggcgatcacccaggcggaagtttctgttggttcttacaactggctgggtaactctaccgtttctcgttacctgtctgttgcgggtaccgacaccctgtacggtacccagctggaagaattcctgaacgcgaccgttctgtctcagatgcgtggtctggcgatccgtctgtcttctcaggaactgaaagacggtttcgacgttcagctggaatcttcttgccaggacaacctgcagcacctgctggtttaccgtgcgtctcgtgacctggcggcgtgcaaacgtgcgacctgcccggcggaactggacccgaaaatcctggttctgccggttggtgcgttcatcgcgtctgttatgaaaatgatcgaacgtggtgacgaaccgctggcgggtgcgtacctgcgtcaccgtccgcactctttcggttggcagatccgtgttcgtggtgttgcggaagttggtatggaccagggtaccgcgctggcgttccagaaaccgaccgaatctgaaccgttcaaaatcaaaccgttctctgcgcagtacggtccggttctgtggctgaactcttcttcttactctcagtctcagtacctggacggtttcctgtctcagccgaaaaactggtctatgcgtgttctgccgcaggcgggttctgttcgtgttgaacagcgtgttgcgctgatctggaacctgcaggcgggtaaaatgcgtctggaacgttctggtgcgcgtgcgttcttcatgccggttccgttctctttccgtccgtctggttctggtgacgaagcggttctggcgccgaaccgttacctgggtctgttcccgcactctggtggtatcgaatacgcggttgttgacgttctggactctgcgggtttcaaaatcctggaacgtggtaccatcgcggttaacggtttctctcagaaacgtggtgaacgtcaggaagaagcgcaccgtgaaaaacagcgtcgtggtatctctgacatcggtcgtaaaaaaccggttcaggcggaagttgacgcggcgaacgaactgcaccgtaaatacaccgacgttgcgacccgtctgggttgccgtatcgttgttcagtgggcgccgcagccgaaaccgggtaccgcgccgaccgcgcagaccgtttacgcgcgtgcggttcgtaccgaagcgccgcgttctggtaaccaggaagaccacgcgcgtatgaaatcttcttggggttacacctggggtacctactgggaaaaacgtaaaccggaagacatcctgggtatctctacccaggtttactggaccggtggtatcggtgaatcttgcccggcggttgcggttgcgctgctgggtcacatccgtgcgacctctacccagaccgaatgggaaaaagaagaagttgttttcggtcgtctgaaaaaattcttcccgtcttaa

SEQ ID NO: 59 - DNA, 2958 bp, Artificial Sequence
  Description of Artificial Sequence: Synthetic polynucleotide
atggaaaaacgtatcaacaaaatccgtaaaaaactgtctgcggacaacgcgaccaaaccggtttctcgttctggtccgatgaaaaccctgctggttcgtgttatgaccgacgacctgaaaaaacgtctggaaaaacgtcgtaaaaaaccggaagttatgccgcaggttatctctaacaacgcggcgaacaacctgcgtatgctgctggacgactacaccaaaatgaaagaagcgatcctgcaggtttactggcaggaattcaaagacgaccacgttggtctgatgtgcaaattcgcgcagccggcgtctaaaaaaatcgaccagaacaaactgaaaccggaaatggacgaaaaaggtaacctgaccaccgcgggtttcgcgtgctctcagtgcggtcagccgctgttcgtttacaaactggaacaggtttctgaaaaaggtaaagcgtacaccaactacttcggtcgttgcaacgttgcggaacacgaaaaactgatcctgctggcgcagctgaaaccggaaaaagactctgacgaagcggttacctactctctgggtaaattcggtcagcgtgcgctggacttctactctatccacgttaccaaagaatctacccacccggttaaaccgctggcgcagatcgcgggtaaccgttacgcgtctggtccggttggtaaagcgctgtctgacgcgtgcatgggtaccatcgcgtctttcctgtctaaataccaggacatcatcatcgaacaccagaaagttgttaaaggtaaccagaaacgtctggaatctctgcgtgaactggcgggtaaagaaaacctggaatacccgtctgttaccctgccgccgcagccgcacaccaaagaaggtgttgacgcgtacaacgaagttatcgcgcgtgttcgtatgtgggttaacctgaacctgtggcagaaactgaaactgtctcgtgacgacgcgaaaccgctgctgcgtctgaaaggtttcccgtctttcccggttgttgaacgtcgtgaaaacgaagttgactggtggaacaccatcaacgaagttaaaaaactgatcgacgcgaaacgtgacatgggtcgtgttttctggtctggtgttaccgcggaaaaacgtaacaccatcctggaaggttacaactacctgccgaacgaaaacgaccacaaaaaacgtgaaggttctctggaaaacccgaaaaaaccggcgaaacgtcagttcggtgacctgctgctgtacctggaaaaaaaatacgcgggtgactggggtaaagttttcgacgaagcgtgggaacgtatcgacaaaaaaatcgcgggtctgacctctcacatcgaacgtgaagaagcgcgtaacgcggaagacgcgcagtctaaagcggttctgaccgactggctgcgtgcgaaagcgtctttcgttctggaacgtctgaaagaaatggacgaaaaagaattctacgcgtgcgaaatccagctgcagaaatggtacggtgacctgcgtggtaacccgttcgcggttgaagcggaaaaccgtgttgttgacatctctggtttctctatcggttctgacggtcactctatccagtaccgtaacctgctggcgtggaaatacctggaaaacggtaaacgtgaattctacctgctgatgaactacggtaaaaaaggtcgtatccgtttcaccgacggtaccgacatcaaaaaatctggtaaatggcagggtctgctgtacggtggtggtaaagcgaaagttatcgacctgaccttcgacccggacgacgaacagctgatcatcctgccgctggcgttcggtacccgtcagggtcgtgaattcatctggaacgacctgctgtctctggaaaccggtctgatcaaactggcgaacggtcgtgttatcgaaaaaaccatctacaacaaaaaaatcggtcgtgacgaaccggcgctgttcgttgcgctgaccttcgaacgtcgtgaagttgttgacccgtctaacatcaaaccggttaacctgatcggtgttgaccgtggtgaaaacatcccggcggttatcgcgctgaccgacccggaaggttgcccgctgccggaattcaaagactcttctggtggtccgaccgacatcctgcgtatcggtgaaggttacaaagaaaaacagcgtgcgatccaggcggcgaaagaagttgaacagcgtcgtgcgggtggttactctcgtaaattcgcgtctaaatctcgtaacctggcggacgacatggttcgtaactctgcgcgtgacctgttctaccacgcggttacccacgacgcggttctggttttcgaaaacctgtctcgtggtttcggtcgtcagggtaaacgtaccttcatgaccgaacgtcagtacaccaaaatggaagactggctgaccgcgaaactggcgtacgaaggtctgacctctaaaacctacctgtctaaaaccctggcgcagtacacctctaaaacctgctctaactgcggtttcaccatcaccaccgcggactacgacggtatgctggttcgtctgaaaaaaacctctgacggttgggcgaccaccctgaacaacaaagaactgaaagcggaaggtcagatcacctactacaaccgttacaaacgtcagaccgttgaaaaagaactgtctgcggaactggaccgtctgtctgaagaatctggtaacaacgacatctctaaatggaccaaaggtcgtcgtgacgaagcgctgttcctgctgaaaaaacgtttctctcaccgtccggttcaggaacagttcgtttgcctggactgcggtcacgaagttcacgcggacgaacaggcggcgctgaacatcgcgcgttcttggctgttcctgaactctaactctaccgaattcaaatcttacaaatctggtaaacagccgttcgttggtgcgtggcaggcgttctacaaacgtcgtctgaaagaagtttggaaaccgaacgcg

SEQ ID NO: 60 - DNA, 2919 bp, Artificial Sequence
  Description of Artificial Sequence: Synthetic polynucleotide
atgaaacgtatcaacaaaatccgtcgtcgtctggttaaagactctaacaccaaaaaagcgggtaaaaccggtccgatgaaaaccctgctggttcgtgttatgaccccggacctgcgtgaacgtctggaaaacctgcgtaaaaaaccggaaaacatcccgcagccgatctctaacacctctcgtgcgaacctgaacaaactgctgaccgactacaccgaaatgaaaaaagcgatcctgcacgtttactgggaagaattccagaaagacccggttggtctgatgtctcgtgttgcgcagccggcgccgaaaaacatcgaccagcgtaaactgatcccggttaaagacggtaacgaacgtctgacctcttctggtttcgcgtgctctcagtgctgccagccgctgtacgtttacaaactggaacaggttaacgacaaaggtaaaccgcacaccaactacttcggtcgttgcaacgtttctgaacacgaacgtctgatcctgctgtctccgcacaaaccggaagcgaacgacgaactggttacctactctctgggtaaattcggtcagcgtgcgctggacttctactctatccacgttacccgtgaatctaaccacccggttaaaccgctggaacagatcggtggtaactcttgcgcgtctggtccggttggtaaagcgctgtctgacgcgtgcatgggtgcggttgcgtctttcctgaccaaataccaggacatcatcctggaacaccagaaagttatcaaaaaaaacgaaaaacgtctggcgaacctgaaagacatcgcgtctgcgaacggtctggcgttcccgaaaatcaccctgccgccgcagccgcacaccaaagaaggtatcgaagcgtacaacaacgttgttgcgcagatcgttatctgggttaacctgaacctgtggcagaaactgaaaatcggtcgtgacgaagcgaaaccgctgcagcgtctgaaaggtttcccgtctttcccgctggttgaacgtcaggcgaacgaagttgactggtgggacatggtttgcaacgttaaaaaactgatcaacgaaaaaaaagaagacggtaaagttttctggcagaacctggcgggttacaaacgtcaggaagcgctgctgccgtacctgtcttctgaagaagaccgtaaaaaaggtaaaaaattcgcgcgttaccagttcggtgacctgctgctgcacctggaaaaaaaacacggtgaagactggggtaaagtttacgacgaagcgtgggaacgtatcgacaaaaaagttgaaggtctgtctaaacacatcaaactggaagaagaacgtcgttctgaagacgcgcagtctaaagcggcgctgaccgactggctgcgtgcgaaagcgtctttcgttatcgaaggtctgaaagaagcggacaaagacgaattctgccgttgcgaactgaaactgcagaaatggtacggtgacctgcgtggtaaaccgttcgcgatcgaagcggaaaactctatcctggacatctctggtttctctaaacagtacaactgcgcgttcatctggcagaaagacggtgttaaaaaactgaacctgtacctgatcatcaactacttcaaaggtggtaaactgcgtttcaaaaaaatcaaaccggaagcgttcgaagcgaaccgtttctacaccgttatcaacaaaaaatctggtgaaatcgttccgatggaagttaacttcaacttcgacgacccgaacctgatcatcctgccgctggcgttcggtaaacgtcagggtcgtgaattcatctggaacgacctgctgtctctggaaaccggttctctgaaactggcgaacggtcgtgttatcgaaaaaaccctgtacaaccgtcgtacccgtcaggacgaaccggcgctgttcgttgcgctgaccttcgaacgtcgtgaagttctggactcttctaacatcaaaccgatgaacctgatcggtatcgaccgtggtgaaaacatcccggcggttatcgcgctgaccgacccggaaggttgcccgctgtctcgtttcaaagactctctgggtaacccgacccacatcctgcgtatcggtgaatcttacaaagaaaaacagcgtaccatccaggcggcgaaagaagttgaacagcgtcgtgcgggtggttactctcgtaaatacgcgtctaaagcgaaaaacctggcggacgacatggttcgtaacaccgcgcgtgacctgctgtactacgcggttacccaggacgcgatgctgatcttcgaaaacctgtctcgtggtttcggtcgtcagggtaaacgtaccttcatggcggaacgtcagtacacccgtatggaagactggctgaccgcgaaactggcgtacgaaggtctgccgtctaaaacctacctgtctaaaaccctggcgcagtacacctctaaaacctgctctaactgcggtttcaccatcacctctgcggactacgaccgtgttctggaaaaactgaaaaaaaccgcgaccggttggatgaccaccatcaacggtaaagaactgaaagttgaaggtcagatcacctactacaaccgttacaaacgtcagaacgttgttaaagacctgtctgttgaactggaccgtctgtctgaagaatctgttaacaacgacatctcttcttggaccaaaggtcgttctggtgaagcgctgtctctgctgaaaaaacgtttctctcaccgtccggttcaggaaaaattcgtttgcctgaactgcggtttcgaaacccacgcggacgaacaggcggcgctgaacatcgcgcgttcttggctgttcctgcgttctcaggaatacaaaaaataccagaccaacaaaaccaccggtaacaccgacaaacgtgcgttcgttgaaacctggcagtctttctaccgtaaaaaactgaaagaagtttggaaaccg

SEQ ID NO: 61 - DNA, 4859 bp, Artificial Sequence
  Description of Artificial Sequence: Synthetic polynucleotide
aaaattccatgcaaaatgctccggtttcatgtcatcaaaatgatgacgtaattaagcattgataattgagatccctctccctgacaggatgattacataaataatagtgacaaaaataaattatttatttatccagaaaatgaattggaaaatcaggagagcgttttcaatcctacctctggcgcagttgatatgtcaaacaggttgccgtcactgcgtcttttactggctcttctcgctaaccaaaccggtaaccccgcttattaaaagcattctgtaacaaagcgggaccaaagccatgacaaaaacgcgtaacaaaagtgtctataatcacggcagaaaagtccacattgattatttgcacggcgtcacactttgctatgccatagcatttttatccataagattagcggatcctacctgacgctttttatcgcaactctctactgtttctccatacccgtttttttgggctagcaccgcctatctcgtgtgagataggcggagatacgaactttaagaaggagatataccatgggtaaaatgtattaccttggtttagacattggcacgaattccgtgggctacgcggtgaccgacccctcataccacctgctgaagtttaagggggaaccaatgtggggtgcgcacgtatttgccgccggtaatcagagcgcggaacgacgctcgttccgcacatcgcgtcgtcgtttggaccgacgccaacagcgcgttaaactggtacaggagatttttgccccggtgattagtccgatcgacccacgcttcttcattcgtctgcatgaatccgccctgtggcgcgatgacgtcgcggagacggataaacatatctttttcaatgatcctacctataccgataaggaatattatagcgattacccgactatccatcacctgatcgttgatctgatggaaagctctgagaaacacgatccgcggctggtgtaccttgcagtggcgtggttagtggcacaccgtggtcattttctgaacgaggtggacaaggataatattggagatgtgttgtcgttcgacgcattttatccggagtttctcgcgttcctgtcggacaacggtgtatcaccgtgggtgtgcgaaagcaaagcgctgcaggcgaccttgctgagccgtaactcagtgaacgacaaatataaagcccttaagtctctgatcttcggatcccagaaacctgaagataacttcgatgccaatatttcggaagatggactcattcaactgctggccggcaaaaaggtaaaagttaacaaactgttccctcaggaatcgaacgatgcatccttcacattgaatgataaagaagacgcgatagaagaaatcctgggtacgcttacaccagatgaatgtgaatggattgcgcatatacgccgcctttttgactgggctatcatgaaacatgctctgaaagatggcaggactattagcgagtcaaaagtcaaactgtatgagcagcaccatcacgatctgacccaacttaaatacttcgtgaaaacctaccttgcaaaagaatacgacgatattttccgcaacgtggatagcgaaacaacgaaaaactatgtagcgtattcctatcatgtgaaagaggtgaaaggcactctgcctaaaaataaggcaacgcaagaagagttttgtaagtatgtcctgggcaaggttaaaaacattgaatgctctgaagcagacaaggttgactttgatgagatgattcagcgtcttaccgacaactcttttatgcctaagcaggtttcgggcgaaaaccgcgttattccttatcagttatattattatgaactgaagacaattctgaataaagcagcctcgtacctgcctttcctgacgcagtgtggaaaagatgcaatttcgaaccaggacaaactactgtcgatcatgacgttccgtattccttacttcgtcggacccttgcgaaaagataattcggaacatgcatggctcgaacgaaaggccggtaagatttatccgtggaactttaacgacaaagtggacttggataaatcagaagaagcgttcattcgccgaatgaccaatacctgtacctattatcccggcgaagatgttttaccgttggattcgctgatctatgagaaatttatgattttaaatgaaatcaataatattcgtattgacggctacccgattagtgttgacgttaaacagcaggtttttggcttgttcgaaaaaaaacgacgcgtaaccgtgaaagatattcagaacctgctgctgtctctcggagctctggacaaacacgggaagctgacaggcatcgataccactatccactcaaactataatacgtatcaccattttaaatctctcatggaacgcggcgtcctgacccgggatgacgtggaacgcatcgttgaaaggatgacctacagcgacgatactaagcgtgtgcgtctgtggctgaataacaactatggtactttaaccgccgacgatgtgaaacacatttcgcgtctgcgcaaacacgattttggccgtttatccaaaatgttcttaacaggtctgaagggtgtccataaggagaccggtgaacgtgcctccatactggatttcatgtggaacacgaacgataacctgatgcagctcctttccgaatgctacacgttcagtgatgaaatcacaaagctgcaagaggcgtattatgcaaaagcccagttgtctttaaacgattttttagactcgatgtacatctctaacgcggtgaaacgtccgatttacagaactctggcagtggtgaacgatattcgaaaagcatgtgggacggcccctaaacgcattttcatcgaaatggctcgtgatggtgaatcaaaaaaaaagagaagtgttacacgtcgcgagcagatcaaaaacctgtaccgctcgattcgtaaagatttccagcaggaagttgattttctggaaaagatcctggaaaataaatctgatggtcaacttcagtcagatgctttgtatctttactttgcacaattagggcgcgatatgtacacgggcgatccaataaagctggagcacatcaaagatcagagtttctataacatagaccatatttacccgcagtctatggtgaaagacgattccctagataacaaagtgctggtgcaaagcgaaattaacggcgagaaaagctcgcgataccctttggacgccgcgatccgcaataaaatgaagcccctttgggacgcttactataatcatggcctgatctccttaaagaaataccagcgtctaacgcgctcgaccccgtttaccgatgatgaaaaatgggactttattaatcgccagttagtggaaacccgtcaatctaccaaagcgctggccattttgttgaagcgtaagtttccagacaccgaaattgtgtattcgaaggcggggttatcgtccgacttcagacatgaattcggccttgtaaaaagtcgcaatattaatgatttgcaccacgctaaagacgcattcttggctatcgttaccggcaatgtgtaccatgaaagattcaatcgcagatggtttatggtgaaccagccgtactcagttaaaactaaaactctttttacccacagcataaagaatggcaacttcgttgcctggaacggcgaagaagatctcggtcgtattgtaaaaatgctgaagcaaaacaaaaataccattcacttcacgcgcttctccttcgatcgcaaagaaggattatttgatatccaacctctgaaagccagcaccggcttagtcccacgaaaagccggtctggatgtcgttaaatacggcggatatgacaaatctaccgcggcctattacctgctggtgaggttcacgctcgaggacaagaaaacccagcacaagctgatgatgattcctgtagaaggcctgtacaaggctcgcattgatcatgacaaggaatttcttaccgattatgcgcaaacgactataagcgaaatcctacagaaagataaacagaaagtgatcaatattatgtttccaatgggtacgaggcatataaaactcaattcaatgattagtatcgatggcttctatcttagtatcggcggaaagtcctctaaaggtaagtcagttctatgtcacgcaatggttccactgatcgtccctcacaaaatcgaatgttacattaaagcaatggaaagcttcgcccggaagtttaaagaaaacaacaagctgcgcatcgtagaaaaattcgataaaatcaccgttgaagacaacctgaatctctacgagctctttctccaaaaactgcagcataatccctataataagtttttttcgacacagtttgacgtactgacgaacggccgttctactttcacaaaactgtcgccggaggaacaggtacagacgctcttgaacattttaagtatctttaaaacatgccgcagttcgggttgcgacctgaaatccatcaacggcagtgcccaggcagcgcgcatcatgattagcgctgacttaactggactgtcgaaaaaatattcagatattaggttggttgaacagtcagcttctggtttgttcgtatccaaaagtcagaacttactggagtatctctaagaaatcatccttagcgaaagctaaggattttttttatctgaaatttattatatcgcgttgattattgatgctgtttttagttttaacggcaattaatatatgtgttattaattgaatgaattttatcattcataataagtatgtgtaggatcaagctcaggttaaatattcactcaggaagttattactcaggaagcaaagaggattacagaattatctcataacaagtgttaagggatgttatttcc

SEQ ID NO: 62 - DNA, 4787 bp, Artificial Sequence
  Description of Artificial Sequence: Synthetic polynucleotide
aaaattccatgcaaaatgctccggtttcatgtcatcaaaatgatgacgtaattaagcattgataattgagatccctctccctgacaggatgattacataaataatagtgacaaaaataaattatttatttatccagaaaatgaattggaaaatcaggagagcgttttcaatcctacctctggcgcagttgatatgtcaaacaggttgccgtcactgcgtcttttactggctcttctcgctaaccaaaccggtaaccccgcttattaaaagcattctgtaacaaagcgggaccaaagccatgacaaaaacgcgtaacaaaagtgtctataatcacggcagaaaagtccacattgattatttgcacggcgtcacactttgctatgccatagcatttttatccataagattagcggatcctacctgacgctttttatcgcaactctctactgtttctccatacccgtttttttgggctagcaccgcctatctcgtgtgagataggcggagatacgaactttaagaaggagatataccatgtcatcgctcacgaaattcactaacaaatactctaaacagctcaccattaagaatgaactcatcccagttggcaaaacactggagaacatcaaagagaatggtctgatagatggcgacgaacagctgaatgagaattatcagaaggcgaaaattattgtggatgattttctgcgggacttcattaataaagcactgaataatacgcagatcgggaactggcgcgaactggcggatgcccttaataaagaggatgaagataacatcgagaaattgcaggataaaattcggggaatcattgtatccaaatttgaaacgtttgatctgtttagcagctattctattaagaaagatgaaaagattattgacgacgacaatgatgttgaagaagaggaactggatctgggcaagaagaccagctcatttaaatacatatttaaaaaaaacctgtttaagttagtgttgccatcctacctgaaaaccacaaaccaggacaagctgaagattattagctcgtttgataatttttcaacgtacttccgcgggttctttgaaaaccggaaaaacatttttaccaagaaaccgatctccacaagtattgcgtatcgcattgttcatgataacttcccgaaattccttgataacattcgttgttttaatgtgtggcagacggaatgcccgcaactaatcgtgaaagcagataactatctgaaaagcaaaaatgttatagcgaaagataaaagtttggcaaactattttaccgtgggcgcgtatgactatttcctgtctcagaatggtatagatttttacaacaatattataggtggactgccagcgttcgccggccatgagaaaatccaaggtctcaatgaattcatcaatcaagagtgccaaaaagacagcgagctgaaaagtaagctgaaaaaccgtcacgcgttcaaaatggcggtactgttcaaacagatactcagcgatcgtgaaaaaagttttgtaattgatgagttcgagtcggatgctcaagttattgacgccgttaaaaacttttacgccgaacagtgcaaagataacaatgttatttttaacttattaaatcttatcaagaatatcgctttcttaagtgatgacgaactggacggcatattcattgaagggaaatacctgtcgagcgttagtcaaaaactctatagcgattggtcaaaattacgtaacgacattgaggattcggctaactctaaacaaggcaataaagagctggccaagaagatcaaaaccaacaaaggggatgtagaaaaagcgatctcgaaatatgagttctcgctgtcggaactgaactcgattgtacatgataacaccaagttttctgacctccttagttgtacactgcataaggtggcttctgagaaactggtgaaggtcaatgaaggcgactggccgaaacatctcaagaataatgaagagaaacaaaaaatcaaagagccgcttgatgctctgctggagatctataatacacttctgatttttaactgcaaaagcttcaataaaaacggcaacttctatgtcgactatgatcgttgcatcaatgaactgagttcggtcgtgtatctgtataataaaacacgtaactattgcactaaaaaaccctataacacggacaagttcaaactcaattttaacagtccgcagctcggtgaaggcttttccaagtcgaaagaaaatgactgtctgactcttttgtttaaaaaagacgacaactattatgtaggcattatccgcaaaggtgcaaaaatcaattttgatgatacacaagcaatcgccgataacaccgacaattgcatctttaaaatgaattatttcctacttaaagacgcaaaaaaatttatcccgaaatgtagcattcagctgaaagaagtcaaggcccattttaagaaatctgaagatgattacattttgtctgataaagagaaatttgctagcccgctggtcattaaaaagagcacatttttgctggcaactgcacatgtgaaagggaaaaaaggcaatatcaagaaatttcagaaagaatattcgaaagaaaaccccactgagtatcgcaattctttaaacgaatggattgctttttgtaaagagttcttaaaaacttataaagcggctaccatttttgatataaccacattgaaaaaggcagaggaatatgctgatattgtagaattctacaaggatgtcgataatctgtgctacaaactggagttctgcccgattaaaacctcgtttatagaaaacctgatagataacggcgacctgtatctgtttcgcatcaataacaaagacttcagcagtaaatcgaccggcaccaagaaccttcatacgttatatttacaagctatattcgatgaacgtaatctgaacaatccgacaattatgctgaatgggggagcagaactgttctatcgtaaagaaagtattgagcagaaaaaccgtatcacacacaaagccggttcaattctcgtgaataaggtgtgtaaagacggtacaagcctggatgataagatacgtaatgaaatttatcaatatgagaataaatttattgataccctgtctgatgaagctaaaaaggtgttaccgaatgtcattaaaaaggaagctacccatgacattacaaaagataaacgtttcactagtgacaaattcttctttcactgccccctgacaattaattataaggaaggcgataccaagcagttcaataacgaagtgctgagttttctgcgtggaaatcctgacatcaacattatcggcattgaccgcggagagcgtaatttaatctatgtaacggttataaaccagaaaggcgagattctggattcggtttcattcaataccgtgaccaacaagagttcaaaaatcgagcagacagtcgattatgaagagaaattggcagtccgcgagaaagagaggattgaagcaaaacgttcctgggactctatctcaaaaattgcgacactaaaggaaggttatctgagcgcaatagttcacgagatctgtctgttaatgattaaacacaacgcgatcgttgtcttagagaatcttaatgcaggctttaagcgtattcgtggcggtttatcagaaaaaagtgtttatcaaaaattcgaaaaaatgttgattaacaaactgaactattttgtcagcaagaaggaatccgactggaataaaccgtctggtctgctgaatggactgcagctttcggatcagtttgaaagcttcgaaaaactgggtattcagtctggttttattttttacgtgccggctgcatatacctcaaagattgatccgaccacgggcttcgccaatgttctgaatctgtcgaaggtacgcaatgttgatgcgatcaaaagctttttttctaacttcaacgaaattagttatagcaagaaagaagcccttttcaaattctcattcgatctggattcactgagtaagaaaggctttagtagctttgtgaaatttagtaagagtaaatggaacgtctacacctttggagaacgtatcataaagccaaagaataagcaaggttatcgggaggacaaaagaatcaacttgaccttcgagatgaagaagttacttaacgagtataaggtttcttttgatcttgaaaataacttgattccgaatctcacgagtgccaacctgaaggatactttttggaaagagctattctttatcttcaagactacgctgcagctccgtaacagcgttactaacggtaaagaagatgtgctcatctctccggtcaaaaatgcgaagggtgaattcttcgtttcgggaacgcataacaagactcttccgcaagattgcgatgcgaacggtgcataccatattgcgttgaaaggtctgatgatactcgaacgtaacaaccttgtacgtgaggagaaagatacgaaaaagattatggcgatttcaaacgtggattggttcgagtacgtgcagaaacgtagaggcgttctgtaagaaatcatccttagcgaaagctaaggattttttttatctgaaatttattatatcgcgttgattattgatgctgtttttagttttaacggcaattaatatatgtgttattaattgaatgaattttatcattcataataagtatgtgtaggatcaagctcaggttaaatattcactcaggaagttattactcaggaagcaaagaggattacagaattatctcataacaagtgttaagggatgttatttcc

SEQ ID NO: 63 - DNA, 4249 bp, Artificial Sequence
  Description of Artificial Sequence: Synthetic polynucleotide
aatcaggagagcgttttcaatcctacctctggcgcagttgatatgtcaaacaggttgccgtcactgcgtcttttactggctcttctcgctaaccaaaccggtaaccccgcttattaaaagcattctgtaacaaagcgggaccaaagccatgacaaaaacgcgtaacaaaagtgtctataatcacggcagaaaagtccacattgattatttgcacggcgtcacactttgctatgccatagcatttttatccataagattagcggatcctacctgacgctttttatcgcaactctctactgtttctccatacccgtttttttgggctagcagtaatacgactcactataggggtctcatctcgtgtgagataggcggagatacgaactttaagaggaggatataccatgcaccatcatcatcaccataacaactacgacgaattcaccaaactgtacccgatccagaaaaccatccgtttcgaactgaaaccgcagggtcgtaccatggaacacctggaaaccttcaacttcttcgaagaagaccgtgaccgtgcggaaaaatacaaaatcctgaaagaagcgatcgacgaataccacaaaaaattcatcgacgaacacctgaccaacatgtctctggactggaactctctgaaacagatctctgaaaaatactacaaatctcgtgaagaaaaagacaaaaaagttttcctgtctgaacagaaacgtatgcgtcaggaaatcgtttctgaattcaaaaaagacgaccgtttcaaagacctgttctctaaaaaactgttctctgaactgctgaaagaagaaatctacaaaaaaggtaaccaccaggaaatcgacgcgctgaaatctttcgacaaattctctggttacttcatcggtctgcacgaaaaccgtaaaaacatgtactctgacggtgacgaaatcaccgcgatctctaaccgtatcgttaacgaaaacttcccgaaattcctggacaacctgcagaaataccaggaagcgcgtaaaaaatacccggaatggatcatcaaagcggaatctgcgctggttgcgcacaacatcaaaatggacgaagttttctctctggaatacttcaacaaagttctgaaccaggaaggtatccagcgttacaacctggcgctgggtggttacgttaccaaatctggtgaaaaaatgatgggtctgaacgacgcgctgaacctggcgcaccagtctgaaaaatcttctaaaggtcgtatccacatgaccccgctgttcaaacagatcctgtctgaaaaagaatctttctcttacatcccggacgttttcaccgaagactctcagctgctgccgtctatcggtggtttcttcgcgcagatcgaaaacgacaaagacggtaacatcttcgaccgtgcgctggaactgatctcttcttacgcggaatacgacaccgaacgtatctacatccgtcaggcggacatcaaccgtgtttctaacgttatcttcggtgaatggggtaccctgggtggtctgatgcgtgaatacaaagcggactctatcaacgacatcaacctggaacgtacctgcaaaaaagttgacaaatggctggactctaaagaattcgcgctgtctgacgttctggaagcgatcaaacgtaccggtaacaacgacgcgttcaacgaatacatctctaaaatgcgtaccgcgcgtgaaaaaatcgacgcggcgcgtaaagaaatgaaattcatctctgaaaaaatctctggtgacgaagaatctatccacatcatcaaaaccctgctggactctgttcagcagttcctgcacttcttcaacctgttcaaagcgcgtcaggacatcccgctggacggtgcgttctacgcggaattcgacgaagttcactctaaactgttcgcgatcgttccgctgtacaacaaagttcgtaactacctgaccaaaaacaacctgaacaccaaaaaaatcaaactgaacttcaaaaacccgaccctggcgaacggttgggaccagaacaaagtttacgactacgcgtctctgatcttcctgcgtgacggtaactactacctgggtatcatcaacccgaaacgtaaaaaaaacatcaaattcgaacagggttctggtaacggtccgttctaccgtaaaatggtttacaaacagatcccgggtccgaacaaaaacctgccgcgtgttttcctgacctctaccaaaggtaaaaaagaatacaaaccgtctaaagaaatcatcgaaggttacgaagcggacaaacacatccgtggtgacaaattcgacctggacttctgccacaaactgatcgacttcttcaaagaatctatcgaaaaacacaaagactggtctaaattcaacttctacttctctccgaccgaatcttacggtgacatctctgaattctacctggacgttgaaaaacagggttaccgtatgcacttcgaaaacatctctgcggaaaccatcgacgaatacgttgaaaaaggtgacctgttcctgttccagatctacaacaaagacttcgttaaagcggcgaccggtaaaaaagacatgcacaccatctactggaacgcggcgttctctccggaaaacctgcaggacgttgttgttaaactgaacggtgaagcggaactgttctaccgtgacaaatctgacatcaaagaaatcgttcaccgtgaaggtgaaatcctggttaaccgtacctacaacggtcgtaccccggttccggacaaaatccacaaaaaactgaccgactaccacaacggtcgtaccaaagacctgggtgaagcgaaagaatacctggacaaagttcgttacttcaaagcgcactacgacatcaccaaagaccgtcgttacctgaacgacaaaatctacttccacgttccgctgaccctgaacttcaaagcgaacggtaaaaaaaacctgaacaaaatggttatcgaaaaattcctgtctgacgaaaaagcgcacatcatcggtatcgaccgtggtgaacgtaacctgctgtactactctatcatcgaccgttctggtaaaatcatcgaccagcagtctctgaacgttatcgacggtttcgactaccgtgaaaaactgaaccagcgtgaaatcgaaatgaaagacgcgcgtcagtcttggaacgcgatcggtaaaatcaaagacctgaaagaaggttacctgtctaaagcggttcacgaaatcaccaaaatggcgatccagtacaacgcgatcgttgttatggaagaactgaactacggtttcaaacgtggtcgtttcaaagttgaaaaacagatctaccagaaattcgaaaacatgctgatcgacaaaatgaactacctggttttcaaagacgcgccggacgaatctccgggtggtgttctgaacgcgtaccagctgaccaacccgctggaatctttcgcgaaactgggtaaacagaccggtatcctgttctacgttccggcggcgtacacctctaaaatcgacccgaccaccggtttcgttaacctgttcaacacctcttctaaaaccaacgcgcaggaacgtaaagaattcctgcagaaattcgaatctatctcttactctgcgaaagacggtggtatcttcgcgttcgcgttcgactaccgtaaattcggtacctctaaaaccgaccacaaaaacgtttggaccgcgtacaccaacggtgaacgtatgcgttacatcaaagaaaaaaaacgtaacgaactgttcgacccgtctaaagaaatcaaagaagcgctgacctcttctggtatcaaatacgacggtggtcagaacatcctgccggacatcctgcgttctaacaacaacggtctgatctacaccatgtactcttctttcatcgcggcgatccagatgcgtgtttacgacggtaaagaagactacatcatctctccgatcaaaaactctaaaggtgaattcttccgtaccgacccgaaacgtcgtgaactgccgatcgacgcggacgcgaacggtgcgtacaacatcgcgctgcgtggtgaactgaccatgcgtgcgatcgcggaaaaattcgacccggactctgaaaaaatggcgaaactggaactgaaacacaaagactggttcgaattcatgcagacccgtggtgactaagaaatcatccttagcgaaagctaaggattttttttatctgaaatgtagggagaccctcaggttaaatattcactcaggaagttattactcaggaagcaaagaggattaca

SEQ ID NO: 64 - DNA, 4679 bp, Artificial Sequence
  Description of Artificial Sequence: Synthetic polynucleotide
aaaattccatgcaaaatgctccggtttcatgtcatcaaaatgatgacgtaattaagcattgataattgagatccctctccctgacaggatgattacataaataatagtgacaaaaataaattatttatttatccagaaaatgaattggaaaatcaggagagcgttttcaatcctacctctggcgcagttgatatgtcaaacaggttgccgtcactgcgtcttttactggctcttctcgctaaccaaaccggtaaccccgcttattaaaagcattctgtaacaaagcgggaccaaagccatgacaaaaacgcgtaacaaaagtgtctataatcacggcagaaaagtccacattgattatttgcacggcgtcacactttgctatgccatagcatttttatccataagattagcggatcctacctgacgctttttatcgcaactctctactgtttctccatacccgtttttttgggctagcaccgcctatctcgtgtgagataggcggagatacgaactttaagaaggagatataccatgactaaaacatttgattcagagttttttaatttgtactcgctgcaaaaaacggtacgctttgagttaaaacccgtgggagaaaccgcgtcatttgtggaagactttaaaaacgagggcttgaaacgtgttgtgagcgaagatgaaaggcgagccgtcgattaccagaaagttaaggaaataattgacgattaccatcgggatttcattgaagaaagtttaaattattttccggaacaggtgagtaaagatgctcttgagcaggcgtttcatctttatcagaaactgaaggcagcaaaagttgaggaaagggaaaaagcgctgaaagaatgggaagcgctgcagaaaaagctacgtgaaaaagtggtgaaatgcttctcggactcgaataaagcccgcttctcaaggattgataaaaaggaactgattaaggaagacctgataaattggttggtcgcccagaatcgcgaggatgatatccctacggtcgaaacgtttaacaacttcaccacatattttaccggcttccatgagaatcgtaaaaatatttactccaaagatgatcacgccaccgctattagctttcgccttattcatgaaaatcttccaaagttttttgacaacgtgattagcttcaataagttgaaagagggtttccctgaattaaaatttgataaagtgaaagaggatttagaagtagattatgatctgaagcatgcgtttgaaatagaatatttcgttaacttcgtgacccaagcgggcatagatcagtataattatctgttaggagggaaaaccctggaggacgggacgaaaaaacaagggatgaatgagcaaattaatctgttcaaacaacagcaaacgcgagataaagcgcgtcagattcccaaactgatccccctgttcaaacagattcttagcgaaaggactgaaagccagtcctttattcctaaacaatttgaaagtgatcaggagttgttcgattcactgcagaagttacataataactgccaggataaattcaccgtgctgcaacaagccattctcggtctggcagaggcggatcttaagaaggtcttcatcaaaacctctgatttaaatgccttatctaacaccattttcgggaattacagcgtcttttccgatgcactgaacctgtataaagaaagcctgaaaacgaaaaaagcgcaggaggcttttgagaaactaccggcccattctattcacgacctcattcaatacttggaacagttcaattccagcctggacgcggaaaaacaacagagcaccgacaccgtcctgaactacttcatcaagaccgatgaattatattctcgcttcattaaatccactagcgaggctttcactcaggtgcagcctttgttcgaactggaagccctgtcatctaagcgccgcccaccggaatcggaagatgaaggggcaaaagggcaggaaggcttcgagcagatcaagcgtattaaagcttacctggatacgcttatggaagcggtacactttgcaaagccgttgtatcttgttaagggtcgtaaaatgatcgaagggctcgataaagaccagtccttttatgaagcgtttgaaatggcgtaccaagaacttgaatcgttaatcattcctatctataacaaagcgcggagctatctgtcgcggaaacctttcaaggccgataaattcaagattaattttgacaacaacacgctactgagcggatgggatgcgaacaaggaaactgctaacgcgtccattctgtttaagaaagacgggttatattaccttggaattatgccgaaaggtaagacctttctctttgactactttgtatcgagcgaggattcagagaaactgaaacagcgtcgccagaagaccgccgaagaagctctggcgcaggatggtgaaagttacttcgaaaaaattcgttataaactgttaccaggggcttcaaagatgttaccgaaagtcttttttagcaacaaaaatattggcttttacaacccgtcggatgacattttacgcattcgcaacacagcctctcacaccaaaaacgggacccctcagaaaggccactcaaaagttgagtttaacctgaatgattgtcataagatgattgatttcttcaaatcatcaattcagaaacacccggaatgggggtcttttggctttacgttttctgataccagtgattttgaagacatgagtgccttctaccgggaagtagaaaaccagggttacgtaattagctttgacaaaatcaaagagacctatatacagagccaggtggaacagggtaatctctacttattccagatttataacaaggatttctcgccctacagcaaaggcaaaccaaacctgcatactctgtactggaaagccctgtttgaagaagcgaacctgaataacgtagtggcgaagttgaacggtgaagcggaaatcttcttccgtcgtcactccattaaggcctctgataaagttgtccatccggcaaatcaggccattgataataagaatccacacacggaaaaaacgcagtcaacctttgaatatgacctcgttaaagacaaacgctacacgcaagataagttctttttccacgtcccaatcagcctcaactttaaagcacaaggggtttcaaagtttaatgataaagtcaatgggttcctcaagggcaacccggatgtcaacattataggtatagacaggggcgaacgccatctgctttactttaccgtagtgaatcagaaaggtgaaatactggttcaggaatcattaaataccttgatgtcggacaaagggcacgttaatgattaccagcagaaactggataaaaaagaacaggaacgtgatgctgcgcgtaaatcgtggaccacggttgagaacattaaagagctgaaagaggggtatctaagccatgtggtacacaaactggcgcacctcatcattaaatataacgcaatagtctgcctagaagacttgaattttggctttaaacgcggccgcttcaaagtggaaaaacaagtttatcaaaaatttgaaaaggcgcttatagataaactgaattatctggtttttaaagaaaaggaacttggtgaggtagggcactacttgacagcttatcaactgacggccccgttcgaatcattcaaaaaactgggcaaacagtctggcattctgttttacgtgccggcagattatacttcaaaaatcgatccaacaactggctttgtgaacttcctggacctgagatatcagtctgtagaaaaagctaaacaacttcttagcgattttaatgccattcgttttaacagcgttcagaattactttgaattcgaaattgactataaaaaacttactccgaaacgtaaagtcggaacccaaagtaaatgggtaatttgtacgtatggcgatgtcaggtatcagaaccgtcggaatcaaaaaggtcattgggagaccgaagaagtgaacgtgaccgaaaagctgaaggctctgttcgccagcgattcaaaaactacaactgtgatcgattacgcaaatgatgataacctgatagatgtgattttagagcaggataaagccagcttttttaaagaactgttgtggctcctgaaacttacgatgaccttacgacattccaagatcaaatcggaagatgattttattctgtcaccggtcaagaatgagcagggtgaattctatgatagtaggaaagccggcgaagtgtggccgaaagacgccgacgccaatggcgcctatcatatcgcgctcaaagggctttggaatttgcagcagattaaccagtgggaaaaaggtaaaaccctgaatctggctatcaaaaaccaggattggtttagctttatccaagagaaaccgtatcaggaatgagaaatcatccttagcgaaagctaaggattttttttatctgaaatttattatatcgcgttgattattgatgctgtttttagttttaacggcaattaatatatgtgttattaattgaatgaattttatcattcataataagtatgtgtaggatcaagctcaggttaaatattcactcaggaagttattactcaggaagcaaagaggattacagaattatctcataacaagtgttaagggatgttatttcc

SEQ ID NO: 65 - DNA, 4240 bp, Artificial Sequence
  Description of Artificial Sequence: Synthetic polynucleotide
aatcaggagagcgttttcaatcctacctctggcgcagttgatatgtcaaacaggttgccgtcactgcgtcttttactggctcttctcgctaaccaaaccggtaaccccgcttattaaaagcattctgtaacaaagcgggaccaaagccatgacaaaaacgcgtaacaaaagtgtctataatcacggcagaaaagtccacattgattatttgcacggcgtcacactttgctatgccatagcatttttatccataagattagcggatcctacctgacgctttttatcgcaactctctactgtttctccatacccgtttttttgggctagcagtaatacgactcactataggggtctcatctcgtgtgagataggcggagatacgaactttaagaggaggatataccatgcaccatcatcatcaccatcatacaggcggtcttcttagtatggacgcgaaagagttcacaggtcagtatccgttgtcgaaaacattacgattcgaacttcggcccatcggccgcacgtgggataacctggaggcctcaggctacttagcggaagaccgccatcgtgccgaatgttatcctcgtgcgaaagagttattggatgacaaccatcgtgccttcctgaatcgtgtgttgccacaaatcgatatggattggcacccgattgcggaggccttttgtaaggtacataaaaaccctggtaataaagaacttgcccaggattacaaccttcagttgtcaaagcgccgtaaggagatcagcgcatatcttcaggatgcagatggctataaaggcctgttcgcgaagcccgccttagacgaagctatgaaaattgcgaaagaaaacgggaacgaaagtgatattgaggttctcgaagcgtttaacggttttagcgtatacttcaccggttatcatgagtcacgcgagaacatttatagcgatgaggatatggtgagcgtagcctaccgaattactgaggataatttcccgcgctttgtctcaaacgctttgatctttgataaattaaacgaaagccatccggatattatctctgaagtatcgggcaatcttggagttgatgacattggtaagtactttgacgtgtcgaactataacaattttctttcccaggccggtatagatgactacaatcacattattggcggccatacaaccgaagacggactgatacaagcgtttaatgtcgtattgaacttacgtcaccaaaaagaccctggctttgaaaaaattcagttcaaacagctctacaaacaaatcctgagcgtgcgtaccagcaaaagctacatcccgaaacagtttgacaactctaaggagatggttgactgcatttgcgattatgtcagcaaaatagagaaatccgaaacagtagaacgggccctgaaactagtccgtaatatcagttctttcgacttgcgcgggatctttgtcaataaaaagaacttgcgcatactgagcaacaaactgataggagattgggacgcgatcgaaaccgcattgatgcatagttcttcatcagaaaacgataagaaaagcgtatatgatagcgcggaggcttttacgttggatgacatcttttcaagcgtgaaaaaattttctgatgcctctgccgaagatattggcaacagggcggaagacatctgtagagtgataagtgagacggccccttttatcaacgatctgcgagcggtggacctggatagcctgaacgacgatggttatgaagcggccgtctcaaaaattcgggagtcgctggagccttatatggatcttttccatgaactggaaattttctcggttggcgatgagttcccaaaatgcgcagcattttacagcgaactggaggaagtcagcgaacagctgatcgaaattattccgttattcaacaaggcgcgttcgttctgcacccggaaacgctatagcaccgataagattaaagtgaacttaaaattcccgaccttggcggacgggtgggacctgaacaaagagagagacaacaaagccgcgattctgcggaaagacggtaagtattatctggcaattctggatatgaagaaagatctgtcaagcattaggaccagcgacgaagatgaatccagcttcgaaaagatggagtataaactgttaccgagtccagtaaaaatgctgccaaagatattcgtaaaatcgaaagccgctaaggaaaaatatggcctgacagatcgtatgcttgaatgctacgataaaggtatgcataagtcgggtagtgcgtttgatcttggcttttgccatgaactcattgattattacaagcgttgtatcgcggagtacccaggctgggatgtgttcgatttcaagtttcgcgaaacttccgattatgggtccatgaaagagttcaatgaagatgtggccggagccggttactatatgagtctgagaaaaattccgtgcagcgaagtgtaccgtctgttagacgagaaatcgatttatctatttcaaatttataacaaagattactctgaaaatgcacatggtaataagaacatgcataccatgtactgggagggtctcttttccccgcaaaacctggagtcgcccgttttcaagttgtcgggtggggcagaacttttctttcgaaaatcctcaatccctaacgatgccaaaacagtacacccgaaaggctcagtgctggttccacgtaatgatgttaacggtcggcgtattccagattcaatctaccgcgaactgacacgctattttaaccgtggcgattgccgaatcagtgacgaagccaaaagttatcttgacaaggttaagactaaaaaagcggaccatgacattgtgaaagatcgccgctttaccgtggataaaatgatgttccacgtcccgattgcgatgaactttaaggcgatcagtaaaccgaacttaaacaaaaaagtcattgatggcatcattgatgatcaggatctgaaaatcattggtattgatcgtggcgagcggaacttaatttacgtcacgatggttgacagaaaagggaatatcttatatcaggattctcttaacatcctcaatggctacgactatcgtaaagctctggatgtgcgcgaatatgacaacaaggaagcgcgtcgtaactggactaaagtggagggcattcgcaaaatgaaggaaggctatctgtcattagcggtctcgaaattagcggatatgattatcgaaaataacgccatcatcgttatggaggacctgaaccacggattcaaagcgggccgctcaaagattgaaaaacaagtttatcagaaatttgagagtatgctgattaacaaactgggctatatggtgttaaaagacaagtcaattgaccaatcaggtggcgcgctgcatggataccagctggcgaaccatgttaccaccttagcatcagttggaaagcagtgtggggttatcttttatataccggcagcgttcactagtaaaatagatccgaccactggtttcgccgatctctttgccctgagtaacgttaaaaacgtagcgagcatgcgtgaattcttttccaaaatgaaatctgtcatttatgataaagctgaaggcaaattcgcattcacctttgattacttggattacaacgtgaagagcgaatgtggtcgtacgctgtggaccgtttacaccgttggtgagcgcttcacctattcccgtgtgaaccgcgaatatgtacgtaaagtccccaccgatattatctatgatgccctccagaaagcaggcattagcgtcgaaggagacttaagggacagaattgccgaaagcgatggcgatacgctgaagtctattttttacgcattcaaatacgcgctagatatgcgcgttgagaatcgcgaggaagactacattcaatcacctgtgaaaaatgcctctggggaatttttttgttcaaaaaatgctggtaaaagcctcccacaagatagcgatgcaaacggtgcatataacattgccctgaaaggtattcttcaattacgcatgctgtctgagcagtacgaccccaacgcggaatctattagacttccgctgataaccaataaagcctggctgacattcatgcagtctggcatgaagacctggaaaaattaggaaatcatccttagcgaaagctaaggattttttttatctgaaatgtagggagaccctcaggttaaatattcactcaggaagttattactcaggaagcaaagaggattaca

SEQ ID NO: 66 - DNA, 4565 bp, Artificial Sequence
  Description of Artificial Sequence: Synthetic polynucleotide
aaaattccatgcaaaatgctccggtttcatgtcatcaaaatgatgacgtaattaagcattgataattgagatccctctccctgacaggatgattacataaataatagtgacaaaaataaattatttatttatccagaaaatgaattggaaaatcaggagagcgttttcaatcctacctctggcgcagttgatatgtcaaacaggttgccgtcactgcgtcttttactggctcttctcgctaaccaaaccggtaaccccgcttattaaaagcattctgtaacaaagcgggaccaaagccatgacaaaaacgcgtaacaaaagtgtctataatcacggcagaaaagtccacattgattatttgcacggcgtcacactttgctatgccatagcatttttatccataagattagcggatcctacctgacgctttttatcgcaactctctactgtttctccatacccgtttttttgggctagcaccgcctatctcgtgtgagataggcggagatacgaactttaagaaggagatataccatggatagtttgaaagatttcaccaatctgtaccctgtcagtaagacattgagatttgaattaaagcccgttggaaagactttagaaaatatcgagaaagcaggtattttgaaagaggatgagcatcgtgcagaaagttatcggagggtgaagaaaataattgatacttatcataaggtatttatcgattcttctcttgaaaatatggctaaaatgggtattgagaatgaaataaaagcaatgctccaaagtttctgcgaattgtataaaaaagatcatcgcactgagggtgaagacaaggcattagataaaattcgagcagtacttcgtggcctgattgttggggctttcactggtgtttgcggaagacgggaaaatacagtccaaaacgagaagtacgagagtttgttcaaagaaaagttgataaaagaaattttacctgattttgtgctctctactgaggctgaaagcttgcctttctctgttgaagaagctacgaggtcactgaaggagtttgatagctttacatcctactttgctggtttttacgagaatagaaagaatatatactcgacgaaacctcaatccactgccattgcttatcgtcttattcatgagaacttgccgaagttcattgataatattcttgtttttcagaagatcaaagagcctatagccaaagagctggaacatattcgtgcggacttttctgccggggggtacataaaaaaggatgagagattggaggatattttttcgttgaactattatatccacgtgttatctcaggctgggatcgaaaaatataacgcattgattgggaagattgtgacagaaggagatggagagatgaaagggctcaatgaacacatcaacctttacaaccaacaaagaggcagagaggatcggctccctctttttaggcctctttataaacagatattgagtgacagagagcaattatcatacttgcctgagagttttgaaaaagatgaggagctcctcagggctctaaaagagttctatgatcatatcgcagaagacattctcggacgtactcaacagttgatgacttctatttcagaatatgatttatctcggatatacgtaaggaacgatagccaattgactgatatatcaaaaaaaatgttgggagattggaatgctatctacatggctagagaacgagcatatgaccacgagcaggctcccaaaagaatcacggcgaaatacgagagggacaggattaaagctcttaaaggagaagagagtataagtctggcaaatcttaatagttgtattgcctttctggacaatgttagagattgccgtgtagatacttatctttccacactgggccagaaggaaggaccacatggtctatctaatctcgttgagaacgtttttgcctcataccatgaagcagagcaattgttgagctttccataccccgaagagaataatctgattcaggacaaggacaatgtggtgttaattaagaatcttctcgacaatatcagtgatctgcagaggttcttgaaacctctttggggtatgggagacgaacccgataaagatgaaagattttatggagagtataattatatccgaggagctctagatcaggtgatccctctgtacaataaggtaaggaactacctcactcggaagccttattcgaccagaaaagtaaaactcaattttgggaattctcaattgcttagtggttgggatagaaataaggaaaaggataatagctgtgtgattttgcgtaaggggcagaacttctatttggctattatgaacaataggcacaaaagaagtttcgaaaacaaggtgttgcccgagtataaggagggagaaccttacttcgaaaagatggattataaatttttgcctgatcctaataaaatgcttcctaaggtttttctttcgaaaaaaggaatagagatatacaaaccaagtccgaagcttttagaacaatatggacatggaactcacaaaaagggagatacctttagtatggatgatttgcacgaactgatcgatttcttcaaacactcaatcgaggctcatgaagattggaagcaattcggattcaaattttctgatacggctacttatgagaatgtatctagtttctatagagaagttgaggatcaggggtataagctctctttccgaaaagtttcggaatcttatgtctattcattaatagatcaaggcaagttgtatttatttcagatatacaacaaggacttttctccctgcagcaaagggacacctaatctgcataccttgtattggagaatgctttttgacgagcgcaatttggcagatgtcatatacaaactggatgggaaggctgaaatctttttccgagagaagagtttgaaaaatgatcatcccacgcatccggctggtaagcctatcaaaaagaaaagtcgacaaaaaaaaggagaggagagtctgtttgagtatgatttagtcaaggataggcactatacgatggataagttccagtttcatgtgcctattactatgaattttaaatgttctgcaggaagcaaagtcaatgatatggttaatgctcatattcgagaggcaaaggatatgcatgtcattggaattgatcgtggagaacgcaatctgctgtatatatgcgtgatagatagtcgagggacgattttggatcaaatttctctgaatacgattaacgatatagactatcatgatttattggagagtcgagacaaagaccgtcagcaggagcgccgaaactggcaaactatcgaagggatcaaggagctaaaacaaggctaccttagtcaggcggttcatcggatagccgaactgatggtggcttataaggctgtagttgctttggaggatttgaatatggggttcaaacgtgggcggcagaaagtagaaagttctgtttatcagcagtttgagaaacagctgatagataagctcaactatcttgtggacaagaagaaaaggcctgaagatattggaggattgttgagagcctatcaatttacggccccatttaagagttttaaggaaatgggaaagcaaaacggcttcttgttttatatcccggcttggaacacgagcaacatagatccgactactggatttgttaatttatttcatgcccagtatgaaaatgtagataaagcgaagagcttctttcaaaagtttgattcaattagttacaacccgaagaaagactggtttgagtttgcattcgattataaaaactttactaaaaaggctgaaggaagtcgttctatgtggatattatgcacacatggttcccgaataaagaattttagaaattcccagaagaatggtcaatgggattccgaagaattcgccttgacggaggcttttaagtctctttttgtgcgatatgagatagattataccgctgatttgaaaacagctattgtggacgaaaagcaaaaagacttcttcgtggatcttctgaagctattcaaattgacagtacagatgcgcaacagctggaaagagaaggatttggattatctaatctctcctgtagcaggggctgatggccgtttcttcgatacaagagagggaaataaaagtctgcctaaggatgcagatgccaatggagcttataatattgccctaaaaggactttgggctctacgccagattcggcaaacttcagaaggcggtaaactcaaattggcgatttccaataaggaatggctacagtttgtgcaagagagatcttacgagaaagactgagaaatcatccttagcgaaagctaaggattttttttatctgaaatttattatatcgcgttgattattgatgctgtttttagttttaacggcaattaatatatgtgttattaattgaatgaattttatcattcataataagtatgtgtaggatcaagctcaggttaaatattcactcaggaagttattactcaggaagcaaagaggattacagaattatctcataacaagtgttaagggatgttatttcc

SEQ ID NO: 67 - DNA, 4574 bp, Artificial Sequence
  Description of Artificial Sequence: Synthetic polynucleotide
aaaattccatgcaaaatgctccggtttcatgtcatcaaaatgatgacgtaattaagcattgataattgagatccctctccctgacaggatgattacataaataatagtgacaaaaataaattatttatttatccagaaaatgaattggaaaatcaggagagcgttttcaatcctacctctggcgcagttgatatgtcaaacaggttgccgtcactgcgtcttttactggctcttctcgctaaccaaaccggtaaccccgcttattaaaagcattctgtaacaaagcgggaccaaagccatgacaaaaacgcgtaacaaaagtgtctataatcacggcagaaaagtccacattgattatttgcacggcgtcacactttgctatgccatagcatttttatccataagattagcggatcctacctgacgctttttatcgcaactctctactgtttctccatacccgtttttttgggctagcaccgcctatctcgtgtgagataggcggagatacgaactttaagaaggagatataccatgaacaacggcacaaataattttcagaacttcatcgggatctcaagtttgcagaaaacgctgcgcaatgctctgatccccacggaaaccacgcaacagttcatcgtcaagaacggaataattaaagaagatgagttacgtggcgagaaccgccagattctgaaagatatcatggatgactactaccgcggattcatctctgagactctgagttctattgatgacatagattggactagcctgttcgaaaaaatggaaattcagctgaaaaatggtgataataaagataccttaattaaggaacagacagagtatcggaaagcaatccataaaaaatttgcgaacgacgatcggtttaagaacatgtttagcgccaaactgattagtgacatattacctgaatttgtcatccacaacaataattattcggcatcagagaaagaggaaaaaacccaggtgataaaattgttttcgcgctttgcgactagctttaaagattacttcaagaaccgtgcaaattgcttttcagcggacgatatttcatcaagcagctgccatcgcatcgtcaacgacaatgcagagatattcttttcaaatgcgctggtctaccgccggatcgtaaaatcgctgagcaatgacgatatcaacaaaatttcgggcgatatgaaagattcattaaaagaaatgagtctggaagaaatatattcttacgagaagtatggggaatttattacccaggaaggcattagcttctataatgatatctgtgggaaagtgaattcttttatgaacctgtattgtcagaaaaataaagaaaacaaaaatttatacaaacttcagaaacttcacaaacagattctatgcattgcggacactagctatgaggtcccgtataaatttgaaagtgacgaggaagtgtaccaatcagttaacggcttccttgataacattagcagcaaacatatagtcgaaagattacgcaaaatcggcgataactataacggctacaacctggataaaatttatatcgtgtccaaattttacgagagcgttagccaaaaaacctaccgcgactgggaaacaattaataccgccctcgaaattcattacaataatatcttgccgggtaacggtaaaagtaaagccgacaaagtaaaaaaagcggttaagaatgatttacagaaatccatcaccgaaataaatgaactagtgtcaaactataagctgtgcagtgacgacaacatcaaagcggagacttatatacatgagattagccatatcttgaataactttgaagcacaggaattgaaatacaatccggaaattcacctagttgaatccgagctcaaagcgagtgagcttaaaaacgtgctggacgtgatcatgaatgcgtttcattggtgttcggtttttatgactgaggaacttgttgataaagacaacaatttttatgcggaactggaggagatttacgatgaaatttatccagtaattagtctgtacaacctggttcgtaactacgttacccagaaaccgtacagcacgaaaaagattaaattgaactttggaataccgacgttagcagacggttggtcaaagtccaaagagtattctaataacgctatcatactgatgcgcgacaatctgtattatctgggcatctttaatgcgaagaataaaccggacaagaagattatcgagggtaatacgtcagaaaataagggtgactacaaaaagatgatttataatttgctcccgggtcccaacaaaatgatcccgaaagttttcttgagcagcaagacgggggtggaaacgtataaaccgagcgcctatatcctagaggggtataaacagaataaacatatcaagtcttcaaaagactttgatatcactttctgtcatgatctgatcgactacttcaaaaactgtattgcaattcatcccgagtggaaaaacttcggttttgattttagcgacaccagtacttatgaagacatttccgggttttatcgtgaggtagagttacaaggttacaagattgattggacatacattagcgaaaaagacattgatctgctgcaggaaaaaggtcaactgtatctgttccagatatataacaaagatttttcgaaaaaatcaaccgggaatgacaaccttcacaccatgtacctgaaaaatcttttctcagaagaaaatcttaaggatatcgtcctgaaacttaacggcgaagcggaaatcttcttcaggaagagcagcataaagaacccaatcattcataaaaaaggctcgattttagtcaaccgtacctacgaagcagaagaaaaagaccagtttggcaacattcaaattgtgcgtaaaaatattccggaaaacatttatcaggagctgtacaaatacttcaacgataaaagcgacaaagagctgtctgatgaagcagccaaactgaagaatgtagtgggacaccacgaggcagcgacgaatatagtcaaggactatcgctacacgtatgataaatacttccttcatatgcctattacgatcaatttcaaagccaataaaacgggttttattaatgataggatcttacagtatatcgctaaagaaaaagacttacatgtgatcggcattgatcggggcgagcgtaacctgatctacgtgtccgtgattgatacttgtggtaatatagttgaacagaaaagctttaacattgtaaacggctacgactatcagataaaactgaaacaacaggagggcgctagacagattgcgcggaaagaatggaaagaaattggtaaaattaaagagatcaaagagggctacctgagcttagtaatccacgagatctctaaaatggtaatcaaatacaatgcaattatagcgatggaggatttgtcttatggttttaaaaaagggcgctttaaggtcgaacggcaagtttaccagaaatttgaaaccatgctcatcaataaactcaactatctggtatttaaagatatttcgattaccgagaatggcggtctcctgaaaggttatcagctgacatacattcctgataaacttaaaaacgtgggtcatcagtgcggctgcattttttatgtgcctgctgcatacacgagcaaaattgatccgaccaccggctttgtgaatatctttaaatttaaagacctgacagtggacgcaaaacgtgaattcattaaaaaatttgactcaattcgttatgacagtgaaaaaaatctgttctgctttacatttgactacaataactttattacgcaaaacacggtcatgagcaaatcatcgtggagtgtgtatacatacggcgtgcgcatcaaacgtcgctttgtgaacggccgcttctcaaacgaaagtgataccattgacataaccaaagatatggagaaaacgttggaaatgacggacattaactggcgcgatggccacgatcttcgtcaagacattatagattatgaaattgttcagcacatattcgaaattttccgtttaacagtgcaaatgcgtaactccttgtctgaactggaggaccgtgattacgatcgtctcatttcacctgtactgaacgaaaataacattttttatgacagcgcgaaagcgggggatgcacttcctaaggatgccgatgcaaatggtgcgtattgtattgcattaaaagggttatatgaaattaaacaaattaccgaaaattggaaagaagatggtaaattttcgcgcgataaactcaaaatcagcaataaagattggttcgactttatccagaataagcgctatctctaagaaatcatccttagcgaaagctaaggattttttttatctgaaatttattatatcgcgttgattattgatgctgtttttagttttaacggcaattaatatatgtgttattaattgaatgaattttatcattcataataagtatgtgtaggatcaagctcaggttaaatattcactcaggaagttattactcaggaagcaaagaggattacagaattatctcataacaagtgttaagggatgttatttcc

SEQ ID NO: 68 - DNA, 4489 bp, Artificial Sequence
  Description of Artificial Sequence: Synthetic polynucleotide
aatcaggagagcgttttcaatcctacctctggcgcagttgatatgtcaaacaggttgccgtcactgcgtcttttactggctcttctcgctaaccaaaccggtaaccccgcttattaaaagcattctgtaacaaagcgggaccaaagccatgacaaaaacgcgtaacaaaagtgtctataatcacggcagaaaagtccacattgattatttgcacggcgtcacactttgctatgccatagcatttttatccataagattagcggatcctacctgacgctttttatcgcaactctctactgtttctccatacccgtttttttgggctagcagtaatacgactcactataggggtctcatctcgtgtgagataggcggagatacgaactttaagaggaggatataccatgcaccatcatcatcaccataccaataaattcactaaccagtattctctctctaagaccctgcgctttgaactgattccgcaggggaaaaccttggagttcattcaagaaaaaggcctcttgtctcaggataaacagagggctgaatcttaccaagaaatgaagaaaactattgataagtttcataaatatttcattgatttagccttgtctaacgccaaattaactcacttggaaacgtatctggagttatacaacaaatctgccgaaactaagaaagaacagaaatttaaagacgatttgaaaaaagtacaggacaatctgcgtaaagaaattgtcaaatccttcagtgacggcgatgctaaaagcatttttgccattctggacaaaaaagagttgattactgtggaattagaaaagtggtttgaaaacaatgagcagaaagacatctacttcgatgagaaattcaaaactttcaccacctattttacaggatttcatcaaaaccggaagaacatgtactcagtagaaccgaactccacggccattgcgtatcgtttgatccatgagaatctgcctaaatttctggagaatgcgaaagcctttgaaaagattaagcaggtcgaatcgctgcaagtgaattttcgtgaactcatgggcgaatttggtgacgaaggtctaatcttcgttaacgaactggaagaaatgtttcagattaattactacaatgacgtgctatcgcagaacggtatcacaatctacaatagtattatctcagggttcacaaaaaacgatataaaatacaaaggcctgaacgagtatatcaataactacaaccaaacaaaggacaaaaaggataggcttccgaaactgaagcagttatacaaacagattttatctgacagaatctccctgagctttctgccggatgctttcactgatgggaagcaggttctgaaagcgattttcgatttttataagattaacttactgagctacacgattgaaggtcaagaagaatctcaaaacttactgctcttgatccgtcaaaccattgaaaatctatcatcgttcgatacgcagaaaatctacctcaaaaacgatactcacctgactacgatctctcagcaggttttcggggattttagtgtattttcaacagctctgaactactggtatgaaaccaaagtcaatccgaaattcgagacggaatattctaaggccaacgaaaaaaaacgtgagattcttgataaagctaaagccgtatttactaaacaggattacttttctattgctttcctgcaggaagttttatcggagtatatcctgaccctggatcatacatctgatatcgttaaaaaacacagcagcaattgcatcgctgactatttcaaaaaccactttgtcgccaaaaaagaaaacgaaacagacaagactttcgatttcattgctaacatcaccgcaaaataccagtgtattcagggtatcttggaaaacgccgaccaatacgaagacgaactgaaacaagatcagaagctgatcgataatttaaaattcttcttagatgcaatcctggagctgctgcacttcatcaaaccgcttcatttaaagagcgagtccattaccgaaaaggacaccgccttctatgacgtttttgaaaattattatgaagccctctccttgctgactccgctgtataatatggtacgcaattacgtaacccagaaaccatattctaccgaaaaaattaaactgaactttgaaaacgcacagctgctcaacggttgggacgcgaataaagaaggtgactacctcaccaccatcctgaaaaaagatggtaactattttctggcaattatggataagaaacataataaagcattccagaaatttcctgaagggaaagaaaattacgaaaagatggtgtacaaactcttacctggagttaacaaaatgttgccgaaagtattttttagtaataagaacatcgcgtactttaacccgtccaaagaactgctggaaaattataaaaaggagacgcataagaaaggggatacctttaacctggaacattgccataccttaatagacttcttcaaggattccctgaataaacacgaggattggaaatatttcgattttcagtttagtgagaccaagtcataccaggatcttagcggcttttatcgcgaagtagaacaccaaggctataaaattaacttcaaaaacatcgacagcgaatacatcgacggtttagttaacgagggcaaactgtttctgttccagatctattcaaaggattttagcccgttctctaaaggcaaaccaaatatgcatacgttgtactggaaagcactgtttgaagagcaaaacctgcagaatgtgatttataaactgaacggccaagctgagatttttttccgtaaagcctcgattaaaccgaaaaatatcatccttcataagaagaaaataaagatcgctaaaaaacacttcatagataaaaaaaccaaaacctccgaaatagtgcctgttcaaacaattaagaacttgaatatgtactaccagggcaagatatcggaaaaggagttgactcaagacgatcttcgctatatcgataacttttcgatttttaacgaaaaaaacaagacgatcgacatcatcaaagataaacgcttcactgtagataagttccagtttcatgtgccgattactatgaacttcaaagctaccgggggtagctatatcaaccaaacggtgttggaatacctgcagaataacccggaagtcaaaatcattgggctggaccgcggagaacgtcaccttgtgtacttgaccttaatcgatcagcaaggcaacatcttaaaacaagaatcgctgaataccattacggattcaaagattagcaccccgtatcataagctgctcgataacaaggagaatgagcgcgacctggcccgtaaaaactggggcacggtggaaaacattaaggagttaaaggagggttatatttcccaggtagtgcataagatcgccactctcatgctcgaggaaaatgcgatcgttgtcatggaagacttaaacttcggatttaaacgtgggcgatttaaagtagagaaacaaatctaccagaagttagaaaaaatgctgattgacaaattaaattacttggtcctaaaagacaaacagccgcaagaattgggtggattatacaacgccctccaacttaccaataaattcgaaagttttcagaaaatgggtaaacagtcaggctttcttttttatgttcctgcgtggaacacatccaaaatcgaccctacaaccggcttcgtcaattacttctatactaaatatgaaaacgtcgacaaagcaaaagcattctttgaaaagttcgaagcaatacgttttaacgctgagaaaaaatatttcgagttcgaagtcaagaaatactcagactttaaccccaaagctgagggcacacagcaagcgtggacaatctgcacctacggcgagcgcatcgaaacgaagcgtcaaaaagatcagaataacaaatttgtttcaacacctatcaacctgaccgagaagattgaagacttcttaggtaaaaatcagattgtttatggcgacggtaactgtataaaatctcaaatagcctcaaaggatgataaagcatttttcgaaacattattatattggttcaaaatgacactgcagatgcgcaatagtgagacgcgtacagatattgattatcttatcagcccggtcatgaacgacaacggtactttttacaactccagagactatgaaaaacttgagaatccaactctccccaaagatgctgatgcgaacggtgcttatcacatcgcgaaaaaaggtctgatgctgctgaacaaaatcgaccaagccgatctgactaagaaagttgacctaagcatttcaaatcgggactggttacagtttgttcaaaagaacaaatgagaaatcatccttagcgaaagctaaggattttttttatctgaaatgtagggagaccctcaggttaaatattcactcaggaagttattactcaggaagcaaagaggattaca

SEQ ID NO: 69 - DNA, 4805 bp, Artificial Sequence
  Description of Artificial Sequence: Synthetic polynucleotide
aaaattccatgcaaaatgctccggtttcatgtcatcaaaatgatgacgtaattaagcattgataattgagatccctctccctgacaggatgattacataaataatagtgacaaaaataaattatttatttatccagaaaatgaattggaaaatcaggagagcgttttcaatcctacctctggcgcagttgatatgtcaaacaggttgccgtcactgcgtcttttactggctcttctcgctaaccaaaccggtaaccccgcttattaaaagcattctgtaacaaagcgggaccaaagccatgacaaaaacgcgtaacaaaagtgtctataatcacggcagaaaagtccacattgattatttgcacggcgtcacactttgctatgccatagcatttttatccataagattagcggatcctacctgacgctttttatcgcaactctctactgtttctccatacccgtttttttgggctagcaccgcctatctcgtgtgagataggcggagatacgaactttaagaaggagatataccatggaacaggaatattatctgggcttggacatgggcaccggttccgtcggctgggctgttactgacagtgaatatcacgttctaagaaagcatggtaaggcattgtggggtgtaagacttttcgaatctgcttccactgctgaagagcgtagaatgtttagaacgagtcgacgtaggctagacaggcgcaattggagaatcgaaattttacaagaaatttttgcggaagagatatctaagaaagacccaggctttttcctgagaatgaaggaatctaagtattaccctgaggataaaagagatataaatggtaactgtcccgaattgccttacgcattatttgtggacgatgattttaccgataaggattaccataaaaagttcccaactatctaccatttacgcaaaatgttaatgaatacagaggaaaccccagacataagactagtttatctggcaatacaccatatgatgaaacatagaggccatttcttactttccggggatatcaacgaaatcaaagagtttggtaccacatttagtaagttactggaaaacataaagaatgaagaattggattggaacttagaactcggaaaagaagaatacgcggttgtcgaatctatcctgaaggataatatgctgaataggtcgaccaaaaaaactaggctgatcaaagcactgaaagccaaatctatctgcgaaaaagctgttttaaatttacttgctggtggcactgttaagttatcagacatttttggtttggaagaattgaacgaaaccgagcgtccaaaaattagtttcgctgataatggctacgatgattacattggtgaggtggaaaacgagttgggcgaacaattttatattatagagacagctaaggcagtctatgactgggctgttttagtagaaatccttggtaaatacacatctatctccgaagcgaaagttgctacttacgaaaagcacaagtccgatctccagtttttgaagaaaattgtcaggaaatatctgactaaggaagaatataaagatattttcgttagtacctctgacaaactgaaaaattactccgcttacatcgggatgaccaagattaatggcaaaaaagttgatctgcaaagcaaaaggtgttcgaaggaagaattttatgatttcattaaaaagaatgtcttaaaaaaattagaaggtcagccagaatacgaatatttgaaagaagaactggaaagagagacattcttaccaaaacaagtcaacagagataatggggtaattccatatcaaattcacctctacgaattaaaaaaaattttaggcaatttacgcgataaaattgaccttatcaaagaaaatgaggataagctggttcaactctttgaattcagaataccctattatgtgggcccactgaacaagattgatgacggcaaagaaggtaaattcacatgggccgtccgcaaatccaatgaaaaaatttacccatggaactttgaaaatgtagtagatattgaagcgtctgcggagaaatttattcgaagaatgactaataaatgcacttacttgatgggagaggatgttctgcctaaagacagcttattatacagcaagtacatggttctaaacgaacttaacaacgttaagttggacggtgagaaattaagtgtagaattgaaacaaagattgtatactgacgtcttctgcaagtacagaaaagtgacagttaaaaaaattaagaattacttgaagtgcgaaggtataatttctggaaacgtagagattactggtattgatggtgatttcaaagcatccctaacagcttaccacgatttcaaggaaatcctgacaggaactgaactcgcaaaaaaagataaagaaaacattattactaatattgttcttttcggtgatgacaagaaattgttgaagaaaagactgaatagactttacccccagattactcccaatcaacttaagaaaatttgtgctttgtcttacacaggatggggtcgtttttcaaaaaagttcttagaagagattaccgcacctgatccagaaacaggcgaagtatggaatataattaccgccttatgggaatcgaacaataatcttatgcaacttctgagcaatgaatatcgtttcatggaagaagttgagacttacaacatgggcaaacagacgaagactttatcctatgaaactgtggaaaatatgtatgtatcaccttctgtcaagagacaaatttggcaaaccttaaaaattgtcaaagaattagaaaaggtaatgaaggagtctcctaaacgtgtgtttattgaaatggctagagaaaaacaagagtcaaaaagaaccgagtcaagaaagaagcagttaatcgatttatataaggcttgtaaaaacgaagagaaagattgggttaaagaattgggggaccaagaggaacaaaaactacggtcggataagttgtatttatactatacgcaaaagggacgatgtatgtattccggcgaggtaatagaattgaaggatttatgggacaatacaaaatatgacatagaccatatatatccccaatcaaaaacgatggacgatagcttgaacaatagagtactcgtgaaaaaaaaatataatgcgaccaaatctgataagtatcctctgaatgaaaatatcagacatgaaagaaaggggttctggaagtccttgttagatggtgggtttataagcaaagaaaagtacgagcgtctaataagaaacacggagttatcgccagaagaactcgctggttttattgagaggcaaatcgtggaaacgagacaatctaccaaagccgttgctgagatcctaaagcaagttttcccagagtcggagattgtctatgtcaaagctggcacagtgagcaggtttaggaaagacttcgaactattaaaggtaagagaagtgaacgatttacatcacgcaaaggacgcttacctaaatatcgttgtaggtaactcatattatgttaaatttaccaagaacgcctcttggtttataaaggagaacccaggtagaacatataacctgaaaaagatgttcacctctggttggaatattgagagaaacggagaagtcgcatgggaagttggtaagaaagggactatagtgacagtaaagcaaattatgaacaaaaataatatcctcgttacaaggcaggttcatgaagcaaagggcggcctttttgaccaacaaattatgaagaaagggaaaggtcaaattgcaataaaagaaaccgatgagagactagcgtcaatagaaaagtatggtggctataataaagctgcgggtgcatactttatgcttgttgaatcaaaagacaagaaaggtaagactattagaactatagaatttatacccctgtaccttaaaaacaaaattgaatcggatgagtcaatcgcgttaaattttctagagaaaggaaggggtttaaaagaaccaaagatcctgttaaaaaagattaagattgacaccttgttcgatgtagatggatttaaaatgtggttatctggcagaacaggcgatagacttttgtttaagtgcgctaatcaattaattttggatgagaaaatcattgtcacaatgaaaaaaatagttaagtttattcagagaagacaagaaaacagggagttgaaattatctgataaagatggtatcgacaatgaagttttaatggaaatctacaatacattcgttgataaacttgaaaataccgtatatcgaatcaggttaagtgaacaagccaaaacattaattgataaacaaaaagaatttgaaaggctatcactggaagacaaatcctccaccctatttgaaattttgcatatattccagtgccaatcttcagcagctaatttaaaaatgattggcggacctgggaaagccggcatcctagtgatgaacaataatatctccaagtgtaacaaaatatcaattattaaccaatctccgacaggtatttttgaaaatgaaatagacttgcttaagatataagaaatcatccttagcgaaagctaaggattttttttatctgaaatttattatatcgcgttgattattgatgctgtttttagttttaacggcaattaatatatgtgttattaattgaatgaattttatcattcataataagtatgtgtaggatcaagctcaggttaaatattcactcaggaagttattactcaggaagcaaagaggattacagaattatctcataacaagtgttaagggatgttatttcc

SEQ ID NO: 70 - DNA, 4363 bp, Artificial Sequence
  Description of Artificial Sequence: Synthetic polynucleotide
aatcaggagagcgttttcaatcctacctctggcgcagttgatatgtcaaacaggttgccgtcactgcgtcttttactggctcttctcgctaaccaaaccggtaaccccgcttattaaaagcattctgtaacaaagcgggaccaaagccatgacaaaaacgcgtaacaaaagtgtctataatcacggcagaaaagtccacattgattatttgcacggcgtcacactttgctatgccatagcatttttatccataagattagcggatcctacctgacgctttttatcgcaactctctactgtttctccatacccgtttttttgggctagcagtaatacgactcactataggggtctcatctcgtgtgagataggcggagatacgaactttaagaggaggatataccatgcaccatcatcatcaccattctttcgactctttcaccaacctgtactctctgtctaaaaccctgaaattcgaaatgcgtccggttggtaacacccagaaaatgctggacaacgcgggtgttttcgaaaaagacaaactgatccagaaaaaatacggtaaaaccaaaccgtacttcgaccgtctgcaccgtgaattcatcgaagaagcgctgaccggtgttgaactgatcggtctggacgaaaacttccgtaccctggttgactggcagaaagacaaaaaaaacaacgttgcgatgaaagcgtacgaaaactctctgcagcgtctgcgtaccgaaatcggtaaaatcttcaacctgaaagcggaagactgggttaaaaacaaatacccgatcctgggtctgaaaaacaaaaacaccgacatcctgttcgaagaagcggttttcggtatcctgaaagcgcgttacggtgaagaaaaagacaccttcatcgaagttgaagaaatcgacaaaaccggtaaatctaaaatcaaccagatctctatcttcgactcttggaaaggtttcaccggttacttcaaaaaattcttcgaaacccgtaaaaacttctacaaaaacgacggtacctctaccgcgatcgcgacccgtatcatcgaccagaacctgaaacgtttcatcgacaacctgtctatcgttgaatctgttcgtcagaaagttgacctggcggaaaccgaaaaatctttctctatctctctgtctcagttcttctctatcgacttctacaacaaatgcctgctgcaggacggtatcgactactacaacaaaatcatcggtggtgaaaccctgaaaaacggtgaaaaactgatcggtctgaacgaactgatcaaccagtaccgtcagaacaacaaagaccagaaaatcccgttcttcaaactgctggacaaacagatcctgtctgaaaaaatcctgttcctggacgaaatcaaaaacgacaccgaactgatcgaagcgctgtctcagttcgcgaaaaccgcggaagaaaaaaccaaaatcgttaaaaaactgttcgcggacttcgttgaaaacaactctaaatacgacctggcgcagatctacatctctcaggaagcgttcaacaccatctctaacaaatggacctctgaaaccgaaaccttcgcgaaatacctgttcgaagcgatgaaatctggtaaactggcgaaatacgaaaaaaaagacaactcttacaaattcccggacttcatcgcgctgtctcagatgaaatctgcgctgctgtctatctctctggaaggtcacttctggaaagaaaaatactacaaaatctctaaattccaggaaaaaaccaactgggaacagttcctggcgatcttcctgtacgaattcaactctctgttctctgacaaaatcaacaccaaagacggtgaaaccaaacaggttggttactacctgttcgcgaaagacctgcacaacctgatcctgtctgaacagatcgacatcccgaaagactctaaagttaccatcaaagacttcgcggactctgttctgaccatctaccagatggcgaaatacttcgcggttgaaaaaaaacgtgcgtggctggcggaatacgaactggactctttctacacccagccggacaccggttacctgcagttctacgacaacgcgtacgaagacatcgttcaggtttacaacaaactgcgtaactacctgaccaaaaaaccgtactctgaagaaaaatggaaactgaacttcgaaaactctaccctggcgaacggttgggacaaaaacaaagaatctgacaactctgcggttatcctgcagaaaggtggtaaatactacctgggtctgatcaccaaaggtcacaacaaaatcttcgacgaccgtttccaggaaaaattcatcgttggtatcgaaggtggtaaatacgaaaaaatcgtttacaaattcttcccggaccaggcgaaaatgttcccgaaagtttgcttctctgcgaaaggtctggaattcttccgtccgtctgaagaaatcctgcgtatctacaacaacgcggaattcaaaaaaggtgaaacctactctatcgactctatgcagaaactgatcgacttctacaaagactgcctgaccaaatacgaaggttgggcgtgctacaccttccgtcacctgaaaccgaccgaagaataccagaacaacatcggtgaattcttccgtgacgttgcggaagacggttaccgtatcgacttccagggtatctctgaccagtacatccacgaaaaaaacgaaaaaggtgaactgcacctgttcgaaatccacaacaaagactggaacctggacaaagcgcgtgacggtaaatctaaaaccacccagaaaaacctgcacaccctgtacttcgaatctctgttctctaacgacaacgttgttcagaacttcccgatcaaactgaacggtcaggcggaaatcttctaccgtccgaaaaccgaaaaagacaaactggaatctaaaaaagacaaaaaaggtaacaaagttatcgaccacaaacgttactctgaaaacaaaatcttcttccacgttccgctgaccctgaaccgtaccaaaaacgactcttaccgtttcaacgcgcagatcaacaacttcctggcgaacaacaaagacatcaacatcatcggtgttgaccgtggtgaaaaacacctggtttactactctgttatcacccaggcgtctgacatcctggaatctggttctctgaacgaactgaacggtgttaactacgcggaaaaactgggtaaaaaagcggaaaaccgtgaacaggcgcgtcgtgactggcaggacgttcagggtatcaaagacctgaaaaaaggttacatctctcaggttgttcgtaaactggcggacctggcgatcaaacacaacgcgatcatcatcctggaagacctgaacatgcgtttcaaacaggttcgtggtggtatcgaaaaatctatctaccagcagctggaaaaagcgctgatcgacaaactgtctttcctggttgacaaaggtgaaaaaaacccggaacaggcgggtcacctgctgaaagcgtaccagctgtctgcgccgttcgaaaccttccagaaaatgggtaaacagaccggtatcatcttctacacccaggcgtcttacacctctaaatctgacccggttaccggttggcgtccgcacctgtacctgaaatacttctctgcgaaaaaagcgaaagacgacatcgcgaaattcaccaaaatcgaattcgttaacgaccgtttcgaactgacctacgacatcaaagacttccagcaggcgaaagaatacccgaacaaaaccgtttggaaagtttgctctaacgttgaacgtttccgttgggacaaaaacctgaaccagaacaaaggtggttacacccactacaccaacatcaccgaaaacatccaggaactgttcaccaaatacggtatcgacatcaccaaagacctgctgacccagatctctaccatcgacgaaaaacagaacacctctttcttccgtgacttcatcttctacttcaacctgatctgccagatccgtaacaccgacgactctgaaatcgcgaaaaaaaacggtaaagacgacttcatcctgtctccggttgaaccgttcttcgactctcgtaaagacaacggtaacaaactgccggaaaacggtgacgacaacggtgcgtacaacatcgcgcgtaaaggtatcgttatcctgaacaaaatctctcagtactctgaaaaaaacgaaaactgcgaaaaaatgaaatggggtgacctgtacgtttctaacatcgactgggacaacttcgttgaaatcatccttagcgaaagctaaggattttttttatctgaaatgtagggagaccctcaggttaaatattcactcaggaagttattactcaggaagcaaagaggattaca

SEQ ID NO: 71 - DNA, 4375 bp, Artificial Sequence
  Description of Artificial Sequence: Synthetic polynucleotide
aatcaggagagcgttttcaatcctacctctggcgcagttgatatgtcaaacaggttgccgtcactgcgtcttttactggctcttctcgctaaccaaaccggtaaccccgcttattaaaagcattctgtaacaaagcgggaccaaagccatgacaaaaacgcgtaacaaaagtgtctataatcacggcagaaaagtccacattgattatttgcacggcgtcacactttgctatgccatagcatttttatccataagattagcggatcctacctgacgctttttatcgcaactctctactgtttctccatacccgtttttttgggctagcagtaatacgactcactataggggtctcatctcgtgtgagataggcggagatacgaactttaagaggaggatataccatgcaccatcatcatcaccataacaaattcgaaaacttcaccggtctgtacccgatctctaaaaccctgcgtttcgaactgatcccgcagggtaaaaccctggaatacatcgaaaaatctgaaatcctggaaaacgacaactaccgtgcggaaaaatacgaagaagttaaagacatcatcgacggttaccacaaatggttcatcaacgaaaccctgcacgacctgcacatcaactggtctgaactgaaagttgcgctggaaaacaaccgtatcgaaaaatctgacgcgtctaaaaaagaactgcagcgtgttcagaaaatcaaacgtgaagaaatctacaacgcgttcatcgaacacgaagcgttccagtacctgttcaaagaaaacctgctgtctgacctgctgccgatccagatcgaacagtctgaagacctggacgcggaaaaaaaaaaacaggcggttgaaaccttcaaccgtttctctacctacttcaccggtttccacgaaaaccgtaaaaacatctactctaaagaaggtatctctacctctgttacctaccgtatcgttcacgacaacttcccgaaattcctggaaaacatgaaagttttcgaaatcctgcgtaacgaatgcccggaagttatctctgacaccgcgaacgaactggcgccgttcatcgacggtgttcgtatcgaagacatcttcctgatcgacttcttcaactctaccttctctcagaacggtatcgactactacaaccgtatcctgggtggtgttaccaccgaaaccggtgaaaaataccgtggtatcaacgaattcaccaacctgtaccgtcagcagcacccggaattcggtaaatctaaaaaagcgaccaaaatggttgttctgttcaaacagatcctgtctgaccgtgacaccctgtctttcatcccggaaatgttcggtaacgacaaacaggttcagaactctatccagctgttctacaaccgtgaaatctctcagttcgaaaacgaaggtgttaaaaccgacgtttgcaccgcgctggcgaccctgacctctaaaatcgcggaattcgacaccgaaaaaatctacatccagcagccggaactgccgaacgtttctcagcgtctgttcggttcttggaacgaactgaacgcgtgcctgttcaaatacgcggaactgaaattcggtaccgcggaaaaagttgcgaaccgtaaaaaaatcgacaaatggctgaaatctgacctgttctctttcaccgaactgaacaaagcgctggaattctctggtaaagacgaacgtatcgaaaactacttctctgaaaccggtatcttcgcgcagctggttaaaaccggtttcgacgaagcgcagtctatcctggaaaccgaatacacctctgaagttcacctgaaagaccagcagaccgacatcgaaaaaatcaaaaccttcctggacgcgctgcagaacctgatgcacctgctgaaatctctgtgcgtttctgaagaagcggaccgtgacgcggcgttctacaacgaattcgacatgctgtacaaccagctgaaactggttgttccgctgtacaacaaagttcgtaactacatcacccagaaactgttccgttctgacaaaatcaaaatctacttcgaaaacaaaggtcagttcctgggtggttgggttgactctcagaccgaaaactctgacaacggtacccaggcgggtggttacatcttccgtaaagaaaacgttatcaacgaatacgactactacctgggtatctgctctgacccgaaactgttccgtcgtaccaccatcgtttctgaaaacgaccgttcttctttcgaacgtctggactactaccagctgaaaaccgcgtctgtttacggtaactcttactgcggtaaacacccgtacaccgaagacaaaaacgaactggttaactctatcgaccgtttcgttcacctgtctggtaacaacatcctgatcgaaaaaatcgcgaaagacaaagttaaatctaacccgaccaccaacaccccgtctggttacctgaacttcatccaccgtgaagcgccgaacacctacgaatgcctgctgcaggacgaaaacttcgtttctctgaaccagcgtgttgtttctgcgctgaaagcgaccctggcgaccctggttcgtgttccgaaagcgctggtttacgcgaaaaaagactaccacctgttctctgaaatcatcaacgacatcgacgaactgtcttacgaaaaagcgttctcttacttcccggtttctcagaccgaattcgaaaactcttctaaccgtaccatcaaaccgctgctgctgttcaaaatctctaacaaagacctgtctttcgcggaaaacttcgaaaaaggtaaccgtcagaaaatcggtaaaaaaaacctgcacaccctgtacttcgaagcgctgatgaaaggtaaccaggacaccatcgacatcggtaccggtatggttttccaccgtgttaaatctctgaactacaacgaaaaaaccctgaaatacggtcaccactctacccagctgaacgaaaaattctcttacccgatcatcaaagacaaacgtttcgcgtctgacaaattcctgttccacctgtctaccgaaatcaactacaaagaaaaacgtaaaccgctgaacaactctatcatcgaattcctgaccaacaacccggacatcaacatcatcggtctggaccgtggtgaacgtcacctgatctacctgaccctgatcaaccagaaaggtgaaatcctgcgtcagaaaaccttcaacatcgttggtaacaccaactaccacgaaaaactgaaccagcgtgaaaaagaacgtgacaacgcgcgtaaatcttgggcgaccatcggtaaaatcaaagaactgaaagaaggtttcctgtctctggttatccacgaaatcgcgaaaatcatggttgaaaacaacgcgatcgttgttctggaagacctgaacttcggtttcaaacgtggtcgtttcaaagttgaaaaacagatctaccagaaattcgaaaaaatgctgatcgacaaactgaactacctggttttcaaagacaaaaaagcgaacgaagcgggtggtgttctgaaaggttaccagctggcggaaaaattcgaatctttccagaaaatgggtaaacagtctggtttcctgttctacgttccggcggcgtacacctctaaaatcgacccgaccaccggtttcgttaacatgctgaacctgaactacaccaacatgaaagacgcgcagaccctgctgtctggtatggacaaaatctctttcaacgcggacgcgaactacttcgaattcgaactggactacgaaaaattcaaaaccaaccagaccgaccacaccaacaaatggaccatctgcaccgttggtgaaaaacgtttcacctacaactctgcgaccaaagaaaccaccaccgttaacgttaccgaagacctgaaaaaactgctggacaaattcgaagttaaatactctaacggtgacaacatcaaagacgaaatctgccgtcagaccgacgcgaaattcttcgaaatcatcctgtggctgctgaaactgaccatgcagatgcgtaactctaacaccaaaaccgaagaagacttcatcctgtctccggttaaaaactctaacggtgaattcttccgttctaacgacgacgcgaacggtatctggccggcggacgcggacgcgaacggtgcgtaccacatcgcgctgaaaggtctgtacctggttaaagaatgcttcaacaaaaacgaaaaatctctgaaaatcgaacacaaaaactggttcaaattcgcgcagacccgtttcaacggttctctgaccaaaaacggttaagaaatcatccttagcgaaagctaaggattttttttatctgaaatgtagggagaccctcaggttaaatattcactcaggaagttattactcaggaagcaaagaggattaca

SEQ ID NO: 72 - DNA, 4455 bp, Artificial Sequence
  Description of Artificial Sequence: Synthetic polynucleotide
aatcaggagagcgttttcaatcctacctctggcgcagttgatatgtcaaacaggttgccgtcactgcgtcttttactggctcttctcgctaaccaaaccggtaaccccgcttattaaaagcattctgtaacaaagcgggaccaaagccatgacaaaaacgcgtaacaaaagtgtctataatcacggcagaaaagtccacattgattatttgcacggcgtcacactttgctatgccatagcatttttatccataagattagcggatcctacctgacgctttttatcgcaactctctactgtttctccatacccgtttttttgggctagcagtaatacgactcactataggggtctcatctcgtgtgagataggcggagatacgaactttaagaggaggatataccatgcaccatcatcatcaccatacccagttcgaaggtttcaccaacctgtaccaggtttctaaaaccctgcgtttcgaactgatcccgcagggtaaaaccctgaaacacatccaggaacagggtttcatcgaagaagacaaagcgcgtaacgaccactacaaagaactgaaaccgatcatcgaccgtatctacaaaacctacgcggaccagtgcctgcagctggttcagctggactgggaaaacctgtctgcggcgatcgactcttaccgtaaagaaaaaaccgaagaaacccgtaacgcgctgatcgaagaacaggcgacctaccgtaacgcgatccacgactacttcatcggtcgtaccgacaacctgaccgacgcgatcaacaaacgtcacgcggaaatctacaaaggtctgttcaaagcggaactgttcaacggtaaagttctgaaacagctgggtaccgttaccaccaccgaacacgaaaacgcgctgctgcgttctttcgacaaattcaccacctacttctctggtttctacgaaaaccgtaaaaacgttttctctgcggaagacatctctaccgcgatcccgcaccgtatcgttcaggacaacttcccgaaattcaaagaaaactgccacatcttcacccgtctgatcaccgcggttccgtctctgcgtgaacacttcgaaaacgttaaaaaagcgatcggtatcttcgtttctacctctatcgaagaagttttctctttcccgttctacaaccagctgctgacccagacccagatcgacctgtacaaccagctgctgggtggtatctctcgtgaagcgggtaccgaaaaaatcaaaggtctgaacgaagttctgaacctggcgatccagaaaaacgacgaaaccgcgcacatcatcgcgtctctgccgcaccgtttcatcccgctgttcaaacagatcctgtctgaccgtaacaccctgtctttcatcctggaagaattcaaatctgacgaagaagttatccagtctttctgcaaatacaaaaccctgctgcgtaacgaaaacgttctggaaaccgcggaagcgctgttcaacgaactgaactctatcgacctgacccacatcttcatctctcacaaaaaactggaaaccatctcttctgcgctgtgcgaccactgggacaccctgcgtaacgcgctgtacgaacgtcgtatctctgaactgaccggtaaaatcaccaaatctgcgaaagaaaaagttcagcgttctctgaaacacgaagacatcaacctgcaggaaatcatctctgcggcgggtaaagaactgtctgaagcgttcaaacagaaaacctctgaaatcctgtctcacgcgcacgcggcgctggaccagccgctgccgaccaccctgaaaaaacaggaagaaaaagaaatcctgaaatctcagctggactctctgctgggtctgtaccacctgctggactggttcgcggttgacgaatctaacgaagttgacccggaattctctgcgcgtctgaccggtatcaaactggaaatggaaccgtctctgtctttctacaacaaagcgcgtaactacgcgaccaaaaaaccgtactctgttgaaaaattcaaactgaacttccagatgccgaccctggcgtctggttgggacgttaacaaagaaaaaaacaacggtgcgatcctgttcgttaaaaacggtctgtactacctgggtatcatgccgaaacagaaaggtcgttacaaagcgctgtctttcgaaccgaccgaaaaaacctctgaaggtttcgacaaaatgtactacgactacttcccggacgcggcgaaaatgatcccgaaatgctctacccagctgaaagcggttaccgcgcacttccagacccacaccaccccgatcctgctgtctaacaacttcatcgaaccgctggaaatcaccaaagaaatctacgacctgaacaacccggaaaaagaaccgaaaaaattccagaccgcgtacgcgaaaaaaaccggtgaccagaaaggttaccgtgaagcgctgtgcaaatggatcgacttcacccgtgacttcctgtctaaatacaccaaaaccacctctatcgacctgtcttctctgcgtccgtcttctcagtacaaagacctgggtgaatactacgcggaactgaacccgctgctgtaccacatctctttccagcgtatcgcggaaaaagaaatcatggacgcggttgaaaccggtaaactgtacctgttccagatctacaacaaagacttcgcgaaaggtcaccacggtaaaccgaacctgcacaccctgtactggaccggtctgttctctccggaaaacctggcgaaaacctctatcaaactgaacggtcaggcggaactgttctaccgtccgaaatctcgtatgaaacgtatggcgcaccgtctgggtgaaaaaatgctgaacaaaaaactgaaagaccagaaaaccccgatcccggacaccctgtaccaggaactgtacgactacgttaaccaccgtctgtctcacgacctgtctgacgaagcgcgtgcgctgctgccgaacgttatcaccaaagaagtttctcacgaaatcatcaaagaccgtcgtttcacctctgacaaattcttcttccacgttccgatcaccctgaactaccaggcggcgaactctccgtctaaattcaaccagcgtgttaacgcgtacctgaaagaacacccggaaaccccgatcatcggtatcgaccgtggtgaacgtaacctgatctacatcaccgttatcgactctaccggtaaaatcctggaacagcgttctctgaacaccatccagcagttcgactaccagaaaaaactggacaaccgtgaaaaagaacgtgttgcggcgcgtcaggcgtggtctgttgttggtaccatcaaagacctgaaacagggttacctgtctcaggttatccacgaaatcgttgacctgatgatccactaccaggcggttgttgttctggaaaacctgaacttcggtttcaaatctaaacgtaccggtatcgcggaaaaagcggtttaccagcagttcgaaaaaatgctgatcgacaaactgaactgcctggttctgaaagactacccggcggaaaaagttggtggtgttctgaacccgtaccagctgaccgaccagttcacctctttcgcgaaaatgggtacccagtctggtttcctgttctacgttccggcgccgtacacctctaaaatcgacccgctgaccggtttcgttgacccgttcgtttggaaaaccatcaaaaaccacgaatctcgtaaacacttcctggaaggtttcgacttcctgcactacgacgttaaaaccggtgacttcatcctgcacttcaaaatgaaccgtaacctgtctttccagcgtggtctgccgggtttcatgccggcgtgggacatcgttttcgaaaaaaacgaaacccagttcgacgcgaaaggtaccccgttcatcgcgggtaaacgtatcgttccggttatcgaaaaccaccgtttcaccggtcgttaccgtgacctgtacccggcgaacgaactgatcgcgctgctggaagaaaaaggtatcgttttccgtgacggttctaacatcctgccgaaactgctggaaaacgacgactctcacgcgatcgacaccatggttgcgctgatccgttctgttctgcagatgcgtaactctaacgcggcgaccggtgaagactacatcaactctccggttcgtgacctgaacggtgtttgcttcgactctcgtttccagaacccggaatggccgatggacgcggacgcgaacggtgcgtaccacatcgcgctgaaaggtcagctgctgctgaaccacctgaaagaatctaaagacctgaaactgcagaacggtatctctaaccaggactggctggcgtacatccaggaactgcgtaactagaaatcatccttagcgaaagctaaggattttttttatctgaaatgtagggagaccctcaggttaaatattcactcaggaagttattactcaggaagcaaagaggattaca

SEQ ID NO: 73 - DNA, 3922 bp, Artificial Sequence
  Description of Artificial Sequence: Synthetic polynucleotide
aatcaggagagcgttttcaatcctacctctggcgcagttgatatgtcaaacaggttgccgtcactgcgtcttttactggctcttctcgctaaccaaaccggtaaccccgcttattaaaagcattctgtaacaaagcgggaccaaagccatgacaaaaacgcgtaacaaaagtgtctataatcacggcagaaaagtccacattgattatttgcacggcgtcacactttgctatgccatagcatttttatccataagattagcggatcctacctgacgctttttatcgcaactctctactgtttctccatacccgtttttttgggctagcagtaatacgactcactataggggtctcatctcgtgtgagataggcggagatacgaactttaagaggaggatataccatgcaccatcatcatcaccatgcggttaaatctatcaaagttaaactgcgtctggacgacatgccggaaatccgtgcgggtctgtggaaactgcacaaagaagttaacgcgggtgttcgttactacaccgaatggctgtctctgctgcgtcaggaaaacctgtaccgtcgttctccgaacggtgacggtgaacaggaatgcgacaaaaccgcggaagaatgcaaagcggaactgctggaacgtctgcgtgcgcgtcaggttgaaaacggtcaccgtggtccggcgggttctgacgacgaactgctgcagctggcgcgtcagctgtacgaactgctggttccgcaggcgatcggtgcgaaaggtgacgcgcagcagatcgcgcgtaaattcctgtctccgctggcggacaaagacgcggttggtggtctgggtatcgcgaaagcgggtaacaaaccgcgttgggttcgtatgcgtgaagcgggtgaaccgggttgggaagaagaaaaagaaaaagcggaaacccgtaaatctgcggaccgtaccgcggacgttctgcgtgcgctggcggacttcggtctgaaaccgctgatgcgtgtttacaccgactctgaaatgtcttctgttgaatggaaaccgctgcgtaaaggtcaggcggttcgtacctgggaccgtgacatgttccagcaggcgatcgaacgtatgatgtcttgggaatcttggaaccagcgtgttggtcaggaatacgcgaaactggttgaacagaaaaaccgtttcgaacagaaaaacttcgttggtcaggaacacctggttcacctggttaaccagctgcagcaggacatgaaagaagcgtctccgggtctggaatctaaagaacagaccgcgcactacgttaccggtcgtgcgctgcgtggttctgacaaagttttcgaaaaatggggtaaactggcgccggacgcgccgttcgacctgtacgacgcggaaatcaaaaacgttcagcgtcgtaacacccgtcgtttcggttctcacgacctgttcgcgaaactggcggaaccggaataccaggcgctgtggcgtgaagacgcgtctttcctgacccgttacgcggtttacaactctatcctgcgtaaactgaaccacgcgaaaatgttcgcgaccttcaccctgccggacgcgaccgcgcacccgatctggacccgtttcgacaaactgggtggtaacctgcaccagtacaccttcctgttcaacgaattcggtgaacgtcgtcacgcgatccgtttccacaaactgctgaaagttgaaaacggtgttgcgcgtgaagttgacgacgttaccgttccgatctctatgtctgaacagctggacaacctgctgccgcgtgacccgaacgaaccgatcgcgctgtacttccgtgactacggtgcggaacagcacttcaccggtgaattcggtggtgcgaaaatccagtgccgtcgtgaccagctggcgcacatgcaccgtcgtcgtggtgcgcgtgacgtttacctgaacgtttctgttcgtgttcagtctcagtctgaagcgcgtggtgaacgtcgtccgccgtacgcggcggttttccgtctggttggtgacaaccaccgtgcgttcgttcacttcgacaaactgtctgactacctggcggaacacccggacgacggtaaactgggttctgaaggtctgctgtctggtctgcgtgttatgtctgttgacctgggtctgcgtacctctgcgtctatctctgttttccgtgttgcgcgtaaagacgaactgaaaccgaactctaaaggtcgtgttccgttcttcttcccgatcaaaggtaacgacaacctggttgcggttcacgaacgttctcagctgctgaaactgccgggtgaaaccgaatctaaagacctgcgtgcgatccgtgaagaacgtcagcgtaccctgcgtcagctgcgtacccagctggcgtacctgcgtctgctggttcgttgcggttctgaagacgttggtcgtcgtgaacgttcttgggcgaaactgatcgaacagccggttgacgcggcgaaccacatgaccccggactggcgtgaagcgttcgaaaacgaactgcagaaactgaaatctctgcacggtatctgctctgacaaagaatggatggacgcggtttacgaatctgttcgtcgtgtttggcgtcacatgggtaaacaggttcgtgactggcgtaaagacgttcgttctggtgaacgtccgaaaatccgtggttacgcgaaagacgttgttggtggtaactctatcgaacagatcgaatacctggaacgtcagtacaaattcctgaaatcttggtctttcttcggtaaagtttctggtcaggttatccgtgcggaaaaaggttctcgtttcgcgatcaccctgcgtgaacacatcgaccacgcgaaagaagaccgtctgaaaaaactggcggaccgtatcatcatggaagcgctgggttacgtttacgcgctggacgaacgtggtaaaggtaaatgggttgcgaaatacccgccgtgccagctgatcctgctggaagaactgtctgaataccagttcaacaacgaccgtccgccgtctgaaaacaaccagctgatgcagtggtctcaccgtggtgttttccaggaactgatcaaccaggcgcaggttcacgacctgctggttggtaccatgtacgcggcgttctcttctcgtttcgacgcgcgtaccggtgcgccgggtatccgttgccgtcgtgttccggcgcgttgcacccaggaacacaacccggaaccgttcccgtggtggctgaacaaattcgttgttgaacacaccctggacgcgtgcccgctgcgtgcggacgacctgatcccgaccggtgaaggtgaaatcttcgtttctccgttctctgcggaagaaggtgacttccaccagatccacgcggacctgaacgcggcgcagaacctgcagcagcgtctgtggtctgacttcgacatctctcagatccgtctgcgttgcgactggggtgaagttgacggtgaactggttctgatcccgcgtctgaccggtaaacgtaccgcggactcttactctaacaaagttttctacaccaacaccggtgttacctactacgaacgtgaacgtggtaaaaaacgtcgtaaagttttcgcgcaggaaaaactgtctgaagaagaagcggaactgctggttgaagcggacgaagcgcgtgaaaaatctgttgttctgatgcgtgacccgtctggtatcatcaaccgtggtaactggacccgtcagaaagaattctggtctatggttaaccagcgtatcgaaggttacctggttaaacagatccgttctcgtgttccgctgcaggactctgcgtgcgaaaacaccggtgacatctaagaaatcatccttagcgaaagctaaggattttttttatctgaaatgtagggagaccctcaggttaaatattcactcaggaagttattactcaggaagcaaagaggattaca

SEQ ID NO: 74 - DNA, 3859 bp, Artificial Sequence
  Description of Artificial Sequence: Synthetic polynucleotide
aatcaggagagcgttttcaatcctacctctggcgcagttgatatgtcaaacaggttgccgtcactgcgtcttttactggctcttctcgctaaccaaaccggtaaccccgcttattaaaagcattctgtaacaaagcgggaccaaagccatgacaaaaacgcgtaacaaaagtgtctataatcacggcagaaaagtccacattgattatttgcacggcgtcacactttgctatgccatagcatttttatccataagattagcggatcctacctgacgctttttatcgcaactctctactgtttctccatacccgtttttttgggctagcagtaatacgactcactataggggtctcatctcgtgtgagataggcggagatacgaactttaagaggaggatataccatgcaccatcatcatcaccatgcgacccgttctttcatcctgaaaatcgaaccgaacgaagaagttaaaaaaggtctgtggaaaacccacgaagttctgaaccacggtatcgcgtactacatgaacatcctgaaactgatccgtcaggaagcgatctacgaacaccacgaacaggacccgaaaaacccgaaaaaagtttctaaagcggaaatccaggcggaactgtgggacttcgttctgaaaatgcagaaatgcaactctttcacccacgaagttgacaaagacgttgttttcaacatcctgcgtgaactgtacgaagaactggttccgtcttctgttgaaaaaaaaggtgaagcgaaccagctgtctaacaaattcctgtacccgctggttgacccgaactctcagtctggtaaaggtaccgcgtcttctggtcgtaaaccgcgttggtacaacctgaaaatcgcgggtgacccgtcttgggaagaagaaaaaaaaaaatgggaagaagacaaaaaaaaagacccgctggcgaaaatcctgggtaaactggcggaatacggtctgatcccgctgttcatcccgttcaccgactctaacgaaccgatcgttaaagaaatcaaatggatggaaaaatctcgtaaccagtctgttcgtcgtctggacaaagacatgttcatccaggcgctggaacgtttcctgtcttgggaatcttggaacctgaaagttaaagaagaatacgaaaaagttgaaaaagaacacaaaaccctggaagaacgtatcaaagaagacatccaggcgttcaaatctctggaacagtacgaaaaagaacgtcaggaacagctgctgcgtgacaccctgaacaccaacgaataccgtctgtctaaacgtggtctgcgtggttggcgtgaaatcatccagaaatggctgaaaatggacgaaaacgaaccgtctgaaaaatacctggaagttttcaaagactaccagcgtaaacacccgcgtgaagcgggtgactactctgtttacgaattcctgtctaaaaaagaaaaccacttcatctggcgtaaccacccggaatacccgtacctgtacgcgaccttctgcgaaatcgacaaaaaaaaaaaagacgcgaaacagcaggcgaccttcaccctggcggacccgatcaaccacccgctgtgggttcgtttcgaagaacgttctggttctaacctgaacaaataccgtatcctgaccgaacagctgcacaccgaaaaactgaaaaaaaaactgaccgttcagctggaccgtctgatctacccgaccgaatctggtggttgggaagaaaaaggtaaagttgacatcgttctgctgccgtctcgtcagttctacaaccagatcttcctggacatcgaagaaaaaggtaaacacgcgttcacctacaaagacgaatctatcaaattcccgctgaaaggtaccctgggtggtgcgcgtgttcagttcgaccgtgaccacctgcgtcgttacccgcacaaagttgaatctggtaacgttggtcgtatctacttcaacatgaccgttaacatcgaaccgaccgaatctccggtttctaaatctctgaaaatccaccgtgacgacttcccgaaattcgttaacttcaaaccgaaagaactgaccgaatggatcaaagactctaaaggtaaaaaactgaaatctggtatcgaatctctggaaatcggtctgcgtgttatgtctatcgacctgggtcagcgtcaggcggcggcggcgtctatcttcgaagttgttgaccagaaaccggacatcgaaggtaaactgttcttcccgatcaaaggtaccgaactgtacgcggttcaccgtgcgtctttcaacatcaaactgccgggtgaaaccctggttaaatctcgtgaagttctgcgtaaagcgcgtgaagacaacctgaaactgatgaaccagaaactgaacttcctgcgtaacgttctgcacttccagcagttcgaagacatcaccgaacgtgaaaaacgtgttaccaaatggatctctcgtcaggaaaactctgacgttccgctggtttaccaggacgaactgatccagatccgtgaactgatgtacaaaccgtacaaagactgggttgcgttcctgaaacagctgcacaaacgtctggaagttgaaatcggtaaagaagttaaacactggcgtaaatctctgtctgacggtcgtaaaggtctgtacggtatctctctgaaaaacatcgacgaaatcgaccgtacccgtaaattcctgctgcgttggtctctgcgtccgaccgaaccgggtgaagttcgtcgtctggaaccgggtcagcgtttcgcgatcgaccagctgaaccacctgaacgcgctgaaagaagaccgtctgaaaaaaatggcgaacaccatcatcatgcacgcgctgggttactgctacgacgttcgtaaaaaaaaatggcaggcgaaaaacccggcgtgccagatcatcctgttcgaagacctgtctaactacaacccgtacgaagaacgttctcgtttcgaaaactctaaactgatgaaatggtctcgtcgtgaaatcccgcgtcaggttgcgctgcagggtgaaatctacggtctgcaggttggtgaagttggtgcgcagttctcttctcgtttccacgcgaaaaccggttctccgggtatccgttgctctgttgttaccaaagaaaaactgcaggacaaccgtttcttcaaaaacctgcagcgtgaaggtcgtctgaccctggacaaaatcgcggttctgaaagaaggtgacctgtacccggacaaaggtggtgaaaaattcatctctctgtctaaagaccgtaaactggttaccacccacgcggacatcaacgcggcgcagaacctgcagaaacgtttctggacccgtacccacggtttctacaaagtttactgcaaagcgtaccaggttgacggtcagaccgtttacatcccggaatctaaagaccagaaacagaaaatcatcgaagaattcggtgaaggttacttcatcctgaaagacggtgtttacgaatggggtaacgcgggtaaactgaaaatcaaaaaaggttcttctaaacagtcttcttctgaactggttgactctgacatcctgaaagactctttcgacctggcgtctgaactgaaaggtgaaaaactgatgctgtaccgtgacccgtctggtaacgttttcccgtctgacaaatggatggcggcgggtgttttcttcggtaaactggaacgtatcctgatctctaaactgaccaaccagtactctatctctaccatcgaagacgactcttctaaacagtctatgtaagaaatcatccttagcgaaagctaaggattttttttatctgaaatgtagggagaccctcaggttaaatattcactcaggaagttattactcaggaagcaaagaggattaca

SEQ ID NO: 75 - DNA, 3982 bp, Artificial Sequence
  Description of Artificial Sequence: Synthetic polynucleotide
aatcaggagagcgttttcaatcctacctctggcgcagttgatatgtcaaacaggttgccgtcactgcgtcttttactggctcttctcgctaaccaaaccggtaaccccgcttattaaaagcattctgtaacaaagcgggaccaaagccatgacaaaaacgcgtaacaaaagtgtctataatcacggcagaaaagtccacattgattatttgcacggcgtcacactttgctatgccatagcatttttatccataagattagcggatcctacctgacgctttttatcgcaactctctactgtttctccatacccgtttttttgggctagcagtaatacgactcactataggggtctcatctcgtgtgagataggcggagatacgaactttaagaggaggatataccatgcaccatcatcatcaccatccgacccgtaccatcaacctgaaactggttctgggtaaaaacccggaaaacgcgaccctgcgtcgtgcgctgttctctacccaccgtctggttaaccaggcgaccaaacgtatcgaagaattcctgctgctgtgccgtggtgaagcgtaccgtaccgttgacaacgaaggtaaagaagcggaaatcccgcgtcacgcggttcaggaagaagcgctggcgttcgcgaaagcggcgcagcgtcacaacggttgcatctctacctacgaagaccaggaaatcctggacgttctgcgtcagctgtacgaacgtctggttccgtctgttaacgaaaacaacgaagcgggtgacgcgcaggcggcgaacgcgtgggtttctccgctgatgtctgcggaatctgaaggtggtctgtctgtttacgacaaagttctggacccgccgccggtttggatgaaactgaaagaagaaaaagcgccgggttgggaagcggcgtctcagatctggatccagtctgacgaaggtcagtctctgctgaacaaaccgggttctccgccgcgttggatccgtaaactgcgttctggtcagccgtggcaggacgacttcgtttctgaccagaaaaaaaaacaggacgaactgaccaaaggtaacgcgccgctgatcaaacagctgaaagaaatgggtctgctgccgctggttaacccgttcttccgtcacctgctggacccggaaggtaaaggtgtttctccgtgggaccgtctggcggttcgtgcggcggttgcgcacttcatctcttgggaatcttggaaccaccgtacccgtgcggaatacaactctctgaaactgcgtcgtgacgaattcgaagcggcgtctgacgaattcaaagacgacttcaccctgctgcgtcagtacgaagcgaaacgtcactctaccctgaaatctatcgcgctggcggacgactctaacccgtaccgtatcggtgttcgttctctgcgtgcgtggaaccgtgttcgtgaagaatggatcgacaaaggtgcgaccgaagaacagcgtgttaccatcctgtctaaactgcagacccagctgcgtggtaaattcggtgacccggacctgttcaactggctggcgcaggaccgtcacgttcacctgtggtctccgcgtgactctgttaccccgctggttcgtatcaacgcggttgacaaagttctgcgtcgtcgtaaaccgtacgcgctgatgaccttcgcgcacccgcgtttccacccgcgttggatcctgtacgaagcgccgggtggttctaacctgcgtcagtacgcgctggactgcaccgaaaacgcgctgcacatcaccctgccgctgctggttgacgacgcgcacggtacctggatcgaaaaaaaaatccgtgttccgctggcgccgtctggtcagatccaggacctgaccctggaaaaactggaaaaaaaaaaaaaccgtctgtactaccgttctggtttccagcagttcgcgggtctggcgggtggtgcggaagttctgttccaccgtccgtacatggaacacgacgaacgttctgaagaatctctgctggaacgtccgggtgcggtttggttcaaactgaccctggacgttgcgacccaggcgccgccgaactggctggacggtaaaggtcgtgttcgtaccccgccggaagttcaccacttcaaaaccgcgctgtctaacaaatctaaacacacccgtaccctgcagccgggtctgcgtgttctgtctgttgacctgggtatgcgtaccttcgcgtcttgctctgttttcgaactgatcgaaggtaaaccggaaaccggtcgtgcgttcccggttgcggacgaacgttctatggactctccgaacaaactgtgggcgaaacacgaacgttctttcaaactgaccctgccgggtgaaaccccgtctcgtaaagaagaagaagaacgttctatcgcgcgtgcggaaatctacgcgctgaaacgtgacatccagcgtctgaaatctctgctgcgtctgggtgaagaagacaacgacaaccgtcgtgacgcgctgctggaacagttcttcaaaggttggggtgaagaagacgttgttccgggtcaggcgttcccgcgttctctgttccagggtctgggtgcggcgccgttccgttctaccccggaactgtggcgtcagcactgccagacctactacgacaaagcggaagcgtgcctggcgaaacacatctctgactggcgtaaacgtacccgtccgcgtccgacctctcgtgaaatgtggtacaaaacccgttcttaccacggtggtaaatctatctggatgctggaatacctggacgcggttcgtaaactgctgctgtcttggtctctgcgtggtcgtacctacggtgcgatcaaccgtcaggacaccgcgcgtttcggttctctggcgtctcgtctgctgcaccacatcaactctctgaaagaagaccgtatcaaaaccggtgcggactctatcgttcaggcggcgcgtggttacatcccgctgccgcacggtaaaggttgggaacagcgttacgaaccgtgccagctgatcctgttcgaagacctggcgcgttaccgtttccgtgttgaccgtccgcgtcgtgaaaactctcagctgatgcagtggaaccaccgtgcgatcgttgcggaaaccaccatgcaggcggaactgtacggtcagatcgttgaaaacaccgcggcgggtttctcttctcgtttccacgcggcgaccggtgcgccgggtgttcgttgccgtttcctgctggaacgtgacttcgacaacgacctgccgaaaccgtacctgctgcgtgaactgtcttggatgctgggtaacaccaaagttgaatctgaagaagaaaaactgcgtctgctgtctgaaaaaatccgtccgggttctctggttccgtgggacggtggtgaacagttcgcgaccctgcacccgaaacgtcagaccctgtgcgttatccacgcggacatgaacgcggcgcagaacctgcagcgtcgtttcttcggtcgttgcggtgaagcgttccgtctggtttgccagccgcacggtgacgacgttctgcgtctggcgtctaccccgggtgcgcgtctgctgggtgcgctgcagcagctggaaaacggtcagggtgcgttcgaactggttcgtgacatgggttctacctctcagatgaaccgtttcgttatgaaatctctgggtaaaaaaaaaatcaaaccgctgcaggacaacaacggtgacgacgaactggaagacgttctgtctgttctgccggaagaagacgacaccggtcgtatcaccgttttccgtgactcttctggtatcttcttcccgtgcaacgtttggatcccggcgaaacagttctggccggcggttcgtgcgatgatctggaaagttatggcgtctcactctctgggttaagaaatcatccttagcgaaagctaaggattttttttatctgaaatgtagggagaccctcaggttaaatattcactcaggaagttattactcaggaagcaaagaggattaca

SEQ ID NO: 76 - DNA, 4291 bp, Artificial Sequence
  Description of Artificial Sequence: Synthetic polynucleotide
aatcaggagagcgttttcaatcctacctctggcgcagttgatatgtcaaacaggttgccgtcactgcgtcttttactggctcttctcgctaaccaaaccggtaaccccgcttattaaaagcattctgtaacaaagcgggaccaaagccatgacaaaaacgcgtaacaaaagtgtctataatcacggcagaaaagtccacattgattatttgcacggcgtcacactttgctatgccatagcatttttatccataagattagcggatcctacctgacgctttttatcgcaactctctactgtttctccatacccgtttttttgggctagcagtaatacgactcactataggggtctcatctcgtgtgagataggcggagatacgaactttaagaggaggatataccatgcaccatcatcatcaccataccaaactgcgtcaccgtcagaaaaaactgacccacgactgggcgggttctaaaaaacgtgaagttctgggttctaacggtaaactgcagaacccgctgctgatgccggttaaaaaaggtcaggttaccgaattccgtaaagcgttctctgcgtacgcgcgtgcgaccaaaggtgaaatgaccgacggtcgtaaaaacatgttcacccactctttcgaaccgttcaaaaccaaaccgtctctgcaccagtgcgaactggcggacaaagcgtaccagtctctgcactcttacctgccgggttctctggcgcacttcctgctgtctgcgcacgcgctgggtttccgtatcttctctaaatctggtgaagcgaccgcgttccaggcgtcttctaaaatcgaagcgtacgaatctaaactggcgtctgaactggcgtgcgttgacctgtctatccagaacctgaccatctctaccctgttcaacgcgctgaccacctctgttcgtggtaaaggtgaagaaacctctgcggacccgctgatcgcgcgtttctacaccctgctgaccggtaaaccgctgtctcgtgacacccagggtccggaacgtgacctggcggaagttatctctcgtaaaatcgcgtcttctttcggtacctggaaagaaatgaccgcgaacccgctgcagtctctgcagttcttcgaagaagaactgcacgcgctggacgcgaacgtttctctgtctccggcgttcgacgttctgatcaaaatgaacgacctgcagggtgacctgaaaaaccgtaccatcgttttcgacccggacgcgccggttttcgaatacaacgcggaagacccggcggacatcatcatcaaactgaccgcgcgttacgcgaaagaagcggttatcaaaaaccagaacgttggtaactacgttaaaaacgcgatcaccaccaccaacgcgaacggtctgggttggctgctgaacaaaggtctgtctctgctgccggtttctaccgacgacgaactgctggaattcatcggtgttgaacgttctcacccgtcttgccacgcgctgatcgaactgatcgcgcagctggaagcgccggaactgttcgaaaaaaacgttttctctgacacccgttctgaagttcagggtatgatcgactctgcggtttctaaccacatcgcgcgtctgtcttcttctcgtaactctctgtctatggactctgaagaactggaacgtctgatcaaatctttccagatccacaccccgcactgctctctgttcatcggtgcgcagtctctgtctcagcagctggaatctctgccggaagcgctgcagtctggtgttaactctgcggacatcctgctgggttctacccagtacatgctgaccaactctctggttgaagaatctatcgcgacctaccagcgtaccctgaaccgtatcaactacctgtctggtgttgcgggtcagatcaacggtgcgatcaaacgtaaagcgatcgacggtgaaaaaatccacctgccggcggcgtggtctgaactgatctctctgccgttcatcggtcagccggttatcgacgttgaatctgacctggcgcacctgaaaaaccagtaccagaccctgtctaacgaattcgacaccctgatctctgcgctgcagaaaaacttcgacctgaacttcaacaaagcgctgctgaaccgtacccagcacttcgaagcgatgtgccgttctaccaaaaaaaacgcgctgtctaaaccggaaatcgtttcttaccgtgacctgctggcgcgtctgacctcttgcctgtaccgtggttctctggttctgcgtcgtgcgggtatcgaagttctgaaaaaacacaaaatcttcgaatctaactctgaactgcgtgaacacgttcacgaacgtaaacacttcgttttcgtttctccgctggaccgtaaagcgaaaaaactgctgcgtctgaccgactctcgtccggacctgctgcacgttatcgacgaaatcctgcagcacgacaacctggaaaacaaagaccgtgaatctctgtggctggttcgttctggttacctgctggcgggtctgccggaccagctgtcttcttctttcatcaacctgccgatcatcacccagaaaggtgaccgtcgtctgatcgacctgatccagtacgaccagatcaaccgtgacgcgttcgttatgctggttacctctgcgttcaaatctaacctgtctggtctgcagtaccgtgcgaacaaacagtctttcgttgttacccgtaccctgtctccgtacctgggttctaaactggtttacgttccgaaagacaaagactggctggttccgtctcagatgttcgaaggtcgtttcgcggacatcctgcagtctgactacatggtttggaaagacgcgggtcgtctgtgcgttatcgacaccgcgaaacacctgtctaacatcaaaaaatctgttttctcttctgaagaagttctggcgttcctgcgtgaactgccgcaccgtaccttcatccagaccgaagttcgtggtctgggtgttaacgttgacggtatcgcgttcaacaacggtgacatcccgtctctgaaaaccttctctaactgcgttcaggttaaagtttctcgtaccaacacctctctggttcagaccctgaaccgttggttcgaaggtggtaaagtttctccgccgtctatccagttcgaacgtgcgtactacaaaaaagacgaccagatccacgaagacgcggcgaaacgtaaaatccgtttccagatgccggcgaccgaactggttcacgcgtctgacgacgcgggttggaccccgtcttacctgctgggtatcgacccgggtgaatacggtatgggtctgtctctggtttctatcaacaacggtgaagttctggactctggtttcatccacatcaactctctgatcaacttcgcgtctaaaaaatctaaccaccagaccaaagttgttccgcgtcagcagtacaaatctccgtacgcgaactacctggaacagtctaaagactctgcggcgggtgacatcgcgcacatcctggaccgtctgatctacaaactgaacgcgctgccggttttcgaagcgctgtctggtaactctcagtctgcggcggaccaggtttggaccaaagttctgtctttctacacctggggtgacaacgacgcgcagaactctatccgtaaacagcactggttcggtgcgtctcactgggacatcaaaggtatgctgcgtcagccgccgaccgaaaaaaaaccgaaaccgtacatcgcgttcccgggttctcaggtttcttcttacggtaactctcagcgttgctcttgctgcggtcgtaacccgatcgaacagctgcgtgaaatggcgaaagacacctctatcaaagaactgaaaatccgtaactctgaaatccagctgttcgacggtaccatcaaactgttcaacccggacccgtctaccgttatcgaacgtcgtcgtcacaacctgggtccgtctcgtatcccggttgcggaccgtaccttcaaaaacatctctccgtcttctctggaattcaaagaactgatcaccatcgtttctcgttctatccgtcactctccggaattcatcgcgaaaaaacgtggtatcggttctgaatacttctgcgcgtactctgactgcaactcttctctgaactctgaagcgaacgcggcggcgaacgttgcgcagaaattccagaaacagctgttcttcgaactgtaagaaatcatccttagcgaaagctaaggattttttttatctgaaatgtagggagaccctcaggttaaatattcactcaggaagttattactcaggaagcaaagaggattaca

SEQ ID NO: 77 - DNA, 4396 bp, Artificial Sequence
  Description of Artificial Sequence: Synthetic polynucleotide
aatcaggagagcgttttcaatcctacctctggcgcagttgatatgtcaaacaggttgccgtcactgcgtcttttactggctcttctcgctaaccaaaccggtaaccccgcttattaaaagcattctgtaacaaagcgggaccaaagccatgacaaaaacgcgtaacaaaagtgtctataatcacggcagaaaagtccacattgattatttgcacggcgtcacactttgctatgccatagcatttttatccataagattagcggatcctacctgacgctttttatcgcaactctctactgtttctccatacccgtttttttgggctagcagtaatacgactcactataggggtctcatctcgtgtgagataggcggagatacgaactttaagaggaggatataccatgcaccatcatcatcaccataaacgtatcctgaactctctgaaagttgcggcgctgcgtctgctgttccgtggtaaaggttctgaactggttaaaaccgttaaatacccgctggtttctccggttcagggtgcggttgaagaactggcggaagcgatccgtcacgacaacctgcacctgttcggtcagaaagaaatcgttgacctgatggaaaaagacgaaggtacccaggtttactctgttgttgacttctggctggacaccctgcgtctgggtatgttcttctctccgtctgcgaacgcgctgaaaatcaccctgggtaaattcaactctgaccaggtttctccgttccgtaaagttctggaacagtctccgttcttcctggcgggtcgtctgaaagttgaaccggcggaacgtatcctgtctgttgaaatccgtaaaatcggtaaacgtgaaaaccgtgttgaaaactacgcggcggacgttgaaacctgcttcatcggtcagctgtcttctgacgaaaaacagtctatccagaaactggcgaacgacatctgggactctaaagaccacgaagaacagcgtatgctgaaagcggacttcttcgcgatcccgctgatcaaagacccgaaagcggttaccgaagaagacccggaaaacgaaaccgcgggtaaacagaaaccgctggaactgtgcgtttgcctggttccggaactgtacacccgtggtttcggttctatcgcggacttcctggttcagcgtctgaccctgctgcgtgacaaaatgtctaccgacaccgcggaagactgcctggaatacgttggtatcgaagaagaaaaaggtaacggtatgaactctctgctgggtaccttcctgaaaaacctgcagggtgacggtttcgaacagatcttccagttcatgctgggttcttacgttggttggcagggtaaagaagacgttctgcgtgaacgtctggacctgctggcggaaaaagttaaacgtctgccgaaaccgaaattcgcgggtgaatggtctggtcaccgtatgttcctgcacggtcagctgaaatcttggtcttctaacttcttccgtctgttcaacgaaacccgtgaactgctggaatctatcaaatctgacatccagcacgcgaccatgctgatctcttacgttgaagaaaaaggtggttaccacccgcagctgctgtctcagtaccgtaaactgatggaacagctgccggcgctgcgtaccaaagttctggacccggaaatcgaaatgacccacatgtctgaagcggttcgttcttacatcatgatccacaaatctgttgcgggtttcctgccggacctgctggaatctctggaccgtgacaaagaccgtgaattcctgctgtctatcttcccgcgtatcccgaaaatcgacaaaaaaaccaaagaaatcgttgcgtgggaactgccgggtgaaccggaagaaggttacctgttcaccgcgaacaacctgttccgtaacttcctggaaaacccgaaacacgttccgcgtttcatggcggaacgtatcccggaagactggacccgtctgcgttctgcgccggtttggttcgacggtatggttaaacagtggcagaaagttgttaaccagctggttgaatctccgggtgcgctgtaccagttcaacgaatctttcctgcgtcagcgtctgcaggcgatgctgaccgtttacaaacgtgacctgcagaccgaaaaattcctgaaactgctggcggacgtttgccgtccgctggttgacttcttcggtctgggtggtaacgacatcatcttcaaatcttgccaggacccgcgtaaacagtggcagaccgttatcccgctgtctgttccggcggacgtttacaccgcgtgcgaaggtctggcgatccgtctgcgtgaaaccctgggtttcgaatggaaaaacctgaaaggtcacgaacgtgaagacttcctgcgtctgcaccagctgctgggtaacctgctgttctggatccgtgacgcgaaactggttgttaaactggaagactggatgaacaacccgtgcgttcaggaatacgttgaagcgcgtaaagcgatcgacctgccgctggaaatcttcggtttcgaagttccgatcttcctgaacggttacctgttctctgaactgcgtcagctggaactgctgctgcgtcgtaaatctgttatgacctcttactctgttaaaaccaccggttctccgaaccgtctgttccagctggtttacctgccgctgaacccgtctgacccggaaaaaaaaaactctaacaacttccaggaacgtctggacaccccgaccggtctgtctcgtcgtttcctggacctgaccctggacgcgttcgcgggtaaactgctgaccgacccggttacccaggaactgaaaaccatggcgggtttctacgaccacctgttcggtttcaaactgccgtgcaaactggcggcgatgtctaaccacccgggttcttcttctaaaatggttgttctggcgaaaccgaaaaaaggtgttgcgtctaacatcggtttcgaaccgatcccggacccggcgcacccggttttccgtgttcgttcttcttggccggaactgaaatacctggaaggtctgctgtacctgccggaagacaccccgctgaccatcgaactggcggaaacctctgtttcttgccagtctgtttcttctgttgcgttcgacctgaaaaacctgaccaccatcctgggtcgtgttggtgaattccgtgttaccgcggaccagccgttcaaactgaccccgatcatcccggaaaaagaagaatctttcatcggtaaaacctacctgggtctggacgcgggtgaacgttctggtgttggtttcgcgatcgttaccgttgacggtgacggttacgaagttcagcgtctgggtgttcacgaagacacccagctgatggcgctgcagcaggttgcgtctaaatctctgaaagaaccggttttccagccgctgcgtaaaggtaccttccgtcagcaggaacgtatccgtaaatctctgcgtggttgctactggaacttctaccacgcgctgatgatcaaataccgtgcgaaagttgttcacgaagaatctgttggttcttctggtctggttggtcagtggctgcgtgcgttccagaaagacctgaaaaaagcggacgttctgccgaaaaaaggtggtaaaaacggtgttgacaaaaaaaaacgtgaatcttctgcgcaggacaccctgtggggtggtgcgttctctaaaaaagaagaacagcagatcgcgttcgaagttcaggcggcgggttcttctcagttctgcctgaaatgcggttggtggttccagctgggtatgcgtgaagttaaccgtgttcaggaatctggtgttgttctggactggaaccgttctatcgttaccttcctgatcgaatcttctggtgaaaaagtttacggtttctctccgcagcagctggaaaaaggtttccgtccggacatcgaaaccttcaaaaaaatggttcgtgacttcatgcgtccgccgatgttcgaccgtaaaggtcgtccggcggcggcgtacgaacgtttcgttctgggtcgtcgtcaccgtcgttaccgtttcgacaaagttttcgaagaacgtttcggtcgttctgcgctgttcatctgcccgcgtgttggttgcggtaacttcgaccactcttctgaacagtctgcggttgttctggcgctgatcggttacatcgcggacaaagaaggtatgtctggtaaaaaactggtttacgttcgtctggcggaactgatggcggaatggaaactgaaaaaactggaacgttctcgtgttgaagaacagtcttctgcgcagtaagaaatcatccttagcgaaagctaaggattttttttatctgaaatgtagggagaccctcaggttaaatattcactcaggaagttattactcaggaagcaaagaggattaca

SEQ ID NO: 78 - DNA, 4111 bp, Artificial Sequence
  Description of Artificial Sequence: Synthetic polynucleotide
aatcaggagagcgttttcaatcctacctctggcgcagttgatatgtcaaacaggttgccgtcactgcgtcttttactggctcttctcgctaaccaaaccggtaaccccgcttattaaaagcattctgtaacaaagcgggaccaaagccatgacaaaaacgcgtaacaaaagtgtctataatcacggcagaaaagtccacattgattatttgcacggcgtcacactttgctatgccatagcatttttatccataagattagcggatcctacctgacgctttttatcgcaactctctactgtttctccatacccgtttttttgggctagcagtaatacgactcactataggggtctcatctcgtgtgagataggcggagatacgaactttaagaggaggatataccatgcaccatcatcatcaccatgcggaatctaaacagatgcagtgccgtaaatgcggtgcgtctatgaaatacgaagttatcggtctgggtaaaaaatcttgccgttacatgtgcccggactgcggtaaccacacctctgcgcgtaaaatccagaacaaaaaaaaacgtgacaaaaaatacggttctgcgtctaaagcgcagtctcagcgtatcgcggttgcgggtgcgctgtacccggacaaaaaagttcagaccatcaaaacctacaaatacccggcggacctgaacggtgaagttcacgactctggtgttgcggaaaaaatcgcgcaggcgatccaggaagacgaaatcggtctgctgggtccgtcttctgaatacgcgtgctggatcgcgtctcagaaacagtctgaaccgtactctgttgttgacttctggttcgacgcggtttgcgcgggtggtgttttcgcgtactctggtgcgcgtctgctgtctaccgttctgcagctgtctggtgaagaatctgttctgcgtgcggcgctggcgtcttctccgttcgttgacgacatcaacctggcgcaggcggaaaaattcctggcggtttctcgtcgtaccggtcaggacaaactgggtaaacgtatcggtgaatgcttcgcggaaggtcgtctggaagcgctgggtatcaaagaccgtatgcgtgaattcgttcaggcgatcgacgttgcgcagaccgcgggtcagcgtttcgcggcgaaactgaaaatcttcggtatctctcagatgccggaagcgaaacagtggaacaacgactctggtctgaccgtttgcatcctgccggactactacgttccggaagaaaaccgtgcggaccagctggttgttctgctgcgtcgtctgcgtgaaatcgcgtactgcatgggtatcgaagacgaagcgggtttcgaacacctgggtatcgacccgggtgcgctgtctaacttctctaacggtaacccgaaacgtggtttcctgggtcgtctgctgaacaacgacatcatcgcgctggcgaacaacatgtctgcgatgaccccgtactgggaaggtcgtaaaggtgaactgatcgaacgtctggcgtggctgaaacaccgtgcggaaggtctgtacctgaaagaaccgcacttcggtaactcttgggcggaccaccgttctcgtatcttctctcgtatcgcgggttggctgtctggttgcgcgggtaaactgaaaatcgcgaaagaccagatctctggtgttcgtaccgacctgttcctgctgaaacgtctgctggacgcggttccgcagtctgcgccgtctccggacttcatcgcgtctatctctgcgctggaccgtttcctggaagcggcggaatcttctcaggacccggcggaacaggttcgtgcgctgtacgcgttccacctgaacgcgccggcggttcgttctatcgcgaacaaagcggttcagcgttctgactctcaggaatggctgatcaaagaactggacgcggttgaccacctggaattcaacaaagcgttcccgttcttctctgacaccggtaaaaaaaaaaaaaaaggtgcgaactctaacggtgcgccgtctgaagaagaatacaccgaaaccgaatctatccagcagccggaagacgcggaacaggaagttaacggtcaggaaggtaacggtgcgtctaaaaaccagaaaaaattccagcgtatcccgcgtttcttcggtgaaggttctcgttctgaataccgtatcctgaccgaagcgccgcagtacttcgacatgttctgcaacaacatgcgtgcgatcttcatgcagctggaatctcagccgcgtaaagcgccgcgtgacttcaaatgcttcctgcagaaccgtctgcagaaactgtacaaacagaccttcctgaacgcgcgttctaacaaatgccgtgcgctgctggaatctgttctgatctcttggggtgaattctacacctacggtgcgaacgaaaaaaaattccgtctgcgtcacgaagcgtctgaacgttcttctgacccggactacgttgttcagcaggcgctggaaatcgcgcgtcgtctgttcctgttcggtttcgaatggcgtgactgctctgcgggtgaacgtgttgacctggttgaaatccacaaaaaagcgatctctttcctgctggcgatcacccaggcggaagtttctgttggttcttacaactggctgggtaactctaccgtttctcgttacctgtctgttgcgggtaccgacaccctgtacggtacccagctggaagaattcctgaacgcgaccgttctgtctcagatgcgtggtctggcgatccgtctgtcttctcaggaactgaaagacggtttcgacgttcagctggaatcttcttgccaggacaacctgcagcacctgctggtttaccgtgcgtctcgtgacctggcggcgtgcaaacgtgcgacctgcccggcggaactggacccgaaaatcctggttctgccggttggtgcgttcatcgcgtctgttatgaaaatgatcgaacgtggtgacgaaccgctggcgggtgcgtacctgcgtcaccgtccgcactctttcggttggcagatccgtgttcgtggtgttgcggaagttggtatggaccagggtaccgcgctggcgttccagaaaccgaccgaatctgaaccgttcaaaatcaaaccgttctctgcgcagtacggtccggttctgtggctgaactcttcttcttactctcagtctcagtacctggacggtttcctgtctcagccgaaaaactggtctatgcgtgttctgccgcaggcgggttctgttcgtgttgaacagcgtgttgcgctgatctggaacctgcaggcgggtaaaatgcgtctggaacgttctggtgcgcgtgcgttcttcatgccggttccgttctctttccgtccgtctggttctggtgacgaagcggttctggcgccgaaccgttacctgggtctgttcccgcactctggtggtatcgaatacgcggttgttgacgttctggactctgcgggtttcaaaatcctggaacgtggtaccatcgcggttaacggtttctctcagaaacgtggtgaacgtcaggaagaagcgcaccgtgaaaaacagcgtcgtggtatctctgacatcggtcgtaaaaaaccggttcaggcggaagttgacgcggcgaacgaactgcaccgtaaatacaccgacgttgcgacccgtctgggttgccgtatcgttgttcagtgggcgccgcagccgaaaccgggtaccgcgccgaccgcgcagaccgtttacgcgcgtgcggttcgtaccgaagcgccgcgttctggtaaccaggaagaccacgcgcgtatgaaatcttcttggggttacacctggggtacctactgggaaaaacgtaaaccggaagacatcctgggtatctctacccaggtttactggaccggtggtatcggtgaatcttgcccggcggttgcggttgcgctgctgggtcacatccgtgcgacctctacccagaccgaatgggaaaaagaagaagttgttttcggtcgtctgaaaaaattcttcccgtcttaagaaatcatccttagcgaaagctaaggattttttttatctgaaatgtagggagaccctcaggttaaatattcactcaggaagttattactcaggaagcaaagaggattaca

SEQ ID NO: 79 - DNA, 3493 bp, Artificial Sequence
  Description of Artificial Sequence: Synthetic polynucleotide
aatcaggagagcgttttcaatcctacctctggcgcagttgatatgtcaaacaggttgccgtcactgcgtcttttactggctcttctcgctaaccaaaccggtaaccccgcttattaaaagcattctgtaacaaagcgggaccaaagccatgacaaaaacgcgtaacaaaagtgtctataatcacggcagaaaagtccacattgattatttgcacggcgtcacactttgctatgccatagcatttttatccataagattagcggatcctacctgacgctttttatcgcaactctctactgtttctccatacccgtttttttgggctagcagtaatacgactcactataggggtctcatctcgtgtgagataggcggagatacgaactttaagaggaggatataccatgcaccatcatcatcaccatgaaaaacgtatcaacaaaatccgtaaaaaactgtctgcggacaacgcgaccaaaccggtttctcgttctggtccgatgaaaaccctgctggttcgtgttatgaccgacgacctgaaaaaacgtctggaaaaacgtcgtaaaaaaccggaagttatgccgcaggttatctctaacaacgcggcgaacaacctgcgtatgctgctggacgactacaccaaaatgaaagaagcgatcctgcaggtttactggcaggaattcaaagacgaccacgttggtctgatgtgcaaattcgcgcagccggcgtctaaaaaaatcgaccagaacaaactgaaaccggaaatggacgaaaaaggtaacctgaccaccgcgggtttcgcgtgctctcagtgcggtcagccgctgttcgtttacaaactggaacaggtttctgaaaaaggtaaagcgtacaccaactacttcggtcgttgcaacgttgcggaacacgaaaaactgatcctgctggcgcagctgaaaccggaaaaagactctgacgaagcggttacctactctctgggtaaattcggtcagcgtgcgctggacttctactctatccacgttaccaaagaatctacccacccggttaaaccgctggcgcagatcgcgggtaaccgttacgcgtctggtccggttggtaaagcgctgtctgacgcgtgcatgggtaccatcgcgtctttcctgtctaaataccaggacatcatcatcgaacaccagaaagttgttaaaggtaaccagaaacgtctggaatctctgcgtgaactggcgggtaaagaaaacctggaatacccgtctgttaccctgccgccgcagccgcacaccaaagaaggtgttgacgcgtacaacgaagttatcgcgcgtgttcgtatgtgggttaacctgaacctgtggcagaaactgaaactgtctcgtgacgacgcgaaaccgctgctgcgtctgaaaggtttcccgtctttcccggttgttgaacgtcgtgaaaacgaagttgactggtggaacaccatcaacgaagttaaaaaactgatcgacgcgaaacgtgacatgggtcgtgttttctggtctggtgttaccgcggaaaaacgtaacaccatcctggaaggttacaactacctgccgaacgaaaacgaccacaaaaaacgtgaaggttctctggaaaacccgaaaaaaccggcgaaacgtcagttcggtgacctgctgctgtacctggaaaaaaaatacgcgggtgactggggtaaagttttcgacgaagcgtgggaacgtatcgacaaaaaaatcgcgggtctgacctctcacatcgaacgtgaagaagcgcgtaacgcggaagacgcgcagtctaaagcggttctgaccgactggctgcgtgcgaaagcgtctttcgttctggaacgtctgaaagaaatggacgaaaaagaattctacgcgtgcgaaatccagctgcagaaatggtacggtgacctgcgtggtaacccgttcgcggttgaagcggaaaaccgtgttgttgacatctctggtttctctatcggttctgacggtcactctatccagtaccgtaacctgctggcgtggaaatacctggaaaacggtaaacgtgaattctacctgctgatgaactacggtaaaaaaggtcgtatccgtttcaccgacggtaccgacatcaaaaaatctggtaaatggcagggtctgctgtacggtggtggtaaagcgaaagttatcgacctgaccttcgacccggacgacgaacagctgatcatcctgccgctggcgttcggtacccgtcagggtcgtgaattcatctggaacgacctgctgtctctggaaaccggtctgatcaaactggcgaacggtcgtgttatcgaaaaaaccatctacaacaaaaaaatcggtcgtgacgaaccggcgctgttcgttgcgctgaccttcgaacgtcgtgaagttgttgacccgtctaacatcaaaccggttaacctgatcggtgttgaccgtggtgaaaacatcccggcggttatcgcgctgaccgacccggaaggttgcccgctgccggaattcaaagactcttctggtggtccgaccgacatcctgcgtatcggtgaaggttacaaagaaaaacagcgtgcgatccaggcggcgaaagaagttgaacagcgtcgtgcgggtggttactctcgtaaattcgcgtctaaatctcgtaacctggcggacgacatggttcgtaactctgcgcgtgacctgttctaccacgcggttacccacgacgcggttctggttttcgaaaacctgtctcgtggtttcggtcgtcagggtaaacgtaccttcatgaccgaacgtcagtacaccaaaatggaagactggctgaccgcgaaactggcgtacgaaggtctgacctctaaaacctacctgtctaaaaccctggcgcagtacacctctaaaacctgctctaactgcggtttcaccatcaccaccgcggactacgacggtatgctggttcgtctgaaaaaaacctctgacggttgggcgaccaccctgaacaacaaagaactgaaagcggaaggtcagatcacctactacaaccgttacaaacgtcagaccgttgaaaaagaactgtctgcggaactggaccgtctgtctgaagaatctggtaacaacgacatctctaaatggaccaaaggtcgtcgtgacgaagcgctgttcctgctgaaaaaacgtttctctcaccgtccggttcaggaacagttcgtttgcctggactgcggtcacgaagttcacgcggacgaacaggcggcgctgaacatcgcgcgttcttggctgttcctgaactctaactctaccgaattcaaatcttacaaatctggtaaacagccgttcgttggtgcgtggcaggcgttctacaaacgtcgtctgaaagaagtttggaaaccgaacgcgtaagaaatcatccttagcgaaagctaaggattttttttatctgaaatgtagggagaccctcaggttaaatattcactcaggaagttattactcaggaagcaaagaggattaca

SEQ ID NO: 80 - DNA, 3451 bp, Artificial Sequence
  Description of Artificial Sequence: Synthetic polynucleotide
aatcaggagagcgttttcaatcctacctctggcgcagttgatatgtcaaacaggttgccgtcactgcgtcttttactggctcttctcgctaaccaaaccggtaaccccgcttattaaaagcattctgtaacaaagcgggaccaaagccatgacaaaaacgcgtaacaaaagtgtctataatcacggcagaaaagtccacattgattatttgcacggcgtcacactttgctatgccatagcatttttatccataagattagcggatcctacctgacgctttttatcgcaactctctactgtttctccatacccgtttttttgggctagcagtaatacgactcactataggggtctcatctcgtgtgagataggcggagatacgaactttaagaggaggatataccatgcaccatcatcatcaccataaacgtatcaacaaaatccgtcgtcgtctggttaaagactctaacaccaaaaaagcgggtaaaaccggtccgatgaaaaccctgctggttcgtgttatgaccccggacctgcgtgaacgtctggaaaacctgcgtaaaaaaccggaaaacatcccgcagccgatctctaacacctctcgtgcgaacctgaacaaactgctgaccgactacaccgaaatgaaaaaagcgatcctgcacgtttactgggaagaattccagaaagacccggttggtctgatgtctcgtgttgcgcagccggcgccgaaaaacatcgaccagcgtaaactgatcccggttaaagacggtaacgaacgtctgacctcttctggtttcgcgtgctctcagtgctgccagccgctgtacgtttacaaactggaacaggttaacgacaaaggtaaaccgcacaccaactacttcggtcgttgcaacgtttctgaacacgaacgtctgatcctgctgtctccgcacaaaccggaagcgaacgacgaactggttacctactctctgggtaaattcggtcagcgtgcgctggacttctactctatccacgttacccgtgaatctaaccacccggttaaaccgctggaacagatcggtggtaactcttgcgcgtctggtccggttggtaaagcgctgtctgacgcgtgcatgggtgcggttgcgtctttcctgaccaaataccaggacatcatcctggaacaccagaaagttatcaaaaaaaacgaaaaacgtctggcgaacctgaaagacatcgcgtctgcgaacggtctggcgttcccgaaaatcaccctgccgccgcagccgcacaccaaagaaggtatcgaagcgtacaacaacgttgttgcgcagatcgttatctgggttaacctgaacctgtggcagaaactgaaaatcggtcgtgacgaagcgaaaccgctgcagcgtctgaaaggtttcccgtctttcccgctggttgaacgtcaggcgaacgaagttgactggtgggacatggtttgcaacgttaaaaaactgatcaacgaaaaaaaagaagacggtaaagttttctggcagaacctggcgggttacaaacgtcaggaagcgctgctgccgtacctgtcttctgaagaagaccgtaaaaaaggtaaaaaattcgcgcgttaccagttcggtgacctgctgctgcacctggaaaaaaaacacggtgaagactggggtaaagtttacgacgaagcgtgggaacgtatcgacaaaaaagttgaaggtctgtctaaacacatcaaactggaagaagaacgtcgttctgaagacgcgcagtctaaagcggcgctgaccgactggctgcgtgcgaaagcgtctttcgttatcgaaggtctgaaagaagcggacaaagacgaattctgccgttgcgaactgaaactgcagaaatggtacggtgacctgcgtggtaaaccgttcgcgatcgaagcggaaaactctatcctggacatctctggtttctctaaacagtacaactgcgcgttcatctggcagaaagacggtgttaaaaaactgaacctgtacctgatcatcaactacttcaaaggtggtaaactgcgtttcaaaaaaatcaaaccggaagcgttcgaagcgaaccgtttctacaccgttatcaacaaaaaatctggtgaaatcgttccgatggaagttaacttcaacttcgacgacccgaacctgatcatcctgccgctggcgttcggtaaacgtcagggtcgtgaattcatctggaacgacctgctgtctctggaaaccggttctctgaaactggcgaacggtcgtgttatcgaaaaaaccctgtacaaccgtcgtacccgtcaggacgaaccggcgctgttcgttgcgctgaccttcgaacgtcgtgaagttctggactcttctaacatcaaaccgatgaacctgatcggtatcgaccgtggtgaaaacatcccggcggttatcgcgctgaccgacccggaaggttgcccgctgtctcgtttcaaagactctctgggtaacccgacccacatcctgcgtatcggtgaatcttacaaagaaaaacagcgtaccatccaggcggcgaaagaagttgaacagcgtcgtgcgggtggttactctcgtaaatacgcgtctaaagcgaaaaacctggcggacgacatggttcgtaacaccgcgcgtgacctgctgtactacgcggttacccaggacgcgatgctgatcttcgaaaacctgtctcgtggtttcggtcgtcagggtaaacgtaccttcatggcggaacgtcagtacacccgtatggaagactggctgaccgcgaaactggcgtacgaaggtctgccgtctaaaacctacctgtctaaaaccctggcgcagtacacctctaaaacctgctctaactgcggtttcaccatcacctctgcggactacgaccgtgttctggaaaaactgaaaaaaaccgcgaccggttggatgaccaccatcaacggtaaagaactgaaagttgaaggtcagatcacctactacaaccgttacaaacgtcagaacgttgttaaagacctgtctgttgaactggaccgtctgtctgaagaatctgttaacaacgacatctcttcttggaccaaaggtcgttctggtgaagcgctgtctctgctgaaaaaacgtttctctcaccgtccggttcaggaaaaattcgtttgcctgaactgcggtttcgaaacccacgcggacgaacaggcggcgctgaacatcgcgcgttcttggctgttcctgcgttctcaggaatacaaaaaataccagaccaacaaaaccaccggtaacaccgacaaacgtgcgttcgttgaaacctggcagtctttctaccgtaaaaaactgaaagaagtttggaaaccggaaatcatccttagcgaaagctaaggattttttttatctgaaatgtagggagaccctcaggttaaatattcactcaggaagttattactcaggaagcaaagaggattaca

SEQ ID NO: 81 - DNA, 329 bp, Artificial Sequence
  Description of Artificial Sequence: Synthetic polynucleotide
tgccgtcactgcgtcttttactggctcttctcgctaaccaaaccggtaaccccgcttattaaaagcattctgtaacaaagcgggaccaaagccatgacaaaaacgcgtaacaaaagtgtctataatcacggcagaaaagtccacattgattatttgcacggcgtcacactttgctatgccatagcatttttatccataagattagcggatcctacctgacgctttttatcgcaactctctactgtttctccatacccgtttttttgggctagcaccgcctatctcgtgtgagataggcggagatacgaactttaagaaggagatatacc

SEQ ID NO: 82 - DNA, 286 bp, Artificial Sequence
  Description of Artificial Sequence: Synthetic polynucleotide
tgccgtcactgcgtcttttactggctcttctcgctaaccaaaccggtaaccccgcttattaaaagcattctgtaacaaagcgggaccaaagccatgacaaaaacgcgtaacaaaagtgtctataatcacggcagaaaagtccacattgattatttgcacggcgtcacactttgctatgccatagcatttttatccataagattagcggatcctacctgacgctttttatcgcaactctctactgtttctccatacccgtttttttgggtagcggatcctacctgac

SEQ ID NO: 83 - DNA, 297 bp, Artificial Sequence
  Description of Artificial Sequence: Synthetic polynucleotide
aatcaggagagcgttttcaatcctacctctggcgcagttgatatgtcaaacaggtttctagagcacagctaacaccacgtcgtccctatctgctgccctaggtctatgagtggttgctggataactttacgggcatgcataaggctcgtaatatatattcagggagaccacaacggtttccctctacaaataattttgtttaacttttactagagctagcagtaatacgactcactataggggtctcatctcgtgtgagataggcggagatacgaactttaagaggaggatatacca

SEQ ID NO: 84 - DNA, 36 bp, Artificial Sequence
  Description of Artificial Sequence: Synthetic oligonucleotide
gtttgagagatatgtaaattcaaaggataatcaaac

SEQ ID NO: 85 - DNA, 29 bp, Artificial Sequence
  Description of Artificial Sequence: Synthetic oligonucleotide
actacattttttaagacctaattttgagt

SEQ ID NO: 86 - DNA, 35 bp, Artificial Sequence
  Description of Artificial Sequence: Synthetic oligonucleotide
ctcaaaactcattcgaatctctactctttgtagat

SEQ ID NO: 87 - DNA, 36 bp, Artificial Sequence
  Description of Artificial Sequence: Synthetic oligonucleotide
ctctagcaggcctggcaaatttctactgttgtagat

SEQ ID NO: 88 - DNA, 38 bp, Artificial Sequence
  Description of Artificial Sequence: Synthetic oligonucleotide
ccgtctaaaactcattcagaatttctactagtgtagat

SEQ ID NO: 89 - DNA, 32 bp, Artificial Sequence
  Description of Artificial Sequence: Synthetic oligonucleotide
gtctaggtactctctttaatttctactattgt

SEQ ID NO: 90 - DNA, 35 bp, Artificial Sequence
  Description of Artificial Sequence: Synthetic oligonucleotide
gttaagttatatagaataatttctactgttgtaga

SEQ ID NO: 91 - DNA, 33 bp, Artificial Sequence
  Description of Artificial Sequence: Synthetic oligonucleotide
gtttaaaaccactttaaaatttctactattgta

SEQ ID NO: 92 - DNA, 122 bp, Artificial Sequence
  Description of Artificial Sequence: Synthetic polynucleotide
gtttgagaatgatgtaaaaatgtatggtacacagaaatgttttaataccatatttttacatcactctcaaacatacatctcttgttactgtttatcgtatccagattaaatttcacgttttt

SEQ ID NO: 93 - DNA, 36 bp, Artificial Sequence
  Description of Artificial Sequence: Synthetic oligonucleotide
ctctacaactgataaagaatttctacttttgtagat

SEQ ID NO: 94 - DNA, 36 bp, Artificial Sequence
  Description of Artificial Sequence: Synthetic oligonucleotide
gtctggccccaaattttaatttctactgttgtagat

SEQ ID NO: 95 - DNA, 35 bp, Artificial Sequence
  Description of Artificial Sequence: Synthetic oligonucleotide
gtcaaaagacctttttaatttctactcttgtagat

SEQ ID NO: 96 - DNA, 85 bp, Artificial Sequence
  Description of Artificial Sequence: Synthetic oligonucleotide
gtctagaggacagaatttttcaacgggtgtgccaatggccactttccaggtggcaaagcccgttgagcttctacggaagtggcac

SEQ ID NO: 97 - DNA, 105 bp, Artificial Sequence
  Description of Artificial Sequence: Synthetic polynucleotide
cgaggttctgtcttttggtcaggacaaccgtctagctataagtgctgcaggggtgtgagaaactcctattgctggacgatgtctcttttaacgaggcattagcac

SEQ ID NO: 98 - DNA, 119 bp, Artificial Sequence
  Description of Artificial Sequence: Synthetic polynucleotide
gaacgagggacgttttgtctccaatgattttgctatgacgacctcgaactgtgccttcaagtctgaggcgaaaaagaaatggaaaaaagtgtctcatcgctctacctcgtagttagagg

SEQ ID NO: 99 - DNA, 23 bp, Artificial Sequence
  Description of Artificial Sequence: Synthetic oligonucleotide
aattactgatgttgtgatgaagg

SEQ ID NO: 100 - DNA, 23 bp, Artificial Sequence
  Description of Artificial Sequence: Synthetic oligonucleotide
tataccataaggatttaaagact

SEQ ID NO: 101 - DNA, 25 bp, Artificial Sequence
  Description of Artificial Sequence: Synthetic oligonucleotide
gtctttactctcacctttccacctg

SEQ ID NO: 102 - DNA, 37 bp, Artificial Sequence
  Description of Artificial Sequence: Synthetic oligonucleotide
atttgaaggtatctccgataagtaaaacgcatcaaag

SEQ ID NO: 103 - DNA, 37 bp, Artificial Sequence
  Description of Artificial Sequence: Synthetic oligonucleotide
gtttgaagatatctccgataaataagaagcatcaaag

SEQ ID NO: 104 - DNA, 36 bp, Artificial Sequence
  Description of Artificial Sequence: Synthetic oligonucleotide
ttgttttaataccatatttttacatcactctcaaac

SEQ ID NO: 105 - DNA, 103 bp, Artificial Sequence
  Description of Artificial Sequence: Synthetic polynucleotide
aaagaacgctcgctcagtgttctgacctttcgagcgcctgttcagggcgaaaaccctgggaggcgctcgaatcataggtgggacaagggattcgcggcgaaaa

SEQ ID NO: 106 - DNA, 122 bp, Artificial Sequence; identical to SEQ ID NO: 92
  Description of Artificial Sequence: Synthetic polynucleotide

SEQ ID NO: 107 - DNA, 85 bp, Artificial Sequence; identical to SEQ ID NO: 96
  Description of Artificial Sequence: Synthetic oligonucleotide

SEQ ID NO: 108 - protein, 1300 aa, Artificial Sequence
  Description of Artificial Sequence: Synthetic polypeptide
MSIYQEFVNKYSLSKTLRFELIPQGKTLENIKARGLILDDEKRAKDYKKAKQIIDKYHQFFIEEILSSVCISEDLLQNYSDVYFKLKKSDDDNLQKDFKSAKDTIKKQISEYIKDSEKFKNLFNQNLIDAKKGQESDLILWLKQSKDNGIELFKANSDITDIDEALEIIKSFKGWTTYFKGFHENRKNVYSSNDIPTSIIYRIVDDNLPKFLENKAKYESLKDKAPEAINYEQIKKDLAEELTFDIDYKTSEVNQRVFSLDEVFEIANFNNYLNQSGITKFNTIIGGKFVNGENTKRKGINEYINLYSQQINDKTLKKYKMSVLFKQILSDTESKSFVIDKLEDDSDVVTTMQSFYEQIAAFKTVEEKSIKETLSLLFDDLKAQKLDLSKIYFKNDKSLTDLSQQVFDDYSVIGTAVLEYITQQIAPKNLDNPSKKEQELIAKKTEKAKYLSLETIKLALEEFNKHRDIDKQCRFEEILANFAAIPMIFDEIAQNKDNLAQISIKYQNQGKKDLLQASAEDDVKAIKDLLDQTNNLLHKLKIFHISQSEDKANILDKDEHFYLVFEECYFELANIVPLYNKIRNYITQKPYSDEKFKLNFENSTLANGWDKNKEPDNTAILFIKDDKYYLGVMNKKNNKIFDDKAIKENKGEGYKKIVYKLLPGANKMLPKVFFSAKSIKFYNPSEDILRIRNHSTHTKNGSPQKGYEKFEFNIEDCRKFIDFYKQSISKHPEWKDFGFRFSDTQRYNSIDEFYREVENQGYKLTFENISESYIDSVVNQGKLYLFQIYNKDFSAYSKGRPNLHTLYWKALFDERNLQDVVYKLNGEAELFYRKQSIPKKITHPAKEAIANKNKDNPKKESVFEYDLIKDKRFTEDKFFFHCPITINFKSSGANKFNDEINLLLKEKANDVHILSIDRGERHLAYYTLVDGKGNIIKQDTFNIIGNDRMKTNYHDKLAAIEKDRDSARKDWKKINNIKEMKEGYLSQVVHEIAKLVIEYNAIVVFEDLNFGFKRGRFKVEKQVYQKLEKMLIEKLNYLVFKDNEFDKTGGVLRAYQLTAPFETFKKMGKQTGIIYYVPAGFTSKICPVTGFVNQLYPKYESVSKSQEFFSKFDKICYNLDKGYFEFSFDYKNFGDKAAKGKWTIASFGSRLINFRNSDKNHNWDTREVYPTKELEKLLKDYSIEYGHGECIKAAICGESDKKFFAKLTSVLNTILQMRNSKTGTELDYLISPVADVNGNFFDSRQAPKNMPQDADANGAYHIGLKGLMLLGRIKNNQEGKKLNLVIKNEEYFEFVQNRNN

SEQ ID NO: 109 - protein, 1300 aa, Artificial Sequence
  Description of Artificial Sequence: Synthetic polypeptide
MSIYQEFVNKYSLSKTLRFELIPQGKTLENIKARGLILDDEKRAKDYKKAKQIIDKYHQFFIEEILSSVCISEDLLQNYSDVYFKLKKSDDDNLQKDFKSAKDTIKKQISEYIKDSEKFKNLFNQNLIDAKKGQESDLILWLKQSKDNGIELFKANSDITDIDEALEIIKSFKGWTTYFKGFHENRKNVYSSDDIPTSIIYRIVDDNLPKFLENKAKYESLKDKAPEAINYEQIKKDLAEELTFDIDYKTSEVNQRVFSLDEVFEIANFNNYLNQSGITKFNTIIGGKFVNGENTKRKGINEYINLYSQQINDKTLKKYKMSVLFKQILSDTESKSFVIDKLEDDSDVVTTMQSFYEQIAAFKTVEEKSIKETLSLLFDDLKAQKLDLSKIYFKNDKSLTDLSQQVFDDYSVIGTAVLEYITQQVAPKNLDNPSKKEQDLIAKKTEKAKYLSLETIKLALEEFNKHRDIDKQCRFEEILANFAAIPMIFDEIAQNKDNLAQISLKYQNQGKKDLLQASAEEDVKAIKDLLDQTNNLLHRLKIFHISQSEDKANILDKDEHFYLVFEECYFELANIVPLYNKIRNYITQKPYSDEKFKLNFENSTLANGWDKNKEPDNTAILFIKDDKYYLGVMNKKNNKIFDDKAIKENKGEGYKKIVYKLLPGANKMLPKVFFSAKSIKFYNPSEDILRIRNHSTHTKNGNPQKGYEKFEFNIEDCRKFIDFYKESISKHPEWKDFGFRFSDTQRYNSIDEFYREVENQGYKLTFENISESYIDSVVNQGKLYLFQIYNKDFSAYSKGRPNLHTLYWKALFDERNLQDVVYKLNGEAELFYRKQSIPKKITHPAKEAIANKNKDNPKKESVFEYDLIKDKRFTEDKFFFHCPITINFKSSGANKFNDEINLLLKEKANDVHILSIDRGERHLAYYTLVDGKGNIIKQDTFNIIGNDRMKTNYHDKLAAIEKDRDSARKDWKKINNIKEMKEGYLSQVVHEIAKLVIEHNAIVVFEDLNFGFKRGRFKVEKQVYQKLEKMLIEKLNYLVFKDNEFDKTGGVLRAYQLTAPFETFKKMGKQTGIIYYVPAGFTSKICPVTGFVNQLYPKYESVSKSQEFFSKFDKICYNLDKGYFEFSFDYKNFGDKAAKGKWTIASFGSRLINFRNSDKNHNWDTREVYPTKELEKLLKDYSIEYGHGECIKAAICGESDKKFFAKLTSVLNTILQMRNSKTGTELDYLISPVADVNGNFFDSRQAPKNMPQDADANGAYHIGLKGLMLLDRIKNNQEGKKLNLVIKNEEYFEFVQNRNN

SEQ ID NO: 110 - protein, 1368 aa, Artificial Sequence [sequence omitted]

SEQ ID NO: 111 - protein, 7 aa, Simian virus 40
PKKKRKV

SEQ ID NO: 112 - protein, 16 aa, Unknown
  Description of Unknown: Nucleoplasmin bipartite NLS sequence
KRPAATKKAGQAKKKK

SEQ ID NO: 113 - protein, 9 aa, Unknown
  Description of Unknown: C-myc NLS sequence
PAAKRVKLD

SEQ ID NO: 114 - protein, 11 aa, Unknown
  Description of Unknown: C-myc NLS sequence
RQRRNELKRSP

SEQ ID NO: 115 - protein, 38 aa, Homo sapiens
NQSSNFGPMKGGNFGGRSSGPYGGGGQYFAKPRNQGGY

SEQ ID NO: 116 - protein, 42 aa, Unknown
  Description of Unknown: IBB domain from importin-alpha sequence
RMRIZFKNKGKDTAELRRRRVEVSVELRKAKKDEQILKRRNV

SEQ ID NO: 117 - protein, 8 aa, Unknown
  Description of Unknown: Myoma T protein sequence
VSRKRPRP

SEQ ID NO: 118 - protein, 8 aa, Unknown
  Description of Unknown: Myoma T protein sequence
PPKKARED

SEQ ID NO: 119 - protein, 8 aa, Homo sapiens
PQPKKKPL

SEQ ID NO: 120 - protein, 12 aa, Mus musculus
SALIKKKKKMAP

SEQ ID NO: 121 - protein, 5 aa, Influenza virus
DRLRR

SEQ ID NO: 122 - protein, 7 aa, Influenza virus
PKQKKRK

SEQ ID NO: 123 - protein, 10 aa, Hepatitis delta virus
RKLKKKIKKL

SEQ ID NO: 124 - protein, 10 aa, Mus musculus
REKKKFLKRR

SEQ ID NO: 125 - protein, 20 aa, Homo sapiens
KRKGDEVDGVDEVAKKKSKK

SEQ ID NO: 126 - protein, 17 aa, Homo sapiens
RKCLQAGMNLEARKTKK

SEQ ID NO: 127 - DNA, 4098 bp, Artificial Sequence
  Description of Artificial Sequence: Synthetic polynucleotide
atgggtaagatgtattatctgggtttggatataggcactaactctgtgggatatgcagtaactgatccctcgtatcacttgttaaagttcaaaggcgaacccatgtggggagcacatgtatttgctgcgggtaatcagagtgccgaaaggcgatctttcagaacatccaggaggcgattagataggagacagcaaagagtaaagcttgtgcaagagatctttgctcctgtcatttcacctatagaccctcgtttttttataagattgcacgaatcggctctatggagagacgatgttgccgaaacagataaacatatctttttcaatgatcccacttatacagacaaggaatactactccgactacccgacaattcatcatttgatcgtcgatcttatggagagctctgaaaagcatgacccccgacttgtctatttggctgtagcttggttagttgctcatagaggtcatttcttgaatgaagtagataaagacaatataggtgatgtactttcttttgatgctttctacccggaatttttggcctttttgtcagacaatggcgtcagtccctgggtctgtgagtcgaaggcccttcaagctactctgctgtctaggaatagcgtcaacgacaaatataaagcattaaaatcgctgatattcggatcgcaaaaaccggaagataactttgacgctaacatctctgaagatggtttaatccaattgctggcgggtaagaaagttaaagtaaacaaactattcccacaagagtccaacgatgctagctttacgttgaatgataaagaagacgctattgaagaaattctaggtactttaacgcctgacgagtgcgaatggatcgctcatattcgcagattgttcgattgggccatcatgaaacacgcgctaaaggatggcaggacgatatctgaatcaaaagtgaagctatacgagcagcatcatcatgacttgactcagttaaagtactttgtgaagacctacctagctaaagagtatgatgatatcttcagaaacgtagactccgagacaactaaaaattatgtagcttattcttaccatgtgaaggaagtgaaaggcacattaccaaaaaataaagcaacgcaagaagaattttgtaaatacgtccttggcaaagtcaaaaacattgaatgttccgaagcagacaaggttgattttgatgaaatgatacaacgacttacggacaattcttttatgccaaagcaagtctcaggtgaaaatagagtaataccataccagttgtactactatgaattaaagacaattttaaacaaagccgcctcatatctaccttttttgacacaatgcggtaaagatgctatttctaaccaagacaaattactgtctataatgacatttcgcataccatatttcgtcggccctttaaggaaagataattcagaacatgcctggttggaacgtaaagcgggtaaaatttacccgtggaactttaatgataaagtagatcttgataaatcggaggaagcctttatccgtaggatgaccaatacttgcacgtattacccaggagaagacgtgttaccattagattcacttatctatgaaaagtttatgatcttgaatgagataaacaatattaggattgacggataccccatttctgttgatgtgaaacaacaagtatttggtttatttgagaagaaaaggcgagtaacagttaaggatattcaaaatctactattatctcttggagcgttggataaacacggtaagctgactggtattgacacgacaatacactctaattataacacttatcatcattttaaatctcttatggagcggggagtattgaccagagatgatgtggaaagaatagtggaaagaatgacatattctgacgatactaagagggtcagactgtggttaaataataattatggaactctaacagctgacgatgttaagcatatctcaagactcagaaaacacgatttcggccgtttgtctaaaatgtttttgacaggattgaaaggtgttcataaggagacaggcgagagagcaagtatactggattttatgtggaatactaacgacaatttaatgcaactactgtccgaatgttacacattctcggatgagatcaccaaattacaagaggcctactacgcaaaagctcaattatcgctaaatgacttcttggactctatgtatatatcaaacgccgttaagagacctatttatcggaccttagcggtagtaaatgatattagaaaggcatgcgggacggcacctaaaagaattttcatcgagatggcgcgagatggagagtctaagaagaaaagatctgtgactcgtagagagcaaattaaaaatctctatagatcaattcgtaaagactttcaacaagaagttgattttctggaaaagatattggaaaataagagtgacgggcagcttcagtctgacgctttatatttgtattttgctcaattaggcagagacatgtacacaggtgatccaatcaaattagaacatattaaagaccaatctttttacaacattgatcatatttatcctcaatcgatggtgaaagatgacagtttggataacaaggtactagtccaaagcgaaatcaatggcgaaaagagttcgcgctatccattagacgcagccattagaaacaaaatgaagccgttgtgggatgcctactataatcatggattaatttctcttaagaaataccagcgtttgacgagatctactccatttacggacgacgagaagtgggattttatcaatcgtcagctagttgaaactaggcaatctactaaagctttagcaatattgttaaagcgtaagtttccagatactgaaatagtttactcaaaggctggactatccagcgattttagacatgaattcggcctggttaagagtaggaatattaatgatctacaccatgctaaagatgcctttctcgcaatagttactgggaacgtttatcatgaaagatttaatagaagatggtttatggttaaccagccatactctgtgaaaactaagacattgtttacccattcaattaagaatggcaactttgtcgcttggaatggagaagaagatcttggacgtatcgtaaagatgttgaaacaaaacaagaacacaatccacttcaccaggttttcctttgataggaaggagggattgttcgatattcaacctctcaaagcttctaccggattggttccacgaaaagcagggttggatgttgttaaatatggaggatacgataaaagcactgccgcgtattatttattagtacgttttacactcgaggataagaagactcaacacaaattgatgatgattcctgttgaaggtctctacaaagcacgtattgaccatgataaagagtttttaacagattatgctcagaccacgatcagcgaaattcttcaaaaggacaagcagaaagtgatcaacatcatgttccctatgggcacgagacatatcaaactgaattcgatgatttctattgatggattctatctttctattggtgggaagagtagcaaaggtaagtcagtactatgtcatgctatggtgccattaatcgtcccacacaagatagaatgttatatcaaggctatggaatcgtttgcaagaaaattcaaagaaaataataaattgaggatcgttgaaaagtttgataaaataactgttgaagataacttgaacttatacgagctttttctacaaaagttgcaacataacccatataataaatttttctctacacaatttgatgtgttgacgaacggtagaagtacattcaccaaattgtctccagaggagcaagtccagactttacttaatatactgagtatatttaaaacttgtcgttcttctgggtgtgatttaaaatcaataaatggttccgctcaagcggctagaattatgatatccgctgatttaactggcttatcaaaaaagtattcagatattagattagttgagcaaagcgcatcaggtctatttgtttcaaaatctcaaaatctcttggaatacttgccaaaaaagaaaaggaaagtttag

SEQ ID NO: 128 - DNA, 4005 bp, Artificial Sequence
  Description of Artificial Sequence: Synthetic polynucleotide
atgagtagtttaacaaagtttaccaataaatatagtaagcaactaactataaagaacgaattgataccggtcggtaagactttggaaaacataaaagaaaatgggttgattgatggagacgagcaattgaatgagaattatcaaaaagcaaagataatagtagatgattttttgagagactttattaataaagctctaaataacactcaaattggtaactggagagagctagccgacgccttgaacaaggaagatgaggataatattgagaaattacaagataagattagagggattatcgtgtctaagtttgagacttttgatctgttcagttcgtattcgattaaaaaggacgagaaaatcatcgatgatgataacgatgtggaagaagaggagctagaccttgggaagaagacatctagcttcaaatacatattcaagaaaaatttgttcaaacttgtccttccttcatatttaaaaacaacaaatcaagataagttaaaaatcatttcttccttcgataattttagtacttattttcgtggttttttcgaaaacaggaaaaatatattcactaaaaagcctatatctacctctatagcttatagaattgttcacgataatttcccaaaatttctagataatatcaggtgttttaatgtttggcaaaccgagtgtcctcagttaatagtcaaggccgacaactaccttaaaagcaagaatgtgattgcaaaagataagtctttggctaactattttacagtcggtgcctatgattattttctgagtcaaaatggtatcgatttctataacaacattattggcggcttaccagcttttgccgggcatgagaagattcagggtttgaacgaatttatcaatcaagaatgtcaaaaggattctgaattaaagtctaagctcaagaataggcacgctttcaaaatggcagtcttattcaaacaaatcctttcagacagagaaaagtcatttgtgattgacgagttcgaatcagacgctcaggtaattgatgctgttaaaaatttttacgcggaacaatgcaaagataataacgtcatatttaatttattgaatctgatcaagaatattgcttttttgtcggatgatgagttagacggcattttcatagagggtaaatacctgtcctctgtgtctcaaaaattgtatagtgattggtcaaagttgagaaatgatattgaagattcggctaattctaaacagggtaacaaagaattagcgaagaaaatcaaaactaacaagggtgatgttgaaaaggctataagtaagtacgagttcagtttatctgaactaaattcaattgttcatgataacacaaaattttccgatcttttatcatgcacattacataaagttgcaagtgaaaaattagtcaaagtaaacgaaggtgattggccaaaacatctaaaaaacaacgaggaaaaacagaagataaaagaacctcttgacgctttattggaaatatacaatactctattaatatttaactgtaaaagttttaacaaaaatggtaatttctatgtcgactacgatcgctgcattaatgagttgtccagtgttgtgtacttgtataataaaactcgtaattattgtacgaaaaagccgtacaacactgacaaatttaagttgaatttcaactccccacaactgggtgagggcttctctaaaagtaaagagaatgattgccttacattattatttaaaaaagatgataattattatgtcggaatcataagaaagggggcaaagatcaacttcgatgacactcaggccatagcagacaacacagataactgtatattcaaaatgaattattttttgctgaaggatgctaaaaaatttatccccaaatgttcaatacaattaaaagaggttaaggcccatttcaaaaagtcggaagatgactatattttgtccgataaggaaaaattcgctagtccgcttgttattaaaaaatccacatttcttctcgctacggctcatgtgaaaggaaagaagggcaatattaagaaatttcagaaagaatactccaaagaaaatcctacggagtatagaaatagtctgaacgaatggatagcattctgcaaagagttcttgaagacctataaagctgccaccatctttgatattacaactttgaaaaaggccgaggaatacgctgacattgtggaattctataaggatgtagataatctttgttacaagttagaattttgccctatcaaaacttcttttatcgaaaatcttatagataatggcgatttatacctgtttagaattaataacaaggacttttcttcaaaaagtacaggcacgaaaaacttacacacattatacttgcaggctatatttgacgagcgaaacttaaacaaccccacgataatgttgaatggaggtgcagagttattctacagaaaagaatctatagaacagaaaaatcggatcacgcacaaagccggtagtatcttagtgaataaagtgtgcaaagatggtacaagtctagatgacaaaatccgtaacgaaatttaccagtatgaaaacaaattcattgatactctttcggacgaagctaaaaaggttctgccaaacgttattaagaaagaggctacgcatgatataacaaaagataaacgtttcactagcgacaaattcttctttcattgtcctttaacaatcaactacaaggaaggtgacaccaaacaatttaataatgaagtgctctcattccttagaggtaaccccgatatcaatattatcggcattgatagaggagaaagaaacctaatctatgtaacagtcattaaccaaaaaggcgaaatattggatagcgtctccttcaatactgtcaccaataagtcatcgaagatagaacaaactgttgattacgaagaaaaattggccgttagagaaaaggaacgtatcgaagcgaagagatcttgggatagcatatccaagattgccaccttgaaggagggttatctaagcgcgatcgtacatgaaatctgcttattaatgattaagcataatgctattgtcgtgttagaaaacctgaatgccggttttaaaaggattagaggtggtttgtcagaaaagtcagtatatcaaaagtttgaaaagatgcttattaataaactcaactacttcgttagcaagaaagaaagtgattggaataaaccgtcaggtttgctcaatggtcttcagttaagtgatcaatttgagtctttcgaaaaattaggaattcaaagtggattcattttttatgtaccagccgcgtacacttcaaaaattgaccctacgaccggatttgccaacgtcttgaatttgtccaaggtcagaaatgttgacgccatcaaaagtttttttagcaacttcaatgaaatctcttattccaaaaaggaagcccttttcaagttttcttttgacctagactcgttatcgaagaaaggattttcatctttcgtaaagtttagcaagtccaagtggaatgtatacacattcggcgagagaattatcaagcccaagaacaaacagggctatagagaagacaagagaatcaacttgacttttgagatgaaaaaattactcaacgaatacaaggtttcatttgatttggagaacaacttgattcccaatttgacatcagctaacttgaaggatacgttctggaaggagttattctttatattcaaaacgacattacaactgcgtaatagtgttacaaacggtaaagaagatgtattaatctcacctgtaaagaatgccaaaggagaatttttcgtatccggtactcacaataagacactaccacaggattgcgacgctaacggtgcgtatcatattgcgttgaaaggattaatgatacttgaaagaaataaccttgttcgcgaagaaaaagacaccaagaagatcatggctattagcaatgttgattggtttgaatacgtgcaaaagaggagaggtgttttgtaa

SEQ ID NO: 129 - DNA, 3717 bp, Artificial Sequence
  Description of Artificial Sequence: Synthetic polynucleotide
atgaacaattatgacgagttcacaaagctataccctatccaaaaaactatcaggttcgaattgaaaccacaagggagaacaatggaacatctggagacattcaacttttttgaagaggacagagacagagcggagaaatacaaaattttaaaagaggccatcgatgaatatcacaaaaagtttatcgacgagcatttaacaaacatgtctttggactggaattcacttaaacaaatttctgagaaatattataagtctcgggaggaaaaagacaaaaaggtctttttgtccgagcaaaagagaatgagacaagaaattgtctcggagtttaaaaaagatgatcggttcaaagatttgtttagcaagaaattgttttctgaattgttgaaggaggagatatacaagaaaggcaaccatcaagaaatagatgctttgaaatcgtttgacaagttcagcggttacttcattggtttacatgaaaataggaagaacatgtatagcgacggcgatgagatcaccgctatatcgaatagaatcgttaacgaaaattttccgaaatttttggataatttgcaaaaataccaggaagctaggaaaaagtaccctgaatggataataaaggcggaatcagctttggtggctcacaacataaagatggatgaagtcttctcgctggaatattttaacaaagtattaaatcaggaaggaatccaaagatacaacttagccttgggtggatacgtaaccaaatcaggtgagaaaatgatgggcttaaatgatgcacttaatctagctcaccaatccgaaaagtcctctaaagggaggatacacatgacaccattgtttaagcaaatcctttcggagaaagaatctttttcatatatccccgatgttttcactgaggatagtcaattgttgcccagcattggtggattttttgcacaaatagaaaatgataaagatggtaacatcttcgatagagccttggaattgataagctcctatgcagaatacgatacggaacgaatatacattagacaagctgacatcaacagagtaagcaatgttatttttggtgagtggggaactttaggtggattaatgcgggagtacaaagctgactcaatcaatgatattaatttggaacgtacgtgcaaaaaagtcgataagtggcttgatagtaaggagtttgctctgtcggatgtactagaagcaattaagagaacaggaaacaatgatgcatttaatgaatatattagtaaaatgaggacggctagagaaaagatagacgccgcacgtaaggaaatgaagtttatttccgagaaaatatctggcgatgaagagtcgattcacatcatcaagaccctactcgattctgttcagcaatttctccatttttttaacctcttcaaagcaagacaagacattcccttagatggggctttttatgccgaatttgatgaagttcattcaaagttgtttgctattgttcctctttacaataaggtccgtaattaccttactaaaaataacttgaacaccaagaaaataaagttaaacttcaagaatccgactcttgccaacgggtgggatcagaataaagtttatgattatgctagcttaatatttctaagagatgggaattattacttaggaatcatcaatccaaagcgtaagaaaaacattaaatttgaacaagggtcaggcaatggcccattctatagaaaaatggtgtataagcaaataccaggacctaacaagaacttgcctcgcgtatttttaacttcaacaaagggtaaaaaagaatataaaccaagcaaagaaattattgaaggttacgaagcagataaacacatcagaggtgataagttcgatctggatttctgccataaattgattgacttttttaaggaatctatagaaaaacataaggactggtccaaatttaatttctacttctcacctacagaaagttatggtgacatttcagaattttatttagacgttgagaaacaaggatataggatgcattttgaaaatatttcagcggaaaccatcgacgaatacgttgagaagggtgatttattcttgttccaaatttacaataaagacttcgttaaagctgcaaccggaaagaaggatatgcataccatatattggaacgctgcattctcgccagaaaacttacaagatgtcgttgtaaagcttaatggagaagctgagctgttctatagagacaagagtgatataaaagagattgtgcatcgggaaggtgaaattctggtgaacagaacttacaatggtcgtacacccgttccagacaaaatacataaaaaactgaccgattatcataatggtaggacaaaggacttgggcgaggccaaggagtacctcgataaagttagatatttcaaggcacactatgatattacgaaagacaggagatatttaaacgataaaatttactttcatgtccctttgacccttaactttaaagctaatggtaaaaagaatttgaacaaaatggtaattgagaagtttttatcggacgaaaaagctcacataatcggaatcgaccgcggagagagaaatttactgtattatagtatcatcgacagaagtggaaagattattgatcagcaatctttgaacgtcattgatgggtttgactatcgggaaaagttaaatcaaagggaaattgaaatgaaggatgcgagacaatcatggaatgccattggtaaaattaaagatctcaaggaggggtacttatcaaaagctgtacacgagataactaaaatggctatccaatataatgcaattgttgtaatggaagaattgaattatggttttaaacgcggcaggtttaaagtcgaaaaacaaatataccaaaagtttgaaaacatgttaattgataagatgaactatcttgttttcaaagatgcacctgatgagagtcctggcggtgtgctgaacgcctatcaattaacaaacccattagagtcctttgctaaactgggtaaacaaactggcattctattttatgttccagccgcttacacctcaaagatcgatccaacgaccggttttgtaaacttatttaatacttcttccaaaacaaacgcgcaagaacgcaaagaattcctacaaaaatttgaatcaatatcctatagcgcaaaagatggaggtatattcgctttcgcttttgactacagaaagtttggcacttccaagacagatcataaaaatgtgtggaccgcttataccaacggagaaaggatgcgttatattaaagaaaaaaagaggaacgaactatttgatccatcgaaagaaattaaagaagctttgacaagcagcggaatcaaatatgatggaggtcaaaacatacttccagatattctcagatctaataataacggtcttatttacacgatgtattcatcttttatcgctgccatccaaatgcgtgtgtatgatggcaaggaagattatattatatctcctattaaaaattcaaagggtgaattttttcgcacggatccaaaaagaagagagcttccaattgacgccgatgctaacggtgcttacaatattgcattgcgtggtgaacttactatgagagccatcgccgaaaagtttgatccggacagtgaaaaaatggcgaaattggagctaaagcacaaggattggtttgaattcatgcagacccgtggcgattga

SEQ ID NO: 130 - DNA, 3897 bp, Artificial Sequence
  Description of Artificial Sequence: Synthetic polynucleotide
atgactaaaacgttcgactccgagttttttaatctctattccttgcaaaagaccgttaggtttgaattgaaaccagttggtgaaactgcctcatttgtcgaagactttaaaaacgagggattgaaaagagtggttagtgaagatgaaagaagggcagtagactatcaaaaggttaaagaaatcattgacgattaccacagagattttatagaagaatctctgaactattttccagagcaggtttcaaaagatgctctagagcaagcgtttcatttgtatcaaaagttgaaagcagcgaaggtggaagaaagggaaaaagctttaaaagaatgggaagcattacagaaaaaattgcgagaaaaagtcgtcaaatgtttcagcgactctaataaagctcgcttttctagaatcgataaaaaagaattgattaaggaagatttaataaattggctggtagcacaaaacagagaggatgatattcctactgttgaaacgttcaataattttactacttacttcactggtttccatgagaacaggaagaatatttactctaaagatgatcacgctactgctataagttttaggttgattcacgaaaacttgcctaaattttttgacaatgtcatcagttttaacaagttgaaagaaggtttcccggaattaaaattcgacaaagttaaagaagatttagaagtagattacgacttgaagcatgcgtttgaaattgaatatttcgttaatttcgtcacacaagctggtatcgaccaatataattacctgcttggaggcaaaactctagaagacggtacgaagaaacaaggaatgaatgaacagattaatttatttaagcaacaacaaactcgcgataaagctagacagattccaaaactgattccacttttcaaacagattctatctgagagaactgaatctcagagttttatccctaagcagttcgagtctgatcaggaactattcgattccctgcagaaattgcataacaactgtcaagataagtttaccgttttgcaacaggcgatcttgggattggctgaggcagatcttaaaaaggtctttattaaaactagtgatctaaacgcattgtctaacactatttttggaaattattctgtgttctcagacgcgctcaatttatataaagagtcgctaaaaactaaaaaggctcaagaagcttttgaaaagttgcctgcacatagtattcatgatttaatccaatacttagaacaatttaattcgtctctcgatgctgaaaagcaacagtctaccgatactgtattaaactactttattaaaaccgacgaattatatagtcgtttcattaaatccacctctgaggcattcacccaagtacaacctctctttgaactggaagctttgagctccaaaagaagacccccagaaagtgaagatgagggggctaaaggccaagaaggtttcgaacaaattaagagaatcaaagcttatctagacactctaatggaggctgtccactttgctaagcctttgtatcttgtcaagggtagaaagatgatagagggtctagacaaggatcaaagcttctacgaagcgtttgaaatggcctaccaggagttggagtctttaatcatccccatttacaataaggccagatcttacctgtctaggaagccatttaaagcggataaattcaaaattaattttgacaataatacacttctatctgggtgggatgctaacaaggagacggctaacgccagcatattgtttaagaaggatggtttatactacctgggaatcatgccaaaaggcaaaactttcttgttcgattatttcgttagttcagaagattctgaaaagttgaaacaacggagacagaaaaccgcagaggaagcgctcgcacaggatggagaatcctattttgaaaaaatacggtataaactcctaccaggtgctagtaagatgttgccaaaggtattttttagcaataaaaatattgggttttacaatccctcagatgatattctacgaattcggaatacggcctctcatactaagaatggtactccccagaagggtcattccaaggtagaatttaacttgaatgactgtcacaaaatgattgatttttttaaatcttccatacagaaacatcccgagtggggatcctttggtttcactttttctgatacgtcggactttgaagatatgagtgctttctaccgagaagttgaaaatcaaggttacgttataagttttgataaaataaaagaaacttacattcagtctcaagttgagcaaggtaacttatatttatttcaaatttacaacaaagattttagtccgtattcaaagggaaagccaaacctgcacactttatactggaaagctctgtttgaagaggctaatttgaataacgtagtggctaagctaaacggcgaagcagaaatctttttcagaagacacagtatcaaagcatctgataaagtggtacatcctgctaatcaagctatagataataagaatccccatactgagaagacgcagtccacatttgaatatgacttggtcaaagacaaaagatatacccaagacaaatttttttttcatgtaccgatatctttaaactttaaggctcagggcgtttcaaagtttaatgataaggtaaatggattcttaaagggcaatcccgacgttaatataatcggtatagatcgaggtgagagacatcttttatactttaccgtggtgaatcaaaaaggagaaatattagtgcaagagtccttgaatacattaatgtctgacaagggtcatgtcaacgattatcaacagaaattggacaagaaggaacaggaaagggacgctgccaggaagtcctggacgacagtagaaaatattaaagaattaaaagaaggttatttatcacatgtggttcataaacttgcacatttaatcatcaaatataacgcaatagtgtgcttggaagatcttaattttggcttcaagaggggtaggttcaaggtcgaaaaacaggtctaccagaagttcgagaaagctctgatcgataaattgaattatcttgttttcaaagaaaaagaattaggagaagttggtcattatcttacagcataccaactcactgcaccatttgaaagcttcaaaaagctaggcaagcaatctgggattttgttctatgttccggctgattatacatcaaagatagatcctaccacaggctttgtaaattttttagatcttaggtaccaatccgttgaaaaagctaaacagttgctgtccgattttaatgcgataagatttaatagtgttcagaattattttgagttcgaaattgattataaaaaattgacaccaaaacgtaaagtaggaacacaatctaaatgggttatttgtacctatggagatgttagataccaaaacagaagaaatcagaaaggtcactgggaaactgaagaagttaacgttactgaaaaacttaaagctctatttgcgagcgattcaaaaacgacgacggtgatcgattatgcaaatgatgataaccttattgatgtaattctggaacaagataaggcatcattttttaaagaactactatggttgttaaagctaaccatgaccctaaggcactccaagataaagtcagaggatgattttatcctctctccagtgaaaaacgaacaaggtgagttttacgactcaagaaaggcgggtgaagtctggcctaaggatgctgatgccaatggagcttatcacatcgctctgaaggggctatggaacttacagcaaattaaccaatgggaaaaaggtaaaactttaaacctcgccataaagaaccaggattggttcagctttatccaagaaaaaccatatcaagaataa

SEQ ID NO: 131 - DNA, 3708 bp, Artificial Sequence
  Description of Artificial Sequence: Synthetic polynucleotide
atgcacacaggaggtctactctcgatggatgctaaggaatttaccggtcaatatccgctgtccaaaactttgcgttttgagcttagacctattggccgaacgtgggataacctagaggcttctggttatttggcggaagatagacatagagctgagtgttatccccgagctaaagaattgctggatgataaccacagggcgttcctgaatagagttctaccgcaaatcgatatggattggcatccaattgctgaagctttctgcaaggtgcacaaaaatccaggtaataaagaattggctcaggattataatttgcagcttagtaagagaagaaaagaaatttccgcttatttgcaggatgctgatggatacaaggggttgttcgcgaaacctgccctggacgaagctatgaaaatagctaaggaaaacggcaatgaatctgatattgaagttttggaagccttcaatggattttccgtttatttcactggttatcatgagagtagggagaatatatactcagacgaagatatggtatccgtcgcctatcgcataactgaagataattttccaaggttcgtgtcgaacgcgttaatttttgataaactaaatgaatcgcacccggatattatttcggaagtgtccggtaatctgggggtagacgatattggtaaatattttgatgtgtccaactacaataatttccttagtcaagcaggaattgatgactacaaccatattataggagggcatacaactgaagacggtctcattcaagcttttaacgtagtgttaaacctaaggcaccaaaaagacccaggttttgagaaaattcaatttaagcaactctacaagcagatactgagcgttaggactagtaagtcatatatcccaaagcaattcgataactcaaaggaaatggtcgactgtatatgcgactacgtctcaaaaatagaaaaatctgaaacagtagaaagagctctgaaattggtaagaaatatatcttcttttgatttaagaggtattttcgtaaataaaaaaaaccttcgaattttgtctaataagttaattggagactgggacgcaatagagacagctttgatgcacagttccagcagtgaaaacgataagaaatcagtgtatgactctgcagaggcattcacccttgatgatatcttcagttctgtgaaaaagttcagcgacgcctccgctgaggatataggaaaccgcgctgaagacatatgtcgtgttatctcagaaacagctcctttcattaacgacttaagggctgtagatttggattctttaaatgatgacggctatgaagcggccgtgtctaaaatacgggaatctcttgaaccctacatggatctatttcacgaattggagatctttagcgtgggtgatgagtttcctaaatgtgctgccttttatagcgagttggaagaggtctcagaacaactgattgaaatcattcctttatttaacaaagcaagaagtttttgcacaaggaaaaggtattcaaccgacaaaatcaaagtcaatttaaaattccctactctggcagatggatgggatctaaataaagaaagggataacaaagccgcaattctaagaaaagacggtaaatactacctggcaattttagacatgaagaaagatctcagtagtattcgtacgagcgatgaggacgagtcttcttttgaaaagatggaatataaattgctcccttctcctgtgaaaatgcttccaaaaatttttgttaaatcgaaagccgccaaagaaaagtacgggttgaccgatagaatgttagaatgctacgataaaggtatgcataagtcgggtagtgcttttgatttgggtttttgtcatgaattgatcgattactataagcgctgcattgccgagtacccaggctgggatgttttcgactttaaatttcgtgagacaagcgattacggatccatgaaagaatttaatgaagacgtcgctggcgcaggttactatatgtcacttagaaagattccatgttccgaagtttatcgtttactggacgagaagtcaatttacttgtttcaaatatataataaggattatagcgaaaacgcacatgggaataagaatatgcatacgatgtattgggagggcttgttctcaccacaaaatttggaatcaccagtcttcaaattgtccggaggcgcagaactttttttcagaaagtcatctattcctaatgacgctaaaacggtacatccgaaaggttcagttcttgttcccagaaacgacgtcaatggtagaagaataccagactcgatctacagagagttgacaaggtattttaaccgtggggattgcaggatcagtgatgaagctaagtcttacctggacaaggtcaagacaaaaaaagcggaccatgacattgttaaggatagaagatttactgtagataagatgatgttccatgttccgattgccatgaattttaaagctataagtaaaccaaatcttaataagaaagttattgatggcataatagatgatcaagatttgaaaatcatcggtatcgatcgtggtgagagaaatcttatttatgtgaccatggtcgataggaaggggaatatattgtatcaagacagtcttaatattttaaatggatacgattaccgcaaagctttagacgtgagggaatatgataacaaagaagctagaaggaattggactaaagtagaaggtattagaaaaatgaaagaaggttatttatctttagctgttagtaaattggccgatatgatcatcgaaaataatgctataatcgtaatggaagatttgaatcacgggtttaaggcaggtcgttccaaaattgaaaagcaggtgtatcaaaaattcgaatcaatgttaatcaacaagttaggatacatggtgctaaaagacaagtccattgaccagtctggtggagcccttcatggttaccaattagccaatcatgttacgaccttagctagcgtgggtaaacaatgtggagtaattttttacatacctgcagcttttacttcgaagattgatcccaccacgggctttgctgatttattcgctctctctaatgtgaagaatgtcgcttctatgagagagttcttctccaaaatgaagtcagtaatatatgacaaggcggaaggcaaattcgcctttacatttgattatttggattataacgttaaaagcgaatgtggacgtaccttatggactgtgtatacagttggtgaacgcttcacctactctagagtaaaccgagagtatgttcggaaagtcccaacagatatcatctatgatgcattacaaaaagctggtattagcgtcgaaggtgaccttagagatagaatcgcggaaagcgacggtgacacattaaagtctatattctacgcttttaaatacgcgttggatatgagagtcgaaaacagagaggaagactatatacagtcacctgtgaagaatgcttctggtgagttcttttgttcaaaaaacgccggaaagtctttgccgcaggattcagatgcaaatggtgcctataatatagctctgaaagggatcctacaactcagaatgttgagcgaacaatacgatccaaatgcagaatcgattagattgccacttataactaacaaggcatggttaacttttatgcaatccggtatgaaaacttggaagaattaa

SEQ ID NO: 132 - DNA, 3783 bp, Artificial Sequence
  Description of Artificial Sequence: Synthetic polynucleotide
atggattctcttaaggatttcactaatttatatccagtctcgaaaacattgcggttcgaattgaaaccagttgggaaaactctagaaaacattgaaaaagccggtatattgaaagaagatgaacacagagcggaatcctaccgccgggtaaaaaagataattgacacataccataaagtgtttattgacagctccttagagaacatggctaaaatggggatagaaaatgaaatcaaggctatgctgcagtctttttgtgaactctataagaaagaccacaggacagaaggagaagataaagctcttgataaaattagagctgttcttagaggtttaatcgttggggctttcactggtgtatgtggaagacgagaaaacacagtacaaaatgaaaagtacgagagtttgttcaaagaaaaattgataaaggaaattttgccagatttcgtgttgtccaccgaggctgagtctcttccattcagcgttgaagaagcaacaaggagcttaaaagagtttgactcattcacttcttattttgctggtttttacgaaaatagaaagaatatttattccacgaaaccgcaaagtactgcgatagcctacagattaattcatgaaaacttgcctaaatttatagataatattttggtcttccagaagattaaagaaccaatcgctaaagaacttgagcacataagagcagattttagcgcaggcggatatatcaaaaaagatgaacggctagaagacatattctcattaaattactacattcatgtcctttctcaagctggtatagaaaaatataatgctttaatcgggaagatagtgacggaaggtgatggtgaaatgaaaggtcttaatgaacatattaacttatataaccaacagaggggtcgagaggataggttgcccttgtttaggcctctatacaagcaaatcctgtccgatagagagcaattgtcttatttacctgaatcatttgaaaaagatgaagagctgcttagagcacttaaggaattttacgatcacatcgccgaagacatcttgggtagaacacagcaattgatgacttcaatttctgaatacgacttgtcccgtatttatgtcagaaatgattctcaacttacagacatctcgaagaaaatgctaggagattggaacgccatttatatggctagagaacgagcctacgaccacgaacaggctcctaaacgtattactgctaaatacgaacgtgatagaatcaaggccttaaaaggtgaagagtcaatttcattggcgaatctgaacagctgtatagctttcttggacaatgtaagggattgtcgagttgacacatacctatcaactttggggcagaaagagggtcctcatggcttaagtaacttggtggaaaacgtcttcgcctcatatcatgaagcagaacagttattgtcgtttccttaccccgaagagaacaaccttattcaggacaaagacaatgtagttttgatcaaaaacctattggataatataagtgatttacaacgtttccttaaacctttgtggggaatgggcgatgaacctgacaaagacgaaaggttttacggtgaatacaactatattagaggagcgcttgaccaggtaatacctttgtacaataaagtaaggaactacttgactcgtaaaccatattctactagaaaagttaaattgaactttggtaattcacagctgctgagtggttgggatcgtaataaagaaaaagataactcctgtgttatcttgcgaaaaggacaaaacttttacttggcaattatgaacaaccgtcacaaaaggtccttcgagaacaaagttctgcctgaatacaaagaaggtgaaccatattttgaaaaaatggactataaattcctgccagatcctaataaaatgttgcctaaggtcttcttgtctaaaaaaggtatagaaatatataaaccatccccgaagttgctggagcaatatggtcatggaacgcacaaaaaaggtgacacttttagtatggatgacttgcacgagttgattgatttttttaaacattccattgaagcgcacgaagattggaaacaatttggtttcaagttctctgacacagccacttacgaaaatgtatcgtccttttatagagaagtggaagatcagggttataaactgtcattccgtaaggttagtgaaagctatgtgtactcgttgatcgatcaagggaagctttatctttttcaaatctataataaagatttctctccttgttcaaagggcacacctaatcttcatacactatactggagaatgcttttcgatgaaagaaatttggctgatgtgatctataaattagacggtaaagctgagatttttttcagagagaaatccctgaaaaacgaccatccaactcatccggcaggtaaaccgattaaaaagaaatcccggcaaaaaaagggcgaagagagtttattcgagtatgatttagttaaggacagacattatacaatggacaaatttcaatttcatgtgcccattactatgaactttaagtgtagtgcagggtctaaggttaatgatatggtaaacgcacatattagagaagctaaagatatgcacgtcatcggtattgatcgcggagaaagaaatttactttacatttgcgttatcgattctaggggcaccatcttggatcaaatctctttgaacactataaatgatattgactatcatgatctactagagagtcgggataaagacaggcaacaagaaagaagaaattggcaaacaattgaaggtattaaagaattaaagcaaggctatctaagccaggctgtacacagaattgccgaattaatggtagcatataaagctgtcgtagctctagaagacttgaacatgggtttcaaaagagggcgccagaaggtcgaaagtagtgtttatcaacaatttgaaaaacagttaatagataagttgaattatctagtggataaaaaaaagcgtcctgaggacattggcggtttattaagagcctaccaattcactgcgccatttaaatcgttcaaagaaatgggtaaacaaaacggttttctattctacatccccgcatggaatacctcaaatatagatccaactaccggtttcgtcaacttatttcatgctcaatatgagaatgtggacaaagcaaaatcattctttcaaaaatttgatagcattagctacaatcctaaaaaagattggtttgaatttgcgttcgattataaaaatttcaccaagaaggctgaaggttccagatctatgtggatattgtgcacccacggaagtagaattaagaacttccgtaattcacagaaaaacggccagtgggacagcgaagaattcgccctaaccgaagctttcaaaagtcttttcgtaagatacgagatagactatacagctgatctaaagacagctattgtggatgagaagcaaaaagacttctttgtcgaccttcttaagttgttcaagttaactgtgcagatgagaaatagttggaaggaaaaagacctagattacttgattagcccagtcgctggtgcagatggcagattttttgatacacgtgaaggcaataaatcactaccaaaagacgcggacgctaatggcgcatacaacatcgcattgaagggtttgtgggctctcaggcagattaggcagacaagtgagggtggtaagcttaagctggcgatttctaataaggaatggttacagtttgttcaagaaagatcctacgaaaaagattaa

SEQ ID NO: 133 - DNA, 3792 bp, Artificial Sequence
  Description of Artificial Sequence: Synthetic polynucleotide
atgaacaatggtactaataattttcaaaacttcatagggatttctagccttcaaaagacattgagaaatgctttaattccaacagaaacgactcaacaattcatagtgaaaaatggtattataaaagaagacgagttgcgtggcgagaatagacaaattttgaaagatatcatggatgactactacagagggttcatctccgaaacattgtcttctattgacgacattgactggaccagcttattcgaaaaaatggaaatacagctgaagaacggagataacaaggacactcttataaaggagcaaacggaatatagaaaggctatacacaaaaagtttgctaatgacgatagatttaaaaacatgtttagtgcgaagttaatttctgatattctacccgagtttgtcattcataataataactactctgcatctgaaaaagaggagaagacccaggttataaagttgttttcaagatttgccacatcatttaaagactacttcaagaacagggcgaattgcttctctgctgatgatattagctcttccagctgtcatagaattgttaacgataatgccgaaattttttttagtaatgccttggtatatagacgcatagtcaagtcactaagcaatgatgatataaacaagattagtggtgatatgaaagatagccttaaagaaatgagccttgaagagatatattcatatgagaagtacggtgaatttataactcaagaaggaatttctttttataacgatatttgtggtaaggttaattcttttatgaatttgtattgccagaagaacaaggaaaataagaatctatataaactacaaaagttgcataaacagattttgtgtatagctgatacatcctacgaagttccgtataaatttgaatctgatgaggaagtttatcaatcggtaaacggttttcttgacaacatttccagcaaacatatcgttgagagactacgtaaaattggagacaactataatggttacaatctagataaaatatacatagtgtccaagttttatgagtctgtctctcaaaagacatatcgtgattgggagaccattaatactgcacttgaaattcattataacaacatattgcctggtaacgggaagagtaaagctgataaggttaaaaaggccgtcaaaaacgacttgcaaaagtctattaccgagataaatgaattagtgtcaaactacaaactatgctcagatgataatattaaagcggaaacatacatccacgaaatttcccacatactgaataactttgaagctcaggagcttaaatataacccggaaatacacttggttgagagcgagttaaaagcatctgagttgaaaaatgtattagacgtcatcatgaatgcgtttcattggtgttcagttttcatgactgaagaattagtcgacaaagataacaatttttatgccgaattagaggaaatatatgatgaaatttatcccgtaattagtttatacaatctagttagaaattatgttacacaaaagccgtatagtaccaagaaaataaagcttaatttcggaatacctacgcttgctgatggttggtcaaaaagtaaagaatatagcaataatgcaataattttaatgagagataacctatattatttgggtatttttaacgctaagaacaaaccagacaagaaaataattgaaggtaatacatctgaaaacaagggcgactataaaaagatgatatacaatttgctcccaggtcctaataaaatgattcctaaggttttcctgagtagcaagactggcgttgaaacttacaagcctagtgcgtatatcctggagggttataaacagaacaagcatatcaaatcctctaaggacttcgatatcaccttttgccatgacttaatcgattattttaaaaattgtatcgcaattcatccagaatggaaaaatttcggatttgattttagtgataccagcacttacgaggatatctctgggttctacagagaagtggagttgcagggctacaaaatcgattggacttacatatctgaaaaggacatagatttgctgcaggagaaaggtcagctatatttgtttcaaatctacaacaaagacttttctaaaaagtctaccggtaatgacaatctgcacacaatgtacttgaagaacttattctccgaggagaacttaaaggacattgtactcaagttgaatggagaagccgagattttttttagaaagagcagtataaagaatcctataatccacaagaagggctcaattctcgtgaataggacgtatgaggcagaagaaaaggaccaatttgggaatatacaaattgtaagaaaaaacatcccagaaaatatctaccaggaattatataagtattttaatgacaaatctgataaggaactgtctgacgaagccgctaagctcaagaatgttgtgggccaccatgaagctgctactaatatagtgaaggactacagatatacctacgataaatatttcctgcatatgccaattactataaacttcaaagcaaataaaacaggttttataaatgatagaatcctgcagtatattgctaaagaaaaggatttacatgtaattgggattgatagaggtgaacgcaatctgatctatgtcagcgtaatagatacttgtggtaatattgtggaacaaaagtcctttaatattgtgaacggatatgattaccaaatcaagttgaaacaacaagagggagcacgccaaattgcccgtaaggaatggaaagagataggtaagatcaaggaaattaaggaaggttatctttcattagttattcacgaaatttcgaagatggtaatcaaatacaacgcaataattgctatggaggacctgtcatatggatttaagaaaggtagattcaaggttgagagacaggtataccagaaatttgaaactatgttgatcaacaaattaaattacttagtctttaaggacatatcaataacggaaaacggcgggcttttaaaagggtatcaacttacatacatacctgataagttgaaaaatgtgggtcatcagtgtgggtgcatcttttatgttccagccgcttacacatcaaaaatcgatcctactactgggttcgtaaacatatttaaatttaaagatctaaccgttgatgcaaaaagagagtttatcaagaaatttgatagcattaggtacgattcagaaaaaaatctattctgttttacttttgactacaacaactttataacgcagaatacagtgatgtcaaaatcgtcctggtcagtgtatacttatggtgttagaattaagagacgtttcgtaaacggtcgtttttctaacgagtccgatacaatcgacatcactaaagatatggaaaaaactttggaaatgacagatataaactggagagatggtcacgaccttagacaagatataatcgattatgaaatcgtacagcatatttttgaaatttttcgcttaacagttcagatgcgtaactctcttagtgagctagaagatagagattatgatagacttatctcgcctgttcttaacgaaaataatatcttctatgactcggcaaaagccggtgatgcacttccaaaagatgctgatgcaaatggcgcgtactgcatcgcattgaaggggctctacgagattaaacaaatcaccgaaaactggaaagaagatggtaaattttctagggataagttgaaaatcagtaataaagattggttcgattttatacaaaataagcgatacttatag

SEQ ID NO: 134 - DNA, 3957 bp, Artificial Sequence
  Description of Artificial Sequence: Synthetic polynucleotide
atgaccaataagtttactaatcaatactcattgtctaaaacgttaagattcgagttaattccccagggaaagacactagaatttattcaagaaaaaggtcttctctctcaggataaacaaagagcagaatcataccaggagatgaaaaaaaccatagataaatttcataagtacttcatcgacttggcactatcgaacgccaagctaacacatttggaaacctacctggagttgtataataaatcggcagagacgaaaaaggaacaaaaattcaaggatgacctgaagaaggttcaagataatctgcgaaaggaaatagtgaagtcgtttagtgatggtgatgcaaagtcaatctttgctattttagacaagaaggaattaataaccgtggaacttgaaaagtggtttgaaaataacgaacagaaagatatttacttcgacgaaaaatttaaaacgtttactacgtactttacagggttccatcagaaccgcaaaaacatgtactccgttgaaccaaactctactgcaatcgcctacagattaatacacgaaaatttgcctaagtttttagaaaatgcaaaggcttttgaaaagataaagcaagtcgaatcgttacaggtaaactttcgcgaattaatgggcgaatttggagatgaaggtcttatttttgtcaatgaattagaggaaatgtttcaaattaattattataacgatgtcttgagtcagaacggcattactatctacaactcaattatcagtggtttcactaagaatgatataaaatataaaggtttgaatgaatacattaataattataatcaaactaaagataagaaggacaggcttccgaaattgaagcaattgtacaagcagattctaagtgataggattagtttgtctttcttgccagacgcatttactgatggcaagcaagtcttaaaggctatattcgatttctacaagattaacctactttcgtacacaattgaaggtcaagaagaatctcaaaatctgctgcttttgattaggcaaactatagaaaatttgtcgtcctttgacactcaaaaaatttacctgaagaatgatacacacctgactacaatatcacagcaggtctttggggatttttctgtcttctccacggccctaaactattggtatgagacaaaagttaatccaaaatttgaaacagaatatagtaaggcgaatgaaaaaaagagagaaattttggataaagcgaaggcagtattcacaaaacaagactatttttctatcgcatttctccaagaagtcttatccgaatatattttgacactcgatcacacctctgatatagttaagaaacattcgtccaactgcatcgcagattacttcaagaatcacttcgtggctaagaaagaaaacgaaacggataaaacttttgacttcattgctaacataaccgctaaataccaatgtattcagggcatattagaaaatgcagaccagtacgaagacgagttaaaacaggaccaaaagttaatagataatctaaagtttttcttagatgctatacttgagttattacattttataaagccattgcatctaaaatcggaaagtattactgaaaaagacactgcgttctatgatgtgttcgaaaattattatgaggctttatctttattgacccccctttacaacatggtccgcaattatgttactcagaagccttactctactgaaaagatcaaattaaactttgaaaatgctcagttgctgaatggttgggatgccaataaggaaggtgactacctgacgactattctaaaaaaagacggtaattatttcttagcaatcatggataaaaaacataacaaggcatttcaaaaatttccagaaggaaaagaaaactatgaaaagatggtttataaattgttgcctggagttaataaaatgttgccaaaagttttttttagcaataagaacatagcttactttaatccatctaaggaactgctcgagaactacaagaaggaaacacataaaaaaggtgatacatttaatttggaacattgccatactctgattgatttttttaaggactctcttaataaacatgaagactggaaatattttgattttcaattttcggaaactaaatcataccaagatctaagtggattttacagagaagttgaacaccaaggttataagattaacttcaagaatatagattctgaatacattgatggtcttgtaaacgagggtaaactattcctgttccaaatctactctaaggacttctcacctttttccaaaggaaaacctaatatgcatacgttgtactggaaggctctatttgaagaacaaaatttgcaaaatgtaatctacaaactgaacggccaagctgaaatattcttcagaaaagcctcaattaagccaaaaaacattattcttcataaaaagaagatcaagattgcgaagaaacattttattgataagaagaccaagacttccgaaattgtaccagtacaaacaatcaagaatctcaatatgtattatcaaggcaagataagtgagaaagagttaacccaggatgatttacgttatatagacaatttctctatattcaacgagaagaacaaaacaatagacattatcaaagataaaaggtttactgttgacaaatttcaatttcatgtgcctatcacaatgaactttaaggccacaggtggttcgtacattaatcaaactgttttagaatatctgcaaaataacccagaggtcaagatcatcggtcttgataggggtgagagacatctggtgtatctaacactcattgatcaacaaggcaacatcttgaagcaagaatcattgaacactatcacagactccaagatctcgactccatatcacaaactccttgacaataaagaaaacgaaagggatcttgccagaaaaaattggggtacagttgaaaatattaaggaactaaaagaaggttacatttcgcaagtagttcacaagattgcaacactcatgttggaagaaaacgcaatcgttgtcatggaagatttaaatttcggatttaagagaggaagatttaaagtagaaaagcaaatctaccagaagttggagaagatgttaattgacaaattgaactacttagtgctgaaagacaaacagcctcaagaattgggcggtctatacaacgctttacaactgacaaataaatttgagtcattccaaaagatgggtaagcagagtggttttttgttttatgttccggcatggaacacatccaaaatcgatccaactacaggcttcgtgaattatttctacactaaatatgaaaatgtggataaagcaaaagctttctttgagaagttcgaggcgatccgttttaacgctgaaaagaagtacttcgagttcgaggtcaaaaagtattcagattttaaccccaaggctgaaggcacccagcaagcatggactatttgcacgtacggtgagcgaatcgaaactaaaaggcaaaaggatcaaaataataagtttgtaagcacacccattaacttgacagaaaagatagaagattttcttggaaaaaaccaaattgtatatggtgacggtaactgtatcaagtcacaaattgcttctaaagacgataaggccttcttcgaaactctgctatactggtttaaaatgacgttgcaaatgagaaacagtgaaactagaactgatatcgactatttaatatcacccgtgatgaacgataatggtaccttttacaattcaagagattacgagaaattggagaaccccacactaccaaaagacgcagacgctaatggtgcctaccatattgctaaaaagggactgatgttgttgaacaagatagatcaagccgacttaactaaaaaagttgatttgtcaatttcgaatagagattggttgcaattcgtccagaaaaataagtaa

SEQ ID NO: 135 - DNA, 4017 bp, Artificial Sequence
  Description of Artificial Sequence: Synthetic polynucleotide
atggaacaggaatactacttgggtttggatatgggaactggttcagtcggttgggctgttacggactccgagtaccacgtgttgagaaaacacggaaaggctttatggggtgtcagactattcgaatcagcatcgaccgcggaagagagaagaatgtttagaacttcaagaagaaggctggatcgtaggaattggcggatagaaattttacaagaaatattcgccgaagaaatctctaaaaaagatccaggattttttctacgtatgaaggaatccaaatactatccggaagataaacgtgatattaatggcaattgtccagagttaccctatgctttatttgtggacgacgatttcaccgataaagattaccataagaagttcccaacaatttaccatctgagaaagatgttaatgaacactgaagaaaccccggatataagactggtctatctagccattcatcatatgatgaaacacaggggacacttcttgctatcaggggatataaatgaaattaaagaatttggtacaacattttctaaattattggaaaatattaaaaacgaagaattagattggaatttagaattaggcaaggaggaatacgcagttgtcgaatcgattctgaaagataacatgttgaacagatcaacgaaaaaaacaaggctgatcaaggctttaaaagcgaaatcaatatgcgaaaaagcagtattgaatttgttagctggggggactgtcaagttgtctgatattttcggattggaagaattgaatgaaacagagagaccgaagatatccttcgccgataatggctacgatgattatataggcgaagtcgaaaatgagctgggcgaacaattctacattatcgagactgccaaggctgtttatgattgggcggtgttagtcgaaatccttggcaaatacacttccatctccgaagctaaggtggcaacctacgaaaagcataaaagtgatttgcaattccttaagaaaattgtccgaaagtacttgaccaaagaagagtacaaggatattttcgtatcaacatcggacaaactgaagaattattcagcttatattggcatgacgaaaattaatggtaagaaagttgatttgcaatccaagagatgttctaaagaagaattttacgatttcattaaaaaaaatgtcctaaaaaagttggagggacaacctgaatatgagtatttaaaggaagaactggaaagagaaactttcctaccaaagcaagttaatcgtgataatggcgttattccataccaaatacacttgtacgaattaaagaagatcttgggtaacttgagggacaaaattgatttaatcaaggaaaatgaagacaaactggtacaattatttgaatttagaataccttactacgtgggccctttaaacaaaatagacgatggtaaggaagggaagttcacatgggcagtcagaaagtccaatgaaaaaatttacccatggaatttcgaaaacgttgtagatattgaagcttctgctgagaaatttattaggagaatgacaaataaatgcacttatcttatgggggaagacgtgttgcctaaagatagtttattatattcaaagtatatggtcttaaatgaattaaacaatgttaaattagatggtgaaaaactttccgtcgaattgaaacaaagattgtatacagatgtattctgcaaatatagaaaagtaactgtaaagaagattaaaaactaccttaaatgtgaaggcattatcagcggaaatgttgagatcactggtatcgatggtgattttaaggcatctttaaccgcatatcacgactttaaggaaatattgacgggtactgagcttgctaaaaaagacaaagagaacattatcaccaatatcgtgctcttcggagacgacaagaaattattgaaaaagagattgaaccgcctataccctcagattacccctaaccaattgaagaaaatctgcgctctgtcttatactggatggggtcgttttagcaagaagtttctagaagaaattactgctccggatcctgaaactggggaagtctggaatataattaccgcgctatgggaatcgaataataatttaatgcaattactatctaatgaatacagatttatggaagaagtcgaaacttacaatatgggaaaacaaacaaaaactttgagctacgaaacagtagagaatatgtatgtctcaccatctgtaaagcggcagatctggcaaaccttgaagatagttaaagaattagaaaaagtgatgaaggaaagtccaaaaagggtttttattgaaatggcccgagaaaaacaagaatctaaaaggacggaaagtaggaaaaagcaacttatagatctatataaagcctgcaaaaatgaagaaaaagattgggtaaaggaattaggtgaccaggaagagcaaaaattgagatctgacaagctgtacttgtattatacgcaaaagggccggtgtatgtattcgggtgaggtaatagaattgaaagatttatgggataacactaagtatgacattgaccatatttacccccagtctaagacaatggacgattcattaaataaccgagttcttgtcaaaaagaagtacaatgccacaaagagcgataagtacccattgaacgaaaatataagacatgaacgaaaaggtttctggaaatcattgttggacggtggatttatttccaaagaaaaatacgagagattgattagaaacactgaactatctccagaggagttagctggctttatcgaaagacaaattgttgaaactagacagtctacaaaagcagttgcagaaatcttaaaacaagtatttccagaatccgaaattgtgtacgtcaaagccggaacagtaagtagatttagaaaagactttgaattattgaaagtacgagaggttaacgacctacatcatgctaaggatgcttatttaaatatagtcgttggtaattcgtattacgtgaaattcacaaaaaacgcatcttggttcatcaaggagaatcctggtaggacatacaacttgaaaaagatgtttacatcaggatggaatatcgaaagaaatggtgaggttgcgtgggaggtaggcaagaagggaaccattgttactgtaaagcaaattatgaataaaaacaatatacttgttacgagacaggtgcacgaagccaaaggagggttgtttgaccagcaaatcatgaagaaaggtaaaggtcagatagcaataaaagagactgatgagcgtttagctagtatagaaaaatatgggggctacaataaggcagctggtgcttacttcatgttggtcgaatcaaaggataaaaaagggaagacgatccggaccatagagtttatccctctgtacttgaagaataagattgagtctgacgaaagcatcgcattgaatttcttggaaaaggggcgcggtctaaaggagccaaaaatattgttaaagaaaattaaaatagacaccctattcgacgtcgatgggtttaagatgtggcttagtggtcgtactggggacagattattattcaagtgtgccaatcagttaatccttgacgagaaaatcattgttacaatgaaaaaaattgttaagtttattcaaaggcgacaagaaaatagagaactaaagttgagtgataaggatggaatcgataatgaagtgttaatggagatttataacacttttgtcgacaaattggagaatacggtgtacagaattaggctatctgaacaggctaaaaccctaattgataaacagaaggagtttgagcgactttctcttgaagacaaatcttcaactcttttcgagatcctacatatctttcagtgtcaatcttctgcagctaatttgaaaatgattggaggtcctggtaaggctggtatattagtcatgaacaacaacatatctaagtgtaataagattagtataattaaccaatcaccgacaggtatctttgaaaatgaaattgatttacttaaa

SEQ ID NO: 136 - DNA, 3858 bp, Artificial Sequence
  Description of Artificial Sequence: Synthetic polynucleotide
atgaaatcattcgactcgttcaccaacttgtactccctgtctaaaacattgaaatttgaaatgcgacctgttggtaacacccaaaagatgttagataatgcaggagttttcgaaaaggataaactgatccagaaaaaatacggtaaaacgaaaccatatttcgataggttgcatcgggaatttatagaagaagctttgactggtgtagaattaattggcttagatgagaatttccgtactctagtcgattggcaaaaagataaaaagaacaatgttgccatgaaggcatacgaaaatagtctacaaagactaagaacagagatcgggaaaattttcaatttgaaggcagaagactgggtgaagaacaaatatccaatattgggtcttaagaataagaatactgatatattgttcgaggaggccgttttcggtattcttaaggcaagatatggtgaagagaaagacacgtttattgaagttgaggagattgataaaaccggtaagtccaaaatcaaccagatctctatcttcgacagttggaagggcttcactggttattttaagaagttcttcgaaactaggaagaacttctataaaaacgatggtacttccacggctattgctacaagaattatcgaccaaaaccttaagcgttttattgataacctatcaattgttgaaagtgttcgacagaaagtagatttggctgaaactgaaaaatcttttagtatctccttatcccagtttttctctatagatttttataataaatgtttgctgcaagatggcattgactactataataaaataattggtggagagacattgaaaaacggagagaagctgattggccttaatgagttgataaatcaatatagacaaaataataaggaccagaaaatccctttctttaaattgctagacaaacagattttgtctgaaaagatcctattcttggatgaaataaagaacgatactgaattgattgaagctttgtcccagtttgctaaaacagctgaagaaaagacaaagattgtgaaaaaattgtttgctgatttcgtagaaaacaattctaaatatgatctagcccagatttatataagtcaagaagctttcaatacaataagtaataagtggacaagtgaaacagaaacttttgctaagtatttattcgaagccatgaagtctggtaaacttgccaaatacgaaaaaaaagataacagttataaatttccagactttatagccctttcacagatgaagtctgccttattgtcgatatccttagaaggtcatttttggaaggaaaaatattataagataagcaagttccaagaaaagactaattgggaacaatttttggctatatttctatatgagttcaattcattattttccgataaaatcaacactaaggatggagagactaagcaagttggctactatttgttcgcaaaagatctgcacaatttgattctatcagaacaaatagatataccaaaagattcaaaggtaactataaaggatttcgcagattccgtcctcaccatttatcaaatggctaaatattttgccgttgaaaaaaagagagcgtggttagcagaatacgagttggactcgttttatactcagccagatactggatacttgcaattctacgataatgcatacgaagacattgtacaggtatacaataaacttagaaattacttaaccaagaagccctacagtgaagaaaaatggaagctgaactttgaaaattcgactttggcaaatggttgggataaaaataaagaaagtgacaactccgcagtgattttgcaaaagggtgggaaatattacttgggtttaatcacaaaaggccacaataagatttttgatgatagatttcaagaaaaattcatagttggtatagaaggtggcaaatacgagaaaattgtctataaattcttccctgatcaagccaaaatgttcccaaaagtttgcttttctgctaaaggattggagtttttccggcctagcgaggagatccttcgtatctacaacaatgctgaattcaaaaaaggagaaacctatagcatagattctatgcaaaaactgatagatttttataaggattgtttaacaaagtacgaaggctgggcctgctatacatttagacatttaaagcccacagaagaataccaaaataacattggtgaattctttcgggacgttgccgaagacggctataggatcgattttcaaggtatctcagatcaatatatccacgaaaagaacgagaagggtgagctgcaccttttcgaaattcataataaggactggaatttggataaggcgagagatggtaaatcgaagaccactcaaaagaacttgcatactttatattttgagtccttgttttctaatgataacgtcgtccaaaattttccaataaagttgaatggacaagcggaaattttctatcggcctaagacagagaaagacaaattagaatcaaagaaagataaaaagggaaataaagtcattgatcacaaacgatactctgagaataaaatatttttccacgtaccattgacactcaacaggactaagaatgactcttatagatttaatgctcagattaataattttttggcaaataacaaggatattaacataattggggtggatagaggtgaaaagcacttggtatattactctgtcatcactcaggcttctgatatattggaaagcgggtctctaaatgaattgaacggtgttaactacgccgaaaagctaggtaaaaaagctgaaaacagagagcaggctcggcgcgattggcaagatgttcaaggaattaaagaccttaaaaaaggctacattagtcaagtagttagaaagttagccgatcttgctattaaacataacgcaatcattattctggaggacctaaatatgcgttttaagcaagttaggggtggcatagaaaaaagtatttatcagcagcttgagaaggctttgatagataagttatcgttcctagttgacaaaggtgaaaaaaatcctgaacaagctggtcatctgttgaaagcttatcagctgagcgcaccttttgaaacatttcaaaaaatgggaaaacaaacaggtattattttctatactcaagcgagttatacaagtaaatctgacccagtgacaggatggagaccacacctttatctaaaatatttttctgctaaaaaggccaaagatgacatcgctaagtttacaaaaatagaatttgtcaacgatagatttgaattgacttacgatattaaagattttcagcaagcaaaagaatacccaaataagacagtgtggaaagtatgctccaatgtggagagatttagatgggataaaaatctcaatcaaaacaagggtggttacacacattatactaatataactgaaaatattcaagaattgtttactaagtacggaattgacataaccaaagacttactaactcagatttcaactattgacgaaaaacaaaatacctcatttttccgcgactttattttttatttcaacttgatctgtcaaattcgtaacacggatgattccgaaattgccaagaagaacggaaaagatgatttcatcctatctccagtggaaccattttttgactcaagaaaagataatggtaataagttgcctgagaacggagatgataacggcgcttataatatcgctcggaagggtattgtaattcttaataaaatatctcagtactctgaaaagaacgaaaactgcgagaaaatgaagtggggcgacttgtatgtatctaatatagattgggataatttcgttactcaagccaacgcgagacattga

SEQ ID NO: 137 - DNA, 3465 bp, Artificial Sequence
  Description of Artificial Sequence: Synthetic polynucleotide
atggaaaattttaaaaacctatatccaattaataagacacttagattcgagcttaggccatacggcaaaacactagaaaattttaagaagtcaggcctattagaaaaagacgcctttaaggcaaattccagaagatcaatgcaggcaattattgatgagaaatttaaagagactatcgaggaaaggttgaaatacactgaattctctgagtgcgatctgggaaacatgacttccaaggataaaaagattaccgataaggctgctaccaacctcaaaaagcaagtcatcttatcgtttgatgatgaaatttttaataactacttaaagccggacaaaaacattgacgccctattcaaaaatgatccgtccaaccccgtaatttcaacttttaagggttttaccacgtactttgtaaatttttttgagattcgtaaacatatcttcaaaggagaatcgtcgggttccatggcctataggataattgatgaaaatcttacgacttacttaaacaatatcgaaaagataaaaaagttaccagaagaattaaagtctcaattggaaggtattgaccaaatagacaaattaaataactataatgagttcataactcaaagcggtatcacacattacaatgaaattatcggtggtatatctaaaagtgagaacgtaaaaatacagggaataaacgaggggatcaatctatactgtcagaagaataaagtaaaattaccaagactaacgccattatacaaaatgattctgtctgatagagtttccaactcgttcgtgcttgatactatagaaaatgatactgaattaattgagatgattagcgacttgattaataaaacagaaatatctcaagacgtaataatgtcagacattcagaacattttcataaaatataaacagcttggtaatttaccggggataagttactctagcatcgtgaatgctatttgctccgattatgacaataattttggtgacggaaaaagaaaaaaatcatatgagaacgataggaagaaacaccttgaaacaaacgtatactcaattaactatatatcggaactgttaacagacaccgatgtatcatctaatataaaaatgagatataaggaacttgaacaaaattaccaggtgtgtaaggagaatttcaatgctaccaactggatgaacattaagaatattaaacagagtgaaaagacaaacttgattaaagatctactagatatactgaaatcaatacagagattctacgatctgtttgatatagttgatgaagacaaaaatcctagtgctgagttttacacgtggctaagtaaaaatgcggaaaagttagatttcgagttcaactctgtttataataaatctaggaattatttaactagaaagcagtattctgataaaaagataaaattgaacttcgactcccctacgttggcaaagggttgggatgcaaacaaagaaatcgataactccaccataataatgcgtaagtttaacaatgataggggggattacgattattttttgggaatttggaacaaatctaccccagcgaatgaaaaaattattccccttgaagacaatggtctttttgaaaaaatgcagtataaattatatccagacccatccaagatgcttccaaagcaatttctgtcaaaaatttggaaggctaaacaccctactactcctgaatttgataagaagtataaggagggccgacacaaaaagggtccagattttgaaaaagaattcctgcatgaattgatagattgttttaagcatggtttggtaaatcatgatgaaaaatatcaggatgtctttggattcaatttgagaaatacagaggattacaactcatatacagaatttctcgaggacgtcgaacgttgcaattataatctcagtttcaacaagatcgcagacacttcaaacttaattaacgacggaaaattgtacgtttttcaaatctggtcgaaagactttagtattgattcaaagggtacaaaaaacctaaatacaatatatttcgaaagtctattctcggaagaaaacatgatcgaaaaaatgttcaaactgtcaggcgaagctgaaatattctaccgtcccgcaagccttaattattgtgaggatatcattaaaaaaggacatcaccatgcagagttaaaagataaattcgattacccaataattaaagataaaagatactcccaggataagttctttttccatgtacctatggttattaactacaagtcggaaaaactaaactcgaagtcattaaataatagaactaacgagaacttgggacaattcacacatataattggtattgatcgtggcgaaagacatttaatatatctgactgttgttgatgtttcaacaggagaaattgttgaacagaaacatcttgatgaaattataaacacagatacaaaaggcgttgagcataaaactcattatctaaataaattggaggaaaagtcgaagactcgcgataacgagagaaagagttgggaagcaattgaaaccataaaagagcttaaagaaggttacattagtcacgtcatcaatgaaatacaaaagttacaagaaaagtataacgctttgattgtaatggaaaatctaaattatggttttaagaattcaagaatcaaagtcgaaaagcaggtctatcagaaatttgaaacggcacttattaaaaagtttaactacattattgataaaaaggacccagaaacttatattcatggttaccaactgacgaacccaatcacaacattggacaaaattggaaaccaaagtggaattgttttatacattccagcttggaatacatccaaaatagaccctgtcacggggtttgtcaacttgttatatgccgacgatttaaagtataaaaaccaagaacaagcaaagtcttttattcaaaagattgataatatttatttcgaaaacggtgaatttaaattcgacatagatttttctaaatggaacaaccgttattcaataagtaaaactaaatggacactcacctcatacggcactcgtatccaaacctttcggaatccccaaaaaaataacaaatgggattctgcagaatacgacttgaccgaggaatttaaattaattcttaatatagacggtacactcaaaagtcaagacgtggagacatacaagaagtttatgtcgttattcaagcttatgcttcagttgaggaactccgttacaggcactgatattgattacatgatttcaccagtaacggataagactgggactcatttcgattctagggaaaatattaaaaatttacctgctgacgcagacgcaaacggcgcatacaatatagcaagaaaagggattatggccattgagaatattatgaatggcatatcagatccattaaagataagcaatgaagactacttaaaatacattcagaatcagcaagaataa

SEQ ID NO: 138 - DNA, 3924 bp, Artificial Sequence
  Description of Artificial Sequence: Synthetic polynucleotide
atgacccagtttgaaggtttcaccaatttgtaccaagtaagtaaaaccttgaggttcgaattgatcccacagggcaagacattgaagcatattcaagagcaaggatttatagaagaagataaagcgagaaacgatcactataaagagttaaaacccattattgacaggatctataaaacatacgccgatcaatgccttcaattagtgcaattagattgggaaaacttgagcgctgccatcgattcctacaggaaggaaaaaacagaagaaacaagaaatgccttaatcgaggaacaagcaacctatagaaacgctatacacgattacttcatcggtagaactgataatctaacagatgcaataaataagagacatgctgagatatataaaggactatttaaagcagaattattcaacggaaaggtgttgaaacagttaggtaccgttacaactactgagcatgaaaatgccttgctgagaagctttgacaagtttactacctacttttcgggtttctacgaaaatcgcaaaaatgtattttctgcggaagatatttcaactgcaatccctcataggattgttcaagataatttccctaagtttaaagagaactgtcacatttttacaaggttaattactgcggttccaagtctaagagaacattttgagaatgtaaaaaaagcgattggtatatttgtatccactagcattgaagaggttttcagcttccctttttataaccaattacttacccaaacacagatcgacctgtacaaccaattgttaggtggtatatcgagggaggctggtacggaaaagattaaaggattaaatgaagttcttaatttggccatacaaaaaaatgatgaaaccgcgcacattatcgcatctttaccacataggtttataccgttattcaagcaaatattatctgatcgtaataccttatcgttcatattagaggagtttaaatctgacgaagaagttatacaatctttttgcaagtataagacgctattgagaaacgaaaacgttctggaaacagccgaagcactgttcaatgaattaaacagtatcgacttgactcatatttttatatcgcataaaaagttggagacaatttcttcagcattgtgcgatcactgggacactttaaggaacgcactatatgaacgtaggatctcagaattgacaggtaagataacgaagtctgctaaagagaaagtgcagagatccctaaaacacgaggatataaatttgcaggagataatttcagctgcaggtaaagagttgtctgaagcgttcaagcaaaagacttccgaaatcttgtcacacgcacacgccgcattagatcaacctttacccactactttgaaaaaacaagaagagaaggagatattaaaatcacaacttgattctttacttggcctttatcatcttttagattggttcgctgttgacgagagcaatgaagtggatccagagttttccgcaagattgaccggtataaagttggaaatggaaccttcgttatcattttacaacaaagctaggaactatgctacaaaaaaaccttattctgtcgaaaaatttaaactgaacttccaaatgcctactctagcaagtggctgggatgttaataaagaaaagaacaatggcgctattttgtttgtaaaaaatggcctatactatcttggaattatgcctaaacaaaaaggtcgctacaaggctttgtcatttgaacctactgaaaagactagcgaaggtttcgataagatgtattacgattatttcccggatgccgctaaaatgatccccaagtgctctactcaattgaaggcagtaactgctcatttccaaacgcataccacgccaatactgctttctaacaactttatagaaccactagaaataacgaaagaaatttacgacctaaataacccagagaaagaaccaaaaaagttccagacggcctacgccaaaaagacaggggaccaaaaaggttaccgcgaggcgttatgtaaatggattgattttactagggactttttatcaaaatacactaaaacgacgtctattgatcttagctccttacgcccgtcctcccaatacaaggatctaggtgagtattacgcagagttgaacccgctattataccatatttccttccaaaggattgctgaaaaggaaattatggacgctgttgaaactgggaaattgtacctgtttcagatttataataaggacttcgcaaagggtcaccatggtaagcctaaccttcacactttgtactggaccggactattctcgcctgaaaatttggctaaaacaagtatcaagttaaacggtcaggccgagttattttatagacccaaatctagaatgaaaagaatggcccatagattaggcgaaaagatgttaaacaagaaattaaaggaccaaaaaaccccgataccagacactctataccaagaactgtacgactatgtgaatcacaggcttagtcacgatttatcagatgaagcgagggctttattgccaaatgtcatcaccaaggaagtatcacatgaaataattaaggatagaaggttcacatctgataaattcttttttcatgtcccaattacattgaattatcaagcagcgaactcaccatctaaatttaatcagcgcgtcaacgcctatttgaaagaacatcccgaaacaccaatcatcggcatagatcgaggtgagagaaacttaatatatataactgtgattgattctacaggaaaaatcctggagcaacgatctttaaataccatacaacagtttgattatcaaaaaaagttggataacagagaaaaagaacgtgttgccgctaggcaggcttggtctgtggtaggaacaattaaggacttaaagcagggctatctgtcccaagttattcatgaaatagtcgatctgatgatacattatcaggcagttgtcgtgttggaaaatttgaattttggctttaaatcaaaaagaactggcatagcagaaaaagctgtgtaccagcagtttgaaaagatgttaatcgataagctaaactgccttgttcttaaagattaccccgcagaaaaagtaggtggtgttcttaatccatatcagttgacagaccaatttacatcctttgcgaaaatgggtacgcaaagcgggttcttattctacgtaccggccccctatacttctaagatcgacccactaacaggttttgtggacccttttgtttggaagacgataaagaaccacgagtcacgcaaacatttcttagagggctttgatttcttgcactacgacgtgaaaactggtgattttatcttacactttaaaatgaacagaaatctctctttccaacgtggactgcccggattcatgccggcttgggacatcgtttttgaaaagaatgaaacgcagtttgacgccaaaggtacaccatttatagcgggtaagagaattgtgccggtcatagaaaaccatagatttacaggtagatatagggatctgtaccctgctaatgaattgattgcattactcgaagagaaaggaattgtgtttcgagatggatcgaatattttacctaagttgttggaaaatgatgattcacacgcaattgatactatggttgccctcataagatcggtattgcaaatgagaaactcaaatgctgctacgggagaggattatataaacagccccgttcgcgatcttaatggtgtttgttttgattcacgttttcagaaccccgaatggccaatggatgccgacgcaaacggagcatatcatattgctcttaaaggccaactactattaaatcacttaaaggaatccaaagacctaaaattgcaaaacgggatatctaatcaggattggctggcttacatacaagaactacgtaactag

SEQ ID NO: 139 - DNA, 3390 bp, Artificial Sequence
  Description of Artificial Sequence: Synthetic polynucleotide
atggccgttaagtcaatcaaagtgaaacttagactggatgacatgccagagattcgtgcggggttatggaaacttcataaggaagttaacgcaggggtaagatattataccgaatggttatcattacttcgacaagagaatttgtacagaaggtccccgaacggcgacggtgagcaagaatgcgataagacggctgaagaatgtaaggcagaacttttggagcgcctgagagcccgtcaggttgaaaatggccatagaggtcctgcgggatctgatgatgagcttttacagctagctagacaattgtatgaattgttggtccctcaggctattggggctaaaggagacgctcaacaaatcgccagaaagttcttgtcacctctggctgacaaagatgccgtgggaggattaggtatcgctaaagcaggtaataaaccaagatgggttagaatgagagaagcaggcgaacctggttgggaagaagagaaagaaaaggccgaaactagaaaaagcgctgacagaaccgcagatgttttacgggccttggctgattttggactgaagcctttgatgagagtgtatactgattcagaaatgtcttccgttgaatggaagcccctaaggaagggacaagcggtcagaacctgggatagggatatgtttcaacaggctattgaaaggatgatgtcatgggaatcctggaatcaaagagtaggtcaagaatacgctaaactggtcgaacaaaagaatagatttgaacaaaaaaattttgtaggtcaagaacatttagtacatttggttaatcaacttcaacaagatatgaaagaggcatctcctggtttggaatcaaaagaacaaacagcacactatgttaccggccgagctttgcgaggttctgacaaagtatttgaaaagtgggggaaattagctcccgatgccccctttgatctatatgatgctgaaattaaaaacgttcaaagaaggaacactagacgttttggatcccatgatctttttgcaaagctagctgagccagaataccaggctctatggcgtgaagacgcctcgtttttgactagatacgcagtatacaattcaatactcagaaaactaaaccatgccaagatgtttgctacattcaccctgcccgatgctaccgctcatcctatttggactagatttgacaagttgggggggaatctacatcagtacacatttttatttaatgaattcggtgaaagaagacacgctattagattccacaagctcctaaaggttgaaaacggcgttgcgagagaagttgatgatgtaacagttcccatttctatgtcggagcaattggataatctattgcctagagaccctaatgaaccaattgctttgtactttcgtgactacggtgcagaacaacactttacaggtgaattcggcggagccaagattcaatgtagacgtgatcaactcgcacacatgcatagaagaagaggcgctcgtgatgtttatttaaatgtgtctgttagagttcaatcccaatcggaggctagaggtgaaagaaggccaccatacgcagcagtttttaggttagtaggtgataatcatagggcatttgtccacttcgacaaattaagtgattatttagcagagcaccctgatgatggaaagttgggcagtgagggattattaagtgggttgagggtaatgtctgtagatcttggtcttcgtacttctgcgagtatctctgtctttagagtagcacgtaaggatgagttgaaacctaatagcaaaggaagagtcccgtttttttttcctattaagggtaacgataacctggtggccgtgcatgaaagatcacaacttttgaaattgccaggagaaacggagtccaaggacttgagggcaattagagaggaacgtcagcgtacattgcgacagctgagaactcaattggcttatttgaggttgttggttaggtgtggttccgaggatgttggcagaagagaaaggtcttgggccaaattgatagaacaaccagtggacgccgcaaatcacatgacaccagattggagagaagctttcgaaaatgaactccagaaattaaagagcctacatggcatatgctctgataaagagtggatggatgccgtatacgaatccgttcgtagagtctggcgccacatgggtaagcaagtacgggactggagaaaggatgttcgttccggcgaaagaccgaagataagggggtatgcaaaggacgttgtaggcggtaattctattgaacagattgagtatttggaaaggcagtacaaatttcttaaatcctggagcttcttcggcaaagtgtcaggacaagtcatcagggctgaaaaaggttccagatttgctattacgctaagggaacatattgatcatgcgaaagaagatagactgaaaaaactagcagatagaataattatggaagcacttggttacgtctatgcacttgatgaaagaggcaaggggaaatgggtagctaaatacccgccttgtcaacttattttattagaagaattaagcgagtaccaatttaacaacgatagacctccatccgaaaataatcagctgatgcaatggtcccataggggtgtttttcaagaattgataaatcaagctcaagtacacgatttgctggtaggtactatgtacgcagcgttttcgagccgttttgatgcaagaactggtgccccaggtatcagatgtcgacgtgttccggccagatgtacacaggaacataaccctgagccatttccgtggtggcttaataagtttgttgtcgagcacacattagacgcatgccctctgagagcagatgaccttatacccactggagaaggcgaaatatttgttagtccattctctgcagaagaaggtgactttcaccagatacatgcagacttaaatgcagcacagaatctccaacaaaggttgtggtcggattttgatatttcgcaaataagactaagatgcgattggggagaggttgatggagaattggtgctgattccaagattaaccggaaagcgaactgccgattcctattctaacaaggtgttttacacaaatactggtgttacctattacgaaagagaaaggggtaagaagagacgtaaagtatttgctcaagaaaaattgtcagaagaggaggcagaactgttagtagaagcagacgaagccagagaaaaatcagttgtgcttatgcgtgacccttccggcattataaatcgtggtaattggacacgacaaaaagaattttggtctatggtcaatcaacgtatcgaaggctacctagttaagcaaatcaggtctagggttccactacaagatagcgcatgtgaaaatacgggtgatatataa

SEQ ID NO: 140 - DNA, 3327 bp, Artificial Sequence
  Description of Artificial Sequence: Synthetic polynucleotide
atggctactagatctttcattttaaaaattgaacctaatgaagaagtgaagaagggtctctggaaaactcacgaagtacttaatcatggcattgcctattatatgaatatcctgaagcttattcgtcaagaagctatatacgagcatcatgagcaagatcctaagaaccctaagaaagtaagcaaagcggaaattcaggctgaattgtgggacttcgtcttgaagatgcagaagtgtaacagttttacgcacgaagttgataaagatgtggtgtttaatattttgagggagctatatgaggagttggtgccctcgagtgtcgaaaaaaaaggagaagctaatcagctgtcaaataaatttttatatcctctggtggatccaaactctcaatcaggtaaaggcactgccagtagtggtcgaaaaccgagatggtataatttgaaaatcgcaggtgatccatcgtgggaagaagaaaaaaaaaaatgggaagaagataaaaaaaaagatccccttgccaaaatactaggtaagctagccgagtatggacttataccattattcattcctttcacggactctaatgaaccaattgtgaaggaaatcaaatggatggaaaaatcacgtaatcagtctgttaggaggttggacaaagatatgtttatacaggctcttgagaggtttttgtcgtgggagtcctggaatttgaaagtgaaagaagaatatgaaaaagtggaaaaggagcataagacgttggaagaaaggattaaggaagatattcaggcctttaagagtctggaacagtacgaaaaagaaagacaggaacagttattgagagatactctaaacactaatgaatataggctttccaagaggggcttgcgaggatggagagagataattcagaaatggttgaaaatggatgagaacgagccatcggagaaatatctagaggtgtttaaagattaccaaagaaagcaccctcgcgaagctggtgattactctgtttatgaattcctttcgaagaaggaaaatcacttcatctggcgaaatcatccagagtacccatatttatatgctacattttgcgaaattgacaagaaaaaaaaagatgctaaacagcaagcgacattcaccctcgctgatcccatcaaccacccattatgggtcaggttcgaagagagatcaggctcgaacctgaataagtacaggatcttgactgagcaattgcatactgagaagttaaaaaagaaattgacggtccaacttgacagattgatttatcccactgaatctggtggatgggaggagaaaggtaaggttgatattgtcctattgccttctcgtcaattttacaaccaaatatttctggacatcgaagagaagggtaaacatgcttttacctataaggatgagagtattaaatttccattgaagggaacgcttggcggcgctagagttcagttcgatagagatcatttgagaagatacccgcataaagtggaatctggtaatgtaggtcggatctactttaacatgacggtaaatattgaacctaccgagtcaccagtcagtaagtctttaaagattcatagggatgatttccctaaatttgtcaacttcaagcctaaggaactaaccgagtggatcaaagacagtaaaggcaaaaagttaaagagcggtattgagtccctggagataggtcttagagtcatgtctatcgatttgggtcaaagacaagcagccgcagcatctattttcgaagttgttgaccaaaaaccggatatcgaggggaaattattttttccaataaaaggaactgagctatacgctgtgcatcgcgcatccttcaatataaaactgccaggagaaacactagtaaaatctagagaggtcttgcgtaaagcacgtgaggacaatctcaaattaatgaatcagaagttaaatttccttaggaacgtgttgcatttccaacagttcgaggacataactgaacgcgagaaaagagtcactaagtggatctcaagacaagaaaatagtgatgtgccattagtgtatcaagacgaacttattcaaataagagagctaatgtataaaccatataaagactgggtggcattcttaaaacaattacacaagcggcttgaagtagaaataggaaaagaagtaaagcattggaggaagagtctgtccgatggtcgcaaaggcctgtacgggatatcacttaaaaatattgatgaaattgacagaacacgaaaatttttgttaagatggtcattgagaccaaccgaaccaggtgaggttagaaggttggaaccaggccaaaggtttgccatcgatcaattaaaccatcttaacgcactgaaagaagatagattgaagaagatggcgaacactattattatgcacgctctaggttattgctatgatgtgagaaagaaaaaatggcaagccaagaaccctgcatgccaaattattttgtttgaagatctttctaattacaatccatacgaagagcgttcacgttttgaaaactctaaattgatgaaatggtctagaagagagattccgagacaggtcgctctacaaggggagatttacggtcttcaagtcggtgaggttggtgctcaattttcttccagatttcatgcaaaaactgggtctccaggcattaggtgttcggtcgttactaaggaaaagttacaggacaaccgtttcttcaaaaatttgcaacgtgaaggccgtttaacacttgataagatagctgtccttaaggaaggcgatctgtacccagataaaggtggtgagaaattcatatctttgagtaaagacaggaaactggttacaacacacgccgacattaacgcagctcagaacttgcaaaagagattctggacaaggacccacggcttctataaggtgtactgtaaagcttatcaagtagatggacaaacggtttatattcctgaatcaaaggaccagaaacaaaaaattatagaagaatttggtgaaggatactttatcttgaaggatggagtttatgagtggggcaatgcaggtaagttaaagataaagaaaggttcatcaaagcaatcaagtagcgaactggtcgattcggatattttaaaggatagctttgatctagctagtgaattgaagggagaaaagttaatgttatacagagatcccagtgggaatgtatttccatctgataagtggatggccgccggagtgttttttggcaaattagagagaatcttgatttctaaactgaccaatcaatactcaatttcgaccatcgaagacgactcttcaaaacaatccatgtga

SEQ ID NO: 141 - DNA, 3450 bp, Artificial Sequence
  Description of Artificial Sequence: Synthetic polynucleotide
atgcctactcgcaccatcaatctgaagttagttttggggaagaacccagaaaatgcgactctaagacgggcactattctctacacatagacttgtcaaccaagcgactaagagaattgaagaatttttactgttgtgtagaggagaagcttatcgtaccgtagataatgaaggtaaagaagctgagatcccacgccatgctgttcaagaagaggcgcttgcttttgcaaaagctgcacaacgacataacggctgtatctccacatatgaggaccaggaaatcttggatgtgcttagacaattgtatgaaagattagtacctagcgtcaatgaaaacaacgaggctggggatgcccaagccgctaacgcttgggtgagtccattaatgagtgcagagtccgaaggtggactatcggtctatgataaagtgttagacccgccgccagtatggatgaaactcaaagaagagaaagcgcctggttgggaagctgcttctcagatttggatacagtccgacgaaggtcaatcgctgctaaataaaccgggtagcccaccacgttggattagaaaacttagatctggtcaaccgtggcaagatgacttcgtttcagaccaaaaaaaaaagcaagatgaactaacgaaaggtaacgcaccactcataaaacaattgaaagagatgggcctcttgcctttagttaatcccttttttagacatttgttggatcccgagggtaagggtgtatccccatgggacagattggccgtaagggccgcggtggcgcacttcatctcttgggaaagttggaaccacagaacaagagctgagtataacagtttgaaactgcgaagagatgaatttgaggccgcatctgatgaattcaaggacgattttacattgctacgacaatatgaggctaagcgacatagtacgcttaagtcaattgccttagctgatgactctaacccgtaccgaattggtgtaaggtccttgagagcctggaatagggttagagaagaatggattgacaaaggcgcaaccgaggaacaaagggttaccatccttagtaagcttcaaacacaattacggggtaaattcggtgatccagacctatttaattggctagcccaagatagacacgtacacctgtggtccccgagagattccgtcacgcccctcgtaaggattaatgccgtcgacaaagtgcttagaagacgtaagccttatgcactgatgacttttgcacatccgagattccatccaagatggattctatacgaagcgcctggtggttctaacttgcgacaatacgctttagattgtactgaaaatgctctgcatattacacttccattactcgtcgacgacgcccatggtacatggattgagaaaaaaatccgcgtaccactcgctcctagtggacaaatacaagatttaactttagaaaaacttgaaaagaaaaaaaacagattatactatagatcaggattccaacaatttgctggattagccggtggtgctgaggtgttgtttcataggccgtatatggaacatgatgagagatcagaagaatctctgttggaaaggccaggcgctgtgtggttcaaattaaccttagatgttgctacccaagcaccacctaactggttagatggtaaaggcagagttaggacacctccagaagttcatcatttcaaaaccgctctgtcaaataaatctaaacatacgagaaccttgcaaccaggattgagagtcctttctgttgatttgggtatgagaacatttgcttcttgttctgttttcgaattgatcgaaggtaaacctgaaacaggtagagcattccctgttgctgacgaaagatcaatggatagtccaaataagttatgggccaagcacgagagaagctttaaactaactctgcctggagaaacaccgagcagaaaggaggaagaagagagaagcattgctagggcagagatttacgcgctgaaaagagatattcaaagactgaaatcactcctaagattaggtgaggaagataatgataatagaagagatgctttgttagagcaattctttaaaggatggggtgaagaggacgtagttcctggtcaagctttccctagaagcctctttcagggattaggcgctgcaccctttaggtcaacacccgaattgtggagacagcactgtcagacgtattacgacaaagcggaagcttgcctggcaaagcatatttccgactggaggaagagaactagacctcgtccgacttcgagagagatgtggtataagacaagatcttaccatggtggcaaaagtatttggatgctagaatacttagatgctgtccgcaaattactactttcatggtcgttaagaggtcgtacttacggagctattaatagacaagacaccgctcgttttggttccttagcttctagattgttgcatcatatcaactctttaaaggaagaccgcatcaaaaccggtgcagatagtattgtgcaggccgcaaggggctatattcctctcccacatggcaagggttgggaacagcgttatgaaccctgtcagttgatattatttgaagatctagctaggtacagatttcgtgtagacagacctcggagagagaattcgcaattgatgcagtggaatcatcgagctatagtagcagaaacgacgatgcaagctgaactatacggtcaaatagtcgaaaataccgctgctggtttctcctcaagatttcatgctgcaactggtgctcctggtgtcagatgtcgctttttgttagaacgagatttcgataatgacctaccaaagccgtacttactgagagaactaagttggatgttaggtaacacaaaggttgaatcagaggaagaaaaattgcgtcttctaagcgagaaaattagaccaggttcattagtcccttgggatgggggtgaacaattcgcgacattacacccgaaaagacaaactctttgtgtcattcacgcagatatgaacgctgctcaaaacctgcaacgcagatttttcggaaggtgtggggaagcctttcgccttgtgtgtcagccacatggtgatgatgttttgaggctagcgtctacaccaggtgcaagacttttgggtgcattacaacaactggaaaatggtcagggagctttcgaattagttcgtgatatgggtagcacatcacaaatgaatcgtttcgtcatgaagtcgttgggcaaaaaaaagatcaagccattacaagacaataacggggatgatgaactagaagacgtgctatctgttttacctgaagaagatgataccggacgaattactgtatttcgggactcttcgggtatattcttcccttgtaacgtttggatcccggcaaaacagttctggcctgcggtccgtgctatgatttggaaggttatggcatcacattcattgggttag

SEQ ID NO: 142 - DNA, 3759 bp, Artificial Sequence
  Description of Artificial Sequence: Synthetic polynucleotide
atgacaaagttaaggcatagacagaagaagttaactcacgattgggcggggtctaaaaagagagaagttctagggagcaatggtaaattacagaatccattgctaatgcccgtcaaaaaaggtcaggtgacagaatttcgaaaagcattttccgcatacgcccgagcaaccaaaggggaaatgacggatggcagaaaaaatatgtttactcactcatttgaaccattcaagaccaagccttcgttacatcagtgcgaactggctgacaaagcctaccagagcttgcattcatatttaccgggttctttggcgcattttcttttatctgcccatgcacttggttttaggatttttagcaaatcaggggaagccactgcattccaagcgtcctcaaagattgaagcttacgaaagcaagttagctagcgagcttgcttgtgttgatttgtctattcagaacttgactatttcaactttgttcaacgcattaacgacttccgtaagaggtaaaggtgaggagacatcggcagatccactgatagctagattttacaccttacttaccggtaaaccactaagcagagacactcagggcccagaacgagatttagccgaggtgataagcagaaaaattgcaagttcttttggaacttggaaggagatgactgccaatccacttcaatctcttcaattttttgaagaggagttgcatgcgctagatgcaaatgttagtttgtcacctgccttcgatgttctgattaagatgaacgacctgcagggtgacttgaagaacagaacgatagtttttgatccagatgctcctgtgtttgaatataatgctgaggatcctgctgacatcatcattaaactgacagctagatatgcgaaagaagcagtgattaaaaatcaaaatgtcgggaattatgttaagaacgctattacgacaactaacgcaaacggactaggttggttgctgaacaaaggcctttccttattgcctgtctccactgatgacgaactattggagtttattggggtcgagagatcccatcctagctgtcatgcgttgatagaacttatcgctcagttagaagcacctgaactgttcgaaaaaaatgttttttctgatactcgttccgaggttcaaggtatgatagattcagctgtaagcaatcatatcgccaggctgtcaagctctcgtaattcattgagcatggactcagaggaacttgagagattgataaaatcttttcaaattcatacaccacattgttcattatttataggggctcaatccttatctcaacaattggaaagcctacccgaagcattgcagtcaggagtgaacagtgctgatattctgctcggctcaacccaatacatgttgacaaattctttggtcgaggagtcaatcgctacgtatcagagaaccttaaatagaattaactacctgtccggcgttgcaggacagattaacggtgctattaagaggaaagctattgatggtgagaagatacatttacccgctgcttggtcagagttaatttctttaccctttattgggcaaccagtgattgatgttgaatcagatttagcccacttaaagaaccaataccagacattgtctaacgaatttgatacgctgatttccgcactgcaaaagaatttcgacttaaattttaataaagccttgcttaatcgaacacaacatttcgaggctatgtgtagatcaacaaaaaagaatgccctttctaagcctgagatcgttagttatagagatttgctagccaggttgacttcttgtctttataggggctctctagtcttgaggagggcgggtatagaagtactgaaaaagcacaagatatttgagtccaactctgaattaagagagcacgttcatgaaagaaaacacttcgtatttgtttctccgctcgatagaaaagccaagaagctcctacgtttgactgactctaggcctgatttattgcacgtaattgatgaaatactacaacatgataatttagagaacaaggatagagaatctttgtggttagttcgatctggttatttactggccggcctaccagaccaactctcctcttcctttataaatcttccaatcattactcaaaaaggcgatcgtcgcttgatagatctcattcaatacgaccaaattaatagagatgcttttgtgatgttggtaacttccgcttttaagtcgaacttaagtgggctgcagtacagagcaaacaaacaatcttttgtggttacgcgcactttgtcaccatatttgggatctaaattggtttatgtgcccaaagataaagattggctggtcccttcccaaatgttcgaggggagatttgcggacattttgcaatccgattatatggtgtggaaggacgctggaagattgtgtgttattgacacagctaagcatttgtctaacattaaaaaatctgtattctcaagtgaagaagtcctcgcgtttttaagagaattgccacaccgtacgtttatccaaactgaggtcaggggtttaggggtgaatgtggacggtattgcatttaataacggggatataccctctctgaagacgtttagcaattgcgtgcaagtcaaagtgagtcggacaaacactagtctggtccaaacattaaatagatggtttgaaggcggtaaggtctcgccgcctagcatccaatttgagagagcatattacaaaaaagatgatcaaatccacgaggacgctgcaaaaaggaagataaggtttcaaatgccagctacagagttggtacacgcgtcagacgacgcaggatggaccccctcctatttacttggtatcgatcccggtgaatatggtatgggtttgtcattggtctcaataaataatggcgaagttttagatagcggatttatacacataaattcattgataaatttcgcttctaagaaatcaaatcatcaaaccaaagttgttccgaggcagcaatacaagtcaccatacgccaactatctagaacaatctaaagattctgcagcaggagacatagctcatattttggatagacttatctacaagttgaacgccctacccgttttcgaagctctatctggcaatagtcaaagcgcagcggatcaggtttggacaaaagtcctcagcttctacacctggggagataatgatgcacaaaattcaattcgtaagcaacattggttcggtgcttcacactgggacattaaaggcatgttgaggcaaccgccaacagaaaaaaagcccaaaccatacattgcctttcccggttcacaagtttcttcttatggtaattctcaaaggtgttcatgttgtggacgtaacccaattgaacaattgcgcgaaatggcgaaggacacatccattaaggagttgaagattagaaattcagaaattcaattgttcgacggtactataaagttatttaatccagacccgtcaacggtcatagaaagaagaagacataatttagggccatcaagaattcctgtagctgatagaactttcaaaaatataagtccaagctcactagaattcaaagaactaataacgattgtgtcacggtctatacgtcattccccagaatttattgctaaaaaaagaggtataggtagtgagtacttttgtgcttatagtgattgtaattcctccttaaattcagaagcaaatgcggctgcgaacgttgcccaaaagttccaaaagcaattgtttttcgaattatag

SEQ ID NO: 143 - DNA, 3864 bp, Artificial Sequence
  Description of Artificial Sequence: Synthetic polynucleotide
atgaaaagaatcttgaactctttaaaggttgccgccctgcgtttgttatttagaggtaaaggatctgaacttgtcaagactgttaaataccctttggtctcgccggttcagggtgcagttgaggagttagctgaggcgatccgccatgataacctacatctgtttggtcaaaaagaaattgttgaccttatggaaaaggatgaaggtacgcaagtttactcagtggttgatttctggttagatacccttcgtttggggatgtttttcagtccatcagcaaacgcattaaaaatcacgctgggtaagtttaattctgatcaggttagcccttttaggaaagtgttagagcagtctccattcttcttggctggtaggctgaaggttgaaccggcagaacgtatattatctgtcgagatccgtaagattgggaagagggaaaacagagttgagaactatgctgctgacgtagaaacgtgttttataggccaattaagttcagatgagaaacagtcaatacaaaaattagctaatgatatctgggatagtaaagatcatgaagagcaaagaatgttaaaggcagatttcttcgctatccctttgattaaggatccaaaggctgtgaccgaagaggatcctgaaaatgaaactgctggtaaacaaaaacccttggagttgtgtgtctgccttgtcccagaactttacacaagaggattcgggtcaatagccgattttttggttcaacgcttaactcttttaagggataaaatgtctacagatactgcagaagattgtttagaatatgtcgggattgaggaggaaaaaggtaacggcatgaactcattgttgggaacgttcttaaagaatttgcaaggcgatggatttgagcagattttccaatttatgttagggagctatgtcggttggcaagggaaggaagatgttttaagagagagattagacttattggctgaaaaagtgaagaggttaccgaaaccaaaatttgctggcgaatggtctggtcataggatgttcttgcatggccaattgaagtcttggtcttcaaatttttttagactatttaacgagacaagggaacttctagagtctattaagtcagatatacagcatgccacaatgctaatatcatatgtagaagaaaaaggtggttatcatcctcaattacttagtcaatatagaaaacttatggaacaactaccagctttgcgtaccaaggtattggaccctgagattgaaatgacacatatgtccgaagcagttcgctcttatataatgatacataaatctgttgcgggttttttaccggatttattagaatcattagatagagacaaggatcgtgagtttctgcttagtatttttccaagaatcccaaaaattgataaaaaaaccaaggaaattgtagcttgggaactgccgggagaaccagaagaaggttatttatttactgctaataacttgttcagaaacttcttagagaatccgaaacatgtcccgagatttatggccgaaaggatcccagaagattggactcgattacgctctgctcctgtctggttcgatggaatggtaaaacaatggcaaaaagtcgttaaccagttagtagaatcaccaggtgctttatatcaatttaacgaatccttcttgagacaaaggttacaggccatgttaactgtgtataagagggacttacaaactgaaaaatttcttaaacttttggcggatgtttgtaggcctcttgtagatttttttggtttgggtggaaatgatattatttttaagagctgtcaagacccaagaaaacaatggcaaaccgttattcctctctctgttccggcagatgtctatactgcttgcgaaggtttggcgattagactaagggagacattaggattcgaatggaagaatttgaaaggtcacgagagagaagatttcttaagattgcaccagttattgggcaatttacttttctggattcgtgatgctaaattggtagtaaaattagaggattggatgaacaacccatgtgttcaggaatatgtagaagcccggaaagctatcgatcttccactagaaatattcggttttgaagtgcctatcttcctgaatggctatctattttcggagttgagacaattagaacttttgcttaggagaaaaagtgtgatgactagctacagtgtaaagactactggatctcctaataggctatttcagctagtttatttacctctaaaccctagtgaccccgaaaagaagaactcaaataactttcaagaacgtttggataccccaactggtttgtcccgtcgtttcctagacctaacccttgatgcattcgcaggtaagttacttaccgatccagttacacaagaattgaagacaatggcaggtttttacgatcatctttttggattcaaattgccatgtaaactcgccgccatgtcgaatcatccaggttcttcttcaaagatggttgtgttagcgaaacccaaaaaaggtgttgcttctaatatagggtttgaaccgatcccagatcccgctcatcccgtatttagggttagatccagttggccagagttgaagtacctcgaggggctattgtatttgccagaagacacacctttgaccatcgaattagcagagacctccgtatcgtgccaaagtgtctcgtcagttgcattcgatttgaaaaacttgacaacgatcttaggtcgtgtgggagaatttagggtcacagctgatcaaccctttaaactaacgcctataatcccggagaaagaagaatcttttattggtaaaacttatttgggtctcgacgcgggtgaaaggagcggcgtcggtttcgctattgttacagtggacggagatgggtacgaagtgcaaagattgggggtccacgaggatacacagcttatggccttgcagcaagttgctagtaaatccttaaaagagccagtatttcagcctctaagaaaaggcacctttagacaacaagaaagaatacggaaatccttacgtggttgctactggaatttttatcatgccttgatgataaaatatagggccaaagtagtacatgaggaatctgtcggaagtagtggtcttgtgggtcaatggttgagggcttttcagaaggatttgaagaaagccgatgttctccccaagaagggcggtaaaaacggtgtagataagaagaagagagagtcctcagctcaagacactctttggggtggtgctttctctaaaaaggaggagcaacagattgcgtttgaggtgcaagctgcaggttcttcgcaattttgtttgaagtgcggatggtggttccaactaggcatgcgtgaagtaaacagggtacaagaatcgggcgtcgtgttagattggaatagaagcatagttacctttttaatagaatcatccggcgaaaaagtttatggtttctccccacagcaattagagaagggtttcagaccagacatcgaaacttttaaaaagatggtaagagactttatgagacctcctatgtttgatagaaaaggcagaccggccgcagcttacgagagatttgttttaggaaggagacatcgaaggtacaggtttgataaagtatttgaggaaagatttgggaggtctgctcttttcatttgtcctagagtaggttgtggaaattttgaccacagctccgaacagtccgcggttgttttggccttgatcggatatattgccgataaggagggaatgtcaggtaagaagttggtttatgtacggctggccgaacttatggccgaatggaaactaaaaaaattagaaagatccagagttgaagaacaatcatccgctcaataa

SEQ ID NO: 144 - DNA, 3579 bp, Artificial Sequence
  Description of Artificial Sequence: Synthetic polynucleotide
atggcagaaagcaaacaaatgcagtgtaggaaatgtggagctagtatgaagtacgaagtcatcggtttgggtaaaaagtcatgtagatacatgtgtcccgattgtggcaaccatacctcggcaagaaagatacaaaacaaaaaaaaaagagataaaaaatatgggtcagccagtaaagcccaatctcaaagaattgctgtagcaggtgctctttaccctgacaaaaaagtacaaactatcaaaacctataaatatccagcagacttgaatggtgaggtgcatgatagcggtgttgccgagaaaatcgcacaagcaatacaagaggacgagattggacttttgggaccaagctcagaatatgcatgctggattgcatctcaaaaacagtctgagccttacagtgtagtcgatttctggtttgatgcagtgtgcgcagggggagtcttcgcctactctggcgctagattattgagtacagttttacagttatccggtgaggaatcggtgcttagagctgccttagcctcgtctccattcgttgacgatataaacttagcgcaagccgaaaagtttttggcggttagcaggcgtacaggtcaagataagttaggtaagagaattggggagtgctttgcagaaggaagattggaagctttagggataaaagatagaatgagggaatttgttcaagctatcgatgttgcacagaccgccggacaacgtttcgctgccaaattgaagatattcggtataagtcagatgccagaagctaagcaatggaataacgattccggactgactgtctgtatactacctgattattatgttcccgaagagaatcgcgcggaccaacttgtagtgttgttaagaagacttcgcgagattgcatattgcatgggtattgaagatgaagcgggtttcgaacatcttggaatagatcctggtgctctttcgaatttttcaaacggtaaccctaagagaggatttctagggaggctgttaaataacgatattattgcgttggcaaacaatatgagtgcgatgactccatattgggaagggcgtaagggtgaactcatagaaaggcttgcgtggttaaagcacagggcagaagggctgtatcttaaagaacctcatttcggtaactcctgggccgatcataggtcacgaattttctcaaggatcgcaggctggttatctggttgcgctggcaagttgaaaattgcgaaagaccaaatttctggagtacgtacagatctatttctgctaaaaagactgctggacgcagttccgcaatcggcgccatcccccgattttattgcgtcaatttcggcacttgacaggtttttagaagctgcagaatcgagccaggaccctgctgaacaagtgagggctctctacgcttttcacttgaacgcacctgcagtccgaagtatagccaataaagcagtgcaaaggtccgacagccaagaatggctgataaaagaactagacgctgttgaccatttagaatttaacaaagcgttcccatttttctctgacacaggaaaaaaaaaaaaaaaaggtgctaatagcaacggtgctccatcggaagaagagtacactgaaacggaatcaatacaacaacctgaggacgcggaacaggaagtaaacggacaagaagggaacggagcgtctaaaaatcaaaagaaatttcaaagaatacctagattcttcggtgaaggctccagatctgaatacagaattttaacggaagctccacagtatttcgatatgttttgtaataacatgagggctatatttatgcagttagaaagtcaaccccgtaaagctcccagagattttaaatgtttcctacaaaatcgattacaaaaattatacaaacagactttcttgaatgcacgaagcaacaagtgtcgcgctctgcttgagtcagttttaatctcttggggagaattttatacatacggtgccaacgaaaagaaatttagattaagacatgaagcttcagaacgcagcagtgacccagattacgtagttcagcaagccttggaaatcgcgcgtcgtctattcctttttggcttcgaatggagagattgctccgctggtgaaagagtggatttggttgaaattcacaaaaaggctatcagttttttgttggctattactcaagctgaggtctctgttggttcatacaattggcttggcaactcaacagtatcgagatatttatccgttgcgggaactgataccttatacggtacccaattggaagaattcctgaacgctacagtgttgagtcaaatgcgtggtctggccattagattgagttctcaagaacttaaggacggttttgatgtgcagctcgagtcttcctgccaggacaatctgcaacacctattggtgtatagggcttcgagagatttggcggcttgcaagcgcgctacttgtccagccgaactcgatcctaagattttagttttaccggtaggtgcattcatcgcttccgtaatgaaaatgatagaaagaggtgacgaacctttagctggtgcttatttacggcataggccacactctttcggatggcaaattagggtccgcggtgttgctgaggtagggatggatcagggtacagcattggcctttcaaaagccaacagagtcagaaccttttaaaattaagcccttctctgcacagtatggaccagttctgtggttgaacagtagtagttattctcaatcacaatatttggacggttttctatctcaaccaaaaaattggagtatgagggtgttgcctcaggcgggttcagttcgcgtcgaacaacgagttgctttgatatggaacttacaagcaggcaagatgagactagaacgctccggtgcgagggcctttttcatgcctgtaccgttttcatttaggccatccggcagtggggacgaagcagttttggcgcccaaccggtacttgggtctgttccctcattccggaggtatagaatacgctgtagtggatgtcctggattctgctggatttaaaattcttgaaagaggcactattgctgtcaatggtttctctcagaaaaggggagagcgccaagaagaagcccatcgtgaaaaacaaagaagggggataagtgatatagggcgaaagaagcctgtgcaggcagaagtcgatgcggcgaacgaattgcatagaaagtacactgatgttgccacaagattaggttgtagaatcgtcgttcaatgggcaccacaacctaaaccagggacagcaccgacagcgcaaactgtttacgcgagggctgttaggacagaagctccgaggagcggcaaccaagaagatcatgcaagaatgaaaagttcttggggttacacctggggtacgtattgggagaaacgaaaaccagaagatattttagggatttctacacaggtgtattggacaggaggtataggcgaatcctgtcctgctgtagcagtcgctttattaggtcatattagagcaacttcaacacaaacggagtgggaaaaggaagaagttgtctttggaagactgaagaagttctttccgagttaa

SEQ ID NO: 145 - DNA, 2958 bp, Artificial Sequence
  Description of Artificial Sequence: Synthetic polynucleotide
atggagaagagaattaataagatacggaaaaaattatctgcggataatgcaacaaagccagtctctcgttcaggccccatgaaaaccctgcttgtaagagtaatgacggatgatttaaaaaagaggttggaaaagcgtagaaaaaaaccagaagtgatgccgcaagtgatctcaaataacgcagctaataatctaaggatgctacttgatgattatacaaaaatgaaagaagcaatcctgcaagtttactggcaggaattcaaggatgaccatgttggactaatgtgcaaattcgcacaaccagcgtctaagaaaattgaccaaaataaattgaaacccgaaatggacgaaaaagggaatttaacaactgccgggtttgcctgctcgcaatgtgggcaaccattatttgtttataaattagagcaggtttcggaaaaaggaaaggcttacacaaattacttcggcagatgtaatgttgccgaacacgaaaaactcatattgttagctcagttgaagcctgagaaagactctgatgaggccgttacttactcgttggggaagtttggtcaaagagctctcgatttttattctattcatgtgacaaaggagtccacacatcccgtcaagcccttggcacaaattgcgggtaatagatacgcttcgggtccagttgggaaggccctttctgatgcatgtatgggcacaattgctagctttcttagtaaataccaggatatcataatagagcatcaaaaagttgtaaagggtaaccaaaagagattagaatcgctgcgtgagttggcgggtaaagaaaacttggaatatccatctgtcactctgcctcctcaacctcatactaaggaaggtgtagatgcgtacaatgaagttatcgctagagtccgtatgtgggtgaatttaaatttgtggcaaaaattgaagttatcgcgtgatgatgcaaaacctcttcttagactaaagggctttcctagcttccctgtagtggaaagacgcgaaaatgaagtcgattggtggaatacaattaacgaagtcaaaaaactgatcgatgcaaagcgagatatgggtcgagttttttggtctggtgttacagctgaaaaaaggaatacgatcttagaaggttacaactacttgccaaatgagaacgatcataaaaaaagagaaggcagtttagaaaatccaaaaaagccagctaagagacaatttggtgatttgctactttacctagaaaaaaagtacgccggagattgggggaaagtctttgacgaagcttgggagagaatagataaaaaaatagcaggattgacgtcacacattgaaagagaagaggcgagaaatgcagaagatgctcagtccaaagctgtcctcaccgactggttgagagccaaagcgtcctttgttctcgaacgcctaaaagaaatggatgagaaggaattttatgcctgcgaaatccagctacaaaaatggtacggagacttgagaggtaacccctttgccgtggaagcagagaaccgtgttgtagatatctccggtttctcaatcggtagcgatggacactccattcagtatcgcaacttgttggcctggaaatatttggaaaacggtaagagggaattctatttacttatgaattatggcaagaaaggtagaatcaggtttactgacggaacagacattaaaaagagtggtaagtggcaaggccttttgtacggtggtggcaaggccaaagtaatagacttaacatttgaccccgacgacgaacaactgataatactgcctttagcttttggtactcgacaggggcgagagttcatttggaatgatcttttgtcactcgagactggtttgataaaacttgcaaatggaagagtcatcgagaagacaatttacaacaaaaagataggtcgcgatgagcctgcactatttgtggccttgacctttgagagaagggaagttgtcgacccatccaatattaaaccagtcaacctaatcggtgtagatagaggtgaaaacatcccagctgttatcgctctgacagaccctgaaggttgccctttgccagaatttaaagattcgtctggtggaccaacagatatattacgtattggggaaggctataaagagaaacaacgtgctattcaggctgcaaaagaagttgaacagaggagagctggaggttacagtagaaaattcgccagtaaaagtagaaacttagcagatgacatggttagaaactctgcccgggatttgttctatcatgcggttactcacgatgcagtcttagtctttgaaaatctatcgcgcggttttggtaggcaaggcaagaggacttttatgacagagagacaatatacaaaaatggaagattggttaaccgcgaagctcgcatatgaaggtcttacttcgaaaacgtacctcagcaaaacgctggctcaatatacttctaaaacttgttcaaattgtggttttactattaccacggcagactacgacgggatgttggtgagattgaagaagacgagcgatggttgggcaacaacattgaataataaggaattaaaagcagaaggacagattacgtattacaatcgttataaacgccaaacggttgagaaagagttgtcagccgagttggatagactaagtgaagagagcggtaacaatgatatctcaaagtggactaaagggaggcgggatgaagccctctttttactaaagaagagattctcacatagacctgtgcaagaacaattcgtttgtttagattgtggccatgaggttcatgcagacgaacaggctgcgttaaatattgcgagaagctggctatttctaaattctaattcaacagagttcaagagctataaatccggaaaacaacctttcgtaggcgcgtggcaagccttctataaaaggagattaaaagaggtttggaaaccaaatgca

SEQ ID NO: 146 - DNA, 2919 bp, Artificial Sequence
  Description of Artificial Sequence: Synthetic polynucleotide
atgaaaagaattaacaaaattagaaggaggctggtcaaagattctaataccaagaaagctggtaagactggtccgatgaaaaccctattagtcagagttatgaccccagatttgagagaaagattggagaacctcaggaaaaagcccgaaaacatcccacaacccattagtaacacatcaagagctaatttaaacaagttattaactgactacactgaaatgaaaaaagcaatattgcatgtttactgggaagagttccagaaagatcctgttgggttgatgtctagagttgctcaaccggccccaaagaatatagatcaaaggaaacttattcctgtgaaggacggcaatgaaagattaaccagctccggtttcgcttgctcccagtgctgccaacccctgtatgtatacaaactggaacaagtaaatgataaaggtaagccacatactaactactttggtaggtgtaatgtatccgagcatgaaagattgatcttgttaagtccccataaaccagaagctaatgatgagttagtaacttatagtttaggtaagttcggacaacgagctttagatttctatagcatccatgttacaagagaaagcaatcaccccgtcaaaccactggaacaaatcggtggtaatagttgtgcgtcaggtccagtaggcaaagctttatcagacgcttgcatgggtgccgtggctagttttttgacgaaataccaagatattatactggaacatcaaaaggtaattaaaaagaatgaaaagagactcgctaacttaaaagatattgcaagtgccaatggtttagcttttcctaaaattaccttgccacctcagccacatacaaaggagggaattgaagcttacaataatgtagtagcccaaatagttatttgggtgaaccttaacctatggcaaaagttaaaaattggtagagacgaagccaaacccctgcagaggctgaagggttttccctccttccccttagtagagagacaagctaatgaagtggactggtgggatatggtgtgcaatgttaaaaaattgattaatgagaagaaagaggatggtaaagtgttttggcagaatcttgctggctacaagagacaggaagctttactgccttatttatcttctgaggaagataggaaaaaaggtaaaaaatttgctagatatcaattcggagacctacttctgcatttagaaaaaaaacatggcgaagattggggtaaagtttatgatgaagcctgggaaagaattgataagaaggtagaaggtctctccaaacatattaaattagaggaagaacgtaggtccgaagacgctcaatcaaaggcagcattaactgattggttgagagcaaaagcctctttcgttattgaaggattaaaagaagccgacaaagatgaattttgtagatgtgagttaaagttgcaaaagtggtatggagacctccgtggtaaaccttttgctattgaggctgaaaattctatactcgatatctctggattttcaaaacaatataactgcgcatttatatggcagaaagatggtgttaaaaagctaaatctatacttaattatcaattactttaaaggtggtaaattgcgttttaagaagataaagcctgaagcctttgaggcaaaccgtttttacactgttatcaataaaaaatctggggaaatcgtaccaatggaagttaatttcaatttcgatgatcctaatcttattattttacctcttgctttcggcaaaaggcaaggtagggagtttatttggaatgatttattgtcgctggaaacggggtctctcaaactcgcaaacggtagggtgatagaaaaaacattatacaacaggagaactcggcaggatgagccagctctttttgtggctctgacattcgagagaagggaagttttagattcatctaacatcaaaccaatgaatttaataggtattgaccggggtgaaaatatacctgcagttattgctttaactgatcctgagggatgtcctcttagcagattcaaggactcgttgggtaaccctactcacatcttaaggattggagaaagttacaaggagaaacaaaggacaatacaagctgctaaagaagtagaacaaaggagggcgggtggatatagtcggaaatatgccagcaaggccaagaatttagctgacgacatggttaggaatacagctagagaccttttatactatgccgtcacccaggatgccatgttgatatttgaaaatttaagtagaggcttcggtagacaaggtaagcgcaccttcatggcagagagacaatatactagaatggaagattggttgactgccaaattggcatacgaaggtctacctagtaagacgtacttatctaaaacactagcgcagtatacttccaagacatgcagtaattgtggtttcacaatcacttctgccgattacgatcgcgtcttggaaaaactaaaaaaaacagcgacaggttggatgactactattaatgggaaagaattgaaggtcgaaggacaaataacttactataatagatataaacggcaaaacgttgtaaaagacctgtcagtcgaactcgatcgacttagtgaagaatctgttaataatgatattagttcgtggacaaaaggtagatccggtgaagctttgagcctcctgaaaaaacgttttagccataggcctgtccaagaaaagtttgtatgtttaaactgtggttttgagacccatgcagacgagcaggccgctcttaatattgctagatcatggttatttttaagatctcaggaatacaagaagtaccagactaacaagacaacaggcaacacagataagcgagcattcgttgagacttggcaatctttttatagaaagaaattgaaggaagtctggaaacca

SEQ ID NO: 147 - DNA, 4077 bp, Artificial Sequence
  Description of Artificial Sequence: Synthetic polynucleotide
atgggaaaaatgtattatctaggcctggacatagggaccaattcagtaggctacgctgtcactgacccctcctaccatttgctgaagttcaagggggaacccatgtggggagcacacgtgtttgcggccggcaaccagagcgcagagcggagaagcttccgcacctccaggagaaggctggatcgcaggcagcagcgtgtgaagctggtccaagagatatttgccccagtgatttcccccatcgatccgcgcttctttattaggctccacgagtccgctctctggcgcgacgacgtggccgaaactgataaacatattttctttaatgacccaacatacactgacaaggagtactattcagattacccaacaattcaccatttgatcgtggaccttatggaaagttcggagaagcatgatcctcgacttgtctatttggccgtggcgtggctcgtggcacataggggccacttcttgaacgaggtggacaaggataacatcggggatgtgttatctttcgacgctttctatcctgaattccttgcttttctgtctgacaatggcgtcagcccgtgggtctgcgaatccaaggccctccaggctacgctattgtcaagaaatagcgtgaacgacaagtacaaggctcttaagtctttgatttttggaagccagaagcccgaggacaactttgatgcaaatatctcggaggacgggctgattcagctcctcgctgggaaaaaggtcaaggtcaataagctgtttccacaggagtcaaatgacgcgagcttcacccttaacgacaaagaggatgccattgaagagatcctggggacactcaccccagacgagtgcgagtggatagcccatattaggcgcctctttgattgggccataatgaaacatgcgcttaaggacgggcgcacgatatccgaaagcaaggtcaaattgtacgagcagcaccaccatgatctgacccagctaaaatattttgtaaaaacatatctggccaaggagtacgatgatatcttccgcaacgtggatagtgagaccaccaaaaactacgtcgcgtactcataccacgtgaaagaagttaagggcacgctgcctaagaacaaggcaacacaagaggagttctgcaagtacgttctcgggaaagttaaaaatatagagtgcagcgaggccgacaaagtggattttgacgagatgattcaacgcctgaccgacaattcgtttatgcctaaacaggtgagtggagagaatcgcgtgattccatatcagctctattactatgaactcaagactattctgaataaggccgctagctatttacccttccttacgcagtgcgggaaggatgccatttctaaccaggataaactcttgagtataatgacatttcgaattccctatttcgtgggtccgcttcgtaaggataacagtgagcacgcttggctggagcggaaggctggcaaaatttatccatggaatttcaacgacaaggtggatctggacaaatccgaagaagcctttatccgcaggatgaccaatacttgcacatactatcctggggaggatgtccttccactggactctctgatctacgaaaagttcatgattttgaatgaaattaacaacataaggatcgatgggtatcctatttccgtcgacgtgaagcagcaggtgttcgggctctttgagaagaagcgacgggtgaccgtgaaggatattcagaatcttctcttatcgctgggagccctggataaacacggaaaactgaccgggatagatactacgattcattctaattacaacacgtatcaccattttaagtcactgatggagaggggcgtcctaacaagagatgacgtggagagaatagtggaacgaatgacatattctgatgacaccaagagagtgcggctttggctgaataacaactacggcactctgacggcggatgatgtaaagcatatttcccgactccgtaagcatgacttcgggcggctgtctaagatgtttctaacaggcctcaagggtgtgcataaggaaactggggagcgcgctagcatcctggattttatgtggaacaccaatgataacctgatgcagctcctgtcagaatgctacacattttcggacgaaatcaccaagctgcaggaggcttactatgccaaggcccaactaagcttgaatgatttcctggattctatgtacatcagcaacgccgtaaaacgaccaatttataggacactggcagtggttaacgacattaggaaagcatgcggaacagctcccaagcgaatctttatcgagatggcccgcgacggcgagagtaagaagaaaaggtcagtgactaggcgggagcagatcaagaacctttaccgctctatccgaaaagacttccagcaagaggttgatttccttgagaagatcttagagaacaagtcagatggacagctccaatccgatgctctgtatctgtacttcgctcagctgggacgagatatgtacactggcgaccccattaaactagaacatatcaaggaccaatcgttttataatatcgaccacatctaccctcagtccatggtgaaagacgatagtctggacaataaggtgctcgtccaaagtgagattaacggagaaaagtcgagcagatatcctttggacgctgcgatccgcaacaagatgaagcccctgtgggatgcttactacaatcatggactgatcagcctgaagaagtatcagagactgacccggagtacccctttcacagacgatgagaagtgggattttatcaatagacaactggtggaaaccaggcagtccacgaaagctctggccattcttctgaagagaaagtttccagacacagagatcgtctattcaaaggccggcctcagttccgactttagacatgagttcggactcgttaaatcacgaaatataaacgatctccaccatgcaaaggacgcattcctcgcgattgtgactggaaatgtctatcacgaaagatttaataggcggtggttcatggttaaccagccatactcagtgaagaccaagacccttttcactcactctattaaaaatggcaacttcgtggcttggaatggtgaggaggatcttggaagaattgtgaagatgttaaaacagaataagaataccatccactttactagattcagctttgaccgaaaagaggggctattcgatattcaaccgttaaaggcttcaacaggtctcgttccacgaaaggccggactggacgtagtgaaatacggcggctatgataagagcaccgcagcttactacctccttgtgcgatttacgctcgaggataagaagacccaacacaagctgatgatgattcccgtggagggactgtacaaagctcgaattgaccatgataaagagtttctcacagattacgcacaaaccaccatctctgagattctccagaaagacaaacaaaaagttataaacataatgtttccaatgggtacaaggcatattaaactgaacagcatgatctccattgatggcttttatttgtccattggaggaaagtctagtaaaggcaagtctgtcctctgccatgccatggtacccctaatcgtcccacacaagattgaatgctacatcaaggctatggagagttttgctcggaaatttaaagagaataataagctgcgtattgtggaaaaattcgacaagataaccgttgaagacaatctgaatctgtacgagctctttctgcagaagctgcagcataacccctataataagttcttctccacacagttcgatgtactgaccaacgggcgatcaactttcacaaagctaagtcctgaggaacaggtgcaaacactcctaaacattctttccatttttaagacctgcagatcttcaggatgcgacttgaagagcattaacgggagcgcacaggcagctaggatcatgatctcagctgacctgacagggctgagtaaaaaatactccgacattcggcttgtagagcaaagcgccagtgggttgttcgttagtaagtcgcagaacctgctggaatacctgtaa

SEQ ID NO: 148 - DNA, 4005 bp, Artificial Sequence
  Description of Artificial Sequence: Synthetic polynucleotide
atgtcttctttgacgaagtttacaaacaaatactctaagcagcttacaattaagaacgaactgattcccgtaggaaagactctggaaaacatcaaagagaatgggctgatagacggcgacgaacaactgaatgagaactatcagaaggccaaaattatcgtggatgacttcctgagggattttattaacaaggccctgaataatacccagatcggcaattggcgggaactggccgacgctctgaacaaagaagatgaggacaatatcgaaaaattacaagacaaaatcaggggcattattgtcagtaagttcgagacattcgatctgttctcttcgtactccattaagaaggacgagaaaatcatcgatgatgacaatgacgttgaggaagaagaactggacttgggtaaaaagacctcatccttcaagtatatttttaaaaaaaatctgtttaaattagtgctccccagttatttaaagacaactaaccaggacaagcttaagattatctcctcttttgacaactttagcacctattttagaggcttctttgaaaatcgcaagaatattttcactaagaagcccataagcacctctattgcctacagaatcgtacatgataacttcccaaaatttttggataacattagatgttttaatgtatggcagaccgaatgtcctcagttaattgtgaaggcggataactacctcaaatccaagaatgtgatcgccaaagataagtctcttgctaactactttacggtcggagcctacgattacttcttatctcaaaacggtattgacttttacaataacattatcgggggattgcctgccttcgccggccatgagaaaattcagggcttaaacgagttcataaatcaggaatgtcaaaaggactcagagctgaaatcaaagcttaagaatcgacacgcatttaaaatggcggtcttgttcaaacagatcctcagcgatagagagaaaagcttcgttattgatgaattcgagagcgacgcacaggtgattgatgccgtgaagaacttctatgcggaacagtgtaaagacaataatgttattttcaacctattaaacttgattaagaatatcgcgtttttaagtgacgatgaactcgacggtatctttatagaaggcaagtacctgtcctctgtcagccaaaaactctactcagattggtccaagctaagaaatgacatcgaggacagtgctaacagcaaacagggcaataaagagctggcaaagaaaatcaagactaataaaggggatgtggagaaggcgatatctaaatatgagttctccctctccgaactgaactccatcgtccacgataataccaagtttagtgatctgttgtcgtgtacactgcacaaagtggccagtgaaaaactcgtcaaggtgaacgaaggcgattggcccaaacacctgaaaaataatgaggagaaacagaagatcaaagaacctttggatgcgttgctcgaaatatataacacactgttgatcttcaactgtaaaagcttcaacaagaacgggaacttttatgtagactacgatcgatgtataaatgaactgagcagcgtcgtttacctgtacaacaagactcgcaattattgtacgaaaaaaccatataacaccgataagttcaagcttaatttcaacagtccccagctgggagaagggttcagcaaatcaaaagaaaacgattgcctgacattactctttaaaaaggatgataattattatgttgggattattaggaaaggcgctaagatcaactttgacgacacacaggccatagctgacaacactgataactgcatctttaaaatgaattactttctgttgaaggacgccaaaaaattcattccaaaatgctctattcagctcaaggaggttaaggcccatttcaagaagtctgaagatgactacatcctctctgacaaggaaaaattcgctagtcctctggttatcaaaaaaagtaccttcttgctggctacagctcacgtgaaaggcaagaaagggaacattaagaagttccaaaaggaatacagcaaagagaatccaaccgagtacagaaattctctgaacgaatggatcgcattctgtaaagaatttctaaagacgtacaaggccgctaccattttcgatattaccaccttgaaaaaagccgaggagtacgccgacatcgtcgaattctataaagacgtggataacctgtgttacaaattggaattctgcccaattaagacctctttcattgaaaacctcatcgacaatggggacctctacttatttagaattaacaataaggatttttcttcgaaatctaccggaactaaaaatctgcacacactgtatctgcaagcaatcttcgatgaacgtaatctcaacaaccctacaataatgctgaacggcggtgctgaactgttctaccgtaaagagagtattgaacagaagaatcgaatcacacacaaagcgggcagtattctcgtcaataaggtgtgcaaagacgggaccagcctggacgataagatcaggaatgaaatatatcagtatgagaacaagtttatcgacaccttgtcggatgaggcaaagaaggtgctacctaacgttatcaagaaggaagctacccatgacataaccaaggataagcggttcacttctgacaagttcttcttccactgtcctctgaccattaactacaaggaaggagacactaaacaattcaataatgaagtacttagctttttgcggggtaatcccgatattaacataattggtatcgaccggggagaacggaacctgatatacgtgacagtaattaatcagaaaggagaaatcctggattccgtatccttcaataccgtgactaataaatctagtaaaatcgagcagacggtcgactacgaggaaaagttagcagtcagagagaaggagagaatcgaggccaaacgttcctgggatagtatcagcaagattgctactctgaaagaaggatatctgtccgctatcgtccatgagatctgtttgttgatgatcaagcacaatgctatagtggttctggagaacctgaacgcaggcttcaagcgaattagagggggcctgtcggaaaaaagcgtttaccagaagtttgaaaagatgctaatcaataagttaaattactttgtaagtaaaaaagaaagcgattggaataagccatcaggacttttaaacgggctgcaactgagcgaccagtttgagtcattcgaaaaactgggtattcagagtggtttcatattctacgtacctgccgcttacacttcaaagatcgatcctacaactggttttgcgaatgtcctgaatctgtctaaggtgaggaatgtggacgcaatcaagtctttcttcagcaacttcaacgagatatcttacagcaagaaagaggctctgtttaaattcagttttgatctggatagcctgagcaagaaaggattctcttctttcgtaaagttttctaagtccaaatggaacgtctacacgttcggagagagaatcattaaaccaaagaacaagcaggggtatcgggaagacaaaaggatcaatctgactttcgaaatgaagaaactattgaatgagtacaaagtctcattcgatttggagaacaatctgatccccaatctgaccagcgctaacctcaaagacacattctggaaggagctgtttttcatctttaagaccaccctgcagctacggaatagtgtcacaaatgggaaagaggatgtactgatctcacctgtgaaaaacgccaagggggagttctttgtgtccggcacccataacaaaaccctgcctcaggactgtgacgcgaacggggcctaccacatcgcgctaaaggggttaatgattctcgaacgtaataatctggtgcgcgaagaaaaagacacaaagaaaattatggccatcagcaacgttgactggtttgagtacgtgcagaagcgtcgaggagttttgtaa

SEQ ID NO: 149 - DNA, 3717 bp, Artificial Sequence
  Description of Artificial Sequence: Synthetic polynucleotide
atgaacaactatgacgagttcactaaactttaccccattcagaaaaccatcagatttgaactgaagcctcagggtcgtaccatggaacacttggaaactttcaactttttcgaggaggacagggatagagctgagaaatacaagatcttgaaagaggccatcgacgagtatcacaaaaaattcatcgatgagcatctcaccaacatgtcgctggattggaacagtctcaagcagatttccgagaagtactataaatctcgggaggagaaagataaaaaggtgtttttgagcgagcaaaagcgaatgcgacaggagatagtctctgaatttaagaaagatgatcggtttaaagacctattttccaaaaagcttttttcagagctgctgaaggaagagatctataaaaaaggcaatcaccaagaaattgatgccctgaaatcattcgacaaattcagtgggtatttcataggactgcatgagaaccggaagaatatgtatagtgatggagacgagatcacagccataagcaatcgaatcgttaacgagaatttcccgaagttcctggataacctgcagaagtatcaagaggctaggaaaaagtaccctgagtggatcatcaaggctgaatcagctctggtggctcacaatatcaagatggatgaagtctttagtcttgagtactttaataaagtccttaaccaggagggcatccagcgctataacctggctctcggtggctacgtcacaaaaagcggagaaaagatgatgggtctcaacgatgcactgaatttggctcatcagtcggagaagtcatctaagggacgcatacacatgacaccactgtttaaacaaatcctgagcgaaaaggaatcattttcctacattcccgacgtattcaccgaggactcacaactgctgcctagtataggggggtttttcgctcagatagagaacgacaaagatggcaacatttttgacagagccttggagttgatttcatcttacgccgagtacgatacggagcgcatttatattcgccaggcggatatcaacagggtttccaatgtgatctttggcgagtggggaacgctgggcgggctgatgcgggaatacaaagccgactcgatcaatgacatcaacctggagagaacatgcaagaaggtcgataaatggttggatagcaaagagttcgccctgagtgacgtcttggaagctatcaaaagaaccggaaataatgacgcgttcaacgagtatatctctaaaatgaggaccgcgagagaaaaaattgatgcagcaaggaaggagatgaagtttatatctgagaagatctcaggcgatgaagagtccatccatattattaaaactcttctggactcagtgcagcaattcctgcacttttttaacctcttcaaggccaggcaggatataccgttagacggggctttttatgccgagtttgatgaagttcattcgaaactttttgctatagtgcctctctataataaagttcgcaattacctgacaaagaataacttaaacacaaagaaaatcaagctcaacttcaaaaacccaacactggcaaacggatgggatcagaacaaggtatatgattacgcctcattgattttcctccgggacgggaattactatctggggatcatcaaccctaagcgcaaaaagaacattaagttcgaacagggatctggcaatggtcccttctataggaaaatggtatacaaacagattcctggccccaacaagaatctcccacgcgtctttctgacgtccactaagggaaagaaggagtacaagccgtctaaagaaattatcgagggctatgaggcagacaagcatattaggggtgacaagtttgacctagacttttgtcataagcttatcgactttttcaaggagtccatagagaagcacaaagattggtcaaagtttaatttctatttttctccaacagagtcctacggggatatctctgagttctatctggatgttgaaaagcaggggtacagaatgcacttcgaaaatatctcagcagaaactatcgatgagtacgtagagaaaggagatctgtttcttttccaaatctacaataaggattttgtgaaggccgccactgggaagaaggacatgcacactatttactggaacgctgcattttcccctgaaaatctgcaggacgtagtagtgaaattaaatggtgaggcagaactgttttaccgcgataaatcagacatcaaggaaatagtgcaccgggaaggcgagattcttgttaaccgaacatataatggcaggacacctgtccctgataaaattcataagaaactgaccgattaccacaacggtcgaaccaaggatctgggcgaggccaaggaatacctcgataaggtgaggtacttcaaagcccattatgacatcaccaaggaccgaagataccttaacgacaaaatctacttccatgtcccactcaccttgaacttcaaagctaacggtaagaagaacctcaataaaatggtgattgaaaaatttctgtccgatgagaaggcccatatcatcggcattgatcgcggcgagagaaatctcctttactattctatcattgatcggtcgggaaagattatcgaccaacaatcactgaatgtcatcgacggattcgactatagagagaagctgaaccaacgggaaatcgagatgaaggacgcgcgccagtcctggaacgctatcggcaaaattaaagatttgaaagaaggttacctctccaaagcagtgcacgaaattaccaaaatggcaatccagtacaatgctattgtggtaatggaggagttaaattacggatttaagcgcgggaggttcaaggttgaaaagcaaatttaccaaaaatttgagaacatgttgattgataagatgaactacctggtgttcaaggacgcacctgacgagtcgccaggcggcgtgttaaatgcatatcagctgacaaatccactggagagctttgccaagctaggaaagcagactggcattctcttttacgtccctgcagcgtatacatccaaaattgaccccaccactggcttcgtcaatctgtttaacacctcctccaaaaccaacgcacaagaacggaaagaatttttgcaaaagtttgagtccattagctactctgccaaagacggcgggatctttgctttcgcattcgactacaggaaattcgggacgagtaagacagaccacaagaacgtctggaccgcgtacactaatggggaacgcatgcgctacatcaaagagaaaaagaggaatgaactttttgacccttcaaaggaaatcaaggaagctctcacctcaagcggtatcaaatacgatggcgggcagaatattttgccagatatcctcagatcgaacaataatggacttatctatactatgtactcctccttcattgcagcaattcaaatgagagtgtacgatggaaaggaggattacattatatcgccaattaagaactccaaaggcgaattcttccgcacggatcctaagcgaagagaactcccaatcgacgctgatgcgaacggcgcctataatatagccctgcggggtgaattaacaatgcgcgctattgccgagaagttcgaccccgattcagaaaaaatggctaagcttgagctgaaacacaaagattggttcgaattcatgcagacaagaggcgactaa

SEQ ID NO: 150 - DNA, 3897 bp, Artificial Sequence
  Description of Artificial Sequence: Synthetic polynucleotide
atgactaagaccttcgattccgagttcttcaacctttattccctgcagaaaactgtaaggtttgagctgaagccggtgggcgagacagccagcttcgtagaggatttcaagaatgagggtctcaaacgggtagttagtgaggatgagaggagagcagtggactatcagaaggtgaaagagatcatcgatgactatcaccgggatttcatagaggagtcgttgaattacttccctgagcaagtatccaaagacgcgctggaacaggcctttcatctttaccagaaactgaaggcagcgaaggttgaggagcgggaaaaggccttgaaagagtgggaagccctgcagaaaaagctcagagaaaaggttgtcaaatgcttcagcgacagcaacaaagccaggttcagtaggatcgataagaaagaactgatcaaagaagacttgatcaattggctggttgcacagaaccgggaagatgatattcccaccgtagagaccttcaacaacttcacaacttacttcaccggcttccatgagaatcgtaaaaacatctacagtaaagatgatcatgcaaccgccatctccttccggttgatccacgagaatctccccaagttctttgacaacgtgataagtttcaataagttgaaagagggatttcccgaactcaagttcgataaagtgaaggaggatctggaagtggattatgaccttaagcacgctttcgagatagagtacttcgtgaactttgtgactcaggccggcatcgatcagtataactacctcctcgggggtaagacgctcgaggacggtactaagaagcaaggaatgaatgagcaaattaatctatttaaacagcagcagaccagggataaggctagacagatccccaagcttattcctctttttaaacagatcctaagtgaaaggacagaaagtcaaagcttcatacctaagcaatttgaaagtgatcaggagctgtttgactccctgcaaaagctgcacaacaattgccaggacaagtttaccgtgctgcagcaggctatcctcggactggctgaggcggatcttaagaaggtattcattaagactagcgacctcaatgcccttagtaacaccatctttggaaattactccgttttcagcgatgccctcaatctatacaaagagagcttgaagactaaaaaagctcaggaagcttttgaaaaattaccggcacattctatacacgaccttatacaatacttagagcagttcaacagcagcctcgacgctgagaaacagcaatccacagacaccgtcctgaattacttcatcaaaaccgatgaactgtactcccgatttatcaagagcacttcagaagccttcacgcaagttcagcctctgttcgagctggaggcactgtccagcaagagacgaccgccagagtctgaagacgagggagccaagggtcaagaggggtttgaacagataaagcgaattaaggcttacttggatactctcatggaggcggtgcatttcgctaagcctttgtacctggttaaaggccgaaaaatgattgaggggctagataaggatcagtctttttacgaggcttttgaaatggcctaccaggaattggaatccttgatcattccaatctataataaagcccggagttatctgagcaggaagcccttcaaagccgacaagttcaaaataaattttgacaataatacgctactgtctggttgggacgctaacaaggaaacagccaatgcttccatcctgtttaagaaagacggcctgtactacctgggaattatgccaaaaggcaaaacttttttgttcgattactttgtgtcatcagaggatagcgagaagttaaagcaaagacggcagaagaccgccgaagaagccctcgcacaagacggagaatcatatttcgagaaaattcgatataagctcctgcctggcgcatcaaagatgttgccaaaagtcttcttttccaacaaaaacatcggcttttataaccccagcgatgatatccttcgcatccggaacaccgcctcacataccaaaaatggaactccacagaagggccactcgaaggttgaattcaaccttaacgattgtcacaaaatgattgatttttttaagagctccattcagaaacaccccgaatgggggtcctttggcttcaccttttctgatacttcagacttcgaggacatgtccgccttctacagggaggtggagaaccagggctatgtcatctccttcgacaaaataaaagagacatacattcagagccaggtcgagcagggaaatctgtacctgtttcagatctataacaaggatttcagtccctatagcaagggcaagcccaatttacataccctgtactggaaggccctgttcgaagaggcaaaccttaacaatgtagttgctaagctgaatggggaagcagagatcttcttccgaaggcacagcatcaaggcaagcgacaaagttgtacatcctgctaaccaggccatcgataacaagaacccgcatacagaaaagacacagtcaacctttgaatacgacctcgtgaaggacaagaggtacacacaagataaattcttcttccacgtgcccatcagcttgaattttaaagcgcagggagtgagcaaatttaacgacaaggtcaacggcttcctgaagggaaaccccgacgtgaatatcatcggaattgatcgcggtgaaagacatctcctctactttactgtggtgaaccagaagggtgagatcctagtacaggagagcctgaacacccttatgagtgataagggccatgtgaatgattaccagcagaagctggacaagaaggaacaggaaagggacgcagcgcggaagtcctggaccactgttgagaatatcaaagaactgaaggagggatatcttagccatgtggtacacaaacttgcacatctgattatcaagtataatgccatagtctgcctggaagacttgaacttcggtttcaagcgaggaaggtttaaagtggagaagcaggtgtaccagaagtttgagaaagcccttattgataagctaaactaccttgtctttaaggaaaaagaactcggcgaagttggccactatttaaccgcctaccaactaaccgcccctttcgagtcttttaagaaactgggaaagcagagcggaatactcttctatgtgcctgcagactacacctctaagatcgaccccactaccggctttgtaaactttctagatctccgctatcagtcagtagaaaaagccaaacagctcttgtcagattttaacgccatccgatttaattccgtccaaaattacttcgagttcgaaatcgactataaaaaacttacccccaagagaaaggttgggacgcagtctaagtgggtaatctgcacttacggtgacgtgagataccagaaccgccgaaaccagaaaggtcattgggaaaccgaggaagtgaatgtgactgagaagctcaaggccctcttcgctagcgacagtaaaacaacaacagttatcgattacgccaatgacgataatcttatagacgtgatcttggaacaagacaaagcctctttttttaaggaattgttgtggttgctgaaacttacaatgacccttaggcacagcaagatcaaatcagaggatgacttcatcctcagcccggtgaagaatgaacagggagagttctacgattcacggaaggctggagaggtgtggcccaaggatgccgacgcgaacggggcctaccacatagctctaaaaggtctgtggaacctgcaacaaatcaatcaatgggagaaaggtaagacactgaacctggccatcaaaaatcaagattggttctcattcatccaggaaaagccttatcaagagtga

SEQ ID NO: 151 - DNA, 3708 bp, Artificial Sequence
  Description of Artificial Sequence: Synthetic polynucleotide
atgcatacgggaggccttttatcaatggacgcaaaagagttcaccgggcagtatccattatctaagacactccgcttcgagctgaggcccattggcaggacctgggacaacctggaggcgtcgggctacctggctgaggacagacatcgcgcagaatgctatccgagagctaaggagcttttggacgacaatcatcgcgcgttccttaaccgggtgctcccacagatcgatatggactggcacccgatcgctgaggctttttgcaaggtccataagaaccctgggaacaaagagctcgcccaggactacaacttgcagctgagcaagcgacggaaagagatttctgcctaccttcaagacgccgatggctacaaagggctcttcgcaaagcccgcattggatgaggccatgaaaatcgccaaggagaacgggaatgaaagtgacatcgaagttctcgaagcgtttaacggatttagcgtgtactttaccggctatcatgagtcaagggagaatatttatagcgatgaggacatggtctctgtggcctaccggattaccgaggataatttcccgaggtttgtttcaaatgcactaatattcgacaagttaaatgagagccacccagacatcatctcggaggtcagcggcaacctcggagttgacgatattggcaaatacttcgacgtgagcaactataacaacttcctctcacaggctggcatcgacgactataatcatattataggcggccacactactgaggatggtctcattcaggcattcaatgtagtcttgaatcttaggcaccagaaggaccctgggtttgaaaagatacagttcaagcagctgtataagcagatattatccgtgcgaacatctaaaagttacatccccaaacagtttgataactcaaaggagatggtggattgcatatgcgattatgtgtcaaaaattgaaaagagcgagactgtggagcgggctctgaagctcgtcaggaacattagctcctttgaccttagaggaattttcgtcaataaaaagaatctgaggatcctgagcaataagctaataggagattgggacgccatagagacagcattgatgcattccagctcaagcgagaatgataagaagtctgtctacgatagcgctgaagccttcacgctggacgatatcttctcttccgtgaaaaaatttagtgatgcgtccgcagaagatatcgggaatcgagccgaagatatctgcagggtaatttcagagaccgcccctttcatcaatgacctgcgcgccgtggacctggatagcctgaatgacgatggttacgaagctgcagtttctaagatcagggagtctctggagccatatatggacttgtttcacgaacttgagatctttagcgtgggcgacgagttcccgaaatgcgcagctttctatagcgagttagaggaggtcagcgagcaattaatcgagatcatacccctgtttaataaggcacggagcttttgtactcgcaagcgctacagcaccgacaagattaaagttaatctgaaatttccaactctcgcagacgggtgggacctaaacaaggaacgcgataataaagccgccatccttagaaaggacggaaagtactatcttgccatcctagatatgaaaaaagatctgagttccattcgtactagcgatgaagacgaatcttctttcgaaaaaatggagtataagctgctcccctcgccagtcaagatgctacccaagatctttgtgaagagcaaagcagccaaggaaaagtacgggctgacggacaggatgctggagtgctacgataagggaatgcataaatcagggtcagcttttgacttgggcttttgccatgagctaatcgattactacaagcgctgtatcgccgagtatccaggatgggacgttttcgactttaaatttcgggagacttctgattatggttcaatgaaggagttcaacgaagatgtcgctggtgccggttactacatgagccttcgcaagattccttgttccgaagtctaccggctactggacgagaaatctatatatttgttccagatatataacaaggactacagtgagaatgcacatgggaataagaatatgcatactatgtattgggaaggtctcttttcaccccaaaatttggagtcacccgtgttcaaacttagcggtggcgcagagctgttctttaggaaatccagtatacccaatgacgccaagacagtccacccaaagggtagcgtcctggtgcccagaaacgatgtgaacggcaggagaatccctgacagcatttaccgagaacttaccaggtacttcaaccgcggcgactgtagaatctctgatgaggcaaagtcttatctggataaggtgaagactaagaaggcagatcatgacattgtgaaagaccgccgctttactgtcgacaaaatgatgtttcacgtgcctatcgcaatgaattttaaggcaatctcaaaaccgaatctgaacaagaaggtgatagatggcattatcgatgaccaggacctcaagatcatcggaatcgacagaggtgagcgaaacctgatatacgtcacaatggtagatcggaagggtaatattctgtaccaggattcactaaacatcctcaatggatatgactatcgaaaagctctcgatgtcagggaatacgacaacaaggaggcgcgacggaattggacaaaggtggaaggcatacggaagatgaaggaaggctatctgtcactagctgtctccaaattggctgatatgattatagagaacaacgccattatcgtgatggaagatctcaaccatggattcaaggcaggaagaagtaaaattgagaagcaggtgtatcagaagttcgaaagcatgcttattaataagttgggttatatggtcttaaaggacaagtctatcgatcagagcggcggcgcactccatgggtatcagctggctaaccatgtcaccacactagcatccgtaggcaaacagtgtggcgtgattttctacattcctgctgcgttcacttctaagatcgatcctaccacgggattcgcagacctgttcgcactgagcaatgttaaaaacgtggcctccatgagggagttctttagcaaaatgaaaagcgtgatttatgacaaggccgagggcaagttcgctttcacatttgactacctggactacaatgtgaaatcagagtgcgggagaaccctgtggaccgtatacacggtaggggaaagattcacttacagtcgagttaatcgggagtatgtccgtaaagtgccaactgacatcatctacgatgcccttcagaaggctggcataagtgttgagggggatctaagggacaggatcgctgaatcggatggcgatactctcaaatcaatcttctacgccttcaagtatgccctcgacatgagggtagagaaccgggaggaggactatatacagtctcccgtgaagaatgcgtcgggagagttcttctgctcaaaaaacgccgggaaatctttgccgcaggattctgatgcaaatggggcttataacattgctctcaaaggcatcctgcagctgcgcatgctatctgaacaatatgacccaaacgctgaaagcattagattgccattgatcaccaataaggcttggctgactttcatgcagagcggtatgaagacatggaaaaactaa

SEQ ID NO: 152 - DNA, 3783 bp, Artificial Sequence
  Description of Artificial Sequence: Synthetic polynucleotide
atggattcccttaaggacttcacaaatctttaccccgtgagtaaaaccctgagatttgaactcaagcccgtgggaaagactctcgagaatatcgagaaggccgggattttgaaggaagacgagcatcgggcggaaagttacagacgggtgaagaagattatagatacttatcacaaggtctttatagacagctctttagagaacatggcaaagatgggcatcgagaacgaaatcaaggccatgctgcagtccttctgcgagctgtataaaaaggatcatcggaccgaaggcgaagacaaggcgctggataagatcagggcagtgctgcgcggcctcattgtgggtgccttcactggggtgtgcgggcggagagagaacactgtgcagaatgagaaatacgagagtttgttcaaagagaaactcatcaaggaaatcctgcccgacttcgtcttaagcacagaagccgaatctctcccattttctgtcgaggaggccacgcgttcccttaaagagttcgacagtttcacttcatactttgccggattttatgaaaaccgtaaaaatatatactccactaaaccacagtcaactgcaatagcttacaggttaatccacgaaaacctgccaaaattcatcgacaatatactcgtctttcaaaaaatcaaggaaccaatcgcgaaggaacttgaacacatccgggctgactttagtgcgggaggatacatcaaaaaagacgagcgcctggaggatatattttcactaaattattatattcatgtactgagccaggctggcatagaaaagtacaacgctctaattgggaaaatcgtgacagaaggtgacggggaaatgaaagggctaaacgaacatattaacttatataaccaacagcggggtcgagaagatcgtctgcccctgttcagacctctgtataagcaaatactctccgacagagagcagctatcatatctgcccgagtcctttgagaaagatgaagagctgctccgggcgctcaaggagttctatgatcatatagccgaggacattttgggcagaactcagcaactcatgacgtctatttctgaatatgatctgtctcgtatctatgtcaggaatgatagccagctgaccgatatatccaagaagatgctgggggactggaacgccatttatatggcgagggagcgagcatacgatcacgagcaggcacccaagagaatcacagccaaatatgagagagaccgcattaaggcgctgaagggcgaagaaagtatcagtctggccaatctgaactcctgcatagctttccttgataacgtgagggattgcagagttgatacttacctgagtaccctgggccagaaggaagggcctcacggcctctctaatctagtggagaatgtatttgcctcctaccacgaagctgagcagctgctgtcatttccgtacccagaggaaaataatttaatacaggataaggacaacgtagtgcttatcaaaaatctactggataacatttccgacctccagcgctttctcaaaccactttgggggatgggcgacgagcctgataaggatgagcgcttttacggcgagtacaactacatcaggggcgccttggaccaggtgattcccctctataataaagtcaggaattacctgacccgaaagccatacagtacaagaaaggtgaaattaaatttcggcaatagtcagctgctgtctggttgggaccgaaataaggagaaagacaacagctgcgtaattctcagaaaaggacagaacttttatttggccatcatgaataacagacacaagagatctttcgagaacaaagtgctccctgagtataaggagggggaaccctacttcgagaagatggactataaattccttcctgatccaaataaaatgctgcctaaagtatttctgtcaaaaaaaggtatagaaatctacaaaccttcacctaagctacttgaacagtatggccacggcacccataaaaaaggggacacgttcagcatggacgacctacacgaactgattgacttctttaagcacagcatagaagctcatgaggactggaaacagttcggattcaaattctcagataccgcgacctacgaaaacgtgtctagtttttaccgggaagtcgaggaccagggctacaagctcagcttcagaaaagttagcgaatcttacgtctactcccttatagatcaaggtaagctgtatctctttcaaatctacaacaaggacttttccccatgtagcaagggcacccccaatctgcacactctctactggcggatgctgttcgacgagcgtaacctggcagacgtgatctacaaattagatggtaaagctgagatcttctttcgtgaaaagagcctaaagaacgatcaccccactcaccccgccggaaagcccattaagaagaaaagtaggcagaagaaaggagaagaatcgctatttgagtacgacctcgtcaaggatcggcattatacaatggataagttccagttccatgtgccaataactatgaatttcaagtgcagtgctggcagtaaggtgaatgacatggtaaacgctcatatccgggaggcaaaggacatgcatgttattggaattgataggggtgagcgtaatctcctctacatctgtgttattgactcccgcggcacaatcctcgatcagatttccttgaatacaattaatgatatagactaccatgacttgcttgagtctcgcgacaaagatagacagcaggagagaagaaattggcagaccatcgaaggcatcaaggaactcaagcaaggctacctttctcaggcagtgcatcgaatagccgagctgatggtggcttataaagccgtcgtggcactagaagacctaaatatgggatttaaacgaggcaggcagaaggtggaatcatccgtataccagcagttcgaaaaacagttgatagacaaactcaattaccttgtagacaagaagaagcggcctgaggacatagggggcctgcttagagcgtatcaatttacagccccattcaagtctttcaaagaaatgggtaaacagaacggttttctgttttacatcccagcgtggaacaccagcaatatagatccaaccactggcttcgtcaatctgtttcatgctcagtatgaaaatgtggacaaggccaaatccttctttcagaaatttgacagcatctcctataacccaaagaaagactggtttgaattcgcctttgactataagaatttcactaagaaggccgagggatcaagaagcatgtggatattgtgcacgcatggctcacgtataaagaactttagaaactcgcaaaaaaacgggcagtgggactcagaagaattcgcactcaccgaggctttcaaatccctcttcgtccggtatgagatcgattacaccgccgatctgaagacggcaatcgtcgacgagaaacagaaagacttctttgtagatctacttaagctctttaagctaaccgttcagatgcgaaacagttggaaagaaaaggatctcgactatctcattagtccagtggctggcgcggatggtagatttttcgatacccgggaaggtaacaagtcccttcccaaagacgccgacgcgaatggtgcctacaatattgcactaaaggggctctgggcgctgcggcaaattagacagacatctgaagggggcaagcttaagctggctatttctaataaagagtggttgcagtttgtgcaggaaaggagttatgagaaggactag

SEQ ID NO: 153 - DNA, 3792 bp, Artificial Sequence
  Description of Artificial Sequence: Synthetic polynucleotide
atgaacaacggcaccaacaacttccagaacttcatcggcatatcgtctctgcagaaaacacttaggaatgccctgattccaactgagacaacacagcagtttattgtgaagaatgggatcatcaaagaggacgaattgcgcggggagaataggcagatcctgaaggacatcatggacgattactacaggggttttatctccgaaacgctgagctcgattgacgatattgactggacgtccctctttgagaagatggaaatccaacttaaaaatggcgataataaagataccctgataaaggaacaaaccgaatatagaaaggctatacacaaaaaattcgcaaatgacgaccgctttaagaacatgttttctgcaaaactgattagcgatattctgcccgagtttgtgattcacaataataactattccgcttcggagaaggaggaaaagactcaggtgattaaactgttttctcggttcgccacttctttcaaagattatttcaaaaatcgcgccaactgtttttccgctgacgacatctcctcctcttcctgccaccggatcgtaaacgacaatgccgagatcttttttagtaacgcccttgtgtatcggaggatagtgaagagcctgtccaatgatgacataaacaaaatttctggcgatatgaaggatagcctcaaagagatgagccttgaagaaatttactcctacgagaagtatggggagttcatcacccaggaggggatttccttctataatgacatctgtggcaaggtgaacagcttcatgaacctgtactgccagaagaataaggaaaacaaaaatctgtacaagcttcagaagttacataagcagatcctgtgtatcgcggatacctcatatgaggttccttataagttcgagagtgatgaagaagtgtaccagtctgtaaatggattcttagacaatatttcgtccaaacatatagtggagagactgagaaagatcggggacaattacaatgggtacaatctcgacaagatttatatcgtgtcgaagttttacgaatctgtgagccagaaaacatacagggattgggaaaccattaataccgcgcttgaaattcactacaataatattctgcctggcaacggaaaaagcaaggccgataaggtaaaaaaggcagtcaaaaatgaccttcagaaaagtatcaccgaaatcaatgagttggtgagcaactacaaattgtgttcagacgataatattaaagcggaaacgtacatacatgaaattagccatattctgaataactttgaggcgcaggaacttaagtacaaccctgaaattcatctcgtcgaaagcgaattgaaggcctctgaattgaaaaacgttcttgacgtgataatgaacgctttccattggtgctctgtgtttatgactgaagagctggttgataaggacaacaacttttatgctgaacttgaggaaatctacgacgagatctaccctgtgattagcttgtataacctcgtcagaaactacgttacccagaagccgtacagcacgaaaaaaataaagctgaactttggtattccgactctcgccgatggatggagcaagtcgaaggaatattccaacaatgccatcattcttatgcgagacaatctgtattacctcggcatctttaacgccaaaaacaagccggataagaaaatcattgaagggaatacgagcgagaataagggcgactataagaaaatgatctacaacttactgccaggtcccaataaaatgattcctaaggtgtttctgtcatcgaaaacaggtgtagaaacatataagcccagcgcatacatcctggaaggctacaagcaaaacaaacacatcaaaagcagcaaggactttgatatcacattctgccacgatctaatcgactacttcaaaaattgcatcgccattcaccctgagtggaagaacttcggctttgacttctccgacaccagtacctacgaagacatttctggattctaccgtgaggttgagctgcagggttataaaattgactggacatacatcagtgaaaaagacatcgatctactgcaggagaaggggcagctctatctcttccagatttataataaggatttcagcaagaagtccactggaaacgacaatctgcatacaatgtatcttaagaacttgtttagcgaagagaatttgaaagatatcgttctaaagttaaacggggaagccgagattttctttcgaaagtcttccattaagaatccaattattcacaagaagggcagtatcctggtcaacagaacctatgaggccgaggaaaaggaccagttcggtaatatacaaattgtgcgcaagaacatccccgagaacatttaccaggagctctataaatacttcaacgacaaaagcgataaggagctttccgacgaggctgccaagctgaaaaacgtggtgggacaccatgaagcagccaccaacatcgtcaaagattatcgttatacatatgacaaatattttctgcacatgcctattacaataaactttaaggcaaacaagaccgggttcatcaatgaccggatactccagtacatcgcaaaagagaaggacctgcatgtgatcggcatcgaccgcggtgaaagaaatctcatttacgtcagcgttatcgacacttgtggaaacattgtggagcagaagtccttcaacattgttaacggctatgactatcagatcaagctcaaacagcaggaaggtgctcgtcagattgcgaggaaagaatggaaagagatcggcaagatcaaggagatcaaagaagggtatctgagcttggtcattcacgagatctccaaaatggtcatcaagtacaacgctattatcgcgatggaagacctctcttacggctttaagaaggggcgctttaaagtggagcgccaggtctatcagaagttcgagactatgcttatcaataagctgaattacttggtctttaaggatatcagtatcaccgagaacggaggactgctgaaaggttaccagctcacatatattcccgataagctcaagaatgtgggccaccaatgcggttgtattttttacgttccagctgcctacacatctaagatcgatcctaccaccggattcgtcaatatatttaaatttaaagatctaaccgttgatgccaagcgtgagtttattaagaaatttgattcaatcaggtacgacagcgaaaagaacctcttctgtttcactttcgactacaacaacttcatcacacaaaatactgtgatgagcaagtcatcatggagcgtttatacttatggtgtaaggataaaaaggcgctttgttaatggaaggttttccaatgaaagcgatacaatagacatcacaaaagacatggagaagacactggagatgacagatattaattggagggacgggcatgaccttagacaggacatcatcgactacgaaatcgtccaacacatttttgagatattcagactcactgtccagatgcgaaacagcctgtcggaactcgaagaccgggactacgatagactgatctccccggtgttaaacgaaaataatattttctacgattctgctaaggcaggagacgctcttcctaaagatgcggacgccaatggcgcttactgtatagcgttgaagggattgtatgagattaaacagatcactgagaattggaaagaagacggtaaattctccagagacaagctgaaaatctccaacaaagactggtttgattttattcaaaataagcgctacctgtaa

SEQ ID NO: 154 - DNA, 3957 bp, Artificial Sequence
  Description of Artificial Sequence: Synthetic polynucleotide
atgacaaacaaatttactaatcagtacagcctgtcaaagaccctccgcttcgaactgattccacaagggaagacccttgaattcatccaggaaaagggtttattatcccaggataaacaacgcgcagaaagctatcaagagatgaagaagacgatcgataaatttcataagtatttcatagatttagccctgagcaacgctaaattgacccacctggaaacctatttggagctgtacaacaagtcagccgagacaaagaaagagcagaagtttaaggacgacctgaaaaaagtacaggacaatttgcgaaaagagatcgtcaagtctttttccgacggagacgccaagtcaatatttgccatcctggacaaaaaggaactcatcactgtggagttggagaagtggtttgagaataatgagcagaaggacatctattttgacgaaaagttcaagacatttactacttacttcaccggatttcaccaaaaccggaagaacatgtactctgttgagccgaactcaaccgccatcgcctaccgccttattcacgaaaatctgccaaagtttctcgagaatgctaaagcctttgagaaaattaagcaggtcgagtcgctccaggtgaactttcgagagctgatgggtgaattcggggacgagggcctgattttcgtgaatgaactcgaagagatgtttcagatcaactactataatgatgtactctcacagaacgggatcactatctacaacagcattatctctggattcactaagaacgatatcaagtataaagggctgaatgaatacatcaacaattataatcagactaaggacaaaaaggacaggctgcctaaattgaaacagctgtataagcagatcctcagtgatagaattagcttgtcatttctcccagatgccttcactgacggaaagcaggtgcttaaggcgatattcgatttctataagatcaacctcctctcttatacaatcgagggccaggaggagtcacagaacctcctgctcctgattcgacaaactattgaaaatctgtcctctttcgatacgcagaagatatacctgaaaaatgacacccatctcactacaatatcccaacaggtattcggagatttctccgtcttcagtacagccctgaattactggtacgagacaaaggtgaaccctaagttcgaaacagagtacagcaaggcgaacgaaaagaagagggagatcctggacaaagccaaagccgttttcaccaagcaagattactttagcatcgcatttctgcaggaagtcctgtctgagtacatactgacactcgatcacacaagcgacatagttaagaagcactcttccaattgtatcgcggactacttcaaaaatcattttgtcgcgaaaaaggagaacgagacagataagaccttcgattttatcgcgaatattaccgcaaagtatcaatgcattcagggtatcttggagaacgccgaccagtacgaagacgagcttaaacaggatcagaagctcatcgacaacctaaagttctttttggacgctatactggaactccttcattttattaagccactacatctgaagagtgagtctatcactgagaaggacactgctttttacgacgttttcgagaattactacgaagcactgtctctgctaacccctctgtataacatggtgagaaactatgtgacacagaaaccttatagtaccgagaagattaagttgaacttcgagaacgcacaattgctgaatgggtgggatgcaaacaaagagggtgattacctcacaacaatcctcaagaaagatggcaattacttcctggccattatggataaaaaacataacaaggcatttcagaaatttcccgaggggaaggaaaattatgaaaagatggtatacaagttgctgcccggggtgaacaaaatgctcccgaaggtgtttttctcgaataagaatatcgcgtactttaacccgtccaaggaactgttggaaaattataaaaaggaaacacacaagaagggggacacttttaatttggagcactgccacacactcattgacttctttaaagatagtctcaacaaacatgaggattggaaatattttgactttcagtttagcgagaccaagtcttatcaggatctgtcgggattttatagggaagttgagcaccagggttacaagataaatttcaagaacatcgatagcgagtacattgacggactggtgaacgaagggaagctgttcctgtttcagatttacagcaaagatttctctcctttctcaaaaggcaagccgaacatgcataccctgtattggaaggccctgttcgaggagcaaaaccttcagaatgtgatttacaagctgaacggtcaggccgagattttttttaggaaggcctctatcaagcccaaaaacatcattctgcacaagaaaaagataaagatcgccaaaaaacacttcattgataaaaagacaaagacttctgagatcgtacctgttcagacaatcaagaatctcaacatgtattatcaggggaagattagcgagaaagagctgacacaggacgatttgaggtacatcgacaacttctctatctttaacgagaagaacaagacaatcgatatcatcaaggacaagcggtttaccgtcgataaattccagttccatgtgcctatcacgatgaatttcaaggccaccggtgggagttatatcaaccagactgtgctggagtatctgcagaacaaccccgaagtaaaaattattggcctggacagaggagagcggcatctggtgtacttgaccctcatcgatcagcagggaaatatcctgaaacaagaatctctgaatactattacggactccaaaatcagcacaccttaccacaagctgcttgataataaagagaatgagagggacttggcccgcaaaaattggggcaccgtcgagaatattaaggaattgaaagaaggatacatctcacaggtggttcacaaaatcgcaaccctgatgttagaagagaacgctattgtggtgatggaggacttaaacttcggatttaaaagaggaagatttaaagtcgagaaacagatttatcagaaactggaaaaaatgctcattgacaaattaaattacctggtgctgaaagataaacagccacaggagctgggtggcctgtataatgctctgcagctgaccaacaagttcgagtcgtttcagaaaatgggcaagcagtcaggcttccttttttacgtgcccgcttggaacacctcaaaaatcgaccctacaacaggctttgtgaattatttctataccaagtatgaaaacgtggacaaggcaaaggcctttttcgagaagtttgaagcaatcaggttcaatgccgagaaaaaatactttgagttcgaggtcaaaaaatatagcgacttcaaccctaaggccgaaggcacgcaacaagcctggacaatatgcacgtatggggagagaattgagactaagcggcagaaggatcagaataacaaattcgtgagcacaccgattaacctgacagagaagatagaggacttcctcggcaagaatcagatcgtgtacggcgacggcaattgcatcaagtcacaaattgcatctaaagatgacaaagcattcttcgaaacactgctgtattggttcaagatgacactccagatgcgaaatagcgaaacaagaacagatattgactacctcatcagccctgtgatgaatgataacggcacgttttacaattcccgggactatgaaaaattagagaacccgacactgccaaaagacgccgacgcaaatggtgcatatcacatcgcaaagaaaggtttgatgctgttgaacaaaattgatcaggctgatctgacaaaaaaggtcgatctgagtatcagtaaccgcgactggttgcagtttgtccagaagaacaaataa

SEQ ID NO: 155 - DNA, 4017 bp, Artificial Sequence
  Description of Artificial Sequence: Synthetic polynucleotide
atggaacaagagtactatctgggcctggacatgggcaccgggagtgtcggatgggcagtcaccgactcagagtaccacgtcctcagaaagcacggtaaggcactttggggagtgcgactcttcgagtccgctagtactgctgaagagaggaggatgtttcgaacttccaggcgcaggctggatcggcgaaactggagaatagagattctccaggagatatttgctgaagagatttcaaagaaggatcctggttttttcctgcgcatgaaagaatctaagtattaccccgaagataaacgcgacatcaacggcaattgtcctgaactgccctatgctctgtttgtcgacgacgatttcaccgacaaagattaccacaagaaattccccaccatataccacctgagaaagatgttgatgaacaccgaggagacacccgacatacgtctggtttacctggctatccatcatatgatgaagcaccgcgggcatttcctgctgtctggagacatcaatgagataaaggaatttggtactacgttctccaagttgttagaaaacattaagaatgaagagttggactggaatcttgaactgggaaaggaagagtatgcagttgtagagtcgattttgaaagataacatgttaaaccggtcaactaagaaaaccaggttaattaaggcactaaaggccaaatcgatatgcgagaaggctgtgctaaatctgctggctggaggcaccgtgaaactgtctgatattttcggcctggaagagctcaatgaaaccgagcggcctaaaatttctttcgccgataacggatacgatgactatattggggaggtggaaaacgagctcggagaacaattctacattattgaaaccgctaaggcagtctatgactgggccgtgctcgtcgagattttaggcaagtacaccagcattagcgaagcaaaggtggctacctatgaaaagcacaaatctgacctccagtttctgaaaaagattgtgcgcaaatacttaacaaaagaagagtacaaggacatctttgtgagcacatcagataagctcaagaattactcagcatacattggaatgacaaagattaacgggaagaaggtggatctccaaagcaaacgttgttcaaaggaggagttttacgatttcataaagaagaacgtgctgaagaaactggagggacaaccggagtacgagtatttaaaggaggagctcgagcgagaaactttcctgcccaagcaagtgaacagagacaatggtgtcattccttaccagattcacttatatgagctgaagaaaatcctggggaacttgagagacaagatagacctcatcaaggaaaatgaagataagttggtccagttgttcgaattcagaatcccatattacgtcggcccgctcaataagatcgacgacggcaaggaaggcaaattcacttgggcggtgcgaaaaagcaacgaaaaaatatacccatggaactttgagaacgtcgttgacatcgaggccagcgccgagaaatttataagacgcatgactaataagtgtacttacctcatgggcgaggatgttctgcccaaggacagcctgctgtattccaagtacatggtgcttaacgagctgaataatgtaaagttagatggtgagaagctcagcgtggagcttaaacagaggctgtacactgatgtgttttgcaagtatcggaaagttaccgttaagaagataaagaattacctgaaatgcgaagggatcatttccggcaacgtggaaattaccggaatcgacggcgattttaaggcgtcgttgaccgcttatcatgatttcaaggagattttaaccggcacggagctcgcgaagaaagacaaggagaacataatcacgaatatagttctgtttggggacgataaaaaacttcttaaaaaacgactcaatcgactgtatccgcagattacccccaaccagctgaagaagatttgcgctctgagctataccgggtggggccggttctctaagaaattcctcgaggagatcacagcaccagacccagagactggtgaggtgtggaatattattacagctctgtgggaatccaataataaccttatgcaattgttgagcaatgaatataggttcatggaggaagtggaaacctacaatatgggcaagcagacaaagaccctatcttacgagaccgttgagaatatgtatgtctccccttcagtgaaacggcaaatctggcaaactttgaagatcgtgaaggagctcgaaaaggtgatgaaagagagcccgaagagggtttttattgaaatggccagagagaaacaggagagcaagagaacagagtctaggaagaagcagctaatcgatttgtataaagcctgcaagaacgaggaaaaagactgggtcaaggagctaggcgatcaggaagaacagaagttgcgctctgataagctgtacttatattatacccagaaaggacggtgcatgtactcaggtgaggtcattgagctgaaagatctgtgggacaatactaagtatgatattgatcacatctaccctcagtcaaaaactatggacgactccctcaacaacagggtgttggttaagaagaaatacaatgctacaaagtccgataaataccctcttaacgaaaacatccggcacgaaagaaagggcttctggaagtccctgctggatgggggttttatcagtaaagaaaagtatgagaggctgatccgaaataccgagctctcccccgaggaactggctggctttatcgaaaggcagatcgtagagactaggcaatctacaaaggcagtcgctgagatcctgaagcaagtgtttcctgagtcagaaatcgtgtacgtcaaagctggcacagtgtcacggttccgaaaggactttgagttgttaaaagttcgggaggtgaatgacctgcaccacgctaaagacgcctatctgaatatcgttgtggggaactcctattatgttaagtttactaagaatgcgtcctggtttattaaggagaacccggggcgcacctataacctgaagaagatgttcacctccggctggaacatagaacggaacggagaagtcgcgtgggaggtgggtaagaaagggaccattgtgaccgtcaaacagattatgaacaaaaacaacatattggtaactcgccaggtgcatgaggccaaagggggcctctttgatcagcagattatgaaaaagggcaaaggacagatcgcaatcaaggaaaccgacgagcgcctggcatccattgagaagtacggaggctacaacaaggcggcaggtgcgtacttcatgctcgtcgagtccaaagataagaaaggcaaaactattagaacaatcgagttcatccctctatatttgaaaaataagatcgaaagtgacgaaagcatcgcccttaacttcttggagaagggccggggcttaaaggaaccaaagattctgctcaagaagatcaagatcgacacactcttcgatgtggatggttttaagatgtggctgtcaggcaggacaggggatcgcttgctgttcaaatgcgcaaatcagttgattctggacgaaaagatcattgtgacgatgaagaagatcgttaaattcattcagcggagacaggaaaacagagaactgaaactctccgataaggatggaattgacaatgaagtcctcatggagatttacaatacctttgtggacaagcttgagaacacagtctatcggatccgactgtccgaacaggcaaagactctgatcgacaaacagaaagaattcgaaagactaagcttagaggacaaaagttcaactctctttgaaattctccacatcttccaatgtcaaagtagtgcagccaacttgaagatgatcgggggtcccggcaaggctggaatcttagtcatgaacaacaacatctccaaatgtaacaaaatctccatcataaaccagtctcccaccggcattttcgagaacgaaattgatttactcaag

SEQ ID NO: 156 - DNA, 3858 bp, Artificial Sequence
  Description of Artificial Sequence: Synthetic polynucleotide
atgaaatctttcgattctttcaccaacctctactcccttagcaaaacccttaagtttgaaatgaggccggtggggaatacacagaagatgcttgacaatgctggcgtctttgaaaaggacaaattaatccagaagaagtatggtaaaacaaagccatattttgaccgattgcatcgggaattcattgaagaggctcttacaggagtagaattgatcggactggacgagaacttccgtaccttagtagactggcagaaggacaagaagaacaacgtggcaatgaaggcctatgagaactcactccagcgccttagaaccgagatcggaaagatctttaatcttaaggcggaagattgggtaaaaaataagtacccgatcctgggactgaaaaacaaaaacacagacatcctgtttgaagaagccgtctttggtatcttgaaggccaggtatggagaggagaaagacacgtttatagaggtagaggagattgataaaacaggcaagagtaagattaatcagatcagtatctttgattcttggaaggggttcacaggctactttaagaagtttttcgaaaccaggaaaaatttctataagaacgatggcacctccacagctatcgcgacacgcatcatagatcagaatctgaaacggttcattgataatctgagcattgttgaatccgtgcgccagaaggtcgacctagctgagactgagaagtctttctctatatcactctcccagttcttctcaatagatttttataataagtgccttctgcaagatggcatagactactataacaagatcatcggcggcgaaactctcaaaaacggtgaaaagctcattggcctgaatgagctcatcaaccaatatagacaaaataacaaggatcagaaaatcccattctttaagctgctagataaacagatcctatcagaaaaaatcctgttcctcgacgaaatcaaaaacgacaccgaactcatcgaggctctctcgcagtttgccaagacggctgaggagaagacgaagattgtgaaaaagctgtttgcagactttgtggagaacaactctaaatacgatttggctcagatttatatctcccaggaagcatttaacacaatctccaataagtggactagcgagactgaaaccttcgccaaatacctgttcgaggccatgaaaagcggcaagctcgccaaatacgagaagaaggacaattcctataagtttcccgatttcatcgcattatctcagatgaagtccgcgctacttagcattagcctggaaggccatttttggaaggagaaatactataagatttccaaattccaagaaaagaccaattgggagcagttcttggctatttttctatacgagttcaactctttgttcagtgacaagatcaacactaaggacggtgagaccaaacaagtggggtactacctcttcgccaaagatcttcataacctgatactgtccgaacagatcgacatacccaaggattcaaaggtgaccatcaaggattttgcggattcggtattgacgatctatcagatggcgaagtatttcgctgtcgagaaaaagcgggcatggctggccgaatacgagttggactccttctatactcaacccgatacagggtacctgcagttttacgataatgcatacgaggatatagtccaggtgtacaataaactcaggaactacctcactaagaaaccatactccgaagaaaaatggaaacttaattttgagaatagtacactggccaatggatgggacaagaacaaggaatcagacaactccgctgtaattctccagaagggtggcaagtattatctgggactgataacaaagggccataacaagattttcgatgaccgttttcaggagaagtttatagtgggcatagagggtggcaagtatgaaaaaatagtctacaagttctttcccgatcaggcgaagatgttccccaaagtatgcttcagtgctaaaggcctcgagtttttccggccatctgaagagatactccgcatctataataacgcagagtttaaaaagggagagacgtactcaatcgactcgatgcagaaactcattgacttctacaaagattgtctcacaaaatacgagggctgggcttgctacacgtttcggcacttgaagccaaccgaggaatatcaaaacaacatcggggagttcttccgtgacgtcgccgaagacggctatagaattgactttcagggcataagtgatcagtatattcacgagaagaatgagaaaggtgagttgcatcttttcgaaatccacaataaagactggaatcttgacaaggctcgcgatggaaaatcaaagactacccagaagaatcttcatacactttacttcgagtccctcttttccaacgacaacgtcgtacagaatttcccaataaaactgaacggccaggccgaaattttttacaggcccaaaaccgaaaaagataaactggaatccaagaaagacaagaagggaaataaggtgatagatcacaaaaggtattccgagaacaagatttttttccacgtacctcttaccctgaacagaacgaagaacgactcttatagattcaatgcccagataaacaactttctcgcaaacaacaaagatatcaatattatcggcgtcgatagaggtgagaagcacttggtatattattctgtgatcacgcaagcatccgatatcttggagtccggttctttgaacgaactgaatggtgtcaactacgccgagaaactcggtaagaaagctgagaatcgggagcaggctagaagggactggcaggacgttcagggtatcaaggacctgaagaagggctacatttctcaggtggttcgaaaactggctgatttggccattaagcacaatgcaatcatcattttagaagatttgaacatgcggtttaaacaagtcaggggggggatagagaaatcaatttaccaacagctggaaaaagctctgattgataaactctcttttttggttgataagggcgaaaagaaccccgagcaagcaggacatctccttaaagcctatcaactgagcgcacctttcgagacattccagaagatgggaaagcaaaccggcatcattttctatacccaggcttcctatacatccaagtctgatccagtgactgggtggagaccccatctctacctcaagtacttttctgccaaaaaagctaaggacgacattgctaagttcacaaaaatcgagttcgtgaacgacaggttcgagctgacttatgacataaaagatttccagcaggccaaggagtacccaaacaagacagtttggaaagtgtgttccaatgtggagaggtttcggtgggacaagaatctgaatcagaataaagggggatatactcactacaccaacattaccgagaacatccaagagttgttcaccaaatacggcatcgacattactaaagatctgctgacacagatctccaccatcgatgagaagcagaacacatctttcttccgggatttcatcttttattttaacttgatctgtcagattagaaataccgacgacagtgagatagctaaaaaaaacgggaaagacgatttcattctctctcccgtggagccgttttttgactcccgcaaagacaatggcaataagcttccggaaaacggggacgataacggcgcctacaacatcgctcgtaagggaatcgttatcctcaataaaataagccagtattccgagaagaacgagaattgtgaaaaaatgaagtggggggacctttacgtcagcaacatcgattgggataactttgtgacacaagccaatgcgagacactag

SEQ ID NO: 157 - DNA, 3465 bp, Artificial Sequence
  Description of Artificial Sequence: Synthetic polynucleotide
atggaaaacttcaaaaacctctaccccatcaacaagaccttgaggtttgagctccggccatatgggaagacactggagaacttcaaaaagtccggtctgctggaaaaggatgcttttaaggctaactctaggaggtctatgcaggccattatcgatgagaaattcaaggagaccatagaggagcgtctgaaatatactgagttttccgagtgtgacctaggaaatatgaccagtaaggacaaaaagatcaccgacaaggcagcgacaaacctgaagaaacaggtgattttaagctttgatgatgagattttcaataactacttgaagccggacaaaaacatcgacgctctgttcaagaatgatccaagcaacccggtcatctctactttcaagggcttcaccacatactttgtaaatttcttcgaaatacggaaacacatcttcaagggagagtcttccggtagcatggcttacagaataatcgatgagaacctaactacatatctaaacaatatcgagaagatcaagaaattgcctgaagaactgaaatctcagcttgagggaatcgatcaaattgacaaactgaacaactataacgagttcatcacccagtccggcattactcattataacgaaattattggagggatttcgaagtctgaaaatgtcaaaattcaaggcattaacgaagggattaatctttactgtcaaaagaataaagtgaagctaccacgcttaactcctctgtataagatgattctctctgatcgggtctctaattcctttgtgctggataccattgaaaatgataccgagttaattgaaatgatctctgatctgataaataagacagagataagtcaggatgttattatgtccgacatccaaaatattttcatcaaatataaacaactcggcaacttgccggggattagctactcatctatagtgaatgctatctgttcggattacgacaataactttggtgacggcaaacgtaaaaaaagctatgagaatgatcgcaaaaaacacctcgagactaacgtgtatagcattaactatatctcagagttactgacagacaccgacgtctccagcaacataaagatgcggtacaaagagctggagcagaattatcaggtatgcaaggaaaatttcaacgccactaactggatgaacatcaaaaacattaagcagtctgagaaaaccaatctgatcaaggaccttcttgacatcctcaagagcatccagcggttttatgatttgtttgacatcgtggatgaagacaaaaatcctagtgctgagttctatacctggctgtctaaaaacgcggagaaactggacttcgagtttaattcagtgtacaacaagagcaggaactacctcacgagaaagcagtactccgataaaaagattaagttgaacttcgatagtcctactctcgccaaggggtgggatgcgaacaaagaaattgataatagcacaattatcatgaggaagttcaacaacgaccggggcgattacgattacttcttggggatctggaataagagcacacctgccaacgaaaagatcatcccattagaggataatggactgtttgaaaaaatgcaatataagctgtatcccgatcctagtaaaatgctgccaaagcaattcctttctaagatctggaaagctaaacatccaactacacccgagtttgataagaagtacaaagaaggtcggcacaagaaggggcctgattttgagaaagagtttctgcacgagttgatcgattgctttaagcatggattggtaaaccacgacgaaaaatatcaggatgtgttcgggttcaatctgcgcaacacggaagactacaactcttatacagagtttctggaggacgtcgaaaggtgcaactataatcttagtttcaataaaatcgctgacacgtctaacttgataaatgatgggaaactctatgtttttcagatctggagcaaggatttcagcatagatagcaagggaacaaaaaacttgaacacaatatactttgaatccctcttctcggaggaaaatatgatcgagaagatgttcaagctctcaggggaagccgaaatattctatcgtccagcaagtttgaattattgtgaagatattatcaagaagggacaccaccacgccgaactgaaggacaaattcgactatcccatcatcaaggacaagcgatatagccaggacaaatttttttttcatgtccccatggttatcaactacaaaagcgagaagttaaactccaaatcacttaacaataggacgaacgaaaatttaggccaattcacgcacatcatcggtatcgaccgcggagagcgacatctcatctacctgaccgtggtggatgtgtccaccggtgagatcgttgagcaaaagcacctggatgaaattataaatacagatacaaaaggcgtcgagcataaaactcattatctcaataaattagaagagaagtccaagacgcgggataatgaaagaaagtcctgggaagcaatcgagacgattaaggagctgaaagaaggctatattagccacgtgatcaatgaaatccagaaattgcaggaaaagtataacgcactgatagtgatggagaacctcaattatgggtttaagaactcgcgtatcaaagtggaaaagcaggtctaccagaaattcgagaccgccctgattaaaaagtttaattacatcattgacaagaaagatcctgaaacctacattcatggataccaactgacgaatccaatcactacactcgataaaattggtaaccagagcggtattgtgttgtacattccggcttggaatacaagcaagattgatccagtcactggtttcgttaacctcctgtatgcagacgatttgaaatacaagaaccaggagcaggctaaaagctttatccagaaaatcgataatatctacttcgaaaatggtgagtttaaatttgatatagatttcagcaaatggaacaaccgctactcaattagcaagacgaaatggacactgacaagctacggaacccggatacagacgttccgaaacccccagaaaaataacaagtgggacagcgccgagtatgacctgaccgaagagtttaaattaatcctgaacatcgatggtactctgaaatctcaggatgtggaaacctataagaaattcatgtctttattcaagctgatgttgcagctgcgaaactccgttactggaacagacattgactacatgattagccctgtgacagataaaactggaacccactttgattcacgggagaatatcaagaacctgcccgccgatgctgatgcgaacggagcttacaacattgctaggaagggcatcatggcaatcgagaatattatgaacggcattagcgaccctctgaagatcagtaatgaggactacctgaagtacattcagaaccaacaagagtaa

SEQ ID NO: 158 - DNA, 3924 bp, Artificial Sequence
  Description of Artificial Sequence: Synthetic polynucleotide
atgacccagtttgagggtttcaccaatctttatcaggtgtcaaaaacactcagatttgagctcatcccacagggtaaaactttaaagcatattcaagagcagggctttatagaggaagacaaagccagaaacgaccattataaggaactaaaaccgatcattgaccgcatctacaaaacctatgccgaccaatgccttcagctcgtccaactcgattgggagaatctgagcgccgctattgacagctacaggaaggagaagaccgaggagactagaaacgccctgatcgaggagcaggcgacctatagaaacgctattcacgattattttatcggccgcaccgacaatttgacagatgccatcaacaagcggcacgccgaaatttataaggggttatttaaggccgagctgttcaatggaaaagtactgaaacagctgggcaccgtaacaaccaccgaacacgagaatgctctgttgaggtccttcgacaagtttactacctactttagcggcttctacgaaaaccgtaaaaacgtgttttccgcggaggatatttcaacagccattcctcataggatcgtgcaggataatttccccaagtttaaggagaactgccatatctttaccagacttatcactgctgtgccaagtttacgagaacacttcgagaatgttaagaaggctataggcatattcgtttccacctccatcgaagaagtattcagttttccattctacaatcagttactcacgcagacccagatagatctctacaatcagctgctcggaggcatttctagagaagcaggcacggaaaagatcaagggcttaaatgaagtactcaatcttgcaattcagaagaacgatgagacagcacacattattgcatctctccctcacagattcattcccctgttcaaacagatcctgtccgatcgcaacacactaagctttatacttgaggagtttaagtcagatgaggaagtgatccagagcttctgtaagtataagactttgctccgtaatgaaaacgtgcttgagacagcagaggctctctttaacgagttgaattccatcgacctgacacacatttttatcagccataaaaagctggaaacgattagctctgccttgtgcgaccactgggacaccctgcgtaacgccctctatgaaaggcgcatttccgagctcaccgggaagatcacaaaaagtgccaaggaaaaagtccagaggtcccttaaacatgaagacatcaacctacaagagatcatctctgcggctgggaaagagctgtcagaagcatttaaacagaagacttccgagatcctgagccacgcacacgccgcattagaccagcccctgcctacaactcttaaaaaacaggaggagaaggagattttaaagagccagctggactcattactcggcctgtatcatctcctggactggttcgccgtggacgaatccaacgaggtggacccagaatttagcgccaggctgacaggaattaaactggaaatggagccaagtttgagcttttacaacaaggctcggaactatgccactaaaaagccctacagcgtggaaaagttcaagctgaattttcagatgccgaccctggcttccgggtgggatgttaataaggaaaagaataatggggctatactgttcgtcaaaaatggtctctactacctgggaatcatgcccaaacagaagggcaggtacaaagccctttcgtttgagccgaccgaaaaaaccagcgaaggctttgataagatgtattacgactatttcccagatgcagccaagatgatcccaaaatgtagcactcagttgaaggcggtaaccgctcactttcagacacacaccactcctatcttgctctccaacaactttattgagccgctggagatcacgaaggaaatctacgaccttaacaacccagagaaggaacccaagaaattccaaacagcttatgctaagaagactggggatcaaaagggctatcgagaggctttgtgtaagtggattgactttacacgggatttcctgagtaagtataccaagaccacatctattgacctgtcctcactgagaccttcctcacaatataaggatctcggagagtattatgccgaactcaaccctctactctatcacatctctttccagaggatcgccgaaaaggaaattatggacgccgtcgagacaggcaagctgtacctcttccagatttacaacaaggatttcgcaaagggccaccacggaaaacccaatttgcacactttgtactggacagggctcttctctcccgaaaatttggccaaaacttcaataaaactgaacgggcaagccgagctgttctatcggcccaagtcacgtatgaagcggatggcccaccggctgggcgagaagatgctcaacaagaaactgaaggatcagaagacgcccataccagacactctttaccaagagctgtatgactacgtgaatcacagactgagtcacgacctgtctgatgaagcccgggctcttcttccaaatgtgattaccaaagaagtttcccacgaaattatcaaggaccggcgcttcacctctgacaaattctttttccacgtcccaatcaccctcaactaccaggcagccaattccccttcaaagtttaaccagcgtgtgaatgcctacctgaaagagcatccggagacccccatcatagggatagacagaggagagcggaatcttatctacattactgtgattgacagcacaggtaagatcttggagcagagatctttaaatacaatccagcagtttgactaccagaagaaactggataaccgagagaaggaaagggttgctgcaagacaggcctggtcagtggtcggcaccatcaaagacctgaagcagggctacttatcccaagtaattcacgaaattgtcgatcttatgattcattatcaagccgttgttgtgctggagaacctgaattttggcttcaaaagcaaacgaacaggtatcgccgagaaagccgtgtatcagcagttcgaaaagatgctcatagacaagctgaactgcttagtgctgaaggattatcctgctgagaaggtcggcggcgtacttaacccataccagctgaccgatcagttcactagtttcgccaagatgggaacgcaaagtggcttccttttctacgtgcccgctccctacacgagtaagatcgaccctctgaccggcttcgtcgacccattcgtctggaagaccatcaagaatcacgaatcacggaaacacttcttagaggggtttgacttcctgcactacgacgtgaagacaggggacttcatcttacactttaagatgaatcgaaacctctccttccagcggggcctgcctggtttcatgcccgcatgggacatcgtgtttgagaaaaacgagacacagtttgacgctaagggaaccccctttattgcggggaagcggattgtcccagtcatcgaaaaccatcggttcaccgggcgataccgggatctgtacccggccaacgagctcatcgcgctgctggaggagaagggtattgtgtttagggatggatccaacattctgcctaagttgctggaaaatgatgattcgcacgccattgataccatggttgcactgattagatccgtactgcagatgaggaatagcaatgctgcaaccggggaggattatattaattccccagtgcgagatctgaatggtgtctgttttgactcgcgctttcagaatccagaatggccaatggatgcagacgctaacggggcgtaccacattgctctgaaaggccagctactcctgaaccacctcaaggagagcaaagatctgaagctgcagaacggcatttccaaccaagactggctcgcctacatacaagaactgcgcaattaa

SEQ ID NO: 159 - DNA, 3390 bp, Artificial Sequence
  Description of Artificial Sequence: Synthetic polynucleotide
atggctgtcaaatccatcaaggttaaattacggcttgatgacatgcccgagatccgcgccgggctctggaaactccataaagaagtgaatgctggcgttagatactacacagaatggctctccctgctgcgccaggaaaatttgtaccgccggtcacctaatggagatggagagcaggaatgcgataaaacagcagaagagtgcaaagccgaattgctggagcgactgcgggcacggcaggttgagaatggacaccgaggtccggcgggatcggacgacgagctgctccagctcgccagacaattatatgaactgctggtgcctcaggctattggggcaaagggtgacgcacagcagattgctagaaaatttctgtctcccctcgccgacaaagacgctgtcggcggccttgggatagccaaagccggcaacaaaccccgatgggtgcgcatgagggaggctggtgagcctggctgggaggaagaaaaggaaaaggccgaaaccagaaagtccgccgacaggaccgcggacgtactccgagcattggccgattttgggctgaagcccttaatgcgagtctacaccgatagtgaaatgtctagcgtggagtggaagccattacgcaaagggcaggcagtgcggacgtgggaccgtgacatgttccagcaagccatcgagcgaatgatgagctgggagagctggaaccagagagtggggcaggagtatgccaagctggtcgagcagaaaaaccggtttgagcaaaaaaattttgtaggtcaggaacacctggtgcatctcgttaaccagctccagcaagatatgaaggaagcttcgcctggattagagagcaaagagcagactgcacactatgtaaccggaagagcactgaggggcagtgacaaagtgttcgaaaaatggggaaaactggctcccgatgccccctttgacctgtacgacgcagaaataaaaaacgtgcagcggcgaaacaccaggcgatttggtagccatgatctgttcgccaaattggcagagccggaatatcaggctctttggcgagaagacgcatcatttctcactaggtacgcggtctataactccattttgaggaaattgaaccacgcaaaaatgtttgccaccttcacgttgcctgacgccaccgctcatcccatttggacacggtttgataagctgggcggcaatctgcatcagtatacattcctgtttaacgagtttggagagcgaagacatgcgatacgattccacaagctactgaaggtcgaaaatggcgtggcacgtgaggtggacgatgtcaccgtgcccatcagcatgagcgaacagctggataatttgttgccgcgggacccaaatgaacctatagccctttattttagggactacggggcggagcaacatttcactggggagtttggcggcgcaaaaattcagtgccgacgcgaccagctcgcccacatgcatagaagacgcggggcccgggacgtataccttaacgtctctgtgagggtgcagtcccagtcagaggcaagaggggaacgcagaccaccttacgcagcagtattcaggctggtaggcgataaccaccgggcgtttgtacactttgataaactttctgactacctggccgaacacccggatgacggcaaattaggatcggaggggctgcttagcggcctgcgtgtgatgagcgtcgatctggggctacggacctctgcttccatctctgtgttccgtgtggcccgaaaggacgagttgaaacctaattcgaagggccgtgtaccattctttttccctattaagggaaatgataatctcgtcgcggtgcacgagcgttcccaactgctgaaactgcctggcgagaccgagtccaaagatctcagagcaatccgggaggagcgacaacgtacacttaggcaactccgcacccagctggcctatctgcgcttgctggtgcggtgcggctccgaggatgtagggagaagagagcgaagctgggcaaagctgatagagcaaccagttgacgccgcgaatcacatgacccccgactggcgcgaagcgtttgaaaatgagctgcagaagttgaaatctctgcatgggatttgctcagataaggagtggatggacgccgtatacgagtctgttcgccgggtatggcggcacatggggaagcaggtgagagattggagaaaggacgttcgctctggggaacggccgaaaattcggggatacgcaaaggatgtcgtgggcggcaatagcattgagcagatcgagtacctggaaaggcaatacaaatttctgaaatcttggtctttctttgggaaggtaagcggacaagttatcagagccgaaaagggatctcgctttgctatcacattgagggaacacattgatcacgccaaagaagacaggttgaaaaagttggctgatcgcattatcatggaagcactcggttacgtctacgcccttgatgagcgcggtaaagggaagtgggtagccaagtatcccccatgtcagctgatcctgctcgaggaactttctgagtatcagttcaataacgaccgtcctccctccgaaaataatcagctcatgcaatggtcccaccggggtgtgttccaagaactgatcaatcaggctcaggtgcacgacctcctcgtaggcactatgtatgcagcctttagctcccgttttgacgcgcgcacaggcgcccctggaatacgatgtaggcgagttcccgcacggtgcactcaagaacataacccggagcctttcccatggtggctcaataagtttgttgtggagcataccctcgacgcttgcccattgagggcggatgacttgattcccacaggcgagggggagatcttcgtgagcccattttctgccgaagaaggggatttccaccaaatacatgccgacttgaatgctgcccaaaatctgcagcaaaggctgtggtcagacttcgacatctcgcaaatcagactgcggtgtgactggggcgaagtagacggcgagctggtgctgatacctagactgacgggtaagcgtaccgccgatagctatagtaataaggttttttatacgaatacgggggtgacatattacgagcgtgagagaggcaagaagcgtcggaaggtgttcgcgcaggagaagctgagcgaagaggaggcggagctactggtagaggcagatgaggcaagagaaaagtccgtcgtcctgatgcgggatcctagcgggattattaacagaggtaattggacacggcagaaagaattctggagcatggtgaatcaaagaatcgagggttacctggtgaagcaaattcgaagccgggtgccccttcaagacagcgcatgtgaaaacactggggacatctag

SEQ ID NO: 160 - DNA, 3327 bp, Artificial Sequence
  Description of Artificial Sequence: Synthetic polynucleotide
atggctactcggtccttcatcctgaaaatcgagccaaatgaagaggtgaaaaagggcctgtggaagacccatgaggtacttaaccacggcatagcatactatatgaatatcctaaaacttatacggcaggaggctatctacgagcatcacgagcaagatcctaaaaatccaaagaaggttagtaaggctgaaatccaggctgaattgtgggacttcgtgctgaagatgcagaaatgcaacagtttcacgcatgaagttgataaggacgtcgtgtttaatatactccgggagctgtacgaagaactggtaccaagctctgtggaaaagaaaggagaggccaaccagctaagtaataagttcctctatcctctcgtggaccccaattcacagagcggcaaaggtaccgcatcttctgggaggaaaccacgctggtacaacttgaagatcgctggcgatcccagctgggaggaggaaaagaagaaatgggaagaggataaaaagaaagaccccctggccaaaatcttaggcaagctcgccgagtacggtctgattccacttttcatcccgttcacagatagcaatgagccgatcgtcaaggagattaagtggatggaaaagagccgcaatcagagtgtgcggaggctggacaaagacatgtttattcaggccctggaacgcttccttagctgggaaagctggaacctgaaggttaaggaagagtacgaaaaagtcgagaaggagcataagactttggaggagcgcatcaaagaagacatccaggcctttaagtctctagaacagtatgagaaagaacggcaggaacagctgctgcgtgatacactgaacacaaacgaatatcgcctgagcaagaggggactcagaggctggagagaaatcattcaaaagtggctcaaaatggatgaaaatgagccgtctgaaaaataccttgaagttttcaaggactaccagcggaagcaccctagagaagccggcgactatagtgtttacgaattcttgagcaagaaggagaatcattttatatggaggaatcacccggagtacccatatctgtacgcaaccttctgcgaaatcgacaagaaaaaaaaagacgccaagcaacaggctacatttactctggccgaccctatcaatcaccctctatgggtccggtttgaggagcgctccggaagcaatctgaataaatatcgtattctgactgaacagttacacacagagaagctcaagaagaaacttacggtgcagctggaccgcctgatatacccaacagagtccggaggatgggaagagaaaggaaaggttgacatcgtactgcttccatctcgtcagttttacaaccagatattcctggacatcgaggagaaggggaaacacgccttcacatacaaggacgagtccataaagttcccactgaagggtactttaggcggtgctagggtgcagttcgaccgcgatcacctgagacggtacccccacaaggtggagagcgggaacgtgggacgaatctactttaatatgacagtgaacattgaacccacagagagtccagttagtaaatccctgaaaattcaccgtgacgactttccgaaatttgtgaatttcaagccaaaggagcttacggagtggatcaaggattcaaagggaaagaagctgaaatctggtatcgaatctctcgagatcggtctccgtgtcatgagcatcgatctgggacagcgccaggcagctgccgccagtatattcgaggtggtagaccaaaagcctgacatcgagggaaagctcttcttcccaatcaaaggcacagagctgtatgcggtgcaccgggcgtcctttaatataaagctgcccggtgaaaccctggtgaagtcacgggaggtgcttagaaaagcgcgagaggataacctcaaactgatgaaccaaaaactgaactttctgaggaacgtcctgcactttcagcagttcgaagatattaccgaacgcgaaaagagagtaaccaagtggatatctcgtcaagagaacagcgacgtcccgttagtctatcaggacgaactcatccaaatacgggagttgatgtataagccctacaaggattgggtcgcctttcttaagcagcttcacaaacgcctagaggtcgaaataggtaaagaggtgaaacattggcggaagtcgctcagcgacgggaggaagggactttatggcatctctttgaagaacattgacgaaatcgatagaaccagaaaatttttgttgagatggtccctccgacccaccgagcctggagaggtgaggcggttagaaccaggacagaggttcgctatcgatcagctgaatcacctcaatgctctgaaggaggaccgcctcaagaaaatggccaatacaatcataatgcacgcccttggctactgctacgacgtccgaaagaagaagtggcaggccaagaatcccgcctgtcaaattatcctttttgaggatcttagcaattacaacccctatgaagagcggtccagattcgaaaatagtaagctcatgaagtggagccgcagggagatcccgcgccaagtggcccttcagggggaaatttatgggctgcaggtaggcgaggtcggggcccaattctcctcgcgctttcatgcgaaaactggaagtcctggaatccggtgctcagtggtgacaaaggagaagttgcaagacaatcggttttttaaaaacttacagcgggagggaaggctgaccctggataagatagccgtacttaaggaaggagatctgtaccctgacaaaggcggtgaaaagttcattagcttgagcaaggaccgaaaacttgtgaccacccacgctgacatcaatgcggcacagaacctgcagaagagattttggactcgcacccacggattctacaaagtttactgcaaagcatatcaagtagacggacagaccgtatacatccccgagtccaaagatcagaagcagaaaattattgaagagtttggggaagggtactttatcctgaaggatggtgtctacgaatggggcaacgctggtaaacttaaaattaagaagggcagctctaaacagtcctccagcgagttagttgattctgatattctgaaagacagtttcgacctggccagcgaacttaaaggggaaaaattaatgctgtaccgggaccccagcggaaacgtctttccatccgataagtggatggccgctggagtgttctttggcaagttagagaggattctcataagtaagctgaccaaccaatactcaatctccacaatcgaggatgactcatccaagcagtctatgtga

SEQ ID NO: 161 - DNA, 3450 bp, Artificial Sequence
  Description of Artificial Sequence: Synthetic polynucleotide
atgcctacacgcactatcaacctgaaactggttcttggcaagaatccagagaatgctacccttcgtcgggcactattttcaacgcatagactggtgaatcaggctaccaaacggattgaagagttcctcttgctttgtcggggggaagcatataggacggtggataatgaggggaaagaggctgaaattccgagacacgccgtgcaggaggaagctcttgcgtttgcaaaggccgctcaacggcacaatggttgcatctctacttatgaagaccaggaaatcctggatgtgctccggcaactgtatgaaaggctggtgccttctgtgaatgaaaataatgaagcaggggacgctcaagccgcaaacgcgtgggtgtcgccactgatgtccgccgagtccgagggagggctcagcgtttacgacaaggtgctggacccacccccagtgtggatgaaactcaaagaggaaaaagctccgggctgggaggctgcttcccagatctggatccagtccgacgaagggcagtcccttcttaacaagcctggttcgcccccgcggtggattaggaaactgaggtcaggccagccttggcaggacgattttgttagcgaccagaaaaagaagcaggacgagctgacaaaggggaatgcgccactgatcaaacaattaaaggaaatgggcttattgcctcttgtgaatcccttttttagacatctgcttgacccggaggggaagggggtgtcaccttgggacagactcgctgttagggccgctgtcgctcatttcatatcatgggaatcatggaaccaccggacacgcgccgaatacaatagtttgaagctgcggagggatgagttcgaagcagcttccgacgaattcaaggacgacttcacgctgcttcggcagtacgaggctaagaggcactccacactgaagagtatagctttagccgatgattcaaacccttataggatcggcgtacgctccctccgcgcttggaaccgcgtccgcgaggagtggatcgacaagggagcgaccgaggagcagcgggtcaccattctcagcaagttgcagacccaactaaggggcaaatttggagatcctgacttgttcaactggctggcgcaggaccggcacgtgcacctctggagccctagagatagtgttaccccactggttaggatcaacgctgttgacaaagtattgcgacggagaaaaccgtacgccttgatgacttttgcccacccaagattccaccctcggtggatactttacgaagccccagggggcagcaatctccgccagtatgcactggattgtaccgaaaatgctctgcacattacactgcctctgctggttgacgatgcacatggcacatggattgagaaaaaaattagggttcctcttgcccccagcggccagattcaggacctgacactagaaaagctcgagaagaagaaaaatcgtctctactaccgttctgggttccagcagtttgccggcctggccggaggtgccgaggtgcttttccatcgaccatacatggagcacgatgagaggagcgaggagagcttattagaacgccctggtgctgtttggttcaaactcaccttggacgtggcaacccaggcccctccaaactggttggacggaaagggccgcgtccgaacgccccccgaggttcaccacttcaagacagccctcagtaacaagtctaagcacacacggaccctccagcccggactcagagtgttatccgtggatctgggaatgcgcaccttcgcctcttgctccgtatttgagctgatcgagggcaaaccagagactggcagagcgttccctgtggccgacgaacgttccatggattcaccaaacaagctgtgggccaagcacgaaagatcctttaaactcacgctccccggcgaaacccccagtcggaaagaagaggaggaacggagcattgcaagagccgaaatctatgcgttgaaaagagatattcagagattaaaaagtcttctgcgcctgggggaagaggataacgataatagacgcgatgcacttcttgagcaatttttcaagggctggggcgaggaagacgtggttccaggtcaggcctttccccggagtctgttccaggggctgggggccgccccattcagatccacccctgagttgtggagacaacactgtcaaacctattatgataaagcagaggcgtgcctggctaaacacatcagcgattggcgcaagagaaccaggcctaggcctacctcacgtgagatgtggtacaagacacgctcttatcacggcggaaagtcaatctggatgctggaatacctcgacgctgtgaggaaactgctcttatcctggagcctcagaggccggacctacggggctatcaacagacaggacacagcaaggttcgggagcttagccagccggctccttcaccacattaactcactcaaagaggatcgaataaagaccggagccgactcgatcgtgcaggcagcccgagggtacatccccctgcctcatgggaagggctgggagcagcgatatgaaccctgccagctgatcttgtttgaggaccttgcccgttatagatttcgcgttgatagacctcgccgtgagaattctcagctgatgcagtggaaccacagagcgatcgtggctgagaccactatgcaggccgagctgtatggacagatcgtggagaacaccgccgcagggttcagttctcggtttcatgctgccaccggagctcccggcgtccggtgccgcttcctcttagagcgtgattttgacaatgacctcccaaagccctatctgctgagggaactgagctggatgctggggaacacaaaagtagaatcggaggaggagaagctacggctcctctccgaaaagatacgtccaggctctctggtaccatgggacggaggagagcagttcgcgacactgcatcctaagagacagacgttatgtgtgattcacgccgatatgaacgccgctcagaatctgcagcgaagattctttggccgctgcggcgaagccttcaggctggtatgtcagccccacggggatgatgtgctgcggctggcctcaacccctggggctagactcttgggggcactccagcagctggaaaatggccaaggggctttcgaactcgttcgggacatgggcagcacaagccagatgaacagattcgtcatgaagagcctgggaaagaaaaagatcaaacccttacaggacaataatggcgacgacgaactggaggacgtgttgtccgtgctgccagaggaagacgacacaggccgcatcactgtcttccgcgactcaagtgggatattctttccttgcaacgtgtggattccggccaaacagttctggcctgccgtcagagccatgatttggaaagtgatggctagtcattcattgggatga

SEQ ID NO: 162 - DNA, 3759 bp, Artificial Sequence
  Description of Artificial Sequence: Synthetic polynucleotide
atgacaaagctgaggcacagacaaaagaagcttacacacgactgggcagggagcaagaaacgtgaggtccttgggtcaaatggaaaactgcagaaccccttgctcatgcctgtaaagaaggggcaggtaacagaatttagaaaagcattctccgcgtacgctcgggcaactaagggggaaatgaccgatggacggaagaacatgttcacccattctttcgagccattcaaaacaaagccgtcattgcaccaatgcgagctggccgataaggcttaccagtctttgcatagttacctccccggttccctggcccatttcttgctttccgcacacgcactgggctttcgtattttctctaaatctggggaggcaactgccttccaggccagctcaaaaatcgaggcctatgagtccaagctcgcttcggagctagcctgtgtcgatttgagtatccagaatttgacgattagtactcttttcaacgctctcacaacttcagttcggggcaagggggaggaaacttcagcagatccccttatcgcacggttctacactctcctgacgggcaagcccctgagccgagacacacagggcccagaacgggacttggcagaggtcatctccagaaagatcgcctcgtccttcggcacatggaaggaaatgactgccaaccctctgcagagcctccagttcttcgaagaagagcttcatgcactagatgccaacgtgtctttatctccagcttttgatgtgttaatcaagatgaatgatctccaaggtgatctgaagaaccgtactatagtgttcgacccagatgcacccgtgttcgagtacaacgctgaggatccagccgatatcatcataaagctgacagctcggtatgcgaaggaggccgtcatcaagaatcagaacgtgggcaattatgtgaaaaacgccattaccaccactaatgccaatgggctggggtggctcctcaataaagggctttcactactgccagtttctactgacgatgagctgctcgaattcattggggtggagagaagccatcccagctgtcacgcgctgatagagctgattgcccagctagaggcgccggaactgtttgagaagaatgtgtttagtgacacccgttccgaggttcagggtatgatcgacagtgcagtgtcgaaccacattgctcggctgtccagcagccgaaactccctgagcatggacagcgaggaattggaacgcttgattaaatctttccagattcatactccccattgttctctgttcataggcgctcagtccttatctcagcagctggagagcttacctgaggcgctgcagtccggagtgaacagcgctgatatcttattaggcagcacacagtatatgctgaccaactctctcgttgaagagtcaattgcaacatatcaaaggacattaaataggatcaattacctgagtggggtggctgggcagattaacggtgctatcaaaagaaaggcaatcgacggcgaaaaaatacacctgcctgccgcctggagtgagctcatctccttacctttcattggacagccggtgattgatgtggagagcgacctggcacacttaaaaaaccagtaccagaccctgtccaatgaatttgacaccctcatttcggccctgcagaagaacttcgatttgaatttcaacaaagcactccttaaccgcacgcagcatttcgaggcaatgtgccggagcacaaaaaaaaatgctttatctaagcccgagatcgtgtcctacagagatctgctggcgcggctgaccagttgcctttatcgaggctcgctggttctcagaagggcgggaatcgaagttctgaaaaagcacaaaatctttgagtcgaatagtgagctgagagaacacgtccacgagcgaaagcacttcgtgttcgttagtccattggacagaaaggcaaaaaaactgttgcgcctgaccgattcccgccctgacttgctccatgtgatcgatgagatcctgcaacatgacaatctggagaataaggacagagagtccctttggctggtccggtctgggtacctccttgctggtctgccggaccagctgagttcttcgtttatcaatctccccataatcacgcaaaagggcgatcgccggctgattgacctgattcagtatgaccagatcaatcgcgatgctttcgtaatgttggtgacaagtgctttcaaaagcaatctctctgggttgcagtaccgcgctaacaagcagtctttcgtggtcacccgcaccctgtctccttacctgggtagtaagctcgtatacgtccctaaagacaaagattggctggtcccatcccagatgtttgagggaagattcgccgatattctgcagagtgactacatggtctggaaggatgccggacgcctgtgcgtgatcgacactgccaaacatctctctaacattaaaaaaagcgtgtttagtagcgaagaagtccttgcttttcttcgagagctgcctcaccggaccttcatccagaccgaggtacgggggttaggagtgaacgtcgatggaatcgcatttaataacggggatatcccgagcttgaagacattctcgaattgtgtgcaggtgaaggtgagtaggactaatactagtctcgtgcagactctaaacaggtggttcgagggtggcaaagtgtcacctccctctattcagttcgaaagagcttactacaaaaaagacgatcagattcacgaggacgcagccaagagaaagatacgcttccagatgccagcaacggaattagtgcacgccagcgatgacgctggttggacccccagctacctgctgggcatcgaccccggtgagtacggaatgggtctcagtttggtgtccatcaacaatggagaggtcctggattctggattcatccacattaattccctgatcaatttcgcgtccaaaaaaagcaatcaccagaccaaagtagtcccccgccagcagtacaagtccccctacgcgaattatctcgagcagtcaaaggattcagcagcaggggatatagctcacattctggatcggctaatctacaaattgaacgccttgcctgtgttcgaggcgctgtctggcaacagtcagagtgctgctgatcaggtatggaccaaagttctatccttctatacatggggagacaacgacgcacagaacagtatacggaagcagcactggttcggtgcctcacactgggatattaaggggatgctgcgccaacccccaaccgaaaaaaaacccaaaccatatatagcctttcccgggagtcaagtgtcatcctatggaaatagtcaaaggtgtagttgttgcggccgcaatcccattgagcagttgcgtgagatggcaaaggacacgagtatcaaggagctgaaaatccgaaatagtgagatccaactattcgatggtacaatcaagctgtttaaccccgacccttccaccgtcatcgagaggcggcggcataacctaggaccctcacgcattcctgtggcagaccgaactttcaagaatattagcccttcttcgttagagttcaaggagctcattactatcgtttctcgaagcatccgccatagccccgaatttattgctaagaaacggggtatcgggtctgagtacttttgtgcttattctgactgcaactcctcactgaactcagaggccaatgccgcggccaatgtggcacagaagtttcagaagcaactctttttcgaactctga

SEQ ID NO: 163 - DNA, 3864 bp, Artificial Sequence
  Description of Artificial Sequence: Synthetic polynucleotide
atgaaacgtattctgaactctctgaaagtcgccgcactgaggctgctgtttcgaggaaagggctcagagctggtgaagaccgtcaagtaccctctggtttcgcccgtccagggtgctgtggaagaactcgccgaagcaatacgccacgacaacctacatttatttgggcagaaggaaatcgtagatctgatggagaaggacgagggcacccaggtctactcggtggtggacttttggctcgacacactccgtctagggatgttcttcagtccaagtgctaatgcccttaagatcactctggggaagtttaacagcgaccaagtttcccctttcaggaaggttctggagcagtcccctttctttctcgcgggtagactcaaagtggagcccgctgaacgtatcctcagcgtggagatccgcaagatcggtaagagggagaatagagtggagaactacgccgcagatgtagagacttgttttatcggtcagctgtctagtgatgaaaagcagtctatccagaagctcgctaacgatatctgggactctaaggatcacgaagagcaaaggatgcttaaggcggatttctttgccattcccctcatcaaagacccaaaggcagtgaccgaggaagatcccgagaatgaaaccgcaggcaaacagaagcctctcgaattatgtgtgtgcttagtgcccgagttgtacacccgcgggttcggttcaatagcggacttcctggtccagcgtctgacactattaagagacaaaatgagcacagacacagcagaagactgccttgagtatgtcggcatagaggaggagaagggtaatgggatgaactcgctgctggggacgttcctcaagaacctgcagggagacgggttcgaacagatcttccaatttatgctcggcagttacgtgggatggcaaggtaaggaagacgtcctacgcgaacggcttgatttgctagcggagaaggttaaaagactgccgaaacctaagtttgccggcgagtggtccggccatcggatgttcctgcatggtcaattgaagagctggtcctctaactttttccgcctgtttaacgagactagggagctcctcgaaagcataaaatccgacatccaacacgcgaccatgttaatcagctacgtcgaagagaaagggggataccacccacaactcttgtcacagtacaggaaactaatggagcagctgccagctctcagaacaaaggtgttagatccagagatagaaatgactcacatgagcgaggcggtaaggtcgtacattatgatccacaagtcggtagcaggatttctgcctgacttactcgagtccctcgatagggacaaggacagggaattcctgctgagtatatttccaaggatccccaaaattgacaaaaaaactaaggaaatcgtggcctgggagctcccaggcgagcccgaagaaggatacctgttcactgccaataatctttttcgcaactttctggagaatcctaaacatgttccacgtttcatggcagaaaggatcccggaagattggacgcgcctgcggtccgctcccgtatggtttgacggcatggtgaaacaatggcagaaagtggtaaaccagctggtggagtcacctggagcattgtatcagttcaatgaaagctttctccgacaacgtttacaggcaatgctgacagtgtataagagagacctgcagacagagaaattccttaagttgttggctgatgtctgcaggcctctggtggacttctttgggctggggggaaacgatatcatcttcaaaagctgccaggacccgaggaaacaatggcaaactgtcattcccttgagtgtccccgctgatgtgtacaccgcgtgtgaggggctggcaatccggcttcgtgagacattgggatttgagtggaagaaccttaagggccatgaaagggaggactttctaagactgcaccagcttttagggaatctgcttttctggattcgagatgccaaactggtggtgaaattggaagattggatgaataatccctgtgttcaggagtacgttgaggctcgtaaggccattgatctcccactggagatcttcggctttgaggtccccatcttcctgaacggatatctgtttagtgaactgaggcagttagaactgctgctccgccgtaagtcggttatgaccagctattcggttaagacaactggcagtccaaacaggcttttccagttagtctacctgccattaaatccttccgaccctgagaaaaaaaattctaataactttcaggaacgcctggacacccccactggcttatcacgtcgcttcctggaccttactctggacgccttcgccggcaagttgctgacagaccccgtgactcaagagcttaaaactatggctgggttctacgatcacctgtttggtttcaagctcccatgtaagctggcagccatgtctaaccaccctggctctagcagcaagatggtcgtgttggccaaacctaaaaaaggggttgcatctaatataggattcgaaccaatccctgatcccgcgcaccccgtattccgggtgagatcatcatggccagagctgaagtatctggaggggttactgtatcttccagaagacactccactgacaatagagctcgcagagacaagtgttagttgtcagagcgtcagtagcgtggcattcgatctgaaaaatctgactactatccttggacgcgtgggtgagttccgtgtgaccgcagaccagccttttaagttgacccccatcatccctgagaaggaggagtccttcataggaaaaacatatctaggccttgatgccggggaacgctcaggcgtagggttcgctatcgtcacagtcgacggggatgggtacgaggtacagcgcctgggggtgcatgaagatacacagctgatggccctacagcaggtggcctctaaaagcttgaaggagccggtgttccagccgctcagaaagggtacttttcggcagcaggaacgtattagaaaatctctcagaggatgttattggaacttctatcacgctctgatgattaagtaccgcgccaaggtagtgcacgaagagagcgtgggcagttccggcctggttgggcagtggttacgagcattccagaaggacctcaagaaagccgatgtgttgccaaaaaagggaggcaaaaacggagtcgataagaaaaagagagagtcttctgcacaagacacattgtggggaggggcttttagcaagaaggaagaacagcagatagctttcgaagtccaagctgctggttctagccagttctgcctgaagtgcggatggtggttccaactcggaatgcgtgaggttaatcgcgtgcaggaatccggcgtcgtgctggattggaatcggagtattgtcacattcctgattgagagctctggcgagaaagtgtatgggttctcccctcagcaactcgaaaaggggttcagaccagacattgaaaccttcaagaagatggttcgggatttcatgcgcccgcctatgtttgaccggaagggtcgcccagcagctgcctacgaaaggtttgtcttgggacgccggcatcggcggtatagattcgacaaggtttttgaagaacgattcggacgatccgcgctattcatttgcccgagggttggctgtggcaactttgaccacagcagcgagcagtcagccgtagtgctggctctaatcggatatattgccgacaaagaggggatgagcggaaaaaagctagtctacgtgcgtctggcagaactaatggcggaatggaaattgaagaaactggagaggagtagagttgaggagcaaagctccgctcagtga

SEQ ID NO: 164 - DNA, 3579 bp, Artificial Sequence
  Description of Artificial Sequence: Synthetic polynucleotide
atggcggagtcgaagcaaatgcagtgcaggaagtgtggagcctctatgaagtacgaagtgatcggcctcgggaagaaaagctgcagatatatgtgtcccgactgcgggaatcacacatctgcaagaaagattcagaataagaagaaaagggacaagaagtatggatctgccagtaaagcacaaagccaacgaatcgcagttgcaggggccttatacccggataaaaaggttcagaccatcaagacttataagtatccagccgacctgaatggtgaggtccatgactcaggggtggccgaaaaaatagcccaagcaatccaggaggatgaaatagggctcctcggcccctcttccgagtacgcctgttggatcgctagccagaaacagagcgagccctacagtgttgtagacttttggtttgacgctgtgtgcgccggaggcgtgttcgcctattctggggctagattgctgtctaccgtcctgcagctatctggggaggagagcgtcctacgcgcagccctggcatcctccccttttgtcgacgatatcaatctggcacaggccgaaaaatttctggcggtgtccaggcgaaccggccaagataagctggggaagcgcattggagagtgcttcgcagagggccgacttgaggccctaggcatcaaggaccggatgcgtgaatttgtccaggctatcgatgtcgctcagaccgctgggcagcgttttgccgcgaaactgaaaatctttgggatttctcagatgcccgaggcaaagcagtggaacaatgacagcggactcaccgtgtgcatcctgcccgactattacgtcccagaagaaaatcgcgcagatcagttggtcgtcctgctaagacgactgagagagatagcatactgtatggggatcgaagatgaggccggttttgaacatcttggaattgatcctggcgcactatcaaatttttccaatggcaatcctaaacgcggatttttgggccgcctgctgaacaatgatattattgccttagcgaacaacatgtccgccatgacgccttactgggagggcaggaagggagaactgattgaaagattggcttggctgaagcaccgtgcagaggggctttatctgaaggaaccgcattttggaaatagttgggccgaccataggtctagaattttttccagaatagccgggtggctttctgggtgcgctgggaagctaaagatcgccaaagaccagatcagcggagtgcgtactgatctgttccttctgaagagactgctggatgcggtcccgcagtccgccccttctcccgacttcatagcctctatctctgccttggatcgcttcctggaggccgcagaatctagtcaggatcctgccgaacaggtgagggccctatacgcctttcatctgaacgcacccgcggtgcgaagcatcgccaacaaggcagtccagcgatccgacagccaagaatggcttataaaggaactggacgctgtggaccacctggagtttaacaaggcctttcccttcttctctgatacgggaaagaagaaaaagaaaggggctaactcgaatggcgctccgtccgaggaggagtacaccgagactgagagcatccagcagcccgaggacgctgagcaagaggttaatggtcaggaaggcaacggggcctcgaagaaccagaagaagtttcagagaatcccccgattcttcggcgaggggagtcgcagcgagtatcgcatcctcactgaagccccgcagtacttcgacatgttctgtaacaacatgcgggccatctttatgcaattagaatcccaaccgcgtaaagctcccagggattttaagtgtttcctgcagaatcggctgcagaaattgtataagcagacattcctgaacgctcgatccaacaagtgccgggcattactagagtccgtattgattagttggggagagttttacacctacggggctaacgagaaaaaatttcgactgcgtcatgaagcttctgagcgctcctcggacccagattacgtggtgcaacaggcgctggagatcgctcggaggctgtttctcttcggctttgagtggagggactgtagcgcaggtgaaagagtggatctggtcgaaatacataagaaagccatatctttcctgttggccatcactcaggctgaggtgtctgtgggcagctataactggctgggcaattctaccgtgagtcggtacctgtccgtggcagggactgataccctttacggcacccagctggaagaattcttaaatgcaaccgtgttatctcagatgcgggggctggctatcaggttatcatctcaggaactgaaggatggatttgacgtacagctggagtctagttgccaggataatctgcaacacttgctcgtgtacagggcttcacgagaccttgccgcctgcaagcgcgctacttgtccagctgagttggatcctaagattctggtactgcccgtgggggcctttatcgctagcgtgatgaaaatgattgaaagaggggatgagcctttagctggagcttatctgagacacagaccccatagtttcgggtggcagatccgcgttcgaggtgtggcagaggtgggaatggaccaagggaccgccctggcgttccagaaaccgaccgagagcgaacccttcaagataaagccgttttccgctcaatacggccccgttctatggctgaacagctccagttatagccagagccagtacctggacgggttcctatcacagcccaagaactggagtatgcgggtgctgccacaggccggctcagtgcgggtagaacagcgcgtcgccttgatttggaatctccaggccggaaagatgaggctggaacggagcggagcgcgggctttcttcatgcccgtcccattcagtttccgccccagtggcagcggcgacgaggcagtcctggctccaaataggtacctgggactctttccacacagcggcggcatagagtacgctgtggtcgatgttcttgactctgccggcttcaaaatactcgagagaggaacaatagccgtcaatggcttctcccagaaacgaggagaaagacaagaggaagcccatcgcgaaaaacaaagacgcggtatctccgatattgggcgcaagaagccagtccaggccgaagtcgatgcggccaacgagctccatcgaaaatacaccgatgttgctactcggctggggtgtcgaattgtcgttcaatgggcaccccaacccaaaccaggcactgcgccgaccgctcagactgtgtacgctagggccgtgaggactgaagcaccaagatccggcaatcaggaagatcacgccaggatgaaatcttcctggggatacacatggggtacgtattgggaaaaaaggaagcccgaggacatcctcggcattagtacccaggtgtattggacaggcgggatcggcgagtcctgcccggctgtcgccgtcgcgctattgggacacatcagggccacctcaacccagactgaatgggagaaagaggaagtcgtgtttgggcgattgaaaaagttcttcccatcctga

SEQ ID NO: 165 - DNA, 2958 bp, Artificial Sequence
  Description of Artificial Sequence: Synthetic polynucleotide
atggagaagcgcatcaataaaattcgcaagaagctgtctgccgataacgccacaaaaccagttagtcgaagcggcccaatgaagaccctgctagttcgagtgatgactgatgatctgaagaaaaggctcgaaaagcgacgcaagaagcctgaggtaatgcctcaggttataagtaacaatgcagcaaacaatctgcggatgctgcttgacgattacacaaagatgaaggaagccattctccaggtgtattggcaggagttcaaggatgatcacgtaggcctgatgtgtaaattcgcgcaacctgcaagcaagaagatcgaccaaaacaagctgaaacccgagatggatgaaaaaggcaatttaacaaccgccggattcgcttgttcccagtgtgggcagccactgttcgtgtacaagttagaacaggtgtcggaaaaaggaaaggcatacactaactactttggacggtgcaatgttgcagaacacgaaaagctgatactgcttgcccagcttaagcccgaaaaagacagcgacgaagcggtgacctacagcctgggaaaattcgggcagcgggcactggacttctattctatccacgttaccaaggagagcacccacccagtgaagccgttggcccaaatcgctggaaaccggtacgccagcggaccagtcggcaaggccctgtccgatgcctgtatgggcacaattgcttctttcctgtccaagtaccaggacatcataatcgagcaccaaaaagttgtgaaagggaatcagaaacgcctggaatcccttcgagaactggccggcaaggagaaccttgagtacccgtccgtgaccctgcctccacagccacataccaaagagggcgtagacgcgtataatgaggtcattgcccgcgttcgcatgtgggttaatttaaacctgtggcagaaattaaaactaagccgagatgatgctaaaccgttactgagattgaagggattccctagctttcctgtggtggagagaagggaaaacgaggttgattggtggaatactattaatgaggtgaaaaagcttattgacgccaagagggatatgggcagggtgttctggagcggggtgactgccgaaaagagaaataccatcctcgagggatacaattacctccccaacgagaatgatcataagaaaagagaggggagcttagagaatccaaagaaacctgcaaagaggcaattcggtgatctcctgctctacctcgagaagaaatacgcgggggactggggaaaagtttttgacgaagcctgggagcgcattgacaagaagatcgccgggctgacgtctcacattgaacgggaagaggcacggaatgcagaggacgcccagtctaaggccgtgctgactgactggctgcgcgcaaaggcctccttcgtgctcgaacgtctgaaggaaatggatgagaaagagttttacgcgtgtgaaatacagctgcagaagtggtacggcgatctaaggggaaatcccttcgcagtggaagccgagaatagggtagttgacatcagtgggttctccatcggcagtgatggacattctatccagtatagaaacctgctcgcctggaagtacttagagaacggcaagagagagttctatctgctgatgaactacgggaaaaaaggtagaattcgctttacagatggcaccgacataaagaagtccggaaagtggcaaggcctcttatacggaggcggcaaagcaaaggtgatagacttgacttttgaccctgacgacgaacagctgataatcttgccgctggcctttggcacaagacaaggtagggaatttatctggaatgatcttctttctctcgagaccggactcatcaagctcgcaaacggaagggtcatcgagaagacaatctacaataaaaagataggccgagacgagccagccctgtttgtggctttgacatttgagcggagagaggtcgtagatcccagcaacatcaaacccgtgaacctgatcggtgttgacaggggcgagaacatcccggcggttatcgcactgacggatccagaaggatgtcctctgcccgagttcaaagattcatcgggagggccaaccgacattttgaggataggggaggggtacaaggagaagcagcgagctatccaggcggccaaagaagtggagcaacgaagagctggtggttattctcgcaagttcgcttccaaaagtcgtaacctggctgacgatatggtgcgcaattctgcccgtgaccttttctaccacgccgttacacacgacgccgtgttagtgtttgaaaatcttagtcgaggcttcgggcgacaggggaagcggacctttatgaccgagagacagtatacaaaaatggaggattggctgaccgccaaactggcgtatgaaggactcacatccaagacctatctctcaaaaactttggcccagtatacatctaagacgtgcagtaactgtggcttcaccattaccacagctgactacgatggcatgctggtccgcttaaaaaagacatctgacggctgggctactaccctcaacaataaagagctcaaagccgaaggacaaattacctattataacaggtataaaagacagactgtcgagaaggagttgagcgcggagctggaccgcctatcagaggagtcagggaacaacgatatctctaagtggactaagggacgccgagacgaggcgttgttcttgctgaaaaagcggttctctcatcgacccgtgcaggagcagttcgtgtgtctggactgcggccacgaggttcatgctgatgagcaagctgctctaaatattgcccgtagttggttgttcctgaacagcaattcaacagagttcaagtcatacaagagcggaaagcagccgtttgtgggcgcatggcaggcattttacaaaagacgcctgaaggaagtgtggaagccaaacgcc

SEQ ID NO: 166 - DNA, 2919 bp, Artificial Sequence
  Description of Artificial Sequence: Synthetic polynucleotide
atgaaaaggattaacaaaatccgaaggcggcttgtaaaggattctaacaccaaaaaggctggcaagacggggcccatgaaaacattactcgttagagttatgacccccgacctcagagagcgactggaaaatttacgcaagaagccagagaacatacctcagccaattagtaatacctctcgggcaaacctaaacaagttgcttactgattacacggagatgaaaaaggccatactgcatgtgtactgggaggagtttcaaaaggaccctgtcgggctaatgagcagggtggctcagcctgcacctaaaaacatcgaccagcggaaactcatcccagttaaggacggaaatgagagattgacaagttcaggtttcgcctgctcacagtgctgtcaaccgctgtacgtttataagttagaacaagtgaatgacaaaggaaagcctcacacaaattattttggccggtgtaatgtctctgagcatgagcgtctgattctgttgtccccgcataaaccggaagctaatgacgagctcgtaacctacagcttggggaagtttggccaaagagcattggacttctattcaatccatgtgacccgcgaatccaatcatcccgtcaagcccttggagcagatagggggcaatagttgcgcttctggccctgtgggcaaagccctgtccgacgcctgtatgggagccgtggcttcattcctgaccaaatatcaggatatcatcttggagcaccagaaagtgatcaagaaaaatgaaaaaaggttagcaaacctcaaggatattgcaagcgctaacggcttggcttttcctaaaatcacacttccacctcagcctcacacaaaggaaggcatcgaggcatacaacaatgtggtggcccagatcgtcatctgggttaacttaaacctgtggcagaaacttaaaattggcagggatgaggcaaaacccttacagcgcctgaaaggattccccagctttccactggtggagcgccaggctaacgaagtggactggtgggatatggtgtgtaacgtcaagaagctcatcaatgaaaagaaagaggacggtaaagtcttctggcagaacctcgccggttacaaacggcaggaggcgctgttaccttatctgtcgagtgaagaggaccggaaaaaaggcaagaaatttgctcgttatcagtttggtgatttgctcctacatttggagaagaagcacggcgaggactggggaaaagtatacgatgaggcctgggagaggattgacaaaaaggtggagggactgtcaaagcacatcaagctcgaagaagagcgcagaagcgaggacgcccaatccaaagcagcgctgactgactggctgcgggcgaaggccagttttgtaatcgaaggccttaaagaagccgacaaggatgaattctgcagatgcgaattaaaactccagaagtggtacggcgatctccgaggtaagcctttcgcaatcgaggccgagaattccatactggacattagtggattcagtaaacagtataattgtgcctttatatggcagaaggatggtgtcaagaaactcaacctgtaccttattattaattatttcaaaggcgggaaactgagatttaagaagataaagcctgaagcctttgaggcgaaccgattctacacagttattaacaagaaatctggtgaaattgtacccatggaggtaaacttcaacttcgatgatcccaatctgattatattgccactagcttttggcaagcggcagggtagggaattcatttggaacgatttgctttcactggaaacagggtcccttaagctggcaaacgggagagtgattgaaaagacattgtacaatcggaggacacgtcaggatgaacctgcccttttcgtggctctgacattcgagcgcagggaggttctggactctagcaatatcaagccaatgaacctgatcggcatagaccgaggagagaatattccggctgtgatcgcactcaccgatcccgaaggatgtcccctttctcggttcaaggactccttaggcaatccaactcatatcctgagaatcggcgagtcatacaaggagaagcagcgaacaattcaggccgccaaggaagtcgagcagaggcgagctggcggctacagccgtaaatacgctagtaaagctaagaacctggccgacgatatggtgcgcaatactgctagagacctgctgtactatgcagtgacgcaggacgcaatgctgatattcgagaatctgtccagaggattcggaaggcagggcaagcggacgttcatggccgagcgccagtatacaaggatggaggattggttaacggccaagcttgcctatgaggggctacctagtaagacctatctgtctaagacgctggctcaatacaccagtaagacctgctcaaactgtggctttacaatcacttctgctgattatgatagagtgctcgagaagctaaaaaaaactgccaccggctggatgactactattaatgggaaggaactgaaagtggaaggacagattacctattataatcgctacaagcgtcaaaacgtcgtcaaggacctgtcggtggaattggacagactcagtgaagagtccgtgaacaatgatatcagctcctggacaaaagggcgcagtggggaggcactcagcttgcttaaaaagaggttttcacatcggccggtccaggagaaatttgtctgcctgaactgcggattcgagacacacgccgacgagcaggcagcactgaacattgccagatcctggctgttccttaggtcccaggaatataagaagtaccagactaacaaaaccacgggaaacacagataaaagggcctttgtcgaaacttggcaatccttttaccggaagaagttaaaggaagtgtggaagccc

SEQ ID NO: 167 - DNA, 4107 bp, Artificial Sequence
  Description of Artificial Sequence: Synthetic polynucleotide
atggataagaaatactcaataggcttagcaatcggcacaaatagcgtcggatgggcggtgatcactgatgaatataaggttccgtctaaaaagttcaaggttctgggaaatacagaccgccacagtatcaaaaaaaatcttataggggctcttttatttgacagtggagagacagcggaagcgactcgtctcaaacggacagctcgtagaaggtatacacgtcggaagaatcgtatttgttatctacaggagattttttcaaatgagatggcgaaagtagatgatagtttctttcatcgacttgaagagtcttttttggtggaagaagacaagaagcatgaacgtcatcctatttttggaaatatagtagatgaagttgcttatcatgagaaatatccaactatctatcatctgcgaaaaaaattggtagattctactgataaagcggatttgcgcttaatctatttggccttagcgcatatgattaagtttcgtggtcattttttgattgagggagatttaaatcctgataatagtgatgtggacaaactatttatccagttggtacaaacctacaatcaattatttgaagaaaaccctattaacgcaagtggagtagatgctaaagcgattctttctgcacgattgagtaaatcaagacgattagaaaatctcattgctcagctccccggtgagaagaaaaatggcttatttgggaatctcattgctttgtcattgggtttgacccctaattttaaatcaaattttgatttggcagaagatgctaaattacagctttcaaaagatacttacgatgatgatttagataatttattggcgcaaattggagatcaatatgctgatttgtttttggcagctaagaatttatcagatgctattttactttcagatatcctaagagtaaatactgaaataactaaggctcccctatcagcttcaatgattaaacgctacgatgaacatcatcaagacttgactcttttaaaagctttagttcgacaacaacttccagaaaagtataaagaaatcttttttgatcaatcaaaaaacggatatgcaggttatattgatgggggagctagccaagaagaattttataaatttatcaaaccaattttagaaaaaatggatggtactgaggaattattggtgaaactaaatcgtgaagatttgctgcgcaagcaacggacctttgacaacggctctattccccatcaaattcacttgggtgagctgcatgctattttgagaagacaagaagacttttatccatttttaaaagacaatcgtgagaagattgaaaaaatcttgacttttcgaattccttattatgttggtccattggcgcgtggcaatagtcgttttgcatggatgactcggaagtctgaagaaacaattaccccatggaattttgaagaagttgtcgataaaggtgcttcagctcaatcatttattgaacgcatgacaaactttgataaaaatcttccaaatgaaaaagtactaccaaaacatagtttgctttatgagtattttacggtttataacgaattgacaaaggtcaaatatgttactgaaggaatgcgaaaaccagcatttctttcaggtgaacagaagaaagccattgttgatttactcttcaaaacaaatcgaaaagtaaccgttaagcaattaaaagaagattatttcaaaaaaatagaatgttttgatagtgttgaaatttcaggagttgaagatagatttaatgcttcattaggtacctaccatgatttgctaaaaattattaaagataaagattttttggataatgaagaaaatgaagatatcttagaggatattgttttaacattgaccttatttgaagatagggagatgattgaggaaagacttaaaacatatgctcacctctttgatgataaggtgatgaaacagcttaaacgtcgccgttatactggttggggacgtttgtctcgaaaattgattaatggtattagggataagcaatctggcaaaacaatattagattttttgaaatcagatggttttgccaatcgcaattttatgcagctgatccatgatgatagtttgacatttaaagaagacattcaaaaagcacaagtgtctggacaaggcgatagtttacatgaacatattgcaaatttagctggtagccctgctattaaaaaaggtattttacagactgtaaaagttgttgatgaattggtcaaagtaatggggcggcataagccagaaaatatcgttattgaaatggcacgtgaaaatcagacaactcaaaagggccagaaaaattcgcgagagcgtatgaaacgaatcgaagaaggtatcaaagaattaggaagtcagattcttaaagagcatcctgttgaaaatactcaattgcaaaatgaaaagctctatctctattatctccaaaatggaagagacatgtatgtggaccaagaattagatattaatcgtttaagtgattatgatgtcgatcacattgttccacaaagtttccttaaagacgattcaatagacaataaggtcttaacgcgttctgataaaaatcgtggtaaatcggataacgttccaagtgaagaagtagtcaaaaagatgaaaaactattggagacaacttctaaacgccaagttaatcactcaacgtaagtttgataatttaacgaaagctgaacgtggaggtttgagtgaacttgataaagctggttttatcaaacgccaattggttgaaactcgccaaatcactaagcatgtggcacaaattttggatagtcgcatgaatactaaatacgatgaaaatgataaacttattcgagaggttaaagtgattaccttaaaatctaaattagtttctgacttccgaaaagatttccaattctataaagtacgtgagattaacaattaccatcatgcccatgatgcgtatctaaatgccgtcgttggaactgctttgattaagaaatatccaaaacttgaatcggagtttgtctatggtgattataaagtttatgatgttcgtaaaatgattgctaagtctgagcaagaaataggcaaagcaaccgcaaaatatttcttttactctaatatcatgaacttcttcaaaacagaaattacacttgcaaatggagagattcgcaaacgccctctaatcgaaactaatggggaaactggagaaattgtctgggataaagggcgagattttgccacagtgcgcaaagtattgtccatgccccaagtcaatattgtcaagaaaacagaagtacagacaggcggattctccaaggagtcaattttaccaaaaagaaattcggacaagcttattgctcgtaaaaaagactgggatccaaaaaaatatggtggttttgatagtccaacggtagcttattcagtcctagtggttgctaaggtggaaaaagggaaatcgaagaagttaaaatccgttaaagagttactagggatcacaattatggaaagaagttcctttgaaaaaaatccgattgactttttagaagctaaaggatataaggaagttaaaaaagacttaatcattaaactacctaaatatagtctttttgagttagaaaacggtcgtaaacggatgctggctagtgccggagaattacaaaaaggaaatgagctggctctgccaagcaaatatgtgaattttttatatttagctagtcattatgaaaagttgaagggtagtccagaagataacgaacaaaaacaattgtttgtggagcagcataagcattatttagatgagattattgagcaaatcagtgaattttctaagcgtgttattttagcagatgccaatttagataaagttcttagtgcatataacaaacatagagacaaaccaatacgtgaacaagcagaaaatattattcatttatttacgttgacgaatcttggagctcccgctgcttttaaatattttgatacaacaattgatcgtaaacgatatacgtctacaaaagaagttttagatgccactcttatccatcaatccatcactggtctttatgaaacacgcattgatttgagtcagctaggaggtgactga

SEQ ID NO: 168 - DNA, 4107 bp, Artificial Sequence
  Description of Artificial Sequence: Synthetic polynucleotide
atggataagaagtattcaattggacttgcgattggcactaacagtgtgggctgggcggtgattacagacgagtataaggtgccgtcaaaaaagtttaaagttctgggcaacactgatcgccattccatcaagaaaaacctaatcggggcccttctttttgatagtggcgaaacggccgaggcgacgcgtctaaaacgtaccgcgcggcgtcgctacacccgacgaaaaaaccgtatttgttaccttcaggagatcttcagtaacgaaatggctaaggtggacgattcattcttccaccgtctggaggagtcctttttagttgaagaagacaagaagcatgagcgacacccaatttttggtaacattgtcgacgaagtcgcctatcacgaaaaatatccgaccatttatcacctgcgcaaaaaactggtcgatagcacggataaagcggatctgcggcttatttacctggcgcttgcccacatgatcaagttccgcggccacttcctgatagaaggagacctgaacccggataatagcgatgtagacaaactgtttattcagctggtccagacctacaaccagctgtttgaagaaaatccgattaatgcgtcaggcgtggatgcgaaagcgatactgagtgcccgcctgtcgaaatctcgccgtctcgaaaatctgattgcacagctgcccggcgaaaaaaaaaacggtctttttggcaatctgatcgcgctgtcactgggcctgacaccaaattttaagagcaacttcgacctggcagaggatgcgaagcttcaactgtcgaaggacacctatgacgatgatctggataatcttctggcacaaatcggtgatcagtatgcggatttattccttgcagcgaaaaacctatctgacgcaattctgttgagcgatatcctccgcgtcaacaccgaaatcactaaagcccccctgtcagcgtcgatgattaaacgttatgatgagcaccatcaggatctgaccttgctaaaggcgctggtgcgacagcagcttcccgaaaaatataaagagatcttttttgatcaatcgaagaatggttatgccggatacattgatggcggagccagtcaggaagaattttacaaattcatcaaaccgatcctggaaaaaatggatggcacagaagaactgcttgtgaaattgaaccgggaagatttactgcgcaaacagcgtacgttcgacaacggctccataccccatcagattcacttaggtgagctgcatgcaatactccgtcgccaggaagatttttatccatttttaaaagacaaccgtgagaagattgaaaaaattttaacttttcgtattccatattacgtcgggcctttggcccgaggtaactctcgattcgcctggatgacgagaaaaagcgaggagaccatcactccgtggaattttgaagaggttgttgataaaggcgcgagcgcccagtcgtttatcgaacgtatgaccaactttgataaaaatctgccgaatgaaaaagtgcttccgaagcattctctgttgtatgaatatttcactgtgtacaatgagttaacgaaagtgaaatatgtgaccgaaggcatgcggaaacctgcttttctgtccggagaacagaaaaaagcaattgtggacctgctgttcaaaacgaaccggaaagtaactgtgaagcagctgaaagaggactacttcaaaaaaatcgaatgcttcgactcagtagagatctctggtgttgaagatcgcttcaacgcgagtctgggaacgtaccatgatttgttgaaaatcatcaaagataaagactttctggataacgaagagaatgaggacattcttgaagatattgttttgacactgactctgtttgaggatcgcgaaatgattgaagagcgcctgaaaacgtatgcccatttattcgatgacaaagtcatgaagcagctgaaacgtcgccgctatactgggtggggcagactttcacgtaaattgatcaatggtataagagacaaacagagcggcaaaactatcttagatttcctgaagagtgatggatttgccaaccggaattttatgcagcttatacatgatgactcgctaacgtttaaagaagacattcagaaggcgcaggtcagcggccagggtgattcgctgcatgaacacattgcaaatcttgccggatcgccagcgatcaaaaaaggcatccttcagacagtaaaagttgtggatgaactggtgaaagtaatgggtcgtcacaagccagaaaatattgtgatcgaaatggcccgggaaaatcagactactcaaaaaggtcagaaaaattctcgcgagcgtatgaaacgtattgaagaaggcatcaaagagctaggcagccagatattaaaggaacatccggttgagaacactcagctgcagaatgaaaaactgtatctgtattatcttcagaacggccgtgacatgtatgttgatcaagaactggatatcaatcgcttgtccgattatgacgtggatcatattgttccgcaaagctttctgaaagacgattctattgacaataaagtactgacacgttcggacaaaaaccgtggtaaaagcgataacgtaccgtcggaagaagttgttaagaaaatgaaaaattattggcgccaactcctgaatgctaaattgattacccagcggaaatttgataacttaaccaaagccgagcggggtggcttaagtgaactggataaagcgggttttattaaacgccaactggtagaaacccgccagataacgaaacatgtagctcaaatcctcgatagtcgcatgaatacgaaatatgacgaaaatgataaattgatccgtgaagtaaaagtgattactcttaaaagcaaattggtatctgattttcggaaagatttccaattctataaggtgagagaaattaacaattaccatcatgcacatgatgcgtatttaaatgcagttgttggcaccgccttaatcaaaaaatatccgaaattagaatctgagttcgtgtatggtgattataaagtttatgatgttcgaaaaatgattgctaagtctgaacaggaaatcggcaaagcgaccgcaaagtattttttttatagcaatattatgaatttttttaaaactgagattaccctggcgaatggcgaaattcgcaaacgtcctctgattgaaaccaatggcgaaaccggcgagatagtatgggacaagggccgtgattttgcgaccgtccggaaagtcctgtcaatgccgcaggtgaatattgtcaagaaaacagaagttcagacaggcggttttagtaaagagtctattctgcccaaacgtaattcggataaattgattgcccgcaagaaagattgggatccgaagaaatatggtggattcgattctccgacggtcgcctatagcgttctagtcgtcgccaaggtcgaaaaaggtaaatccaaaaaactgaaatctgtgaaagaactgttaggcattacaatcatggaacgtagtagttttgaaaagaacccgatcgacttcctcgaggcgaaaggctacaaagaagtcaagaaggatttgattattaaactcccaaaatattcattatttgagttagaaaacggtaggaagcgtatgctggcgagtgctggggaattacagaaagggaatgagttagcactgccgtcaaaatatgtgaactttctgtatctggcctcccattacgagaaactgaaaggtagcccggaagataatgaacagaaacaactatttgtcgagcaacacaaacattatctggatgaaattattgaacagattagtgaattctctaaacgtgttattttagcggatgccaaccttgacaaggtgctgagcgcatataataaacaccgtgataaacccattcgtgaacaggctgaaaatatcatacatctgttcacgttaaccaacttgggagctcctgccgcttttaaatatttcgataccacaattgaccgcaaacgttatacgtctacaaaagaggtgctcgatgcgaccctgatccaccagtctattacaggcctgtatgaaactcgtatcgacctgtcacaactgggcggcgactga

SEQ ID NO: 169 - DNA, 4107 bp, Artificial Sequence
  Description of Artificial Sequence: Synthetic polynucleotide
atggacaagaaatattcaatcggtttagcaataggaactaactcagtaggttgggctgtaattacagacgaatacaaggtaccgtccaaaaagtttaaggtgttggggaacacagatagacactctataaaaaaaaatttaataggcgctttacttttcgattcaggcgaaactgcagaagcgacacgtctgaagagaaccgctagacgtagatacacgaggagaaagaacagaatatgttacctacaagaaattttttctaatgagatggctaaggtggatgattcgttttttcatagactcgaagaatctttcttagttgaagaagataaaaaacacgaaaggcatcctatctttggaaacatagttgatgaggtggcttaccatgaaaaatatcccactatatatcaccttagaaaaaagttggttgattcaaccgacaaagcggatctaaggttaatttacctcgcgttggctcacatgataaaatttagaggacatttcttgatcgaaggtgatttaaatcccgataactctgatgtagataaactgttcatccagttggttcaaacatataatcagttgttcgaagagaaccccattaacgcatcaggtgttgatgctaaagcaatcttatcagcaaggttgagcaagagcagacgtctggaaaacttgattgcccaattgccaggtgaaaagaagaacggtctttttggaaatttaattgcactttcacttgggttgacaccgaattttaaaagcaatttcgacctcgctgaggatgctaaactccagttatctaaggatacatatgacgatgatttggataatctattggcccagataggtgatcagtatgcagatttgtttttggcagctaagaatttatcagatgcaattctactgagcgatattttaagggtgaatacagaaataactaaagcacctttgtctgcatctatgataaaaagatacgatgaacaccatcaagatctcacactattaaaagctttagttagacaacaattaccagaaaaatataaagaaatctttttcgatcagtccaagaacggatacgccggctatatagatggcggtgcctcccaagaagaattttacaaatttatcaaacccattttggaaaagatggatggtactgaagaattattggtcaaattaaacagggaagatttattaagaaaacaaaggacctttgataatggttctattccacaccaaatccatctaggggaattacatgcgattcttagaagacaagaagatttttatccattcttgaaagataacagggaaaagatagagaaaatcttaacttttagaattccctactacgtcgggcccttagctagggggaattctagattcgcctggatgacacgcaaatcagaagaaacaattacgccttggaattttgaagaagttgttgataaaggagcctctgctcaatcttttattgaacgaatgaccaattttgataagaatttacccaatgaaaaggtcttacccaaacattcactcctatacgagtactttactgtttacaatgagttgacaaaagtgaagtatgttaccgagggtatgcgaaaacctgctttcttgagtggtgaacaaaagaaggccattgttgacttgttattcaaaactaacagaaaggtcactgtgaagcagcttaaagaagattatttcaaaaagatcgaatgtttcgactcggtagaaattagtggtgtggaagatagatttaatgcttctcttggaacatatcatgatctactaaagatcatcaaagataaagatttcttggacaatgaagaaaatgaagatattcttgaagacatcgtgttgacacttacattgtttgaggacagagaaatgattgaagaaaggctgaagacctacgcccatttgtttgatgataaagtcatgaaacagttaaagaggagaaggtataccggatggggtaggctgtctcgcaaattgattaatggtattcgtgataaacaatcgggtaaaacaatcctagatttcctgaagtccgatggtttcgccaacaggaattttatgcaattgattcatgacgattctttgacttttaaagaggatattcagaaagcacaggtctcaggacagggcgattcactccatgaacatatagctaacctggctggctcccctgctattaagaaaggtatcttgcaaaccgtcaaagtagtagacgaacttgttaaagttatgggaagacacaaacctgaaaatatcgttattgaaatggctcgcgaaaaccagacaacacaaaagggtcaaaagaattcgagagagagaatgaagcgtatcgaagaaggtattaaagaacttgggtcccaaatacttaaagaacatccagtagaaaacactcagcttcaaaatgaaaaattatacttatattatcttcagaatggccgcgatatgtatgttgaccaagagttagatataaataggttgtctgattacgacgtggatcatattgtacctcaatcttttctaaaagatgattcaattgataataaggtattaacgagaagtgataaaaatagaggtaaatctgacaacgtgccaagcgaagaggtggtgaagaaaatgaaaaattattggcgtcaactgttgaacgccaagttaattacgcagagaaagtttgataatctaacaaaagctgaaagaggaggcctatctgagttagataaggccggttttatcaaacgtcagttagttgaaaccaggcaaatcacgaagcacgttgcccaaattctagattcaaggatgaataccaaatacgatgaaaacgataaactgattcgggaagtcaaggttataactctaaaaagcaaactagtttcagattttcgcaaagattttcaattttacaaagttcgagaaatcaataattatcatcatgctcacgacgcgtacttgaacgcggtcgttggtacagctttaataaagaaatatcctaaactggaatcggaatttgtatatggggattacaaagtatacgacgtgagaaagatgatcgctaaatctgaacaagaaattgggaaagcaactgccaaatattttttttacagcaacataatgaatttttttaaaacggaaattacattggcaaatggcgaaattagaaagcgcccattgatagagaccaatggagagactggggaaatcgtgtgggataaaggacgtgattttgccacagtgaggaaagtgttaagtatgccacaagttaatattgtaaaaaagaccgaggtccaaacgggtggatttagcaaagaatcaattttacctaagagaaattcagataaattaattgcccgcaaaaaggattgggatcctaaaaaatatggtggttttgattccccaacagttgcttactccgtcctagttgttgctaaggttgaaaaaggaaagtctaagaaacttaaatccgtaaaagagttactgggaattacaataatggaaagatcctctttcgaaaagaaccctattgacttcttggaggcgaaaggttataaagaagtcaaaaaagatttgatcataaaactaccaaagtattctctatttgaattggaaaacggcagaaaaaggatgttggcaagcgctggtgaactacaaaagggtaacgaattggcattgccgagtaaatacgtgaattttctatatttggcatcacattacgaaaagttaaagggatcacccgaggataacgagcagaaacaactgtttgttgaacaacacaaacattatcttgatgaaattatagaacaaattagtgagttcagtaagagagttattttagccgatgcaaatttagacaaagttttatctgcttataacaaacatagagataagcctataagggaacaagccgaaaatattattcatttgtttacgttaacaaatttaggggcaccagcagcattcaagtacttcgatacgactatcgatcgtaagcgttacacatctaccaaagaagttcttgatgcaactttgattcatcaatctataacaggcttatatgaaactagaatcgatctgtcacaacttggtggtgactaa

SEQ ID NO: 170 - DNA, 4107 bp, Artificial Sequence
  Description of Artificial Sequence: Synthetic polynucleotide
atggacaagaagtactcaattgggcttgctatcggcactaacagcgttggctgggcggtcatcacagacgaatataaggtcccatcaaagaaattcaaagtccttggcaatacggaccgacattcaatcaagaagaacctgattggagctctgctgtttgattccggtgaaaccgccgaggcaacacgattgaaacgtaccgctcgtaggaggtatacgcggcggaaaaataggatctgctatctgcaggaaatatttagcaacgaaatggccaaggtagacgacagcttcttccaccggctcgaggaatctttcctcgtggaagaagacaaaaagcacgagcgccaccccattttcggcaatatcgtggacgaggtagcttaccatgaaaagtatccaactatttaccacttacgtaagaagttagtggacagcaccgataaagccgaccttcgcctgatttacctagcacttgcacacatgattaagttccgaggccacttcttgatagagggagacctgaatcctgacaattccgatgtggataaattgttcatccagctggtacagacatacaatcagttgtttgaggaaaatccgattaatgccagtggcgtggacgccaaggctatcctgtctgctcggcttagtaagagtagacgcctggaaaatctaatcgcacagctgcccggcgaaaagaaaaatggactgttcggtaatttgatcgccctgagcctgggcctcacccctaactttaagtctaacttcgacctggccgaagatgctaagctccagctgtccaaagatacttacgatgacgatctcgataatctactggctcagatcggggaccagtacgctgacctgtttctagctgccaagaacctcagtgacgccattctcctgtccgatattctgagggttaacactgaaattacaaaggccccgctgagcgcgagcatgatcaaaaggtacgacgagcatcaccaggacctcacgctgctgaaggccttagtcagacagcaactgcccgaaaagtacaaagaaatctttttcgaccaatccaagaacgggtacgccggctacattgatggcggggcttcacaagaggagttttacaagtttatcaagcccatcctggagaaaatggacggcactgaagaactgcttgtgaaactcaatagggaagacttactgaggaaacagcgcacattcgataatggctccataccccaccaaatccatctgggagagttgcatgccatcttgcgaaggcaggaggacttctacccctttcttaaggacaacagggagaaaatcgagaaaattctgactttccgtatcccctactacgtgggcccacttgctcgcggaaactcacgattcgcatggatgaccagaaagtccgaggaaacaattacaccctggaattttgaggaggtagtagacaagggagccagcgctcaatctttcattgagaggatgacgaatttcgacaagaaccttccaaacgagaaagtgcttcctaagcacagcctgctgtatgagtatttcacggtgtacaacgaacttacgaaggtcaagtatgtgacagagggtatgcggaaacctgcttttctgtctggtgaacagaagaaagctatcgtcgatctcctgtttaaaaccaaccgaaaggtgacggtgaaacagttgaaggaggattacttcaagaagatcgagtgttttgattctgttgaaatttctggggtcgaggatagattcaacgccagcctgggcacctaccatgatttgctgaagattatcaaggataaggattttctggataatgaggagaatgaagacattttggaggatatagtgctgaccctcaccctgttcgaggaccgggagatgatcgaggagagactgaaaacatacgctcacctgtttgacgacaaggtcatgaagcagcttaagagacgccgttacacaggctggggaagattatcccgcaaattaatcaacgggatacgcgataaacaaagtggcaagaccatactcgacttcctaaagagcgatggattcgcaaatcgcaatttcatgcagttgatccacgacgatagcctgaccttcaaagaggacattcagaaagcgcaggtgagtggtcaaggggattccctgcacgaacacattgctaacttggctggatcaccagccattaagaaaggcatactgcagaccgttaaagtggtagatgagcttgtgaaagtcatgggaagacataagccagagaacatagtgatcgaaatggccagggaaaatcagaccacgcaaaaggggcagaagaactcaagagagcgtatgaagaggatcgaggagggcatcaaggagctgggtagccagatccttaaagagcacccagttgagaatacccagctgcagaatgagaaactttatctctattatctccagaacggaagggatatgtatgtcgaccaggaactggacatcaatcggctgagtgattatgacgtcgaccacattgtgcctcaaagctttctgaaggatgattccatcgacaataaagttctgacccggtctgataaaaatagaggcaaatccgacaacgtacctagcgaagaagtcgtcaaaaaaatgaagaactattggaggcagttgctgaatgccaagctgattacacaacgcaagtttgacaatctcaccaaggcagaaagggggggcctgtcagaactcgacaaagcaggtttcattaaaaggcagctagttgaaactaggcagattactaagcacgtggcccagatcctcgactcacggatgaatacaaagtatgatgagaatgataagctaatccgggaggtgaaggtgattactctgaaatctaagctggtgtcagatttcagaaaagacttccagttctacaaagtcagagagatcaacaattatcaccatgcccacgatgcatatcttaatgcagtagtggggacagctctgatcaaaaaatatcctaaactggagtctgaattcgtttatggtgactataaagtctatgacgtcagaaaaatgatcgcaaagagcgagcaggagatagggaaggccacagcaaagtacttcttttacagtaatatcatgaactttttcaaaactgagattacattggctaacggcgagatccgcaagcggccactgatagagactaacggagagacaggggagattgtttgggataagggccgtgacttcgccaccgttaggaaagtgctgtccatgccccaggtgaacattgtgaagaagacagaagtgcagacgggtgggttctcaaaagagtctattctgcctaagcggaatagtgacaaactgatcgcacgtaaaaaggactgggatccaaaaaagtacggcggattcgacagtcctaccgttgcatattccgtgcttgtggtcgctaaggtggagaagggaaaaagcaagaaactgaagtcagtcaaagaactactgggcataacgatcatggagcgctccagtttcgaaaaaaacccaatcgattttcttgaagccaagggatacaaggaggtaaagaaagaccttatcattaagctgcctaagtacagtctgttcgaactggagaatgggaggaagcgcatgctggcatcagctggagaactccaaaaagggaacgagttggccctcccctcaaagtatgtcaattttctctacctggcttctcactacgagaagttaaaggggtctccagaggataatgagcagaaacagctgtttgtggaacagcacaagcactatttggacgaaatcatcgaacaaatttccgagttcagtaagagggtgattctggccgacgcaaaccttgacaaagttctgtccgcatacaataagcacagagacaaaccaatccgcgagcaagccgagaatataattcaccttttcactctgactaatctgggggcccccgcagcatttaaatatttcgatacaacaatcgaccggaagcggtatacatctactaaggaagtcctcgatgcgacactgatccaccagtcaattacaggtttatatgaaacaagaatcgacctgtcccagctgggcggcgactag

SEQ ID NO: 171 - DNA, 4805 bp, Artificial Sequence; identical to SEQ ID NO: 69
  Description of Artificial Sequence: Synthetic polynucleotide

SEQ ID NO: 172 - DNA, 20 bp, Artificial Sequence
  Description of Artificial Sequence: Synthetic oligonucleotide
aattcaaaggataatcaaac

SEQ ID NO: 173 - DNA, 20 bp, Artificial Sequence
  Description of Artificial Sequence: Synthetic oligonucleotide
aatctctactctttgtagat

SEQ ID NO: 174 - DNA, 19 bp, Artificial Sequence
  Description of Artificial Sequence: Synthetic oligonucleotide
aatttctactgttgtagat

SEQ ID NO: 175 - DNA, 19 bp, Artificial Sequence
  Description of Artificial Sequence: Synthetic oligonucleotide
aatttctactagtgtagat

SEQ ID NO: 176 - DNA, 15 bp, Artificial Sequence
  Description of Artificial Sequence: Synthetic oligonucleotide
aatttctactattgt

SEQ ID NO: 177 - DNA, 18 bp, Artificial Sequence
  Description of Artificial Sequence: Synthetic oligonucleotide
aatttctactgttgtaga

SEQ ID NO: 178 - DNA, 16 bp, Artificial Sequence
  Description of Artificial Sequence: Synthetic oligonucleotide
aatttctactattgta

SEQ ID NO: 179 - DNA, 19 bp, Artificial Sequence
  Description of Artificial Sequence: Synthetic oligonucleotide
aatttctacttttgtagat

SEQ ID NO: 180 - DNA, 19 bp, Artificial Sequence
  Description of Artificial Sequence: Synthetic oligonucleotide
aatttctactgttgtagat

SEQ ID NO: 181 - DNA, 19 bp, Artificial Sequence
  Description of Artificial Sequence: Synthetic oligonucleotide
aatttctactcttgtagat

SEQ ID NO: 182 - DNA, 19 bp, Artificial Sequence
  Description of Artificial Sequence: Synthetic oligonucleotide
aatttctactattgtagat

SEQ ID NO: 183 - DNA, 255 bp, Artificial Sequence
  Description of Artificial Sequence: Synthetic polynucleotide
atgaataacggcactaataacttccagaatttcattggcatatcttccttacagaaaacacttagaaatgctttgatcccgacggagactacacagcagtttatcgtgaagaacggcataattaaggaggatgaattgaggggagagaaccgtcaaatactcaaggatatcatggatgactactatagagggttcattagcgaaactctttcttccatcgatgatatagattggacttccctcttcgagaagatg

SEQ ID NO: 184 - DNA, 255 bp, Artificial Sequence
  Description of Artificial Sequence: Synthetic polynucleotide
atgaataatggcaccaataacttccagaacttcatcggaatctcctcccttcagaaaacactgagaaatgctcttatccctactgaaactacacaacaattcattgtaaagaacggaataattaaggaagatgaattgcgtggtgagaacaggcaaatactcaaggacatcatggatgactattaccggggattcatttcagagactttatcctccattgatgatatagattggacgtcgttgttcgagaaaatg

SEQ ID NO: 185 - DNA, 255 bp, Artificial Sequence
  Description of Artificial Sequence: Synthetic polynucleotide
atgaacaatggtaccaataatttccagaacttcatcggaatttcatcactccagaagacccttaggaacgcccttattccaaccgaaacaacacagcaattcatagtcaagaacggcatcattaaggaggatgagcttcgcggggagaatcgacaaatactcaaagatattatggatgattattacagaggattcattagtgaaaccctcagtagcatcgatgatatcgattggacaagtctattcgagaaaatg

SEQ ID NO: 186 - DNA, 255 bp, Artificial Sequence
  Description of Artificial Sequence: Synthetic polynucleotide
atgaataacgggaccaacaacttccagaatttcattggtatatccagccttcagaagaccctaagaaacgctcttatccctactgagactacacagcagtttatagtcaagaatgggattataaaggaagatgaattaagaggagagaatcgacagatactcaaagacataatggatgattactaccgtgggttcatatcagaaaccctctcgtcgattgatgatattgactggactagtctattcgagaagatg

SEQ ID NO: 187 - DNA, 255 bp, Artificial Sequence
  Description of Artificial Sequence: Synthetic polynucleotide
atgaataatggaactaacaactttcagaacttcatcggaatctctagtttgcagaaaacccttcgaaacgcattgatacctacagagacgacacaacaattcattgttaagaacggcattattaaagaggacgagcttagaggagagaataggcaaatactcaaagacattatggatgactattaccgtgggtttattagcgaaactttaagctccattgatgacatagactggacctcattgtttgagaagatg

SEQ ID NO: 188 - DNA, 255 bp, Artificial Sequence
  Description of Artificial Sequence: Synthetic polynucleotide
atgaataatggaacgaacaacttccagaacttcattggtatctcgtctctacagaagactttacgtaacgctctaatacctaccgagactacacaacaattcatcgttaagaacggaatcataaaggaggatgaactaagaggagagaacaggcagatccttaaggatatcatggatgattactatcgaggctttatctcagagaccttgtcaagtattgatgatatcgattggacgtcactatttgagaagatg

SEQ ID NO: 189 - DNA, 255 bp, Artificial Sequence
  Description of Artificial Sequence: Synthetic polynucleotide
atgaacaatggcacaaacaactttcagaatttcatcggtatatcttctcttcagaagacgcttaggaatgccttgattccaactgagactacacaacagtttatagttaagaacggaatcattaaggaagatgaattacggggagagaatcgtcaaattctaaaggatatcatggatgactattatcgcgggtttatctcggagactctcagctcaatcgatgacatcgattggacctccttattcgagaagatg

SEQ ID NO: 190 - DNA, 255 bp, Artificial Sequence
  Description of Artificial Sequence: Synthetic polynucleotide
atgaacaacggtacaaataatttccagaatttcatcggtatctccagtttacagaagaccttgcgtaacgctctaatcccgacagaaacaactcaacaattcattgtgaagaatggaattataaaggaggatgaacttagaggtgagaatagacagatattgaaggacataatggacgactactatcgcgggttcatatcagagactctgagtagcattgacgatattgattggacctcactcttcgagaagatg

SEQ ID NO: 191 - DNA, 255 bp, Artificial Sequence
  Description of Artificial Sequence: Synthetic polynucleotide
atgaacaatggcactaacaacttccagaatttcatagggatctcttctcttcagaagactcttcggaacgcactaatacctactgaaacaactcaacagtttatcgttaagaacggtataatcaaagaagacgaattgcgtggtgagaatcgtcaaatccttaaggatatcatggatgactattatcgaggattcatctccgagacactttcctcaatcgatgatatagattggacatccctcttcgagaagatg

SEQ ID NO: 192 - DNA, 255 bp, Artificial Sequence
  Description of Artificial Sequence: Synthetic polynucleotide
atgaacaatggcactaataatttccagaacttcattggaatctcttctctccaaaagacacttagaaatgctttaattccaacggaaacgactcaacaattcatcgtaaagaacggaattattaaggaagatgagttgagaggtgagaacaggcagattctaaaggatatcatggatgattattacagaggtttcatctctgaaacgctgtcttcaatagatgacatcgattggacgagtctatttgagaaaatg

SEQ ID NO: 193 - DNA, 255 bp, Artificial Sequence
  Description of Artificial Sequence: Synthetic polynucleotide
atgaacaatggaacgaataacttccagaacttcataggaatatcctctttgcagaaaacattaaggaatgcacttattcctacagaaactacccaacaatttatcgtcaagaatggaatcattaaagaggatgaactccgtggagagaataggcaaattctaaaggatatcatggacgattactatagagggttcatctcagaaaccctctcgtctatagatgatattgactggacaagcctcttcgagaagatg

SEQ ID NO: 194 - DNA, 255 bp, Artificial Sequence
  Description of Artificial Sequence: Synthetic polynucleotide
atgaataacggaacgaataacttccagaatttcatcggtatttcgtccctgcagaaaacacttagaaatgctctcatcccaactgagactacgcagcagtttatagtgaagaacggcataattaaagaggatgagctaaggggcgagaatagacaaatcttgaaagacattatggatgactactaccgcggcttcatatctgagactctttcatctattgacgatatagactggaccagtttatttgagaagatg

SEQ ID NO: 195 - DNA, 255 bp, Artificial Sequence
  Description of Artificial Sequence: Synthetic polynucleotide
atgaacaacggtacgaataactttcagaacttcataggtatctccagtcttcaaaagactcttcgtaatgcgcttattcctactgaaactactcaacaatttatcgtgaagaatggcattattaaggaagacgagctaagaggagagaataggcagatacttaaggatataatggacgattactacagaggatttatctcagaaacactctcttctatcgacgatatagattggacttcgctgttcgagaagatg

SEQ ID NO: 196 - DNA, 255 bp, Artificial Sequence
  Description of Artificial Sequence: Synthetic polynucleotide
atgaataatgggaccaataacttccagaattttattggtatttcctctttgcagaagaccctaagaaacgcgctgatcccaactgagacgacacagcaattcatcgttaagaacggaattattaaagaggatgaacttcgcggagagaaccgccagatactgaaggatattatggatgactactatcgtggtttcatatccgagactttgtcttctatagacgatatcgattggacttctttatttgagaaaatg

SEQ ID NO: 197 - DNA, 255 bp, Artificial Sequence
  Description of Artificial Sequence: Synthetic polynucleotide
atgaacaacggtactaacaacttccagaatttcatcggtattagttcattgcagaagactcttagaaacgcactaattcccaccgaaacaacccaacagttcatagtcaagaacggtataattaaggaagatgagctaagaggtgagaatagacaaatcttgaaggatatcatggatgactattatagaggctttataagtgagacgctatcttctattgatgacattgactggaccagtttgtttgagaagatg

SEQ ID NO: 198 - DNA, 255 bp, Artificial Sequence
  Description of Artificial Sequence: Synthetic polynucleotide
atgaataacggtacaaataatttccagaattttattggaattagttctctgcaaaagaccttgcgtaatgcacttataccaacagaaacaacccaacaattcattgtcaagaatggtataatcaaagaggatgagctaagaggagagaatagacaaattctaaaggatatcatggacgactactaccgtggttttatctcagagaccttgtcctctatcgacgacatagattggacatctttgttcgagaagatg

SEQ ID NO: 199 - DNA, 255 bp, Artificial Sequence
  Description of Artificial Sequence: Synthetic polynucleotide
atgaataatggaacaaataacttccagaacttcattggaatttcatctttgcagaaaacgttgcgaaatgcgttgattcctactgaaacgacgcaacaattcattgtgaagaatggtatcatcaaagaggatgagcttcgaggtgagaatagacagatcctcaaagacatcatggatgattactatagaggatttatatctgaaaccttgtcctccattgatgacatcgattggacttcactcttcgagaagatg

SEQ ID NO: 200 - DNA, 255 bp, Artificial Sequence
  Description of Artificial Sequence: Synthetic polynucleotide
atgaacaacggaacaaacaacttccagaatttcatcggtatctcctctctccagaagactcttcgcaatgcgcttattcctacagaaaccacacagcaattcatagttaagaacggaattataaaggaggatgagttgagaggtgagaacagacagatactgaaagatattatggatgattactaccgtggatttatatcggagactctgtcaagtattgatgatatagattggactagtctattcgaaaagatg

SEQ ID NO: 201 - DNA, 255 bp, Artificial Sequence
  Description of Artificial Sequence: Synthetic polynucleotide
atgaacaatggaactaataatttccagaacttcattggtatcagttcgctccaaaagactttaagaaatgctttaatccctactgaaactacacagcagttcattgtaaagaatggaataattaaggaggacgaattacgtggagagaaccgtcagatcctcaaggatatcatggatgattattatcgtggcttcatcagcgaaacgttatcgtcaatcgatgacatcgattggacatcattattcgaaaagatg

SEQ ID NO: 202 - DNA, 255 bp, Artificial Sequence
  Description of Artificial Sequence: Synthetic polynucleotide
atgaacaacggaactaataacttccagaacttcattggaatatcatctttgcagaagacattgcgcaacgcccttatccctacagagactacgcagcaatttatcgttaagaacggcataataaaggaagatgagcttcgtggtgagaaccgacagattcttaaggatattatggatgactattaccgtggattcatttcggaaactttatctagtatcgacgacatcgactggacgagcttatttgagaaaatg

SEQ ID NO: 203 - DNA, 255 bp, Artificial Sequence
  Description of Artificial Sequence: Synthetic polynucleotide
atgaataacggtactaacaacttccagaatttcatcggtatcagctctctgcaaaagaccttacgtaatgccctgataccgacagagactacccagcagttcatcgttaagaatggaatcatcaaggaagatgaattacgcggcgagaatcgtcagatactgaaggatatcatggatgattattatcgtggctttatctctgaaaccctgagcagcatagatgacatcgattggacgagcttatttgagaagatg

SEQ ID NO: 204 - DNA, 255 bp, Artificial Sequence
  Description of Artificial Sequence: Synthetic polynucleotide
atgaataacgggaccaataactttcagaacttcatcggtatttcgagcttgcaaaagacactgaggaacgccctgatcccgacagagacaacgcagcagttcatcgtgaagaacggtattatcaaggaagatgaactgcgcggcgagaaccgacagattctgaaagatatcatggatgactactatcgtgggttcatttccgagacgctgtcttcaattgacgacattgactggacgagcctgtttgagaagatg

SEQ ID NO: 205 - DNA, 255 bp, Artificial Sequence
  Description of Artificial Sequence: Synthetic polynucleotide
atgaacaatggcacgaataactttcagaacttcattggaatttcgagtttacaaaagacgttacgtaacgcgctcatcccgaccgaaacgactcagcaattcatcgtcaagaatggcattatcaaagaagatgaacttcgaggggagaaccgccagattctgaaagacatcatggatgactattaccgtgggttcattagcgaaacattatctagcatcgatgacattgattggacgagtctctttgagaagatg

SEQ ID NO: 206 - DNA, 255 bp, Artificial Sequence
  Description of Artificial Sequence: Synthetic polynucleotide
atgaataatggtacgaataacttccagaatttcatcggtatatcttctctgcagaaaacgttgcggaatgccctaatcccgacagaaaccactcagcaatttatcgtgaagaacggcattatcaaagaagatgaactgagaggagagaatcgccagatactcaaagatatcatggacgattactatcgcggcttcatctcggaaacgctgagtagtattgacgacattgattggacatctctgtttgagaagatg

SEQ ID NO: 207 - DNA, 255 bp, Artificial Sequence
  Description of Artificial Sequence: Synthetic polynucleotide
atgaacaacggtactaacaacttccagaactttattggtatctcgagcctgcaaaagaccttgcgtaacgctttaatcccgacggaaacgacccagcaattcattgtaaagaacggtattatcaaggaggacgaattacgtggtgagaaccgccaaatcctcaaagatataatggatgattattacagaggattcatcagcgagacgctcagttctattgatgacatcgactggaccagtctgtttgagaagatg

SEQ ID NO: 208 - DNA, 255 bp, Artificial Sequence
  Description of Artificial Sequence: Synthetic polynucleotide
atgaacaatggaactaacaatttccagaacttcattgggatcagttccctgcaaaagacgcttcgaaacgcactcataccgaccgaaactactcaacaattcatcgtcaagaacggcataatcaaagaagatgaactccgtggcgagaaccgtcaaattctcaaagatattatggacgattattatcgtggctttatttccgaaacattatcatcgatcgatgatattgattggacgtctttatttgagaagatg

SEQ ID NO: 209 - DNA, 255 bp, Artificial Sequence
  Description of Artificial Sequence: Synthetic polynucleotide
atgaataatggtacgaataacttccagaatttcattggtattagctcactccaaaagaccttacgcaacgcattaattcctaccgagaccacccaacagtttatagtgaagaacggaataatcaaagaagacgaacttcgaggtgagaaccgacaaattctgaaggacataatggatgattactatcgcgggtttatctcggaaaccctctctagcattgacgatatcgactggacaagtttatttgagaagatg

SEQ ID NO: 210 - DNA, 255 bp, Artificial Sequence
  Description of Artificial Sequence: Synthetic polynucleotide
atgaacaatgggactaacaatttccagaacttcattggcatttcaagtctgcaaaagactctgcgtaatgccttgattcctaccgaaactacacagcagtttatcgttaagaacgggatcattaaagaagatgagctgcgaggcgagaatcgccaaatcctgaaggatattatggacgactattatcgtggcttcatcagcgaaaccctgtcttcgatagatgacattgattggacgtcattgtttgagaagatg

SEQ ID NO: 211 - DNA, 255 bp, Artificial Sequence
  Description of Artificial Sequence: Synthetic polynucleotide
atgaacaatggtacaaataacttccagaactttattggtatcagctctctgcaaaagaccctgcgcaatgcgcttattccaacggagacgacccaacagtttattgtcaagaacggcatcattaaagaggatgagctgcgcggtgagaatagacaaatcctgaaggatattatggatgattattatcgtggcttcatctccgaaacgttaagttctattgacgacatcgattggacatcgctctttgagaagatg

SEQ ID NO: 212 - DNA, 255 bp, Artificial Sequence
  Description of Artificial Sequence: Synthetic polynucleotide
atgaacaatggtaccaataatttccagaatttcatcggtatctcttctctgcagaagacgctacgtaatgcgttaatcccaaccgagacaactcaacagttcattgtgaagaacgggatcatcaaagaagatgaattacgcggagagaatcgccaaatcctgaaggacatcatggatgactattatcgtggattcatatctgaaaccctgagctctatcgacgatattgactggacctctctctttgagaagatg

SEQ ID NO: 213 - DNA, 255 bp, Artificial Sequence
  Description of Artificial Sequence: Synthetic polynucleotide
atgaacaacggcactaataacttccagaatttcattggcataagcagcctgcaaaagacgctgcggaacgcgctgatcccgaccgaaacaactcagcagtttatcgtcaagaatggtattattaaagaggatgaactgcgcggagagaatcgtcagatccttaaggatatcatggatgactactatcgtggctttattagtgaaacgttgtcttctatcgatgatattgactggacctcattgtttgagaagatg

SEQ ID NO: 214 - DNA, 255 bp, Artificial Sequence
  Description of Artificial Sequence: Synthetic polynucleotide
atgaacaatggcaccaataacttccagaacttcatcggcatctctagcttgcagaaaaccctgcgtaacgctctcattcccaccgaaactacccaacagttcatagtcaagaacggtattattaaggaggatgaactccgcggtgagaatcgtcagattctgaaagatatcatggatgattattaccgcggtttcatttctgaaacgttaagctcgatcgacgatatcgattggacgagtctgtttgagaagatg

SEQ ID NO: 215 - DNA, 255 bp, Artificial Sequence
  Description of Artificial Sequence: Synthetic polynucleotide
atgaacaacggtacgaataacttccagaactttatagggatatcgagcctgcagaaaactttacgcaacgccctgattccaacggagacgacgcaacagtttattgtaaagaatgggattatcaaagaagacgaattacgcggcgagaaccgtcagattctgaaagatatcatggatgattattatcgtgggttcatcagtgaaacgctgtcgtctattgacgatatcgattggacgtcactgttcgagaagatg

SEQ ID NO: 216 - DNA, 255 bp, Artificial Sequence
  Description of Artificial Sequence: Synthetic polynucleotide
atgaacaatggaaccaacaacttccagaactttattggtatcagctcgctgcaaaagaccctgagaaatgctctgattccaacggaaactacgcagcaatttatcgtaaagaatggtattattaaagaagatgaacttagaggagagaatcgtcagatcctgaaagacattatggatgattattacagggggttcatctcagaaacgttaagctcaattgacgacattgattggactagcctgttcgagaagatg

SEQ ID NO: 217 - DNA, 255 bp, Artificial Sequence
  Description of Artificial Sequence: Synthetic polynucleotide
atgaacaatggtaccaacaatttccagaatttcatcggcattagcagtctgcagaagaccttacgcaacgcactgattccgacagaaaccacacagcagttcatcgtaaagaatggaattataaaggaggacgagctgcgaggcgagaatcgacagatcctgaaagacatcatggatgactattaccgtggattcatttcggagaccctgtcttctattgacgacattgattggaccagtttatttgagaagatg

SEQ ID NO: 218 - DNA, 255 bp, Artificial Sequence
  Description of Artificial Sequence: Synthetic polynucleotide
atgaacaatggtaccaacaacttccagaatttcatcggcatttccagcctgcaaaagactctgcggaatgcgctgattccaaccgagacgacgcaacagttcattgtaaagaacggcattatcaaagaagatgagctgaggggtgagaatcgccagatcctcaaagatattatggatgactattatcgtgggtttatatccgaaacgttgtcatcaatcgatgacatagattggacatctctgttcgaaaagatg

SEQ ID NO: 219 - DNA, 255 bp, Artificial Sequence
  Description of Artificial Sequence: Synthetic polynucleotide
atgaataatggtacgaacaactttcagaatttcattgggatctccagtctccagaagacgttacgcaacgcattaataccgacagaaactactcaacaattcattgtgaagaatggaatcattaaggaggatgaactgcgcggcgagaatcgtcagatattgaaggatatcatggatgattactacagaggtttcatctcagaaaccttgtctagcatcgatgatatagattggacgagcctgtttgaaaagatg

SEQ ID NO: 220 - DNA, 255 bp, Artificial Sequence
  Description of Artificial Sequence: Synthetic polynucleotide
atgaataatggtacgaacaactttcagaattttatcggtattagtagccttcagaagacattgcgcaacgctctgatcccgactgaaacaacccagcagttcattgtcaagaacggcattattaaggaagacgaactgcgaggtgagaaccgtcagatactgaaggatattatggacgattattatcgcgggttcatttcagaaaccctctcgagcattgatgatattgactggaccagtttgttcgagaaaatg

SEQ ID NO: 221 - DNA, 255 bp, Artificial Sequence
  Description of Artificial Sequence: Synthetic polynucleotide
atgaacaatggtaccaacaacttccagaatttcatcgggatcagctcgctccagaagaccctgcgcaatgcactgatcccgactgagaccacacagcagttcattgtaaagaacggtattatcaaggaagacgagcttcgcggcgagaacagacaaatcctcaaggatatcatggatgattattatcgcggcttcatttctgaaaccctgtcctctatcgatgatatcgattggacctcattatttgagaaaatg

SEQ ID NO: 222 - DNA, 255 bp, Artificial Sequence
  Description of Artificial Sequence: Synthetic polynucleotide
atgaataacggaactaacaactttcagaatttcatcggtatcagcagcttgcaaaagacactgcgtaatgcgctgatcccgacggaaacgacgcaacagtttatcgtgaagaacgggattatcaaagaagatgaactgcggggcgagaaccgacaaatcttgaaagatatcatggatgattattatcgtgggtttatctcagaaactctcagcagcatcgacgatatcgactggacctctttgttcgagaagatg

SEQ ID NO: 223 - DNA, 3792 bp, Artificial Sequence
  Description of Artificial Sequence: Synthetic polynucleotide
atgaataacggcactaataacttccagaatttcattggcatatcttccttacagaaaacacttagaaatgctttgatcccgacggagactacacagcagtttatcgtgaagaacggcataattaaggaggatgaattgaggggagagaaccgtcaaatactcaaggatatcatggatgactactatagagggttcattagcgaaactctttcttccatcgatgatatagattggacttccctcttcgagaagatggaaatacagctcaagaatggagataacaaggatactcttatcaaagaacagactgagtatcgtaaagcaatccataagaaatttgctaatgacgatagattcaagaacatgtttagcgctaagctaatatcagacatcttgcctgagtttgttatccataataacaattatagtgcttccgagaaggaagagaagacacaagttataaagttgttctcacgattcgctacttcatttaaagactattttaagaaccgcgctaattgtttctctgctgacgatatctcttcttcttcttgtcatcgtatagttaatgacaacgctgaaatcttcttctcaaacgctctcgtttatagaagaatcgttaagtctttaagtaacgatgatattaacaagattagcggtgatatgaaagacagccttaaggagatgtcattggaagaaatttatagttacgagaaatatggcgaatttatcacacaggagggtatctcgttctataatgacatatgtggaaaggtgaacagcttcatgaatctatattgccagaagaataaggagaataagaacttatacaaacttcagaagctgcataaacaaatactttgcattgcagataccagctacgaggtcccgtataaattcgagtctgatgaggaggtttatcagtcagtaaacggattcttagataacatcagtagtaaacacattgtggaacggttaaggaagattggagacaattacaacggatataatttggataagatatacatcgtttctaaattctacgagagtgttagccagaaaacctacagagattgggaaaccataaatactgctttagagattcactacaacaacatccttccaggaaacggtaagagtaaagctgacaaagttaagaaggctgttaagaacgatctgcagaaatcaataacagaaatcaatgaattagtttctaattacaagctttgctctgatgataatatcaaagctgaaacctacattcatgaaatctcgcatatcctgaacaacttcgaagcacaagaattgaagtacaatcccgagatacatcttgtagagtcagaattgaaggcttcggaacttaagaatgtactagatgtcataatgaatgctttccactggtgctcagtattcatgaccgaggaattagttgataaggataacaacttctacgccgaattagaagaaatttacgatgagatataccctgtcatcagcttgtacaaccttgtgaggaattatgttacccagaaaccttactctactaaaaagatcaaacttaacttcggaatccctactctggcagatggttggtccaagtcgaaggagtattcgaataacgcaataatacttatgagagataatttatattaccttggtatcttcaacgcgaagaacaaaccggataagaaaattatagagggtaacacgtctgagaacaaaggtgattataagaagatgatatacaatttactgcctggtcctaacaagatgatacctaaggtattcctctctagcaagactggagtggaaacttataagccgtctgcctatattctcgaagggtacaagcagaacaagcacataaagagttcgaaggatttcgatattactttctgtcatgacctaatagactactttaagaactgtattgctatccaccctgaatggaagaacttcgggtttgatttcagtgatacatctacctacgaggatatatctggattctacagagaggttgaacttcagggttacaagattgattggacatacatctctgagaaagatattgatcttctgcaggagaagggacaattgtatctcttccagatctataataaggacttctcgaagaagagtactggaaacgataaccttcacacaatgtatctcaagaatttgttttcagaggagaatctcaaagatattgttctcaaacttaatggcgaggcagagatattcttcaggaagtcgtcgataaagaacccgatcatccataagaaaggatcaatcttagtcaacagaacttatgaagccgaagagaaggaccaatttggaaatatacaaatagttagaaagaacattccggagaatatttaccaggaattatataaatacttcaatgacaagtcagataaagaattgagcgacgaagcggctaaactcaagaacgttgttgggcaccacgaggcagctactaatatcgttaaggattaccgttatacatatgacaagtatttcttacacatgccaattacaatcaatttcaaggcaaataagactggctttattaacgaccgaattcttcaatacatagcaaaggagaaagatctgcacgtgataggaattgaccgtggagaaagaaatctcatctacgtgtctgttatcgacacttgtggtaacatagtagagcagaagtcatttaatatagtaaatgggtacgactaccaaataaagttaaagcagcaagagggagcacgtcagatcgcaaggaaggagtggaaggagattggaaagataaaggagattaaagaaggatatctaagtcttgtcatacatgagatttccaagatggtgatcaagtacaatgctattattgctatggaagatttgagttacgggttcaagaagggaagattcaaagtagagcggcaagtatatcagaagttcgaaacaatgttgatcaataaattgaattacttggtcttcaaagatatttctatcacagagaacggaggccttctcaaaggctatcaacttacctatattcctgataagctcaagaacgttggacatcaatgcgggtgcattttctacgttccagcggcatacacctcgaagatcgatcctactacgggattcgtgaacatatttaagtttaaggatcttactgtggatgcaaagagggaatttattaagaagttcgattctataaggtacgactctgaaaagaatttgttctgctttacatttgattataataacttcataacacagaataccgttatgtctaagagttcgtggtccgtgtacacatacggagtgcgtattaagagacgcttcgtcaatgggcgcttctctaatgagtcagataccatcgacatcactaaagacatggaaaagactctagagatgacggacattaactggagagatgggcacgatctaagacaagatattatcgattacgaaattgtacagcatatatttgagatctttagactgacagtccaaatgcgtaattcactttctgaactcgaggaccgtgactatgatcgtttaatctcgccggtgctgaacgagaataatatcttttatgatagtgcgaaggctggagacgctcttccgaaggatgctgatgctaacggtgcatattgtattgctttgaaaggtctttatgaaattaaacagattactgagaactggaaagaagatgggaagtttagtcgtgacaaacttaagatttcaaacaaggattggttcgacttcattcagaacaaacgctacctgtga

SEQ ID NO: 224 - DNA, 3792 bp, Artificial Sequence
  Description of Artificial Sequence: Synthetic polynucleotide
atgaataatggcaccaataacttccagaacttcatcggaatctcctcccttcagaaaacactgagaaatgctcttatccctactgaaactacacaacaattcattgtaaagaacggaataattaaggaagatgaattgcgtggtgagaacaggcaaatactcaaggacatcatggatgactattaccggggattcatttcagagactttatcctccattgatgatatagattggacgtcgttgttcgagaaaatggaaatccagttgaagaatggagataataaagatacgttgatcaaagaacagactgagtacaggaaggctatacacaagaaatttgcaaatgacgatcggttcaagaatatgttcagtgctaaactcatttctgatatacttcctgaatttgttattcataataacaattattccgcttcagagaaggaagagaagactcaagtgatcaaattattctctaggtttgctactagcttcaaggattactttaagaaccgtgctaactgcttctcggccgatgacatttcatccagttcttgccacagaatagtaaatgataacgcagagatatttttctctaatgctttggtctatcgtagaattgttaaatctttgtctaacgacgatatcaacaagatatcaggagatatgaaagactctcttaaagaaatgtctcttgaagaaatttattcttatgagaagtacggagagtttattactcaggaaggcatctctttctataacgatatatgcggtaaagttaattcatttatgaatttgtactgccagaagaataaggagaataagaatctttacaaactgcagaagctacataagcagattctgtgcatcgccgatacgtcttatgaggtgccgtacaagttcgagagcgacgaggaggtgtatcaatccgtcaacggattcctagataatatcagcagcaagcatatagttgagaggctacggaagatcggagataattacaatggatataatttggacaagatctatattgtttcaaagttctatgaatccgtttcacagaaaacctaccgggattgggaaaccattaacactgcacttgagattcattataacaacatccttccaggaaatggcaaatcgaaggcagacaaagtcaagaaagcagttaagaatgaccttcagaagtccataactgaaattaacgagcttgtctcaaattacaaattatgctctgatgataacattaaagctgagacgtatatccatgagatctctcatatcttaaataatttcgaagctcaagaacttaagtacaatccagaaattcatttggtggaaagcgaacttaaggcttcagagctaaagaatgtcctagatgtgattatgaatgcatttcattggtgtagtgtgttcatgactgaggagttagtggacaaagataataatttctatgcagagctcgaggaaatctacgacgaaatttacccggttatctcattgtacaacctagttagaaactacgtgacccagaagccatactctactaaaaagattaaattaaacttcggtatccctaccttagcggatggttggtctaaaagcaaggagtattccaacaacgcaatcatcttgatgagggacaatctttattacttaggtatatttaacgcgaagaataagccagataagaagattatagaaggcaatacctcagagaacaaaggagattacaagaagatgatttacaatctgctgccgggaccgaataagatgatcccaaaggtcttcctttcatctaagacaggagttgaaacatataagccgagtgcatatatactcgagggttataagcagaacaaacatattaagtcaagcaaagacttcgacatcaccttctgccacgatcttatcgactatttcaagaactgtattgcaatacacccggagtggaagaacttcggcttcgacttctcagatacttctacctatgaggacatttctggtttctacagggaagttgaacttcaaggttacaagattgattggacatatatttctgagaaggatatagacctgttacaagagaagggccagctttacttgtttcaaatatataataaggacttctcaaagaaatctacgggtaacgataatttacacactatgtacttgaagaatctattctcagaggagaatctcaaagatattgtcttgaaattgaacggagaagccgagattttcttccgtaagtctagcataaagaacccgatcatccacaagaaagggagcatattggtcaatagaacctacgaagctgaagagaaggaccaattcggaaacattcagatagttcggaagaatatccctgagaatatttatcaggagttgtacaagtatttcaacgataaatctgataaggagctgagcgatgaagctgctaagttgaagaacgttgttggtcatcacgaagctgctacaaacatagttaaggattatcggtacacttatgataaatatttccttcatatgccaattactatcaacttcaaggcaaataagactggctttatcaacgacaggatcttacaatacattgcgaaggagaaagacttgcatgtcatcggtattgatcgtggcgaaagaaacctcatctacgtgtccgtcattgacacatgcggtaatatcgtagagcagaaaagcttcaatatcgtaaacggttatgattatcaaattaagttgaaacagcaagaaggtgctcgtcagattgcgagaaaggagtggaaggagatcggaaagataaaggagatcaaagaaggatacctgtccctcgttatccacgaaattagcaagatggttatcaagtataatgcgatcattgctatggaggatctaagttatggatttaagaaaggaaggttcaaggttgaaaggcaggtttatcagaagtttgaaactatgttgattaacaaactaaactacttggtgttcaaagacatttcgatcactgagaatggaggattgcttaagggttaccaactcacatacatacccgataaactgaagaatgttggtcaccaatgcggctgtatattctacgtaccggctgcatacacatcaaagatcgatcctactaccgggtttgtgaatatctttaagtttaaggatcttactgttgacgcgaagagagagtttatcaagaagtttgactccatacgttatgattctgagaaaaacctcttctgcttcaccttcgattataacaatttcataacacagaatacagttatgagcaaatcctcttggagtgtctacacatacggagttcgaataaagaggagattcgtaaacggtcgtttctctaatgaatctgataccattgatatcactaaggacatggagaagaccctcgaaatgaccgacatcaactggagagacggacatgatctgcgacaagacatcattgattacgaaatcgttcagcatatcttcgaaatcttccgattgacggtccagatgcggaatagcctatctgagctcgaagacagagattatgatcgccttatatcgcccgtgttgaatgagaataatatattctacgacagcgcaaaggccggagatgcgctgcctaaagatgctgatgcaaacggagcatactgtatcgccttgaagggtttatacgagatcaaacaaataaccgagaactggaaggaagatgggaaattctctcgcgataagttgaagatttctaataaggactggtttgatttcatacagaataagagatacctttaa

SEQ ID NO: 225 - DNA, 3792 bp, Artificial Sequence
  Description of Artificial Sequence: Synthetic polynucleotide
atgaacaatggtaccaataatttccagaacttcatcggaatttcatcactccagaagacccttaggaacgcccttattccaaccgaaacaacacagcaattcatagtcaagaacggcatcattaaggaggatgagcttcgcggggagaatcgacaaatactcaaagatattatggatgattattacagaggattcattagtgaaaccctcagtagcatcgatgatatcgattggacaagtctattcgagaaaatggagattcagcttaagaatggagacaataaggacactctcatcaaggaacaaactgaatatcggaaggcaattcataagaaattcgcaaatgacgataggttcaagaatatgttctcagctaagctaatctctgatatcctaccagagtttgttattcataataacaattacagtgccagcgagaaggaggagaagacccaagttattaaattattctccaggtttgccactagctttaaagactacttcaagaatcgggctaactgcttctccgccgatgatatatctagttcatcatgccatcgaattgttaatgacaacgcagaaatcttcttctctaatgccttagtctaccgaaggatcgttaagtctttgagtaatgacgatattaataagatcagcggagatatgaaagattctctaaaggagatgagtttagaagaaatctactcttacgagaaatatggcgaatttataacccaagagggtatcagtttctacaatgacatttgtggcaaggtcaactctttcatgaacctgtattgtcagaaaaataaagagaacaagaatctttacaaattgcagaagttgcataaacaaatactttgcattgctgatacttcctacgaggttccatataagttcgagagcgatgaggaggtttaccagagtgtaaacggatttcttgataacatatcctcaaagcacatagtggagcgtttgagaaagatcggagataactacaacgggtacaacttagacaagatatatattgtgtccaagttctatgaatctgtaagccaaaagacgtatcgggattgggaaacaataaatactgcccttgagattcactataataacatcttgccaggcaacggtaagtctaaagcagataaagtaaagaaggcagtcaagaacgacttgcagaagtctatcaccgagattaatgaacttgtttctaattataagttatgtagcgatgataacatcaaggctgagacctatatccatgaaattagccacatcctcaataacttcgaagctcaggaattgaagtataatccggagatacatttggttgaatccgaactcaaagcatcagaacttaagaacgtcttggatgtcatcatgaatgccttccactggtgtagtgtattcatgaccgaagagttagttgataaagataacaacttctacgcggagttggaagagatttatgatgagatttatccagttatctctctctacaacctagttagaaactatgttactcagaaaccttattccactaagaagattaagttaaacttcgggattccaactcttgctgacggatggtctaaatcaaaggagtattctaacaatgcaattatccttatgagagataacttatattacttaggaatcttcaacgctaagaataaacctgacaagaagatcattgaaggtaatacgagcgagaacaaaggagattacaagaagatgatttataacttgcttccaggacctaacaagatgatccctaaagtgttcttgtcctcgaagacaggtgttgaaacttacaagccatctgcgtatatcttagaaggatataagcagaacaaacatatcaagtcgtctaaagacttcgatatcactttctgtcacgatctgatagactactttaagaattgtattgctattcatccagaatggaagaacttcggattcgatttctcagacacatcgacttatgaagatattagtggattctatagagaagtcgaacttcaaggctataagattgactggacctatatttcagagaaggatattgatttactgcaggagaagggacaactctacttatttcaaatatacaacaaggacttctctaagaaatcaactggcaatgataatttacacacgatgtacttaaagaatctcttctctgaagagaaccttaaggatatagttctgaagttaaatggcgaggcggagatattcttcagaaagtcatcgatcaagaacccaattatccacaagaagggatccatactagtcaatcgtacatatgaagctgaagagaaagatcaattcggtaatatccagattgtgcgcaagaacataccagagaacatctaccaagagttgtataagtactttaacgataaatctgacaaagaacttagcgacgaagcagctaagcttaagaacgttgtgggacatcacgaagcagctaccaatattgtgaaggattacagatacacgtacgataagtactttcttcacatgccaattaccataaacttcaaagctaacaagactggattcattaacgatcgaattctacagtacattgcaaaggagaaagatttacatgtgattggaatagaccgaggcgagcggaaccttatttacgtatctgttatagatacttgtggaaacatcgtagagcagaagtcgtttaatatcgtgaatggatacgactatcagatcaagctaaagcagcaggaaggagcccggcaaatagctcgtaaggagtggaaagaaatcggtaagatcaaggagattaaagaaggatatctcagtcttgtaatccatgagatctcaaagatggtcattaaatataacgcgatcatagccatggaagacttatcttacggatttaagaagggcaggtttaaagtcgaaagacaagtttatcagaagttcgaaacgatgttgattaataagcttaattatctagtcttcaaggatatctctataaccgagaacggaggcttgttgaagggataccagttgacctatatccctgataaacttaagaacgttggtcatcagtgcggctgtatattctatgttccagcagcttatacatccaagatagaccctacgacagggtttgttaatatctttaaatttaaggacttaacggtggatgccaagcgtgaatttattaagaagtttgacagtatccggtacgactccgagaagaatctgttctgtttcactttcgattacaataacttcattacgcagaacacagttatgtccaagagttcatggagtgtttatacctacggagttaggatcaagaggagatttgttaacgggagattctcaaacgagtcagatacaattgatatcactaaggatatggagaagacattggaaatgactgatataaattggagagatggacacgatttaagacaggacattattgattatgaaattgttcagcatatcttcgaaatatttaggctaacagttcaaatgcgtaattcattgagtgaacttgaggatcgggactacgatagattgatatcgcccgtattgaacgagaataacatattctacgattccgcgaaggctggagatgctttaccaaaggatgctgacgcgaacggtgcttactgcattgctttaaagggactttatgagatcaagcagattacagagaattggaaagaagatggtaagttctctagagataagctcaagattagtaataaagattggtttgatttcatacagaataagcgttatctttag

SEQ ID NO: 226 - DNA, 3792 bp, Artificial Sequence
  Description of Artificial Sequence: Synthetic polynucleotide
atgaataacgggaccaacaacttccagaatttcattggtatatccagccttcagaagaccctaagaaacgctcttatccctactgagactacacagcagtttatagtcaagaatgggattataaaggaagatgaattaagaggagagaatcgacagatactcaaagacataatggatgattactaccgtgggttcatatcagaaaccctctcgtcgattgatgatattgactggactagtctattcgagaagatggaaattcagcttaagaacggagataataaggatactttgattaaggagcaaacagagtaccgtaaagctatccataagaagttcgccaatgatgatagattcaagaatatgttctctgcgaagttaataagcgacatattgcctgaattcgtaatccacaataataactattccgcgtcagagaaggaggagaagacacaggtgatcaaacttttctcaagatttgctacgagtttcaaggactactttaagaaccgtgcgaactgcttctcagcagatgatatctcatctagcagctgccatcggatcgttaatgataacgcagaaatctttttctcaaatgctcttgtttatagaagaattgttaaatccttgagtaatgatgacattaacaagatttcgggagatatgaaggattctttgaaggaaatgtcgcttgaggaaatatattcgtatgagaaatatggtgagtttatcactcaagagggaatttcgttctataatgatatctgtggaaaggttaactcattcatgaatctgtactgtcagaagaacaaagagaacaagaatttatacaaactccagaagttgcacaagcaaatactctgtattgctgatacatcttacgaggttccatacaagttcgagagcgacgaggaggtctaccagtctgttaatggcttcttagataacatctctagtaaacatattgttgaacgactgagaaagattggagacaactataacggttataacctagataagatttatattgtgtcaaagttctatgagagcgtttctcagaaaacgtatcgtgactgggaaacaatcaacacagcattggaaattcattataataatattcttcctgggaacggaaagtcaaaggcagataaggttaagaaagctgtgaagaatgatttgcagaagtctattacagagatcaatgaacttgtgagcaactacaaactttgtagcgatgataacattaaagcagaaacttatatacatgaaatatcacatattcttaataacttcgaagcacaagagctaaagtacaatcctgaaatccatttagtggagagcgagctcaaggccagtgaattgaagaatgtgctagacgtcatcatgaatgctttccactggtgtagtgtgtttatgactgaagaattagtggataaggataataatttctatgctgagctcgaagaaatatacgacgagatttatccagtaatctccctctacaatctcgttagaaactatgttacccagaaaccttactcaactaagaagattaaactcaactttggcatacctacactggctgacggttggtcgaaatcaaaggaatatagtaacaacgcgatcattctcatgcgtgacaatttatattatttaggtatctttaacgcgaagaataaacctgacaagaagatcattgagggaaatacgagcgagaacaaaggagattataaaaagatgatttacaacctgttgcctggtccaaataagatgataccaaaggtattcctatcttcgaagactggagttgaaacgtacaaaccatctgcatacatactggagggttacaaacagaacaaacatataaagtcaagcaaggatttcgacataaccttctgtcatgatttgatagactacttcaagaactgtatcgccatccatccagaatggaagaactttggtttcgatttctccgacacttcgacatatgaagacatctccggtttctatagggaagttgaactccagggttataagatcgactggacatacatctcagagaaagacatagatttgcttcaggagaagggtcagctgtacctgtttcagatctacaataaggatttcagcaagaagtccactggtaatgataatttacatacaatgtatttgaagaacttgttcagtgaagagaatttgaaagatattgtgcttaagcttaatggagaagctgaaatatttttccgaaagtccagcataaagaatccgataattcacaagaagggttctatactggtgaataggacatacgaagctgaagagaaagatcagttcgggaatattcaaatcgttagaaagaacattccagagaatatctatcaagaactatataaatacttcaacgataaatctgacaaagaacttagtgatgaggctgcgaaattgaagaatgttgttggacaccatgaagctgcaacaaatatcgttaaagattatagatatacttacgataaatatttccttcacatgcctataacgatcaatttcaaagctaacaagacaggatttattaatgacaggatcctgcaatacattgctaaagagaaggacttacacgtcatcggtatcgaccgcggcgagagaaatttgatttatgtttctgttattgatacttgtggtaatattgtggagcagaagagctttaatatcgtgaatggatatgattatcagattaagttaaagcaacaagagggagcgaggcaaatcgctaggaaggagtggaaagagataggcaagattaaggaaattaaggagggctacttgtctttggtaattcatgagatttctaagatggttattaaatacaatgcaattattgccatggaggatttgagttacggcttcaagaaagggcgattcaaagttgagcggcaagtttatcagaaattcgaaacgatgcttattaataaattgaactatttagtatttaaagacatttctataaccgagaacggcgggttattaaagggatatcaattgacatatatacctgataagttaaagaatgtgggtcatcagtgtggttgcatcttttatgtacctgcagcgtatacatccaagatagatccgactactggatttgtgaatatctttaagtttaaggatttgaccgttgacgcaaagcgtgaattcatcaagaaattcgatagcatcaggtatgactctgagaagaatctcttctgcttcaccttcgattataacaatttcattacacagaatacggtgatgtctaagtcctcttggtccgtttatacatatggtgttagaatcaagaggagatttgtcaacggtcgtttctcaaacgagagcgatacgattgacattactaaggatatggagaagacgctcgagatgactgatattaactggcgggatgggcatgaccttagacaggacattatagattacgagatcgttcagcatatatttgaaatattcagactcacggttcaaatgaggaactcactctcagagctcgaggatagagattatgatcgcctcatatcacctgtactcaatgagaacaatatcttttatgattctgctaaggctggtgacgctcttccaaaggatgctgatgcaaacggagcgtattgtatcgcactcaagggtctatacgagattaagcagatcaccgagaactggaaggaggatgggaagtttagtagggataagctcaagatttctaacaaagattggttcgacttcattcagaataagagatatctgtga

SEQ ID NO: 227 - DNA, 3792 bp, Artificial Sequence
  Description of Artificial Sequence: Synthetic polynucleotide
atgaataatggaactaacaactttcagaacttcatcggaatctctagtttgcagaaaacccttcgaaacgcattgatacctacagagacgacacaacaattcattgttaagaacggcattattaaagaggacgagcttagaggagagaataggcaaatactcaaagacattatggatgactattaccgtgggtttattagcgaaactttaagctccattgatgacatagactggacctcattgtttgagaagatggagatacaactgaagaatggagataataaggatacattaatcaaggagcagactgagtaccgaaaggcaattcacaagaaatttgctaacgatgacaggtttaagaatatgttctctgctaaactgatatctgatatactgccggagtttgtgatacacaacaataactattctgctagtgagaaagaagaaaagactcaggtcatcaagttattctcaagattcgccacttcattcaaagactactttaagaaccgagccaactgcttcagtgcagacgatatctcgtcttcttcatgtcatcgcatagtgaacgataacgcagaaatatttttctcgaatgctctcgtttatagacgcatcgtcaagagccttagtaatgacgatatcaacaagatctccggcgatatgaaagattcattaaaggaaatgtctcttgaggagatttattcatatgagaagtacggagagtttataactcaagaaggaatttccttctataatgacatttgcgggaaagtaaattcgttcatgaatttatactgtcagaagaacaaggagaataagaacttatacaaattacagaaacttcataagcagattctttgcattgccgatacaagctatgaggttccgtacaaattcgagtctgatgaagaggtttaccaaagcgtcaatggcttcttagataacatatcgtctaaacatatcgtcgaacgtttacgaaagattggagataattataatgggtataatctcgacaagatttacatagtctccaagttctacgagtcagtttctcagaagacatacagagattgggagacgattaatactgctctggaaatccattataataacattctcccagggaatggtaagtccaaggctgataaagtcaagaaggcagtgaagaacgatctgcagaaaagcattaccgagataaacgaactggtctctaattacaagctctgcagcgatgacaatatcaaggctgagacctatattcacgagattagccacattcttaataacttcgaagcgcaagaattaaagtataatcctgaaatacacttggtcgagtcagagctcaaggcgtccgaacttaagaacgtgttagacgttatcatgaatgcattccactggtgctccgtattcatgacagaggagctcgttgacaaggataacaatttctatgctgagttagaagagatatacgatgaaatttacccagtgatatctctttacaatcttgtgcggaactacgtgacacagaaaccttactccactaagaagatcaagttaaacttcggtattccgacattagctgatgggtggagtaagtctaaggaatactctaacaacgcgattatacttatgagagataacctctattatcttggaatcttcaatgcaaagaacaaacccgataagaagataatcgagggaaacacttctgagaacaagggtgattataagaagatgatctacaatttattgcctggaccaaataagatgatccctaaagtgttcctatcttcaaagacaggagttgagacctataagccgtctgcttatatcctcgagggatacaaacagaataaacatataaagagttctaaagacttcgacattacattctgccacgaccttattgactactttaagaactgcatcgctattcatccagaatggaagaactttggcttcgacttctctgatacttcaacctatgaggacattagtggattctatagagaggtggagcttcaagggtacaagatcgattggacatacattagcgagaaagacattgatctgctacaagagaagggacaactttatctattccagatttataacaaagacttctctaagaagagtaccggaaatgacaatttgcataccatgtatctcaagaatttattctcagaggagaacttgaaagacattgtgctaaagctaaatggagaagcagagatattctttcgcaagtcctccatcaagaacccgatcattcacaagaagggttcgatattggttaacaggacatatgaagctgaggagaaggatcagttcgggaatattcagatcgtccggaagaacattcctgagaatatttatcaggaattgtataaatacttcaatgataagagcgataaagaactgtctgatgaagccgccaagctcaagaatgttgtagggcatcacgaagctgctactaacattgtcaaggattatagatacacttatgataagtatttcttacatatgcctataacaatcaacttcaaggctaacaagaccgggttcataaatgataggattcttcaatatattgctaaggagaaggacctgcatgttataggtatcgacagaggcgaaagaaacctcatatacgtctctgttattgatacttgcggtaacatcgttgaacagaagagctttaacatcgtaaatggatacgattatcaaattaaattgaagcaacaagagggtgcccgacaaatcgcgcgtaaggaatggaaggagattggtaagattaaggaaattaaggagggatatctgagccttgtcattcatgaaatatcaaagatggttatcaaatacaatgctattatagctatggaagacctgtcatacggttttaagaaaggtagatttaaggttgaacgccaggtttatcagaagtttgaaactatgctaattaacaaacttaattacttagtgtttaaggatatatccatcacagagaacggtggattgcttaagggataccaacttacgtacattccggataagctcaagaacgtaggacatcaatgtgggtgcatcttctatgttccggctgcttacacctcaaagatcgatccaacaaccggtttcgtaaacatcttcaagttcaaggatctgacggtcgatgcgaaacgagaattcataaagaaatttgattcaataagatacgattcagagaaaaacttattctgcttcacatttgattataataacttcataacacagaacacagtgatgagtaaatcatcatggtctgtatatacctacggagtcagaattaaacgtaggttcgttaatgggcgcttctctaacgaaagtgatacgattgacattacgaaggacatggaaaagacgctcgagatgactgatatcaattggagagatgggcacgatttgcggcaagacatcattgactatgaaatcgtgcaacacatattcgagatctttcgcctcacagttcaaatgcgtaattccctgagtgaattagaagatagagactatgatagacttattagccctgtgctgaacgagaacaacatattctacgatagtgctaaggcaggtgatgctcttcctaaggacgctgatgcaaacggcgcatattgtatcgctctcaaaggactctacgagatcaagcagatcacagagaattggaaagaagatgggaagttctctcgagataagttaaagattagtaacaaagattggtttgatttcatccagaacaagcgatacctttag

SEQ ID NO: 228 - DNA, 3792 bp, Artificial Sequence
  Description of Artificial Sequence: Synthetic polynucleotide
atgaataatggaacgaacaacttccagaacttcattggtatctcgtctctacagaagactttacgtaacgctctaatacctaccgagactacacaacaattcatcgttaagaacggaatcataaaggaggatgaactaagaggagagaacaggcagatccttaaggatatcatggatgattactatcgaggctttatctcagagaccttgtcaagtattgatgatatcgattggacgtcactatttgagaagatggaaatccaactaaagaacggtgataataaagatacgttaatcaaggagcagacggagtatcgcaaagcgatccataagaagtttgctaacgatgatagattcaagaacatgttctcagctaagctcatcagcgatatccttccggagttcgtaattcacaataataactattcagcatcagagaaggaggagaaaacgcaagttataaagctattctctaggttcgcaacgtctttcaaggattactttaagaatagagccaattgcttcagcgcagacgatatttcctcatcctcttgtcatagaatagtgaatgataatgccgaaatattctttagtaatgcattggtttataggagaattgtgaaatccttgagtaatgatgatatcaacaagattagcggcgacatgaaggattcccttaaggagatgagtttggaggaaatatacagttatgagaagtatggagagtttatcacccaagaagggataagtttctataacgacatatgcgggaaagtcaatagcttcatgaacttgtattgccagaagaataaggagaacaagaatctttacaagcttcagaaattacataagcagattctgtgtattgctgatacatcatatgaggtcccttataaattcgagtctgacgaagaggtctatcaaagtgtgaatgggttccttgataatatcagttctaaacatattgtggagcgtttgagaaagattggagataattacaatggatacaacttggacaagatctatatcgtttctaagttctatgaatctgtgtcacagaagacatatcgggattgggaaacaattaacaccgctttggaaatacactataacaatatcttgccaggaaatggtaaatctaaggctgataaggtgaagaaggcagtgaagaatgatctccagaaatctattacagagatcaacgaattagtgtcaaactataagttatgttctgatgacaacatcaaggcagagacttacatccatgaaatctcacatatcctgaacaacttcgaagctcaagagctaaagtacaaccctgagatccacttggtggaatctgaactcaaggcgtctgaactcaagaatgtgctcgatgttatcatgaatgcatttcattggtgcagtgtattcatgactgaggaactcgtagacaaggataacaacttctatgctgagctagaggaaatatatgacgagatatacccggtaatctctctgtataatcttgttagaaactacgtcacacagaagccgtattctaccaaaaagatcaagcttaactttggtataccaactctcgctgacgggtggtctaaatcgaaggagtattcaaataatgctatcatattgatgcgtgataacctttattatttaggaatctttaacgcaaagaataaacctgacaagaagatcatagagggtaatacatcagagaacaagggcgattacaagaaaatgatttataacttgttgcctggaccaaacaagatgatacccaaggtcttcctctcgtctaagactggtgtggagacttataaaccctctgcctacatacttgaaggatataagcagaacaagcatatcaaatctagcaaagactttgatattacgttctgtcatgaccttatcgattacttcaagaactgcatcgctatccacccagaatggaagaacttcggcttcgacttctctgatacgagtacatatgaggatatatctggattctaccgtgaagttgaattgcaaggatacaagattgattggacatatatttcagagaaagacatcgacttgttgcaggagaaagggcaactgtatctctttcagatttataataaagacttcagtaagaaatcgactggtaacgacaatcttcatacgatgtatttgaagaatctattctccgaagagaaccttaaggatatcgtgttgaaactcaatggagaagccgagatattcttccggaagtcatcaataaagaacccgattatccacaagaagggctcgatcctcgtcaacagaacgtacgaagctgaagagaaggatcaatttgggaacattcaaattgtacgtaagaatataccagagaatatttatcaggaactctataaatacttcaacgataagtcggacaaagaactgagtgatgaggccgctaagctaaagaacgtcgttggccatcatgaagcagctaccaatattgtcaaggattataggtatacttatgacaaatatttcttgcatatgccaatcaccataaatttcaaagctaacaagaccggattcattaacgatcgaattctgcaatacatagcgaaggagaaggatctccacgttattggaattgatcgcggagaaaggaatttaatatacgtttccgttattgatacgtgtgggaacatcgtggaacagaagtcctttaatatagttaacggatacgattaccaaatcaaacttaagcaacaggaaggcgctagacaaattgcccgtaaggagtggaaagaaattggaaagataaaggagatcaaggaaggttatttatctcttgttattcatgagattagtaagatggttatcaagtacaatgccattatagctatggaagatttgagttacggtttcaagaagggtaggttcaaagttgaacgacaggtctatcagaaatttgagaccatgctaattaacaagctcaattacttggtcttcaaggatatatctattacagagaacggcggacttctgaaaggataccagcttacttacatcccggataaactgaagaatgttggacatcagtgcggctgtatattttacgtgcctgctgcctatacttctaagatcgacccgaccaccggattcgtcaacatattcaaattcaaagatctgaccgttgatgctaagcgggagtttatcaagaaatttgacagcattagatacgactctgaaaagaatttgttctgtttcacattcgattacaataacttcatcacccagaacaccgtgatgtccaagtcatcgtggagcgtgtacacatatggtgttaggattaagcggaggttcgttaatgggagatttagtaatgagtcagatactatagacattacaaaggacatggagaagacacttgagatgacagatatcaactggagagacggacatgacttacgccaagatattattgattatgagattgtgcaacacatattcgaaatatttcgtctgaccgtgcaaatgcgaaactcgctgtcggaactagaggatagagattacgataggttgatctctcctgtgcttaacgagaataatattttctatgattcagctaaggctggagatgctttacctaaggacgctgacgcgaacggagcatattgcatcgctcttaagggattgtacgaaattaagcagattaccgagaactggaaggaagacggaaagttctcccgggacaaattaaagatctctaacaaggattggttcgatttcattcagaataagagatacctgtag

SEQ ID NO: 229 - DNA, 3792 bp, Artificial Sequence
  Description of Artificial Sequence: Synthetic polynucleotide
atgaacaatggcacaaacaactttcagaatttcatcggtatatcttctcttcagaagacgcttaggaatgccttgattccaactgagactacacaacagtttatagttaagaacggaatcattaaggaagatgaattacggggagagaatcgtcaaattctaaaggatatcatggatgactattatcgcgggtttatctcggagactctcagctcaatcgatgacatcgattggacctccttattcgagaagatggaaatccagttaaagaatggtgacaataaagatactttaattaaggaacagactgaatacaggaaggccatccacaagaagttcgccaacgatgatcgtttcaagaatatgttctcggctaagttgatctcagatatacttccagaatttgtcatccacaataacaactatagtgccagcgagaaagaagagaagactcaagtaattaaactgttctcacgatttgcgacaagcttcaaggactacttcaagaatagggctaattgtttctcagcagatgacatatcgtcgagtagttgccaccggatcgtcaacgataatgctgagatcttcttctcaaacgcgctcgtatatcgtagaatagttaagtctctttcgaacgatgatattaacaagatttccggagatatgaaagactctctgaaggaaatgagccttgaggagatttatagctacgagaaatacggagaattcattactcaggaaggaatttccttctacaatgatatatgtggcaaggtgaactcgttcatgaacttatactgtcagaaaaacaaagagaacaagaacctctataagctacagaaacttcataaacaaatcctgtgcatcgcggacacaagctatgaagttccgtacaagtttgaatcagatgaggaagtgtaccagtcagttaatggcttcctagataacatatcatcgaagcatatcgtggaacggctccggaagattggtgataattataatggatacaacttggataagatctatatagtaagcaaattctacgagtcagtttctcagaagacgtatcgtgactgggaaacaatcaacacagcactggagattcattacaacaacatcttgccagggaacggtaagtcgaaagctgataaggttaagaaagcagttaagaacgatctgcagaagtccataacagagataaatgagctagttagcaattacaagttgtgctcagatgataatataaaggcagaaacctacattcacgaaatttcacatatcttgaataactttgaggctcaagagctcaagtacaatccagaaatccatctagttgagtctgaactgaaagctagtgagttaaagaatgtattggacgttattatgaacgcgtttcactggtgttccgtctttatgacagaagagcttgttgataaagacaataacttctacgctgagttagaagagatttatgacgaaatttaccctgttatatcgctgtataacctagtaagaaactatgttactcagaagccgtatagcaccaagaaaatcaagctaaactttggtataccaactctcgccgatggatggtccaagagcaaggaatattcaaataatgccattattctgatgagagacaatctttattatctgggaatctttaatgcaaagaataagccagataaaaagataattgaaggcaataccagtgagaataagggtgattacaagaagatgatctataatttactcccaggtcctaataagatgattcctaaggtgttccttagtagtaagacaggagttgaaacctataagccaagtgcttatatcttggagggttacaaacagaataagcatattaaatccagcaaggatttcgatataacattctgccacgaccttatcgattactttaagaattgtatagctatccatccagaatggaagaactttgggtttgacttctctgataccagtacttatgaggatatttccggattctatagagaagttgagctgcaagggtataagatagattggacgtatatcagtgagaaagacattgatttgctccaagagaagggacagctgtacttatttcagatttataataaagacttcagcaagaaatcaactgggaacgataaccttcacactatgtacttgaagaacctattctcagaggagaaccttaaagacatagttctgaaactcaacggagaggctgagatcttcttccgtaaatcttccatcaagaatccgataatccacaagaagggaagtatcttagttaacagaacttacgaagctgaggagaaagatcaatttgggaacatccaaatcgtgaggaagaatatccctgagaatatctaccaagaattgtacaagtactttaacgacaagagcgataaggaactctcagatgaagcggctaaattgaagaatgttgttgggcaccatgaggcagccactaacatagttaaggactacagatacacttatgataaatacttcctacatatgcctattacgataaacttcaaggctaataagactggattcattaacgatcgtatattacagtacatagccaaagagaaagatttgcacgtaatcgggatcgatcgaggagaacgaaatctaatctacgtttctgtgatcgatacatgtggtaacattgttgagcagaaatcattcaacatcgtgaatggatatgattaccaaataaagctgaagcagcaggaaggagctcgacaaattgccagaaaggagtggaaggaaatcggaaagataaaggagatcaaggaaggttatctatctctcgtaattcatgagataagcaagatggttattaagtacaacgcaattatcgctatggaggacctgtcatatggattcaagaaaggacgtttcaaggtagaacgacaagtgtatcagaagttcgaaaccatgcttatcaacaagcttaactacctggtcttcaaagacatctcaatcacggagaatggtggactgcttaaaggctaccaacttacttatatccctgacaagctgaagaacgtgggacatcaatgcggttgtatattctatgttcctgcggcgtatacatcaaagatcgaccctactacaggatttgtaaatatcttcaagttcaaagatctcactgttgacgcaaagcgtgaattcatcaagaaatttgattcaatacgatacgattcagagaagaacttgttctgtttcacatttgattacaacaacttcataacccagaatactgtgatgtccaagagcagttggtccgtgtacacttacggtgtgagaattaagaggaggttcgttaatggaagattcagtaatgagtctgataccatagatatcacgaaagatatggagaagacattggagatgacggacatcaattggcgggatggacacgatcttcgacaagatattatcgattacgaaatcgtacaacatatatttgagatctttcggcttacagttcaaatgagaaactcattgtctgagcttgaagatcgtgactatgatagactcatttcgccggtactaaatgagaataatattttctacgactccgctaaagctggtgatgcattacctaaagatgccgatgctaatggagcgtactgtatcgccttgaagggattgtatgagattaagcaaatcaccgagaattggaaggaagatggaaagttctctagagataaattgaagatatccaacaaagattggtttgactttatccagaacaaacgatatttgtaa

SEQ ID NO: 230 - DNA, 3792 bp, Artificial Sequence
  Description of Artificial Sequence: Synthetic polynucleotide
atgaacaacggtacaaataatttccagaatttcatcggtatctccagtttacagaagaccttgcgtaacgctctaatcccgacagaaacaactcaacaattcattgtgaagaatggaattataaaggaggatgaacttagaggtgagaatagacagatattgaaggacataatggacgactactatcgcgggttcatatcagagactctgagtagcattgacgatattgattggacctcactcttcgagaagatggaaattcaattgaagaacggcgataataaggatactctgatcaaagaacaaactgaataccgtaaggctattcacaagaaatttgctaatgacgatagatttaagaatatgttctctgctaaattgatctcagatattctcccggaatttgttatccacaataataattactctgcatctgagaaagaggagaagactcaagtcattaagctcttctcacgcttcgccacttcgttcaaggattactttaagaaccgtgctaactgcttctcagcagatgatatatcttctagctcttgccatagaatagtaaatgataacgcagaaattttcttttctaatgcgctcgtatatcgacgaatagtgaagtctctttcgaacgacgatattaacaagatatccggagatatgaaagacagtctcaaagagatgtctcttgaagagatttatagttacgagaaatacggagaatttattacgcaagaagggatcagtttctataacgatatctgtggtaaggtgaattcgttcatgaatctatactgtcagaaaaataaagagaacaagaacctctacaaacttcagaagcttcataagcagatactttgtattgcagatacgagctatgaggttccatacaagttcgaatccgatgaagaggtctatcagagtgttaatggcttccttgacaatatctcttctaaacacatcgtagaaagacttcgaaagatcggagacaactacaatggctataacctggataagatctacattgtgtccaaattctacgagagtgtttctcagaagacttatcgcgattgggaaacaattaacaccgcattggagattcactacaacaacatattacctggaaacggtaaatctaaggctgataaagttaagaaggcagtgaagaacgatcttcagaagtctattactgagatcaatgagctagtgagcaactacaaattgtgcagcgatgacaacatcaaagctgagacttacatccacgaaatatctcacattcttaacaactttgaagcacaagaacttaagtacaatccagagattcatcttgtggagagcgaattgaaggcaagtgaacttaagaatgtgctcgatgttattatgaacgcgtttcactggtgctccgtgtttatgactgaggagttggtagataaggataataatttctacgcagagttggaggaaatttacgatgagatttaccctgtgataagcttgtataacctggttcgtaactacgtgactcagaaaccatacagcaccaaaaagattaagctaaatttcggaataccgaccctcgctgacggatggtctaaatctaaagaatattctaataatgcgataatactcatgcgggataacctctattacttgggaatctttaacgcaaagaataagccagataagaagataattgagggtaatacttcagagaacaaaggagattacaagaagatgatttataacttgcttcctggacctaacaagatgatacctaaggtgttcttgagtagtaagaccggtgtagagacgtacaaacccagtgcttatatattggagggttacaaacagaacaaacacatcaagagttctaaggacttcgatatcactttctgtcatgatctcatcgattactttaagaactgcatcgcaatacatccagaatggaagaatttcggatttgacttctctgatacttctacatacgaggatatttctggattctacagggaagttgagttgcagggatacaagatcgactggacctacatctcggagaaggacatcgatctcttacaagagaaagggcaactctatctgtttcaaatatataataaggatttctcaaagaaatctacaggtaacgacaacttacatacaatgtatcttaagaacctattctccgaggagaacctcaaagacatagtgttgaagctaaatggtgaggcagaaattttcttccggaagtcttctattaagaatccgataattcacaagaagggtagcatcttagttaaccggacttatgaagctgaagagaaggatcagttcggtaacattcagattgtccggaagaatataccggagaatatttatcaagagctatataaatacttcaatgataagtctgataaagaactctcagatgaagctgctaagttaaagaacgtagttggtcatcatgaagctgctactaatattgtgaaagattatagatatacctacgataaatacttcttgcatatgccaattacgataaactttaaggcaaataagacagggtttattaacgatagaatactccaatatattgccaaggagaaggatttgcacgttatcggtattgatcgcggtgaaaggaatcttatatacgtgtcggtgatcgatacttgtggaaatatagtagagcagaaatcattcaacatcgtgaacggatacgactatcaaattaagcttaagcagcaagagggtgctcggcaaatagctagaaaggaatggaaagagattggtaagatcaaagagatcaaagaaggatatctctctctggtcatacatgagatatcaaagatggttattaagtacaatgccattattgctatggaggatttatcctatgggttcaagaaaggtcgatttaaggtggagaggcaggtttaccagaagttcgagaccatgctaatcaataaacttaactacttggtgttcaaagatatcagtatcacagagaatggaggcctattgaagggttatcaactcacgtatattcctgacaaactcaagaacgtaggccatcagtgtggttgtatcttttacgttccggcagcttacacatcgaagattgatcccactacagggttcgtaaatatcttcaaattcaaagatcttactgtcgacgccaagagagagtttattaagaagtttgactctattcgttatgattccgagaagaacctattctgcttcacattcgattacaacaactttatcacacagaacaccgtcatgagtaagtcaagttggtcagtttacacgtacggtgttagaatcaagagaaggttcgtcaatgggaggttctcaaacgagtcagatacaatagatattactaaggacatggagaagacattagaaatgacagacatcaactggagagatggacatgatttacgtcaggatattatagattatgaaattgttcaacatatattcgaaatattcaggctgactgttcaaatgagaaatagcctgtcagaactagaagatcgagattacgacagactcattagcccggtactcaacgagaataatatattctacgattctgctaaagctggagatgctcttccgaaagatgctgatgctaatggtgcatactgcatagctctgaaaggattgtacgaaatcaagcaaatcactgagaactggaaggaagacggtaaattctctcgtgacaagctaaagatttcgaacaaagattggtttgatttcatccagaacaaacgatacctgtaa

SEQ ID NO: 231 - DNA, 3792 bp, Artificial Sequence
  Description of Artificial Sequence: Synthetic polynucleotide
atgaacaatggcactaacaacttccagaatttcatagggatctcttctcttcagaagactcttcggaacgcactaatacctactgaaacaactcaacagtttatcgttaagaacggtataatcaaagaagacgaattgcgtggtgagaatcgtcaaatccttaaggatatcatggatgactattatcgaggattcatctccgagacactttcctcaatcgatgatatagattggacatccctcttcgagaagatggaaatccagttaaagaacggagataacaaagatacgttgatcaaggagcaaactgaatatcgtaaagctatacataagaagtttgctaacgatgatagattcaagaatatgtttagtgctaaactcatttccgatatattgcctgagttcgtaatacataataataactatagtgcttccgagaaagaagagaaaactcaggtgatcaaacttttctcccggttcgctacttctttcaaagattattttaagaatagagcaaactgcttcagcgctgacgatatcagttcgtcttcatgccacagaattgtaaatgataatgcggagattttcttttcaaacgcattagtatataggagaatcgttaaatccctgagtaatgatgatatcaacaagattagcggcgatatgaaagattcactaaaggagatgtctcttgaagagatctatagttacgagaaatacggcgaatttatcacacaggagggaatcagtttctataacgatatatgcggcaaggtcaactcattcatgaacctgtactgtcagaagaacaaagagaataagaatctttataagctgcagaagcttcataaacaaattctctgcattgctgacactagttatgaggttccctataaatttgagtccgatgaagaggtttatcaatcggttaacggattccttgataacatttcatccaaacatatagtggagaggctcagaaagatcggtgataactataacggttataaccttgacaagatatatatagtgtccaagttctacgaatctgtttcacagaagacttacagagattgggaaacgataaacacagcgctggaaattcattataacaacatacttccaggcaatgggaaatctaaggcggataaggttaagaaagctgtcaagaatgatctacagaagtctattacagaaatcaatgaacttgttagtaattataagctttgcagcgacgataatattaaggcagagacgtatatacacgaaatcagtcatatactgaataactttgaggcacaagaactcaaatacaatcccgagattcatcttgttgaatcagaattgaaggctagcgagttgaagaatgtgcttgatgttatcatgaacgcgttccattggtgctctgtgtttatgacagaagaactagtcgataaagacaataatttctatgccgaacttgaagagatttatgatgaaatataccctgttatcagtctgtacaaccttgtgcgtaattacgttactcagaaaccatattccacaaagaagatcaagcttaatttcggtattccaactttagcagatggttggtctaaatccaaagaatatagcaacaatgctattatacttatgcgtgacaacctctattaccttggtatcttcaatgcaaagaataaaccggataagaagataatcgaaggtaatacgtctgagaacaaaggagattacaagaaaatgatttataacttgcttcctggccctaataagatgattcctaaagtgttcttgtcatctaagactggagtcgagacctacaaaccttctgcgtatatacttgagggctataagcagaataagcacatcaagagctcgaaagactttgatattacattctgtcacgaccttatagattacttcaagaattgcattgctattcatccagagtggaagaatttcggattcgatttctcagatacgtctacatacgaggatattagtggattctatagagaggtcgagcttcaaggatataagatcgattggacctacatatcggagaaggatattgatttgctccaagagaaaggtcagttatacctatttcaaatttacaataaggacttctcaaagaagagcacgggcaatgataatcttcatacgatgtatctaaagaacctcttctccgaggagaatcttaaagatattgttcttaaattgaatggagaggctgaaatctttttccgcaagagtagtattaagaatcctataatccacaagaagggctcaattctagtgaacaggacatacgaggcggaggagaaggaccaattcggaaatatacagatcgtacgtaagaacattcccgagaatatttaccaggagctttacaagtactttaatgataaatcagataaggaattgtctgacgaggctgctaaacttaagaatgttgtgggacatcacgaagcggctactaacatcgttaaagattatcgttacacctatgataaatacttccttcatatgccgattaccattaatttcaaggcgaacaagactggattcatcaatgataggatactgcaatatattgctaaggagaaagatctccatgttattggtattgatcgtggtgaacgcaatttaatttatgtcagcgttattgacacctgtggtaacattgtcgaacagaaatcatttaatatcgtcaacggatatgattaccaaatcaagctcaaacaacaagaaggagctagacagattgccaggaaggaatggaaggagattggcaagattaaggagattaaggagggttacttaagccttgtgatacatgaaatatctaagatggtcatcaagtataatgcgattattgccatggaggatctcagctacggatttaagaaaggacgatttaaggtagagcgtcaggtttaccagaaatttgaaacaatgctgataaataagcttaattatttagtgtttaaggacatttcaatcactgagaacggaggtttattgaaaggctatcagctcacttatattccggataaactcaagaatgtaggacaccagtgtgggtgtatcttctatgtgcccgcggcttatacctccaagattgatccaaccacagggttcgttaacatcttcaagttcaaagatctgactgttgatgccaagagggaattcataaagaagtttgacagtatcaggtacgattctgagaaaaacctcttctgctttacatttgactacaacaatttcattacccagaatacagtgatgtcaaagagctcttggtcagtttatacatacggtgtaagaattaagcgccggtttgttaacggaagattctctaacgagagtgacactatcgatatcacgaaggatatggagaagactttggaaatgacagacattaattggcgggacggtcacgatctaaggcaagacatcatagactacgaaatagttcaacatatattcgagatctttaggctaaccgtgcaaatgagaaattcattgtctgagctggaagatcgggattatgaccgtttgatctctcccgttctaaatgagaataacatcttctatgattcagctaaagctggagatgcacttccgaaagatgctgacgcaaatggtgcttattgcattgctctcaagggcttgtacgaaataaagcaaattactgagaattggaaagaggatggcaagttctccagggataaactgaagatatccaacaaagattggttcgactttatacagaacaagcgctatttgtaa

SEQ ID NO: 232 - DNA, 3792 bp, Artificial Sequence
  Description of Artificial Sequence: Synthetic polynucleotide
atgaacaatggcactaataatttccagaacttcattggaatctcttctctccaaaagacacttagaaatgctttaattccaacggaaacgactcaacaattcatcgtaaagaacggaattattaaggaagatgagttgagaggtgagaacaggcagattctaaaggatatcatggatgattattacagaggtttcatctctgaaacgctgtcttcaatagatgacatcgattggacgagtctatttgagaaaatggagatacagctcaagaatggtgataacaaggatactctaatcaaggaacagaccgagtatcgtaaggctatacacaagaagttcgcaaacgatgatagatttaagaacatgtttagcgcgaaactgatttccgatattctgccggagttcgtcattcataacaacaactattccgcttcagagaaggaagagaaaacgcaagtgattaagttattctctagattcgccacgagcttcaaagattattttaagaaccgagcaaactgcttctctgcagatgacattagttcttcgtcttgccaccgtattgtaaatgacaatgcagagatattcttcagcaacgctctagtatatcgtcgaatagttaagtccttgtcaaacgatgacattaataagatcagcggtgatatgaaagattcattgaaagaaatgagtttggaagaaatctattcatatgagaagtacggagaattcattactcaagagggaatctccttctataacgacatctgcggcaaagtaaatagctttatgaatttgtattgtcagaagaacaaagagaataagaatctatataaattgcagaaacttcacaagcaaatcttgtgtattgcagatacaagttacgaagtaccgtacaaattcgaatcagatgaggaggtttatcagtctgtcaatggcttcttagacaacattagctctaagcatattgtcgagaggttgcgcaagattggagataattacaatggatataacctcgataagatctatattgttagtaagttctacgagagtgtatcgcagaagacgtatagagattgggagacaatcaatacggctttggaaatccactacaacaacatcttaccagggaatgggaagtctaaggcagacaaagtgaagaaagctgtaaagaacgacttacagaagtcaatcacggaaataaacgagctcgtatccaactataaattatgcagtgacgataatattaaagccgaaacatatatccatgaaataagtcatattcttaacaactttgaagctcaagagctgaagtataacccggaaatccaccttgtcgagtcggagttaaaggctagtgagctcaagaacgtgctcgatgtgattatgaatgccttccattggtgtagtgtgtttatgacagaggaattagtcgataaggataataacttctacgccgaactagaagagatatatgatgaaatttacccagttatctctttatacaacctagttcgaaattacgttacgcagaaaccatactcgacgaagaagattaagttaaacttcggtataccgacacttgctgacggatggtcaaagagcaaggaatattcgaataatgcaatcatcttgatgcgtgataatctctattatctcgggatctttaatgctaagaacaagccagataagaaaattatagagggaaatactagtgagaacaaaggcgattacaaaaagatgatatacaacttgctccctggacctaataagatgattccgaaggtatttctttcttccaagactggtgttgagacatacaagcccagcgcttacatccttgaaggttataaacagaacaaacatatcaagtcgtctaaggatttcgacataacgttctgtcatgacttaatcgattacttcaagaactgcatagcaattcatcctgagtggaagaatttcggatttgatttctctgatacttctacgtatgaagatatatccggcttctatcgggaagttgaattgcaagggtataagattgattggacctacatctcagagaaagacattgatttgctccaggagaagggccaattatatttgttccagatttataataaagatttctctaagaagtcaaccggcaatgataatcttcacacaatgtatctcaagaacttatttagcgaagagaacctaaaggatatagtgcttaagcttaatggagaagctgagatctttttcaggaaatcctcaataaagaatccaatcattcacaagaaaggaagcatcttagtgaatcgaacatacgaagcagaggagaaagatcaatttggtaatattcaaatcgttagaaagaacatcccagagaatatttaccaagaattgtacaagtacttcaacgataagtctgataaagaactttcagatgaggccgcgaagctcaagaacgttgtaggtcatcatgaagcagctactaatatcgtgaaagattacagatatacctacgataagtatttcttgcatatgccgataacaatcaacttcaaagcaaacaagacaggtttcattaacgataggatactccagtacatcgccaaggagaaggatttacatgtaatcgggattgatcggggggaacggaaccttatatacgtttctgtgatagacacttgtggtaatatcgttgagcagaagagctttaatatagttaatgggtatgactatcagattaaactcaaacaacaagagggcgctagacagatcgcgagaaaggaatggaaagaaatcggtaagattaaagaaattaaagaaggctatttgtctctcgtcatacatgaaatatccaagatggtgatcaagtataatgctatcattgccatggaagacctcagttacggatttaagaagggaaggttcaaggttgaaagacaggtttaccagaagtttgaaactatgcttattaataagttgaactacttagtgttcaaagatatttcaattacagagaatggagggctccttaaaggttaccaattgacttacatcccggacaaactgaagaacgttggccatcagtgcggatgcattttctatgttccagcagcatatacaagcaagatagatccgacaaccggcttcgtgaacatatttaagttcaaagacttaacggttgacgccaaacgtgaatttataaagaaatttgatagcataagatatgattcagagaaaaacttgttctgcttcactttcgattataacaacttcataactcagaacacagtgatgagcaagagcagctggtctgtctatacttatggtgttagaattaagaggcgattcgtgaacggtagatttagtaatgagtctgatacaatcgatatcacgaaggatatggagaagacattggagatgacggatataaattggcgtgatggtcatgatctaaggcaggacataatagattacgagattgttcagcacatctttgagatatttagacttaccgttcaaatgcggaactctttatctgaactggaagatagagattacgatagactcatctcgcctgttctgaacgagaataacatattctatgactctgccaaggcaggagacgcacttcctaaggatgcagatgcaaacggagcctattgtatagcactcaagggactctacgagatcaagcaaattactgagaattggaaagaagatggaaagttctcgagagacaagttaaagatttcgaataaggattggtttgatttcattcagaacaagcgttatctttga

SEQ ID NO: 233 - DNA, 3792 bp, Artificial Sequence
  Description of Artificial Sequence: Synthetic polynucleotide
atgaacaatggaacgaataacttccagaacttcataggaatatcctctttgcagaaaacattaaggaatgcacttattcctacagaaactacccaacaatttatcgtcaagaatggaatcattaaagaggatgaactccgtggagagaataggcaaattctaaaggatatcatggacgattactatagagggttcatctcagaaaccctctcgtctatagatgatattgactggacaagcctcttcgagaagatggagatccagctgaagaatggtgataataaggacactctaatcaaggaacagaccgagtatcgcaaggctattcacaagaaatttgcgaacgatgatcggttcaagaatatgttctctgctaagttgatttcagatatcctcccggagttcgttattcataacaacaactattcggcttcggagaaggaggagaaaacacaggttatcaaactctttagcagatttgctactagtttcaaggactacttcaagaatagggcgaactgtttctctgcagatgacatttcgtcttcttcttgccataggattgtcaatgataacgcagagatatttttctcaaacgccctcgtatacagacggattgttaaatctttgtcaaacgacgacataaacaagataagtggtgatatgaaggattctctaaaggagatgtccttggaagaaatttatagttatgagaaatacggagaattcatcacccaagaaggaatatcgttctataacgatatatgcggtaaagtaaactcgtttatgaacctttattgtcagaaaaacaaagagaataagaatctttacaagcttcagaaactgcataaacaaatcctttgtattgctgatacttcttacgaggtaccgtataagttcgaaagcgatgaagaagtgtatcagtctgtaaatggctttctggataatatctcttctaaacacattgtggaacgtttgcgaaagataggagataattataatggatacaatctcgataagatttacattgtgtcaaagttctatgaaagtgtctctcaaaagacgtatcgagattgggagactattaatacagcattggagatccattacaataacatacttccaggaaacggcaagagtaaagctgataaggttaagaaagctgtaaagaacgatttgcaaaagagtattactgagatcaatgaactagtatccaactacaaactttgttcggacgacaatataaaggccgagacctatattcacgagatatcgcatattctcaacaactttgaggcccaagaattaaagtataatccagagattcacctggttgagtctgaactgaaggcaagcgaactgaagaatgtgttagacgtgattatgaacgccttccactggtgtagtgtgtttatgacagaagaacttgttgacaaggataataatttctatgctgagttggaagagatttacgatgaaatatatcctgttatctctctttacaatctcgttcgtaactacgtaacgcagaagccttattctacgaagaagattaaattgaatttcggaattcccacgctcgctgatggatggtcgaaatctaaggagtactccaataatgctataattctcatgagagataatctgtactatctaggaatattcaatgcaaagaacaagccagacaaaaagattatagaaggcaatacgtctgagaacaagggcgattacaaaaagatgatctataacctcctccctgggcccaacaagatgattccgaaagtattccttagttcaaagactggtgtagagacatataaaccgagtgcttacatcctcgaagggtataagcagaataagcacattaagagctcaaaggatttcgatatcactttctgtcacgatctcattgactactttaagaattgtattgctattcatcccgaatggaagaactttggtttcgacttctctgatacaagcacctacgaggacatatccggattctacagagaggttgagcttcagggatataagatagattggacttacataagtgagaaggatatcgatctcttgcaggagaaaggtcagttgtacttattccaaatttataacaaagacttctccaagaagtctaccgggaatgacaacctccatactatgtatctcaagaacttgtttagtgaggagaatcttaaggacattgtgttaaagcttaatggtgaggcagagatcttctttaggaaatcttctatcaagaaccctataatacacaagaaaggcagtatattagttaatcgtacatacgaagcggaagagaaagaccaattcggtaacatccagatcgtaagaaagaatattcctgagaatatataccaggaactctataagtacttcaacgataagagcgacaaggaattgtcagacgaggctgctaaattgaagaatgttgtgggtcatcacgaagctgcaactaacatcgtgaaagactaccgttacacatatgataaatactttctccatatgccgataacaattaacttcaaggcaaataagacaggcttcatcaatgatagaattctccaatatatagctaaggagaaagacttgcacgtaatcggaatagatcgaggtgaaaggaatctaatatatgtctctgtaatagatacatgtgggaacattgtagagcagaaatctttcaatatcgttaacggttacgattatcagatcaagctgaaacagcaagaaggtgctcggcagattgctcgtaaggagtggaaggagattggtaagatcaaggaaattaaagaaggttacctgtcactcgtaatacacgaaataagcaagatggtcatcaagtataacgcgattattgctatggaagatctctcgtatggcttcaagaaaggaagattcaaagtagagcgacaagtataccagaaattcgagactatgctaattaataaacttaattaccttgtgtttaaggatatttctattacagagaatggtgggttgttgaaagggtatcagcttacgtatatacctgataaactaaagaacgttggccatcaatgcggatgtatcttttacgttcctgctgcatacacgtctaagattgatcctaccactggtttcgtaaatatctttaaattcaaggatttgacagttgatgctaaacgggaattcattaagaaatttgatagcatccgttacgacagcgaaaagaatctgttttgcttcacctttgattataataatttcatcacgcagaatactgtaatgagtaaatcatcatggtccgtttacacttatggagtgagaattaaacgtaggttcgttaacgggaggtttagtaatgaaagcgacacaatcgatattaccaaggatatggagaagacgcttgaaatgactgatatcaattggagggatggtcatgatttgcgtcaagatattatagactatgaaatcgtgcaacacatctttgaaatatttaggctaactgttcaaatgagaaactcattatctgaattagaggacagagattacgaccggcttatttcacctgtcttaaatgagaataacatattttacgattcggctaaggctggcgacgctcttcctaaagatgctgatgccaatggtgcatattgtatcgcactgaagggactttacgaaataaagcagattactgagaactggaaggaggacggaaagttcagcagagataagcttaagatatcaaataaagattggttcgacttcatccagaacaagcgatacttgtga

SEQ ID NO: 234 - DNA, 3792 bp, Artificial Sequence
  Description of Artificial Sequence: Synthetic polynucleotide
atgaataacggaacgaataacttccagaatttcatcggtatttcgtccctgcagaaaacacttagaaatgctctcatcccaactgagactacgcagcagtttatagtgaagaacggcataattaaagaggatgagctaaggggcgagaatagacaaatcttgaaagacattatggatgactactaccgcggcttcatatctgagactctttcatctattgacgatatagactggaccagtttatttgagaagatggaaatacaactgaagaatggtgataataaggataccctgatcaaggagcaaactgaatacaggaaggctatccacaagaagtttgctaacgatgatagattcaagaatatgttctccgctaaattgatctctgatatactaccggaatttgtgatacataacaataactactcagcctcagagaaggaggagaaaactcaagttatcaagttgttctctcggtttgccacctcctttaaagactacttcaagaacagagctaactgtttctctgcagacgacatttcttccagtagttgccatcgaatcgtcaatgacaatgctgaaatattcttctctaacgcacttgtctacaggcgtatcgttaagagtttaagcaacgatgatatcaataagatttctggagatatgaaggattctcttaaagagatgagtcttgaagaaatctattcatatgagaagtatggtgagtttatcacccaggaagggatctcattctataacgatatttgtggcaaagtcaatagcttcatgaacttatattgtcaaaagaacaaggagaacaagaatttgtacaaacttcagaaacttcataaacaaatattgtgtattgctgatacctcctatgaggttccatacaagtttgaaagcgacgaggaagtgtatcaaagtgtgaacggattcttggacaatatttctagcaagcatattgttgaaagacttcgtaagataggagataattacaacggatacaacttagacaagatctatatcgtctctaagttctacgaatctgtgagtcaaaagacatacagggattgggaaacaataaataccgcacttgagatccattataacaatattctaccgggaaatggcaagagcaaagcggataaagttaagaaagctgtgaagaatgatctccagaaatctataacagagattaatgaattggtaagcaactacaaactttgttccgatgataacattaaagcggagacctacatccatgagatatctcatattcttaataactttgaggctcaagagcttaaatataatccggagattcatctagtagagtccgagctaaaggcatctgaacttaagaatgtcttggacgtcatcatgaacgcattccactggtgctctgtgtttatgacagaagagcttgtggataaagataacaatttctatgcggaactcgaggagatttacgatgagatctacccagtcatctctttgtataatttggtgcgaaattatgtgactcagaaaccgtattcaacaaagaagattaagttaaacttcggtattccaacattagcagacggctggtctaagtctaaagagtatagcaataatgccataatccttatgagagataatctgtattatttgggcatattcaacgctaagaacaaacctgataagaagattatcgaagggaacaccagtgagaacaagggtgattacaagaagatgatctataacttattacccggtcctaacaagatgattcccaaggtgtttctttcatctaagaccggtgtggaaacttataagccatctgcgtatattctcgagggatataaacagaataaacacattaagtctagtaaggatttcgatatcacattctgtcacgatttaattgattactttaagaactgcatcgccatccatcctgagtggaagaacttcggtttcgacttctcagatacgagcacctatgaagacatctctggcttctatcgtgaggttgagctccaaggttataagattgattggacatacatctcggagaaagatattgatttgctgcaggagaagggtcagttgtacctctttcaaatttataataaagatttctccaagaaatcaactggaaacgataaccttcacacaatgtacctaaagaatctattctctgaagagaatcttaaagacattgtcctgaaattgaatggtgaggcggaaatcttttttcgtaagagcagtatcaagaatcctattattcacaagaaaggatcgatcttggttaatagaacatatgaagcagaagagaaggatcagttcgggaatattcaaatcgttcgaaagaacatcccagagaacatatatcaagagctttacaaatacttcaacgataagtcagacaaggagttaagtgatgaggcagccaagcttaagaatgtagtcggacaccatgaagcagctaccaacatcgtgaaggattaccgctatacctatgataaatactttctccatatgcctatcaccattaatttcaaagcaaacaagacaggatttatcaatgataggatattgcagtatattgccaaggagaaagatttacacgttattgggattgatcggggtgaacgtaatttgatctacgttagcgttattgacacctgcggaaatatcgtcgagcagaagtcgtttaatatcgtcaacggatatgattaccagataaagctcaaacaacaggaaggtgctcgtcagatcgctcgtaaggagtggaaggaaattggcaagattaaagagatcaaggagggttacctcagcctcgttatccacgagatttcgaagatggtgataaagtacaatgcaatcattgctatggaggatctaagctatggattcaagaaaggaaggttcaaggttgagagacaagtttaccagaagttcgagactatgctcattaacaagctgaattacttggtatttaaggatatctctataactgagaatggcgggctgctgaaaggataccaactcacgtatatcccagacaaattgaagaatgtaggacaccagtgcggttgtatattctacgtgcctgccgcatatacttctaagattgatccaacaactggatttgtgaacatatttaaatttaaagatcttacagtcgacgcaaagagggagttcataaagaagttcgattctatccgttacgatagtgagaagaatttgttctgctttaccttcgattacaataacttcattacacagaacactgttatgtctaaatcaagttggagcgtatatacttacggagttagaatcaagcggcgatttgttaacgggagattctctaacgaaagcgatacaatcgatataactaaagacatggagaaaactttagaaatgacagatatcaattggagagacggacatgacttgagacaagatattatagattatgaaatagtgcagcacatcttcgagatcttccgcctgacagtgcaaatgaggaatagccttagtgaactagaagatagagattacgatcgtctcataagtccagtgctaaatgagaacaatatattctatgactctgcaaaggcaggtgatgctttacctaaggatgcagacgcgaatggagcctattgcatagcccttaaagggctttatgagattaagcagattacggagaactggaaggaagatggaaagttctccagagacaagctgaagatctctaataaagattggttcgacttcattcagaacaagagatatttatga

SEQ ID NO: 235 - DNA, 3792 bp, Artificial Sequence
  Description of Artificial Sequence: Synthetic polynucleotide
atgaacaacggtacgaataactttcagaacttcataggtatctccagtcttcaaaagactcttcgtaatgcgcttattcctactgaaactactcaacaatttatcgtgaagaatggcattattaaggaagacgagctaagaggagagaataggcagatacttaaggatataatggacgattactacagaggatttatctcagaaacactctcttctatcgacgatatagattggacttcgctgttcgagaagatggagattcagttgaagaacggagacaacaaagacactttgatcaaagaacagaccgaataccgtaaagcgatacacaagaagtttgccaatgatgaccgatttaagaatatgttctcagcgaagctgatttctgatattctcccagaatttgtaattcacaataataattactctgcatcggagaaggaggagaaaactcaagttatcaaattattctctcgtttcgctaccagtttcaaagattactttaagaatagagccaactgtttctcagctgatgacatttcttcatctagctgtcacagaatcgttaatgataatgctgagatctttttctctaacgcactagtgtataggaggatcgtcaaatccctgtcaaacgatgacatcaacaagatctctggtgacatgaaggactctttaaaggagatgagcttggaggagatctacagctatgagaaatacggtgaatttatcactcaggaaggaatatcgttctataacgacatctgtggcaaggtgaacagtttcatgaacctttattgtcagaagaacaaggagaataagaacttgtataagcttcagaagcttcacaaacaaatattatgcatagccgatacctcttatgaagtgccttacaagttcgaaagcgatgaggaggtttatcaatcagtgaacggctttctggacaatatctcctcgaagcatatcgttgaacgtttgagaaagattggcgataactataatggatacaatcttgataagatttatatagtgagcaagttctatgagtcggtgagccagaagacgtatcgagattgggagactatcaatactgccttggaaattcattataataacatcctgccaggaaacggtaagtccaaggcagataaagtcaagaaagcagttaagaatgacctacagaagtcaattacagaaattaatgagttggtgtccaactacaagctgtgcagcgacgacaatattaaagccgagacttacatacatgaaatctcccatatactcaacaatttcgaggcgcaagaattaaagtacaacccggaaatccatctggttgaatcagaactgaaagctagtgaactaaagaatgtacttgatgttatcatgaacgcatttcattggtgctctgtatttatgacagaggagcttgtagataaagataacaatttctatgctgaattggaggagatttatgacgagatctatccagtcatctctctgtataatttggttcgtaattacgtgactcagaagccatattcgactaagaagattaagttgaacttcggaatcccgaccttggcagatggttggtctaagtctaaggaatattccaacaatgcgattatcctcatgagagataacctttactatctgggaatatttaacgctaagaacaaaccggacaagaagattattgaaggtaatacctccgagaataaaggcgactataagaaaatgatttataacctcttaccagggcctaataagatgattccaaaggtgtttctctcaagtaagacaggtgtagaaacttacaaaccttctgcatatatcctggaaggttacaagcagaacaagcatatcaaatcctctaaggacttcgacattactttctgtcatgacttaattgactactttaagaattgtattgcaatccatccggaatggaagaacttcggatttgacttctctgacacatctacttacgaggatattagcggattctaccgtgaggttgagctgcaaggatataagatagactggacttatatttcagagaaagatattgatctgttgcaggagaagggtcagctctatctcttccaaatttacaataaggacttcagcaagaaatctaccggcaacgataatctacacaccatgtatctgaagaacctgttttcagaggagaacttaaaggatatagttcttaagcttaatggagaggctgagattttcttccgcaaatcatcaattaagaatcccattatacataagaagggctcaatcttggtgaatcggacctatgaagccgaggagaaggaccaattcggaaacatccaaatagttagaaagaacataccagagaacatttatcaggaactttataaatatttcaatgataagtccgataaagaactctcagatgaagctgccaaacttaagaatgtcgttggacaccatgaggctgccactaatatcgtgaaggactacaggtatacatacgacaagtacttcctgcacatgccgattacgattaacttcaaggcgaacaagactggattcatcaacgatagaatactgcagtatattgctaaggagaaggatcttcatgttattggaatcgatcgtggtgagcgaaatcttatatatgtctcagttatagacacatgcgggaatatcgtggaacagaaatcctttaatattgtaaatgggtatgactaccaaataaagttgaaacagcaggagggtgcgagacagattgctagaaaggagtggaaagagattgggaagatcaaggaaatcaaggaaggttacctaagcctcgttatacacgagatttccaagatggtaataaagtacaatgcaataattgctatggaggatctttcttatgggttcaagaaaggtaggttcaaagtagaacgtcaagtctaccagaaatttgaaacgatgctcatcaacaaacttaattacttggtatttaaggatatcagtataacagagaacggtgggctcttgaaagggtaccagttgacatatattccggacaagctaaagaacgtgggacatcagtgtgggtgcatcttctacgttcctgctgcatatacaagcaagattgatccaacgacaggatttgtgaacatatttaagtttaaagatttgacagtggatgcgaagagagagtttatcaagaagtttgattctattagatatgactcggaaaagaatctgttttgtttcaccttcgattacaataatttcattactcagaatactgtgatgtcaaagagctcatggtcggtctatacatacggagtgagaatcaaacggagatttgttaacgggagattcagtaatgagtccgacacgattgatattactaaggacatggagaagactctagaaatgacggatatcaattggcgtgatgggcatgatctaagacaagatatcatagactatgaaatcgtgcagcatatcttcgaaatattcaggcttactgttcaaatgcggaattctttaagcgagttggaggaccgggactatgacaggcttatttcaccagttctgaacgagaacaacatcttctacgattctgctaaagccggagatgctctgcctaaggatgcggatgctaatggagcttactgcatcgctctcaaaggactttacgagatcaagcaaattaccgagaattggaaggaagatgggaaattctcacgagataaactcaagatatcgaacaaggattggtttgactttatacagaacaaacgttatctttga

SEQ ID NO: 236 - DNA, 3792 bp, Artificial Sequence
  Description of Artificial Sequence: Synthetic polynucleotide
atgaataatgggaccaataacttccagaattttattggtatttcctctttgcagaagaccctaagaaacgcgctgatcccaactgagacgacacagcaattcatcgttaagaacggaattattaaagaggatgaacttcgcggagagaaccgccagatactgaaggatattatggatgactactatcgtggtttcatatccgagactttgtcttctatagacgatatcgattggacttctttatttgagaaaatggagattcaacttaagaatggcgataataaggacacattaatcaaggaacaaactgagtacagaaaggcaattcataagaagtttgcaaacgacgacagattcaagaatatgttctcagcgaaactgatctcagatattcttccggagttcgttatacataataacaattactcggcatctgagaaggaggagaagactcaagttattaaactcttcagcaggttcgcaacaagcttcaaggattattttaagaatagggcaaattgtttctcagctgatgatatttcgtcatccagttgccacagaatcgtgaatgacaacgctgaaatctttttctctaacgctcttgtttataggcgcattgtgaagtcgttatctaatgatgatattaacaagatctctggcgacatgaaagactcattgaaagagatgtctttagaggaaatttattcctacgagaagtatggagagttcattacgcaggagggaatatcgttctacaacgatatctgcggcaaggtcaatagctttatgaacttgtactgccagaagaacaaagagaacaagaatctttataagcttcagaaactacataaacagattctatgcatagccgacacttcctatgaggtaccttataagtttgaaagtgacgaggaagtttatcaaagtgtgaacggatttctggataatatttcttctaagcacattgtggagagattgcgaaagatcggagataattacaatggctacaaccttgataagatttacattgttagcaaattctacgaatccgtttcacagaaaacttaccgggactgggagactattaacacagctttggagatacattacaataatatcctacctggtaacggtaaaagcaaggcagacaaggttaagaaagccgtgaagaatgatttgcagaaatctatcaccgaaatcaacgagcttgtgtctaactacaaactttgtagcgacgataatatcaaggcagagacttacatacatgagatttctcacatattaaacaacttcgaagctcaagaacttaagtacaacccggagatccacttggttgagagcgaattgaaagctagtgaactaaagaatgtgcttgatgtgattatgaacgcgtttcattggtgctctgtgtttatgaccgaggagttagttgacaaagataacaatttctacgccgagcttgaagaaatttacgatgaaatctacccagtcatcagcctttacaacctagtaagaaattacgttacacagaaaccatatagtactaagaagattaagctcaacttcggaatacctactctcgctgatgggtggtctaaatcaaaggaatacagtaataacgcaataatcttgatgcgggacaatctatactacttaggaatattcaacgcgaagaataagcctgacaagaagattattgagggcaatacgtcagagaacaagggagattataagaagatgatttacaacttgctgcctggacctaataagatgattcctaaagtctttttatcatcgaagactggtgttgagacatataaaccctccgcttatattctcgagggctataaacagaataaacacatcaagtcatccaaggactttgatattacgttctgtcatgatttgatagattacttcaagaactgtatcgcgattcacccggagtggaagaatttcgggtttgatttcagtgatacatcgacatacgaagatatttccgggttctacagggaggttgagttacaaggatacaagatagattggacgtacatatctgagaaggatatagacctcctacaagagaaaggccagctctatctctttcagatttacaataaagacttctcgaagaagtctactggcaacgataatcttcatacaatgtatttaaagaatctattcagtgaagagaatctcaaagacatcgtgctgaaattgaatggagaagctgaaatattcttccgaaagtcatcgatcaagaaccctataatccacaagaagggttcaatactggtgaatcgcacatatgaggctgaagagaaggaccaatttggtaacattcagatcgttcggaagaatattcctgagaacatctaccaagaactttataagtactttaacgataaatctgataaagaattatccgacgaggctgctaagctaaagaacgttgtgggccatcatgaggcggctactaatattgtgaaggattataggtacacatatgacaagtacttcttacacatgccaatcaccataaactttaaggccaacaagactggatttattaatgatagaatcttgcaatatatcgctaaagagaaggacttacacgttattgggattgatcgtggagaaagaaatttgatttacgtttcagtcattgatacatgtggaaatattgttgagcagaaaagtttcaacatcgtgaatggttacgattatcaaataaagcttaagcagcaggagggagctaggcagattgctcgtaaggagtggaaagaaatcggcaagataaaggagatcaaagagggttacttgagtttggtaattcacgagatttcaaagatggtcattaaatataatgctataatagctatggaagatctttcatatggatttaagaaaggacggttcaaagtagaaagacaagtgtaccagaagtttgaaaccatgctcattaacaagctgaattatttggtgtttaaagacatctctattaccgagaatggcggacttctgaaaggataccagttgacttatataccagataaacttaagaacgtgggtcaccagtgcggttgtatcttctacgtgcctgctgcctatacgagtaagatcgatcctaccacaggcttcgtgaacatcttcaagtttaaggatcttacagttgatgctaagagggagttcattaagaaatttgatagcatacgatacgactctgagaaaaatttgttctgtttcacgttcgattacaataatttcataacacagaacactgtgatgtccaagagctcctggagtgtttacacctatggagtaaggatcaaacggagattcgtaaatgggcggtttagtaatgaaagtgatacaatcgatattactaaggatatggaaaagacactagagatgactgatatcaattggagagatggtcacgatcttagacaagatataatagattatgagatagtacagcatatattcgagatcttccggttgaccgttcaaatgaggaatagcctgagcgaactcgaggatagggactatgacagacttatttctccagtccttaacgagaataacatcttctatgactcagcgaaggcaggtgacgcacttccgaaagacgcggacgccaacggagcctactgcattgcactcaaaggtctgtacgagattaagcagattactgagaactggaaagaagatgggaaattctctcgagacaaactcaagatttccaataaagactggtttgatttcattcagaacaaacgctacctgtga

SEQ ID NO: 237 - DNA, 3792 bp, Artificial Sequence
  Description of Artificial Sequence: Synthetic polynucleotide
atgaacaacggtactaacaacttccagaatttcatcggtattagttcattgcagaagactcttagaaacgcactaattcccaccgaaacaacccaacagttcatagtcaagaacggtataattaaggaagatgagctaagaggtgagaatagacaaatcttgaaggatatcatggatgactattatagaggctttataagtgagacgctatcttctattgatgacattgactggaccagtttgtttgagaagatggagatacaattgaagaacggtgataataaagacaccctcattaaggagcagaccgaataccgtaaggcaatccacaagaagtttgcgaacgatgataggtttaagaacatgttctctgccaagttgatcagtgacatacttccagagtttgttatccacaataacaattattcggcttctgagaaagaggagaaaacccaagtcattaagttattctcaaggtttgctacctcattcaaagattactttaagaatcgtgctaactgtttctcagctgatgacatctcgagctcatcttgtcaccgaatagtgaacgataacgcggaaatatttttctcgaacgcactggtttatagacggatcgtgaaatccttgagtaatgatgatatcaataagattagtggagatatgaaagatagcctgaaagagatgtctcttgaggaaatttattcctacgagaagtacggtgagttcataacccaggagggaataagcttctacaacgatatttgtggtaaagttaactcatttatgaacctctattgtcagaagaataaggagaataagaatttgtacaagttacagaagcttcataaacaaatcttgtgcatagctgatacttcctacgaggttccttacaaatttgagagcgacgaggaggtatatcaatcagtaaatggattccttgataatatatcctctaagcacattgttgagagacttcgaaagattggtgataattataatggatataacctggataagatttatatcgtttccaagttctacgagtcagtttctcagaaaacttatcgtgattgggaaactattaacactgctttggagatccattataacaatatattgcccggcaatggtaagtcaaaggcagataaggttaagaaagcagtgaagaatgatttacagaaatccatcacggagataaatgagcttgtgtctaattataaactttgttcagatgataatatcaaagctgagacttacatacatgagatctcccacatacttaacaacttcgaagcccaagagctaaagtacaatccagaaattcatctcgtagagagcgaattgaaagcctcggagctcaagaacgtccttgatgtcataatgaacgccttccactggtgctctgtcttcatgacagaagaactcgttgacaaggataacaacttctacgcagagttagaggagatctatgatgaaatttacccagtgatctccttatacaacttggttaggaattacgttacacagaaaccttattcaacgaaaaagatcaagctaaacttcggaatccctactttagcagatggatggtcaaagagtaaggagtacagcaataacgcgattatcctgatgcgtgacaatttgtattacctcgggatctttaatgctaagaataagcctgacaagaaaataatcgaaggtaatacgagtgagaacaaaggtgactataagaagatgatttacaatctcttgccgggtcctaataagatgattcctaaggtcttcctcagtagtaagactggagtggagacttataagccatccgcatatattcttgaaggctataagcagaataaacacatcaagtcttccaaagatttcgacattacgttctgccatgatcttattgattattttaagaactgtattgctattcacccagagtggaagaacttcggatttgacttcagtgatacttcaacttacgaagatatctctggattctacagagaagttgagctacagggttataagatagattggacctatatatcagagaaagatattgatttactgcaggagaagggacaactctatctgttccagatctataacaaagacttcagcaagaaatcaacgggaaatgataatctacatacaatgtacttaaagaatctattttctgaggagaacttgaaggacatagtgttgaaacttaacggagaggcagaaattttcttcaggaagtcgtcgataaagaatccgatcatacacaagaaagggtctattcttgtgaaccgtacgtacgaagcagaagagaaagaccaattcggaaacatccaaattgtccgcaagaatataccggagaatatctaccaagaactttacaaatactttaatgataaatcagataaagaactatctgatgaagcggctaaattaaagaatgtagttggtcaccatgaggctgcaacgaatatagttaaagattatcgttacacatatgataaatactttctccatatgccaattactattaacttcaaggctaataagacagggtttatcaacgatagaattctccaatacatagctaaggagaaagacttgcacgtcattgggatcgatagaggagaacggaatttaatatatgtttctgtgattgacacttgcggcaacattgtggaacagaaatctttcaatatcgtcaatggatacgactaccagatcaaacttaagcaacaggagggtgccagacaaattgctcggaaagaatggaaggagataggaaagattaaggaaatcaaggagggataccttagtttagtcattcatgagattagtaagatggttatcaaatacaatgctattatcgcaatggaagatctttcttatggatttaagaagggaaggttcaaggtcgagcgacaagtctatcagaagttcgagaccatgttaattaacaagctaaactatctcgtgtttaaggatatcagtattacagagaatggtggacttcttaaaggctaccaacttacctatatacctgacaaacttaagaacgtcggccatcagtgtggttgtatattctacgttcctgcagcatatacatctaagatcgatccgactaccgggttcgtcaatatctttaagttcaaagatctcactgttgatgcgaagcgggagttcataaagaaatttgattctattcgatatgattctgagaagaatttgttctgtttcacatttgactacaataactttataacccagaataccgttatgtcaaagagtagctggtctgtttacacgtacggtgtgaggatcaagagacggtttgtgaacggaagattctctaatgagtcagatactatagatataactaaggatatggaaaagacattggagatgacagatatcaattggagagacgggcatgaccttagacaagacattatcgattatgagattgttcagcacatcttcgagatattcagactgacagtgcaaatgaggaattcattgagtgaactagaagatcgagactatgacagacttatttctccagttctcaatgagaacaatatcttctatgactctgctaaagctggagatgcgcttcctaaagatgcggacgctaatggagcctactgtattgctctcaaaggcctttacgagataaagcaaattacggagaattggaaggaagacggtaaattcagtcgtgataaattgaagatctccaataaggattggtttgacttcatccagaacaagagatacctttga

SEQ ID NO: 238 - DNA, 3792 bp, Artificial Sequence
  Description of Artificial Sequence: Synthetic polynucleotide
atgaataacggtacaaataatttccagaattttattggaattagttctctgcaaaagaccttgcgtaatgcacttataccaacagaaacaacccaacaattcattgtcaagaatggtataatcaaagaggatgagctaagaggagagaatagacaaattctaaaggatatcatggacgactactaccgtggttttatctcagagaccttgtcctctatcgacgacatagattggacatctttgttcgagaagatggagattcagttgaagaatggcgataacaaagatacgcttataaaggaacaaacggagtataggaaggccatacataagaaatttgctaatgatgatagatttaagaatatgttctctgcaaagcttatttccgatattcttccagaatttgtcattcataacaataattattccgcatcggagaaggaggaaaagacgcaagtgattaaattattctctcgatttgcgacctctttcaaagactactttaagaaccgcgccaactgcttcagcgcagatgatatcagctctagttcgtgtcataggattgtcaatgataacgctgagatcttctttagtaacgcgttagtttatcgaaggatcgttaagtctttgagcaatgatgacataaacaagattagcggtgatatgaaggatagcctgaaggagatgtctctagaggaaatatactcttatgagaagtacggagaattcatcacccaagaaggcatatcgttctataatgatatatgcggcaaggtcaactcattcatgaatttgtactgtcaaaagaataaagagaataagaacttatacaagcttcagaagcttcacaagcagatcctgtgtatagctgatacatcatacgaagtcccatacaaatttgagagtgatgaggaggtttaccaatcagttaacggatttcttgataatatttcatcaaagcatatcgttgagaggcttagaaagataggagataattacaacgggtataacctagataagatctatattgtctcaaagttctatgaatctgttagtcagaagacatatagggattgggagacaattaataccgcactggagatccattataacaatatcctccctgggaatggtaagtcgaaggcggacaaagtcaagaaggcggtgaagaacgatttacagaaatctattaccgagatcaatgagttagtgtctaattataagctttgttcggatgataacattaaggctgagacatacatccacgagatttctcacatattaaataacttcgaagctcaagagttgaaatataatcctgagattcatctggtggaatctgagttgaaagcaagcgagctcaagaatgtgcttgacgttataatgaatgcattccattggtgcagcgtgtttatgacagaggaactcgtagacaaggataataacttctatgctgaattggaagaaatatatgacgagatttatcctgtgatctcattatataatctagtccggaattacgttactcagaagccgtattcgacgaagaagattaagctcaatttcggcattccaacattagctgatggatggagcaagtccaaagaatacagcaataacgcaattatcctaatgcgagataacctttactacctcggtatctttaatgcgaagaacaaacccgacaagaaaatcattgagggaaatacttcagagaacaaaggcgattataagaaaatgatttataacctcttgccagggccgaacaagatgattcccaaggtatttctctctagtaagaccggagtagagacgtacaaacctagcgcttacatcctggaaggatacaaacagaataagcacattaagtcaagtaaggacttcgacatcactttctgccacgatttaatagattactttaagaactgcattgcaatacaccctgaatggaagaatttcggattcgatttctctgacacaagcacatatgaagacataagcggcttctatagagaagtagaacttcaaggctacaagattgattggacatatattagtgagaaggacatagacctccttcaggagaaaggtcaattgtatttgtttcaaatctacaataaagacttctctaagaagagtaccggaaatgacaaccttcacacgatgtacttaaagaatctgtttagtgaggagaatttgaaggacatcgtgctgaaattgaatggagaagcagagatcttttttagaaagtcgtcaattaagaatccgatcatacacaagaaagggtctatcttggtcaatcgaacctacgaagctgaagagaaggaccaatttggaaatatccagatagtgaggaagaatattccagagaatatctaccaagaactttacaagtacttcaatgataaatccgataaggagcttagcgacgaggcggccaagcttaagaatgttgttggacatcatgaagccgctacaaacatcgtcaaagattacagatatacttatgacaaatactttcttcatatgcccatcacaataaatttcaaggcgaataagaccggatttattaatgatcggatactccaatacatagctaaggagaaagacctccatgttatcggtatagatcgcggagaacgtaacttaatctatgtttctgttatcgacacttgtggaaatatcgtggagcagaagtcatttaacattgtcaacggctatgattatcaaattaagctgaagcagcaagaaggtgcacgtcagattgcacgtaaagagtggaaagaaataggcaagattaaggagattaaagagggatatttgagcttggtcattcacgaaatatctaagatggtcattaagtataatgctattattgctatggaggatttgtcatatggattcaagaaaggccgcttcaaagtagaacgacaagtttatcagaagtttgaaactatgctaattaacaaactcaattatcttgtatttaaagacatctctattactgagaatggtgggcttctaaagggatatcaacttacctatatcccagataagttgaagaatgttggtcatcaatgtggatgtatcttctatgtgccggctgcttacacatccaagattgatccaactacgggtttcgttaatatctttaaattcaaggatttaactgtggatgcgaagagagaatttataaagaaattcgacagcattaggtatgattctgagaagaacttgttctgtttcacgtttgattacaataactttattactcagaatactgttatgtcaaagtcatcatggagcgtctatacgtatggtgtcagaatcaagagacgtttcgtgaatggaagattctcaaacgaatcagacactattgatattactaaagatatggagaagacacttgaaatgacggatataaattggcgtgatgggcatgatcttagacaagatatcattgattatgagatagttcagcacatcttcgaaatctttagacttaccgtgcaaatgcggaacagtttatccgaacttgaagatagagactacgaccgcttgatatcgcctgtgttgaacgagaacaatatcttttacgacagtgcaaaggcgggtgatgctttgccgaaggatgcggatgctaacggagcgtattgcattgccttgaaaggactctatgaaattaaacaaataacagagaactggaaggaagacggcaagttctcacgtgataaattgaagatctctaacaaagactggttcgacttcattcagaataagcgctatctttag

SEQ ID NO: 239 - DNA, 3792 bp, Artificial Sequence
  Description of Artificial Sequence: Synthetic polynucleotide
atgaataatggaacaaataacttccagaacttcattggaatttcatctttgcagaaaacgttgcgaaatgcgttgattcctactgaaacgacgcaacaattcattgtgaagaatggtatcatcaaagaggatgagcttcgaggtgagaatagacagatcctcaaagacatcatggatgattactatagaggatttatatctgaaaccttgtcctccattgatgacatcgattggacttcactcttcgagaagatggagatccaattgaagaacggcgataacaaagacactcttatcaaagaacaaacagaatatcggaaagcaattcataagaaatttgcgaatgatgatcgattcaagaacatgttctctgccaagctgatttccgatattctccctgagtttgttatccataataataactattcggctagtgagaaggaagagaaaacccaagtgattaaactattctcccgcttcgctacaagtttcaaagattatttcaagaatcgtgcgaattgtttctcggccgatgacattagtagctcttcttgccatagaattgtcaacgataatgcagaaatcttctttagcaatgctcttgtgtatagaagaattgttaaatcgttaagcaacgatgatatcaataagatcagcggagatatgaaagactcattgaaggagatgagtctcgaagaaatatactcttacgagaagtacggagagtttattactcaagaagggatatctttctataatgatatctgtggaaaggttaattccttcatgaatttgtattgccagaagaataaagagaataagaacctctacaaactacagaagcttcataaacagatactgtgcatcgcagatacatcatatgaagtcccatataaatttgagtctgacgaagaggtttaccagtctgtgaacggctttcttgataatatctcatcgaagcatattgtggagagacttagaaagatcggcgacaattacaacggttacaatttggataagatctatattgtatcgaagttctacgaatcagtgtctcagaagacatacagagattgggaaactattaatacagctttggaaatacactacaacaatatccttccagggaatggaaagtctaaggctgacaaggtaaagaaggcagttaagaatgatcttcagaagtccataactgaaataaacgagttggtttccaattacaaattgtgcagcgatgataacatcaaagctgagacatatattcacgagatctcacatatcttgaataacttcgaggcacaagagctaaagtacaaccctgaaattcatctcgtggaatctgagcttaaggcttctgaactcaagaatgtgcttgatgttataatgaacgcgttccattggtgctctgtgttcatgacagaggaactcgttgacaaagacaataatttctacgctgaattagaggagatctacgacgagatttatcctgtgatatctttgtacaatttggtgcgtaactatgtgacacagaagccatatagtaccaagaagattaagctcaacttcggaatcccaactttggctgatggttggagtaagagcaaggaatactctaacaacgcgataatactgatgagggacaatttatattatctgggcatattcaacgctaagaacaagccggataagaagatcattgagggtaacacttcagagaacaaaggagattataagaaaatgatctacaacctgttgccaggccctaacaagatgattcctaaggtatttctctcgagcaagaccggtgtagaaacgtacaagccatccgcatatatcctggaaggttacaaacagaacaaacatataaagagttctaaggacttcgatattaccttctgtcatgatcttattgattacttcaagaactgtatagctatccatcccgagtggaagaacttcggatttgatttctcggatacatcaacatatgaggatatcagtggtttctaccgtgaggttgaattgcagggttataagatcgactggacatatatctcagagaaagatatcgatttgttacaggagaaaggccaactttatctatttcaaatatacaataaggactttagtaagaaatccacagggaatgacaacttgcacacgatgtatctgaagaacctattttctgaggagaacttgaaagatatcgtgctcaaactaaacggcgaagctgagatattcttccgtaagtcgagcatcaagaatccgatcattcacaagaaaggtagcatcctagtgaatagaacctacgaagcagaagagaaagatcagtttggaaacatccagattgtacgcaagaatatacctgagaatatataccaagagttgtacaagtatttcaacgacaagtcggacaaggaactcagcgatgaggctgctaaacttaagaatgttgttgggcatcatgaggcagcaacaaacatagtgaaggattacaggtatacgtacgataaatacttcctacacatgcctattactataaacttcaaggctaacaagaccggatttatcaatgatcgaatcttgcaatatatagctaaggagaaggacctgcatgttatcgggattgatagaggtgagcgaaacttaatttatgtatctgtcattgatacgtgtgggaatattgtcgagcagaaatcctttaatatcgttaacggttacgactaccagattaagctcaaacaacaggagggtgctaggcaaattgcccggaaggaatggaaggaaattggtaagattaaggaaatcaaggaaggctatttatcacttgttattcatgaaatcagtaagatggtcatcaaatataatgctattatagccatggaggatctttcatacggcttcaagaaaggtcgcttcaaggtcgaacggcaggtttatcagaaattcgagaccatgttaatcaataaactcaactatctcgtgttcaaggacatttcaattacagagaacggtggtttgcttaaaggataccagcttacatatatacccgacaaacttaagaatgttggacatcaatgcggatgcatattctacgttccagcagcttatacatccaagatcgatccaacaaccggcttcgtcaacatattcaaattcaaagatcttacggtagacgcaaagagagagtttattaagaagttcgactcaattcgttacgatagcgagaaaaacctgttctgcttcacatttgattataataacttcataacacagaataccgttatgtcgaaatctagctggtctgtttatacatacggagttcggatcaagagacgcttcgtcaatggccggtttagtaatgaaagcgataccatagatatcactaaagatatggagaaaaccttggaaatgacagacatcaattggagagatggtcacgatcttaggcaagatattattgattacgaaatcgtccagcatatctttgagatcttcaggcttacggtgcaaatgcgtaactctctaagcgaattagaggatcgtgactatgataggcttatatcacctgtccttaacgagaataatatcttctacgacagcgcaaaggcgggtgatgcactccctaaggacgctgacgctaacggtgcttactgcatagcacttaaaggactctacgaaattaagcagataacagagaattggaaggaagacggaaagttctcaagagataagcttaagatttcaaataaggattggttcgacttcatacagaataagagatatctttaa

SEQ ID NO: 240 - DNA, 3792 bp, Artificial Sequence
  Description of Artificial Sequence: Synthetic polynucleotide
atgaacaacggaacaaacaacttccagaatttcatcggtatctcctctctccagaagactcttcgcaatgcgcttattcctacagaaaccacacagcaattcatagttaagaacggaattataaaggaggatgagttgagaggtgagaacagacagatactgaaagatattatggatgattactaccgtggatttatatcggagactctgtcaagtattgatgatatagattggactagtctattcgaaaagatggaaattcaattgaagaatggtgataataaggatactctcattaaggagcagactgaataccgcaaggcaatacataagaaatttgcgaatgatgaccgctttaagaatatgttctccgcaaagttgattagcgatatcctcccagagttcgttatccacaacaataactattccgcttccgagaaagaggagaagacacaagttatcaagctcttcagtcggtttgctacgtcattcaaagattactttaagaatagggcaaactgtttctcggctgacgatatttcatcttcttcttgtcatcggattgtgaatgataatgcagagatctttttctctaacgcgttagtatatagacgcatcgtgaagtctctttccaacgatgatataaataagatttccggtgatatgaaggattccctgaaagaaatgtctttagaggagatttattcctatgagaaatacggtgagtttatcacgcaagaaggtatcagtttctacaatgatatctgtggaaaggttaattcatttatgaacctttattgccagaaaaataaagagaacaagaacttatataagcttcagaaactccataagcaaatcttatgcatcgcagatacatcttatgaggtgccatacaaattcgaatctgacgaagaggtatatcagtctgttaatgggttccttgacaatataagttcaaagcacatagttgagagactgcgtaagattggtgacaattacaacggatacaatttggataagatttacatcgtctccaaattctacgaatctgtttcacagaagacttatagggactgggaaactattaatacggccctagaaattcattacaacaacatattaccgggaaatggcaagtctaaggctgataaggtaaagaaagcggttaagaacgatcttcagaagtcaatcaccgaaattaacgaattagtttcgaactacaaattatgctcagacgataatatcaaggcggagacgtacatacatgagatatcgcacatccttaacaacttcgaggcccaggagctcaagtataatccagagatccatcttgtagaaagtgaactgaaggcctccgaattgaagaacgtgctggatgtgattatgaatgcatttcattggtgttcggtatttatgactgaagagttagtcgacaaggataataacttctacgcagagctcgaggagatatatgacgaaatttacccggtaatttcgctttataatcttgttaggaactacgtaacacagaagccttacagcactaagaagattaagttgaacttcggaataccaactctcgctgatggctggtcaaagtctaaggagtacagcaataatgctattatcttgatgagagataatttgtactatctcgggatctttaatgccaagaataaacctgacaagaagatcattgagggaaataccagcgagaacaagggtgattacaagaagatgatatataatctcttaccagggccaaataagatgataccgaaggtcttcctatcatcaaagacaggtgtggagacttacaagccgagcgcatatatattggaaggatataaacagaataaacatatcaagagtagcaaagacttcgatattactttctgccacgaccttattgattacttcaagaactgtatagcaatacatccggaatggaagaacttcggatttgacttctcagacacctcgacctatgaagatatttccgggttctatagggaggttgagcttcaaggttacaagatcgactggacgtacatttctgagaaagacattgacctgcttcaagagaaaggccagctatatttgttccagatttataacaaagacttctctaagaaatcaacagggaatgataacttgcacacgatgtacctcaagaatttattctccgaagagaacctcaaagacatagtgttgaaattgaacggagaagctgaaatattcttccgtaagagcagtatcaagaatcctataatccataagaagggcagcatcctagttaatagaacttacgaggctgaagagaaggatcaattcgggaatatacaaattgttaggaagaatattcctgagaatatatatcaggaattatacaaatactttaatgataagtcagataaagaactgtcggatgaggctgctaaactgaagaacgtagttggtcaccatgaagctgctactaatattgttaaggattaccgatacacttacgacaaatatttcctccacatgcctattacaatcaatttcaaagctaataagacaggattcatcaatgataggatcttacaatatatcgctaaagagaaagatctgcatgtgattggaatcgaccgaggagaacggaatcttatttatgtgtcagtgattgacacttgcgggaatattgttgagcagaaatcattcaacattgttaacggctatgattatcagattaagttgaaacaacaggagggagcaagacaaatagcacgaaaggaatggaaagaaattggtaagatcaaagagatcaaggaaggatacttgtctttggtgatacacgagatttccaagatggttatcaaatataacgccataatcgcaatggaagacctaagctacggcttcaagaaaggacgtttcaaagtcgagcgccaagtataccagaaattcgaaaccatgttaataaacaaactgaactatttagtgttcaaggatatctcgataactgagaatggaggtttgctcaaaggctatcagcttacatacataccagacaaattaaagaatgttggacaccagtgcgggtgcatcttctatgttccggcggcttatacttcaaagattgatcctactactggtttcgtgaacatctttaaatttaaggacctaactgttgatgccaagagagaatttatcaagaaatttgacagtattcgttacgatagtgagaaaaacctattctgcttcacgtttgattacaacaacttcattacccagaatactgtcatgtctaagagttcatggtctgtttacacttacggagtcagaatcaagagaagattcgtgaatgggcgtttcagtaacgagtcggatactatcgatatcactaaggacatggagaagacccttgagatgaccgatattaactggcgtgatgggcatgatctccgccaggatatcattgactacgaaattgtccagcacatctttgagatcttccgtttgacagttcagatgagaaatagtcttagcgaattggaagacagagactatgacagattaatcagcccagtgcttaacgagaataacatcttctatgatagtgccaaggcaggcgatgcgttacccaaggatgctgacgcaaacggagcatactgtattgcactcaaagggctttacgaaatcaaacaaattacagagaattggaaggaagatggtaagttctctagggacaaacttaagatctctaataaagattggttcgatttcattcagaacaagcgctatctgtaa

SEQ ID NO: 241 - DNA, 3792 bp, Artificial Sequence
  Description of Artificial Sequence: Synthetic polynucleotide
atgaacaatggaactaataatttccagaacttcattggtatcagttcgctccaaaagactttaagaaatgctttaatccctactgaaactacacagcagttcattgtaaagaatggaataattaaggaggacgaattacgtggagagaaccgtcagatcctcaaggatatcatggatgattattatcgtggcttcatcagcgaaacgttatcgtcaatcgatgacatcgattggacatcattattcgaaaagatggagattcaacttaagaatggtgataataaagataccttaattaaggaacagactgaatacagaaaggcaatacacaagaaattcgcgaacgatgatcggttcaagaacatgttctcagctaagctcatatcagatatattgccggaattcgtaattcataataacaactatagcgcgtctgagaaggaggagaagactcaggttattaagttattctctcgatttgctacgtccttcaaagattattttaagaatagagctaactgtttctccgcggacgatattagctcttcatcatgccatcgcatcgtcaacgacaatgctgagatcttcttctcgaacgctctggtctatcgtagaatagttaaatctttgtcaaacgacgatatcaacaagattagcggagatatgaaagatagtctgaaggaaatgagtcttgaagagatttatagctatgagaagtacggagagttcataacacaggaaggtatttccttctataacgatatctgtggaaaggttaactcattcatgaatttgtactgtcagaaaaataaagagaataagaatctatacaagctacagaaacttcataagcaaatcctatgtatcgcagatactagttatgaggtcccttataaatttgaatcggatgaagaggtttatcaatctgtcaatgggttccttgataacatctcctctaagcatattgtagagcgtttgcgaaagattggagataattacaacggttacaatctggataagatttacatcgtttctaaattctatgagagcgtgtctcaaaagacatacagagactgggagaccatcaacactgcactagaaatacactataataatatcctgccaggaaatgggaaatctaaagctgataaggtcaagaaggcagttaagaacgatttacagaagtcgataacagagataaatgaattagtgagcaactacaaactttgttctgatgataatattaaagctgaaacatacattcacgagatttctcatattcttaacaacttcgaagcccaagaattaaagtataatccagaaatccaccttgtcgagagcgagcttaaggcctcagagctaaagaatgtacttgacgttattatgaatgcgttccactggtgtagcgtgttcatgacagaggaactagtcgacaaggataataatttctatgctgagttagaagaaatatacgatgagatctatccggtgatatcattatacaaccttgtccgaaactacgtgacgcagaaaccttatagcactaagaagataaagttaaacttcgggattcctacattagcagatggatggtctaagagcaaggaatactccaataatgctatcattctaatgcgagacaacttatactatttgggtatctttaacgccaagaataaaccagataagaaaatcatcgaagggaatacgtccgagaacaaaggagactataagaagatgatttataacttgctgcctggacccaataagatgattcctaaagtgttcttatcatcgaagacgggcgtcgagacgtacaaaccgtccgcatatatccttgaaggttataagcagaacaagcatattaagtcaagtaaggacttcgacataaccttctgtcatgatttgatcgattactttaagaactgcattgccatacatcccgaatggaagaacttcggctttgatttcagcgacacttcaacttatgaggacatttctggcttctatagagaagtggagcttcaaggttataagatcgattggacatatattagtgagaaggacatcgaccttctccaagagaaaggacagttatatctctttcaaatttataacaaagacttctcgaagaagtcaactggtaacgataatctccacacaatgtaccttaagaatttatttagtgaggagaacttaaaggatattgttcttaaattaaacggtgaggcagagatattttttcgcaagagcagtattaagaaccctatcatccacaagaaaggatctatcttggtgaatcgtacgtacgaagcagaagagaaggatcagttcggaaacattcagattgtgcggaagaacatccctgagaacatctatcaagaactttataagtactttaacgacaagtcagataaagaacttagcgatgaagctgcaaagctgaagaatgtagttggtcatcatgaggctgctaccaacattgtcaaagattaccgatatacttatgataagtacttcctacacatgcccatcaccatcaacttcaaagccaataagactggcttcatcaatgatcggattctgcaatacattgcgaaggagaaagacctacacgtcattggtatagacagaggcgaaagaaatcttatttacgtgtctgtcatcgatacatgtggtaatatcgtcgagcagaaatcattcaatattgttaatggctatgactatcaaatcaagcttaagcaacaagaaggagcacgccagattgcaagaaaggaatggaaagaaataggcaagatcaaggaaattaaggaaggatacttatcgcttgttatacacgaaatcagtaagatggttatcaaatacaatgctataatagctatggaggacctctcgtacggattcaagaagggacgattcaaagttgaaagacaagtttatcagaaattcgagactatgctcatcaacaaactgaactatctagtctttaaagatatctcaatcacggagaatggcggtcttctcaagggataccaacttacgtatattccggataaattgaagaacgttggtcatcagtgtggatgtatattctatgttccagctgcctacacatcaaagatcgatcccactacgggattcgtaaacatatttaaattcaaggacctaacagtggacgccaagagagaatttatcaagaaatttgattccattaggtatgattccgagaagaacctgttttgcttcaccttcgactataataacttcataacacagaatacggtgatgtccaagtcgtcttggagtgtctacacatatggtgttcgtataaagagaagattcgtaaatggtcgattctcaaacgagtctgacactattgatatcacgaaggacatggaaaagacactagagatgactgatataaactggagagatggtcatgacctgaggcaggatatcatcgactatgagatcgttcagcatatcttcgagatctttcgtcttacggttcaaatgcggaattccctttcagaacttgaggatcgagattacgatcgtctgatttctcctgtgcttaatgagaacaacatcttctatgattctgctaaggccggagatgccttgcctaaggacgcagacgctaacggtgcatactgtatcgctctcaaggggttgtatgaaattaagcaaattaccgagaattggaaggaagatgggaagttctctagggataaattaaagattagcaacaaggattggttcgatttcattcagaacaagagatatctttga

SEQ ID NO: 242 - DNA, 3792 bp, Artificial Sequence
  Description of Artificial Sequence: Synthetic polynucleotide
atgaacaacggaactaataacttccagaacttcattggaatatcatctttgcagaagacattgcgcaacgcccttatccctacagagactacgcagcaatttatcgttaagaacggcataataaaggaagatgagcttcgtggtgagaaccgacagattcttaaggatattatggatgactattaccgtggattcatttcggaaactttatctagtatcgacgacatcgactggacgagcttatttgagaaaatggaaatacagcttaagaatggtgataataaagatactttgattaaagaacaaacagaatataggaaagctattcacaagaaatttgcaaacgatgataggtttaagaacatgttctctgcaaagctaatcagcgatatcttgccggaattcgtgatccacaacaacaattattcagcatctgagaaagaagagaagacccaggttattaagttgtttagccgattcgcgactagcttcaaagattattttaagaatagagcaaactgtttctctgcagatgacatttcttcatcatcttgccataggatcgtcaatgacaatgctgagatcttcttctcgaacgccttggtatatcgaaggatcgtaaagagcttatcgaacgatgatataaataagatttccggtgatatgaaagattctctcaaggaaatgtcactcgaagaaatttattcctatgagaagtatggagagtttatcacccaagagggaatttctttctacaacgatatctgtggtaaagtgaactcgttcatgaatctgtactgccagaagaacaaagagaataagaacctttacaaacttcagaaactccataaacaaattctctgtatcgccgatacttcctacgaagttccttataaattcgaaagcgacgaagaagtttaccaatctgtcaacggtttcttggataacatatcatcgaagcatattgtggagcgccttagaaagataggtgacaattataacggatataatctagacaagatctacatcgttagtaaattctacgaatcagtttcgcagaagacttatagggactgggagactatcaatacagcactcgaaatccattataataacatactgccgggaaatgggaagtctaaggcagataaagtcaagaaagcggtgaagaacgatttacagaagtccataactgaaattaacgagcttgtttccaattacaaattatgttctgatgacaatattaaggcggagacatatattcacgaaatatctcatattctgaacaatttcgaagcgcaagagctcaagtataatccggagatccatttggtggaatcggaacttaaggcgagtgaactaaagaacgtgctcgatgtcatcatgaacgccttccattggtgttcggtattcatgacggaagagttggttgacaaagataacaacttctatgctgagttggaggagatctatgatgaaatatatccggtgatttcgctatataacttagtgaggaactacgtcacacagaagccatactccacgaagaagatcaagctcaacttcggtatccctactctggctgacggatggtcaaagtccaaggagtacagtaataacgctataatcttgatgagagataatttatactatctaggtatctttaatgctaagaacaaaccagataagaaaattatcgaaggaaatacatctgagaacaaaggagactataagaagatgatctacaatctccttcctggcccaaataagatgattccgaaagtgtttttgtcttccaagacaggtgttgaaacttacaaaccttctgcatacattctagaagggtataagcagaacaaacatattaaatcatctaaagacttcgatatcacgttctgccacgatctgattgattattttaagaattgcattgctatccaccctgaatggaagaacttcggatttgactttagcgatacatctacatatgaggatatttcaggtttctatagagaggttgaactacagggatataagattgattggacatatatttcagagaaggacatagatctcttgcaggagaagggtcaactttatctatttcaaatttacaataaggacttctctaagaagtcaactgggaacgataacctacacacaatgtatctcaagaatctgttctctgaggagaatctgaaggatatcgtactcaaacttaacggtgaagccgagatcttcttcaggaagtcatctattaagaacccgattatacataagaaaggatcaattctggttaaccgaacatatgaagctgaggagaaagatcaatttggtaatattcaaatcgtccgaaagaacattccagagaacatctatcaggagctttacaaatatttcaacgacaagtcagacaaagagctatctgacgaggcagcaaagttgaagaacgtggttggtcatcacgaagccgctacaaatattgttaaggattatcgttatacgtacgataagtatttccttcatatgccgattacgattaacttcaaagcaaataagacgggcttcattaatgatcgaatactacagtatatagccaaggagaaagatcttcatgttattggaatcgacagaggagaacgtaatcttatatacgtgtctgttatagatacctgtggaaatatcgtggaacagaagagcttcaacattgtgaatgggtacgattatcagatcaagcttaagcaacaggagggagccagacagatagcaagaaaggagtggaaagaaattggaaagattaaagaaattaaggagggctatctcagccttgtcatccacgaaattagtaagatggtcatcaagtacaatgccattatagctatggaggatttatcatacggatttaagaagggcagattcaaagtagaacggcaagtttaccagaagtttgaaacaatgcttatcaataagctgaactacttggtctttaaggacatttcaataacagagaatggaggactgcttaaaggataccagcttacatacatacctgataagctgaagaatgttggacatcagtgtggctgtatcttttatgtgcctgctgcatatacatcaaagatagaccctacaacgggatttgtgaacatatttaagttcaaggacctaacagtggacgcaaagagagaatttattaagaagttcgatagcattcgatatgacagtgagaagaatctcttctgcttcaccttcgactacaacaatttcattactcagaataccgtgatgtccaagtcttcttggtctgtgtacacatatggagttagaatcaaacgtagatttgttaatgggcgattctcgaatgagtctgatactattgatataacaaaggacatggaaaagacactagaaatgactgatatcaattggagggacggccatgatctgaggcaggatatcattgattacgaaatagtccaacatatctttgaaatcttcagattgactgtgcagatgcgtaattctctcagtgaacttgaagacagagattacgatcgcttgatcagcccagttctcaatgagaacaatatcttctacgattcagcgaaggctggagacgcacttcctaaagacgccgatgctaacggagcatattgtattgcacttaagggactctatgaaatcaagcagattactgagaactggaaagaagatggcaagtttagccgtgacaagttgaagattagcaacaaggactggttcgacttcatccagaataagaggtatctctag

SEQ ID NO: 243 - DNA, 3792 bp, Artificial Sequence
  Description of Artificial Sequence: Synthetic polynucleotide
atgaacaacggaactaataacttccagaactttatagggatctcaagccttcaaaagacgctgcgcaacgcgttgattcccaccgaaacgactcaacagtttatcgtaaagaatggcattatcaaggaggatgagttgcgaggcgagaatcgccagatcctcaaagatatcatggacgattattaccgaggctttatcagtgaaaccttaagcagcatcgatgacatagattggacctcactctttgaaaagatggaaatacaactgaagaatggagataataaagatacgctcattaaggaacagacagaatatagaaaggcaatccacaagaagttcgctaatgatgacagatttaagaacatgttctctgccaagctgataagcgacatactgcccgaatttgtaattcataataacaattacagcgccagtgagaaggaggagaagacacaggtgattaagttattctccaggttcgcaacctccttcaaggactacttcaagaaccgcgccaattgcttcagtgcagacgatatcagtagctcatcctgtcacagaatcgtgaacgataacgcggaaatcttcttctcgaacgctctggtgtatcgacgaattgtcaagtctctgtcaaatgatgacataaataagatcagcggtgacatgaaggactctctcaaggaaatgtctctcgaagaaatttatagctacgagaaatacggcgagtttatcacacaggaaggaatcagcttctataacgatatttgcggcaaggtcaactccttcatgaacctgtattgtcaaaagaataaggagaataagaatctctataaattgcagaagttgcataaacagattctctgtatagccgacacatcatacgaggtgccatacaagtttgagtctgatgaggaagtgtatcaatcagttaatggattcctggacaatatttccagcaagcatattgtcgagcgactgaggaagattggagataactataacggatataatctggacaagatctacatcgttagtaaattctacgaatccgtttctcagaagacttaccgcgattgggagactattaacactgctttggaaattcattataacaacatattgcctggtaacggcaagagcaaggcggacaaagttaagaaagcagtgaagaatgacttacagaagtctataaccgaaatcaatgagctggtgtccaattacaaactctgctcagacgataatatcaaagcggaaacttatattcacgaaattagccacattctcaacaacttcgaagcacaggaactgaagtataatccggaaattcacctggtggaatcagagctgaaggcaagcgagcttaagaatgttctggatgttatcatgaatgcgttccattggtgctcagtctttatgacggaggaactcgtcgacaaagataacaatttctacgccgaactggaggaaatctacgacgagatttaccctgtgattagcctgtacaatctggtacggaattatgtgacccagaagccatatagcacaaaaaagattaaattgaacttcggcatacctaccctggcggatggctggtcaaagtcgaaggaatatagcaataatgcgataatccttatgcgggacaatctgtactacctcggcatattcaacgctaagaacaagccagacaaaaagattattgaagggaatacaagtgagaacaagggagactacaagaagatgatctataatctcctgcccgggcccaacaagatgatacctaaggtgttcctgagcagcaagaccggagtagaaacgtataagccatcggcttacatcctggaaggctataagcagaataaacatatcaagtctagcaaggatttcgacataactttctgccacgatttaatcgattacttcaagaactgtatagctatccaccctgaatggaagaactttggatttgactttagtgatacttcaacttacgaggatatctcaggcttctaccgggaagtggaacttcagggttataagatagactggacatacataagcgagaaggacattgatctcctgcaagagaaaggtcagctttacctgttccagatttacaacaaagactttagcaaaaagagtactggaaacgacaacttgcacacaatgtacttaaagaacctgtttagcgaggagaaccttaaagatattgttcttaagctaaatggagaagccgaaatattcttccggaaatcatctattaagaatccaataatccacaagaaaggcagcatcctcgtaaatcgtacatacgaggctgaggagaaggatcagtttggcaatatacaaattgtgcggaagaacatacctgagaacatttatcaggaactttataaatacttcaatgataagtcggataaggagctcagcgatgaagcagctaaactcaagaacgtggtgggccaccacgaagcagccaccaacatcgtgaaagactacaggtacacctacgacaagtacttcctgcatatgcccatcacaatcaatttcaaagcaaacaagacaggtttcattaatgacagaattctgcagtatatagccaaggagaaggatctacatgtcatagggattgatcgcggtgagcggaatttgatttacgtatcagtgatcgacacttgcggaaatattgttgagcagaagagcttcaatatagtaaatggatacgactatcagattaagcttaaacagcaggaaggcgctaggcagattgcacggaaagagtggaaagaaatcggaaagatcaaagagatcaaagagggttacttaagcttggtcatccacgagatttccaagatggtcatcaagtacaacgctataattgctatggaagatctgagctacggattcaagaaaggtaggttcaaagtggaacgacaagtttaccagaaattcgagacaatgctcatcaacaaactcaactacctcgtctttaaagacatctctataaccgagaatggtggtttacttaaaggatatcaactgacatatattcctgataagctaaagaatgtgggccatcagtgtggatgtatcttctatgtgcccgctgcctataccagcaagattgaccctactaccggatttgttaatatatttaagtttaaggacctcaccgtggacgccaaacgagagtttatcaagaagtttgactccattagatacgattctgagaaaaacctgttctgctttacgttcgattacaataacttcatcacccagaacactgtgatgtcgaagagcagctggagcgtttacacctacggagtgcgtattaagagaaggtttgtcaacggacggtttagcaatgagtccgatactatcgatatcaccaaagacatggaaaagactctcgagatgaccgatatcaattggcgtgatggccatgatcttaggcaagatatcattgattacgagatagtgcagcacatctttgaaatctttagactcactgtgcagatgcgaaactccttgtccgaactggaagaccgggactacgatcgattgatatctccagttctcaatgagaataatatcttttacgacagcgccaaagcaggcgacgctctcccgaaggacgctgatgcaaacggtgcctactgcatagccctgaagggcctgtatgagattaagcaaattaccgagaattggaaagaagacggcaagttctctagggacaaactgaagatttcgaataaggactggtttgacttcatccagaacaagagatacctctaa

SEQ ID NO: 244 - DNA, 3792 bp, Artificial Sequence
  Description of Artificial Sequence: Synthetic polynucleotide
atgaataacgggacaaataactttcagaactttatcggcattagcagcttgcagaagacgctgagaaacgccctcatcccaacagaaaccacacagcaatttatcgttaagaatggaattattaaggaggatgagcttcgtggcgagaatcggcagatcttgaaagatattatggatgactactatcgcggtttcatttctgagactttgtcctccatcgacgatatcgattggaccagcctctttgagaagatggagattcaattgaagaacggtgacaacaaggatactctcatcaaagaacagaccgagtatcgaaaggccatccataagaagtttgcgaacgacgatcgatttaagaacatgtttagcgccaaactcatcagtgacatcttgcccgagttcgtaatccacaacaataattactcggctagcgagaaagaagagaaaacccaggtgattaagctgttctctcgcttcgctacgtcctttaaagattatttcaagaatagggctaattgtttctcggccgatgacatctcttcctcgtcttgccatcgaattgtgaacgataacgccgagatatttttctctaacgccttagtgtaccgcagaatcgttaagagtctgagtaatgatgatatcaacaagataagcggcgacatgaaggattctctgaaagagatgagcctggaagaaatctatagttatgagaaatacggtgaatttatcacacaggagggaatttcgttctacaatgacatctgcggcaaggtcaactccttcatgaacttgtattgccagaagaataaagagaacaagaatttatacaagctccagaagctgcataaacagatcttatgcattgccgacacgtcctacgaggttccgtacaagttcgaatcggatgaagaggtctatcagtccgtaaacggcttcttagacaacatctccagtaaacacatcgtcgaacgactgagaaagattggcgacaattacaatggatacaatctggataagatctacatcgttagtaaattctacgagagtgtttctcagaaaacttaccgggattgggaaactataaatacagctctggaaatccattataacaatattctgccagggaatggtaagagcaaggcggataaggtcaagaaggccgtgaagaatgacctccagaaatccatcactgagataaacgaacttgtcagcaattataaactctgttccgacgacaatatcaaggccgaaacctacattcacgagattagtcatattctcaataatttcgaagcacaggaacttaaatacaatccagaaatccacctcgttgagtctgagctgaaagctagtgagctaaagaatgtgctggatgtaatcatgaatgccttccactggtgctcggtgtttatgaccgaggagttggtggataaagataataatttctacgctgagcttgaagaaatatacgacgagatatacccagtgatctccctctataacctcgtacggaactacgtcacccagaaaccttattcaacgaagaagattaagttgaactttggcattcccacgttggccgacggctggtccaagagtaaggaatactccaacaatgcaataatactgatgagggataacttgtattatctcggtatcttcaacgctaagaataaacccgataaaaagatcatagagggaaatacatcagagaacaagggtgactacaagaagatgatctataatctgctcccaggccctaacaagatgataccaaaggtatttttgtcatccaagactggcgttgagacctataaaccaagtgcgtacatactggagggttataagcagaacaagcatattaagagttctaaggacttcgacataacgttctgccatgacctgattgattactttaagaactgcatagcaattcatccggaatggaagaatttcggatttgacttcagtgacactagtacctacgaagacattagcggtttctatcgggaggttgaactgcaaggatataagattgattggacttatatctctgagaaggatatcgacctgctgcaagagaaagggcaattatatttgtttcagatctacaataaagacttctccaagaaatccacagggaatgataatcttcacacaatgtatctgaagaacctgttctctgaggagaatctgaaagatatcgtgctaaagttgaatggtgaggctgagatcttcttccggaagtcctctataaagaatcccatcatccataagaagggctcgatcttggtgaatcgaacctatgaggccgaggagaaggaccagttcggtaacatccagatcgtgcgaaagaatattcccgagaatatctaccaggaattatataagtatttcaatgacaagtctgataaagagctctctgatgaggccgccaagctcaagaacgttgtaggccaccacgaagctgccaccaacatagtgaaggattatcggtatacttacgacaaatacttcctccacatgcccatcactatcaacttcaaagccaacaagaccggcttcataaatgaccgcattctgcagtacatcgcaaaggagaaggacctgcatgtgattggtattgaccgaggcgagcgtaacctcatatatgtttctgtaattgacacttgcggcaatatcgtggaacagaaatccttcaatattgtcaatggatacgattaccagatcaaacttaagcagcaagagggagccagacagatagcgaggaaggaatggaaagaaatagggaagataaaggaaatcaaagagggttatctgagccttgtcattcatgagatctctaagatggttattaagtacaatgccattatcgcgatggaagacctgtcatatggattcaagaaaggacgcttcaaagtggaacgccaggtctaccagaaattcgagacaatgctcattaacaagctgaattacctggtgtttaaggatattagcataactgagaacggaggcctcctcaaagggtaccagctcacttacatacctgataagttaaagaacgtcggccatcagtgcggttgtatattctatgttcccgccgcctacacatccaagatagatcccaccacgggattcgtcaacatctttaaatttaaagacttgactgttgacgccaagcgagaattcattaagaagtttgattccatcaggtacgactccgaaaagaatctcttctgtttcacatttgactataataacttcattacgcagaatactgtcatgtccaagtcttcatggtcagtctatacctatggcgtgcgtatcaagagaagattcgttaacggtaggtttagtaacgagagcgacactatcgacataactaaagacatggagaagacactggagatgacagacataaattggcgagatggccatgacctgagacaggacataatcgactacgagatcgtgcagcatatattcgaaatcttccggctgacggttcagatgaggaacagcctgagtgagctcgaagaccgagattacgacagactgatttcacctgtcctaaatgagaataatattttctacgatagtgcaaaggcaggcgacgccttacctaaggatgctgacgcaaacggcgcatattgtatagcgctaaagggattgtatgagatcaagcagataaccgagaattggaaagaggatggcaaattctcacgggacaagttgaagatatcgaataaggattggttcgatttcattcagaacaaacgatatctgtga

SEQ ID NO: 245 - DNA, 3792 bp, Artificial Sequence
  Description of Artificial Sequence: Synthetic polynucleotide
atgaacaacggaaccaacaactttcagaacttcatcgggatttcgagcttgcagaagacacttcgcaacgctcttatacccaccgaaacaactcagcaattcatagttaagaatggcataatcaaggaggacgaactgcgtggcgagaatcgacagatccttaaagatatcatggatgactactatcggggctttatatccgaaaccctctcctcaattgatgatattgattggacttccttatttgagaagatggaaattcagctcaagaatggcgacaataaagacaccctgattaaagaacagaccgaataccggaaagcaatacataagaagttcgctaatgacgaccggttcaagaacatgtttagtgccaaactgatatctgatatccttcccgaattcgttatccacaataacaactactcagcctcagagaaggaggaaaagacccaggtaatcaaattgttctctagattcgccacctctttcaaagactacttcaagaaccgcgccaattgtttctctgccgatgacattagttcctcttcatgtcacagaattgtcaacgataacgctgaaatctttttctctaacgctcttgtgtacaggcggatagtcaagtcactgagcaacgatgatataaacaagatatccggcgatatgaaggattccctcaaagaaatgtcactcgaggagatttatagttatgagaaatacggtgaatttataacgcaggagggcatcagcttctacaacgatatttgcggcaaggtgaattctttcatgaatctgtactgccagaagaataaagagaacaagaacctctataagcttcagaaactgcacaagcagatcctgtgtattgccgacacttcatatgaggttccgtataaattcgagtctgatgaggaggtttatcaaagcgtgaacggctttctggataacatttcttcaaagcatattgtggagcggttgagaaagatcggtgacaactataacggatataatctcgataagatctacattgtctccaagttctacgagtccgtgagtcaaaagacctacagagactgggaaaccattaacacggccctcgagatacattacaacaatatattaccaggcaatggaaagtctaaagccgacaaggtgaagaaagcagtaaagaatgacctgcagaaatcaatcactgagatcaacgagctggtctccaactataagctatgctccgacgataatattaaggcagaaacatatatccatgagatcagccatattctcaacaactttgaagcccaagagctgaagtataaccctgaaatccatctggttgagagcgaactcaaggctagtgaattgaagaatgtcctcgacgtcatcatgaacgccttccactggtgcagcgtattcatgacagaagagttggttgacaaagacaacaacttctacgccgaattggaagaaatctacgacgaaatttaccctgtgatcagtctatataatttggtgcgaaattatgtcacgcagaagccctactccaccaagaagattaagttaaactttgggatacccacactagccgatggatggagtaaatccaaagaatattctaacaatgcaattatactcatgagggacaacctctactacctcggaatctttaatgctaagaataagcccgacaagaagataatcgaaggcaacactagcgagaacaaaggcgactacaagaagatgatttacaacctactgccaggacccaacaagatgatccctaaggtgttcctctccagtaagaccggcgtagagacgtataaaccaagcgcctacatcctagagggctacaagcagaacaagcatattaagagtagcaaggacttcgacatcacattctgtcacgatctcattgattacttcaagaactgtattgcaatacatccagaatggaagaactttgggttcgacttcagcgatactagcacctacgaggacatctccggattctatagagaagtggaattacagggttataagatagactggacttacatttctgagaaagacatagaccttctccaggagaaagggcagttgtacttatttcagatatacaataaggacttcagtaagaagtcgaccgggaatgataatctccataccatgtacctgaagaatttattcagtgaagagaatcttaaggacattgtcctgaagctgaacggtgaagcagaaatattctttcgcaagtccagtatcaagaatccaattatacacaagaaaggctcaatacttgtaaataggacatatgaggctgaagagaaagatcaatttggcaatattcagatcgtgagaaagaacattccggagaatatctatcaagagctgtataagtactttaatgacaagtccgacaaggaactgtccgatgaagccgccaagttaaagaatgttgtaggtcaccacgaggctgcgacgaacatcgtaaaggactaccgatacacctacgataagtactttctccacatgccaataacaatcaacttcaaggcgaacaagactggattcatcaacgacagaatcctgcagtacatcgcaaaggagaaggaccttcatgtgattggtattgacagaggcgagaggaaccttatctacgtgagcgttattgacacatgcggaaatattgttgagcagaaaagtttcaatatagtgaatgggtacgattaccagatcaaactaaagcaacaagagggcgcccgacagattgctcggaaggaatggaaggagatcggcaagatcaaggagatcaaagagggatacctgtccctggttattcacgagatctccaagatggtgatcaagtataacgcaatcatcgctatggaagacctgagctacggcttcaagaagggaaggtttaaagtggagcggcaggtgtaccagaagtttgagaccatgttgattaacaagctgaactacctagtgttcaaggatatatccattacagagaacggtggtttgcttaaaggatatcaactgacctacattccggataaactcaagaacgtgggacaccaatgcggatgtatcttctacgtgccggcagcttacacctcaaagatcgatccgacgaccggcttcgtaaacatctttaagttcaaggatctgacggtagacgctaagagagagttcataaagaaattcgactctataaggtatgattccgagaagaacctgttctgcttcacctttgactataataacttcattacccagaataccgtgatgtctaagagttcgtggagtgtgtacacatacggagtaaggatcaagcggagatttgttaacgggagattctctaacgaatccgacacgatcgacattactaaggacatggagaagactctcgaaatgaccgacatcaattggagggacggtcatgacctgcgacaggacattatcgactacgagatcgtgcagcacatatttgagatattccgcctgacggtccagatgagaaattctttgagtgagcttgaggatagggattacgatcgactaatttctcctgtcctgaacgagaacaatatcttctatgacagcgccaaggccggcgacgcccttcctaaggatgccgacgccaacggcgcttactgcattgccctgaaaggattatacgagatcaagcagataaccgagaattggaaagaggacggcaagttctctagggacaaactgaagatctccaacaaggattggtttgacttcatacagaataagagatacctttag

SEQ ID NO: 246 - DNA, 3792 bp, Artificial Sequence
  Description of Artificial Sequence: Synthetic polynucleotide
atgaacaatggaaccaacaatttccagaattttatcggcatttcctcgttgcaaaagacccttaggaacgcactgatcccgacagaaactactcagcagttcattgtcaagaatggaatcatcaaagaggacgagctgagaggcgagaatcgtcagatccttaaagacatcatggacgactactatcgcggattcatcagcgagacactcagcagtatagacgacatcgattggacatctctgtttgaaaagatggagatccagcttaagaatggtgacaacaaagacactctgatcaaagagcagaccgagtaccggaaggccatccacaagaagtttgccaacgacgacagattcaagaatatgttctccgccaagctaattagcgacatcctgcccgagtttgtcatacacaataacaattactcggcgagcgagaaagaggagaagacacaggttataaagctattctctcgcttcgctactagcttcaaggactacttcaagaacagagcgaattgtttctcggccgatgacatctcctcctcttcgtgtcaccgcatcgttaatgataacgctgagatctttttctctaacgctctagtgtaccgcaggatcgtgaaatcccttagtaacgacgacatcaacaagatcagcggtgacatgaaagacagcctgaaggagatgagtctggaagaaatctacagctatgagaaatatggcgaattcatcacccaagaaggaatcagtttctacaacgatatttgcggtaaagtgaactctttcatgaacttatactgccagaagaacaaggagaataagaacctttataaactccagaagttgcacaaacaaatcctgtgcatcgctgacactagttatgaagtaccttataaattcgaatcagacgaggaagtataccaatctgttaatgggtttcttgacaacatctcttcaaagcatatagtggaaaggttgaggaagataggcgataattataatggttataatctagataagatctatatcgtatcaaagttctatgagtccgtgtcacagaagacctatagagactgggaaactatcaacacggctttagagatacactataataacatcctacccggcaacggtaagagcaaggccgacaaggtgaagaaagctgtgaagaatgatctacagaagagcatcactgagataaacgaactcgtctctaattataaactgtgctcggacgacaatattaaggccgagacttatatccacgagatctcacacatcttaaacaactttgaggcgcaggaactcaagtacaatcccgagatccatctagttgaatctgaactgaaggcaagtgaacttaagaacgtgctggacgttatcatgaatgctttccactggtgcagtgtctttatgacagaggagctggtggacaaggataataatttctacgctgaactggaggaaatctatgatgaaatctacccagtgatctccttgtacaacctggtgaggaactacgttactcagaaaccgtactctacaaagaagattaagcttaacttcggtatacccactctagcagacggatggagcaagagtaaggagtattctaataatgcaataatattaatgagagacaatttgtattacctcgggatatttaacgctaagaacaaaccagacaagaagatcatcgagggaaacacatcagagaacaaaggagattataagaagatgatctacaacctgttgcctggcccgaataagatgatccctaaagtcttcctcagtagcaagacgggagtcgaaacatataagccctccgcttacatcttggaaggctataagcagaataagcacattaaatcatccaaggacttcgatataaccttctgccatgacctaattgactactttaagaattgcattgccattcatcctgagtggaagaacttcggtttcgatttctccgacacatcaacttacgaagacatttctggcttctaccgggaagtagagctccaaggctacaagatcgactggacctacattagcgagaaggacatcgacctgctgcaagagaaaggccagctttacctgttccagatctacaacaaagatttcagcaagaagtcaacaggaaatgataaccttcacactatgtatttgaagaacctgttcagcgaggagaaccttaaggacattgtgcttaaactcaacggagaagcagaaatcttcttcagaaagagcagcattaagaatcccattattcacaagaagggatccattctggtgaacaggacatatgaagccgaagagaaggatcagtttgggaatattcagatcgtgaggaagaatataccagagaatatctatcaggagctctacaagtacttcaacgacaagagcgacaaggagttatccgatgaagctgcgaagctaaagaacgtagtcgggcatcatgaggccgccacaaatatcgttaaggattatcgctatacttatgacaagtacttcctgcacatgcccattacaattaacttcaaagccaacaagaccggattcatcaatgaccgcattctgcaatacatcgccaaggagaaagacctgcacgtcattggcatagaccgaggagagcgtaaccttatttatgtgtccgtcatcgacacttgtggcaatattgtggagcagaaatcatttaatatcgtgaatggatacgattatcagatcaaactcaagcaacaggagggcgcccgccagattgcaaggaaagaatggaaagagatcggcaagatcaaagaaattaaagaaggttatctgtctctagtgatccatgagatttccaagatggttatcaagtacaatgcaattatcgcaatggaagacctgtcttacggcttcaagaaaggtcggttcaaggttgagaggcaggtgtaccagaagtttgagacaatgctgatcaataagttgaattacctggtcttcaaagacatttccataacagagaacggcggccttcttaaagggtatcaattaacttacatccctgacaaactgaagaacgtgggacaccaatgtggttgtatcttctatgttcctgccgcttacactagcaagatcgatcccacaaccggatttgtcaatatcttcaaatttaaagatctcaccgtcgatgcaaagagggagtttattaagaagttcgatagcatcaggtacgactctgaaaagaatctgttctgtttcactttcgactacaataacttcatcactcagaacacggtcatgtcaaagagttcatggtccgtatacacctacggcgtgaggatcaaacgtaggtttgtcaatgggcgcttcagtaatgaatctgacacaatcgacattacaaaggacatggagaaaactctagagatgactgatatcaattggcgagacggccatgacttgcgccaagatatcatcgactacgaaatcgttcagcacatattcgagatatttcggctgacagtccagatgcgtaactccttgagcgagctggaagatcgggattatgaccggctgatcagtcctgtcctaaatgagaataacatattctacgactctgctaaggccggcgacgctttgcccaaggatgcagatgccaatggtgcctactgcatcgccttgaaaggcctgtacgagattaagcagattaccgagaactggaaggaagacggcaagttctcccgggacaaactgaagatctctaataaggactggttcgacttcattcagaataagagatacttataa

SEQ ID NO: 247 - DNA, 3792 bp, Artificial Sequence
  Description of Artificial Sequence: Synthetic polynucleotide
atgaataacggtaccaacaatttccagaatttcatcgggatctcaagtctccagaagaccttaaggaacgcactgatacctaccgaaacgacccaacagtttattgtaaagaacgggattattaaggaggatgaactgagaggcgagaaccgtcagattcttaaggacatcatggacgattactaccgtggcttcattagtgagacccttagcagtatagacgatattgactggacgtccctgtttgagaaaatggaaattcagctgaagaatggtgataacaaggatacattgattaaagagcaaactgaataccgcaaggcgattcataagaagttcgccaacgacgaccgcttcaagaatatgttctctgccaaattaataagcgacatcctgcccgagtttgtaattcacaacaataattattcggcatctgagaaagaagagaaaacgcaggtcatcaaactgtttagtaggttcgctacgtcattcaaggattatttcaagaatcgcgcaaattgcttctccgctgatgacatcagttcctcttcatgccacaggatcgtgaatgacaatgcagagatatttttctccaatgccctagtttaccgccgcatagtgaagagtctgtcgaatgacgacatcaataagatctccggtgatatgaaggattctttgaaggagatgagcctggaagagatctactcttatgagaaatatggcgaattcatcacccaggagggcatatcgttctacaatgatatctgtgggaaggtcaatagcttcatgaacttatattgtcaaaagaataaggagaacaagaacctctataaactgcagaagcttcataagcaaatcttatgcattgccgacaccagctacgaagtgccttacaagtttgagtccgatgaagaggtttaccagtccgtgaatgggtttctcgacaatatttcatcaaagcacatagttgagagactccgaaagatcggtgacaattataatgggtataacctggataagatctacattgtgagtaaattctatgaatcggtgagccaaaagacttacagggactgggagactatcaatactgcgctggagatacattataacaatatcctacccgggaacggcaagagcaaagcggacaaagtgaagaaggcagtgaagaacgacttacagaaatctatcaccgaaataaatgaactcgtgagcaattacaagttgtgttcagacgacaatattaaggcagagacctatattcatgagatctcacacatcctgaataactttgaggcacaggagttaaagtataaccctgaaatccacctggtggaatctgaactcaaagcctcagagttgaagaatgtgctggatgtcattatgaacgccttccactggtgcagcgtgttcatgacagaggagctcgttgacaaagacaataacttctacgctgagctcgaggagatctacgatgaaatttatccagtcatctccctttataatctggttcggaactatgtgacacagaaaccctacagcaccaagaagattaagctcaacttcggcatacctacccttgccgacggctggtccaagagcaaggaatactctaacaacgccataatcctaatgcgcgataacctgtattatctaggaatatttaacgcgaagaataagcccgataagaagatcattgagggtaacacctcggagaataagggagattataagaagatgatttacaacctcctgccaggacccaataagatgataccgaaagtctttctgtcctctaagactggcgtggaaacctacaaaccctctgcctatattctggaaggctataaacagaacaagcacattaaatcatcgaaggactttgatattacgttctgtcatgatttaattgactactttaagaattgcattgcgattcatcctgaatggaagaactttgggtttgacttctccgatacttcaacctatgaggacatcagcggcttctatagagaggtagaactccagggatacaagattgattggacttacatctccgagaaggacatcgacttattgcaggagaaagggcagctgtacttatttcagatctacaacaaagacttctctaagaagtctaccggaaatgataatctgcatactatgtatttgaagaacctcttcagcgaggagaaccttaaggatattgtgctgaagttgaacggtgaggccgagatcttcttccgaaagagctctattaagaacccaattattcacaagaaagggtccatcctggtgaacagaacctacgaggctgaggagaaagatcagtttggtaatatacagattgttagaaagaacatccctgagaatatctaccaggaattgtacaagtactttaacgataagtcagataaagagctaagcgatgaggccgccaagttgaagaatgtcgttggtcaccacgaggctgccacaaacattgtgaaggactatcgctacacatatgacaaatatttcctgcacatgccaatcacaatcaacttcaaggctaacaagacaggtttcatcaatgaccgcatactgcagtatattgcgaaagagaaagatttgcatgtcataggtattgaccgaggagagaggaatctaatttacgtgagcgttatcgatacgtgtggaaatattgttgagcagaagagtttcaatatagtcaatggatacgattaccagatcaagttgaaacagcaggaaggtgctaggcagattgcgcgcaaagagtggaaggagataggaaagattaaagaaataaaggaaggatatctttctctagttattcacgaaatttctaagatggtcattaagtacaatgctatcattgccatggaagacttgtcctacgggtttaagaagggacgctttaaggtagagaggcaagtctatcagaagtttgagaccatgctcatcaataagctgaactacctggtctttaaagatatcagcataactgagaatggtggcttactgaaaggttatcagttaacatatattccagataaattaaagaacgtcggacaccagtgcgggtgtatcttttatgtgccggccgcttacacgtcgaagatcgatccgaccactggatttgtcaacatctttaaatttaaagatctaaccgttgacgccaagcgcgagttcatcaagaagttcgattcaatccgttatgactccgagaaaaacctgttctgtttcacattcgactataataatttcattacacagaacactgtgatgtctaaatcttcttggtccgtttatacatacggcgtgagaattaagagacgattcgttaatgggagattctccaatgagtccgacaccattgatatcacgaaggacatggagaaaacgcttgagatgacagacattaattggagagatggccatgacctaagacaggacatcattgactacgaaattgtgcagcacatatttgagatctttaggcttactgtacaaatgagaaattccttatcagaacttgaagatcgcgattacgatcggctgatctctccagttcttaatgagaataatattttctacgacagtgccaaggccggtgacgctttgcctaaggacgccgatgccaacggcgcatactgcatcgctctgaaaggattgtacgagatcaagcaaatcacagagaactggaaggaagatgggaagttctcgcgagacaaactgaagatttctaacaaggactggtttgatttcatacagaacaagaggtatctttaa

SEQ ID NO: 248 - DNA, 3792 bp, Artificial Sequence
  Description of Artificial Sequence: Synthetic polynucleotide
atgaacaacgggacgaacaacttccagaacttcatcggtatttctagcctccaaaagactctcagaaacgccttaattcccaccgagactacacaacaattcattgtgaagaatggtattatcaaggaggacgaactacgcggagagaatcggcagatattgaaggacatcatggatgactactatagaggatttatcagtgagacgctgtcctcaatcgatgatattgactggacaagtctgtttgagaagatggagattcaactcaagaatggagacaacaaagacaccttaattaaggaacagacagagtaccggaaggccattcacaagaagtttgcaaacgatgatcgtttcaagaatatgttcagcgcaaagctgatttccgacatcctgcccgagttcgtgatccataacaataattactcggcatcagagaaagaagagaaaactcaggtaatcaaattgttctcacgattcgccacctctttcaaagactacttcaagaatagagcgaactgtttctccgctgacgacatttcatcaagtagctgtcaccgcattgtgaatgacaacgcagaaatcttcttcagcaatgctcttgtctaccgcaggattgtaaagagcctgtcaaacgatgacatcaacaagattagtggagacatgaaagactccttgaaagagatgagcctggaagagatttactcctacgagaaatatggtgaatttattacccaggaaggcatcagtttctacaatgacatctgtggtaaggttaactccttcatgaatttgtattgccaaaagaataaagagaacaagaacttgtataagctccagaagctccataaacagattctttgcatcgccgacaccagctatgaggttccctataagttcgaatctgacgaagaggtgtatcagagcgttaacgggttcctcgacaatatttcatctaaacacattgtggagagactgaggaagataggagataactacaacgggtacaacctagataagatttacatcgtgagcaaattctacgagtccgtgtcacagaagacttatagagattgggaaactattaacacggcgctagagatacattataataatatcctgccaggaaatgggaagtctaaggcagacaaggtaaagaaggctgtgaagaatgacctgcagaagtccataacagaaataaacgaactggtgagtaactataagctgtgctctgatgataatatcaaagcagagacttacatccatgagatctctcacattctcaacaacttcgaggcacaggagctgaagtacaatcccgagattcacttagtcgagtccgagttgaaagcttctgaactgaagaatgttctagacgttatcatgaacgccttccactggtgttctgtgttcatgaccgaagagcttgtcgataaagacaacaatttctatgctgaactggaggagatctatgacgagatttacccagtcatatctctctataatcttgtacgcaactacgtcactcagaaaccgtactccacgaagaagattaagctgaacttcgggatacctacactcgcggacggatggtcaaagagtaaggagtactcaaataatgctataatactgatgcgggacaatttgtattaccttggtatatttaatgcaaagaacaaaccagataagaagattatagagggtaatactagcgagaataaaggcgactataagaagatgatatacaatctgctcccaggcccaaacaagatgatcccaaaggtcttcctctcatcgaagacgggtgtggaaacttataagccatccgcatacattctggaagggtacaagcagaataaacatattaagtcatctaaggacttcgatattactttctgccatgatcttatagattatttcaagaattgcatcgccattcatcccgagtggaagaacttcgggttcgacttcagcgacacctctacttatgaggatatctctggcttctatcgcgaagtggagttgcagggttataagatcgactggacctacatttctgagaaggacattgaccttcttcaggagaagggccagctgtatttgtttcagatctacaataaagacttctccaagaagtccacagggaatgacaatcttcatactatgtatttgaagaatcttttctcagaagagaacctgaaagacattgttctgaagctcaacggcgaggccgaaatcttcttcaggaagagtagcataaagaatcctatcatccacaagaagggctccatcctggtcaatcgaacttatgaggcagaggagaaggaccagttcggcaacattcagatcgtccgtaagaatattcccgagaatatttaccaggagttatataaatacttcaatgataaatctgataaagagctgtccgacgaagctgccaagctgaagaatgtggttgggcatcatgaagccgccaccaacatcgttaaggactaccgctatacatacgacaaatatttcctccacatgcctataacaattaacttcaaggccaacaagaccggtttcataaacgacaggatactccagtacatagcaaaggagaaggacctgcacgttattggcatcgaccgcggcgagagaaacctgatttatgtgagtgtgattgatacgtgtggtaatatcgtggagcagaagtcattcaacatcgtgaatgggtacgactatcaaattaaattgaaacagcaggaaggtgcaaggcaaatcgcccggaaggaatggaaagaaattggcaagattaaggaaattaaagaaggatatcttagtctggttatccatgaaattagcaagatggtgataaagtacaacgctatcattgctatggaggacctgtcctatggcttcaagaagggacggtttaaagtagagagacaggtataccagaagtttgagaccatgctgatcaacaagctgaactatctggtgttcaaagatatctccattactgagaatggcggcttacttaagggatatcagctgacttatattcctgacaagctaaagaacgtgggacaccagtgtggttgtatcttttacgtgccagctgcttatacctctaagattgatcccactactgggtttgtgaatatctttaaatttaaggacctgactgtagatgcgaagcgggagtttattaagaagtttgacagtattcgctatgactcagaaaagaacctcttctgctttactttcgattacaataacttcattactcagaatacagtcatgtccaagtcatcctggtccgtgtatacgtacggtgtgaggattaaacggaggttcgttaatggaaggttctccaatgagagtgacacaatagacattacaaaggatatggagaagacacttgagatgacggacataaactggagggatggtcatgacctacgacaggatatcattgactatgagatcgtacagcacatatttgagatatttcggctgacggtgcagatgcggaactccctctcagagctcgaagaccgcgactatgaccgtttgattagccctgtattaaacgagaacaacatcttctacgattccgctaaagctggagacgcattaccaaaggacgccgacgcaaacggtgcttattgcatagccttgaagggactctacgagatcaaacaaattactgagaactggaaggaagatggcaagtttagccgggataaattaaagatttctaataaggattggtttgacttcattcagaacaaacgctacctttaa

SEQ ID NO: 249 - DNA, 3792 bp, Artificial Sequence
  Description of Artificial Sequence: Synthetic polynucleotide
atgaataacggcactaataatttccagaatttcataggcataagcagtttgcagaagaccctgaggaatgccctcattcctactgaaaccacacagcagtttattgtcaagaacggaataatcaaagaagacgagctccgcggcgagaacagacagatactcaaagacataatggatgattactaccgcggcttcatttcagagaccttgtcatctatcgacgatattgattggacttccctgttcgagaagatggagattcagttaaagaatggcgacaacaaagataccttaattaaagaacaaaccgaataccgcaaagcaatccataagaagtttgccaatgatgaccgcttcaagaacatgttctccgcaaagttgatatcggatattttaccggaatttgtgatccataataacaactacagcgcttccgagaaagaagaaaagactcaggtgattaagctgttctcacggttcgcaaccagtttcaaggattatttcaagaaccgggcaaattgctttagcgccgacgatatctcctccagctcttgccaccgcattgtcaacgacaatgcagagatcttttttagcaatgccttggtgtatcgaagaatcgtcaagtccctaagcaacgacgacatcaataagatatccggcgatatgaaggattcccttaaggaaatgtcgctcgaggaaatttactcttacgagaaatatggcgaatttattacgcaggagggaatttccttctataacgatatatgcggcaaggtaaactcctttatgaatctgtattgtcagaaaaacaaggagaacaagaatttgtataagctgcagaaactccacaagcagatcctttgtattgctgatactagctatgaggtgccgtataaattcgagagtgatgaagaggtctatcaatccgtgaacggcttcttagataacatctcaagcaaacatatcgtagagcggttacggaagattggagacaactataatggctataatcttgataagatttacatcgtgtctaaattctacgaaagtgtttcgcaaaagacttaccgggactgggagacaatcaacaccgcactagagatccactacaataacatcctgccagggaacggcaagagcaaagccgataaagtaaagaaagctgtcaagaacgacctgcaaaagagcatcactgagattaacgaactcgtgtcaaactataagctttgctctgatgataatatcaaagcagaaacctatattcacgaaatttcgcacattctgaacaacttcgaggcacaggaactcaaatataatccggagatccacctggtggagtctgagctgaaagcatctgagttaaagaatgtacttgacgtgatcatgaatgcattccactggtgctccgtgtttatgaccgaggaactggtcgacaaggacaacaatttctacgcggagctggaagagatatacgacgaaatataccctgtcatttcactttataatctggtgcgcaactatgtcacccagaaaccatattcaaccaagaagatcaagctgaatttcggcatccctacgcttgcagatggttggtctaagtctaaggagtattccaacaacgctatcattctcatgcgtgataacctctactacctcgggatctttaacgctaagaacaagcctgataagaagattattgagggaaatacatcggagaacaaaggagattacaagaagatgatatataatctgctgccgggaccgaataagatgatccctaaggtgttcctgagttcgaagaccggtgtcgagacctataagccaagcgcttacattctcgaaggctacaagcagaacaaacatataaagagtagcaaagatttcgacataactttctgccatgatttgattgactattttaagaactgtattgcgattcacccagaatggaagaacttcggcttcgactttagtgatactagcacatacgaggacatttcgggattctacagggaggtggaactgcagggatacaagatcgactggacgtacatctctgagaaggatatagatctccttcaggagaagggtcagttatacctgttccagatctataacaaggacttctcaaagaagtctactggaaacgacaatctccacactatgtaccttaagaatttattcagtgaggagaatctcaaggacattgtgctcaagctgaacggagaagccgagattttctttcgcaagagttcgatcaagaaccctattattcacaagaaaggcagtattctggtgaacagaacttacgaagccgaggagaaggaccagttcggtaacattcaaattgtccggaagaacattcccgagaatatataccaggagttgtataagtactttaatgacaagagtgacaaggaactcagcgacgaagccgccaaacttaagaacgtggttggtcatcacgaggccgcaactaatatcgttaaagattataggtacacctacgacaagtatttcctgcacatgcccataacaatcaactttaaggcaaacaagactggctttatcaatgaccggattctccaatatatcgccaaggagaaggacctccacgtgattggtatcgaccggggtgaaagaaacctaatttatgtgtccgtgatagacacttgtgggaacattgtcgagcagaaatccttcaacatcgtaaatggatacgactatcaaataaagcttaagcagcaggagggagcccggcagatagctagaaaggagtggaaagagattggtaagattaaggagataaaggaagggtacttgagccttgtcattcacgaaattagcaagatggttattaaatacaatgctattatcgcaatggaagacctgtcctacggctttaagaaagggagattcaaagttgagagacaagtgtatcagaaatttgagactatgcttatcaataaactcaactacctggtgttcaaggatataagtatcacagagaatggcgggctccttaagggctatcagctgacatatatcccagacaagcttaagaatgtaggacaccagtgcggatgcatattctacgttcccgcagcctacacatccaagatcgatccgactaccggcttcgtgaatatctttaaattcaaagacctcacagtcgatgccaagagagagttcataaagaagttcgattctattaggtatgacagtgaaaagaacctattctgctttactttcgattacaacaactttattacacagaataccgtaatgtctaaatcttcttggtccgtgtacacatatggcgtgcggatcaagaggcggtttgtgaacggacggttctctaacgagagtgacaccatcgacatcactaaagacatggagaagaccttggagatgaccgatatcaattggagagatgggcatgacttgcgtcaggatattatcgattacgagatcgtgcagcacatatttgagatctttcgattaacggtgcaaatgcgcaacagcctatcagagctggaggatagggactacgatcggttaatatctcccgtacttaatgagaataacatattctatgactcggctaaagcaggcgatgctttacccaaggacgctgacgcaaatggcgcctactgtatagctcttaagggcttgtatgagatcaagcagatcacagagaattggaaagaggatgggaagttctctcgtgacaagctcaagatcagtaataaggactggtttgactttatccagaataagagatacctgtga

SEQ ID NO: 250 - DNA, 3792 bp, Artificial Sequence
  Description of Artificial Sequence: Synthetic polynucleotide
atgaataatgggacgaataatttccagaatttcatcggtatatcctcactgcagaagaccctgagaaatgctcttatacctaccgagacaacgcaacagtttatcgtgaagaatggaataataaaggaggatgagcttcgtggtgagaaccgccaaatattaaaggatatcatggacgattattatcgcgggtttatttcagagacactgagctccattgatgacatcgactggacctcactcttcgaaaagatggagatccagctcaagaacggcgataataaggacacactcatcaaggagcagaccgaataccggaaagcaattcataagaagtttgccaacgatgaccggttcaagaatatgttctccgctaaactgatttcggatatcctgccggagttcgtcattcacaataacaattattcggcaagcgagaaagaggagaagactcaagtgatcaagctgttctccaggttcgccacttctttcaaggattactttaagaacagggccaattgtttcagcgccgatgacatctcgtcttcctcttgtcaccggatcgtgaatgacaatgccgagatatttttctcaaatgctctggtatacaggaggatcgtgaagtctttatctaacgatgatattaacaagatttccggcgacatgaaagattctctcaaggaaatgagcctggaggaaatttactcttacgagaagtacggcgagtttatcacacaggaaggcatttcattctacaatgatatatgcggcaaagtaaactcattcatgaacctctattgccaaaagaataaggagaacaagaacttgtacaagttgcagaaacttcacaagcagatactgtgtatcgctgacactagttatgaggtaccatacaagttcgaatcagatgaagaggtataccagagtgttaatggtttcctggacaacatctcatcgaagcatattgtggaaagactgcggaagattggcgacaattataatgggtacaaccttgacaagatctacatagtttctaaattctacgaaagtgtctcacagaagacataccgcgattgggagactatcaataccgcgctcgagattcattataacaatatactgccgggaaacggaaagagcaaagccgacaaggtcaagaaggctgttaagaatgatctacaaaagagtatcacagaaatcaatgaactcgttagtaattacaagctctgttctgacgacaatatcaaagccgaaacctatatacacgaaatcagccacatcttgaacaacttcgaggcccaagaactgaaatataatccggagattcatctggtcgaaagcgaactcaaggccagtgaacttaagaacgtgcttgatgtgatcatgaatgcctttcactggtgtagtgtcttcatgactgaagagctggtggacaaggataacaacttctacgcagaattggaggaaatctatgatgagatctatccagtcatttctctgtataacctggtcaggaattacgtcactcagaagccatactcgaccaagaagattaaattgaactttggcatccctaccctggcagatggttggagcaagtctaaggaatacagcaacaatgccatcatactgatgagggataacctctactacttgggcatcttcaatgcgaagaataaaccagacaagaagatcatcgaaggcaatacgtcagagaacaagggtgattataaaaagatgatttacaatctgctacctggccctaacaagatgatcccaaaggtgttcctgtctagcaagaccggagtggaaacatataaacctagcgcctacatccttgagggatataagcagaataaacacattaagtcttctaaagatttcgatattacgttctgccatgacctgatcgactactttaagaattgtatcgccatacatccagagtggaagaacttcggctttgatttctccgacacatcaacttatgaggacatttctgggttctatcgcgaagtggagctacagggctataagattgactggacttacataagtgagaaagacatcgacttgctgcaggagaagggtcaactttatctcttccaaatttacaacaaagacttcagtaagaagtcaactggtaatgacaatctccacaccatgtacctaaagaacctgtttagcgaggagaatctcaaggatatcgtcttgaagctgaacggagaggctgaaatattcttccgaaagtcctctataaagaacccaattattcataagaaaggcagcatactggtgaacagaacctacgaggctgaagagaaggaccagtttggaaacattcagatcgtaaggaagaacatcccggagaacatctatcaggagctgtacaaatatttcaatgataaatccgacaaggagctttccgacgaggcagcgaaactgaagaacgtcgttgggcaccacgaagccgctactaacatagtcaaagactatagatatacatacgacaaatacttcttgcacatgcctatcaccattaatttcaaggctaacaagactggtttcattaatgaccgcatcctgcagtatattgccaaggagaaagacctgcacgttatagggattgaccggggcgagcgaaacctgatttacgtcagcgtgattgatacatgcgggaatattgtagagcagaagtcatttaacatcgtgaatggttatgactaccagattaagctgaagcaacaggagggagcgagacagattgcccgaaaggaatggaaggaaatcggtaagatcaaagagatcaaagaaggatacctgtctctcgttatccacgaaataagtaagatggtgataaagtacaatgctattatcgcgatggaagatctgtcctacggttttaagaaaggccgcttcaaggtggaacgacaggtgtaccagaagttcgagaccatgctgatcaacaaactgaactatctggtgtttaaagacatctcaatcacagagaatggaggtttactgaaaggataccagctcacgtatatcccagacaaactcaagaatgttggccatcaatgtggttgtatcttctatgttcccgccgcctacacttcaaagatcgatcccaccaccgggttcgtgaacatcttcaagtttaaagatttaacagtggacgcaaagagagagtttataaagaagtttgattcaattcggtacgattctgagaagaatctgttctgctttactttcgactataataacttcattactcagaatactgttatgtcaaagagcagttggtcggtctatacctatggcgtcagaatcaagcgtagattcgtaaatggacgatttagcaatgaatcagacacaattgatatcactaaggatatggagaagaccctggaaatgaccgacatcaattggcgcgacgggcacgacctaagacaagacattatagactatgaaatagtccagcacatattcgaaatattccgtttgactgtccagatgagaaatagcctgagcgaattggaggaccgagattacgatcgtctgatttctcctgtcctgaatgagaacaacatcttctacgacagcgccaaagcaggcgacgctctcccaaaggacgctgacgccaatggcgcgtactgcattgccctgaaaggtctgtatgagatcaagcagatcactgagaactggaaggaagacggcaaatttagtagggacaaacttaagatctctaacaaggactggtttgacttcattcagaacaagcgttatctctga

SEQ ID NO: 251 - DNA, 3792 bp, Artificial Sequence
  Description of Artificial Sequence: Synthetic polynucleotide
atgaacaacggcactaacaactttcagaatttcataggcataagttccctccagaagacccttaggaatgctcttatcccaactgaaaccacccaacaattcatagtgaagaacggcataatcaaagaagatgagttgagaggtgagaatcggcagatattgaaggacataatggatgattactaccgtggctttatttccgaaactttgtcatccattgacgatattgattggacaagtctctttgagaagatggaaattcagctgaagaatggagacaataaggacaccttaatcaaggagcagacagagtaccggaaagccatccataagaagtttgccaacgatgatcgatttaagaatatgttctctgcgaagctcatctctgatatcctgcctgagtttgtgatccataataacaactatagcgcctccgagaaggaagaaaagactcaggtcattaagctgttcagtcggttcgctacatccttcaaggattatttcaagaatcgggcaaactgcttcagtgctgacgacataagctccagcagttgccaccggatcgtgaatgacaatgctgaaatattcttctccaatgcccttgtgtatcgtagaatcgtcaagtccctctctaacgatgacatcaacaagattagcggagacatgaaggacagcctcaaagaaatgagcctggaagaaatttattcctacgagaaatatggcgagttcataacgcaggagggaatctctttctacaatgatatttgcgggaaggtcaattcgtttatgaatctgtactgccaaaagaacaaggagaacaagaatctgtacaagttgcagaaactgcacaaacagatactctgcatcgccgacacctcctacgaagtaccgtataagttcgagtctgacgaggaagtgtaccagagtgtgaacgggttcctggacaacatcagttcaaagcatatagtcgagcgactgcggaagatcggcgataactacaatggatacaacctggataagatttatattgttagcaaattctatgagtcagtcagtcagaagacgtatagagactgggagaccatcaatacggctttggagatccattacaacaacattctgccaggtaacgggaagtccaaagccgataaggtcaagaaggctgtaaagaacgacctgcagaaatctatcacagagataaacgagctggtttctaactacaagctctgtagcgatgataatatcaaagcggaaacttacattcatgagatctcacatatccttaacaacttcgaagctcaggagcttaagtacaatcccgaaatccacttggttgagagtgagttaaaggccagtgagttaaagaatgtactcgatgtgatcatgaacgcgttccattggtgtagtgtgttcatgaccgaggagctagtagacaaagataacaacttctatgccgagcttgaggagatttacgacgagatttatcctgtcattagtttatataacctggttcgcaattacgttacacagaagccttactctacgaagaagattaagcttaacttcggtattccgacattggcggacggctggagcaagtcaaaggagtacagtaataacgccataatactaatgagggataatctctactacctagggatatttaacgccaagaataagcctgacaaaaagattatagaaggcaacacttccgagaataaaggtgattacaagaagatgatttacaatcttctcccaggaccaaataagatgatccctaaggtgtttctttctagcaagactggagttgagacttacaagccaagcgcctatattctagaaggttataaacagaacaagcacatcaagtcttccaaggacttcgatataacgttctgccacgacctcatagactatttcaagaactgtatagcgattcatccagagtggaagaacttcgggttcgacttctcagataccagcacatacgaagacatcagtggcttctatcgggaggtggaactgcagggttacaagatcgattggacttacatctcagagaaagatattgatctgcttcaggagaagggacaactctatctctttcagatctataacaaagatttctccaagaagtcgacaggaaacgataatctgcacaccatgtacctcaagaacttgttctccgaggagaatctgaaagacatcgtgttaaagctgaatggtgaagccgaaatattcttccggaagtcatctataaagaatccaatcatccataagaaaggtagcatactcgtgaacaggacctacgaagccgaagagaaagaccaattcggcaacattcagatcgtccggaagaacattcccgagaatatctatcaggagctgtataaatactttaatgataagtcggataaagagctcagcgatgaggctgcgaaactcaagaacgtcgtcggccatcatgaagccgcaacgaatattgtgaaggattacagatatacttacgataaatatttccttcatatgcccataaccatcaatttcaaagccaacaagacagggttcattaatgatcggattctccagtatatcgccaaggagaaggatctccacgtcattggaatagaccgcggtgagaggaatttaatttatgtctctgtcattgacacttgcggcaatatagtcgagcagaagagcttcaacatcgtgaatgggtacgattatcagatcaagcttaagcaacaagaaggagcgcgccagatcgctaggaaagaatggaaggagatcggcaagatcaaggaaatcaaggaagggtacttaagcctggtaatccatgagatttcgaagatggtcattaagtataatgctatcatagctatggaggacctgtcctacgggttcaagaaaggcaggtttaaagtggagcgccaggtgtaccagaagttcgagactatgctaatcaacaagctcaattatctggtgttcaaggacatctcaatcacggagaatggaggcctgctgaaagggtaccaattaacttacattcctgataaactgaagaacgtgggccaccaatgcggatgcatcttctatgttccagccgcatatacatccaagattgatcccactaccggattcgttaacatcttcaagtttaaagatctgacggtggacgcaaagcgcgaattcatcaagaaatttgattcaattcgttatgacagcgagaagaatctattctgctttacctttgactacaataacttcataactcagaataccgtgatgtctaaatcatcttggtctgtgtatacctacggtgtgagaattaagaggaggtttgttaatggcaggtttagcaacgagtccgacactatcgacatcacgaaggacatggagaagactttggagatgacggacatcaactggcgagacgggcatgatctccgacaggacatcattgattatgagatagtccaacacatctttgaaatcttccggctgactgtccagatgcgcaattccctgagtgaattagaagatcgcgattatgatcgtctgatcagcccagtgttaaatgagaacaatattttctatgattcagctaaggctggtgacgcattacctaaggacgctgatgcaaacggtgcatattgtatagccctgaagggcctgtatgagatcaaacagatcacagagaattggaaagaggatgggaaattctctcgggataagcttaagatttccaacaaggactggttcgatttcattcagaacaagaggtacctgtaa

SEQ ID NO: 252 - DNA, 3792 bp, Artificial Sequence
  Description of Artificial Sequence: Synthetic polynucleotide
atgaataatggcaccaacaatttccagaactttataggtatctctagccttcagaaaaccctaagaaacgcactcattccgacagaaaccacacaacagtttattgtgaagaatggaatcataaaggaggacgaattgcgtggtgagaatcggcagatactgaaggatataatggatgactattaccgcggcttcatttctgagaccctgagtagtatcgacgacatcgactggacatccctattcgaaaagatggaaatccaacttaagaatggtgacaataaggataccctcataaaggagcagacagagtatagaaaggcgatacacaagaaattcgcaaacgacgatcggttcaagaatatgttctcggccaaattgatatctgacatacttcccgaattcgtaatccacaataataactattctgctagtgagaaagaagaaaagacccaggtcatcaaactcttctcccggttcgccacatcattcaaagactactttaagaaccgggcaaactgtttctccgccgacgatatatctagttccagttgtcaccgcatcgtgaacgataatgcagagatattcttcagcaatgctctggtgtataggagaatcgtgaaatcgttgagcaacgatgacatcaataagatctccggcgatatgaaggatagcctgaaggaaatgtcccttgaggagatctattcttatgagaaatacggtgaatttatcacacaggagggcattagtttctataatgatatatgtggcaaagtgaactcctttatgaacctctactgtcagaaaaataaagagaacaagaacctctacaagcttcagaaacttcacaaacagatactgtgcatcgcagatacctcatacgaggtgccatacaagttcgagagcgacgaggaggtgtaccagagtgttaatgggttcctcgataacatctcgtcaaagcacattgttgaacggctgcgcaagattggagataattataatggttataatctggataagatatatatcgtgtccaagttctacgagtccgtatcccaaaagacctaccgggattgggagaccatcaacaccgcactggaaatccactacaacaacattctgccaggaaatggcaagagtaaagcagacaaggtcaagaaagccgtgaagaatgacttgcagaagtccattaccgagataaacgagctggtatctaactataaactttgttccgatgataatatcaaggccgaaacctacatccatgaaatctctcatatcttgaataacttcgaggcccaggagctcaaatataatccagagatacaccttgtcgagagcgagcttaaggcgtcggagctcaagaacgtgctggacgtgatcatgaatgcgtttcactggtgtagcgtctttatgacggaagaactagtggataaagataataatttctacgcagagctggaggagatatatgacgagatctacccagtcatttcactgtacaaccttgtcagaaactatgttacccagaaaccatactccactaagaagattaagctgaacttcggtattcctaccttggccgatggttggtctaagtccaaagagtacagcaacaacgctatcatcttaatgcgggacaatctgtactatcttggcatctttaatgcaaagaataagcccgacaaaaagattatagagggcaataccagtgagaacaagggcgactataagaagatgatttataatctgctgccaggtccgaacaagatgataccaaaggtctttctttcctcaaagactggtgtggaaacatacaagccttccgcttacatcctcgagggctacaaacagaacaagcatatcaaatcgagcaaagacttcgacattacattctgccatgacctgatcgattacttcaagaattgcatcgctatccaccctgaatggaagaacttcggattcgacttctcagatacatccacttacgaggacatttctggcttctacagggaagtcgagctccagggttataagatcgactggacatacatctcagagaaagacattgacctgctacaggagaaaggacagctgtacctgtttcagatctataataaagacttcagcaagaagtctactggtaacgacaacttgcacactatgtatctgaagaatctcttctccgaggagaatttgaaggatatcgtgctgaaactcaatggagaggcagaaatcttcttccggaagagctcaataaagaatcctatcattcataagaaaggctctatattagtcaaccgaacatacgaggctgaagagaaagatcaattcgggaacatacagattgtgcgaaagaacattcccgagaatatctaccaagagctatacaagtactttaatgataagtctgataaggagctgagcgatgaggcagctaaactcaagaatgtcgtgggtcaccatgaagcagcaaccaacattgtcaaagactacagatacacatacgataagtatttccttcacatgccaattacaattaacttcaaggctaataagactggctttataaatgacagaatcttacagtacattgccaaggagaaagacttgcatgtcattggaatcgatcggggtgaaaggaatcttatatacgtaagcgttattgatacgtgtggaaacatcgtggaacaaaagagctttaacatcgtaaatggatatgactaccagattaagctgaagcagcaggaaggagcccgccagatcgctcggaaggaatggaaagaaataggaaagattaaggaaataaaggagggttacttgtctctggtgatccatgaaatctcaaagatggtcatcaagtataacgcgatcatagctatggaagacctgtcctacgggttcaagaagggtagatttaaggtcgaacgccaggtttaccagaaattcgagaccatgctaattaataagctgaattatctcgtgtttaaggacatcagtataactgagaacggaggcctcctgaagggataccagctgacgtacatacccgacaagctaaagaatgttggacaccagtgcggatgcatattctatgttcccgcggcatatacttccaagatcgatccaacaaccggctttgtgaacatcttcaagtttaaagatctgaccgtcgatgcgaagagagagttcataaagaaatttgacagcataaggtacgatagcgagaagaatctattctgtttcacctttgactacaacaatttcatcacccagaacacagtgatgtctaagtcttcctggtccgtgtatacgtacggtgtaaggattaagaggcgctttgttaacggtcggttctccaacgaatctgacacgatagacatcacaaaggacatggaaaagacacttgaaatgaccgatattaactggagagacgggcatgatctgagacaggatattatcgattacgaaatcgttcagcatatattcgagatctttaggctgacggtccagatgcgcaacagcctgtcggagctcgaggatagagactatgatcgcttaatcagcccagtactgaatgagaataatatattttacgactctgctaaagcaggagatgcccttccaaaggatgccgatgcaaatggagcctactgtattgcattaaagggcttatacgagattaaacagatcactgagaattggaaggaagacgggaaattctcacgggataagcttaagatttctaataaggattggtttgacttcattcagaacaagcgatacctgtaa

SEQ ID NO: 253 - DNA, 3792 bp, Artificial Sequence
  Description of Artificial Sequence: Synthetic polynucleotide
atgaataatgggacaaacaacttccagaactttattggcataagcagcctccagaagaccctacgaaatgctctcatcccaacagagacaacccagcagtttattgtaaagaacggcataattaaggaggatgaactgcgcggcgagaataggcagatcctaaaggatatcatggacgattactatcgtgggttcattagcgaaaccctttcctcaatagacgacatcgattggacatccttgttcgagaagatggagatccagctcaagaatggtgacaataaagatacgctgataaaggagcagacagaatacagaaaggccatccacaagaaatttgccaacgatgaccgatttaagaatatgttctctgccaaactaatatctgacatccttcccgaatttgtcattcacaacaataactacagcgcctccgagaaggaagagaagactcaagtgatcaagttatttagtagatttgcgacatccttcaaggactactttaagaacagggccaactgcttctcagccgacgacatttcatcatcttcctgtcacagaatcgttaacgataacgctgagatattcttctcaaatgccctggtgtacaggcgtattgtgaaatcactgtccaatgatgatattaataagatctccggtgatatgaaggactcattaaaggagatgagcctcgaagagatttactcatacgagaaatacggtgaattcattacccaggagggcataagtttctacaatgacatttgcggcaaagtgaatagctttatgaatctgtactgtcagaagaacaaggagaacaagaatctgtataagctgcagaagttgcataagcaaatactgtgtattgctgatactagttatgaggttccgtacaagtttgaatcggacgaggaagtttatcaatccgtgaacggtttcttagacaacatttcgagtaaacatatcgtagaacgactgaggaagattggcgacaactacaatggctataatcttgacaagatttacattgtatccaagttctatgaaagtgtctcacaaaagacctatcgagactgggagaccattaacactgccttggagattcactacaacaacattctgcctggcaatgggaaatccaaagctgataaagtcaagaaggccgtgaagaatgacctgcagaagtccataaccgagatcaatgagctggtttcaaattacaagttgtgctccgatgacaacattaaagctgaaacctacatccacgaaatctctcacatcctcaataacttcgaagcccaagagctgaagtataatcccgagattcacctagtggagagcgagctgaaggctagtgaactcaagaacgtactggacgtaataatgaacgcgtttcactggtgctccgtcttcatgaccgaagaattggttgacaaggataataacttctacgccgagcttgaggaaatatacgacgagatctatcctgtcatctctctgtacaacctcgtaaggaattacgtgactcagaaaccgtacagcacaaagaagattaagctgaacttcgggatccctacactggctgatgggtggtctaagtccaaggaatactccaataatgccatcatcctcatgagggacaacctgtattacctaggcatattcaacgccaagaacaaacccgacaagaagataattgaaggaaacactagtgagaataagggcgattacaaaaagatgatttataatctgctacccgggcctaacaagatgattccaaaggtctttttaagtagtaagacaggagtggagacttacaagcccagtgcatacatccttgaaggctataagcagaataagcacataaagagctccaaggacttcgacattaccttctgccatgacctgattgactacttcaagaattgcattgccatccatccagagtggaagaacttcgggtttgactttagtgatacttctacgtatgaggacatcagtgggttctatcgggaggtcgagctgcagggttataagatcgattggacctacataagcgagaaggacattgacctgctacaggagaaaggccagttgtacctgttccagatatataacaaggacttctctaagaagtcaacaggaaacgacaatttgcacaccatgtaccttaagaaccttttctctgaggagaatctgaaggacatagtgcttaagcttaacggcgaggccgaaatattctttcggaagagctcaatcaagaatccgataatccataagaaaggctcaattctagtgaacaggacatatgaggcagaagagaaagaccagttcgggaacattcagattgtcagaaagaatatacccgagaatatataccaggagctgtataagtatttcaacgataaatccgacaaagaactatcagatgaggcagcaaagcttaagaatgtggtaggacaccacgaagcagctaccaatatagttaaggattatagatacacttacgataagtacttcctgcacatgccaataacaattaatttcaaagccaataagaccggattcataaacgataggatactccaatatattgcaaaggagaaagacctgcatgtgatcgggattgaccgtggcgagcggaatcttatttacgtgtccgtgattgacacatgtggcaacatcgtggaacagaaatccttcaacattgttaacggctatgactatcagattaaactgaagcagcaggaaggagcacggcagattgctcggaaagagtggaaagagataggtaagattaaggaaatcaaggagggctatctgtcgctggtgatacatgagatctcaaagatggttatcaaatacaacgccatcattgcaatggaggacctctcatacgggtttaagaaaggaaggttcaaggtggaaaggcaagtgtaccagaagttcgaaacaatgcttatcaacaagctcaactacctcgtgttcaaggatataagcatcaccgagaatggcgggttactgaagggctatcagttaacctatataccggataaactgaagaacgtgggtcaccagtgcggatgtatattctacgtccctgcagcatatacgagtaagatcgacccaaccaccggatttgtgaatatattcaagttcaaggacctgacggtcgatgcgaagcgcgaattcattaagaagttcgattcaatccggtatgacagcgaaaagaacctgttctgctttacgttcgattataataatttcattactcagaataccgtcatgagcaagagctcctggtcagtgtacacctacggtgtgagaatcaaacgccgatttgttaatgggcggttcagtaatgagtctgacaccattgacattactaaggacatggagaagacactggaaatgactgatatcaactggagggatggccatgatctacgacaggacatcatagactatgagatagtacagcatatctttgagatctttagacttactgtacagatgaggaatagcctgagtgaacttgaagatcgcgactacgaccgcctcattagtcctgttctaaatgagaataacatattctacgattccgcgaaagcgggcgacgcattgcctaaagacgccgacgccaatggagcatattgcatcgcacttaaaggtctctatgagattaaacagatcactgagaactggaaggaagatgggaagttctcccgggataagctaaagatttccaacaaagactggtttgatttcattcagaacaaacgatatttgtga

SEQ ID NO: 254 - DNA, 3792 bp, Artificial Sequence
  Description of Artificial Sequence: Synthetic polynucleotide
atgaacaacgggactaacaactttcagaacttcattggaattagcagtctgcagaaaaccctacggaacgcccttattcctacagagaccacccagcagtttatagtcaagaatggtattatcaaggaggatgagttacgtggcgagaatcggcaaatcctcaaggacatcatggatgactactatcgcggctttatttctgagacactgtcctcaatagatgacattgactggacaagtctgtttgagaagatggaaatccaactcaagaatggtgataataaagatacactgattaaagaacagacggaatacaggaaagcaatacataagaagtttgctaacgacgaccgatttaagaatatgttctcagcgaagttaatttctgacatcctcccagagttcgtcatacacaataacaattacagtgccagcgagaaagaggagaaaacacaggtaattaagcttttctctcggttcgctacctctttcaaagactattttaagaatcgtgccaactgtttctcagcggatgacatctcgtccagctcctgtcacagaattgtcaatgataacgccgagattttcttctctaacgccttagtctacaggcggattgtgaagagcttaagcaacgatgatataaataagattagcggtgacatgaaggactcgctcaaggagatgtctcttgaagagatctacagctacgagaaatacggcgaatttattacacaggagggaatctccttctataacgacatctgcggcaaagtaaactcattcatgaacctctattgccaaaagaataaagagaataagaatctatacaagttacagaagctacacaaacagatactgtgtatcgccgacacctcttacgaggtaccttacaagtttgaatcagacgaagaggtctaccagtctgtgaatggtttcctggacaatatttccagtaagcatatcgtcgagagactccgaaagatcggagataactacaatgggtataacctcgataagatatacatcgtatctaagttctatgaaagtgtctcccagaagacttatagagactgggagaccattaacaccgcattggagatccactataataatatcctgcccgggaatggcaagagtaaagcggacaaagtgaagaaggccgtgaagaacgatttgcaaaagagtatcaccgaaatcaacgagctggtaagcaactataagctgtgctctgatgacaatattaaggctgagacctatattcacgaaatttctcatattctgaataactttgaggcacaagaacttaaatataatccagagatccatctggtcgagtccgaactgaaagcaagcgagttgaagaatgtgctggacgtaattatgaacgcgttccactggtgttctgtattcatgaccgaagagttggtagacaaagacaataacttctacgccgagctcgaagaaatctacgacgagatctatccagtcatttccctttacaacctcgtccgcaactatgttacacagaaaccgtattctactaaaaagataaagctgaacttcgggattcctacactcgcagatggttggagtaagagtaaggaatattctaataacgctattatattgatgagagacaacctgtactatctcgggatctttaacgcgaagaacaaacccgataaaaagattatcgaaggtaatacaagtgagaacaaaggcgattataaaaagatgatttacaatttactgccagggcccaacaagatgattcccaaggtgttcctgagctccaagaccggcgtggagacctataaacccagcgcttacatccttgaaggctacaagcagaataagcacattaagagctccaaagacttcgacattacattctgccacgacctgattgactacttcaagaactgcatcgccatacatccggaatggaagaatttcggctttgacttcagcgacaccagcacatatgaggatatatcaggtttctatcgggaggtggagctgcagggctataagatcgactggacatacatctcagagaaagatatagatctgctccaggagaaaggacagctatacctatttcagatctataataaggacttctccaaaaagagcactggaaatgacaacctccatacaatgtaccttaagaacctcttctctgaggagaatctgaaggatattgttctgaaactcaatggtgaggctgagatcttctttcgaaagagtagcatcaagaacccaattatccataagaaaggctctatcttggtgaatagaacgtatgaggccgaggagaaagatcagtttggtaacattcagatcgtgcggaagaacataccagagaatatttaccaagagctctataaatacttcaacgacaaatctgacaaggaactgtcagacgaagctgccaaactgaagaatgtggttgggcaccacgaagccgccaccaacatcgtcaaggattaccggtatacctatgacaagtatttcttgcacatgccaattactataaactttaaggcgaataagaccgggtttatcaacgatagaatccttcaatacatcgccaaggagaaggacctccacgttattggtatagatcgcggtgaacgcaacttaatttacgtcagtgttattgacacatgcggaaatatcgtagaacagaagagcttcaacatcgttaatgggtacgattatcagatcaaactgaagcaacaggagggagcaaggcagatcgctcgcaaggaatggaaagaaatcgggaagatcaaagagattaaagaagggtacctttccctagtaattcacgagatttctaagatggtgatcaagtacaacgccattattgctatggaagatctgtcctacgggttcaagaaaggacggtttaaggtggagcgccaggtgtatcagaagttcgagacaatgctcattaacaaactgaattaccttgtattcaaagatattagcattaccgagaatggcgggctgttgaagggatatcaactaacttatatacctgataaacttaagaatgtcggtcaccagtgcggctgtatcttctacgtgccagcagcctacacgagcaagattgacccgacaactgggtttgtgaatatatttaagttcaaggaccttaccgtggatgcaaagagggagtttataaagaaatttgacagtatccggtacgactcagagaaaaatttgttctgcttcaccttcgattacaataacttcattacccagaacactgtaatgtctaaatcatcttggtctgtgtacacatatggcgtgaggatcaagagacgctttgtgaatgggagattctccaacgaatccgacacgatcgacataactaaggacatggagaagacgctagaaatgactgacatcaactggcgagatgggcatgatctgcgacaagatattatcgattatgagattgtacagcatatcttcgagatattccgactgacagtacagatgagaaactctctgagtgagctggaggatcgtgattacgaccgtttaatcagccctgtgttaaacgagaacaatatcttctacgattctgctaaggccggagatgctcttcccaaagacgctgatgctaatggcgcgtactgtatagctttgaaaggactgtatgaaatcaaacagattacagagaactggaaggaggacggcaagttcagtagagataaattaaagatttccaacaaagattggtttgatttcatacagaacaagcggtacctgtaa

SEQ ID NO: 255 - DNA, 3792 bp, Artificial Sequence
  Description of Artificial Sequence: Synthetic polynucleotide
atgaataacggcactaataactttcagaactttattggaattagtagcctccaaaagacgctaaggaacgcattaatccctacagagaccacgcagcagtttatcgtcaagaacggcatcattaaagaagatgaactcagaggggagaataggcagatcctcaaggacataatggacgattattacaggggctttatctccgaaacactttcctctatagatgacatcgactggacatccttgtttgagaaaatggaaatccagcttaagaatggcgataacaaggataccctcattaaggagcagacagagtataggaaggccatccataagaagttcgccaatgacgacaggtttaagaacatgttctccgcaaagctgatctccgacatcctacctgagtttgttatccataacaacaattattctgctagtgagaaagaagagaaaacacaggtgattaagctctttagccgattcgcaacgtcatttaaagattactttaagaatcgggcaaattgtttcagcgcagacgacataagctcctcaagctgccaccgaattgtgaatgataacgccgagattttctttagtaacgcactagtgtaccggcggatcgtgaagtcgctcagtaatgacgatatcaacaagatctcgggcgacatgaaggatagcctcaaggaaatgagcctggaggagatttatagttatgagaagtatggcgagttcattactcaggagggcatcagtttctacaatgacatttgtgggaaggtgaactctttcatgaatttgtactgtcaaaagaacaaagagaacaagaatctctataaattgcagaagctccataaacaaatactctgtatagcggacacatcttatgaagtgccctataaatttgaaagtgacgaggaagtgtaccagagtgtcaatgggtttctggataatatctcctccaaacatatagttgagcgcctgcgaaagatcggagacaactacaatggttataatctggataagatttatatcgtttccaaattctatgagtcagtttcacagaagacctaccgggattgggaaactatcaacacagctctggaaatccactacaataacattctgcccgggaatggaaagagcaaagccgacaaggtgaagaaggccgttaagaatgacctccaaaagagtattactgaaatcaatgagctagtcagcaattacaaactctgcagcgatgacaatattaaggcagagacgtacattcacgagataagccatattctgaataacttcgaagctcaagaacttaagtataatccagagattcacctggtggaatctgaactcaaggcatcagaactaaagaatgtattggacgtaatcatgaatgcctttcactggtgctctgtgttcatgacagaggaactcgtcgacaaggataacaacttctatgccgagctggaagaaatatacgacgagatctatcctgtcatcagcctgtacaacctggttcgcaattatgtaactcagaaaccttacagcacaaagaagatcaaactaaactttggtatcccgaccctggctgacggttggagtaagtccaaggagtacagtaacaacgccatcattctgatgagggataacctgtactacttgggtatatttaatgcaaagaacaagccagacaaaaagataattgagggcaacacatccgagaacaagggagattacaagaagatgatatataatcttctgccagggcctaacaagatgataccaaaggtgtttctcagttcaaagaccggcgtggagacttacaagccctcggcgtatatattggaaggatacaagcagaacaagcatatcaaatcttcaaaggacttcgacataacattctgtcacgacctcattgattacttcaagaattgcatagccattcatccagagtggaagaacttcggcttcgatttcagcgacactagtacatatgaagacatttctgggttctatagggaggtcgagctgcaaggctataagatcgattggacttatatctctgagaaagacatcgatcttctgcaggagaaaggtcagctctacctgttccaaatctacaacaaggatttctctaagaagtctaccggtaacgataacctccacactatgtatttaaagaacctattcagcgaggagaatctgaaagacatcgtgctgaagctgaatggcgaagctgagatattcttcagaaagagttctatcaagaatcccataattcataagaaaggttccattcttgtcaataggacttacgaggccgaggagaaggaccagtttggcaacatccagatagtgcggaagaacatccctgagaacatttatcaagagctctacaaatatttcaatgataaatccgacaaggagctctcagatgaagctgcgaagctcaagaatgtagtcggacaccatgaggctgccaccaatattgtcaaagactaccgctacacatacgacaaatacttcttgcacatgccgattacgataaacttcaaagccaacaagaccgggttcattaacgaccgaatcctccagtatatcgctaaggagaaagacctccacgttatcggaatagacagaggcgagagaaatttgatttacgtctccgtgatcgacacttgtggaaatatcgttgagcagaagtcctttaatatcgtaaacggctatgactatcagattaagctgaaacagcaggagggcgcaagacagattgctaggaaggagtggaaggagatcggcaagatcaaagaaattaaggagggatatctgagcttggtcattcatgagatttccaagatggtaatcaagtacaatgccatcatagccatggaggatctttcctatgggtttaagaaaggaagatttaaagtggaacggcaggtttaccagaaatttgagacaatgctgattaacaagctgaactatttggtatttaaagatatctccatcacagagaatggcggattgctgaagggctaccagttaacctatataccagacaagctcaagaacgtcggccaccagtgtgggtgtatcttctacgttcctgccgcttatacaagcaagatagacccaaccacagggtttgtgaatatcttcaaattcaaggatttaaccgttgatgccaagagagagttcatcaagaagttcgactccattcgatacgactctgagaagaacctattctgcttcaccttcgattataataactttattacccagaataccgtcatgagcaaatcctcatggtcagtctacacttatggtgtgagaatcaagagaaggttcgtgaatggacgattcagtaatgaatccgacactattgacatcaccaaagatatggaaaagacgctggagatgaccgacatcaattggagagacgggcatgacctccgtcaggatataattgactacgaaatcgtgcagcatatatttgaaatatttcggcttaccgtgcaaatgcggaatagcctttccgaactggaagaccgagactatgatcgattaattagccccgtcctgaacgagaataacatcttttacgacagtgccaaagctggtgatgccctgccgaaagatgccgatgctaatggtgcatattgtatagcccttaaaggtctctacgaaattaaacaaatcacggagaattggaaggaggatggcaaattctctagagacaaactgaagatcagtaacaaggactggttcgatttcatccagaataaacgttatctgtga

SEQ ID NO: 256 - DNA, 3792 bp, Artificial Sequence
  Description of Artificial Sequence: Synthetic polynucleotide
atgaataacgggaccaataacttccagaacttcatcgggatctcctctctccagaaaaccctaagaaatgcactgattcccacagagacgacccagcagtttatcgtcaagaacgggatcattaaagaggatgagctgcgtggagagaataggcagatcttaaaggacatcatggatgactattaccgagggtttatcagcgagaccctttccagcatagatgacatcgactggacctccttgttcgagaagatggagatacagttgaagaatggcgataataaggatactctgattaaagagcagaccgaataccgcaaagccatccacaagaaattcgctaacgacgataggtttaagaacatgttctctgcgaagcttattagtgacattctgcccgagtttgtgattcataacaataattattccgcatcagagaaggaagagaagacccaggtgatcaaattattctctcggttcgcgacctcattcaaagactacttcaagaacagagcaaattgtttctctgctgatgatataagctcctcgtcatgtcatagaatcgtgaatgacaacgcagaaatctttttcagcaatgctctggtgtaccgcaggatagtgaaatctttgtccaacgacgatatcaacaagatatctggcgatatgaaagactccctaaaggagatgtcattggaggagatctattcctacgagaagtacggcgagtttatcacccaagaaggaatcagcttctataacgacatttgtggtaaagtcaattccttcatgaacttatactgccaaaagaacaaggagaacaagaacctctacaagctacagaaattgcacaagcagatcctatgtattgcagacacttcttatgaggtgccttacaagtttgagagcgatgaggaagtataccagtccgtcaacggcttcttggacaatattagttccaagcacatcgtggagaggctaagaaagattggagataactataacgggtataacctggataagatttacatcgttagtaagttctacgaatctgtgtctcagaagacctacagggattgggagacgattaacacagcactcgagatccactataacaacattctccctggaaacgggaaatccaaggcagacaaagtaaagaaagcagtaaagaatgacttacagaaatcgatcaccgagatcaatgagttggtgtcaaactacaaactttgctccgatgataacatcaaagcagaaacctatatacacgaaatctctcacatcctgaataactttgaggcacaggaactcaagtacaacccagagatccacctagtagaaagtgagttgaaggcctctgaactgaagaatgtgctggacgtgataatgaatgcctttcattggtgtagcgtcttcatgacggaggaactggttgataaagacaacaacttctacgctgaactagaggagatttacgacgagatttacccagttatctcactctacaacctggtgcgcaattacgtcacgcagaagccttatagtactaaaaagattaagctcaacttcggtatccctaccctcgccgacggatggtctaaatccaaggagtatagcaacaacgcaatcatccttatgagagacaatctgtactacctaggtatatttaatgcaaagaataagcctgataagaagataatagaaggaaacacctctgagaataaaggtgactacaagaaaatgatttacaatcttctgccaggcccaaataagatgattccgaaggtattcttaagcagtaagaccggagtggagacatacaaaccttccgcctacatattagagggctacaaacagaataaacatatcaagagctcgaaggactttgacataacgttctgccacgatctgattgattactttaagaattgtattgcgattcatccagaatggaagaactttgggttcgatttcagtgatacaagtacttatgaggacatctccggcttctaccgagaagtggagctgcagggatacaagattgattggacttatatctcggagaaagacatcgacctgttgcaggagaagggacagctctatttattccagatatacaacaaagacttctccaagaagagtactggcaatgataacttacatacaatgtacttaaagaacctgttctctgaagagaatctgaaagacattgtactgaaacttaatggcgaggccgagatctttttcaggaaatcctctattaagaatccaatcattcacaagaaaggctccatccttgtaaatcgaacatacgaagcagaagagaaagatcagtttggcaatatccagattgtccggaagaacattcctgagaatatttaccaggaactatataaatacttcaatgataagtctgacaaggaactttccgacgaggctgctaaactgaagaatgtggttggccatcatgaagcagcgactaacattgtcaaggactaccgttatacatatgacaagtacttcctgcatatgcctatcactatcaatttcaaggccaacaagacagggttcatcaatgacagaatcttgcagtatattgctaaggagaaagatttgcatgtcatcggaatcgacagaggcgagcggaatctcatctatgtgtctgttatcgatacttgtggaaatatcgtggaacagaagtcattcaatatagtaaacggctacgactatcagattaagcttaagcagcaggagggtgcgagacagattgcccgcaaagaatggaaggaaattggtaagataaaggagatcaaggaaggctatcttagtcttgtgatccatgaaatttcgaagatggttatcaagtacaatgccatcattgccatggaagaccttagttacgggttcaagaaaggccggttcaaggttgaacgtcaggtctatcagaagtttgaaacaatgctgatcaacaagcttaattatctggtgtttaaagatatatccatcactgagaacggaggcctcctgaagggctaccagctaacctacataccagacaaactcaagaacgtgggacaccagtgtggttgcatcttctatgtgccagccgcctatacctctaagatagatccaacaaccgggttcgttaacatcttcaaattcaaggacttgaccgtcgatgcaaagcgagagttcatcaagaagtttgattctatcagatacgattccgagaagaatctgttctgtttcacatttgactataataacttcattacacagaatacggtgatgtcgaagtcttcttggtccgtgtacacttatggagtgagaatcaaacgccggttcgtcaatggaaggttcagcaatgaatccgacaccattgacatcacaaaggatatggagaaaactttggaaatgactgatataaattggcgcgacggtcatgatctaaggcaggatatcatagattatgagatcgttcagcacatatttgagatctttcgcctgacagtccagatgcgcaattctctttccgagctggaggacagggactatgatcgcctgatctcacctgtcctgaacgagaacaatattttctacgattcggctaaggctggtgatgctcttcccaaggacgcagacgcaaacggcgcatactgcatagcacttaaagggctgtatgagatcaaacaaatcaccgagaattggaaggaggatgggaagttcagccgcgataagctgaagatttccaataaggattggtttgacttcatacagaataagcgttatctttag

SEQ ID NO: 257 - DNA, 3792 bp, Artificial Sequence
  Description of Artificial Sequence: Synthetic polynucleotide
atgaataacggaactaacaatttccagaatttcatcggcatatcgagtcttcagaagactcttcgaaatgcccttattccaaccgaaaccacgcaacagttcatcgtgaagaatggtattatcaaagaggatgagctgcgcggcgagaataggcaaatactcaaggatatcatggacgattattaccgaggattcatcagcgaaacattgtcaagtattgacgatatcgactggacatccctctttgagaaaatggagatccaattgaagaacggcgacaacaaggatactctaataaaggagcagaccgagtataggaaagctatccataagaagtttgcaaacgatgatcgctttaagaatatgttcagtgcaaagctaataagcgatatactgcccgagtttgtcatccacaacaacaattattccgcgtctgagaaggaagagaaaactcaagtgatcaagctgttcagcagatttgccaccagctttaaagattactttaagaaccgggccaattgtttctctgccgacgacatctctagttctagttgccaccgaatcgtcaatgacaatgccgaaattttcttctcaaacgccctcgtttaccggcgaatagtcaagagcctgagtaacgacgacattaacaagatttccggcgatatgaaggacagtttgaaggaaatgagtctagaggaaatctatagctacgagaagtatggtgagttcatcactcaggaaggcatctcattctacaacgacatctgcggcaaggtgaattctttcatgaacctttactgccagaagaataaggagaataagaatctttataaactccagaagctccacaagcagatcttgtgcatagccgataccagctatgaagtaccttacaagttcgaatcggacgaggaggtgtatcagtctgtgaatggtttcttggacaatatatcctctaagcacatcgtggaaaggctgcgcaagatcggcgataactacaacgggtataacttggacaagatttatattgtgagtaaattctatgagagtgtcagccagaaaacctatcgagactgggaaactataaacactgccttggagatacactacaacaacatccttcccggaaatggaaagtcaaaggccgacaaggtgaagaaagcagtgaagaacgacttgcagaaatctattacagagatcaacgagcttgtgtcaaattataagctttgctcggatgataacatcaaggctgaaacctacattcacgagatttcgcacatcttgaacaacttcgaggcacaggagttgaaatacaatcctgagattcatttggtggaatcagagcttaaagcctcggagctcaagaacgtgttggatgtgataatgaatgcctttcattggtgcagtgtgtttatgactgaagagctcgttgataaggacaataatttctacgcggaactggaggagatctacgacgagatttatccagtgatcagtctgtacaatctggtaagaaattatgtgacccagaagccttactctaccaagaagattaagctaaacttcggaattcccactctcgccgacggctggtccaaatccaaggagtactccaacaacgcaattatccttatgcgggataatctgtactacttaggaatatttaacgctaagaacaaacccgacaagaagatcatcgaaggcaacacctctgagaataaaggagattacaagaagatgatttataatcttctgcccggtcccaacaagatgatacccaaggtcttcctgtcctcaaagactggtgttgagacctacaaaccgagtgcctatatcctggaaggatacaagcagaataagcatattaagagctctaaagactttgatatcacattctgccacgacctgatcgattatttcaagaactgcatcgccatccatcctgaatggaagaactttggattcgacttcagcgacacatccacttacgaagatatttcaggcttctacagagaggtggaactgcaaggctataagattgactggacgtacatctccgagaaggacattgatttgctgcaggagaagggccaactgtacctgtttcagatatacaacaaagacttctctaagaagtcaactgggaatgacaatcttcacaccatgtatctcaagaatctgttttccgaagagaacctgaaagacattgtgctcaaacttaatggtgaagcggagatattcttccggaaatcgagcattaagaacccgattatccataagaaaggctccattctggtcaatagaacatacgaggctgaagagaaagatcagttcggaaacattcagatagtgaggaagaatatccctgagaacatctaccaggaactttataagtactttaacgacaagagcgataaggaactatccgatgaagctgctaaactgaagaacgtggtaggccatcatgaggcggctactaacatcgtgaaggattatcggtatacttacgacaagtacttcttgcacatgcccataacaatcaatttcaaggccaataagacaggcttcatcaatgacaggatacttcaatacatagctaaggagaaggacctgcacgtgattggcattgaccggggggagcgcaaccttatatacgtgtctgtgatcgacacatgcgggaacatagttgagcagaagtcattcaacattgtgaacgggtatgattaccaaatcaaactcaagcagcaggagggtgccaggcagattgcacgaaaggaatggaaagagataggtaagattaaggaaatcaaggaaggatatttgtctctggtcatccacgagatcagcaagatggtgatcaaatacaacgcaatcatcgccatggaagacctcagctacggatttaagaaaggacgcttcaaagtagaacgccaagtctatcagaaatttgagaccatgttaatcaacaagttaaattacctggtgttcaaggatatctcgatcactgagaacggagggctgttgaagggctaccaattaacctacattcccgacaagctcaagaacgtcggccatcagtgtggatgcattttctacgtacctgccgcgtatacttccaagattgacccaacgacaggatttgtgaatatatttaagttcaaggacttgaccgtggatgcaaagagagaatttataaagaaattcgactctataaggtatgacagcgagaaaaatttgttctgcttcacatttgactacaataactttatcacacagaacacggtgatgagcaagtctagctggtccgtctacacgtatggcgtccgcattaagcgacggtttgtgaatggccgcttcagcaacgagtctgacacaatcgacattacaaaggacatggagaagacactcgagatgactgacataaactggagagacggacacgaccttcgccaagacatcatagactacgagatcgtgcagcatatatttgaaatattcagactgaccgttcagatgcggaatagcctctccgaattagaagatcgcgactacgacaggttaatcagccctgtattaaatgagaataacatcttttatgatagcgccaaagctggcgacgccctacctaaggacgccgatgccaatggtgcatattgcatcgcactcaagggactgtatgagatcaagcagataacagagaactggaaggaagatggcaagtttagcagggacaagctgaagatctccaataaggattggttcgatttcattcagaataaacgctatctttga

SEQ ID NO: 258 - DNA, 3792 bp, Artificial Sequence
  Description of Artificial Sequence: Synthetic polynucleotide
atgaacaatggtaccaataactttcagaacttcattgggattagtagcctccagaagaccctacggaacgccttgatccctaccgagacaacgcagcaatttatcgttaagaacggcataatcaaagaggacgagcttagaggagagaatcgccaaatcctgaaagacattatggatgattattatcgaggattcatcagtgagactctaagtagcatagacgatatagattggacctccttattcgaaaagatggagattcagctaaagaacggcgataataaagacacactcatcaaagaacagactgagtaccggaaggccatccataagaaatttgcaaacgatgaccggttcaagaatatgttcagcgccaagctcatttcagacattctgcccgagttcgttatccacaacaataactattccgcaagcgagaaggaggaaaagacacaggtgatcaagttgtttagtcgtttcgctacctctttcaaggattactttaagaatagagccaactgtttctctgctgatgacatctcttcatccagctgtcatcggatcgtgaacgataacgccgaaatatttttctctaacgctcttgtgtaccggagaattgttaagagcttgtccaatgacgatattaataagatttccggtgatatgaaggatagtctgaaagaaatgtccctggaggaaatctattcatatgagaagtatggtgagttcatcactcaagaaggaataagtttctacaatgatatatgcggcaaagtaaatagcttcatgaatctgtattgccaaaagaacaaagagaataagaacttgtacaaacttcagaaactgcacaagcaaattctctgcatcgccgacacctcctacgaagtgccatataaatttgagtcggatgaggaggtgtatcagtccgtcaacggtttcttggacaatatctctagcaagcacatagttgaaagactcaggaagataggagataattacaacggctacaacttggacaagatctacattgtcagcaagttctacgagagcgtgagccaaaagacctatagggattgggaaaccatcaatacagcgctggaaatccattacaataatatactgccagggaacggcaagagtaaggcagataaggtaaagaaggccgttaagaatgatctgcagaaatctattactgagataaacgaactcgtttccaattataaactgtgctcggatgataatataaaggccgaaacctacattcatgagatttctcacattctgaataacttcgaagcgcaagaactcaaatataacccagagattcacttggtagagtcagaactgaaggcatctgagcttaagaacgtattagatgtcattatgaatgccttccactggtgcagcgtctttatgactgaggaattggtcgataaagataacaacttctacgccgaactcgaagagatctacgacgagatctacccagtgatcagcctctataacctggtgaggaactacgtaacacagaaaccttacagcacaaagaaaataaagctgaactttggcatccctacactagcggacgggtggtccaagtccaaagagtatagtaataatgctattattctcatgcgggacaacctgtactatctcggcatatttaacgctaagaacaagcctgataagaagatcattgagggtaatactagcgagaataaaggtgattataagaagatgatctataatttattgcccggacctaataagatgatcccaaaggtgttcctctccagcaagactggcgttgaaacttacaagccctctgcatatatcctcgaaggatataaacagaataagcacattaagagctccaaggatttcgacatcacattctgccatgacctcatagactattttaagaattgcatcgccatccatcccgagtggaagaacttcggctttgatttcagtgacacaagcacctatgaggatattagtggattctatagggaggttgaactgcagggctacaagatcgactggacgtacatctctgagaaagacattgaccttcttcaggagaagggacagctgtacttgtttcagatctataataaagatttctccaagaaatccacaggcaacgataatctgcacactatgtatctgaagaacctctttagtgaggagaatttgaaagacatcgtgctcaagctgaatggcgaggccgagatcttctttaggaaatcgagcatcaagaacccgatcatccataagaaaggcagtatattagtgaaccggacttacgaagctgaggagaaagatcagttcggcaatatccaaattgtgcggaagaacatccctgagaacatctaccaggagctgtacaagtacttcaatgacaagtcagacaaggaactctctgatgaggccgctaaactgaagaacgtggtgggtcaccatgaagcggcaactaacatcgttaaggactaccgctatacctatgacaagtactttctgcatatgccaattactatcaactttaaagcgaataagactggatttatcaatgatcggatcctacagtacatcgctaaggagaaagacctgcatgttataggcatcgaccgcggagaaaggaatttgatttacgtgtcagtcatcgatacgtgtggcaacattgtggagcagaaatccttcaacattgtcaatggctacgattaccagattaaattgaagcagcaagaaggagctcgccagatcgcccgtaaggagtggaaagagatcggaaagatcaaggaaatcaaagaaggctatctatcactggttatccacgagattagtaagatggtaatcaagtacaacgctatcattgccatggaggatctctcttatggctttaagaaaggccggttcaaggtcgagaggcaagtttatcagaaattcgagactatgttgattaacaagcttaattacctggtatttaaggatatatctatcaccgagaatggtggcctcctcaaagggtatcagcttacgtatattcccgacaagctgaagaatgtcggtcatcaatgcggatgtatcttttacgtaccagcagcatacacatcaaagatcgacccaactactggatttgtcaacatctttaagtttaaggacttaactgtggacgcgaagagggagttcataaagaaatttgatagcatccggtacgactcagagaaaaatctgttctgcttcacatttgactataacaatttcattactcagaatactgtcatgtccaagagcagctggtcagtgtacacatatggagttcgcatcaagagacgatttgtcaatgggaggttctccaacgagagcgatactattgacatcaccaaagatatggagaagactttagagatgaccgacattaactggagggatggtcacgaccttcgccaagacatcatcgactacgaaattgtgcagcatatcttcgaaatctttaggctgacagtacagatgcggaattctttgtccgagctcgaggaccgggactacgatcggctgatttctcccgtcttaaacgagaacaacatcttctatgactctgccaaagccggagatgctcttccaaaggatgcagatgctaatggagcttactgtatcgccctgaaaggtctatacgagattaagcagattacggagaactggaaagaggatggcaagtttagcagagataagctgaagattagcaataaggattggttcgatttcatccagaataagagatatctatag

SEQ ID NO: 259 - DNA, 3792 bp, Artificial Sequence
  Description of Artificial Sequence: Synthetic polynucleotide
atgaataacggtactaacaactttcagaatttcattggcatcagctccctccagaagaccctaagaaatgctcttataccaacagagaccacacaacagttcatagtcaagaatggaataattaaggaagacgagttgagaggtgagaaccgacagatacttaaggatattatggacgattactacagaggctttatctctgaaacgttatcctccatcgacgacattgattggacgagcctctttgagaagatggaaatccaactgaagaacggcgacaataaggatactctgattaaggagcagacagaatacaggaaggcaatacacaagaagtttgccaatgatgaccgcttcaagaatatgttcagcgcaaagttgatctcagatattctgcctgaatttgttattcataataataattattcagctagcgagaaagaggagaagacccaagtaattaagctgttctcgcgcttcgccacaagcttcaaggactattttaagaaccgcgctaactgtttctccgccgacgatatttcgtccagcagctgccacagaattgttaatgacaacgctgagattttcttctccaatgcccttgtgtaccggagaatcgtcaagtccctgagtaacgacgatataaataagatttccggagacatgaaagattccctgaaggaaatgagcctggaagagatttacagctatgagaaatacggtgaattcattacgcaggaaggcatctcattctacaatgatatctgtggcaaggttaactcgtttatgaacttatattgccaaaagaataaggagaataagaacctctacaagttacagaagcttcacaaacagattctgtgtatcgcagatacatcttacgaagtgccatataagttcgaatcagacgaggaagtgtaccaaagtgtcaatggcttcctggataatattagcagtaagcacattgtcgaaaggctgaggaagattggagacaattacaatggctataatctggacaagatctacatcgtctccaaattctatgagagcgtcagtcaaaagacatatagagactgggaaactataaacacagctctggagattcattacaacaacattctgcccggaaatgggaagtccaaagctgacaaagtcaagaaagcagtaaagaatgatctccagaagtcaatcactgagatcaacgagctggtctcaaattacaagttgtgtagtgatgataacatcaaggctgagacttatatccacgagatttctcacatcctcaataacttcgaagcacaagagctgaagtacaatcctgagatccatcttgtagagagtgaattgaaagccagcgagctgaagaatgtgctggacgtgattatgaacgccttccattggtgcagtgtgttcatgaccgaagagctagttgacaaggataataatttctacgccgagcttgaggaaatctacgacgaaatatatccagtgatttctctgtacaacctagttaggaactatgttacccagaagccatactctacgaagaaaatcaagctgaacttcggaattcccaccttagcggacggctggagtaagtctaaagaatattccaacaatgccatcattctgatgcgggataatctctactatctgggaatctttaatgcaaagaacaaacccgataaaaagattatagaaggcaacacaagcgagaataagggtgattataagaagatgatctacaacctgctccctggtcccaacaagatgattcctaaagtgtttctgtcaagcaagaccggcgtggaaacctacaagccgtctgcctacatattggagggatataaacagaataaacatattaaatcctccaaagacttcgatatcaccttctgccacgaccttattgactactttaagaactgcatcgccatccaccctgagtggaagaacttcgggttcgacttctccgacaccagcacttatgaagatataagcgggttctatagggaggttgaactgcaaggctacaagatcgattggacctatatatctgagaaagacattgacctgttacaggagaagggacagttatatttatttcagatctacaacaaggacttcagcaagaaatcaacaggtaatgataatttgcatacaatgtacctcaagaatcttttctcagaagagaacttgaaggacattgtgttgaagctgaacggcgaggctgaaatattcttccgcaagtcctctatcaagaacccaatcatccataagaaaggaagcatactggtcaaccgaacctacgaagccgaagagaaggatcaattcggaaacatacaaatagtgagaaagaacattcccgagaacatttaccaagagctctataagtatttcaatgacaagtccgacaaagaattgtcagacgaggccgctaagctcaagaacgtggtagggcaccacgaggctgccacaaatattgttaaggattaccggtatacgtacgataagtacttcttgcacatgcccatcacaataaacttcaaagctaacaagaccggctttatcaatgaccgtatcttgcagtatatcgccaaggagaaagacctacatgttataggaatagaccgtggagaaagaaatctgatatacgtgagcgtgattgatacttgcggcaatattgtcgagcagaagagcttcaacattgtgaacgggtatgattaccaaatcaagttaaagcagcaggagggcgcccggcagatcgcccgaaaggaatggaaggaaattggaaagattaaggaaatcaaggaaggctatctaagccttgttattcatgaaatttccaagatggttatcaaatacaacgcgatcattgcgatggaagacctgtcctatggctttaagaagggacgtttcaaggtggagcggcaggtgtaccagaaatttgagacaatgctgattaacaaattgaattacctcgtctttaaggatatctcaatcaccgagaacggtggactgttgaagggataccagctaacatatattcctgacaaattaaagaacgtaggtcaccagtgcggctgcatcttttacgtgcctgcggcatacacctcgaagatcgacccaaccactggtttcgtgaacatattcaaattcaaggacttaaccgttgatgctaaacgcgagttcatcaagaagttcgactccatccggtatgacagcgagaagaatctgttctgctttacctttgactacaacaactttattacacagaacaccgtaatgagtaagagctcctggtctgtctatacgtatggtgttcggattaagcggcgcttcgtgaatgggcgtttctccaatgagtctgacacaattgatatcacgaaagatatggagaagactcttgagatgaccgacatcaactggagagacggccacgatttgcggcaagacatcatcgactacgagatcgtgcagcatatctttgaaatcttccgtctgacagtccagatgcgtaatagcctgtcagagctcgaagatagagattatgacagactgatcagtcccgtgctgaatgagaacaatatattctacgactccgcaaaggctggcgacgccctccctaaggacgctgacgccaatggcgcctattgcatagcactgaaaggcctgtatgaaattaaacagatcacagagaattggaaagaggatgggaaattctctagagataagcttaagatcagcaataaggactggtttgacttcatccagaacaagagatatttgtga

SEQ ID NO: 260 - DNA, 3792 bp, Artificial Sequence
  Description of Artificial Sequence: Synthetic polynucleotide
atgaataacggcacgaacaatttccagaactttatcggtatatccagtcttcagaagacccttcggaatgctcttatacctaccgagactacacagcaattcattgtcaagaatgggataattaaagaagacgagcttagaggtgagaataggcagatcctgaaagacatcatggacgactactatcgcggtttcatcagcgagaccctttcttctatagatgatattgactggaccagtctgttcgagaagatggagattcaactgaagaatggagataacaaggataccctgattaaagagcaaaccgagtaccgaaaggccatacataagaagttcgccaacgatgatcgcttcaagaatatgtttagcgccaagctgattagtgatatcctgcccgagttcgtgatccacaacaacaactattctgcctcggagaaagaggaaaagactcaagtgattaagctcttctcacggttcgccacatctttcaaagattactttaagaatcgagctaattgcttctcagcagacgacatatcatcatcctcctgccacagaattgttaacgataatgccgaaatcttcttcagtaacgctctggtatacagacggatcgtcaagagcttgagcaacgacgacatcaataagatctcaggcgatatgaaggacagcctaaaggaaatgagtctggaggaaatctatagctatgagaaatatggagaatttattacccaggagggaattagtttctataatgacatctgcgggaaagtgaattctttcatgaatctgtactgtcagaaaaataaggagaataagaacctctataaactgcagaagctgcataagcaaatcctgtgcatcgcagatacgagctacgaagtcccatacaagttcgaaagcgatgaagaagtgtatcagagcgtgaatggcttcctggataacatttcctcgaagcatatcgtggaacgcctgaggaagatcggagacaattacaacggctacaacctcgataagatatatatcgtcagtaagttctacgagtctgtgagccagaagacataccgagactgggaaacaattaatacagctcttgagattcactacaacaatattcttccaggaaacggaaagagtaaggctgataaagtcaagaaggctgtaaagaatgatctccagaaatcgataacggagattaacgagcttgtcagcaactacaagctgtgttctgacgacaatatcaaggccgagacttatatacatgaaatcagccacattctgaataatttcgaagcgcaggagctcaagtacaacccagaaatacacctggtcgaatcggaactgaaagcttccgaactaaagaacgtgctcgacgtgatcatgaacgcattccactggtgcagcgtgtttatgaccgaggaattagtagacaaagataacaacttctacgctgagctcgaagaaatctatgacgagatctatcccgtaatatccctgtataacctggtgcgaaactacgtgacacagaaaccgtatagtaccaaaaagatcaaactcaacttcggaattccaaccctggctgatggctggtccaagagcaaggagtacagcaacaatgcaattattctgatgcgcgataatctctactacctgggcatcttcaacgctaagaataaacccgataaaaagatcattgaaggtaataccagtgagaacaagggagattacaaaaagatgatttacaatcttctgcccggccctaacaagatgatccctaaagtcttcctgagtagtaagacaggtgtggaaacatacaaaccctccgcctacatcctggagggctataaacagaataagcacatcaaatctagtaaagacttcgatattactttctgccacgatttaatagactactttaagaactgcatcgccatccatccagagtggaagaacttcggattcgactttagcgacacttccacctatgaggatatctctggcttctacagggaggtagagctccagggctacaagatagattggacatatatatctgagaaggatattgatctgctgcaggagaaaggccaactctatctgttccagatctataataaagatttctcgaagaagtcaaccgggaacgataatctgcacacgatgtatctaaagaatctattctctgaggagaatctgaaagatattgtgctgaagcttaatggagaggcagagatattttttcggaagagcagtattaagaatcccataatccataagaaaggaagtatcctggtcaataggacgtatgaggctgaggagaaggatcaattcgggaacatacagatcgtccgtaagaacatccctgagaacatctaccaggagctgtacaaatacttcaacgataagtccgacaaggaactcagcgatgaggcggccaagctaaagaatgttgtcggccatcacgaagcagctacaaatatcgtgaaggactaccggtacacttacgacaaatactttctgcatatgccgatcacaatcaatttcaaagccaataagactggtttcatcaatgacaggattctccaatatattgctaaagagaaggatctccacgtcatcggcatcgaccgtggtgagcggaatcttatttatgtctccgtcattgatacttgtgggaatattgttgagcagaaatcgttcaacattgtcaatggatacgattaccagatcaagttgaagcaacaggagggagccagacagatcgcccgcaaagaatggaaagagatcggtaagattaaggaaatcaaggaaggatacctcagcctggttattcatgaaatcagtaagatggtcatcaagtataacgctattatcgccatggaagatctgtcatatggatttaagaaaggacggttcaaggtggagagacaggtataccagaaattcgagactatgctgatcaataaactgaactatttggtctttaaggatatatcgattaccgagaatggtgggctattgaagggttatcagctgacatacattcccgataagttaaagaacgtcgggcaccagtgcggctgtatcttctacgtccctgctgcttacacttcaaagattgatccaaccaccggatttgtgaacatcttcaagttcaaggacctgacagtagatgccaagagagaatttatcaagaagtttgacagcattcggtacgattccgagaagaatctgttctgcttcactttcgactataacaacttcatcactcagaacaccgtcatgtctaagagcagttggagcgtatatacttatggagtgcggatcaagcgacgattcgtgaacggcagattcagtaacgagagcgacacgattgacattaccaaagatatggagaagacactcgaaatgacggatatcaattggcgagacggccatgacctacggcaagatataatagactacgagatcgtccaacacatcttcgaaatattccgcttgacagttcagatgaggaacagtttgtcggagttagaggaccgggactacgacagattaatatcgcctgtcctcaacgagaacaacatattctatgacagtgccaaagctggcgacgcacttccgaaagacgccgacgcaaacggagcttactgcatcgctctgaaaggtctgtatgaaatcaagcagattaccgagaactggaaggaggatggaaagttctcccgcgacaaattaaagatttcaaacaaggattggtttgacttcattcagaataaacggtatctgtag

SEQ ID NO: 261 - DNA, 3792 bp, Artificial Sequence
  Description of Artificial Sequence: Synthetic polynucleotide
atgaataatggcaccaacaactttcagaactttattggaatttcatcactccagaagaccttaagaaacgcccttatacctacagagaccactcagcaatttatcgttaagaacggtattatcaaagaggacgagctgagaggcgagaacagacagattctcaaggacatcatggatgactactacagaggctttatttcagaaacactgagttccatagatgacatagactggacctccttgtttgaaaagatggagatccagttgaagaacggtgataataaggacactctgataaaggagcagacagagtacaggaaggcaatccataagaaattcgcaaacgacgatcggttcaagaatatgtttagcgccaagctcatttcagacatactgcctgagttcgtcatacataataataattattccgcctccgagaaagaggagaagacccaggtaattaagttgtttagccgattcgcaacgtctttcaaggactacttcaagaatagggcgaactgcttctctgcagatgatatttcttcctcctcttgccatcgaatagtgaacgacaatgcagagatatttttctccaacgcgttggtgtaccggcggatcgtcaaatccctaagcaatgacgacatcaataagatcagcggcgacatgaaagacagtctcaaagagatgagtctggaagaaatttacagttatgagaaatacggagaatttatcactcaggaaggaatcagcttctataacgatatatgtggcaaggtgaactccttcatgaacctttactgtcagaagaacaaagagaataagaatctgtacaaactgcagaaactgcataaacaaatactgtgtatcgccgacaccagttatgaggttccctacaaattcgagtctgacgaggaagtgtaccaaagcgtgaatggcttcctggataatatcagttcaaagcacatagttgagcgacttcgcaagatcggtgataattacaacggatacaatctggataagatctatatcgtatccaaattctacgaaagtgtgagtcaaaagacgtatagagattgggagacaataaacaccgcactggaaatccactacaacaacatactacccggcaacggcaagagtaaagctgacaaagtgaagaaggctgtcaagaatgatcttcagaagtcaattaccgagataaatgaattggtgtctaactataagctgtgctccgacgacaacatcaaggcggagacgtatatccatgagatctcgcacatcttgaataactttgaagctcaagagctgaagtataaccctgagatccacctggtcgaatcagagctcaaagcttccgaactcaagaacgttctcgacgtgatcatgaacgctttccattggtgtagcgtatttatgaccgaggagttggtcgacaaagataataatttctacgcagaacttgaagagatttacgacgaaatctaccctgtgatttccctatataacctggtcagaaactacgtaactcagaaaccctactcaactaaaaagatcaaactgaacttcgggataccaacattagctgacggctggagcaagtctaaggaatatagcaacaacgctattatcctcatgcgggacaacctttactacctgggaatctttaacgcaaagaataaacctgataagaagatcattgagggaaacacttccgagaacaagggagattacaagaagatgatctataatctattgccggggccgaacaagatgatacctaaagtatttcttagctcaaagacaggcgtggaaacctacaaacccagtgcctacatcctcgaaggctacaagcagaacaaacatataaagagctccaaggacttcgacattacattctgccacgacctaatcgactacttcaagaattgtattgctatccatccagaatggaagaacttcggcttcgatttctctgatactagtacttacgaggatatctccggattctaccgggaagtcgagctgcaaggttataagatagactggacatatatatctgagaaagacatcgacctgctgcaggagaaggggcagctctatctgttccagatctacaataaagacttctctaagaagagcacaggaaatgataatctgcacacgatgtacctgaagaatttgtttagtgaagagaacctgaaggatatagtgttgaagttaaatggagaggcagagatcttcttccggaagtcatccattaagaatcctattatccataagaaaggtagcatacttgtgaatcgaacatacgaagctgaggagaaggaccagttcggtaacattcagattgttcgcaagaatatacccgagaatatttaccaggagttgtacaaatactttaacgacaagagtgataaggagctgtctgatgaagcggccaagctaaagaacgtcgtcgggcatcacgaggccgccaccaacattgtgaaggattatcgttacacgtatgataaatacttcctgcacatgcccatcaccatcaacttcaaggcaaataagactggctttatcaacgaccggatattgcagtatatagctaaggagaaggatttgcacgtgatcggcatcgaccgcggtgagaggaaccttatctacgtttctgtgatcgatacttgcgggaatatcgtggaacagaagagcttcaatatcgtaaacgggtatgattaccagatcaagctcaaacagcaggagggtgctcggcaaattgctagaaaggaatggaaggaaattggtaagatcaaggaaattaaagaaggctatctcagcctggttatccatgaaatcagtaagatggtcatcaaatacaatgctatcattgctatggaggacctgtcctacggattcaagaagggacgctttaaagtcgagcgacaggtttaccagaaattcgagaccatgttgataaacaagctaaattacctggtgtttaaagacataagtatcaccgagaatggcggcctgctgaagggttatcaattgacttatattccagataagctgaagaacgttggacaccagtgtggatgtatcttctacgtgccagctgcctatacctccaagatcgatccgactacaggctttgtgaatatcttcaagttcaaggacctgaccgtcgatgctaagcgggaattcatcaagaagtttgactcaatcagatacgattccgagaaaaacctattctgcttcacctttgattataacaatttcattacacagaacaccgtgatgtcaaagtcaagctggtctgtatatacatatggcgtacgtatcaagcggagatttgttaatggtagattctctaatgagtcggatacgattgacataaccaaggacatggaaaagaccttggagatgacagatatcaattggcgggatggccacgatctcagacaggacataattgattatgaaattgttcagcacatatttgaaatattcaggctcaccgtgcagatgcggaacagtctgagcgaactggaggatagagactacgacaggctgatcagcccggtactaaatgagaacaacatcttctatgactctgctaaggcaggagacgcgctgcccaaggatgccgatgcaaacggtgcctactgtatcgccctcaaaggtctctatgagattaagcagatcacggagaactggaaagaagacggcaagttctcgcgagacaagctcaagatttctaacaaggattggttcgactttatccagaacaagcgctacctgtga

SEQ ID NO: 262 - DNA, 3792 bp, Artificial Sequence
  Description of Artificial Sequence: Synthetic polynucleotide
atgaataacggaacaaataactttcagaacttcattggcattagcagtttacagaagaccctgaggaacgccctcattccaaccgaaacaacacaacaattcatcgtaaagaatggcatcatcaaagaggacgagcttaggggtgagaatcgacagattctgaaagacatcatggacgattactatagaggttttatctctgagactctgtcttccattgacgacatcgactggacgtccctgttcgagaagatggagatacagcttaagaatggagataacaaggacaccttaattaaggagcagactgagtacaggaaggctatccacaagaaattcgctaacgacgatcgattcaagaacatgttctcagccaaactgatttccgacatcctcccggaattcgtgattcataataataattactcagcctcggagaaggaggagaagacacaggtgatcaaactgttctctcgattcgccacaagcttcaaggactattttaagaatcgggcaaattgtttctccgctgatgatatatcttcttcttcttgtcaccgtatcgtcaatgacaatgctgaaatcttcttctctaatgctcttgtttataggagaattgtgaaatctttgagtaatgacgacataaacaagatatctggtgatatgaaagatagcctgaaggaaatgtctttagaagagatctacagctacgagaagtacggagagttcatcactcaggaagggatcagtttctataatgacatctgcggtaaagtgaatagcttcatgaatctctactgtcagaagaacaaagagaataagaatctctataaactccagaagttacacaagcagatcctctgtatagcagatacgagttatgaagtgccgtataagttcgagagcgacgaggaagtgtatcagtccgtgaacgggttcctcgataatatctctagtaagcatatcgtcgagagactgcggaagattggtgataactacaacgggtataatctagataagatttacattgtgagtaagttctacgagagcgtatcacagaaaacttaccgcgattgggagacaattaatactgcgttggagatccattacaacaacatactgccagggaacggtaaatcgaaggccgataaggtgaagaaggcagtcaagaatgatctccaaaagagcattaccgaaattaatgagctggtctccaattataagctgtgcagcgatgataacatcaaagcggaaacctatatccacgaaattagccacattcttaataatttcgaagcgcaagaactcaaatacaatccagaaatacacctcgtggagagtgaattgaaggcatctgaactaaagaatgtcctggatgttataatgaacgccttccattggtgcagtgtattcatgacggaggagctggtcgacaaggataataatttctacgcagaactcgaggagatttacgatgaaatctacccggtcataagcctctataatttggtccggaattatgtgacacagaagccctacagcaccaagaagatcaaactgaacttcggaatcccgacattagccgacggctggtccaagagcaaagaatactcaaacaacgccataatcctcatgcgggacaatctgtactacctgggcatcttcaatgccaagaataaaccggataagaaaattatcgagggcaatacctctgagaataagggtgactacaagaagatgatctacaacctgctgccaggacctaataagatgattcctaaggtctttctgagcagcaagactggagtggagacctacaaacccagtgcctacatactggaaggttataagcagaacaaacatatcaagagctctaaagacttcgatattacgttctgtcacgacctgattgactactttaagaattgtattgccatccacccagaatggaagaacttcgggtttgatttctccgacacaagcacctacgaagatatctccggcttctatcgcgaagtcgaactccaaggttacaagatcgactggacttatattagcgagaaggatattgacctgcttcaggagaagggtcagctttatttatttcagatttataacaaggacttctcgaagaaatctaccggcaatgacaatctccacacaatgtatctcaagaacctcttctccgaggagaatctgaaggacatcgtattgaagctgaatggcgaggcagaaatattcttccggaagtctagtatcaagaatccaatcattcataagaagggaagtattctagtaaacagaacttatgaagctgaggagaaggaccagtttggaaatattcagattgtgcgaaagaatattcctgagaacatttatcaggagctgtacaaatacttcaacgataagagcgataaggaactttccgacgaagctgcgaaattgaagaacgtagtgggtcaccatgaggcagctaccaacatagtgaaggactaccgttatacctacgataaatacttccttcacatgccaataaccataaatttcaaggcaaataagacaggatttatcaatgaccgtatactgcagtacattgccaaggagaaggacctgcatgttatcggcatcgatcgcggtgagagaaacttgatctatgtcagtgtgatagatacatgcgggaacatcgtggagcagaaaagtttcaatattgttaatggctacgattaccaaatcaagcttaagcagcaagagggtgcacggcagattgcaaggaaagaatggaaagaaatcggcaagatcaaagaaataaaggagggatacctgtccctggtgatccacgagatctctaagatggtcatcaagtataacgccatcatagccatggaagatctgagttacgggtttaagaagggccggtttaaggtagaacgacaggtgtaccagaaattcgagacgatgctgatcaataagctgaactacctggtattcaaggacattagcattactgagaatggcggactgctcaagggctaccagctaacttacatccctgacaagcttaagaacgttgggcaccagtgtggctgtatattttacgttccggctgcttacaccagcaagattgatcctacaaccgggtttgtgaacatatttaagttcaaggacctgaccgtcgacgcaaagagggagttcattaagaagtttgactctatcaggtacgactcagaaaagaatttattctgtttcaccttcgactataacaatttcatcacccagaatacagtgatgagcaagagcagttggtctgtatatacctatggcgtgcggattaagcggagattcgttaacggccggttctcaaacgagtccgacaccatcgatattacgaaagacatggagaagacattggagatgaccgatattaactggagggacggccatgatctgcgacaagacatcattgattacgaaattgttcagcatatctttgagatctttaggctgaccgtccagatgcgaaacagtctctccgaactggaggaccgcgactacgacaggttaatttctccggtacttaatgagaataacatcttttacgattcggctaaagcgggcgacgccttacctaaagatgctgatgccaacggagcttattgcattgctttgaaaggcctgtatgaaattaagcaaattactgagaactggaaggaagacggcaagtttagcagggataagcttaagatcagcaataaggattggttcgacttcattcagaacaagaggtacctgtga

SEQ ID NO: 263 - DNA, 4005 bp, Artificial Sequence
  Description of Artificial Sequence: Synthetic polynucleotide
atgagttcgctcacgaagtttaccaataaatattcgaagcagttaacaataaagaacgaactgatacctgttggcaagacattggagaacattaaagagaatggactaatagatggagatgaacaattgaatgagaattaccagaaggccaagattattgtggacgacttccttagggatttcataaacaaggctctgaataacacacaaatcggcaactggagagagctagcagatgcattaaataaagaggacgaagataatatcgagaagttgcaggataagattcgtggtattatcgttagtaaatttgagacgttcgacctattctctagctatagtattaagaaagatgagaaaataattgacgacgacaacgatgtcgaggaggaagaattggatcttggaaaaaagacttcttcgtttaagtacatattcaagaagaacttattcaaactcgttcttccatcatatcttaagaccacgaaccaggataagcttaagatcataagctccttcgataatttctcaacttactttcgtggtttcttcgagaatcgtaagaatatctttactaagaagccaatttcaactagtattgcctatagaattgtacatgataacttccctaaatttctagataatattcgttgcttcaatgtatggcaaacagagtgtccacaattaatagtgaaagctgacaattatttgaagagtaagaacgtaatcgcaaaggacaagagtttagccaactactttactgttggtgcatatgattacttccttagtcagaacggtatcgacttctataataacattattggtgggttacccgccttcgctggacatgagaagatacagggtttaaacgagttcattaatcaagagtgtcagaaggattccgaattgaaatccaaattaaagaacaggcacgcattcaagatggcggtgttatttaaacagatattatccgatagagagaaatccttcgtcatcgacgaatttgaaagtgacgcacaggtaattgatgccgttaagaatttctacgccgaacaatgtaaggataacaatgttatcttcaacttattgaacctaattaagaatatagcctttctgtcggacgatgagctagacgggatattcattgaaggtaagtatttatcctctgtttctcagaagctctattcagattggtcgaaactgagaaacgatattgaggactcagctaattcaaagcaaggtaacaaagaattagcgaagaaaataaagacaaataagggtgatgttgagaaagctattagtaaatatgaatttagcttaagcgaattaaatagtattgtccacgataatactaagttctctgacttgctctcatgtactttacacaaagttgcatctgagaaacttgtgaaagtcaacgaaggtgattggccgaagcatctaaagaacaacgaagagaaacagaagattaaagaaccacttgatgcactattagaaatatacaatacattattaatcttcaattgtaaatcatttaataagaatggcaacttctatgtagactatgatagatgtattaatgaattatcgagcgttgtttacttatacaacaagacccgtaactactgtaccaagaaaccttataacactgacaagttcaaattgaatttcaattctccacaattgggtgaagggttctccaagtcgaaagagaacgattgtttgaccttgttgtttaagaaggatgacaactattacgtgggtataatccgtaaaggcgccaagattaatttcgacgacactcaagctatagctgacaataccgataattgtatctttaagatgaactactttctattaaaggatgccaagaagtttatccctaagtgttctatacagttgaaggaagttaaagcccacttcaagaaatctgaggatgactacatcctttctgataaagagaaattcgcttcacctttggttataaagaagtctacattcttattagcaaccgctcacgtgaaaggaaagaagggcaacataaagaaatttcagaaagagtactcgaaagagaatcctaccgaatataggaattcgttgaatgaatggatagccttctgtaaagagttcctcaagacttataaggccgccacaatcttcgatataaccacccttaagaaagctgaggaatatgccgatattgtagaattctataaagatgttgataatttatgctacaagctcgagttctgccctattaagacgtctttcattgagaacttaattgataatggtgacttgtatctatttaggattaataacaaggatttctcttcgaagtcaacaggcaccaagaatttgcacaccttgtatcttcaagctatcttcgacgaaagaaatcttaacaatcctaccattatgttaaacggtggtgctgagttattctatcgcaaagaatcaattgaacaaaagaaccgtattactcataaagctggaagtattctcgtgaataaagtgtgcaaagatggtacctctctagacgacaagattagaaacgagatctaccaatacgagaacaagtttatagataccttgtctgatgaagctaagaaggtacttcctaacgtcattaagaaagaggccacccatgatattacgaaagataagagattcacttcggataagttcttctttcattgtccattgacgataaattataaggagggtgatactaaacagttcaataatgaagtactttccttcctccgtggtaatccggacattaatataattggtatcgacagaggtgagagaaacctaatatatgttactgtcataaaccagaaaggcgagatattggatagtgtaagtttcaatacagtaacgaacaagtctagtaagattgaacagacggttgattatgaggagaaactagctgttagagagaaagaacgtatagaagcgaagagatcttgggattctataagtaagattgcgactctcaaagaaggttatttatcagccatcgtacacgaaatttgcttacttatgattaaacataatgcaatcgtagtcctggagaacctcaacgctggcttcaagagaatacgaggtggtttgtcggagaaatctgtttatcagaagtttgaaaagatgttgataaataaattaaattacttcgtaagcaagaaagagtcagattggaataaaccatcaggattgttaaatggactgcaactttctgatcaatttgagtccttcgagaagcttggcattcaatcaggtttcatattctatgttccagccgcatatacgtctaagattgacccaacaactggatttgccaacgtactcaacttgtccaaagttcgcaatgttgatgccatcaagagcttctttagtaactttaacgaaattagttatagcaagaaagaggcattatttaaatttagcttcgatctcgactccctaagtaagaaaggtttctcttcattcgttaagttctctaagtcaaagtggaacgtatataccttcggagagagaataatcaaaccgaagaataaacaagggtacagagaagataagcgtataaacttgacgtttgaaatgaagaagttattgaatgaatacaaggtgtctttcgatctggagaacaacctaataccgaatctgacaagtgcaaacctaaaggacaccttctggaaagaactgttcttcatattcaagacaacactgcagctaagaaattcagttacaaacggtaaggaggatgtattgattagcccagtcaagaatgccaagggcgaattctttgttagcggtactcataataagactttacctcaggactgtgacgccaatggtgcgtatcatatagctctcaaaggtttaatgattctggagaggaataatttagtcagagaagagaaagatactaaaaagattatggccatttcaaacgtggactggttcgagtatgtgcagaagaggcgaggcgtcttgtaa

SEQ ID NO: 264 - DNA, 4005 bp, Artificial Sequence
  Description of Artificial Sequence: Synthetic polynucleotide
atgtctagtttgactaaatttaccaataaatattcgaaacaactcactataaagaatgaattgatccctgttggcaagactctagagaacataaaggagaatggtctgatagatggtgatgaacaacttaacgagaattatcagaaggcaaagattatcgtggacgacttcttacgcgacttcattaataaggcactaaataacacccaaatcggtaactggcgggagttggcagacgcgctgaataaggaagacgaagataacatcgagaagttgcaggacaagattagaggcatcatagtgtctaaatttgaaaccttcgatttgttttcttcatatagtataaagaaagacgaaaagatcattgacgatgataatgatgtggaagaagaagaattagatttgggtaaaaagacttcgtctttcaagtatatatttaagaagaacttattcaaacttgtgttgccatcatacctgaagactaccaaccaggataaactaaagataattagctctttcgacaatttctcaacttactttcgtggcttctttgagaaccgaaagaatatatttactaagaaaccaataagcacaagtatagcttatagaattgtccatgataactttcccaagttcttggataacattaggtgcttcaacgtctggcagacggagtgtccgcaattgatcgtcaaggccgataattatctcaagagcaagaacgtgatcgctaaggataaatccctagcaaattacttcacagttggtgcctacgattatttcttatctcagaatgggatagatttctataacaatatcataggtggtctaccagccttcgccggacatgaaaagattcaaggcttaaacgaattcataaatcaagagtgtcagaaagacagtgaacttaaaagtaagttaaagaatcgacatgcgttcaagatggccgtcctatttaaacagatattgtcagatcgggagaagtcatttgttattgacgaatttgaatccgatgctcaggttattgatgctgttaagaacttctatgcagagcaatgtaaggataataatgttatattcaatttgttaaatctaataaagaatattgctttcctcagtgacgacgaacttgatggtatatttatagagggaaagtatttaagttctgtctcacagaaattatattctgattggtctaagttaagaaacgatatagaagattctgctaactccaaacaaggtaataaagagctggcgaagaagattaagaccaataagggtgacgttgagaaagctatctctaaatacgaattctcgctgtcagaattgaactcgatagtccacgataatactaagttctcggatttgttgtcttgcacattgcacaaggtcgcatccgagaagctggttaaagtcaacgaaggagattggccgaagcacctcaagaacaatgaagagaaacaaaagattaaggaaccattggatgcacttctcgaaatttacaatacccttcttatctttaattgtaagagcttcaataagaatggaaacttctacgttgactatgatagatgtattaacgaattatccagtgttgtatacttatataataagacgaggaattattgtactaagaagccatataacactgacaaattcaagctgaactttaactcaccacagctcggtgaagggttctcgaagagtaaagagaacgattgtttaaccttgctctttaagaaagatgataattattatgtaggtatcataaggaagggtgcgaagattaacttcgacgatacccaagcaatcgccgacaacactgacaactgcatcttcaagatgaactacttcttgttgaaggacgcaaagaaatttatcccgaagtgtagcattcagttgaaagaagttaaggcccactttaagaagtcagaggatgattacatactatctgataaagagaaatttgcaagtcccttagttatcaagaaatctactttcttactggctactgcacatgtcaagggtaagaagggtaatataaagaaatttcagaaggagtatagtaaggagaacccaacagagtacagaaatagtctaaacgagtggattgcattctgtaaggagttcttaaagacttataaagctgcgaccatattcgatatcacaaccctaaagaaagcagaggaatatgctgatattgtagaattctataaagatgtcgacaacctttgctacaagctggagttctgtccgattaagacttcgtttatagagaaccttatagataatggagatttatacctattccgtataaacaacaaagacttctcttcaaagtctactggcaccaagaaccttcatactttgtacttacaagctatattcgatgaacgaaacttaaacaacccaactataatgctcaacggtggtgctgagttgttctacaggaaggaatcgattgaacaaaagaatagaatcactcataaagcaggtagcattctcgtcaacaaagtttgtaaggatggtactagtttagacgacaagatacgtaacgaaatctatcaatatgagaacaagttcattgatacattgagtgacgaagcaaagaaagtcttaccaaacgttatcaagaaggaagcaacccatgatataactaaagacaagagattcacctcagataaattcttcttccactgcccacttacaattaattacaaagaaggtgatacaaagcaattcaataatgaagtacttagctttcttcgtggaaatccagatattaacattattggaattgatagaggtgaaagaaatttaatttatgtcactgtgattaatcagaagggagagatcttggattccgtatcatttaacactgttactaacaaatcatcaaagattgagcaaactgtagattatgaggagaagctagctgttagggagaaagaaagaatagaagcgaagagatcttgggattctattagtaagattgctactttgaaagaaggctatttatctgctatcgtgcatgaaatctgtttgctgatgattaaacacaatgcaattgttgttctagagaacttaaatgcaggtttcaagcgtatacgaggaggtctgtccgagaagagcgtataccagaaattcgaaaagatgctgattaataaactaaattacttcgttagtaagaaagaatcagattggaataaaccaagtggtcttctcaatggtctacagttatcggaccagttcgaatcattcgagaaattgggtattcagtccggatttatcttttatgttccggcggcatatacatctaagatagacccgacaactgggttcgccaacgtccttaatctttcaaaggtccgtaacgtagatgcgattaagtccttcttctcaaacttcaatgaaattagctattcgaagaaggaggccctgttcaaattttctttcgatctagactcgctaagcaagaaagggtttagctccttcgttaaattctcaaagtcgaagtggaatgtgtacacatttggagaaagaataattaaacctaagaataagcaaggttatagggaagataagagaattaatctaacctttgagatgaagaagttgctcaatgaatacaaggttagctttgatttggagaacaatttgatcccgaacctcacctcagcgaatttgaaagacactttctggaaagaattattcttcatattcaagacaactttacaacttaggaactcagttacaaatgggaaggaagacgtcctaatatctccggttaagaatgctaaaggtgaattcttcgtgtccggaactcacaataagacactccctcaagactgcgacgcaaacggagcctatcatatcgctctaaagggtctgatgatacttgaacgaaataatttagtaagggaagagaaagacaccaagaaaattatggcgatctctaatgtagattggttcgaatacgttcagaagcgtagaggagtgctgtaa

SEQ ID NO: 265 - DNA, 4005 bp, Artificial Sequence
  Description of Artificial Sequence: Synthetic polynucleotide
atgtccagcctgactaagttcactaataagtattctaaacaattgaccataaagaatgaactaatcccagtcgggaagactctagagaatataaaggagaacggtctaattgacggtgatgaacaactaaacgagaactaccagaaagcgaagataatagttgatgacttcttaagggacttcattaacaaagctttaaataatactcagattggaaattggagggagctagccgatgctttgaataaagaagacgaagataatattgagaaattacaggataagattcgaggtatcattgtgagtaaatttgaaacatttgatcttttctcttcttactctatcaagaaagatgaaaagatcattgatgacgataacgacgttgaggaggaagaattagatttgggcaagaaaacgtcaagcttcaagtatatctttaagaagaatttattcaaattggtccttccctcttacctaaagactacaaaccaagataaacttaagataatttcctccttcgacaacttctccacatacttcagagggttcttcgagaatagaaagaacatcttcacaaagaaacctatttctacttctattgcatatcgtatagtgcatgataactttccgaaatttcttgataacattaggtgctttaatgtctggcaaaccgagtgtcctcagctgatagttaaggcagacaattatttaaagtctaagaacgttattgctaaagacaaatcacttgctaattatttcactgtaggagcatacgattatttcctctcccagaacggtattgacttctacaataacattattggcggtttacctgctttcgcgggtcatgagaagattcaaggattgaatgaatttattaatcaggaatgtcagaaggactcagaattgaagagtaaattgaagaatagacacgcgtttaagatggcagtcctcttcaaacaaatcctatcagatagagagaaatcctttgttatcgatgaattcgaaagcgacgctcaagtgattgatgccgttaagaacttctatgcggaacaatgtaaggataacaatgttatattcaacttacttaacttgattaagaatatcgctttcttaagtgatgatgaactcgatggtatatttatagagggtaagtatctctcgtcagtgagtcagaaactttattcagactggagtaagttaagaaacgatatcgaggattctgcaaatagtaagcaaggaaataaagaattagcgaaaaagatcaagacaaacaaaggcgatgttgagaaggccatttccaaatacgaattctccctatctgaattaaattccatagttcatgacaacaccaaattctccgacctcctgagttgcactcttcataaagtggcatcagagaagttggtcaaggtgaacgaaggagattggccgaagcacttgaagaataacgaagagaaacagaaaattaaagagcctctcgatgcattattagagatatataatacgctgctgatattcaattgtaagagtttcaataagaacggtaatttctacgtagattatgataggtgtataaatgaattgagttcggtagtatacctatataacaagacaaggaactactgcacgaagaaaccctataataccgataaatttaagttaaacttcaatagtccacagttaggcgaaggtttctctaaatctaaagagaatgattgccttaccctcttgttcaagaaagatgacaattattatgttggaatcattaggaagggcgcaaagattaactttgatgatacacaagctatagccgacaacacagataattgtatattcaagatgaattactttctgttaaaggacgcgaagaaattcattcccaaatgctcgattcaactgaaagaggtgaaggcacactttaagaagtcagaggatgactacatcttgagcgacaaagagaagttcgcatcaccattggtgattaagaagtccacgtttctattagctacagcacatgttaaaggcaagaaaggtaatataaagaaattccagaaggagtattccaaggagaacccaactgaatatagaaatagtttaaatgaatggattgcattctgtaaagagttcttgaagacttataaggcagcaactatatttgatattacaaccttaaagaaagctgaagaatatgcggatatagtagagttctataaggatgtcgacaatttgtgctacaagttagaattctgccctataaagacctctttcattgagaacctcatcgataacggtgatctatacctgtttcgaattaataataaagacttctctagtaagagtaccggaaccaagaacttgcatacactttacttacaggctatctttgatgaacgaaatttgaataatcctactataatgttaaatggaggagctgaactattctataggaaagaaagtatagagcagaagaacagaattacacataaagcgggtagtatactagttaacaaggtatgtaaagatggaacgagcttagacgataagataagaaacgagatctatcaatatgagaataaatttattgacaccctatctgatgaggccaagaaagtcttgccaaatgttattaagaaagaagccacccatgatataacgaaggataagagatttacttctgataaatttttctttcattgtcctttgacgataaactataaagagggagatacaaagcaatttaacaacgaagtactatcgttcttaagaggtaacccagatattaacataatcggtattgatcgaggtgaacgaaatctgatatatgtcactgtgattaaccagaaaggcgagatccttgactccgtaagtttcaacactgtaacgaacaagagttcgaagattgaacagacagtcgattatgaagagaagcttgctgttagagagaaagaaagaattgaagctaaacggtcgtgggactcaatttcgaagatagccaccctgaaagaaggttatctatctgccatcgtacatgaaatatgcttactaatgattaagcacaatgcaatagttgtacttgagaatctgaatgctggattcaagagaattagaggtggtcttagtgagaagagtgtatatcagaagttcgagaagatgttaattaacaaattgaattatttcgtttctaagaaggaaagtgactggaacaagccgagcggtctactcaatggtctacagctatcagaccagttcgagtcatttgagaagctaggaattcagagtggtttcatattctatgttccggcggcttatacatccaagatagatcctacgactgggtttgccaacgttctaaatctatctaaggttcggaatgtagatgcaatcaaatcgttcttctctaactttaatgaaatctcatattcgaagaaagaagcattattcaaattctccttcgatttagattcattgagtaagaaaggatttagttctttcgtaaagttctctaagtctaaatggaatgtatacaccttcggcgagaggataattaaaccaaagaataagcaaggataccgtgaagacaagagaattaatcttacatttgaaatgaagaagttattaaatgaatacaaggtgagtttcgatcttgagaacaacctgattccaaacctcactagcgctaatttgaaagatactttctggaaagagctatttttcatcttcaagacgacgttgcagctaagaaactcagttacaaacggaaaggaggatgtgctaatttcaccggtcaagaatgctaagggtgagttctttgtaagcggtactcataacaagacacttccacaagattgtgatgcaaacggagcttatcatattgctcttaaaggcttgatgatccttgaaagaaacaacttggtgagagaagagaaggataccaagaagattatggctatctccaatgtcgactggttcgaatatgtacagaagcgacgaggtgttctttga

SEQ ID NO: 266 - DNA, 4005 bp, Artificial Sequence
  Description of Artificial Sequence: Synthetic polynucleotide
atgtcgtctcttaccaaatttacgaacaagtattctaagcaactcactataaagaacgagctgattcccgttggtaagactcttgagaatattaaagagaatggattaattgatggcgatgaacaattaaatgagaattaccagaaagccaagattattgttgatgacttcttacgggacttcattaacaaggccctcaacaacactcaaattggtaattggagagaattagctgatgctcttaataaagaagatgaagacaatattgagaagttgcaagacaagattagaggtataattgtgtccaagttcgagacattcgacctgttctcaagttactcaattaagaaagatgagaagattattgatgacgataatgatgttgaagaagaagaactggacttgggaaagaaaacgtcctcctttaagtacatctttaaaaagaacttgtttaaattagtactacccagctaccttaagactaccaatcaagataaactcaagattatatcctcctttgacaactttagcacatacttcagaggattctttgagaaccgtaagaacatattcactaagaagcccatttctacaagcatagcttacaggatcgttcatgataacttcccgaaattcctagataacataagatgcttcaatgtttggcaaaccgaatgtccacagttaatagtcaaggcagataactacctaaagagcaagaatgtcattgccaaagacaagtcacttgccaattatttcactgtaggagcttatgattatttcttatcccagaacggtatcgacttctataataatattattggcggacttcccgcgttcgctggacacgaaaagattcaaggtttaaatgaatttatcaatcaagaatgccagaaagattcagaactcaaatcgaaattaaagaatagacacgcattcaagatggccgtcttatttaaacagatactctcagacagagagaaatcatttgtaatagatgaatttgaaagcgatgcgcaagttatcgatgcagtgaagaatttctatgctgagcaatgtaaagacaacaacgtcatctttaatctgctaaatctaatcaagaatattgctttcttgtcagatgacgaattggatgggatatttatagagggcaaatatttgtcaagcgtatcccagaaactttacagcgattggagcaagctaaggaacgacatcgaagattcagcaaactctaaacagggaaacaaggaattagctaagaagataaagacaaacaaaggtgatgtcgagaaagctatctccaagtacgaatttagcttgagcgagttaaacagtatcgttcacgacaacactaagttctcagacctgctgtcgtgtacgttacataaggtcgcttcagagaagttggttaaggtaaatgaaggtgattggcccaagcacttaaagaataacgaagagaagcaaaagattaaagaacctttggacgcgttattagaaatatacaacacactgctcatcttcaattgcaagagcttcaacaagaatggtaatttctatgtcgactatgatcgttgcattaatgaactatcgtctgtagtctacctttataataagactagaaactattgtacaaagaaaccatataatactgacaaatttaagttgaatttcaatagcccacagcttggcgagggtttcagcaaatctaaagagaatgattgcctaaccttgttattcaagaaggatgataactattatgttggaattatacgaaagggtgcgaagattaactttgacgatactcaggcaatcgcggacaacactgacaattgcatattcaagatgaactacttcttgttaaaggacgcaaagaagtttattcccaaatgctctatacagttgaaagaagtcaaggctcattttaagaaatccgaagatgattatatcctaagcgacaaagagaagttcgccagccctttagttataaagaaaagcacattcttattggcaacagctcatgttaagggtaagaagggtaatataaagaagtttcagaaggaatatagcaaagagaaccctactgaatatagaaactctttgaacgaatggattgccttctgtaaggagttcctgaagacctacaaggcagccacaatattcgacataactactttaaagaaagctgaagaatacgcggacatagttgagttctacaaagatgttgataacttatgctataaattggagttctgccctataaagacatccttcattgagaacttaatcgataacggcgatttatatctgttcagaattaacaacaaggacttctcttctaaatctacgggtactaagaaccttcataccttatacctacaagcaatattcgatgaacgaaatttgaataatcctactataatgctaaatggtggtgcagagctattctatcggaaggaaagtattgaacagaagaatagaatcacgcataaagctgggtctatccttgtaaacaaagtgtgcaaagacgggacttcccttgacgataagatacgcaatgaaatatatcagtatgagaataaatttattgatacgttgagtgacgaagctaagaaagtattgcctaatgttatcaagaaggaagctacacacgatatcactaaagacaagagattcacaagcgataaattcttctttcattgcccactgaccattaactacaaagaaggcgatactaaacaatttaacaatgaggtgctgtcattcttaagaggtaatcctgatataaacatcattgggattgatagaggagaaagaaacttaatatatgttaccgttataaaccagaaaggtgagatcttagattccgtatcattcaatactgtcacgaataaatcaagtaagattgagcaaactgtcgattacgaagagaagctcgccgtaagagagaaggagcgtatcgaagccaagagatcttgggatagtattagtaagattgctaccctaaaggaaggttatctgtctgctattgtccacgaaatatgtttactaatgattaagcacaatgctatagtggtcttggagaatcttaatgctggcttcaaacgcatcagaggtggtctttccgagaaatctgtttaccagaaatttgagaagatgctaataaacaagcttaactacttcgtttccaagaaggagagtgactggaacaagccatctggtttattaaatggattgcagttgagtgatcaattcgaaagtttcgagaaattaggtatccaaagtgggttcatcttttacgttcccgcagcttacacatctaagattgacccaacgactggcttcgctaacgtgttgaatctttccaaagtacgtaatgtagacgccattaagtccttcttctccaactttaacgaaatatcctattcaaagaaggaggcactattcaagttcagctttgatttggattctctatcgaagaaaggattctctagctttgttaaattctccaagagtaagtggaatgtttatacgttcggcgaacgtataattaaaccaaagaataagcaaggttaccgagaagacaagaggataaatttgacgtttgagatgaagaaacttctaaatgaatataaggtatctttcgaccttgagaacaacttaattccaaacctgacatcggcaaatctgaaggatactttctggaaagagctcttctttatattcaagacaactctacaattgcgaaattccgtaactaacggtaaggaagacgtattaatttctccagttaagaatgccaagggagaattctttgtatctggtactcacaacaagactttgccacaggattgcgacgcaaatggtgcctatcacattgcattgaaaggtctaatgatcctcgagagaaataatttggtcagggaagagaaagacacgaagaaaattatggctatctcaaatgttgattggtttgaatatgtgcagaagagacgtggtgttctctaa

SEQ ID NO: 267 - DNA, 4005 bp, Artificial Sequence
  Description of Artificial Sequence: Synthetic polynucleotide
atgtcttcccttaccaagtttactaataaatattcgaagcagttaactatcaagaatgaattgatcccagtaggaaagaccttagagaatatcaaagagaacggacttatcgatggtgacgagcagttgaatgagaactaccagaaggctaagatcattgttgatgatttcttgagggactttattaacaaggcacttaacaatacacaaattggtaattggagggaactggcagatgctttaaataaagaagacgaagataatattgagaagttgcaagataagattagaggaattatagtctccaaatttgaaaccttcgacctgttctccagttattcaatcaagaaagacgagaagatcatcgatgacgacaatgatgtagaagaggaagaattagacttggggaagaaaacatcctcattcaaatatatatttaaaaagaatttgtttaagctagttctaccttcttacttaaagaccacaaatcaagataaactaaagattatctcctcgttcgacaatttctccacctatttcagaggtttctttgagaatcgaaagaatatctttactaagaaaccaatttcaacatctatagcttataggatcgttcatgacaactttcccaagttcttggataatatacgctgcttcaacgtatggcagacagaatgccctcagttaattgttaaggctgataactatctgaagtccaagaatgttatcgccaaggataagagcttggctaattacttcaccgttggtgcttatgattacttcttatcacagaacggtattgacttctacaataatattattggtggtcttccagcctttgccggtcacgagaaaattcagggcctaaacgagtttataaatcaagaatgccagaaagattctgagcttaagtctaaattgaagaataggcatgctttcaagatggcagtactcttcaagcaaattctttcagacagagagaaaagctttgtcattgatgagttcgaatcagatgctcaggtaatcgatgctgtcaagaacttctacgctgagcaatgcaaagacaataatgttatatttaacttgcttaacttaatcaagaacattgccttcctaagcgatgatgagttggatggtatctttattgaaggcaagtatttatcttctgtctcccagaaactgtattctgactggagtaaactaaggaatgacattgaggattctgccaattcgaagcaaggcaacaaagaactagcgaagaaaatcaagacgaataagggtgacgttgagaaggcaattagtaaatatgaattcagtttgtcagaacttaactcaattgtccatgataatacgaaattctccgacttattgagctgtacactccacaaggtggcatcagagaaattggttaaagtgaatgaaggtgattggcccaaacatttaaagaacaacgaagagaaacagaagattaaagaaccgctggatgcgttgttggaaatatataataccctactaatctttaattgtaaatcctttaataagaatggaaatttctacgtggattatgatcgctgtataaatgagctttcaagtgtggtgtatttgtataacaagactagaaattactgtacgaagaaaccatacaacacagacaaattcaaactaaacttcaattcgccacagcttggagaaggattcagcaagagtaaggagaatgactgtttaacattactatttaagaaagatgacaattactatgttgggattatccgcaaaggagctaagatcaacttcgatgatacccaagcaatcgcagataacacagacaattgtatcttcaagatgaattacttccttctgaaagatgcaaagaaatttattcccaagtgttctattcaactgaaggaagtcaaggcgcacttcaagaaatcagaagacgactatatattaagcgataaagagaagttcgcgagccctctggttattaagaagagcaccttcctccttgcaacggcgcatgttaaaggcaagaagggaaatattaagaaatttcagaaggaatacagcaaggagaacccgacagaatatcgtaatagtttgaacgaatggatagctttctgtaaagaattcttgaagacttacaaagccgctacaatattcgacatcactactctgaagaaagcagaggaatatgccgatattgtcgaattctacaaggacgtggataatctctgttataagttggaattctgtccgatcaagacttcgtttattgagaatctgattgacaacggagatttatacttattccggattaacaataaagacttcagttcgaagagtaccggaaccaagaatttgcatacattgtatctacaagctatatttgatgaaagaaatctgaataatcccacaattatgttgaatggcggcgctgaattattctatcgcaaagaaagcatcgaacagaagaacaggataacacacaaagcaggctctatattggtgaacaaggtttgtaaggatggcacatctctcgatgataagatacgtaacgaaatttatcaatacgagaataaattcatagatactttaagtgacgaagccaagaaagtcctgcctaacgtcataaagaaggaagctactcatgatatcacaaaggataaacgctttacctctgataagtttttcttccattgtcctttgaccataaactataaggagggtgatactaagcagtttaataacgaagtactatcattcttgcgaggcaatcctgatatcaatatcatcggcatagacagaggcgaaagaaacttgatatatgtaaccgttataaatcagaaaggtgaaattctggattcagtctcgttcaatacagtaactaataagagctcgaagattgaacaaactgtagattacgaggagaagttagcagtgagagagaaggaaaggattgaagcaaagagaagttgggattcaatatccaagattgctaccttgaaagaaggttacctatctgcgatcgtacacgaaatttgcctgcttatgataaagcataacgctattgtagtcctggagaatcttaatgccgggtttaaacgtattcgaggaggcttgtcagagaagtcagtataccagaaattcgagaagatgttgataaataaacttaactacttcgtatcaaagaaagaatctgactggaataagccatcgggattattgaatggactacaattgagcgatcagtttgaaagcttcgagaaactaggtattcagtctggtttcatattttatgtaccagcagcctatacttcgaagattgatcctactactggcttcgcaaacgtgttaaacctgtcaaaggtacgcaacgtagatgcaatcaagtcattcttctctaactttaacgagatatcgtatagcaagaaagaggctttattcaagttctcattcgatctcgactcgttaagtaagaaaggattcagtagtttcgtcaagttctcgaaatccaaatggaatgtctatacatttggcgaaagaattatcaaaccaaagaataagcagggttacagagaagacaagagaataaacttgactttcgaaatgaagaaattgttaaatgagtataaggtatctttcgatcttgagaataatttgattcctaatttgacatctgcgaatctaaaggacaccttctggaaggagcttttctttatctttaagacaacacttcaactaagaaattcagtgactaacggtaaagaagatgtcttaatctctccggtgaagaatgctaagggtgagttcttcgtctcgggcacccataacaagacgctgccgcaagattgcgatgctaacggagcgtaccatatagcattaaagggtttaatgattctggagagaaacaacctagtgagggaggagaaggatacaaaaaagatcatggcaatttccaatgtagattggtttgagtatgtgcagaaaagacgaggagtcctgtag

SEQ ID NO: 268 - DNA, 4005 bp, Artificial Sequence
  Description of Artificial Sequence: Synthetic polynucleotide
atgtcgtccctcacaaagtttacgaataaatatagcaaacaactaacaatcaagaacgaattaataccagttgggaagacgttagagaatattaaggagaacggcctgatagacggcgatgaacaattaaacgagaattatcagaaagcaaagattatcgtcgacgacttcttaagagatttcataaataaagccttaaataacacacaaattggcaattggcgggaattggcagacgcattgaacaaagaagacgaggataatattgagaaactgcaagataagatccgaggaatcattgtctcgaaattcgaaaccttcgatttattctcgagttatagtatcaagaaagacgagaagattatagatgacgataatgacgttgaagaagaagaattggacttaggtaaaaagacgtctagcttcaaatatatctttaagaagaatctcttcaagctagtactaccatcttatcttaagacgactaatcaagataaactgaagataatttcatcgtttgataactttagcacatacttcagaggtttctttgagaaccgaaagaatatatttacaaagaagcccatttcaacttcaatagcttacagaattgtccatgacaacttccctaaattcttagataatattagatgcttcaacgtgtggcaaacggaatgccctcaattaattgttaaggctgataactatctaaagtctaagaatgtgatcgctaaggataaatcgctggctaattatttcacggtaggtgcatatgactacttcttaagtcagaatggtatcgacttctacaataacattattggaggtttacctgctttcgcaggtcatgagaagatacaaggactcaacgagttcattaaccaagaatgtcagaaggatagcgagcttaagtccaaacttaagaacagacacgcctttaagatggctgtactattcaaacagatattaagtgacagggagaaatctttcgttattgatgaattcgaaagtgatgcacaagtgattgatgctgtaaagaatttctatgctgaacagtgcaaagataacaatgtgatattcaacttactaaatttgatcaagaatattgctttcttaagtgacgatgaactagatggtatcttcattgaaggcaaatacttgagtagtgtttcgcagaaactttactctgactggtctaaactaagaaacgacatagaggactccgcaaattctaagcagggtaataaggaacttgcaaagaagattaagacaaataaaggcgatgtggagaaggctatctcgaaatatgaattctctctgtcagaactaaatagtattgttcacgataacaccaagttctcagacttgcttagttgcactcttcataaggttgcttcagagaaactggtcaaagttaacgaaggtgattggcctaagcatttaaagaataatgaggagaaacagaaaataaaggaaccactagatgcactgctcgaaatttataataccctattaatctttaactgcaagtcatttaataagaatggtaacttctatgtggattacgatagatgtattaatgagttgagtagtgttgtctacttatacaacaagacacgaaactattgtacaaagaaaccgtacaacaccgacaaattcaagttaaacttcaacagtcctcaattgggagaaggtttctctaaaagcaaggagaatgattgcctaactttattgtttaagaaggatgataattattacgtaggaataattcggaagggtgcaaagatcaatttcgatgacacacaagctattgctgataacacagataattgtatatttaagatgaactacttcctactaaaggacgcgaagaagtttatacctaaatgcagtatccaattaaaggaagttaaagcacatttcaagaagtccgaagatgactacatcctgagtgataaagagaaattcgcttcacctctggttataaagaaatcaacgttcctcttagccaccgcccacgttaaaggcaagaagggtaacataaagaagtttcagaaagagtacagtaaggagaaccctacggaatacagaaattctttgaatgagtggatagcgttctgcaaagagttcctaaagacttataaagcagcaaccatattcgatattactacactcaagaaagccgaggaatacgctgacatcgtggaattctataaagatgtcgataatctctgttacaaacttgagttctgtccaatcaagacatcattcatagagaacttaatagataatggagacttgtacctatttaggattaacaacaaagacttcagctccaaatcgacgggaactaagaatctgcatacgctatatctccaagctatatttgatgaacgaaatttgaataacccaacaataatgttgaatggcggagcagaattattctatagaaaggaatccatagaacaaaagaaccgtataactcataaggcaggatctatactggtcaataaggtttgtaaggatggtacgtcgttagatgataagataagaaacgaaatttatcaatatgagaacaaatttatagataccttatccgatgaggcaaagaaagtcctacctaacgttataaagaaagaggccactcatgacataacgaaagacaagagatttactagtgataaattcttctttcattgtcccttgacgattaattataaagaaggtgacacgaagcaattcaataatgaagtactttccttcttaagaggaaacccagacatcaacattatcggcattgaccgcggagaacgtaacttaatttatgtaactgttataaatcagaagggagaaatattagactcagtatcctttaacacggtaaccaacaaatcaagcaagattgaacaaacagtcgattatgaagagaaattagccgtgagagagaaagaacgtatagaggcgaagagaagctgggattcaatatcgaagattgccactttgaaagaaggttatctgtccgcaattgtacatgagatttgtctgttaatgattaagcataacgcaattgtcgtattagagaacttaaatgccggatttaagaggatcagaggaggtcttagcgagaagtcggtttaccagaagttcgagaagatgcttatcaataaacttaattactttgtgagtaagaaggaaagcgattggaacaagccgtcgggacttctgaacggcctgcaactttctgatcaatttgaaagctttgagaagttaggtattcaatcgggattcatattctacgttccagctgcgtacactagcaagatcgatcccaccacaggtttcgctaatgttctaaacttgtctaaagtccgtaatgtggatgctatcaaatcattcttctccaacttcaatgaaatatcgtacagtaagaaggaggccttgtttaaattcagtttcgatcttgatagtctttccaagaaaggtttctccagcttcgtgaagttctctaagtcaaagtggaatgtttatacattcggagaaagaatcattaaacctaagaataaacaaggatacagggaagacaagaggattaaccttactttcgaaatgaagaaattattaaacgaatataaggttagcttcgacttggagaataatttgattccaaatttaacatctgctaatttaaaggatacgttctggaaagagcttttcttcatattcaagacgactttacaattgagaaatagtgtaactaacgggaaggaggatgttcttatatctccggtaaagaatgctaaaggtgaattctttgtttcaggaacccataacaagacacttccacaagattgcgatgccaacggtgcttatcatattgccttgaagggtctgatgatattggaaagaaacaatcttgtgagggaagagaaagatactaaaaagataatggctatttcaaacgttgactggttcgaatatgttcagaaaagacgtggtgtgttatga

SEQ ID NO: 269 - DNA, 4005 bp, Artificial Sequence
  Description of Artificial Sequence: Synthetic polynucleotide
atgtcctctttaaccaagttcacaaataaatatagtaaacagttgacgataaagaatgaattaattcctgttggtaagacacttgagaacattaaagagaacggtcttattgatggtgatgaacaattgaatgagaattaccagaaagccaagataattgtagatgactttcttagggactttataaacaaggcgttgaataatacccaaattggaaactggagggaattggccgacgccttaaacaaagaagatgaagataacatagagaaacttcaggacaagattagaggaattatagttagcaagtttgagacatttgatcttttctcaagctactctatcaagaaggatgagaaaatcatagatgatgataatgatgttgaagaagaagaattggatctgggcaagaagaccagcagctttaaatatatcttcaagaagaacttgtttaagttagtcttgccaagttaccttaagacgacgaaccaggacaaactcaagataatttcatcctttgataacttctcgacctactttcgcgggttcttcgagaaccgcaagaatatcttcacgaagaagccaatctcaacatcaattgcctatcgcattgttcacgataattttcctaagtttcttgacaatattcgttgctttaatgtatggcaaaccgaatgtcctcaattgattgtgaaagcggacaactatttgaaatccaagaatgtgattgctaaagataagagtttagcgaattacttcaccgtgggcgcttatgattacttcctatcacagaacggtattgacttctacaacaatattattggcggcctaccagcgttcgcaggacacgagaagatacaaggtttaaatgagtttataaatcaggaatgtcagaaagactctgaattaaagagtaagttaaagaacagacatgcctttaagatggccgtcctctttaaacaaattcttagcgatagagagaaaagtttcgtaatcgacgaattcgagagtgatgctcaggtcatcgacgcagtcaagaatttctacgccgagcaatgtaaagataataacgtgatcttcaatctgttaaacttaattaagaatatcgccttcctatcggatgatgaattagacggcatattcatcgaaggaaagtatttgtcaagtgttagtcagaagttgtactccgattggtccaagttaaggaacgatatcgaggattccgctaattcgaaacaaggaaataaggaactagccaagaagattaagacgaataagggtgacgtggagaaagcaatttcgaaatatgaattctccttatccgagttgaactctattgtacatgataacactaagttcagtgatctattatcgtgtacactacacaaagtggcctccgagaaactggttaaggtgaatgaaggtgattggccaaagcatttgaagaataacgaagagaagcagaagattaaggaacctctcgacgccttgcttgaaatttataataccttgctaatatttaattgtaaatcatttaacaagaatggtaatttctacgttgattatgatcgttgtattaatgaactatcttcggttgtttatttgtacaacaagacgcgaaactattgcactaagaagccttataacacagataagtttaagctaaactttaacagtcctcagttaggtgagggtttctctaagagtaaggagaacgattgcttgacattattgttcaagaaagacgacaattactacgtgggtattattcgtaagggagccaagattaactttgatgatacacaagcaatagcagataatacagataattgcatctttaagatgaactacttcttactgaaggatgctaagaaatttatacccaagtgtagcattcaattgaaggaagttaaggctcatttcaagaaatctgaagatgattacatcttatccgataaagagaagttcgcgtcacctctagttataaagaaatcaactttcttacttgcaaccgctcatgttaaaggaaagaagggtaacattaagaaatttcagaaagaatatagcaaagagaatccaacagagtatagaaactctcttaatgagtggattgcgttctgcaaagaattcctgaagacttataaagctgcaaccatctttgacataacaactttgaagaaggctgaagagtacgcagatatcgttgagttctataaagacgttgacaatctttgctataaattggaattctgtccaatcaagacttctttcattgagaatttaattgataacggagatttatacttattccgcataaacaataaagatttcagttccaagtctactggtacaaagaatctccatacgctatatttacaagctatatttgacgaacgcaatttgaataacccaacaattatgcttaatggtggtgcagaactcttctaccgcaaagaatctattgaacaaaagaacagaattacacataaagcgggttctatcctcgtgaataaagtttgcaaagatggtacgagtttggacgacaagatccgtaatgagatttatcaatatgagaataagtttattgatacactttcagatgaagcaaagaaagtccttccgaatgttattaagaaggaagcgacacacgatattaccaaagacaagagattcacttccgataagttcttctttcattgtccactgactattaattataaggaaggtgatacgaagcaattcaataatgaagtgttgagcttcttaagaggtaatccggacattaatataattggtattgatagaggtgaaagaaatttgatttatgttacagttattaaccagaagggtgaaatactggattctgttagcttcaatacagtcaccaataagagttccaagattgaacaaaccgtcgattacgaagagaagctggcagtaagagagaaagaaagaatagaagcaaagagatcgtgggactcaatatcaaagatcgctaccctgaaagaaggttacctatcagccatcgtgcatgaaatctgtctgctaatgatcaagcataatgccattgttgtcctagagaacttaaacgctggattcaagagaattagaggtggactcagtgagaagtctgtctaccagaaatttgagaagatgctcatcaacaagctaaattacttcgtaagtaagaaagaatcagattggaataaacctagcggccttctaaacggtttgcaactttctgatcaatttgaatccttcgagaaattaggcatccaaagtggctttatattctatgtgccagcagcttacaccagcaagattgatccaactactgggttcgcaaatgttcttaacttgtctaaggtacgtaacgttgacgcaatcaaatccttcttctctaacttcaacgaaatttcttattcaaagaaggaagctctgtttaaattctcatttgatcttgattcgctttcgaagaagggcttctcttcattcgtcaagttctcaaagagtaaatggaacgtttacacattcggtgagagaatcattaagccaaagaataaacagggttacagggaggataaacgtattaacctgacatttgaaatgaagaagttattgaacgagtataaagtctcattcgacttagagaacaacttaattccaaaccttacatccgccaatcttaaagacactttctggaaggaacttttcttcatattcaagacaaccttgcaactaagaaactccgttacgaatgggaaggaagacgtattaatatctcctgtcaagaatgctaaaggtgagttcttcgtttccggtacacacaacaagacccttccacaagattgtgacgctaatggtgcatatcacattgcacttaaaggtctgatgatacttgaacgtaacaatttagtaagagaggagaaggataccaagaagattatggcaatttcaaatgttgattggtttgaatacgtgcagaagcgccgaggagttctttaa

SEQ ID NO: 270 - DNA, 4005 bp, Artificial Sequence
  Description of Artificial Sequence: Synthetic polynucleotide
atgtcttctctcacgaagtttacaaacaaatacagcaaacagttaacaataaagaatgagttgatccctgttggtaagacgctagagaatatcaaagagaatggattaatcgacggtgacgagcaactaaacgagaattaccagaaggcaaagattattgttgatgatttcctgagagatttcattaacaaggcactcaataatactcagatcggtaattggagagaattggctgatgcattaaacaaagaggatgaagataacattgagaaattacaggacaagattagaggcatcatagtatctaagtttgagacgttcgatttgttctcctcgtattcaataaagaaggatgagaaaataatcgacgacgacaacgacgtcgaagaggaggaactagatctaggcaagaaaacatcctccttcaagtacatcttcaagaagaatctattcaaattagtgttgccctcctacctcaagaccaccaatcaagacaagctaaagattatcagctcgttcgacaatttctctacttactttcgtggtttctttgagaaccgtaagaacatcttcacaaagaagccaatatcaacatcaatagcctacaggattgttcatgataatttccctaagttcttagataatattaggtgcttcaatgtatggcaaacagaatgtccgcaacttatagttaaggctgataattatttgaagtccaagaacgttattgccaaggataaatcccttgctaactacttcacagttggtgcatacgattactttctatctcagaacggcattgacttctataataatatcatcggaggccttcctgcgttcgccgggcatgagaaaatccaaggactgaacgaatttatcaaccaagaatgtcagaaggactcagagctaaagtctaaactaaagaatcgtcacgcattcaagatggcggtattattcaaacaaatattgagcgatagggagaaatccttcgtaattgatgagtttgagtcagacgcgcaagtaattgatgcagtaaagaatttctatgccgaacaatgtaaggataataatgttatcttcaatttgctaaatctaatcaagaacatcgcattcttgagtgacgatgaactggatggcatctttattgaaggtaagtacctgtcatctgtttctcagaaattatatagtgattggtccaagttgagaaatgacatcgaagattcagctaattctaagcaaggcaacaaagagctggcgaagaaaattaagaccaataaaggagacgtcgagaaagcgatctctaaatatgaatttagcttgtcagaactgaattctatcgttcacgacaatacgaagttctccgacctgttaagttgtactttacacaaggtagcatcagagaagcttgtaaaggtgaatgaaggcgactggccaaagcacttaaagaacaatgaagagaaacagaagatcaaagagccattggacgccttactagaaatatacaacaccctactaatcttcaactgtaaatctttcaataagaatgggaacttctacgttgattacgacagatgtattaatgagttatcctctgtcgtttacttatataacaagacgcgaaattactgtacaaagaaaccatacaacactgataagttcaaacttaacttcaattcaccacaattaggagaaggtttctctaaatccaaggagaatgattgcctaactttactgtttaagaaagacgacaactattatgtcgggataatccgtaagggagctaagatcaactttgatgatacccaggcaatcgccgataacactgataattgtatattcaagatgaactacttcctgctgaaagatgccaagaaatttatccctaagtgtagcattcaactaaaggaggttaaagcacactttaagaagtcggaagatgactatatattgtctgataaagagaaatttgcatcaccgttggtaatcaaaaagagtaccttcctgttagctactgcacacgttaaaggaaagaaaggaaacataaagaaattccagaaagaatactcgaaggagaatccaactgaatatagaaactcacttaatgaatggatcgcgttctgtaaggaatttctgaagacttataaagctgctacgatcttcgatataacaacattaaagaaggccgaggaatacgcagacatcgtagagttctacaaagatgttgataatctttgttataaacttgagttctgtccaataaagacctccttcatagagaacctgattgacaatggtgatctttatctattcagaattaataacaaagatttcagttcgaagagcactggtaccaagaatttacatactttatatctgcaagctatcttcgatgagagaaatcttaacaatccaactattatgttaaatggcggagctgagttattctataggaaagaatccatcgaacagaaaaataggatcacccataaagctggctccattctagtcaataaggtatgcaaggatggtacttctttggatgacaagattagaaacgaaatttaccagtacgagaacaaattcatagacacattgagcgacgaagccaagaaggtattaccaaacgttataaagaaggaggccacgcatgatataactaaggacaagaggtttacttcagataagttcttctttcattgtccattgaccattaattataaggaaggagacactaagcagtttaacaacgaagtcttatcattcttacgaggcaaccctgacattaatataattggtatagatagaggcgagagaaatcttatctacgttactgttatcaatcagaagggtgaaatcctggattctgtgtctttcaataccgttacgaataagagctcaaagattgaacaaacggtcgactacgaggagaagttagccgtaagagagaaggaaagaatcgaagctaagagatcatgggattcaatttcaaagattgctaccttgaaggaagggtacttaagtgctattgttcatgaaatttgcctattaatgataaagcacaacgcgatagtagtcctcgagaacctaaacgccggctttaagagaatacgaggtggccttagtgagaaatctgtgtaccagaagtttgagaagatgctcattaataagttaaactacttcgtttcaaagaaagaatcagattggaacaaaccttcgggtctactaaacggtctacagctttccgaccagtttgagagctttgagaagctaggtattcagtcgggtttcatcttttacgtcccagccgcatatacatccaagattgatccgacaacaggattcgcaaatgttctaaacctaagcaaagtaagaaatgtggacgccatcaaatcgttctttagtaacttcaatgagatttcatattccaagaaagaagcgttgttcaaatttagctttgatcttgattcattatcgaagaaaggcttctcgtcatttgtgaaatttagtaaatctaagtggaacgtttatacctttggcgaaaggattattaaaccgaagaataaacaaggctacagagaggacaagagaattaatttgacattcgagatgaagaaactattaaacgaatataaagtatcattcgatctcgagaataatctgataccgaatttaacaagcgctaacttgaaggataccttctggaaggaactgttcttcatatttaagacaactctacaattgcggaattcggtgaccaacggcaaagaagacgtcctgatttcacctgtgaagaacgccaagggagaattctttgtgtctggaacccataacaagacactgccacaggattgtgacgctaacggcgcatatcacatcgcattgaaaggtttgatgatcttggaacgtaataacttggtccgtgaggagaaagacacgaagaaaattatggctatttcaaatgttgattggtttgaatatgtgcaaaagagacgtggagtgttatag

SEQ ID NO: 271 - DNA, 4005 bp, Artificial Sequence
  Description of Artificial Sequence: Synthetic polynucleotide
atgtcctcccttacaaagtttacgaataagtattccaaacaacttactataaagaatgaattaatccctgttggtaagactctggagaacatcaaagagaacggtttgatcgacggagacgaacaattaaacgagaactatcagaaggccaagataatcgttgatgacttcttaagggacttcataaacaaggcattaaataatacacaaattgggaattggcgtgagttggctgatgcacttaacaaagaagacgaagataacatagagaagctacaggacaagattagaggtattatagtttcgaaattcgaaacgttcgatttattctcttcatactcgattaagaaagatgagaagataattgatgatgataacgatgtcgaagaggaggaactggatttaggcaagaaaacatcatcctttaagtatatatttaaaaagaatctattcaagttagtcttaccatcctatcttaagactaccaaccaagacaaattgaagatcattagctcattcgataatttctcaacatactttagagggttctttgagaatcgcaagaacatctttaccaagaagcccatatctacttcaatagcttatagaattgtgcacgataacttcccgaagttcttggataacataagatgctttaatgtttggcaaactgagtgtccacaattgattgttaaggcagataattaccttaaatcgaagaatgtgattgctaaggataagtctttagcaaattacttcacagtgggtgcatatgattacttcctatcacagaacggtattgacttctacaataacatcataggaggactgccagccttcgccggacatgagaagattcaaggtttaaatgaatttatcaatcaagaatgccagaaggattcagaattgaagagcaaacttaagaatcgccatgcattcaagatggccgttctatttaaacaaattctatcggacagagagaagtcatttgttatagacgaatttgaatccgacgcccaagtgatcgatgcggtaaagaatttctacgcggagcaatgtaaggacaataatgttatattcaatcttcttaacttgataaagaacattgcattcttgtcggacgacgaattagacggcatctttattgaaggtaaatacctttcttccgtttcccagaaactgtattctgattggagcaaattgaggaacgacattgaagactcagccaattccaaacaaggcaataaggaattagcaaagaaaatcaagacgaacaaaggagatgtagagaaggcgatcagcaaatacgagttctctttgtccgaactaaattcaattgtacacgataacaccaaattctccgatctactttcatgtactttgcacaaagttgcgtcggagaagttggttaaggttaacgaaggagactggcctaagcatctgaagaacaacgaagagaaacagaagatcaaagagccgcttgatgccctacttgaaatttataacacactgctgatctttaattgtaagtcgtttaataagaatggaaacttctacgttgattatgatagatgcataaacgaattaagttccgttgtttatctatataataagactagaaactactgtaccaagaaaccgtataataccgataagtttaaattaaactttaacagtccgcaacttggcgagggcttcagtaaatctaaagagaacgattgtttaacactcctgttcaagaaagacgacaattactacgtaggcatcattcgtaaaggtgcgaagataaacttcgatgacacccaggccatagctgataatacggacaattgtatcttcaagatgaattatttcttactcaaagatgctaagaagtttatacctaagtgttccatacaactgaaagaggtcaaggctcactttaagaagtctgaggacgattacattctttcggacaaggagaaattcgcctcacctctggtaatcaagaagagtacgttcttgctggctaccgcacatgtcaagggcaagaaaggtaacattaagaaatttcagaaggaatatagtaaggagaacccaactgaatatagaaattccctaaatgagtggatcgctttctgcaaagagttccttaagacctataaagctgccaccatatttgatataactactttaaagaaggcggaggagtatgccgatattgttgagttctataaggatgttgataatttatgctataagttggagttctgtccgatcaagacgtctttcatcgagaatttgatagacaacggtgatttatatttatttaggattaacaataaagatttctcctctaagtccacaggtacaaagaatttgcatactttatatttacaggcaatcttcgatgaaaggaatttgaataatccaaccatcatgctgaatggcggagctgaactcttctatcgtaaggaatccatcgaacagaaaaatcgtatcacccacaaggctggttctatcctagtaaacaaggtatgcaaagacggaacctctttagatgacaagattagaaacgagatttaccagtacgagaacaagtttatcgatactctaagtgatgaggcgaagaaagtactacccaatgtgattaagaaagaagctacccatgacattaccaaggacaagcggttcacgtctgacaaattcttctttcattgtcctttgaccattaactataaggagggagataccaagcaatttaataatgaagtgttgtctttcctaagaggtaacccagacattaatataattgggatcgacagaggtgaacgaaatttgatttatgttacggtgattaaccagaaaggtgaaatactagatagtgtttcgttcaacacagtaacaaacaaatcctctaagattgaacaaactgtggactacgaggagaagttggctgtgagagagaaagaaagaattgaagctaagaggtcgtgggatagtatcagcaagattgctactttgaaggaagggtacctgagtgctatcgttcatgaaatttgcttgctgatgattaagcataatgccattgtcgtcctggagaatttaaatgcaggctttaagagaatacgaggaggattatctgagaaaagcgtatatcagaagttcgagaagatgctgataaacaagctcaactatttcgtgtctaagaaggaatccgattggaacaaaccctctggactgttgaatggtttgcagctgtctgatcaattcgaatcattcgagaaattaggtattcaatctggtttcatattctacgtcccggctgcctatacttccaagattgacccaaccactggctttgctaacgtactcaatcttagcaaagtcagaaacgtagatgctataaagtccttcttctctaatttcaacgaaatcagctacagcaagaaggaagcgttattcaaattctcattcgatttagattccctatccaagaaaggtttctcctcgtttgtgaaattctctaagtctaagtggaatgtttatacatttggcgaaaggataattaaaccaaagaataagcaaggttaccgtgaagataagcgtattaaccttacattcgaaatgaagaaattgcttaatgaatataaggtttcattcgacttggagaataatttaataccgaatcttacctctgcaaatttaaaggatacattctggaaagaattattctttatcttcaagacgacacttcaattaagaaatagtgtaaccaacggtaaggaagacgtacttatatcgcctgtgaagaatgcgaagggtgaattctttgtatcgggaacacacaacaagacattgccacaagactgtgacgcgaacggtgcgtaccatattgcacttaagggtttgatgatcttggagcgtaataatcttgttcgagaagagaaggatactaagaagataatggctatttctaatgttgactggtttgagtatgtccagaagagaagaggtgtcctataa

SEQ ID NO: 272 - DNA, 4005 bp, Artificial Sequence
  Description of Artificial Sequence: Synthetic polynucleotide
atgtctagtctgaccaaatttaccaataagtacagtaaacaattgacaatcaagaatgaattaatacctgtcggcaagacgctagagaatatcaaggagaatggactaattgacggtgatgaacaattaaacgagaactatcagaaggccaagattattgttgacgacttcttgagagacttcattaataaagctttaaacaacacgcaaatagggaattggcgtgagctagcggatgcattgaataaggaagacgaggataacatagagaaattacaagacaagattagaggtattatcgtatccaagtttgagacgtttgacctattctccagctattccataaagaaagatgagaagataatcgacgatgacaatgatgttgaagaagaagaattagacctgggaaaaaagacttcaagcttcaagtacatctttaaaaagaatttgtttaaattagtcttgccaagttatctcaagaccactaaccaagataagctcaagatcattagttcatttgataacttctcgacttactttagaggattctttgagaataggaagaatatatttactaagaaacctattagtacctctatcgcctataggattgttcatgataactttccaaagttcttggataacataagatgtttcaatgtgtggcaaactgaatgtcctcagttaatcgttaaagcggataactaccttaagagtaagaatgtgatagcgaaagataagtcattagcgaattacttcacggtcggcgcttacgattacttcctctcgcagaatggaattgacttctacaataacattatcggcggtttgcctgcgtttgcaggtcatgagaagatacaaggtttgaatgaatttattaatcaagaatgtcagaaagactccgaattgaagagcaagttaaagaatagacacgcgtttaagatggcagtgctattcaaacaaatcttatcagaccgagagaaatcatttgttatcgatgagtttgaatctgatgcacaagttattgatgctgtaaagaatttctacgcagaacaatgtaaggataataacgtaatctttaacttattgaatttaatcaagaacattgccttcttgtctgatgatgagttagatggcatattcatagagggtaagtatctatcgtcggtaagtcagaagctctactcagattggtctaaattgcggaatgatattgaagattcagcaaacagcaaacaaggtaacaaggaattggctaaaaagatcaagactaataaaggagatgtcgagaaggcaatttctaaatacgagttctctcttagtgaattaaattcaattgttcacgataacaccaaatttagtgatttgttaagttgtacattacataaggtggcctcggagaagttggttaaggttaacgaaggtgattggccgaagcacctaaagaataatgaggagaaacaaaagattaaagagccactggatgctctcctcgaaatttataatactctactaatattcaattgcaaatctttcaacaagaatggaaatttctatgtcgactacgatagatgtatcaatgaattatcctctgttgtttacctatataataagactagaaactattgtacgaagaagccatataatacagataaatttaagttgaacttcaattctcctcagttgggtgaaggcttctccaaatcgaaagagaacgattgcttgacactgctatttaagaaggatgataactactatgtaggtattataaggaagggtgcgaagatcaacttcgatgatacacaagctattgccgacaacactgacaattgtatattcaagatgaattatttcttgttgaaggacgcaaagaagttcatccctaaatgttcgatccaattgaaagaggttaaggctcatttcaaaaagagtgaagatgattacattctatcagataaagagaagtttgcttctccattggttataaagaaatcgacattcctgttagctactgcccacgtcaaagggaagaagggtaatatcaagaagttccagaaagagtattcgaaggagaacccgaccgaatataggaactcactcaacgaatggatcgcgttctgcaaagaatttctcaagacgtacaaggctgctacaatcttcgatataacaacactgaagaaagcagaagaatacgccgacatcgtagagttctataaagacgtcgataatttatgttacaaactggaattctgtccgataaagacctcatttatagagaatttaattgataacggtgacttatatctatttagaattaataataaggacttcagcagtaagtcaaccgggacaaagaacctacatactctttacttgcaagctatctttgatgagcgtaatctgaacaatccaactattatgttgaatggtggagctgaactgttctacaggaaggagagtatagaacagaaaaatagaataacgcacaaagctggttcaatattggtaaataaagtgtgcaaagacggtactagtttagacgacaagatcagaaacgaaatttatcagtacgagaacaaatttatcgataccctttctgacgaagctaagaaggtactgccaaatgtgattaagaaagaagccacccacgatatcacgaaggataagagattcactagtgataagttcttcttccattgtcctttgactattaattacaaggaaggagatactaagcagttcaacaatgaggttctgtctttcttgagaggaaatcctgacattaacattatcggaatcgatcgtggagaaagaaatttaatttatgtaactgttatcaaccagaagggagagatactagatagcgtttctttcaatacggtgacaaacaagagttctaagattgagcaaactgtagattatgaagagaaacttgccgtcagagagaaggaacgcatagaagcgaaacgtagttgggattctatctctaagatagcaactttaaaggaaggttatttatcggccatagtacacgagatttgcttgctaatgattaagcataatgctatagtagttctcgagaatttaaacgcgggttttaagagaattagaggaggtctatcggagaagagtgtttaccagaagttcgaaaagatgctaattaacaaattgaactacttcgtttcgaagaaagaatcagattggaataaaccatctggtctgcttaatggattacaattgtctgatcaattcgaaagtttcgagaagttaggtatacaaagtggatttatattctatgtgccagctgcttatacttcaaagattgaccctactaccgggttcgctaacgtcttgaacctttctaaggtccgtaatgtagacgcaatcaagagttttttctcaaatttcaatgaaatatcatactcaaagaaggaagctctcttcaagttctctttcgacctggattcactatctaagaaaggcttctcctcctttgttaagttctccaagtctaaatggaatgtttatacattcggagaacgaattatcaagccaaagaataagcaaggttacagggaagataagagaatcaatttaacattcgaaatgaagaagttgttgaatgaatataaagtgtcctttgatctagagaataatttgatcccaaacttaacaagtgcaaatcttaaggataccttctggaaggaactgttctttatatttaagaccactctgcagcttagaaacagtgttaccaatggtaaagaagatgttctgataagtccggtaaagaatgctaaaggtgagttctttgtttcaggtacacacaacaagactttgccacaagactgcgacgcaaatggagcttaccacatcgctttgaagggtttaatgatcttggagaggaacaacttagttagagaggagaaggatactaagaagatcatggcaatttccaacgtggattggttcgaatatgtgcagaagaggcgtggtgtcttgtga

SEQ ID NO: 273 - DNA, 4005 bp, Artificial Sequence
  Description of Artificial Sequence: Synthetic polynucleotide
atgtccagtctaactaagtttacgaataagtattcaaagcaactcactatcaagaatgaactaatacctgtagggaagactttggagaacatcaaggagaatggtttgatagatggtgatgagcagctaaacgagaactatcagaaagccaagataatagtagatgacttcttaagggacttcataaacaaggctttgaataatacgcaaattgggaattggcgggagctcgctgatgcgctgaacaaggaggacgaagataacattgagaagcttcaggataagattagaggtattattgtgagtaaatttgaaacatttgatctctttagtagttactctataaagaaagatgaaaagattatcgatgatgataatgacgtagaagaagaggaactggacttaggcaaaaagacaagttcatttaaatatatattcaagaagaacttatttaaactcgtattacccagttatctcaagacgacaaaccaagacaaactgaagatcatatcatctttcgacaacttctctacatacttccgaggcttcttcgagaacaggaagaatatattcacgaagaagcccatatccacgtcaattgcatatagaattgtacatgataacttccctaagttcttagataatataaggtgcttcaatgtatggcaaacagaatgtcctcaattgattgtcaaagcagataactatttgaagagcaagaatgtcattgctaaagataagtccctagcaaattatttcacggtgggtgcttacgattacttcttgtcacagaacggtatcgatttctataataacattataggcggtcttcctgctttcgctggccacgaaaagatacaaggtcttaacgaatttataaatcaggaatgtcagaaggatagcgagttgaagtctaaattgaagaatagacacgcatttaagatggctgtcctattcaaacaaatattatctgatagagagaagtctttcgttattgatgaatttgaaagtgatgcacaagtgatcgatgccgtaaagaacttctacgcagaacaatgtaaggataacaacgtgatattcaatctacttaacttgatcaagaatattgcattcttatctgatgatgaattggacggtatctttatcgaaggcaaatacctttctagcgtgtctcagaaactctatagcgactggtccaaattacggaatgacattgaagatagtgcaaattcgaagcagggaaataaagaattagctaagaaaattaagaccaacaagggcgacgtcgagaaggcgatttctaagtatgaattctctttatcagaattaaacagtatagttcatgataatacgaagttctccgatctgctaagttgtacactacacaaggttgcttccgagaaattagttaaggtcaatgaaggtgattggcctaagcatctaaagaacaatgaagagaagcagaagattaaggagcctctggatgcactattggaaatctataacactctacttatcttcaattgtaaatcatttaacaagaatggtaacttctatgtggattacgatagatgcatcaacgaattatcaagcgtggtctacttgtacaataagacccgaaattactgtaccaagaaaccatataacactgacaagttcaagctgaacttcaattctcctcaattaggtgaaggattcagcaaatctaaggagaacgactgtttgacactcctctttaagaaagatgataactattacgtcggcattattaggaaaggagctaagatcaacttcgatgatactcaagcgatagcggataatactgataattgtatattcaagatgaactatttcctattgaaagacgctaagaagtttattccaaagtgttccattcaactgaaagaagtgaaggcccatttcaagaaatcagaggatgattatatcttgagtgataaagagaagtttgcctctccgctggtcataaagaaatctaccttcctgcttgcaaccgctcatgttaaaggtaagaaaggcaacattaagaaattccagaaagaatactcaaaggagaatccgactgaatacaggaactctttgaacgaatggatagcgttctgtaaagagttcctgaagacttataaagcggcaacaatatttgacatcacgacattgaagaaggccgaagaatacgctgatatcgtcgagttctataaagatgtagataacttgtgttacaagctagagttctgtccaattaagacatctttcatagagaacctgattgataacggagatttgtatctatttagaattaataacaaggacttctctagcaagtccactggtactaagaatttacatacattgtatctccaagccatcttcgatgaacgtaatctcaataatcctacaattatgttgaatggtggtgcggaattgttctaccggaaggagtctattgaacagaaaaatagaattacacataaagccggatctattctagttaataaggtttgcaaggatggtacttcactggacgacaagatcaggaatgaaatctaccagtacgagaacaaattcattgatactttgtccgatgaagctaagaaagtgttacctaacgttatcaagaaggaggctacccatgatatcaccaaggataagcggttcacctcagataagtttttctttcattgcccacttacgataaactacaaagaaggagacaccaaacagtttaataacgaagtattatccttcttacgaggcaaccctgatattaatattataggtatcgacagaggtgagcgtaacttgatctatgtaactgttattaatcagaagggagagatattagactcggtgagtttcaacacagtcacaaacaaatcaagcaagatcgagcaaacggttgattatgaagagaagttagcggttagagagaaagagcgaatcgaagcaaagaggagttgggacagtatttctaagattgctactttgaaagagggatacttatctgctattgtgcacgagatttgtctattgatgattaagcataatgcaattgttgtactagagaacttaaatgcaggattcaagaggatcagaggtggtttatctgagaagtcggtctatcagaagttcgagaagatgttaattaacaagctaaactatttcgtctctaagaaagaaagtgactggaacaaaccatctggcctattaaacggtcttcaattgagcgaccagttcgaaagtttcgagaagttgggaatccaaagtggattcatattctatgtgcccgccgcttatacttcgaagatagatcctactactggatttgcgaatgtccttaatctaagtaaggttagaaatgtagacgccataaagtcgttcttctctaacttcaacgagatatcttactctaagaaagaggcgttgttcaaattcagctttgatctagactccctttctaagaagggcttctcctccttcgtgaaattttcaaagagtaaatggaatgtttacactttcggtgagagaattattaaaccaaagaacaagcaaggataccgagaagataaacgaattaatcttacgtttgaaatgaagaaattgttaaacgagtataaggtctcatttgatttggagaataacttgatacctaatcttacttcagcgaatttgaaagatactttctggaaggagttgttcttcatcttcaagaccaccttacaactcaggaattctgttacgaacgggaaagaggacgtgttgattagcccagtaaagaatgctaagggagaattcttcgtaagcggtactcataataagacactaccacaagactgcgatgccaatggtgcctatcatattgctttgaaaggcctgatgatattagaacggaataatcttgtaagggaagagaaggatactaaaaagattatggctatctccaatgtcgactggtttgaatacgttcagaagcggcggggggtattgtag

SEQ ID NO: 274 - DNA, 4005 bp, Artificial Sequence
  Description of Artificial Sequence: Synthetic polynucleotide
atgtcttccttaactaaatttactaataagtattccaagcagcttacaataaagaatgaattgatccctgttgggaagacattagagaacatcaaagagaacgggctaattgatggcgatgagcagcttaacgagaattaccagaaagcaaagatcatagtggatgatttccttagagacttcataaataaagctttgaacaacactcaaataggaaattggagagaattagctgacgcactaaacaaggaggacgaggacaacatagagaaactccaggataagatacgaggaatcattgttagcaagtttgaaacattcgacctcttctcttcatacagtataaagaaagacgaaaagatcattgatgatgataatgatgtcgaagaagaagaactggatttaggtaaaaagacctcctcgttcaaatatatctttaaaaagaacctattcaaactcgtccttccaagttatctaaagacgactaatcaagataaacttaagatcatttcatcgttcgacaacttctcaacctacttccgtggattctttgagaatcgtaagaatatctttactaagaagcctatttctacttctattgcttacagaatcgttcatgacaacttccctaagtttctagataacattagatgcttcaacgtctggcaaacagaatgtccacaactaatagtgaaagctgataactatctaaagtcgaagaatgtcatcgcgaaggataaatcactcgcgaattactttacagtcggtgcctatgattatttcttgtcacagaacggaatagacttctataacaatatcataggtggtttaccagcgtttgcagggcacgagaagatacaaggtttaaatgaatttattaatcaagaatgtcagaaggatagtgaattaaagagtaaactaaagaaccgtcacgcatttaagatggctgtgttattcaaacagatcttatccgatagggagaaatcatttgtcatcgatgagtttgaaagtgacgctcaagtcatagatgcggttaagaacttctatgccgagcaatgtaaagataataatgtgatctttaacttgctcaacttgataaagaatattgccttcttgtcagatgatgaactagatggaatatttattgagggtaagtatctgtcttcggtaagtcagaaactgtactctgattggagtaagttacgtaatgacatcgaagacagtgcaaattctaaacagggaaataaagagttggcgaagaaaattaagaccaacaagggcgacgttgagaaggcaatttctaaatacgaattctcactctccgagttgaactctattgtccatgacaatactaagttctccgacttactatcgtgcactttgcataaggttgcatctgagaaattggtcaaggtcaacgagggagattggccgaagcatttgaagaataacgaagagaagcagaaaataaaggaaccattggacgcactacttgaaatctataacacattattaatctttaattgtaagtcattcaataagaatggtaatttctatgttgattacgataggtgcataaatgagttgagcagcgtcgtatatctttacaacaagacaagaaactactgtactaagaagccatacaatacggacaaatttaagcttaacttcaattcaccacagctaggcgagggcttctccaaatcaaaggagaatgattgcttgacgcttctatttaagaaagacgacaactactacgtgggtataatccgtaagggtgctaagataaacttcgatgatacccaagccatagcggataacactgataactgtatctttaagatgaattacttcttgttgaaagatgcaaagaaatttattcccaaatgttccattcaattgaaggaggttaaagcgcactttaagaaatccgaagacgactatatactcagtgataaagagaaattcgcttcgccgctcgttattaagaaatcgacattcttacttgccactgcacatgtgaaaggaaagaagggcaacattaagaaattccagaaagaatattcgaaggagaatccaaccgagtacagaaatagtttaaacgaatggatcgcattctgcaaagaatttttaaagacatataaggcagcaactatctttgacattactacactgaagaaggcagaggaatacgctgatatcgttgaattctacaaagacgttgataatttgtgttataaattggaattctgccctattaagacatcatttatcgagaacctaatcgataacggcgatttgtacttgttcaggatcaacaataaagatttcagttcaaagtctaccggaactaagaatctacacacgttgtacttacaagctatcttcgatgaacgaaatttgaacaacccaactatcatgttaaatggtggagccgaattattctacaggaaggagtcaatagaacagaaaaacaggatcacacacaaagcgggctcgatacttgtcaacaaagtttgcaaagatggaacatcacttgatgataagataaggaacgaaatataccagtatgagaataaattcattgatacattgtccgatgaggcgaagaaagttctccctaacgtaatcaagaaagaagccactcacgatattacgaaggataagagatttacgtccgataagttcttctttcattgtccattaacaattaattacaaagaaggtgatacgaagcaatttaacaatgaggtgttgtctttcttacgcggaaatccagatattaatattataggaatcgacagaggtgaaagaaatttaatatacgtaaccgtaattaaccagaagggtgaaatacttgactctgtttctttcaacacagttaccaataaatccagcaagattgaacaaacagttgattatgaagagaagttagccgtaagagagaaggaaagaatcgaagcgaagagaagttgggactcaattagcaagattgccacattgaaagaaggctatttgtcagcaatcgttcacgagatctgcttgttgatgattaaacacaacgctattgtagtactagagaatctaaatgctggctttaagcgaatacgtggcggcctaagcgagaagtcagtttaccagaagttcgagaagatgttaattaataagttaaactactttgttagcaagaaggaatcggattggaacaaaccctcaggcttgctgaatggattacaactatccgaccagttcgagagtttcgagaagttgggtatacaatctggctttatattctatgttccagccgcctatacctctaagatagatccgacgacagggttcgcaaatgtattaaatttgtccaaggttaggaacgtggacgcaatcaagtctttcttcagtaactttaatgaaatctcatactccaagaaagaagccttgtttaagttctcgtttgatttggacagtttgtctaagaaaggattctctagcttcgtcaaattctcaaagagtaaatggaacgtctatacgtttggcgaacgcatcatcaagccgaagaataaacaaggttatagagaagacaagaggataaatttaactttcgaaatgaagaagttgctgaatgaatataaggtatcatttgatttagagaacaatttaattcctaacctaaccagtgctaatctcaaggacactttctggaaagaactattctttatctttaagacaacgcttcagcttagaaactccgtgactaatggtaaggaagatgtattgataagccctgtcaagaatgccaaaggcgagttctttgtctccggtacccataacaagacgcttccgcaagattgcgatgcaaacggagcataccacatagctttgaagggtcttatgatacttgagcgtaacaaccttgttagggaagagaaagacacgaaaaagattatggctatttcaaatgtagactggtttgaatacgtacagaagaggagaggtgtgttatga

SEQ ID NO: 275 - DNA, 4005 bp, Artificial Sequence
  Description of Artificial Sequence: Synthetic polynucleotide
atgtcgagtctgacgaagtttacaaacaaatacagtaaacaacttaccatcaagaatgagttaataccggtcggcaagacactagagaatattaaagagaatggtttgatcgacggagatgaacaattgaatgagaactatcagaaggccaagataatagtggatgacttccttagggacttcataaacaaagcccttaataatacccaaatcggcaactggagagaattggcagatgcactaaacaaagaagacgaagataacatagagaagttgcaagataagattagaggaattattgtaagtaagtttgaaacattcgatctatttagcagttacagtattaagaaagacgagaagattattgacgacgataatgacgttgaagaagaggagctggatctgggtaagaagacaagcagtttcaaatatatatttaagaagaacctctttaaattagtacttccgtcttaccttaagacaactaaccaagataagcttaagatcatttcgtcattcgataacttctctacctactttcgggggttctttgagaaccggaagaacatatttaccaagaaaccgatttccacatcgattgcatataggattgttcacgacaactttcctaaattcttagacaatattcgttgtttcaatgtttggcaaactgaatgcccgcaacttatagtgaaagcagacaattatctaaagtcaaagaacgtgattgcgaaggataagtcattagctaattactttactgtaggcgcttatgactacttcctgtcacagaatgggattgacttctataacaatattattggtggtttacccgcatttgccggtcatgaaaagattcaaggtttgaacgaatttattaaccaagaatgtcagaaggactccgaacttaagagtaaattaaagaacagacatgcgttcaagatggcagtattatttaaacaaatactgtctgatagggagaagtccttcgtcattgatgaattcgagtcagatgcccaagttatcgacgccgttaagaatttctatgcggaacaatgtaaagacaataacgtaatcttcaatctattaaacttgataaagaatatcgcattcctctcagatgatgaattagacggtatattcatagagggtaaatacctgagctcagtctcccagaagttgtattcagactggtctaagttacgtaacgatattgaagattccgcaaactccaagcagggtaacaaagaattagccaagaagatcaagaccaataagggtgatgtggagaaggcaatctcaaagtatgaattcagtttgtctgaattaaacagtatcgttcacgacaacaccaaattctctgatttgctatcttgcaccttacataaagtcgcttcagagaagcttgttaaagttaacgaaggagattggcccaagcacctcaagaataatgaagagaagcagaagataaaggaacctttagatgctctcctggaaatatataataccttgctcatattcaattgtaaatccttcaacaagaacggtaacttctatgttgactatgatagatgtataaacgaactttcctctgtggtctatctttataacaagactagaaactattgtacaaagaaaccgtacaatactgataaattcaagcttaatttcaatagtcctcaactaggtgaagggttcagtaagtcgaaagagaatgattgtttgacattgttatttaagaaagacgataattactatgtcggtatcataaggaagggtgcaaagataaatttcgacgatacacaagccatagctgataatactgataactgtatcttcaagatgaattacttcttactgaaggatgcaaagaaattcataccaaagtgttccatccagcttaaggaagttaaagcccattttaagaaatccgaagatgattatatattgagcgacaaggagaagttcgcttcaccgttggtcattaagaaatccacgtttctacttgcaaccgctcatgttaagggaaagaagggcaatatcaagaagtttcagaaggaatacagtaaggagaatccaaccgagtacagaaatagcctgaatgaatggattgcgttctgcaaagagttcttaaagacttacaaggctgcaactatctttgatatcacaactctaaagaaagcggaagagtacgcagacatcgttgagttctataaagatgtagataacctatgttacaagttagagttctgtccgataaagactagcttcatagagaacttgatcgataatggcgacttatatttgttccgtattaacaataaggatttctcttccaagtctacaggcactaagaacctccatactttatatttgcaagctatcttcgatgagaggaatcttaataacccaactatcatgttgaatggaggagccgaactcttctatagaaaggaatccattgaacagaaaaacagaataactcacaaagctggatccatattggttaataaagtctgcaaagatggtacaagcttagatgacaagataaggaacgagatctatcaatatgagaataaatttatcgataccctttcggatgaagcgaagaaggttctgcccaatgttatcaagaaagaagccactcatgatatcactaaggacaagaggttcacctcggataagttcttctttcattgtcctcttaccatcaactacaaggagggtgacactaagcaatttaataatgaagtactgtctttcctaagaggtaatcccgacataaatatcattggaattgatcgtggtgaaaggaacttaatctatgttacagtcattaatcagaaaggtgaaatcctagattctgtatcgttcaatactgtcactaataaatcttcgaagattgagcaaacggttgactacgaggagaaattggcagtaagagagaaggaaaggatcgaagcgaagagatcatgggactctattagcaagatagcgacacttaaggagggttatctatctgcgattgtacatgaaatctgtttattaatgataaagcacaacgcaattgtagttcttgagaaccttaacgcgggatttaagcgtattagaggcggtttgtcagaaaagagcgtttaccagaagttcgagaagatgttgattaataagctaaattacttcgtgtccaagaaggagtcggactggaacaagccatcaggcctcctcaatggtttgcagctctcggatcaattcgaatcatttgagaagctaggtattcaaagcggatttatcttctacgtgccagcagcttatacttctaagattgacccgacaacaggcttcgcaaacgttcttaatttgagcaaggtgcgaaacgttgacgctataaagagtttcttctctaactttaacgaaatttcctatagtaagaaagaagccttattcaagttttctttcgacctagattcactatcaaagaagggattctcatcctttgttaaattcagtaagagtaagtggaatgtgtataccttcggcgaacgtataatcaagcctaagaataagcagggttaccgcgaggataagaggataaatttgacattcgaaatgaagaagttattaaatgaatataaagtttcattcgacttagagaacaacttaatcccaaatctcacatccgcaaatttgaaagatactttctggaaagaactattcttcatctttaagacgactctgcagcttcgcaatagcgttaccaatggcaaagaagatgttctaattagtcccgtaaagaatgctaaaggtgagttcttcgtctctggcacacacaacaagacacttcctcaggactgtgatgcaaatggtgcatatcatatcgcactgaaaggcctcatgatcctagaaagaaataatctcgttcgtgaagagaaagacacgaaaaagatcatggctatatcgaacgtagattggtttgaatatgttcagaagagaagaggagtcttgtaa

SEQ ID NO: 276 - DNA, 4005 bp, Artificial Sequence
  Description of Artificial Sequence: Synthetic polynucleotide
atgtcttccctaaccaagtttactaacaagtattctaaacaactgactataaagaatgagttgattcccgtggggaagacacttgagaatattaaagagaacgggttgattgatggagatgaacagttgaatgagaactatcagaaggcaaagatcatagtagacgacttcctgagggacttcatcaataaagccttaaataatacacagataggcaattggagagaattggctgacgctttgaataaagaagatgaagacaatatcgagaaactgcaggacaagattcgtggcatcatcgtatccaaatttgagactttcgatttatttagttcatattctattaagaaagatgagaaaatcatagatgatgataatgacgtggaagaagaggaattggaccttggtaaaaagacctcttcatttaaatacatcttcaagaagaacctattcaagcttgtacttccgagttatttaaagactactaaccaagacaagctgaagattatatccagcttcgacaatttcagcacttactttagaggcttcttcgagaaccgaaagaatatattcacgaagaagccgatatccacatctattgcctataggatagtccacgataactttccaaagttcttggacaatataagatgtttcaacgtttggcaaaccgaatgtccacaactgatcgttaaggcagacaactatttgaaaagcaagaatgttattgctaaagataagagccttgcaaattatttcacagtaggtgcttacgattacttcttgtctcagaatggaattgatttctataataatataataggtggtttgcctgcgttcgctggtcacgagaagattcaaggcctaaatgagttcataaatcaagagtgtcagaaagattctgagctaaagtctaaactcaagaataggcacgcattcaagatggcggtactctttaaacaaatcctatcagacagagagaaatctttcgttattgacgaatttgagtcagatgcacaagttatagatgctgttaagaatttctatgccgaacaatgtaaagataataacgttatatttaatttattaaacctaataaagaatatcgcattccttagcgatgacgaattggatggtatatttatcgaagggaagtatctttccagcgtttcacagaagctgtactcggactggtcgaagttgagaaacgacatagaggattccgcaaattctaagcaaggaaataaagaattagctaagaagatcaagactaacaagggtgatgtggagaaggcaatctcaaagtacgagtttagtttgagcgaattgaactccatagtgcatgataacactaaattctctgatttgctttcttgcactctccataaagttgcttctgagaaattggtcaaggttaacgaaggagattggccgaaacatctgaagaacaatgaagagaagcaaaagatcaaagaacccttggatgctttattggaaatttacaacaccttgttaatctttaattgcaaatcatttaataagaatggtaacttctatgtggattacgacaggtgcattaatgaattgtcttctgtcgtttacctgtataacaagactaggaactactgcactaagaaaccatataatactgataaatttaaacttaacttcaactcaccacaacttggagaaggcttctctaagagtaaggagaatgattgtctgactttgctcttcaagaaggatgataattattatgtaggcataatccggaaaggtgctaagatcaatttcgacgacactcaagccatagccgataataccgataattgtatcttcaagatgaattacttcttgctaaaggatgcgaagaaatttatacctaaatgtagtattcaactcaaggaagtcaaggcacatttcaagaaatctgaggacgattatatcttgtctgacaaggagaaatttgcttcgccgttggttatcaagaagtccaccttcctcttagctactgcccatgtaaagggaaagaaaggcaatataaagaagtttcagaaagaatactccaaggagaaccctactgaatacagaaatagtttgaatgaatggattgccttctgcaaagaatttcttaagacttacaaggctgcaaccatcttcgatataacaactctaaagaaagctgaagaatatgccgatatcgtggaattctacaaggacgttgataatttgtgttacaagttagagttctgtcctataaagactagtttcattgagaatctaattgataatggtgacttatatctgtttcggattaacaacaaggacttcagcagcaaatccaccggtaccaagaatctccacaccctatacctgcaagccatcttcgacgaaagaaacttgaataatccaactattatgctgaatggcggcgcagagttattctataggaaagagagtattgaacaaaagaacagaataactcataaggctggaagtatattggtaaacaaagtatgtaaagatggaacctcattagatgataagatcagaaatgaaatataccaatacgagaataaatttattgacactttatcagatgaagctaagaaagtccttccaaacgttattaagaaggaagctactcatgatattactaaagacaagagatttacgtctgataagttcttctttcattgcccactaactattaattataaagaaggcgatactaaacagtttaataatgaggtcttaagtttcctacgtggcaatcctgacattaatataattggaattgatagaggtgaaagaaacttaatatacgtcacagtaataaatcagaaaggagaaatccttgatagtgtctcatttaacaccgtgacaaataaatcgtctaagatcgaacaaaccgttgactacgaggagaaattagctgtcagagagaaagaaaggattgaggctaaacgctcatgggatagtattagtaagatagccactttaaaggagggatatttgtcggccattgttcacgaaatttgcttgctaatgatcaagcataatgcgatcgtagttcttgagaatttaaacgcaggttttaagagaattagaggtggtctttctgagaagtccgtttaccagaagttcgagaagatgttaattaacaaattaaattacttcgtatccaagaaggagagcgattggaataagccatctggtctcttaaacggtttacaacttagcgatcagttcgaatccttcgagaaactgggtatccagtctggctttattttctacgtcccagcagcatatacatctaagatagatcctactactggcttcgcaaacgttctaaatttatcgaaggttaggaacgttgatgcaattaaatcgttcttttcaaatttcaacgaaatctcttacagtaagaaggaagctttgtttaagttctcctttgatcttgacagtttatccaagaaaggcttctcatcattcgtaaagttctctaaaagtaagtggaacgtttataccttcggagaacgaattattaagcctaagaataaacaagggtatagagaggataagagaataaaccttactttcgaaatgaagaagttgttaaatgaatataaagtatcatttgatctggagaataacctgatcccaaatcttacttcagcgaatttgaaggataccttctggaaggaattgttcttcatattcaagacaacgttacaacttcgaaatagtgttacaaatggtaaagaggatgtgttaatttctccggtcaagaacgcaaagggtgaattcttcgtttctggtacacacaacaagacactgccacaagattgtgacgctaatggtgcttaccatattgctctaaagggattgatgatcttggaacgcaacaacttggtcagagaagagaaagacaccaaaaagataatggctatctcaaatgtggattggtttgaatatgtacagaaaagaagaggagtactctga

SEQ ID NO: 277 - DNA, 4005 bp, Artificial Sequence
  Description of Artificial Sequence: Synthetic polynucleotide
atgagttcattaacaaagtttacaaataaatatagcaaacaattgaccataaagaacgagttaattccagtaggtaagactttggagaacatcaaagagaacggtctgatagatggtgacgaacaactcaatgagaattatcagaaggcaaagattatcgttgacgacttcttaagggactttatcaataaggctctgaacaacactcagattggtaattggagagagttagcggatgcattgaataaagaagacgaggataacatagagaagcttcaagataagatcagaggtataattgtgagtaagttcgaaacattcgatttattctcatcttatagtataaagaaagatgaaaagataattgatgacgataatgatgtcgaagaagaagagttagacttgggcaaaaagacaagtagctttaaatacatcttcaagaagaatctattcaaactggtacttccgtcatacttgaagacaacaaatcaggataagctaaagatcatttcatcattcgacaacttctctacttacttcagaggcttcttcgagaatagaaagaacatcttcaccaagaaacctatttcaacatccattgcgtaccgcattgttcacgataacttcccaaagtttctagataacataagatgctttaacgtgtggcaaaccgaatgtcctcaactgatagtgaaagcagataattacctcaagtctaagaatgttattgcaaaggataaatctttagccaattatttcacagtgggtgcatacgactacttcttgtcacagaacggtattgacttctataacaacattataggtgggttacctgctttcgctggtcacgagaaaatccagggtttaaatgagtttattaaccaagaatgtcagaaagactcagaacttaagtctaagttaaagaacagacatgcatttaagatggccgtcttattcaaacaaattctaagtgatcgtgagaagtccttcgttattgacgaattcgaatctgatgctcaagttattgatgccgttaagaatttctacgccgaacaatgtaaggataacaacgtcatattcaacttgttaaatttgatcaagaatatagcattcttatctgacgatgaattagatggcatatttatcgaaggtaaatatttaagctctgtttcacagaagttgtactcggattggtctaaactcaggaacgacattgaagattctgctaattcgaagcaaggtaacaaagaattggctaagaaaattaagacaaacaagggagatgtagagaaggcaataagcaaatatgagttctctctatcagaattgaactccattgtacatgataatactaagttctctgacttgttgagttgtacattgcataaagttgctagtgagaagctggtgaaagtgaacgaaggtgactggccgaagcatctgaagaacaacgaagagaagcagaaaattaaggagccgttggacgcgttgttagaaatctataatactttattaatctttaattgtaagtcatttaacaagaacgggaatttctatgtagattatgatagatgcatcaacgaattgtcttctgttgtctacttgtataataagacaagaaattactgtacaaagaaaccatacaatacagataagttcaaactaaacttcaattctccacagttgggagaaggtttctccaagtccaaggagaacgactgcctgacactattattcaagaaagacgataactattatgtgggtataattaggaagggcgcaaagattaactttgacgatactcaagctattgcggataacacagataattgtatcttcaagatgaattatttcttattgaaagacgcaaagaagtttattcctaaatgttccattcaactaaaggaagtcaaggcacactttaagaaatctgaagacgattatatacttagtgataaagagaaatttgcgtctcctttggttattaagaagagtaccttcctccttgccacggcccacgttaagggcaagaaaggaaacataaagaaattccagaaggaatattctaaagagaacccgactgaatatagaaactccttaaatgagtggatcgcgttctgcaaagagttcttgaagacgtacaaagcagcaaccatcttcgatatcacaaccctaaagaaagccgaggaatatgccgatatcgttgagttctataaggacgttgataacttgtgttataaattagaattctgtccaatcaagacatcatttattgagaatttaatcgataatggtgatttatatctcttccgtattaacaataaggatttctcgagtaaatctactggtacaaagaatttacatacactgtatttgcaagcgatcttcgatgaaagaaatctgaataacccaacgatcatgctaaacggcggagctgaactattctaccggaaggaatccatcgaacaaaagaatcgaatcactcacaaggccggatctatcctagtgaataaggtatgtaaggatggtacatctttggatgacaagatacgaaatgaaatataccaatacgagaataagttcatagacacactatctgacgaagcaaagaaagtccttccaaatgtaataaagaaagaagctacccatgacattactaaagacaagagattcacgagcgataagttcttcttccactgcccattgaccataaattacaaggaaggtgacactaaacaattcaataatgaagttctatcctttctaagaggcaatcctgacatcaatattatcggtattgaccgaggcgaaagaaacttaatttatgtgactgttataaaccagaaaggtgaaatattggactctgtttcctttaatactgtgacgaacaagtcttctaagatcgaacaaactgttgattatgaagagaaattggctgtgagagagaaagaaaggatcgaagcgaagagaagctgggattccattagtaagatagccacattgaaagaaggttacttgtcagctatagttcatgaaatttgtctgctgatgatcaaacataacgctatagttgtcttagagaatttgaacgctggctttaagagaataagaggcggcttgagtgagaagtcagtctaccagaagttcgagaagatgttgatcaacaaacttaactatttcgtaagtaagaaagaatcagattggaataaaccttccggtttgctaaatggactacagttatcggatcaatttgaaagtttcgagaagttgggtatacagagcggctttatcttctacgtacctgcagcatatacttcaaagattgatccaactaccggtttcgcaaacgtgctgaatctctcgaaggttcggaatgttgacgccatcaagagtttcttttctaacttcaatgagatttcgtattctaagaaagaagctctattcaaattctctttcgatctagattcattgtctaagaagggcttctcgagcttcgttaaattcagtaagagcaagtggaatgtctatacctttggcgagaggattatcaaacctaagaacaaacagggctacagggaagataagagaattaacttgaccttcgaaatgaagaagctattgaacgaatacaaagtttccttcgatctagagaataatctgataccaaacctaaccagtgcaaatctgaaagataccttctggaaagagttgttcttcatatttaagaccactttgcaattgcgtaactctgttaccaacggcaaggaggacgttctcatctcacccgtcaagaatgctaagggtgagttcttcgtctcagggacacataacaagactttaccgcaggactgcgatgcgaacggagcataccatatagcgttaaagggcttaatgatactggaaaggaataatttggtccgagaagagaaggatacgaagaagataatggccatctccaacgttgattggttcgagtatgttcagaagagaagaggagttctataa

SEQ ID NO: 278 - DNA, 4005 bp, Artificial Sequence
  Description of Artificial Sequence: Synthetic polynucleotide
atgagctcattgaccaaattcaccaacaaatattcaaagcaattaacaattaagaacgaattaattccggttggcaagactctggagaacattaaggagaacggtttgatcgatggtgatgaacaattgaatgagaactaccagaaggcgaagattatcgttgacgacttccttagggacttcattaacaaggctcttaacaacactcaaattggaaattggcgggaacttgcagacgcgctaaacaaagaagatgaagataacattgagaagttacaagacaagattagaggaattatcgtttccaagttcgaaacattcgacctgttctcatcctatagcataaagaaggatgagaagataattgatgatgataacgacgtcgaagaggaagagttggatttgggcaaaaagacttcttccttcaagtatatcttcaagaagaatttgttcaaattagtactgcctagttatctgaagaccactaatcaggataaattaaagatcatttcttcattcgataacttctctacttacttcagagggttcttcgagaatagaaagaacatatttaccaagaaacctatttcaacctctattgcatacagaattgtacatgataatttccctaagttcttagacaacattagatgcttcaacgtctggcaaaccgaatgcccacagcttattgtcaaagcagacaattacttgaagagcaagaatgttatcgctaaagataagagcttggccaactatttcactgtgggtgcctacgactacttcctaagccagaacgggatagatttctataacaatataattggtggattaccagcatttgctggtcacgagaaaattcaaggtttaaacgaatttattaaccaagaatgtcagaaagactctgagttgaaatctaaattaaagaacagacatgcgttcaagatggcagtgctgtttaaacaaatacttagtgatagggagaaatcgttcgttatagacgaattcgagtcagatgcccaagtaatcgatgctgttaagaatttctacgcagaacaatgtaaagataataatgtcatctttaatttactcaatctgataaagaatattgcattcttgtcagatgatgaattagatgggatcttcattgaaggcaaatacctatcttccgtgtctcagaaattatattctgattggtcaaagttgaggaatgacatcgaggattcagcaaactccaagcaaggtaacaaagaattagccaaaaagattaagacaaacaaaggagacgttgagaaagcaatctccaagtacgaatttagtttatcagaactaaatagtatagttcatgataacactaagtttagtgatctgttgtcttgcactttgcataaagttgcaagcgagaagttagttaaagtcaatgaaggtgactggcctaaacatctaaagaacaatgaagagaagcagaaaatcaaggaacctctggacgcattattggaaatttataataccttgttaatattcaattgtaagtcatttaacaagaatggtaatttctatgttgattacgatagatgtataaatgagctatcttctgtggtttacttgtataacaagactagaaattattgcacgaagaagccatacaatactgacaagttcaaattaaactttaatagtcctcagctgggagaaggtttctcgaagagcaaggagaatgactgtctcacactactatttaagaaggacgacaattattatgttggtataataaggaaaggtgctaagatcaactttgatgatacacaagctatagcagacaacactgataattgcatctttaagatgaattatttcttattgaaagacgctaagaaatttatcccgaagtgttctattcaactcaaggaagtcaaagcccacttcaagaagtccgaagatgactacatactatccgataaagagaagttcgcatcgccgttagtgattaagaagtctacgttcttgctagctaccgctcatgtgaaaggaaagaagggtaacataaagaaatttcagaaggaatattcaaaggagaatcctacggaataccgtaactcgttaaatgaatggattgcattctgtaaagaattcctcaagacatacaaggctgcgactatattcgatattacaactcttaagaaagcagaggaatacgctgacatcgtagagttctataaggacgttgataacctatgctacaagctggaattctgtccgataaagacctccttcatagagaacttgattgataatggtgatctgtacttgtttagaataaataacaaggacttctcatctaagagtaccggaacgaagaaccttcacactttatatttacaagcaatattcgatgaaagaaatttaaataatcctacaataatgttaaacggaggagcagaattgttctatcgcaaggaaagcatcgaacagaagaacagaatcactcacaaggcgggcagtatcttagtaaataaggtgtgtaaagatggtactagtcttgatgataagatacgcaatgaaatttatcaatatgagaacaaatttatagatacactatcagatgaagctaagaaagttctcccaaacgttattaagaaagaggctacgcatgacattaccaaggacaagaggttcacatcagacaaattcttctttcattgcccgcttacaatcaactacaaagagggcgatactaaacagtttaacaatgaagttctaagtttcttaagaggtaatcctgacattaacatcatcggaattgatcgcggagaaagaaacttgatttatgtaactgtgattaatcagaagggagagatcttggactctgtttcgttcaataccgtcaccaataaatcttccaagattgagcaaacagtcgactacgaggagaaattggctgtcagagagaaagaaagaatagaagcgaagaggagctgggatagcatcagtaagattgcaacgctgaaagaaggttatttgtcggctatagtacatgaaatttgtttgttgatgataaagcacaacgcaattgtggtactcgagaatctcaatgcaggtttcaagcgaataagaggaggattaagtgagaaatcagtataccagaagttcgagaaaatgttgattaataagctaaattactttgtctcgaagaaagaaagcgactggaacaaaccatctggactattgaatggacttcaactttctgatcaatttgagtcatttgagaagttgggcatacaaagtggcttcatattctatgtgcctgcggcttacactagtaagatcgatccaactacgggattcgcaaacgtactgaatttatctaaggtcaggaatgtcgacgcaataaagtccttcttctccaacttcaatgaaatttcatattctaagaaggaagctttgtttaagttctcgttcgatctggattctctttcaaagaaaggattctcaagcttcgtaaagttctctaagagtaaatggaacgtttataccttcggagaaagaatcattaaaccgaagaataagcaaggttacagggaagataagagaattaatttaacctttgaaatgaagaagctcttaaatgaatacaaagtaagcttcgacctagagaacaatttaataccgaatcttacatccgccaatttgaaagacacattctggaaagagttattctttatattcaagaccaccttgcaactgagaaacagcgttactaacggcaaggaagatgtcttgatttctccggttaagaatgccaagggtgagttcttcgtttctggcacgcacaacaagactctgccgcaagactgtgatgccaacggcgcctaccatattgctctcaagggtctaatgattctggaacgtaataatttagtaagagaagagaaggacacgaagaaaataatggccatctccaatgttgactggtttgaatacgttcagaagaggagaggagtcctgtaa

SEQ ID NO: 279 - DNA, 4005 bp, Artificial Sequence
  Description of Artificial Sequence: Synthetic polynucleotide
atgtcaagtctgaccaaatttacgaacaagtatagcaaacagctaactattaagaacgaattgatacctgttggaaagacattggagaacattaaggagaatggattaatagatggtgatgagcaactgaatgagaactatcagaaggcgaagatcattgttgatgacttcctacgggactttattaacaaggcgttaaacaacacccaaataggaaattggcgtgaattagccgatgctctaaataaagaggatgaagataatatcgagaaattgcaggataagattcgtggtatcatcgtaagcaagttcgaaactttcgatctcttctcaagttactcaattaagaaagatgaaaagattatcgacgatgacaacgatgtcgaagaagaagagttagatttgggaaagaagacttcctccttcaagtatatcttcaagaagaacttatttaaacttgtgctaccatcatacctgaagactacgaaccaagataaactgaagatcatctctagtttcgacaatttcagtacctatttcagaggattcttcgagaacagaaagaatatattcactaagaaaccaatctccacttccatcgcttaccgtatcgttcatgataacttcccaaagtttctagataatattagatgcttcaatgtttggcaaaccgaatgtccacaactaattgtcaaggccgataactatttgaaatccaagaacgttattgcaaaggacaagtctttggctaattactttacggtcggcgcgtatgattacttcttgagccagaatggtatcgatttctataacaatataatcggcggtctgcctgccttcgctggccatgagaagatccagggtcttaatgaatttataaaccaagaatgtcagaaggatagcgaattgaaatccaagttgaagaatcgtcatgcattcaagatggcagtactatttaaacagatactatcggatagagagaaatcctttgtaattgacgaatttgagagtgacgctcaagttattgatgctgtgaagaacttctatgctgaacaatgtaaggataataatgtaatatttaacttattgaatctaattaagaatatcgcgtttctatcagatgacgaactggatggaatctttattgaaggtaagtatttatcgtcagtaagtcagaaattatattcagattggtctaaattgagaaatgatatcgaagatagcgccaattcgaaacaaggcaataaggaactagcaaagaagatcaagaccaataagggtgacgtggagaaggcaattagtaaatacgagttctctctatccgaattaaattcaatcgttcatgataatacgaagtttagtgatttgttatcctgtacattgcataaagtagcgtcagagaaactcgttaaagtaaacgaaggtgattggcccaaacatttgaagaataatgaggagaaacagaagatcaaagaaccgttggacgcgctgctggaaatatacaacaccttgcttatattcaactgcaagtccttcaataagaatggtaacttctatgtggattacgatcgttgcattaacgaactttcctccgtagtttacttatacaataagacacggaattattgcaccaagaaaccatataacacagacaaatttaagctgaacttcaactcacctcaactcggtgaaggtttctccaaatctaaagagaacgattgcctgacattattattcaagaaggatgataattattacgttgggattattcgaaagggagcaaagataaacttcgatgatacgcaagctattgctgataatacggataactgtatctttaagatgaactatttcttactaaaggatgcaaagaagtttatccctaaatgtagcatacaattgaaggaagtgaaagctcattttaagaagagcgaagatgattacatactgtctgataaggagaagttcgcatcaccgttagttataaagaaatccacctttcttctggctactgcccacgttaaggggaagaagggaaatataaagaagtttcagaaggagtatagtaaagagaatcctacagagtacagaaattcactcaatgaatggatcgctttctgtaaagaattcttaaagacctacaaggcggccacgatcttcgatataacaactttaaagaaagctgaagaatacgccgatattgttgaattctacaaagatgtagataatttatgctataagctagaattctgcccaattaagacctcgttcattgagaacttaatcgacaacggtgatttgtatctgttcaggattaataataaggacttctctagcaaatcaacaggaaccaagaatcttcataccttatatcttcaagcgatcttcgacgagagaaacttgaacaatccaacaattatgctaaacggtggtgctgaactattctatcgaaaggagtcgatcgaacagaagaatcggattacgcacaaggcgggtagtatcttagtaaataaagtctgtaaggatggtacctcattagacgacaagataaggaatgaaatatatcaatacgagaataaatttatagatacattatctgatgaagctaagaaggtccttcctaacgtaataaagaaggaagctacccatgatattactaaggataagagattcacatcggataaattcttcttccactgcccattgacaataaattataaagagggagatactaaacagttcaacaatgaagtgctctctttcttaagaggcaaccctgacattaatataattggtatagacaggggtgaacgtaatttaatatatgttactgttatcaatcagaaaggtgaaatcctagatagcgtgtccttcaatactgttacaaataaatcttcaaagattgaacaaacagttgactatgaagagaaattggcagttagagagaaagaacgtattgaagcaaagaggagttgggacagcataagtaagatcgcgacattgaaggaaggatatttatcagccatcgttcatgagatatgtctgttgatgatcaaacataatgcgatagtggtccttgagaacctaaatgctggctttaagagaatcagaggtggtctaagtgagaaaagcgtttatcagaaatttgagaaaatgttgataaacaagcttaactactttgtctcaaagaaagaatccgattggaataagccaagtggtcttctaaatggattacaacttagtgatcaatttgagtctttcgagaagcttgggatccaatccggattcatcttctatgttcctgcagcctatacttcgaagattgaccctacgaccggctttgccaatgtattaaatttgagcaaagttagaaacgttgatgctatcaaatcttttttctctaacttcaatgaaattagctatagcaagaaagaagcattatttaagtttagctttgatctcgacagtctatcaaagaagggattctcttcattcgttaagttctcgaaatctaagtggaatgtatataccttcggagaaagaattatcaaaccgaagaataaacaaggataccgtgaagataagcgtatcaatttgacgttcgagatgaagaaattgttaaacgaatataaagtgtcgttcgacttagagaataatcttattcccaatttgacttccgctaatctcaaagacaccttctggaaagaactattctttatattcaagactacgctacagttgaggaactcagtaacaaatggaaaggaagatgtgttgatcagtccagttaagaacgccaaaggtgagttctttgtatctggtacccataataagactttgcctcaggattgtgatgcaaatggtgcataccacattgccttgaaaggactcatgatattagaaagaaacaaccttgtgagggaggagaaggacaccaaaaagatcatggcgatatcaaatgtagattggtttgagtatgtccagaagcgcagaggtgtgctataa

SEQ ID NO: 280 - DNA, 4005 bp, Artificial Sequence
  Description of Artificial Sequence: Synthetic polynucleotide
atgtcttctttgactaagtttacaaataaatattccaaacaattaaccattaagaatgaactaattccagtaggcaagacactcgagaacatcaaagagaatggtcttattgatggagatgaacagctgaacgagaattaccagaaggctaagattattgtagacgacttccttcgcgatttcataaataaagcgttgaataacactcaaattggtaattggagagaattggctgatgcattgaataaggaggatgaagataatatagagaagctgcaagacaagatccgtggaattattgtgagtaaatttgaaacgttcgatctattctcgtcttattcaataaagaaggacgagaagatcatcgatgacgataacgatgttgaagaagaagaactggacttgggaaagaagacttcatccttcaagtatatattcaagaagaacctgttcaaattagttctgccaagttatcttaagacgactaatcaagataaactcaagatcatttcctcgtttgacaacttcagtacatactttagaggtttctttgagaatcgcaagaacatcttcactaagaagcctatttctaccagcattgcttatagaattgttcatgataactttcccaagttcttagacaatataagatgcttcaacgtatggcaaaccgagtgtccgcaattgattgtcaaggctgacaattatctaaagtcgaagaatgttatcgctaaagacaagtcattagctaattactttacggtcggtgcttacgactacttcctttctcagaacggcatcgacttctataacaatatcataggaggacttcccgcctttgccggtcacgagaaaatacaaggtttgaatgaattcatcaatcaggaatgtcagaaagattcggaattgaagtccaagcttaagaatagacatgctttcaagatggctgtgctctttaaacaaatcttgtctgatcgtgagaaatcgttcgttattgatgaatttgagtctgatgctcaagtgatcgatgcggttaagaatttctatgcagaacaatgtaaggacaataatgtaatattcaacctcctaaacttgattaagaacatcgctttcttgtctgatgacgaattggatggtatctttatcgaaggcaaatacttatcgtctgtatcgcagaagctatattctgattggtctaaattgagaaatgatattgaggactcagccaattctaaacaaggtaacaaggagcttgctaagaagattaagactaataaaggtgatgtggagaaagctatttccaagtatgagttctcactttcagagttgaattcgattgttcatgataatactaagttctctgatttgttgagttgtaccctccacaaagtagcaagtgagaagttggtcaaagtaaatgaaggtgattggccaaagcacttaaagaacaatgaagagaaacagaagattaaggaaccattagatgcgctattggaaatttataacacactactgatattcaattgtaagagctttaacaagaatggaaatttctacgtagattacgataggtgtatcaacgaactatccagcgtcgtttatttatataacaagacccgtaactattgtacaaagaaaccttacaacactgataagttcaaacttaacttcaatagcccacaacttggcgaaggtttcagtaagagcaaggagaacgactgtttaacactgttgttcaagaaggacgataattactatgtgggaataattagaaagggtgcaaagattaatttcgacgatacacaggcaattgctgataataccgacaactgtatattcaagatgaactatttcttgctaaaggatgccaagaagtttattcctaagtgtagcatacaactcaaggaagttaaggcacactttaagaagtccgaagatgattacatcctcagtgataaggagaagtttgcaagccccttagttatcaagaaaagtacattcctattggctacagcgcatgttaaggggaagaaaggcaatataaagaaatttcagaaggaatacagcaaggagaatccaactgaatatagaaattctttaaatgaatggattgccttctgtaaagaattccttaagacgtacaaagccgcaactatatttgacataactacactaaagaaggctgaagaatacgctgatatcgttgagttctataaagatgtagacaacctgtgttacaagttagagttctgtccgattaagacttcgttcattgagaacttgatagataatggcgacttgtacttgttcagaattaataataaggacttctccagcaagagtacgggcactaagaatttacacacattatatttgcaggctatatttgacgagcgtaatctgaacaatcctacaatcatgttaaacggaggagccgaactgttctatcgtaaagaatcaatagaacagaaaaatcgtattactcataaggcaggtagtatactagtcaataaagtctgcaaagatggtacttcactagatgataagattagaaacgagatttatcaatacgagaataaattcattgatacgttatctgatgaagcaaagaaagttctgccaaatgtaatcaagaaagaagcgactcatgatattaccaaggataagaggtttaccagtgataaattcttcttccactgtcctcttactatcaattacaaagagggagataccaaacaatttaataacgaagttctcagcttccttcgagggaatccagacattaacatcatcgggatcgacaggggcgaaagaaatctgatatacgtcacagttattaaccagaagggtgaaatcctggattctgttagtttcaacactgttactaacaagtcgagtaagattgagcaaactgttgattacgaagagaagttagccgttcgcgagaaagagcgaatcgaagccaaacgcagctgggactctataagtaagattgcgaccctcaaagaaggttacctgtcggcaatcgtccacgagatttgtttgctaatgattaagcataatgcgatcgtggtgttagagaacttaaatgcaggatttaagagaatccgtggtggtttgtccgagaagtcagtgtatcagaagtttgagaagatgttaattaataagttgaactacttcgtgagcaagaaggaatctgactggaataaaccgtccggtctccttaacggtttgcaattgtctgatcaattcgaatctttcgagaagcttggtattcaaagcggattcatattctacgtacctgcagcgtatactagtaagattgatcctaccactgggttcgcaaatgtattaaatctaagtaaagtcagaaatgtcgacgctattaagagtttctttagcaacttcaatgaaatctcgtattccaagaaagaggctttattcaaattctctttcgatctggattcattaagcaagaaaggtttctcaagctttgtaaagtttagtaaatccaaatggaatgtttatacattcggtgaacgtattattaagcctaagaataagcaaggttatagggaagacaagagaataaatctaacctttgagatgaagaaactactgaatgaatacaaagtgagctttgacctagagaacaatttaatacctaatttgacttctgctaacttgaaagacacattctggaaggagctgttcttcatattcaagacaactttgcagttaagaaactcagttactaacggcaaagaagatgtgctaataagtccagtgaagaatgctaagggtgagttctttgtgtccgggacccataataagacattaccacaagactgtgatgcaaatggagcataccatattgctctaaagggattgatgatcctcgagagaaacaatttagtgagagaagagaaggatacaaagaaaatcatggcaatttccaacgttgactggttcgaatatgtccagaagagacgtggggtcctctag

SEQ ID NO: 281 - DNA, 4005 bp, Artificial Sequence
  Description of Artificial Sequence: Synthetic polynucleotide
atgagttctctcaccaagttcacaaacaagtatagtaaacaactcacgataaagaatgaacttatcccagtgggcaagacacttgagaatatcaaagagaatggcttaatcgacggtgatgaacaactaaatgagaattatcagaaggcaaagatcattgtggatgactttcttagagatttcataaataaggcattgaacaatactcagattgggaactggcgagaattagcagatgctttgaataaagaggacgaagataatattgagaaacttcaagacaagatcagagggatcattgtaagcaagtttgaaacgttcgatctgttctcaagctatagtattaagaaagacgagaagataatagacgatgataacgatgtagaagaagaagagcttgatttaggtaaaaagaccagttcattcaaatacatcttcaagaagaacttatttaagctagtcttaccatcttacttaaagacaacgaatcaagataagcttaagatcatctcttcattcgacaatttctctacctatttcagagggttcttcgagaaccgaaagaatatatttacgaagaagccgatatctactagtatcgcatatagaatagtgcatgataacttccctaaattcctagataatattcggtgctttaatgtttggcaaaccgaatgccctcaactgatcgtgaaggcagataactatttgaaaagtaagaatgttattgccaaagataaatcattggccaattacttcaccgtcggagcttatgattactttctgtctcagaatggcattgacttctataacaatattataggtggtttaccagcatttgccggtcatgagaaaattcaagggttgaatgaattcatcaatcaggaatgccagaaagactcggaacttaagtctaaactaaagaatcgccatgcgttcaagatggctgttctgttcaaacaaatattgtcagatcgtgagaagtcattcgtgatagatgaattcgaatctgatgcacaagtaatagatgcagtgaagaacttctacgcggagcagtgtaaggacaataacgtgatatttaatttgttaaatcttataaagaatattgccttcctttctgacgacgaactagatggtatatttattgaaggtaagtatctttcttccgtgagccagaagttgtattcggattggagcaagctaagaaacgatatcgaagattcggcaaattccaaacaaggtaataaagaactagcaaagaagatcaagacaaataagggtgatgttgagaaagcgataagtaagtacgagttctcactttctgaactaaattccatagtgcatgataacactaagttctcagatttactgtcttgcacattgcacaaggttgcctcagagaagttggtgaaagtaaacgaaggcgattggccgaagcatctaaagaataatgaagagaagcagaagattaaagagccactagatgccttacttgaaatctataacaccttacttatctttaattgcaagtcctttaataagaatggtaatttctacgttgattatgatagatgtattaatgaactctcatctgttgtttacttgtacaataagactagaaattactgtactaagaaaccttataacacagataaattcaaactcaacttcaattcacctcaattaggtgaagggttctctaagtcgaaagagaatgactgcctaacgttgttgtttaagaaagatgataactattacgttggtattattagaaagggagccaagatcaatttcgatgatactcaagcaattgctgataatactgataattgtatctttaagatgaattacttcttactcaaagacgctaagaagttcatcccgaagtgtagtatccaattaaaggaagttaaagcgcattttaagaagtccgaagatgattatatattatcagataaggagaaattcgctagtccattggttataaagaaatcgactttcttgttagcgaccgcacatgttaagggtaagaaaggcaatatcaagaaattccagaaggaatactctaaagagaatcctacagaatatagaaatagcttgaatgaatggatcgctttctgtaaagagtttctcaagacttacaaggccgcaactatctttgacataactaccttgaagaaggcagaagagtacgccgatattgtagaattctataaagatgtcgataacctttgctacaagttagaattctgtccgattaagacttcgttcattgagaatttgattgacaacggtgatctttacttgttcagaattaacaataaggatttcagctcgaaatcaactgggaccaagaacctccacacattatatttgcaagccatctttgatgaaagaaatcttaacaaccctactattatgctaaatggcggtgctgaattgttctacagaaaggaatcaattgaacagaagaatagaataacgcataaggctggttctatcctagtgaataaagtatgtaaagacgggacatctcttgatgataagattaggaacgaaatttatcaatatgagaacaaatttatcgacacattgtccgatgaggctaagaaggtgctgccgaacgtgattaagaaggaagccacacatgatattaccaaggataagagatttaccagcgacaagtttttctttcattgccctttaacgattaattacaaagaaggtgatactaaacaatttaacaatgaggttcttagcttcctacgcggtaatccagatattaatataattgggattgatcgaggtgagaggaacttgatctatgttacagttattaaccagaaaggtgaaatacttgactctgtctcatttaatacagtaactaacaagagttcaaagatcgaacaaactgttgattacgaagagaagttagcagttcgtgagaaggagagaatcgaggctaagagaagctgggattctatttctaagattgctacactgaaggaaggttatctaagtgccatagtacatgaaatctgcctattgatgattaagcataatgcaatcgtggtgttggagaatctcaatgcaggatttaagagaatcagaggaggattatctgagaagtcagtttaccagaaattcgagaaaatgttgattaacaaattgaattactttgtgagcaagaaggaatccgactggaataaaccttccggcctgctcaatgggttacaattatcggatcagttcgaaagcttcgagaaattaggcatacaaagcgggttcatcttctacgtgccagcggcgtatacctcgaagatcgatcctacaaccggatttgcaaacgttctgaacctgtccaaggtaagaaacgtagacgcaattaaatcgttcttctcaaactttaatgaaatctcatattctaagaaagaagctttgtttaagttctcgtttgacttggactctttaagtaagaagggcttctcctcattcgtgaaattcagcaaatctaaatggaatgtttatacgttcggagaaagaataattaagcccaagaacaaacagggttatagggaagataagagaattaatttgactttcgaaatgaagaagttattgaatgaatataaagtaagctttgatttggagaacaatttgataccaaaccttacatctgctaatttgaaagacaccttctggaaagaactcttctttatattcaagactactcttcaattgcgtaactcagttacaaacggtaaagaagatgtactaataagtccagtaaagaatgccaagggtgaattctttgtgtcgggaacacataataagacattgccgcaggactgtgatgcaaatggagcatatcatattgcactgaagggtttaatgattctagaaaggaataacttggtgagagaagagaaggatactaagaagataatggccatctcaaatgttgattggtttgaatacgtccagaagagacgtggcgttctatga

SEQ ID NO: 282 - DNA, 4005 bp, Artificial Sequence
  Description of Artificial Sequence: Synthetic polynucleotide
atgtcgtctttgacgaagttcacgaacaaatattctaaacaacttaccattaagaacgaacttattccagtagggaagacgttggagaacatcaaagagaacggattaattgatggagatgaacaactaaatgagaactaccagaaggcgaagattatagtagacgactttcttagggatttcataaataaagccttaaacaatacccaaattggtaattggagagaactggctgatgctcttaataaagaagatgaagataatatagagaagttacaagacaagatcagaggtataattgtatctaaattcgaaacattcgacctattctcatcatattctatcaagaaagacgagaagattattgatgatgataacgatgtcgaggaagaggaattggatttaggaaaaaagacaagtagctttaaatatatatttaagaagaacctattcaagttggtcctcccttcttacttaaagacaaccaaccaggacaagctcaagattatttcctcgttcgacaacttcagtacctactttcgaggattctttgagaacagaaagaatatctttacaaagaaacccatatccacgagcatcgcttatagaatcgtgcacgacaacttcccgaaattccttgataatataagatgctttaatgtttggcaaacagagtgtccacagttaattgtcaaagccgacaattatttgaagagtaagaatgttattgctaaggataaatctctcgcaaactactttactgtaggtgcgtacgattatttcttgagtcagaatggtattgacttctataataatataataggtggtttgccagcgttcgctggtcatgagaagattcaaggtttgaatgagtttatcaaccaagagtgccagaaggatagtgaactcaagtccaaattgaagaatagacatgccttcaagatggccgtcttatttaaacaaatactatcagatagagagaagtcattcgtgattgatgagtttgagtcagatgcacaagttatagatgctgtgaagaacttctatgctgagcaatgtaaggacaacaatgtgatctttaacttactaaacctgattaagaacatagccttcctttctgacgacgaattagatggtatattcatcgaaggtaagtatttgtcttccgtctcacagaaattatactctgattggtctaagctaagaaatgatattgaagattccgctaattctaaacagggcaacaaggaattagcaaaaaagatcaagaccaacaagggtgatgtcgagaaagctatctctaaatacgagttctccttgagtgaattgaatagcattgtacacgacaatactaaatttagcgatctactctcctgtactttgcacaaggttgcctccgagaagctggtgaaggttaatgaaggcgattggcccaagcacttaaagaacaatgaagagaaacagaagattaaggaaccactggatgccctcttagaaatctataatactttgttgatatttaattgtaaatcgttcaacaagaatggaaatttctacgtggactatgatcgatgcattaacgagttaagttcagttgtatacctgtataataagactcgtaactactgtacaaagaaaccttataatactgataaatttaaacttaactttaacagcccgcaacttggagaaggattctctaaatctaaggagaacgattgtttgactttgctcttcaagaaagatgacaattactatgtgggcattatccggaagggcgccaagatcaactttgacgatacacaagccattgccgacaatacagataactgtatctttaagatgaattatttcttgcttaaggatgctaagaaatttatcccaaagtgtagtattcagcttaaggaagttaaggctcattttaagaaatctgaggatgactatattctgtccgacaaagagaagtttgcctcgccactggttattaagaagtctacattcttactagcaacagctcatgtaaagggaaagaaaggaaacataaagaaattccagaaggaatattccaaggagaatccaactgagtacagaaattctttgaatgaatggattgcgttctgcaaagaattcctgaagacatataaagccgcaacgatcttcgacattactacactaaagaaagcagaggagtatgccgatattgtcgaattctataaggatgtcgacaacctctgttataaattagaattctgtccaattaagactagcttcatcgagaacctgattgataatggagatctatatctctttcgtatcaataataaggacttcagttccaagagtaccggcaccaagaatttgcacaccctgtatttacaagcgatcttcgatgagcgaaatttaaacaatccaaccataatgctaaacggaggtgctgaattgttctaccgcaaggagtcaatcgaacagaagaacaggataacgcataaggcagggtctatactggttaataaagtatgtaaggatgggacctctttggatgacaagatacgtaatgaaatctatcaatatgagaataagttcatagataccttgtcggatgaagcaaagaaggtgctcccgaatgtgattaagaaggaagctactcatgacattactaaagataagagatttacttctgacaagttcttcttccattgtccgctaactatcaactacaaagaaggcgatactaaacaatttaacaatgaagtcttaagcttcttgagagggaatccggacataaatattattggaattgatagaggtgagagaaacttaatttatgtgacagttatcaaccagaaaggtgaaattcttgattctgtatcattcaatacagtcacaaacaaatcatctaagattgaacagacagttgactatgaagagaagcttgcggttagagagaaagagcgtattgaagctaagagaagctgggattctattagcaagatcgctactttgaaagaaggttatttatcagctattgttcatgaaatctgcttgttaatgattaagcacaatgcaatagtggtactcgagaacctgaatgctggctttaagagaattcgaggtgggttatccgagaagtcagtttatcagaaattcgagaagatgttaattaataaattaaattactttgttagtaagaaggaaagcgactggaataagcctagcggtttgcttaatggattacaattatcagatcaatttgagagcttcgagaagctaggaattcaatctggatttatcttctatgtccctgctgcatatacatctaagatagatccaaccacgggcttcgcgaatgtgttgaacttgagtaaggttagaaatgtagatgctattaagtcgttcttctcaaactttaatgaaatttcctatagcaagaaggaagccttatttaaattctctttcgacttagactcgctgtccaagaagggtttcagctcatttgtaaagttctcaaagagcaaatggaatgtctacacattcggagaaaggatcatcaaacccaagaataaacaaggctatcgagaggacaagaggattaatttgacgttcgaaatgaagaagctgttaaacgaatacaaagtatcctttgacctagagaacaatttaattcctaatttgacttctgcaaaccttaaagacactttctggaaggaattattcttcatattcaagacgactttacagctccgtaacagcgtgactaatggtaaggaggatgtgttgataagtcctgtcaagaatgctaagggcgagttctttgtaagtggtacacataacaagacactaccacaggattgcgacgccaacggtgcgtaccatattgccttaaagggtttgatgattctcgagcgaaataatttggttagggaagagaaagataccaagaagatcatggcaatttccaatgttgattggtttgaatatgtacagaagagaagaggagttctctag

SEQ ID NO: 283 - DNA, 4005 bp, Artificial Sequence
  Description of Artificial Sequence: Synthetic polynucleotide
atgtcgtcactgacgaaattcactaacaagtacagcaagcaactgacgattaagaacgaactgataccggttgggaagacgttagagaatatcaaagagaatggcctgattgatggtgacgaacagttaaacgagaactatcagaaggcgaagattatcgtcgacgatttcttgcgtgacttcattaataaagccctcaacaacacccagatcggaaattggcgtgaacttgccgatgctctgaataaggaagatgaagataacatcgagaagctccaagacaagatacgtggtatcatcgtttctaaattcgaaacctttgatctctttagtagctatagcatcaagaaagatgagaagattattgatgatgataacgatgttgaagaagaggaattggatctcggtaagaagacctcgtcatttaaatatatctttaagaagaatctgtttaaattggttctgccgtcgtatcttaagacaacgaaccaagataaattaaagattataagttcgtttgataacttcagcacctatttccgtggcttctttgagaatcgtaagaacatattcaccaagaagccgattagcacttcgatcgcatatagaattgtacatgacaactttccgaagttcctggataatatacgctgcttcaacgtatggcagactgaatgtccgcagctgattgttaaagcagataactatttgaaatctaagaacgtaatagcgaaagataaatctctggcgaactacttcacagttggcgcatatgattacttcctgtctcagaacggaatcgatttctacaacaacattattggtggtcttccagcgtttgccggtcacgagaagattcaaggtttaaatgaattcatcaatcaggaatgtcagaaagactcagagctgaaatccaaattgaagaaccgccatgcgttcaagatggcagtgctgtttaagcagatcttgtcagatcgtgagaagtccttcgtgattgacgaatttgaatcggatgctcaggttatcgatgcggtaaagaatttctatgcagaacagtgtaaagataacaacgtgatcttcaatttgctgaacctgatcaagaatattgcgttcctgagcgacgacgaactggatggtatatttatcgaaggcaagtatttatcttctgtaagtcagaaactctatagcgattggagcaagctgcgtaacgatatcgaggattccgcgaactctaaacaaggcaataaagaactggctaagaaaataaagacaaataaaggtgatgtcgagaaggctatatcgaaatatgaattctccctgagcgaactgaatagcattgtgcacgataacaccaaattctcagatttgctgtcatgtacgttacataaggtggcttcggagaagctggtaaaggtgaacgaaggagactggcctaagcatctgaagaacaatgaagagaagcagaagatcaaagagccgttggacgcgctgttggagatttacaatacattactcatcttcaattgtaagtcgtttaacaagaatggcaatttctatgtagactatgatcgctgtattaacgaactctcttcagttgtctacctctataacaagacacgcaactactgcacgaagaaaccgtataacaccgacaagttcaaattaaacttcaacagtccgcagttaggcgaagggttctccaagtcaaaggagaatgactgtcttactctgctgttcaagaaagacgataattactacgtgggtataattcgtaaaggtgcaaagataaactttgatgacactcaggccattgccgacaacaccgacaactgtatcttcaagatgaattacttcctactgaaagacgctaagaaattcattccgaaatgcagtatacagttgaaagaggttaaagcacactttaagaaatctgaagatgactatatattgtctgataaagagaagtttgcatctcccttagtaattaagaaatctacatttctgttagctaccgcccatgttaaaggtaagaaaggtaacatcaagaaatttcagaaagaatattcgaaggagaatccaactgagtatcgtaacagcttaaatgaatggatcgcgttctgtaaagaattcctcaagacgtataaagcggctacaatctttgatatcaccactttaaagaaagcggaagaatatgcggatatcgttgaattctacaaagatgttgacaatctttgctacaaacttgagttctgtcccatcaagacgagctttatcgagaacttgattgataatggtgatttgtacctctttagaattaacaacaaggacttcagctccaagtcaacgggaacaaagaatcttcataccctgtacctgcaagcgatcttcgatgagaggaatttaaacaatccgacaattatgctaaacggtggcgcggaactattctatagaaaggaaagtattgaacagaagaatcgcataacccataaggctggcagcatccttgtaaacaaagtgtgcaaagacggtacttctctcgatgataagattcgtaatgaaatctaccagtacgagaataaattcatcgacaccctgagcgacgaagctaagaaagtgctccctaatgtgatcaagaaagaagcgacacacgacattaccaaggacaaacgtttcacctcggacaaatttttctttcattgtccactgactatcaactataaggagggagacactaaacaattcaacaacgaagtactctcgttcctgcgtggtaatccagacattaacataatcggaatcgatcgtggtgaacggaacctgatttatgttaccgtaattaatcagaaaggagaaatacttgattcagtctcgttcaatacggttaccaataagagctcaaagatcgagcagacggttgactacgaagagaaattagcggttcgcgagaaagaaagaatcgaagccaagcggtcatgggattctatctcgaagatagcgaccttgaaggaaggttatctgtctgcgattgttcacgaaatctgtctgctgatgatcaaacataatgccatcgtggttctggagaacctgaacgccggatttaaacgcattagaggtggcttgtcagagaagtctgtctaccagaaattcgaaaagatgctgattaataaactgaattacttcgtttctaagaaagagagtgattggaataaacctagcgggttattgaacggcttacagctgtctgatcagtttgaatcgttcgagaaactgggtatccaatctgggtttatcttttatgtaccagctgcgtacaccagcaagattgacccaacaacaggcttcgcaaacgtcctgaacctgagtaaagtgcgtaacgtggatgcaatcaaatcatttttctcgaacttcaatgaaatatcgtactccaagaaagaagcgttgttcaaattctctttcgatctcgattcgctgagcaagaagggcttctccagcttcgttaaatttagcaaatccaaatggaatgtttacacattcggcgaacgtattattaaaccaaagaacaaacaaggatatagagaagataaacgtattaatctgacatttgaaatgaagaaactgctgaacgagtataaagtcagctttgatctcgagaacaacctgattcccaatctgaccagcgccaacctcaaagataccttctggaaagaattattcttcatcttcaagacgacgctgcaactccgaaattcggtaaccaacggtaaggaagatgtacttatttcgccagttaagaatgccaagggtgaattctttgtttccggcacccataataagacactgcctcaagattgcgacgcgaacggtgcctatcacatcgcgctgaagggcctgatgatattagagcgtaacaacttagttcgtgaagagaaggacacgaagaaaatcatggcgatttccaacgtagattggtttgagtatgtgcaaaagagaagaggtgtgctttga

SEQ ID NO: 284 - DNA, 4005 bp, Artificial Sequence
  Description of Artificial Sequence: Synthetic polynucleotide
atgtcctccttaactaaattcaccaacaaatacagtaagcagctgacgattaagaacgaactgatcccggtgggcaagacgctagagaatattaaagagaatgggttgattgatggcgatgaacaattaaatgagaactaccagaaagccaagatcattgttgatgatttcctccgtgactttattaataaagcgttgaataatacgcaaatcggcaattggcgagaactggccgatgcgttaaataaagaggatgaggataacatcgagaaattgcaagataagattcgtggaattattgtgtctaaatttgaaacctttgacctattctcaagctactcgattaagaaagatgagaagattattgacgatgataatgacgtggaagaagaagaactggaccttggaaagaaaacttcaagcttcaagtatatctttaagaagaatttgttcaaactggtgctaccatcctacttaaagactacgaaccaagataaactgaagatcatttctagctttgataatttcagcacctactttagaggattcttcgagaaccgtaagaatatcttcactaagaaaccgattagcacctcaatcgcttatcgcattgtgcatgacaactttccaaaatttctggataacatccgttgcttcaatgtgtggcagacggagtgccctcagttaattgtgaaagccgataactatctgaaatcgaagaatgtgattgccaaagacaagagcctggccaattacttcaccgttggagcctacgattatttcctgtcacagaatggaattgacttctataacaatattattggtggtcttcctgcattcgcaggtcatgagaagattcagggcttaaacgagtttattaaccaggaatgccagaaggatagtgaacttaagtctaaattaaagaatcgtcacgcctttaagatggccgtactgttcaagcagattctgagtgaccgtgagaagtcatttgtgatcgatgaattcgagtctgatgcgcaggtaattgacgcggtcaagaatttctatgcggagcagtgcaaagataacaatgtcatatttaacctgctcaatctgatcaagaatattgcatttctgtctgatgatgaactggatggcatcttcattgaaggcaaatatctcagctctgtctcccagaaattgtacagtgattggagcaaattgcgcaacgatattgaagattcagcgaatagcaaacagggcaataaagaactggctaagaaaatcaagacaaataagggagacgttgagaaggcgataagtaaatatgaattcagtttatcagaacttaacagtattgttcacgataacaccaaattctcggatctgctgtcgtgtactcttcacaaagtggcatcagagaaattggtaaaggtgaacgaaggagattggccgaaacatttaaagaacaatgaggagaagcagaaaatcaaggaaccgctggatgcactgttagaaatttacaatactctgctgatatttaactgcaagagctttaacaagaatggaaacttctatgttgattatgatcgctgcattaatgaactgtctagcgttgtttatttatacaacaagacgcgtaactattgtactaagaagccttacaataccgacaaattcaaacttaatttcaatagcccgcaactgggtgaagggttctcgaaatcaaaggagaatgattgcttgaccttgctatttaagaaagacgacaattattacgttggcattattcgtaagggcgcgaagatcaatttcgacgacactcaggcgatcgcagataatactgataactgcatatttaagatgaattatttcctgctgaaagatgctaagaaattcattcccaagtgtagcattcagttgaaagaggttaaagcccattttaagaaatctgaagacgactatattctttccgataaagagaagtttgcgagtccgctggtgattaagaaatctacgttcctgctggcaacagctcatgtcaaaggtaagaagggtaatataaagaaatttcagaaagaatacagtaaagagaaccctaccgaataccggaattccctgaatgaatggatagcgttctgtaaggagtttttgaagacatacaaagcggcgaccatatttgatatcacgactttaaagaaggcggaagagtatgccgacattgttgaattctacaaggacgtggataatctttgttataaacttgaattctgtccgattaagacgagctttatcgagaatctgattgataatggcgatctgtatttatttcgcattaataataaagactttagttctaaatctacgggtacgaagaacctgcataccctgtatttgcaggccatattcgacgagcgtaatctgaacaacccgactatcatgctgaatggcggcgcagagttattctatcgcaaagaaagtatcgaacagaagaatcggataacccacaaagctggtagcattcttgttaataaagtttgcaaagacgggacaagccttgatgataagatccgtaacgaaatctaccagtatgagaataagttcattgataccttaagtgatgaagcaaagaaggtcctccctaatgtgattaagaaggaggcgacgcacgatataacgaaagacaaacggttcactagtgacaaattcttcttccattgcccgttgactatcaattataaggaaggtgatacgaaacagttcaataatgaggttctgtcctttctgagaggaaatcccgatattaatattataggtattgatcgcggcgaacgcaaccttatctacgttacggtgatcaaccagaaaggtgagattcttgattcagtctcattcaatactgttacaaacaagagctctaagatcgaacaaacggtggattacgaagagaaactggccgttcgagagaaggaacgtatcgaggcaaagagaagctgggattcaatcagcaagatcgcgacgctgaaagaaggttacttgtcagcgatcgtacatgagatttgtctgctgatgattaagcataacgccattgtcgtgttagagaatctgaacgccgggtttaaacgcatccgcggtggcctctctgagaaatcagtatatcagaaatttgagaagatgctgattaacaagctgaattatttcgtgtcgaagaaagaatcggactggaacaaaccgagcggcctgctgaacggccttcagctgagtgaccaatttgaatctttcgagaagctgggcatccagtcaggtttcatcttctacgtccctgcagcatacacaagcaagattgatcctacaaccggctttgctaacgtgttaaatctgagtaaagtgcgtaatgtggatgcgatcaagagcttcttctccaacttcaatgagatttcgtactcaaagaaagaagctctgtttaaattcagcttcgacctcgattcattaagtaagaaaggattctcttcatttgtgaagttctcaaagtcgaaatggaacgtctatacgtttggcgaacgcatcattaaaccgaagaacaaacagggctatcgcgaagataaacgtatcaacctcacgtttgaaatgaagaaattgctgaatgaatataaggtttctttcgacctcgagaataatcttattcctaatctgaccagtgctaatctgaaagacacattctggaaagaacttttcttcatatttaagacaacactgcagctgcgcaactcggttacgaatgggaaagaagatgttctgatcagcccggttaagaatgctaagggtgagttcttcgtgtctggcacacataataagaccttgccacaggactgcgacgcaaatggcgcctaccatatagcgctgaaaggactgatgatcttggaacgcaataatttagttcgtgaagagaaggataccaagaagatcatggccatctcgaatgtagattggttcgaatatgttcagaaacgtcgtggtgtgctgtaa

SEQ ID NO: 285 - DNA, 4005 bp, Artificial Sequence
  Description of Artificial Sequence: Synthetic polynucleotide
atgtctagcctgacgaaatttacaaataagtattcgaaacagcttactataaagaacgaactgatcccggttggtaagactctggagaacatcaaggagaatggtttgatagatggagacgaacaactgaacgagaactaccagaaagctaagatcattgttgatgactttctgcgcgacttcattaataaagctcttaacaacacccaaattggtaattggcgggaactggcggacgctctgaacaaagaagatgaagacaatatagagaaactccaggacaagatccgcggtattattgtgagtaagtttgaaaccttcgacctcttctcctcgtatagcataaagaaggacgagaaaatcatcgatgatgataatgatgtagaggaagaagagttggacctgggcaaaaagacatcatcgttcaaatacatctttaagaagaatctatttaaattagtccttccgtcttacctcaagacgaccaaccaggacaagttgaagattatttcatcattcgataatttctcaacctatttccgtggcttctttgagaatcgaaagaacatatttaccaagaaaccaatctcgactagcattgcatatcgcatcgtccatgataacttccctaaattcctggacaatattcgttgctttaacgtgtggcaaaccgagtgtcctcagctaattgtcaaagcggataattatctgaaatcaaagaatgtaattgcgaaagacaaatccctggcgaactacttcacggtcggtgcatatgattatttcttgtcccagaatgggattgacttctacaacaacatcataggcggtctcccagcgtttgccggtcatgagaaaattcagggtcttaacgagttcattaatcaggaatgccagaaggactcggaactaaagagtaaactcaagaaccgtcacgcatttaagatggcggttctgtttaaacagattctgagtgatcgcgagaagagctttgtcatagatgaatttgagtctgacgcgcaggtgattgatgcggtgaagaatttctatgctgaacagtgcaaagataataatgtcatcttcaatctccttaacctcataaagaacattgcgtttctttcggacgacgagctggatggaatctttattgagggcaaatatctcagctctgtcagccagaaactttatagcgattggagcaagctccgcaatgatattgaggatagcgcaaacagcaagcagggtaacaaggaattagcaaagaaaattaagacaaataaaggtgacgtcgagaaggccattagtaagtatgaattctccctcagcgaattaaactctatagtccacgataataccaagttcagtgatctattgagttgtacactgcataaagttgcaagtgagaaactagtgaaagtgaacgagggtgattggccgaaacatcttaagaataatgaagagaagcaaaagattaaagaacctctcgatgctttactggagatctataatacactgcttatctttaattgtaaatcattcaacaagaatggcaacttctatgtggactacgatcgctgtataaatgaattgtcgagcgtggtctacttatacaacaagacacgcaactattgtacaaagaagccctataatactgataaattcaagctgaacttcaattcgccgcagctgggcgaaggcttcagtaagagcaaagagaacgactgcctgacccttctatttaagaaagacgacaactactacgtcggaataatccgcaaaggtgccaagattaatttcgacgacacgcaggcgattgccgacaatacagataactgcatattcaagatgaattacttcttgctgaaggatgccaagaaattcattccgaaatgttcaatccagcttaaagaagtcaaagctcactttaagaaatcagaagacgactatatcctgtccgacaaagagaagtttgcttcgccgctggtaataaagaaaagtacgtttctgcttgcgaccgcgcacgttaaagggaagaaaggaaatattaagaagttccagaaagaatattcgaaagagaatccgacagaatatcgtaatagcctgaatgagtggatcgctttctgcaaagagttcctgaagacctataaagcggccaccatcttcgacatcacgacactcaagaaagcggaggaatatgcagatatcgtggagttctacaaagacgttgacaacctttgctataaacttgaattctgcccgatcaagactagtttcattgagaaccttattgataatggtgatctgtatttgtttcgcatcaataataaagatttctcctccaagtctactggcacaaagaacttacataccttgtatctccaggcgatcttcgatgaacgtaatttaaataacccgacgatcatgttaaatggtggcgcagaactcttctaccgtaaggagagtattgaacaaaagaaccgtataacccataaagctgggtccatcctggtgaataaagtgtgcaaagatgggacgtcgttagacgataagattaggaatgagatttaccaatatgagaataagtttatcgacaccctctctgatgaagcgaagaaggtgctaccgaatgtgatcaagaaagaagccacacacgacatcacgaaagacaaacggtttacctcagataaattcttctttcattgtccgctgaccatcaattataaagagggagatactaaacagtttaacaatgaggtattaagcttcttaagaggcaatccagatattaacattattgggattgatcgtggtgaaagaaatctgatttatgtaaccgttataaatcagaaaggagaaatcctggactccgtaagctttaacaccgtaactaataagagtagcaagatagaacaaacggttgattacgaagagaaattagctgtgcgggagaaagagcgtattgaagcgaagcgcagttgggatagcataagtaagatcgcgaccctcaaggaaggctacttaagcgcaatagtacatgaaatctgcttactcatgatcaaacacaatgcgattgttgtcctggagaatctcaacgccggcttcaaacgcatacggggtggtctgagtgagaagtcagtttatcagaagtttgagaagatgcttattaacaaattgaattactttgtgtctaagaaagagagcgactggaacaaaccctctggtttactgaacggcttacagctcagcgatcagtttgaatcatttgagaagttgggtattcagagcggattcatattttatgtaccagcagcctatacaagcaagatcgatccaaccacaggcttcgctaatgttctgaacctgagcaaagtgcgcaacgtagatgctatcaaatcattcttctccaatttcaatgaaatcagttacagtaagaaggaagccttgttcaagttctcgtttgatctggattcgctctcaaagaaaggattcagcagctttgtaaagttcagcaagagcaaatggaatgtctatacgtttggtgaacgaatcatcaagccaaagaataagcagggttaccgcgaagataaacgcattaatctcacctttgaaatgaagaagttgcttaacgaatataaagtttctttcgacttggagaacaacttgatacctaatctgacgagcgctaatttgaaggatacattctggaaagagctcttctttatcttcaagactaccctgcaactgcgcaatagcgttaccaacggcaaagaggacgtgctcatttcaccggtaaagaatgctaagggtgagttctttgtgagcgggactcataacaagacacttccgcaggactgcgacgcgaacggcgcctatcatattgcgcttaagggcctcatgatcctggaaaggaacaatctcgtgcgcgaagagaaagatacgaagaaaataatggccattagcaatgtagactggtttgaatatgtgcagaagcgtcgcggtgtcctctag

SEQ ID NO: 286 - DNA, 4005 bp, Artificial Sequence
  Description of Artificial Sequence: Synthetic polynucleotide
atgagctcactaaccaagttcaccaacaagtactccaaacagctgaccattaagaatgaactgattcctgttggcaagaccttggagaatattaaggagaacggcttgattgatggcgatgaacaactgaatgagaattatcagaaagctaagatcatcgttgatgatttcttacgtgacttcatcaacaaagctcttaataacacccaaatcggcaattggagggagctggcggatgctctcaataaagaggatgaggacaatatcgagaagctgcaagacaagatccgtgggatcatcgtttccaaatttgaaacattcgacctcttctcaagctactcaattaagaaagatgagaagatcattgatgacgataatgatgtagaggaggaagagctggacctgggcaagaaaacctcatcgtttaagtatatcttcaagaagaatttgtttaaactggtattgccaagttatttaaagaccactaatcaggataaattaaagatcatctctagctttgacaacttcagcacgtatttcagagggttcttcgagaatcgcaagaatatctttactaagaaaccgatttccaccagtatcgcatatagaattgtccatgacaacttcccgaagttcttagataacatcagatgtttcaacgtgtggcagaccgagtgcccgcagctgatcgtgaaggcagataactatctgaagtccaagaatgtgatcgcaaaggataagagtttggccaattacttcacggtcggtgcttatgattactttctttcgcagaacggcatagatttctataacaacatcattggtggactgccggcgttcgcgggccatgagaaaattcagggacttaacgagttcattaatcaggaatgtcagaaagactctgagttgaaatcgaaactgaagaatagacacgctttcaagatggcagttttgtttaaacagatactctcagatcgtgagaaatcattcgtgatcgatgaatttgaatctgatgcccaggtgattgacgcagtgaagaatttctatgccgagcagtgtaaagataacaacgtgatattcaatttgttaaatctgatcaagaatattgcattccttagcgacgacgaactggacggtatctttattgaaggaaagtatttatctagcgtgagccagaagctgtattccgattggtcgaaactgcgtaatgacatagaggattccgccaacagcaaacaagggaataaagaacttgcaaagaaaatcaagaccaataaaggtgatgttgagaaggcaattagcaagtacgaattcagcttatctgaattgaactctattgttcatgacaacaccaaatttagtgacttgctgtcatgtacattgcataaggtagcgtctgagaagctggttaaagttaacgagggcgactggccgaaacaccttaagaacaatgaagagaagcaaaagatcaaagaaccgttagatgcgctcctcgaaatttacaatactcttctcatatttaactgtaagagcttcaacaagaatggtaatttctatgttgactatgatcgctgtattaatgaacttagtagcgtggtttacttatataataagactcggaactactgcactaagaaaccgtataacaccgataagttcaaactgaactttaacagtccgcagctgggtgagggcttcagcaagtcgaaggagaacgactgtctgacgctgttatttaagaaagatgataattactacgttggcattatccgcaaaggtgctaagattaacttcgacgatacgcaggccatagcggataacaccgacaattgcatcttcaagatgaactacttcctcctcaaagatgctaagaaattcattccgaaatgctcgattcaattgaaggaagttaaggcccacttcaagaaatccgaagatgattatattctgtcagacaaagagaagttcgcaagtccactcgtaattaagaaatcgacctttctgcttgcaaccgctcatgtgaaagggaagaaaggcaacataaagaaatttcagaaggagtattcaaaggagaatccgacagagtaccgcaacagcttaaacgagtggattgcgttctgtaaggaattcctgaagacctataaagccgcgactatatttgacattacgaccctgaagaaggcggaagaatatgctgatattgttgaattctacaaggatgtagataacctgtgctacaaattagagttctgcccgattaagaccagctttatcgagaacctcatcgacaacggcgatctgtacctgtttcgcatcaacaataaagacttcagctcgaagagcaccggcacgaagaacctgcacacactgtaccttcaggcgatatttgatgaacgcaatttgaacaatccaacgatcatgctaaacggaggtgcggaactcttctatcgtaaagagagtatcgaacagaagaaccgtattacccataaagctggaagcatattagtgaacaaggtttgcaaagatgggacctctcttgatgacaagatccgcaatgaaatataccaatatgagaacaagtttatcgatacgctgagtgacgaggccaagaaggtgctgccgaacgtaatcaagaaagaagcaacccacgatattacgaaagataagagatttacatcggataaatttttcttccactgcccgctgaccatcaactataaggaaggagatactaaacagtttaataacgaggttctgtcgtttctgcgtggcaatccggatattaacatcatcggtatcgaccgcggagaacgtaacctgatttatgtaaccgttattaaccagaagggtgaaatacttgacagcgtctctttcaacacggtgaccaataagtcttccaagatcgaacagactgttgattatgaagagaagctggcagtgcgcgagaaagaacgtatcgaagctaagcgttcctgggactctatcagcaagattgccacccttaaagaaggttacctgagcgccatcgttcatgaaatttgcttgctgatgattaagcataacgccattgtggtcttggagaaccttaacgctggatttaaacgtattcgcggcggtttatctgaaaagagcgtttatcagaagttcgagaaaatgctgattaataaattaaactatttcgtcagcaagaaagaaagcgattggaataaaccatctggtctcctaaacgggttgcagttaagtgatcagtttgaatcattcgagaaactgggcattcagtcaggtttcatattttacgtcccggcggcttatacctcaaagattgatcccaccacgggtttcgctaatgtacttaacctaagtaaagtgcgtaacgtggatgcaattaaatcgttcttctcgaacttcaatgaaatctcgtacagcaagaaagaagcgctctttaagttctcatttgacttagattcgctgtcgaagaagggatttagttcatttgttaagtttagtaaatccaaatggaatgtgtacacgttcggtgaacggattattaaacccaagaataaacagggatatcgtgaagataaacgcattaatctgacatttgaaatgaagaaattattaaacgaatacaaggtaagcttcgatctggagaacaacctaattcctaacttaaccagcgcaaacttgaaggatacgttctggaaagaactattcttcatcttcaagaccactctgcagcttcgcaactctgtgacgaacggtaaagaagacgtacttatttcaccggtaaagaacgccaaaggtgaattctttgtttcgggcacccacaataagaccctgccacaggactgcgatgcaaacggcgcatatcatattgccttgaaaggattaatgatcttagaacgcaataatctcgttcgcgaggagaaagatacaaagaagatcatggccattagcaacgttgattggtttgaatacgtacagaagcgccgtggcgttctctaa

SEQ ID NO: 287 - DNA, 4005 bp, Artificial Sequence
  Description of Artificial Sequence: Synthetic polynucleotide
atgagctctcttacgaagttcacgaacaaatacagcaaacagctgactattaagaatgaattgattccagtaggcaagacgctggagaacattaaagagaacggcctgatcgacggcgatgaacagctgaacgagaattaccagaaggccaagattattgttgatgacttcttaagagatttcataaataaggcgttgaacaatactcagattggtaattggcgcgaactggcagatgccttgaataaagaagatgaagataacattgagaagttacaggataagatccgtggtattattgtttctaagtttgaaactttcgacctgttctcaagctatagcatcaagaaagacgagaagatcatcgatgatgataatgatgtggaagaagaggaactcgatctgggaaagaaaacatcgtcattcaaatatatcttcaagaagaatctgttcaaattagtgctgcctagctatctcaagacgacaaaccaggataagctaaagataatttcttcattcgataatttctctacttacttccgcggtttctttgagaaccgaaagaatatctttacgaagaagccgatctcaacctcgattgcctaccgtattgtccatgataacttcccgaaattcctggataacattagatgcttcaacgtgtggcaaacggaatgcccgcagcttatcgttaaagcagataactatctgaaatcaaagaatgttatcgcgaaagacaagagcctggcgaactacttcacggtgggcgcgtacgactactttctgagccagaatggtattgatttctacaacaacatcattggcggcttaccggcattcgcgggccacgagaagatccaagggctgaatgaatttatcaaccaagagtgtcagaaagatagtgagcttaagagcaaactgaagaatcgccatgccttcaagatggccgtcctctttaaacaaattctgagcgatcgtgagaaatcctttgtgatcgacgagtttgagtcagatgcacaggtgattgacgccgtgaagaatttctatgcggaacagtgcaaagataataatgtgatatttaatctgctgaaccttataaagaacatcgcgtttctatcagatgacgaattagatggtatatttattgagggcaaatatctgtcaagcgtgagccagaaactgtatagcgattggtccaaactgcgtaacgatattgaagactccgccaattcgaaacagggtaacaaagagttggctaagaaaatcaagactaacaaaggcgatgtagagaaggcgattagcaaatatgagtttagtctgtccgaattaaatagtattgttcatgataacacgaaatttagtgacttgctgtcgtgtaccctgcataaggtcgcaagtgagaaactcgttaaggtgaacgaaggtgattggccgaaacatcttaagaataatgaagagaagcaaaagattaaggaacctttggacgcgctgctggaaatttataacacgctgctgatctttaattgcaagagtttcaacaagaacggaaacttctatgtcgactatgacagatgtattaacgaactgagctcagtcgtttacctgtacaataagacgcgcaattattgcaccaagaaaccgtacaacaccgataaattcaaactgaacttcaactcaccgcagctcggtgaaggattcagcaagtccaaggagaatgattgtttaacactgctctttaagaaagacgataattattatgtcggtattattcggaagggtgctaagatcaactttgacgatacccaggcgattgcagacaataccgataattgtatctttaagatgaactactttctgctgaaggacgcgaagaagtttatccctaaatgttcaatccaacttaaagaagtcaaagcacactttaagaaatccgaagacgattacatccttagcgataaagagaagttcgcaagcccgctggtgattaagaaatctactttcctgctggcgactgcccacgttaaaggaaagaaaggcaatatcaagaaatttcagaaggaatatagcaaagagaacccgacagaataccgtaattcgctgaacgaatggatcgcattctgtaaggaattcttaaagacctataaagcggccacaatctttgacattaccaccctaaagaaagcagaggagtatgcggacattgtcgaattctacaaagatgtggacaatttatgttacaaacttgagttctgtcccattaagacgtcctttatcgagaatctgattgataatggcgacttatatctctttcgtattaacaataaggacttcagttcgaaatcgacgggaacaaagaatttgcataccttgtatctacaggcgatctttgatgaacgcaacctgaataacccgacgatcatgcttaatggaggtgcagaactcttctatcgtaaagaatcgatcgaacaaaagaaccgcatcactcataaagctggctctattctggtcaataaggtgtgcaaagacggtacgtcattggatgataagattcgcaatgagatttaccagtacgagaataaatttatcgatacgctgagtgatgaagcaaagaaagtcttgcctaacgtgattaagaaggaggcaacgcatgatattacgaaggataagcggtttacatccgacaagttcttctttcattgtccgctcaccataaactacaaagaaggcgacactaaacaattcaataatgaggttctttcatttctgcgcggtaacccggatatcaacatcattggcattgatcgtggtgaacgcaacctgatttatgttaccgttatcaatcagaaaggcgaaatactggacagtgtatcgttcaatacggtaaccaataagagttctaagatcgaacagacggtcgactacgaagagaaactggcagtacgtgagaaagagcggattgaggccaagcgttcctgggatagcatttctaagattgctactctcaaagaaggttacctgtcagcgatcgtgcacgagatttgtttacttatgattaaacacaatgcgatagtggtgcttgagaatttaaatgccggcttcaaacgtattcgtggtggcttatcagagaagagcgtgtatcagaagttcgagaaaatgcttattaacaaactgaattacttcgtttccaagaaagaatctgattggaacaaaccatctggcctgttaaacggcctgcaactctctgaccagtttgaatcatttgagaagctgggcatccagagtggattcatcttctatgtaccggcagcgtacacatcaaagattgatcctacaaccggcttcgcaaacgtgctgaatcttagtaaagtgcgcaatgtggatgcaattaaatccttcttctcgaactttaacgaaatcagctacagcaagaaagaagccttattcaaattttcgttcgatttggatagcctctctaagaaagggttctcaagcttcgtgaaattcagcaagagcaaatggaatgtgtatacctttggtgaacgcattattaagcctaagaacaaacaagggtaccgtgaagacaagagaattaacctaacgtttgaaatgaagaaactccttaacgagtacaaagtgtcgtttgatctggagaataatctcatcccaaacctgaccagtgcaaacctgaaggacactttctggaaagaactgttcttcatattcaagaccaccttgcagctgcgaaattcagtcaccaacggtaaagaagatgtgctgatctcgccggtaaagaatgcaaagggtgaattcttcgtaagtgggactcataataagacgctgccgcaggactgtgacgcaaatggcgcctatcacatagcgctgaaaggcttaatgatcctggaacgcaacaaccttgtacgtgaagagaaggatacgaagaagattatggcgatctccaatgttgactggtttgaatacgtgcagaagcgccgtggagttctgtaa

SEQ ID NO: 288 - DNA, 4005 bp, Artificial Sequence
  Description of Artificial Sequence: Synthetic polynucleotide
atgagttctcttacaaagtttacaaacaaatattctaaacagctgacgataaagaacgagctgattccagtggggaagacccttgagaatatcaaggagaacggtttgattgacggtgatgagcagctgaacgagaactatcagaaagcaaagattatcgtcgatgactttcttcgcgatttcattaacaaagctttaaacaacacgcagattggcaactggagggaactggccgatgctctgaataaagaagatgaggacaacatcgagaaattacaggataagatcagaggtatcatcgtcagcaaattcgaaacgtttgacctgttcagcagttatagcattaagaaagatgagaagatcatagacgacgataatgacgttgaagaggaggaacttgatctgggtaagaaaacatcgtcattcaaatatatattcaagaagaacctcttcaaattagtgctacctagttacctaaagacgaccaatcaagacaaactgaagatcatttcgtctttcgataactttagcacgtactttcgcggcttctttgagaaccgcaagaacatcttcaccaagaaacccatttctactagtattgcgtatcgtattgtgcatgataatttccctaagttcttagataacattcgttgctttaacgtatggcagacagagtgtcctcaactgatcgtcaaagctgataactaccttaaatcgaagaacgtcatagccaaagacaagagcctagccaactacttcaccgtaggtgcatacgactacttcctgagtcagaacgggatcgacttctataataatatcattggaggactgccagcattcgcagggcatgagaagatccagggcctgaatgagtttattaaccaggaatgtcagaaggactctgagctgaagagcaaactcaagaatcgtcacgcgtttaagatggcggttctctttaaacagattctgtcggaccgtgagaaatctttcgtgattgatgagtttgaatctgacgcccaggtcatcgatgcggtaaagaatttctatgcggagcaatgtaaagataacaacgtaatcttcaacctgctcaatctgataaagaacatagcgtttctgtcagatgatgaactggatggtatctttattgaaggtaaatacctgagttctgttagccagaaactgtactcggattggtctaaacttcgcaacgatatcgaagatagtgctaactcgaaacagggtaacaaggaactggcgaagaagattaagacgaataagggtgacgttgagaaggcgatcagcaaatatgagttctcgctatccgaattgaattccattgttcatgataacaccaaatttagcgatctcctgtcatgcacactacataaagttgcgagtgagaagctggtcaaagtgaatgaaggtgactggccgaaacatcttaagaacaacgaagagaaacagaagattaaggaaccgctggatgcgctgctggaaatctataatacgctgctaatatttaactgtaagagctttaacaagaatggaaacttctacgtggattatgatcgttgcatcaatgaattgagctctgtggtgtacctctacaataagacgcggaactactgcactaagaaaccgtataataccgataagtttaaactgaactttaactctcctcaactgggagaagggttctctaaatcaaaggagaatgactgtcttacactgctgtttaagaaagatgataactactatgttggcattatcagaaagggtgccaagatcaactttgatgacacgcaggcgatcgcggacaatacggataactgcatattcaagatgaattacttcttgctcaaagatgcgaagaaattcatcccaaagtgtagcatccagctcaaagaagtcaaagcccacttcaagaaaagcgaagacgattacattctgtcagataaagagaaatttgctagcccattggttatcaaaaagagtacgttcttgctggccaccgcgcacgtaaaggggaagaaaggaaacatcaagaaatttcagaaagaatattctaaagagaatccgactgagtaccgtaacagcttgaatgaatggatcgctttctgcaaggagttcctaaagacgtataaggcagctactatctttgacataactacgctcaagaaagccgaggagtatgctgacattgtcgaattctataaagacgtagataacctgtgctataaactagaattctgcccgataaagaccagtttcatcgagaatctgattgataatggtgatttatacttattccggatcaacaataaggacttcagcagtaagagcacgggcacaaagaacctacatactttgtatttgcaggcaatcttcgacgaacgtaatcttaacaacccgaccattatgctgaatggaggcgcggagctgttctatcgcaaggaatcaatcgaacagaagaaccgcatcacccacaaagcgggatcgatcctggtgaacaaggtatgtaaggacggcacatccctcgacgataagatacggaatgagatttaccagtacgagaacaaatttattgatacccttagcgatgaagcaaagaaggttctgccgaatgttatcaagaaagaagcgacccacgatattacgaaagataagcgattcacttcagataagttcttcttccattgcccgttaactatcaattacaaggaaggagatacgaaacagtttaataatgaagtactcagctttctccgcggtaacccagatattaatattataggtatagatcgaggcgaacgtaacctgatttatgtaacggtcattaaccagaaaggagaaattctcgactctgtgtcattcaacacagtaaccaataagtcatcaaagattgaacagacagttgattatgaagagaagctggctgttcgcgagaaggaacgtattgaagcgaagcgctcatgggatagcattagtaagattgcgaccctcaaggaaggttacctgtcggcgattgttcacgaaatttgtctgctaatgattaaacataacgcgattgtagtcctggagaatctaaacgccggattcaaacgcatcagaggaggactgtcggagaagtctgtatatcagaaattcgagaagatgctgatcaacaaactgaattacttcgtttctaagaaagaatcagactggaacaaaccgtcgggactcttaaacggtctgcagctgtccgatcaattcgaaagcttcgagaaattgggcattcagagcgggtttatattctatgtgccagctgcatatacatcaaagattgaccctacgacaggattcgccaacgttctgaatttgtctaaggttcgcaatgttgatgcgatcaagtcatttttctccaacttcaatgaaatcagctattctaagaaagaagccctatttaaatttagtttcgacctggacagcctgtcgaagaaaggctttagcagcttcgtgaagttctcgaaatcgaagtggaacgtctacaccttcggagaacgcattatcaaacctaagaataagcagggatatcgtgaagacaagcgaattaacctgactttcgaaatgaagaagctgctgaacgaatataaagtatcgttcgaccttgagaacaacctgatcccaaatcttacatcggctaacttaaaggataccttctggaaagaactcttctttatcttcaagaccaccttgcagctgcgtaatagtgtaacaaatggcaaagaagacgtcctcatcagtccggttaagaacgctaaaggagaattctttgtctcgggcacccacaataagaccttaccgcaggactgcgacgccaacggtgcttatcacatcgcacttaaaggattgatgatcctcgaacgcaataacctggtccgggaggagaaagatacaaagaaaattatggcaatcagcaacgtagactggttcgaatatgtgcagaagcgacgtggcgtattgtaa

SEQ ID NO: 289 - DNA, 4005 bp, Artificial Sequence
  Description of Artificial Sequence: Synthetic polynucleotide
atgtccagcctgaccaaatttactaacaaatacagtaagcaactcacaataaagaatgagctgataccagtcggtaagaccttagagaatattaaggagaatggcctcatcgatggcgatgaacagctgaatgagaactatcagaaagccaagattatcgtggatgactttctgcgcgacttcataaacaaggcactgaacaacacgcaaattgggaattggcgtgaactggctgatgcgctgaataaagaggacgaagacaatatcgagaaacttcaggataagatacgtggcatcatcgtttctaaatttgagaccttcgatctattctcatcgtatagcattaagaaagatgagaagatcattgacgatgataacgacgtagaagaagaagaactggatttgggaaaaaagacgagctcctttaagtatatcttcaagaagaacctgtttaaactggtcttaccgtcatacttaaagacaacgaatcaggataaactgaagattatttcctccttcgataatttctctacctactttcgtgggttctttgagaaccgaaagaatatcttcactaagaaaccaattagcacctcgatcgcgtatcgtatagtgcatgacaacttcccgaagttcttggataacatccgctgctttaatgtttggcaaactgagtgcccacagctaatagttaaagctgataactatctgaaaagcaagaacgtgatagccaaagataaatctctggcaaactacttcaccgtaggtgcatatgactacttcctctcccagaacggtatcgacttctataataacattatcggaggactgccagcgttcgccggacacgaaaagattcagggtttaaatgaatttattaaccaagaatgtcagaaggatagtgaacttaaatccaagttaaagaacagacacgccttcaagatggcggttctattcaaacagatcctgagtgatagagagaaatcatttgttattgacgaattcgaatctgatgcccaggtgattgatgcggtaaagaatttctacgctgagcaatgtaaagacaacaatgtgatcttcaacttactgaatctgataaagaacatcgcgtttctgtctgacgacgaactggatggaatctttattgagggcaagtatttgtcatcagtgagccagaaactgtatagcgattggtccaaactgcgcaacgatatagaagattcggcaaacagtaaacagggaaataaggagctcgccaaaaagatcaagactaacaaaggcgatgttgagaaggccattagtaagtatgaattctcgttgtcagaactgaacagtatcgttcatgataataccaaattctcagacctgctgtcatgcacgcttcacaaagtcgcgtcagagaaactggtcaaagttaatgaaggcgattggccgaagcacctaaagaataacgaagagaagcaaaagattaaggaaccgctggatgcactcttagaaatctataacacgttgctgatctttaactgtaagagtttcaataagaacggtaatttctatgtggactacgatcgttgtatcaatgaactgagctcggtggtctacctttataataagacgcgtaactactgtactaagaaaccgtataacaccgacaaatttaagctgaacttcaatagtccgcagcttggcgaaggcttcagtaaatcgaaagagaacgactgcctgaccctgctgtttaagaaggacgataattactacgtaggaattattcgtaagggcgctaagattaacttcgacgacacgcaggccatcgccgacaacacggataactgtatcttcaagatgaactacttcctcttgaaagacgctaagaaattcatcccgaagtgcagcattcagctgaaggaggttaaggcacattttaagaaatcagaagatgattatatactcagtgataaagagaaatttgctagcccgctagtcattaagaaatcaacgttcctgctggcgactgcgcatgttaaaggtaagaaaggaaatatcaagaaatttcagaaagagtatagtaaggagaatccgacggagtatcgcaattctttgaacgaatggattgcattctgtaaggagttcctgaagacgtacaaagccgcaaccatctttgacattacgacccttaagaaggctgaagaatatgcggatatcgttgaattctataaagatgttgataacctgtgctataaactggagttctgtccgattaagacctcatttatcgagaatctgattgacaatggcgacctgtatctattccgtatcaataacaaagacttctcctctaaatctaccggcacaaagaatctgcacaccctttacctgcaggcgatcttcgatgagcgaaatctgaacaatccgacaatcatgctgaatggtggcgccgaactattctaccgcaaagaaagcattgaacaaaagaaccgaataacacacaaagccggcagcattctggtgaataaagtctgtaaagatggtacaagcttggacgacaagattcgcaacgaaatttaccaatacgagaacaaatttattgatacgctgtcggatgaggccaagaaagtgctgcccaacgtgataaagaaggaagccacgcatgatattaccaaagataaacgtttcacctcagataagttcttctttcattgtccgctaacgattaactacaaggagggtgataccaaacagtttaacaatgaggtcctgtcgttcctgcgcggtaatccggacataaacatcatcggtatcgaccgaggcgagcgtaacctgatttacgtgaccgtgattaaccagaaaggcgagatattagatagcgtgagctttaataccgttaccaacaaatcgtcgaagattgagcagactgtggactatgaagagaaactggccgtccgggagaaggagcgtattgaagccaagagatcttgggattctatcagcaagattgctactctcaaggaagggtacctatcggcaatcgttcatgaaatctgtttgcttatgatcaaacataatgcgatagtagtgctggagaacttgaatgcgggattcaaacgtattcgaggcggcttatctgagaaaagcgtataccagaagttcgaaaagatgctgattaacaaacttaactactttgtgtctaagaaagagtccgattggaataagccctcgggtctgcttaatgggctgcaattgtctgatcagttcgagtcgtttgagaagttgggtattcagtctgggttcattttctatgttccggccgcgtatacgtcaaagatcgacccgacgactggtttcgcgaatgtccttaatctgagtaaggttcgcaatgttgatgcgatcaagagtttcttcagcaacttcaatgaaatctcatactcaaagaaggaagcgctattcaaattctcattcgatttagattcgttgtcaaagaagggcttcagttcattcgttaagttcagcaagagcaaatggaacgtttacacattcggcgaacgcattatcaaacccaagaacaagcagggctaccgcgaagataagcgaattaacctgacattcgaaatgaagaaactgttaaatgagtataaagtgagctttgatcttgagaataatctgattccaaatctgacatccgctaacctgaaagacacattctggaaggaattgttctttatcttcaagacaacattacagctgcgcaacagtgtgacgaatggcaaggaagatgtgctgattagcccggtaaagaacgcgaagggtgaattctttgtttctggtacccataacaagactcttcctcaagactgtgacgcaaatggtgcctatcatatcgccctgaaaggtctgatgatcctggagcgcaataatcttgttcgtgaggagaaggacactaagaagattatggctatttctaacgttgattggtttgagtatgttcagaaacggcgcggtgttctataa

SEQ ID NO: 290 - DNA, 4005 bp, Artificial Sequence
  Description of Artificial Sequence: Synthetic polynucleotide
atgagctctttaaccaaattcaccaacaaatattcaaagcagctgaccattaagaacgaacttatcccggttgggaagacccttgagaatatcaaagagaatggtctgattgatggagatgagcagcttaacgagaattatcagaaggctaagattattgttgacgactttcttcgtgacttcattaataaggcacttaacaatactcagatcggtaattggcgcgagcttgctgacgctttgaacaaagaagacgaagacaatatagagaaactgcaggataagattcgtggaataatcgttagtaaattcgagacattcgatttgtttagctcgtactctattaagaaagacgaaaagattatagacgatgataatgacgttgaagaagaagaactggatctgggcaaaaagactagtagcttcaagtatatatttaagaagaacttatttaaactggttctgccgtcatatttaaagaccaccaatcaagataaactaaagattattagtagtttcgacaacttctcgacatactttcgcgggttctttgagaatcgcaagaacatctttacaaagaagcccattagcacgagcatcgcctaccgcatagtccatgacaatttcccgaaatttcttgacaacattcgttgctttaacgtttggcagaccgaatgcccgcagcttatcgttaaagcggataactatctcaagtcgaagaacgtgattgccaaagacaagagcctggcgaattactttaccgtgggcgcctatgattacttccttagtcagaacgggattgatttctacaacaatattataggcggtctgccggcctttgctggacatgagaagatccagggcctcaatgaatttattaaccaggagtgccagaaagatagcgagctgaaatcgaaactcaagaaccgccatgcgtttaagatggccgtactgttcaaacaaatcctctctgaccgagagaagagctttgttattgatgaatttgaaagtgatgctcaggtgatcgatgcggtgaagaacttctatgccgaacaatgtaaagataataatgtgatcttcaacctgcttaacctgattaagaacattgctttcctgtcggatgatgaattggacggcatattcattgaaggcaagtatctctcttcagtttcacagaagctttactctgattggagcaagctgcgaaacgatattgaagacagtgccaacagtaaacagggtaataaagagctcgcaaagaagattaagacgaataagggtgatgtggagaaggcaattagtaagtacgaatttagcctgagcgaactgaattctatagtacatgataacaccaaattctcagacctgttgtcatgtacacttcacaaagtggcatcagagaaattggtgaaggtgaacgaaggagactggccgaagcacctaaagaacaacgaagagaagcagaagattaaggaaccgctcgacgcattactggaaatttacaatacgctgctgatatttaattgtaaatctttcaacaagaacggtaatttctatgtcgattacgatcgctgcatcaacgaactttcttctgtggtgtacctgtataacaagactagaaattattgtactaagaaaccgtacaataccgataaatttaaactgaacttcaatagcccacaattgggagaaggattcagtaagagcaaggagaatgattgcttaaccttactcttcaagaaagatgataactactacgtgggaattattcgcaaaggcgcaaagattaacttcgatgatacacaggctattgcggataataccgataactgtatcttcaagatgaactacttcctgctgaaagatgcgaagaaatttataccgaaatgctccattcagctgaaggaagtgaaggcgcattttaagaaaagcgaagatgattatattctgtcggataaagagaagtttgcctcaccactggtgatcaaaaagagcacattcttgctggcaacggcacacgttaaagggaagaaagggaacatcaagaaatttcagaaggaatattccaaagagaatccgacagagtatcgtaacagtctgaacgaatggatcgcgttctgcaaggaattcctaaagacatataaggctgctaccatcttcgacataaccaccctgaagaaagcagaggaatatgccgacatcgtagaattctacaaagatgtggacaatctgtgctataaactggagttctgtcctatcaagacctcgtttatcgagaaccttattgacaacggtgacttgtacctgttccgcatcaataacaaagactttagttcaaagagcacaggtaccaagaatctgcacaccttatacctgcaggcgatatttgatgaacgtaacctgaataatccgacgattatgctgaatggaggcgcagaattgttctaccggaaagaaagcatcgaacagaagaaccgtatcacccacaaagcgggaagcatattggtcaataaagtgtgtaaggatggcactagtctggatgataagatacgcaacgaaatttatcagtatgagaataagtttattgacacgctgagcgatgaagccaagaaggtactgccgaatgtgataaagaaagaagctacgcacgatattaccaaggataagcgctttactagtgacaaattcttctttcattgtccactgactataaattacaaagaaggtgacaccaaacagttcaacaacgaggttctgagctttctacgcgggaacccagatattaacattattggtattgatcgaggagaacggaatctgatttacgtgaccgtgattaatcagaagggcgaaattctggattcggtaagctttaacacagttacgaataaatctagcaagatcgagcagacggtagattacgaagagaagcttgcagtgcgcgagaaggaaagaattgaagctaagagatcatgggatagcattagcaagattgcgacgctgaaagaaggctacctgtcagccatcgttcatgaaatctgtctactgatgattaaacataatgccatcgtggtacttgagaacttaaacgcaggatttaaacgcattcgaggaggcttaagtgagaagtctgtttaccagaaatttgagaagatgctgattaataaactgaattacttcgtcagcaagaaagaatcggattggaataaaccctctgggctcttgaacggcctgcagctttctgaccagtttgaatcattcgagaaactcggcatccagtcgggcttcatcttctacgttcctgcggcctatacttcgaagatcgatccgacgacgggattcgctaacgtcctgaacctgagcaaagtccgtaatgtggatgccataaagagctttttctcaaactttaatgagatttcctattctaagaaagaagcactgtttaagttctcgttcgatctggattcattgtctaagaaaggcttctcgtcattcgtcaaattctcgaagtccaaatggaatgtgtatacgtttggcgagcgcattatcaagccaaagaacaagcagggctatcgagaggacaaacggattaacctgacattcgaaatgaagaagctattaaacgaatacaaggtgtcattcgacctggagaataacttgatccctaacttgacctcagcaaatttgaaagatacgttctggaaagagctgttcttcatcttcaagactacacttcagctgcgcaatagtgtaaccaacggtaaagaagacgtgcttatctcacccgtgaagaatgcgaaaggtgagttcttcgtatccggaacccataataagactctgccgcaagattgcgacgcgaacggagcatatcatattgcgctaaagggtttgatgatactagaacgcaacaatcttgttcgtgaagagaaggataccaagaagatcatggcaataagcaacgtggactggttcgagtatgtacagaagaggcgcggtgtactctaa

SEQ ID NO: 291 - DNA, 4005 bp, Artificial Sequence
  Description of Artificial Sequence: Synthetic polynucleotide
atgagctcattaaccaaatttaccaataaatacagtaagcaattaacgataaagaatgagctgatcccggtggggaagacacttgagaatattaaggagaacggtcttattgatggtgatgaacagctgaatgagaactatcagaaagctaagatcattgttgatgactttctgcgcgacttcattaacaaggccctgaataacacgcagataggcaattggcgcgaattagcggacgccctgaacaaagaagatgaagacaacattgagaagttacaggacaagattcgcggcatcatcgtgtccaaattcgaaacgtttgatctgttcagctcctattctataaagaaagatgagaagattattgatgatgataacgacgtagaagaggaagaacttgacctcggtaagaaaacttcaagctttaaatatatctttaagaagaacctgttcaaactggtgcttccgtcttaccttaagactactaatcaggacaaattgaagatcatcagttcgtttgataatttcagcacatactttcgcggcttcttcgagaatcgaaagaacatctttaccaagaaaccgatctcaacctcaattgcctatcgcatcgttcatgataacttcccgaaatttctggacaatatccgctgcttcaacgtctggcagaccgagtgtccgcaattaatcgttaaagctgacaactatctgaaatctaagaacgtcatcgcgaaggataagagtttagcgaactactttacagtaggcgcttacgattactttctgtcgcagaatggcattgacttctataacaatatcatcggtggcttaccagccttcgcaggtcacgagaagattcaaggcctcaacgaatttattaatcaggaatgtcagaaggactctgagctaaagagtaagttgaagaatcgtcacgcgtttaagatggccgtactgttcaaacagattctgagcgatcgtgaaaagagctttgtgattgacgagttcgagtcagacgcgcaggttatcgacgcagttaagaatttctatgcggaacaatgcaaagataacaacgtcatctttaacctgctcaatctgataaagaacatagcgttcctcagcgacgatgaactagacggaatattcatcgaaggtaaatacttaagttcggtcagccagaaactgtattctgactggagcaagctgcgtaatgacatcgaggattccgccaactcgaaacagggtaataaagaactggccaagaaaattaagacaaacaaaggtgacgttgagaaggcgattagcaaatacgaattcagcttaagtgaattgaattctattgttcatgataataccaagttctctgatctgttatcttgtaccctccacaaagtggcgagcgagaagttggtgaaagtgaatgagggtgattggccgaaacatctgaagaataatgaagagaaacagaaaatcaaagaaccgttagatgctctcctcgaaatttacaatacactgcttatcttcaattgcaagagcttcaacaagaatgggaacttctacgtggattacgaccgttgtataaatgaactgagctcggttgtgtatttatataacaagacacgaaattattgtaccaagaaaccttataatacggataaattcaagctgaacttcaactcacctcagctaggagaaggcttctctaaatctaaagagaacgattgcctcacgctcttattcaagaaagatgataattactatgttggaatcattcgtaagggtgccaagatcaacttcgacgatacccaggcgattgctgataatacggataattgcatcttcaagatgaattacttcttgttgaaggatgccaagaaattcattccgaaatgctccatccagctgaaagaagttaaggcacactttaagaaaagcgaagacgattatattctgagcgacaaggagaagtttgcctcgccgttagtcatcaagaaatcaactttcttgttggcgaccgcacacgtgaaaggtaagaagggcaacattaagaagttccagaaggaatacagcaaagagaaccctaccgaatatcgtaattctctgaacgaatggattgcattctgtaaagagtttctaaagacgtataaagcggccaccatcttcgacatcacaaccttgaagaaagcggaggagtatgcggatattgttgaattctataaagatgtggacaacctttgttacaagttggagttctgccctataaagaccagctttattgagaacctgattgacaatggcgatctctatttatttcggatcaataataaagacttctcctccaagtcaaccgggactaagaatctgcacactttgtatttacaagcgatctttgacgaacgtaatctcaataacccaaccattatgctgaacggtggcgccgaattgttctatcgtaaagaatcgattgagcagaaaaatcgtattactcataaagcaggaagcattctagtaaataaagtgtgcaaagatggaacgagcctggacgacaagatccgtaacgaaatttaccagtatgagaataaattcatagatacccttagtgatgaagcaaagaaagtgctgccgaatgtgattaagaaagaagcgacccatgacatcaccaaggataagagattcaccagtgacaaattcttcttccattgcccgctgaccatcaactacaaagagggtgatacgaaacagtttaacaatgaggtgctgagctttctgcgtggtaacccggatatcaatattatcggtatcgatagaggtgaacgcaacctgatatacgttaccgttatcaaccagaaaggcgaaattctggattctgtgtccttcaacacggttaccaataaatcctcaaagattgaacaaaccgtggattacgaggagaagctggccgtccgagagaaggaacgaattgaggccaaacgctcttgggactctatcagcaagatcgccacgttaaaggagggttatctgagtgcaatcgttcatgaaatatgtcttcttatgattaagcataacgcgatcgtagtccttgagaacctgaacgcagggtttaagcgcattcgaggtggtttaagcgagaagagtgtatatcagaaattcgagaagatgttgattaacaagctgaactactttgtatcgaagaaagaaagcgattggaataaaccttctggtctgctgaacggcctacagctcagtgatcaatttgagtccttcgagaagttgggcattcagtcgggtttcatattttatgtcccggcggcgtatacgagtaagatcgatccgaccacgggatttgcgaacgtcctgaatctgtcgaaagttcgcaatgtcgatgcgatcaaatcgttcttctcgaacttcaacgaaatctcctactccaagaaagaagcactcttcaaattctcgtttgatctggatagtttatctaagaagggtttctctagctttgttaagttctctaaatctaagtggaatgtttatacctttggtgaacggattatcaaaccaaagaacaagcaaggttatcgtgaagacaagaggatcaatctgacgtttgaaatgaagaagctattgaatgaatataaggtctcgtttgatttagagaacaacttgattcccaatctgaccagcgctaatttgaaagatacattctggaaagaattgttctttatcttcaagacgaccctgcaactgcgtaatagtgtaacgaacggcaaagaggacgtgctgataagcccggttaagaatgcaaagggcgagttcttcgttagcggtacacataacaagactttgcctcaggactgtgatgccaacggagcttaccacatcgccctgaaaggtcttatgattcttgagcgcaacaatcttgtacgcgaggagaaagatacgaaaaagattatggctatatcaaacgtcgactggttcgaatatgtacaaaagaggcgtggtgtactgtga

SEQ ID NO: 292 - DNA, 4005 bp, Artificial Sequence
  Description of Artificial Sequence: Synthetic polynucleotide
atgagcagcttaacgaaatttactaataaatattcgaaacagctgacgatcaagaacgagcttattcccgtgggcaagacgttagagaacatcaaagagaatggactgattgacggcgacgaacagctgaacgagaattatcagaaggccaagatcattgttgatgactttctgcgtgacttcattaataaagccctgaataatacgcaaatcggtaactggagagagctggcggatgcgttgaacaaagaagatgaggataatattgagaagcttcaggacaagattcgcgggattattgtcagtaagttcgagacattcgatttatttagtagctatagcataaagaaagatgaaaagataatcgatgatgataacgacgtagaagaggaagaactggacctgggtaaaaagactagcagctttaagtacatctttaagaagaatctgtttaaattagttctgccgtcatatttaaagactactaatcaggacaaactcaagattataagcagtttcgataactttagtacttacttccgcggcttcttcgagaacagaaagaatatcttcaccaagaagcccatcagcacctcgatcgcgtatcgtatcgtgcatgacaacttccctaagttcctggataatatccgctgtttcaacgtttggcaaaccgagtgcccacaattgattgttaaagccgataattatctgaaaagcaagaatgtgatcgctaaggataaatctctggctaattacttcaccgttggcgcatacgactacttcttgtcccagaatggcatcgacttctataataatataatcggtggcttaccggcctttgcaggccatgagaagattcagggcttaaatgaatttattaaccaggaatgccagaaggactctgaactgaaatctaaacttaagaatcgtcatgcgtttaagatggcagttctgtttaaacaaattctgtccgatcgtgagaagagctttgtaatagacgaatttgaaagcgacgcacaggtcattgacgcggtcaagaacttctatgccgagcaatgcaaagataacaatgttatctttaacctgcttaaccttataaagaatatcgcatttctgtcagacgatgaacttgacggaatcttcatcgaaggcaaatatctgagctccgtttcccagaaactgtattcagactggagcaaactgcgcaatgacattgaagattccgccaatagcaaacagggtaacaaggaactcgctaagaaaattaagaccaacaaaggtgatgtggagaaggctatctcgaaatatgaattctccttaagtgaactcaatagcatcgtgcatgataatactaagttctctgatttgctgagttgcaccttgcataaagttgcctctgagaagttagtgaaagtgaacgagggagactggccgaagcatctgaagaataatgaggagaaacaaaagatcaaagaaccgttggatgcactgctggaaatctataatacgctgcttatctttaactgcaaatcgtttaataagaacggtaacttctatgttgattatgaccgctgcattaatgaattatcatcagttgtttacctgtacaacaagacccgcaactactgtacgaagaaaccatacaacactgataaatttaaattaaactttaacagccctcagttgggtgaaggattctcgaaatcgaaagagaatgattgcctgaccctcttgtttaagaaagacgataactattatgttggcatcatccgcaaaggagcaaagataaacttcgacgatacacaagcgatcgctgacaacaccgacaactgcatcttcaagatgaattacttcctgttgaaagacgcgaagaaatttatcccgaaatgtagtatccagctgaaagaagtgaaagcgcattttaagaaaagtgaggacgattatattctgagcgataaagagaaatttgcgagcccactggtaatcaagaagagcactttccttctggcgacagctcatgtcaagggcaagaaaggtaacatcaagaagtttcagaaagaatactctaaggagaacccgactgaatatcgtaattctctcaatgaatggatcgcgttctgcaaagaatttctgaagacttacaaggcagctacaatctttgacattacgacacttaagaaggccgaagaatacgccgatatcgtggagttctacaaggatgtagacaacctgtgttataaattagagttctgtccgattaagacaagctttattgagaacctgattgataatggcgacctgtatctgttcagaattaataataaagacttctcttctaaatcgacgggtacaaagaatttacacaccctgtaccttcaggcaatcttcgacgaacgaaatcttaataacccaaccataatgcttaacgggggagcagaattgttctatcggaaggagagcattgagcagaagaatcgcattacccataaggccgggtctattctagtcaataaagtttgtaaagacggcacgtcactggacgacaagattcggaacgagatctaccaatatgagaacaaattcattgacaccctgagtgacgaggccaagaaggtgttaccgaacgttataaagaaagaggcaacccacgacatcacgaaggataaacgtttcacctctgataagttcttctttcattgcccgttaacaatcaattataaggagggcgatactaagcagttcaacaatgaagtgctttcattcttgcgtgggaatccggatattaacatcatcggcatcgatcgaggcgagcgtaatcttatctatgttacggtgataaaccagaaaggagagattctggactctgtgtcattcaatactgtcacgaacaaatcttccaagatagaacaaacagtagattatgaagagaagttagccgttcgtgagaaagaacgtatcgaagccaagcgttcttgggattcgatctcgaagatcgccacgttgaaagaaggttatctttccgcaatcgtgcatgaaatttgtctgctgatgattaaacataatgcgatcgtggtgttagagaacctgaatgcagggttcaagaggattcgtgggggtctgtccgagaagtcagtttatcagaaatttgagaaaatgctgattaataaactcaactatttcgtgagtaagaaagaatcggactggaacaaaccgtccggacttctgaatgggctccaactgtcagatcagttcgaaagcttcgagaaacttggtatccagagtggtttcatcttctatgttccggcggcctatactagcaagatcgatcctactaccggcttcgccaatgtcttgaatttgtctaaagtgcgcaatgttgatgcgattaaatctttctttagcaatttcaatgaaatctcatactcaaagaaggaagcattatttaagttctcatttgacctggatagcctgtccaagaaagggttctcgtcgtttgtgaaattctccaaatctaaatggaatgtatacacctttggtgaacgtattatcaaacctaagaacaagcaaggttatcgtgaggacaagcggattaacctgacgttcgaaatgaagaaactcttgaacgagtataaagtgagcttcgaccttgagaataatctgattcccaatctgacctccgcaaacttgaaagataccttctggaaagaactgttcttcatctttaagaccacattacagcttcggaattcagttacaaatggtaaagaagatgtcctgattagcccagttaagaacgctaagggcgagttctttgttagcggaacacacaataagacactaccacaggattgcgatgctaatggtgcctatcatatcgcgttgaaaggcctgatgattctggagcgtaacaatttagtgcgtgaagagaaagacaccaagaagattatggcgataagtaatgtcgactggtttgaatatgtgcagaaacgtcggggagtcctgtga

SEQ ID NO: 293 - DNA, 4005 bp, Artificial Sequence
  Description of Artificial Sequence: Synthetic polynucleotide
atgtcgagcttaaccaaatttaccaataaatactctaaacagctgaccataaagaacgaacttattccggtgggtaagacgctggagaatatcaaagagaacggtttgattgatggcgatgaacagcttaacgagaattatcagaaagcaaagattattgtggatgacttcttgcgtgatttcattaataaagcactgaacaacacccaaattggcaactggcgtgaactcgccgatgcattaaacaaggaggatgaagataacattgagaagctgcaggacaagatccgcggcattattgtctctaaattcgagacattcgatttgttctccagctacagtattaagaaggatgagaaaattattgatgacgataatgatgtagaagaggaggaattagatctcggcaagaagacatcgtcgttcaagtatatcttcaaaaagaacctattcaaactggtgctgccatcttacctcaagaccaccaaccaggacaaactcaagatcatcagctcgttcgataactttagcacatacttccgtgggttctttgagaaccgtaagaacatcttcaccaagaaaccaatctcaacgtcgattgcataccgaattgtacatgataatttcccgaaatttctggataatatccgctgcttcaacgtctggcagaccgagtgcccacagctgattgtgaaagcggataactatctcaagtcaaagaacgtcattgcgaaagataaatccttagctaactacttcactgtcggtgcctatgattatttcttgtctcagaatggtatcgatttctataacaacattatcggcggactgccggccttcgctggtcatgagaagattcagggtctgaacgagttcatcaaccaggaatgccagaaggatagcgaactaaagagtaaacttaagaatcgccatgccttcaagatggccgtcctatttaaacaaattctgtcagatcgtgagaagtcgtttgtaattgatgagtttgagtcggatgcccaagtgattgatgccgtgaagaacttctacgctgagcagtgcaaagataacaacgtcatcttcaacctgctgaacctgatcaagaatattgcgtttctgtctgacgatgagctggacggcatattcattgaaggtaaatatcttagcagcgtgagtcagaaactgtacagtgactggtcaaagctacgcaacgacatcgaagactcggcaaatagtaaacagggaaacaaagaactggcaaagaaaatcaagactaacaaaggtgatgtagagaaagcgatctcgaagtatgaattctcgctgtccgaactgaactcgatcgtgcacgataatactaagttctctgatctcctgagctgtaccctgcacaaagtagctagcgagaagttagtgaaagtcaacgaaggagactggcccaaacacctaaagaataatgaagagaagcagaagatcaaagaaccattggacgcactgttagaaatctacaacaccttactgatatttaattgcaagtcatttaataagaatggtaatttctatgtagattatgaccggtgcatcaatgaactgagctcagttgtctatctctataacaagacccgaaactattgcacgaagaaaccgtacaataccgacaaatttaaattgaactttaattctcctcaactgggcgaaggctttagcaaatccaaggagaacgattgcctaacgttattatttaagaaagacgacaactattatgtgggaattattcgaaagggtgccaagattaactttgatgatacccaagccatcgcagacaacacggacaattgtatctttaagatgaactatttcctattgaaagatgcaaagaaattcatacctaaatgctcaatccagctgaaagaagtgaaggcccactttaagaaatcagaggatgactatattctgtctgacaaagagaaatttgcatcaccgctcgtcataaagaaatctacattcttgctggcgaccgctcacgttaaaggcaagaaaggtaacattaagaaatttcagaaggaatattcgaaggagaacccaactgaataccgcaactctctgaacgaatggatcgccttctgcaaagaattcctaaagacgtacaaagccgcaacgatattcgatattactacgcttaagaaggcggaagaatatgcagatatagtggaattctataaagatgtagataatctgtgttacaagttggagttctgtccaatcaagacaagcttcattgagaatctgatcgacaacggcgatctgtatctgtttcgcatcaataataaggatttctcatcaaagagtactggtacaaagaaccttcatacgctctacctgcaggccatatttgatgagcgcaacctaaataacccaacgatcatgttgaatggaggagcggaattattctaccgtaaagaaagtatcgaacaaaagaatcgtattacccacaaagcaggaagcattctggtgaataaagtgtgcaaagacggtactagccttgatgacaagatccgtaacgaaatttatcaatatgagaataagtttatcgatactctgtcagatgaagcaaagaaagtgttgccgaatgtgataaagaaagaggcgacgcacgatataaccaaagacaaacgctttacgtctgataaattcttctttcactgtccactgacaatcaactataaagagggtgataccaagcaatttaataacgaggtgctgtcgttcttaagaggtaacccagacatcaatattattggtattgaccgtggcgaacgtaacttgatttatgttaccgtgattaatcagaaaggcgaaatcctggatagtgtgtcgtttaataccgtcaccaataagagctcaaagatcgaacagacggttgattacgaagagaagttggcggtcagagagaaggaacgtattgaagctaagaggagctgggatagcataagtaagattgccacgctgaaggagggttacctatcggcaattgtccacgaaatctgcctgctgatgattaaacacaatgccatcgttgtactggagaacctgaatgctgggtttaagagaatccgggggggcctgtccgagaagtctgtttaccagaaattcgagaagatgctgattaataagctcaattacttcgtttcaaagaaagaaagcgattggaacaaaccgtccggcttgcttaacgggttacagctctcggaccaatttgaatcgtttgagaagttaggcattcagtctggattcatcttctatgtgccggcagcatataccagcaagattgacccgactacgggatttgcgaacgtgctgaacttaagcaaagtgcgcaatgtggatgccattaaatcgttcttcagcaactttaacgagattagctatagcaagaaagaggcgctgtttaagtttagctttgacttggatagcctctcaaagaagggcttcagtagtttcgtcaaattctccaaaagtaagtggaatgtctatacatttggcgagcgcattattaagccaaagaataagcagggttatcgtgaagataaacgaatcaaccttacctttgagatgaagaaactgctgaacgaatataaagtatcgttcgaccttgagaacaacttaatcccgaatctgacctcggcgaacctcaaagataccttctggaaagaactgttctttatcttcaagaccaccctgcaattacgtaatagcgtaacaaatggcaaagaggacgtattaatttctcccgttaagaatgcgaagggagaattcttcgtttctggtacgcacaataagaccctgcctcaggactgcgacgcgaacggtgcgtaccatattgcacttaaaggcctgatgatcctcgagcgtaacaatttagtgcgggaggagaaggatacgaagaagattatggctatctccaacgtcgattggtttgaatacgttcagaaacgaagaggggttctataa

SEQ ID NO: 294 - DNA, 4005 bp, Artificial Sequence
  Description of Artificial Sequence: Synthetic polynucleotide
atgagtagcttgacgaaatttactaacaagtacagcaaacaactgacaatcaagaatgagctgataccggttggcaagactttagagaatattaaagagaatggcttaattgatggcgatgaacaattgaatgagaattatcagaaggcaaagatcattgtagatgatttcctgcgcgacttcattaacaaggccctgaacaacacgcagatcggcaactggcgggaactggcagacgcactaaacaaagaagatgaagataacattgagaagctgcaagacaagattcgcggaattattgttagcaaatttgaaaccttcgatctgttcagctcctattctataaagaaagatgaaaagattatcgatgatgacaacgatgtggaggaggaagaactggatctgggcaagaagacgtcaagcttcaagtacatctttaaaaagaacttgtttaaactcgtcttaccgagctatttaaagaccactaaccaggataaactcaagatcatttcttcattcgataactttagcacctacttccgcggcttctttgagaatcggaagaatatatttaccaagaaaccgatttccaccagcattgcatatcgtatcgtccatgataactttccgaaattcctggacaacatcaggtgcttcaatgtttggcagacagaatgtcctcaactcatagtcaaagccgataactatctgaagagcaagaacgtcattgcaaaggataagagtctggcaaactacttcactgtcggtgcatacgattacttcttgagccagaatggtattgatttctacaataatattattggcgggctgccggcctttgccgggcatgaaaagatacagggtctgaacgaattcattaatcaggagtgccagaaggattctgaactgaaatccaagctgaagaacaggcacgcttttaagatggccgttctgttcaagcaaatcctgtctgatcgcgagaagagctttgtcattgatgaatttgagagcgatgcacaagttattgacgcagtaaagaacttctacgcagaacagtgcaaagataacaacgtcatattcaatctcctgaacctgataaagaatattgctttcttgagcgatgatgaactggatggtatcttcatcgagggtaagtaccttagtagtgtaagtcagaagctttacagtgattggagcaaactacgtaacgacatcgaagactcagcgaacagcaagcagggcaataaagaattggcaaagaagattaagacaaacaaaggtgatgtggagaaggcaatttcgaagtatgaattctccttatctgaactgaattcaattgtacacgacaatactaaattctcagaccttctttcgtgcacgcttcataaagtggcatcagagaagctcgttaaggtgaacgagggtgattggcctaaacacctgaagaacaatgaagagaagcagaagattaaagaaccgttggacgctttactggaaatttataatacgttactcatctttaactgcaaatcattcaataagaacggcaatttctatgtggattacgatcgctgcattaatgagctctcaagtgtagtttacttatataacaagactcgaaattactgcacaaagaaaccttataatactgataaatttaaactgaacttcaactctccgcagcttggtgagggattctcgaagagtaaggagaatgattgcctgactctgctattcaagaaagacgacaactactacgtcggcattattcgtaaaggtgccaagattaatttcgatgatacccaggcgatagctgataacactgataactgtatcttcaagatgaattatttcctacttaaagatgctaagaaattcattcctaagtgctcaatccaactgaaagaggtcaaagcacactttaagaaaagcgaagacgattatatcctgagcgataaggagaagtttgctagcccgctggttattaagaagagcacctttctactcgcaaccgcgcacgtgaaaggcaagaaaggtaatatcaagaaattccagaaagaatatagcaaagagaacccgacggagtacagaaactctctgaatgagtggattgcgttctgcaaagaatttctaaagacgtataaagcagcgacgatattcgacattaccaccctaaagaaagctgaagagtacgccgatatagtcgagttctacaaagatgttgacaacctgtgttataagctggaattctgtcctataaagacgtccttcatcgagaatttaattgataacggagatctgtacctgtttcgtatcaacaataaagatttctcaagcaaatctacgggtacaaagaatttgcataccctgtacctccaggccatattcgatgagcgcaatctgaacaacccaacgatcatgctgaacggaggggccgagctcttctatcgcaaagagagcattgaacaaaagaatcgtattacacacaaagctggctcgattctggtaaataaagtgtgcaaagacggtacctccctggatgataagattcgcaacgagatttaccaatatgagaacaaatttatcgatacactcagcgatgaggccaagaaagtgttgccgaacgtgatcaagaaagaggccacgcatgatattacgaaagataaacgctttaccagtgataagttcttcttccattgtccgctgaccatcaactataaggagggagatactaaacagttcaacaacgaagtgctctcgttcctgcgtggcaacccggatattaacataattggcattgatcgcggagaaagaaacctaatctacgtgacagtaatcaaccagaagggcgaaatcttagatagcgtgagctttaataccgttaccaacaaatcgtcgaagatagaacagaccgttgactatgaagagaaacttgcagtgcgcgagaaggaacgtatcgaagccaaacgttcgtgggattcgatcagtaagatcgcgactttaaaggaaggttacctttcagcgattgtgcatgagatctgtttgctgatgattaaacataatgccatcgtggtcctggagaacctgaatgcaggttttaagagaattaggggaggactgagtgagaagagcgtgtatcagaagtttgagaagatgctgattaataaattaaactacttcgtatcgaagaaagaatccgactggaacaaaccgtcaggacttctgaacggtcttcagttgagcgaccagtttgagtccttcgagaagttgggtatccagagtggcttcatcttctatgtaccggcggcttacacctctaagattgatcctacaaccggctttgcaaatgtgctgaatctgtctaaggttagaaacgttgatgccataaagagtttcttctcgaactttaatgaaatctcttactcgaagaaagaagcgctgtttaagttctcattcgaccttgatagtctgagcaagaaaggcttcagttcatttgttaagttcagcaaatctaaatggaatgtgtacacgttcggcgagcgaattattaaacccaagaataaacagggttatcgggaagataaacgcattaatctgaccttcgaaatgaagaagttgctgaatgagtacaaagtctctttcgatcttgagaacaatctgattccaaaccttacttccgctaacctcaaggatacattctggaaggaacttttcttcatcttcaagactacactccagctgcgtaatagtgtaactaatggcaaagaagacgtgctgattagcccagtaaagaatgctaaaggtgagttctttgtgtccgggacccacaataagacgctgccgcaggattgtgatgcgaatggtgcctatcacatcgcgctgaaaggattaatgattctcgaacggaataatctggtgcgcgaggagaaagatacaaagaaaatcatggcaattagcaatgttgattggtttgagtacgtacagaaacgtagaggagtgctgtga

SEQ ID NO: 295 - DNA, 4005 bp, Artificial Sequence
  Description of Artificial Sequence: Synthetic polynucleotide
atgtcctcgctgaccaagttcactaataagtacagcaaacagttgacgatcaagaatgaactgatcccggtgggtaagaccctcgagaatatcaaagagaatggactgattgatggcgacgaacagctgaacgagaactaccagaaagccaagatcattgtagatgacttcctgcgcgatttcataaacaaagcactgaataacacccagatagggaactggcgggagttggccgacgcgttgaataaggaagacgaagataacattgagaaactgcaagacaagatcaggggaattattgtttcgaaattcgagacctttgatttattcagtagttacagtatcaagaaggacgagaaaataatcgacgacgataatgatgttgaagaagaagaattggatctgggcaagaaaacaagctccttcaaatatatcttcaaaaagaatttgttcaaattagttctgccaagctatctgaagacgactaaccaggacaagctcaagattatttcgagctttgataacttcagtacctacttccgagggttctttgagaatcgaaagaatatctttacaaagaaaccgatcagtaccagcatcgcatatcgtattgttcatgataactttcctaaattcctggataatattcgctgtttcaacgtctggcagactgaatgtccacagctaatcgttaaggcggacaactacctcaagtccaagaacgttatagccaaggacaaatcgttagctaattacttcacagtgggagcgtacgattactttctatctcagaacggtattgacttctacaacaatataataggaggactgccggcgttcgcaggtcacgagaaaatccagggtcttaacgagtttattaaccaggaatgtcagaaggattcggaactcaaatccaaattaaagaaccgccacgcttttaagatggctgtcctgttcaaacagattctcagtgatcgtgagaagagtttcgtgattgatgagtttgagagtgatgcgcaggtaatagacgctgtgaagaacttctatgccgagcagtgcaaagataataatgtcatctttaatctgcttaatttaattaagaacattgcctttctttccgatgatgaactggatggaatctttatcgaaggcaaatacttaagcagtgtgagccagaagttgtactcagattggtctaaactgcgcaacgacatcgaagatagcgcgaactctaaacaaggcaataaggagctcgcgaaaaagattaagactaacaaaggcgacgttgagaaagcaattagcaaatatgagttctcactgagcgaattaaacagcatcgtgcacgataacaccaaatttagcgacctgctgtcatgcacgctccacaaagtggcatctgagaaactggttaaagttaacgaaggcgattggccgaaacatctaaagaataatgaagagaagcagaagattaaagaaccgttggacgcactactggaaatttataacacgctgctgatattcaactgtaagagtttcaataagaacggcaatttctatgtcgattatgatcggtgtataaatgaactgtcgtcagtcgtttatttgtataataagacccgcaactattgtaccaagaaaccctacaataccgataaatttaaattaaactttaattcaccgcaactaggtgagggtttctctaagagcaaagagaacgactgtctgaccctgctgttcaagaaagacgataactattacgtcggcattatccgcaagggcgccaagattaacttcgatgacacgcaagccattgctgacaacactgacaattgtatattcaagatgaactacttcctgctcaaagatgcgaagaagtttattccgaaatgttcaattcagcttaaggaggtgaaagcgcacttcaagaaaagcgaagacgactatattctatctgataaagagaaattcgcatctcctttggtgatcaagaagtccacattcctgctggcgacggcccatgtgaaagggaagaagggtaacatcaagaagttccagaaagaatattccaaagagaacccaacagaatatcgtaactctctgaatgaatggattgctttctgcaaagaattcctcaagacgtataaggcagctaccatctttgatatcacgacgctgaagaaagccgaggaatatgccgatatagtggagttctacaaagatgttgacaatctttgctataaacttgagttctgtccgattaagacgtcatttattgagaacttaatcgataatggcgatctgtatctcttccgcattaataacaaagacttcagtagtaagagcaccggaacgaagaacttacataccctgtacctgcaggcgatcttcgatgaaagaaatttgaataacccaaccatcatgctgaacggaggtgcggagctgttctatcgcaaagaatccattgaacagaagaaccgcattacgcataaagcaggcagcattcttgtaaacaaagtatgcaaagacggaaccagtctggacgacaagatccggaatgaaatctaccaatatgagaataaatttatcgacacgctctcagatgaagcaaagaaagtactgcccaatgttatcaagaaagaggcgacgcatgacatcactaaagataagagattcacgagcgataaatttttcttccactgtcctttgacaattaattacaaagaaggcgatactaaacagtttaataatgaagttctgtcgttccttagaggcaatccggacattaatattattggtatcgatagaggagaacggaacttaatttatgtcactgtgattaatcagaagggcgagatactagactcggtgtcgttcaacaccgtgaccaacaaatcgtctaagattgaacaaacggttgattatgaggagaaactggccgtgcgcgagaaagaaagaattgaggccaaacgtagttgggattccattagtaagattgctaccctgaaagagggttatctgagcgcgatcgtgcatgagatttgcctgttgatgattaagcacaacgcgattgtggttctcgagaacctgaatgcgggctttaaacgtatccgtggcggtcttagcgagaagtcggtctaccagaaattcgagaagatgcttataaacaaattaaattacttcgtgtcaaagaaggaatcggattggaataaaccaagtggactgctcaacgggctgcagctaagtgatcagttcgaatcattcgagaagttgggcattcagagtggtttcatattctatgtaccggctgcgtacacctctaagatagatccgacgaccggatttgcaaatgtattaaatctgtctaaagtacgtaacgtggatgcgattaaatctttctttagcaacttcaacgaaattagttacagtaagaaagaagccttgttcaagtttagctttgacctggattcactgtccaagaagggtttctctagcttcgttaaattcagtaagtcaaagtggaacgtttatacattcggtgaaagaatcattaaacctaagaacaaacaagggtaccgtgaagataagcgtattaacctcacctttgaaatgaagaaactgttgaacgaatacaaagtgagtttcgacctcgagaataacttgattcctaacttgaccagcgctaatcttaaggataccttctggaaagaattgtttttcatctttaagacgactctccagcttcgtaatagcgtaacgaacggtaaagaagatgtactgatttctccggtgaagaacgcgaagggcgaattcttcgtcagtggcacccataataagacccttccgcaggattgcgatgccaatggtgcctaccatatcgcattgaaaggtttgatgatcctggagcgcaataacctggttcgtgaggagaaggacacaaaaaagattatggctattagcaatgttgattggtttgaatacgtacagaagcgtcgtggcgtgctgtaa

SEQ ID NO: 296 - DNA, 4005 bp, Artificial Sequence
  Description of Artificial Sequence: Synthetic polynucleotide
atgtcgagcttaacgaaatttacaaacaaatactccaagcaactgaccattaagaacgagctcattccagtcgggaagacgttagagaatattaaagagaacggcttgatcgatggcgacgaacagctgaacgagaattaccagaaggcaaagatcatcgtagatgactttctgcgcgacttcataaataaagcattgaataacacgcaaatcggcaactggcgcgaactggccgatgccctgaataaagaagatgaagacaacattgagaagctgcaggataagattagaggaattatcgttagcaagtttgaaacctttgatttgtttagtagctatagcattaagaaggatgaaaagatcattgatgacgataatgatgtggaggaagaagaattggatctgggtaagaagacctcttcgtttaaatatatattcaagaagaatctgtttaagctggtgttaccttcttatctcaagacaaccaatcaggataagttaaagatcatatcgtcattcgacaacttcagcacctatttccgcggcttcttcgagaatcggaagaacatctttactaagaaaccgatctcgacgtctattgcctaccggattgtacacgacaatttcccaaagttcttggacaacatccggtgcttcaatgtatggcagacagaatgcccgcagctgatcgtgaaagcggataactatctgaaaagcaagaacgtaattgccaaagataaatctctggctaattatttcacggtaggtgcgtatgattactttctgtctcagaatggaattgacttctacaacaatatcattggtggattaccagccttcgccggccatgagaagattcaaggtcttaatgaatttattaaccaggaatgccagaaagattcagagttaaagagtaaactaaagaaccgtcacgcgtttaagatggcggtgttatttaaacagatcttaagcgatagagagaagagtttcgtcattgatgaattcgaaagcgatgctcaggttatcgacgcagtcaagaatttctatgccgaacagtgtaaagacaataatgtgatattcaacctgctgaatcttattaagaacatagcgtttctgagtgacgatgagctggacggaatatttattgaaggcaaatatctctcgtctgtttcacagaaactttatagcgactggagcaaactgcgtaatgacatagaagatagcgcaaacagcaagcaaggtaacaaagagctggctaagaagataaagaccaacaagggtgacgtagagaaggcgatcagcaagtatgagttctctttgagtgaactgaattctatcgtacacgacaacacgaaatttagcgacctccttagttgcactcttcacaaagttgcgtcggagaaacttgttaaagtaaacgagggtgattggccgaaacatctgaagaacaatgaagagaaacagaagattaaagaaccgctggatgcactgctggagatttacaatacacttctgatcttcaactgcaagagcttcaacaagaacggtaatttctacgtagattatgatcgttgtatcaacgaactctcgtctgttgtgtacctgtataataagacccgtaactattgtacgaagaagccgtataataccgataaattcaaactcaacttcaattcaccgcagctgggcgaaggcttctcgaaatctaaggagaacgactgtctgaccctcctgttcaagaaggatgataactactatgttggtattatacgcaaaggtgctaagatcaacttcgatgatacccaggcgatcgccgacaataccgataactgcatcttcaagatgaattacttcctgctgaaagatgcaaagaaattcatcccgaagtgctctatccagctgaaagaggtaaaggcccactttaagaaatcagaagatgattacattcttagcgataaagagaaatttgcgagtccgttagtcattaagaaaagtacctttctgctggcaacggcgcatgtgaaagggaagaaaggcaatataaagaaattccagaaagagtatagtaaagagaacccgacggaatatcgtaacagtctgaacgaatggattgcgttctgtaaagaatttctgaagacatataaggccgccacaatattcgatattacaacgcttaagaaggcggaagaatatgcggacattgtcgaattctataaagatgtggacaatctgtgctataaactggaattctgccctattaagacgagctttattgagaacttaatagataatggtgatctttatctctttcgcattaataacaaagacttctcgtcaaagagtacaggcacgaagaatcttcatacattatatttgcaggccatatttgatgagaggaacctcaacaacccgacaattatgttgaatggcggcgcggaactattctaccgtaaggaatctatcgaacagaagaatcgtatcacccataaagccggctctattctcgttaacaaagtttgtaaagatgggacaagtctggacgataagattcgcaatgagatttatcaatatgagaacaaatttatcgacacgctgtcggacgaggccaagaaggtcctgcctaacgtcatcaagaaagaagcgacacacgacatcaccaaggataagaggtttaccagcgataaattcttctttcattgccctctgaccattaactataaagagggtgataccaaacagtttaataacgaggtgctcagctttctgcgaggcaatccggatatcaacattattgggatagaccgaggcgagcgcaacctgatttacgtaaccgttatcaaccagaagggcgagattctggatagcgtgtctttcaatactgttacgaataagagcagtaagatcgaacagaccgtggattacgaagagaagctggcggtgcgtgagaaagaacgtattgaggcaaagcgctcttgggattcaattagtaagattgctactctgaaagaaggatatttatctgccatcgtccacgaaatttgcctcctgatgattaaacataatgcaatagttgtgctggagaacctcaacgccgggtttaagcgtattagaggaggcctgagcgagaagtcagtttaccagaaattcgagaagatgctcatcaataaactgaactacttcgtatctaagaaagaaagcgattggaacaagccgtctgggctactcaacggcctacaactgagtgatcagtttgaatcatttgagaagctaggtattcagtcagggtttatcttctatgttccggcggcgtatacctcgaagatcgaccctacgaccggcttcgccaatgtcctgaatttatctaaagtccgaaatgtagatgcgattaagtcattctttagtaacttcaacgaaattagctattctaagaaagaagccctgttcaaattctcatttgatcttgattctctgtccaagaagggctttagctccttcgtcaaattctcgaagtctaagtggaatgtatacacgttcggcgagcgtattatcaagcctaagaacaaacaaggttatcgtgaggacaagaggattaatctaaccttcgaaatgaagaagttgttaaacgaatacaaagtttcgttcgatcttgagaataatctgataccaaatctcacttcagctaacttgaaggatactttctggaaagaactgttctttatctttaagaccactctgcagcttcggaactctgtaaccaacggcaaggaggatgtactgatttcaccagttaagaatgctaaaggtgaattctttgtctccggcacacacaataagaccctgccgcaggattgcgacgcgaatggagcctaccatattgcactgaaaggtttaatgatcctggaacgcaacaacctggtcagggaggagaaggacacgaaaaagatcatggcaatatctaacgtcgattggttcgagtacgtacagaaacgacgcggtgtattgtga

SEQ ID NO: 297 - DNA, 4005 bp, Artificial Sequence
  Description of Artificial Sequence: Synthetic polynucleotide
atgtcctctttgactaagtttactaataaatatagcaaacagcttaccattaagaacgagctgattccggtaggtaagaccttggagaatatcaaggagaacggcttaattgatggcgacgagcaactgaacgagaattatcagaaagcaaagattattgttgacgatttcttacgtgacttcattaataaggcgcttaataatacccagatcggaaattggcgcgaactggcggatgcattgaataaggaggatgaggacaacatagagaaactgcaagacaagatccgtggtatcattgtcagcaaattcgagaccttcgatttattctcgagttattcgataaagaaagatgagaagatcatagatgacgataatgacgtcgaagaagaagaactggatctaggaaagaaaaccagctcattcaaatatatattcaagaagaatttattcaaattggtcctgccttcttacttaaagacaacaaatcaggacaaactgaagattattagttcgttcgacaatttctcaacatacttccgcgggttcttcgagaatcggaagaatatcttcacaaagaagccgatttctacgtctattgcataccggatagtgcatgacaactttccgaagtttctggataacattcgttgctttaatgtttggcaaaccgagtgtccacagctgattgttaaagcagacaattacctaaagagcaagaacgttattgcgaaggataaatccctggcgaattactttaccgtcggtgcgtacgattacttcctatctcagaacggcattgatttctataacaacattattggcggtttaccggccttcgccggtcacgagaagatccaaggtctcaacgagtttatcaaccaggagtgccagaaggacagtgagcttaagagtaaactaaagaatcgacatgcgttcaagatggccgttctgtttaaacagattctttctgacagggagaaatcatttgtgatcgatgaatttgaaagcgatgcgcaggtgatcgacgcggtaaagaacttctacgcagaacagtgcaaggacaataatgtcatatttaacctgctgaacctgataaagaatatagcgttcctttcggatgacgaattagacggaatatttatcgaaggtaagtatctgagctcggtcagccagaaactgtacagtgattggagcaaactgaggaatgatatagaagattctgctaactcgaaacaaggtaataaggaactcgctaagaaaattaagacaaataaaggtgatgtagagaaagccatttcaaagtacgaattctcactgagcgaactgaattcaatcgtgcatgacaacacaaagttcagcgatttgctgtcgtgtaccttgcacaaagttgcatctgagaagttggtgaaggttaatgagggcgattggccgaagcacctaaagaacaatgaggagaaacaaaagataaaggaaccactggatgcactgcttgaaatttacaataccctgctgatattcaactgtaaatcattcaataagaatggcaacttctatgtggattacgaccgctgcatcaatgaactgagctctgtagtttatctttataataagacgcgtaattattgcacaaagaaaccttacaacaccgacaaatttaaactgaactttaacagcccgcagcttggtgaaggcttctcgaagagcaaagagaatgactgtctgacgctgctgtttaagaaagatgataattattatgttggtattattcgtaaaggagcaaagatcaacttcgacgacacacaggcgatcgcagataacactgacaattgcatatttaagatgaactatttcttactgaaagatgcaaagaagttcatcccgaaatgttctattcaactcaaagaagttaaagcgcactttaagaagtctgaagatgattatattctgtctgacaaagagaagtttgcaagtcccttggtgattaagaaatcgacgttccttctggccaccgcgcacgttaaaggcaagaaaggcaacataaagaaatttcagaaggagtactctaaagagaatcctacagaataccgtaatagtttgaatgagtggattgcattctgcaaggaattcctcaagacttataaagccgcaacaatattcgatattacgacccttaagaaagcagaagaatacgctgatattgttgaattctacaaagatgtagataacttatgttataaactggagttctgcccgataaagactagcttcatcgagaatctgattgacaatggcgatttatatttgttccggattaacaacaaagatttcagtagcaaatccactggtacgaagaatctgcacactctttacttacaagctatctttgatgaacgcaacctcaataacccgaccatcatgctgaatggtggcgcagaactgttctatcgtaaagaaagcatcgagcaaaagaaccgtatcacgcataaagccggttcgattctcgtgaacaaagtgtgtaaagatggcacatcactggatgacaagatacgcaatgaaatctatcagtatgagaataaatttattgatactctgtcagatgaggctaagaaagtgctgcctaatgtaatcaagaaagaggcaacccatgatattaccaaggataaacggttcacgtctgataagttcttcttccattgtcctttaactatcaactacaaagagggcgatactaagcaatttaataacgaagttctttcctttcttagagggaacccggacatcaacattattggcattgaccgtggtgaacgtaacctgatctatgtgaccgttattaatcagaaaggtgaaatcctggactccgttagtttcaataccgtaacgaataagtcttctaagattgaacagactgtggattatgaagagaaactagccgtccgagagaaagagcgaatagaagctaaacgtagctgggattcaatctctaagatcgcgaccttgaaagaagggtatctgagtgcgatcgttcatgagatttgcttactgatgatcaaacacaatgctatcgtggttctggagaatcttaacgcaggctttaaacgtattcgaggagggctttcagagaagtcggtgtatcagaaattcgagaaaatgcttattaataaactgaactacttcgtttcaaagaaagaaagtgattggaataaaccaagcggcctgttaaacggtttacagctgagtgatcagtttgaaagcttcgagaagctgggcattcagagtggattcatcttctatgttcctgcggcatataccagtaagattgatccaaccactggctttgctaatgtactgaatttaagtaaagttcgtaacgtcgacgccattaaatcattcttctctaactttaacgaaatcagctacagtaagaaagaagcgctgtttaagttctcattcgatttagattcgctgagtaagaaagggttctcgagctttgttaagttctctaagagtaaatggaacgtatacaccttcggtgaacgtataattaagccaaagaacaagcaaggatatcgcgaagacaagcgtatcaatctgacattcgagatgaagaaactcctgaacgagtataaggtttcgttcgatctggagaataacttgattccgaacctaacgtctgcgaatctgaaggatactttctggaaagaactatttttcatcttcaagactaccctgcagttgcgcaacagtgttactaatggtaaggaagacgtcttgattagtccggtcaagaatgccaagggcgagttctttgttagcggcacgcacaacaagactctgccacaagactgtgatgcgaatggtgcatatcacatcgcgttgaaaggtcttatgatcctggagcgcaataaccttgtccgcgaagagaaagataccaaaaagattatggcaatttccaacgtggattggttcgaatacgtccagaaacggcgcggcgttctgtga

SEQ ID NO: 298 - DNA, 4005 bp, Artificial Sequence
  Description of Artificial Sequence: Synthetic polynucleotide
atgagctcacttaccaaatttaccaataagtatagtaaacagctgaccattaagaatgaactgattccggtgggcaagacattggagaatattaaagagaatggacttattgatggagacgagcagcttaatgagaactatcagaaggcgaagatcatcgtggatgactttctgcgggatttcattaataaagcattgaataacacgcaaatcggcaattggcgtgaacttgctgatgctcttaataaagaagacgaggataatattgagaagctacaggataagatccgtggaatcatcgtgagcaagttcgagacgttcgacctgttcagttcgtatagcataaagaaagacgagaaaataattgacgacgataacgacgttgaagaagaggaactggatctagggaagaaaacgtcaagctttaagtatatctttaagaagaacttgtttaaactggtattaccgtcgtatctgaagacaacgaatcaggacaaattgaagatcataagctctttcgataacttcagtacgtacttcaggggcttcttcgagaaccggaagaatatcttcacaaagaagccgattagtactagcatcgcttaccgaattgttcacgataactttccaaagttcttggataatattcgctgcttcaacgtgtggcagactgagtgcccgcaactcattgttaaggccgataattatctcaagagcaagaatgtgatcgctaaagataaatctctcgctaactacttcacggtgggagcgtacgattactttctgtctcagaacggtatagatttctacaataatattattggtggccttccagccttcgccggccacgagaagatccagggcctgaacgagttcattaaccaggaatgtcagaaagattcggaactgaaatctaaactgaagaaccgccacgcctttaagatggccgtactatttaaacagattctgtcggaccgggagaaatctttcgtgatcgatgagtttgaatcagacgcccaggttatcgacgctgtaaagaatttctatgcagagcagtgtaaagataataacgtcatcttcaacctgttaaacctgataaagaacatcgctttcctttctgatgatgaactggatggtatatttattgagggcaaatacctttcttccgtatcacagaagctgtattctgactggagtaaattaagaaacgatatcgaagattcagccaatagcaagcaaggaaacaaggagttagcgaaaaagatcaagaccaacaaaggcgatgtagagaaagctatcagtaagtatgaatttagcttgagcgaacttaattcaattgtacatgacaacactaaatttagtgatctgttatcctgcaccctgcataaagttgcgtcagagaagctggttaaggtgaatgagggcgactggccgaaacatctaaagaacaatgaagagaaacagaagattaaggaaccacttgacgcactgctggaaatttacaacactctgttaatatttaattgtaaatcattcaacaagaacggcaatttctacgtcgactacgatagatgcattaacgaattatcatcagtggtctacctctacaacaagactcgtaactattgtactaagaagccgtataatactgataaatttaaactgaatttcaatagtccacagctgggcgaaggctttagtaaatcgaaagagaacgactgtctgactctgctgttcaagaaggatgacaactactacgtcggcattattcgtaaaggtgctaagattaacttcgatgatacccaggcgatagcggacaacacggataattgtatatttaagatgaattacttcctgctgaaagatgccaagaaatttattccgaaatgctcaatccagctcaaggaagtcaaggcacacttcaagaagtcagaagatgattacatactttcggataaagagaaatttgccagtcctctggtgattaagaaaagcacgttcttattagccaccgcccacgttaaaggcaagaaaggcaatataaagaagttccagaaagagtatagtaaagagaacccgaccgaatatagaaactcgcttaacgaatggatcgcgttctgcaaagagttcttgaagacatacaaggcggcaaccatcttcgatattacgacgctaaagaaagcagaagagtacgctgatatcgtggagttctataaagacgtcgataacctgtgctacaaattagaattctgtccaatcaagacgtcatttatagagaatctgattgataacggtgatttatacctatttcgcatcaataacaaagacttctcgagcaagagcaccgggactaagaaccttcatacactctacttgcaagcaatattcgacgagcgcaacctgaacaatccgacaattatgcttaatggtggtgctgaactcttctatcgtaaagaatctatcgagcagaagaaccgcatcacgcacaaagctggaagtattctggtaaataaagtgtgcaaggatggtacatcattagatgataagatccgtaatgaaatctaccagtacgagaacaaattcatcgacacgctgtcagatgaagcgaagaaagtgcttcccaatgtcattaagaaagaagcaacccacgatatcactaaagataaacgatttactagcgacaaattcttctttcactgccctctgaccataaactataaagaaggcgacactaaacaattcaataacgaagtgctgagcttcctgagggggaatccggatattaatattattgggatcgatcgaggggagcgcaaccttatctacgtcactgtcattaaccagaaaggtgagattcttgattcagtttcgttcaatacggttaccaacaagagctctaagattgaacagaccgtagattacgaagagaagctggctgtgcgggagaaagagcgtatcgaagccaagcgcagctgggattctatttccaagattgcgacgctgaaagaaggatatctgagcgcgatcgtgcatgaaatttgtctgcttatgatcaaacataatgctatcgtcgtacttgagaatctgaatgcagggtttaaacgcatccgcggtggtttgagtgagaagtctgtgtatcagaagtttgaaaagatgttaattaataaactaaactacttcgtgagtaagaaagaatcggattggaataagccgtcagggttgctgaatggcctccagctttcagatcagttcgaatcctttgagaaactgggcattcagtcgggctttattttctatgttccagccgcatatacctctaagattgatcctacaaccggctttgcgaatgtgttgaatctttcgaaggtgcgtaatgtggatgcgattaagtcgttcttctctaatttcaatgaaatttcttactcgaagaaagaagccctgtttaaattctcatttgatctggattcgctaagcaagaaaggcttctcaagctttgtgaagtttagtaagagtaaatggaatgtatacaccttcggtgaacgtatcattaagccaaagaataaacagggttatcgagaagataaacgcattaatctcacgttcgaaatgaagaagctgttgaacgagtacaaggtgtctttcgatctcgagaataatctgattcctaacttaacgagcgccaacttgaaggatacgttctggaaggaactgttcttcatctttaagaccactttacaactccgcaactctgtgacgaatggcaaagaggatgttctgattagccctgtcaagaatgcgaaaggtgaattcttcgtctcaggcacccacaataagaccttgccgcaagactgcgatgccaatggtgcgtatcacattgcgttgaagggactaatgattctggaacggaataacctggtacgggaggagaaagacacgaagaagatcatggcgatctcgaatgtggactggttcgaatacgtgcagaagcgccgtggcgtcctgtaa

SEQ ID NO: 299 - DNA, 4005 bp, Artificial Sequence
  Description of Artificial Sequence: Synthetic polynucleotide
atgtccagtttaaccaaatttaccaataaatattcgaagcaactgacaatcaagaacgagcttattccggtggggaagacccttgagaacatcaaagagaatggtctgatcgacggcgatgagcaactgaatgagaattatcagaaagcgaagataattgtggacgacttcttacgcgactttatcaataaagccttaaataacacccaaatcggtaactggcgtgaattggcagatgctttaaacaaagaggacgaagacaacattgagaaattacaggataagattcgtggtattattgtctccaagttcgaaacattcgacttatttagctcctattctataaagaaagacgaaaagataattgacgatgataacgatgtggaagaggaagaacttgatctggggaagaaaacatcttcattcaagtatatattcaagaagaacttgttcaaactggtgctcccaagctacctaaagaccaccaatcaggataaattaaagattatcagttccttcgacaacttctcaacatactttcgtggattctttgagaatcgcaagaacatattcactaagaaacccattagcacctctattgcgtatcgcatcgttcatgataacttcccgaaattcctggataacatcagatgcttcaatgtgtggcagactgaatgtccacagctgattgtcaaagcagataattacctaaagtctaagaacgttattgcgaaggataagagtctggccaactacttcacggtaggtgcgtatgattatttccttagccagaatgggattgatttctataataacattattggtgggttgccggcgtttgcaggtcatgagaagatacaaggcctcaacgaatttatcaaccaagaatgtcagaaggacagtgagctgaagtctaaactcaagaaccgtcatgcattcaagatggcggtgctgtttaaacaaatcctgtcggatagggagaagtcgtttgtaatagacgaatttgagtctgatgcgcaagtcatcgatgctgttaagaacttctacgcagaacaatgcaaagataataatgtcatattcaacctgttgaacctcataaagaacatcgccttcctgagtgacgatgagctggacggtatattcattgaggggaagtacctatcttccgtttcacagaaactctatagtgactggagtaagttgagaaacgacattgaggattcggcgaacagcaaacaaggcaacaaagagctggcaaagaagattaagaccaacaaaggagacgttgagaaagccatcagcaaatatgaattcagcctgagcgagttgaactcgattgtccacgataatactaagttctcagatctcttgtcttgtaccctccacaaagtagcctcagagaagttggtcaaggtcaacgaaggagattggccgaaacacctcaagaacaatgaagagaaacaaaagattaaggaaccattagatgcgctgctggaaatatacaataccttattaatctttaactgcaagtcatttaataagaatggtaatttctatgttgattacgatcgctgcattaacgaactgagctctgtagtttacttgtacaacaagactcgcaattactgcacgaagaaaccgtataataccgacaaattcaagctgaacttcaatagcccgcagctgggagaagggtttagcaaatctaaagagaacgattgtctaacgttgctgtttaagaaagatgacaactattatgtgggcattattcgtaaaggtgctaagataaactttgatgatacccaggctattgcagataacaccgataactgtatattcaagatgaactacttcctattgaaagacgcaaagaaattcatcccgaaatgctccatccagcttaaagaagttaaagcgcactttaagaagtcagaagatgattacatcctgtcagataaagagaagtttgcgagcccactggtaataaagaaaagtacctttctgctggcgacagcccatgttaagggcaagaagggtaatattaagaaatttcagaaagaatatagcaaagagaacccgacagaatatcgtaattcgctgaacgaatggatcgccttctgtaaagagttcttaaagacatataaagccgcgacgatctttgatattaccaccctcaagaaagcagaggaatatgcagacattgttgagttctataaggacgttgacaacttatgttacaaactggaattctgtcctattaagacttcctttatcgagaacctgattgataatggtgacctgtacttgtttcgaattaacaacaaagatttcagcagcaaatcgaccgggaccaagaacctacatacactctatttgcaggcaatattcgatgagcgtaacctcaataaccctaccattatgctgaacggcggcgcagagctattctaccgtaaagaatctatcgagcagaagaatcgcatcacccataaagcaggttcgatcctggtgaataaagtatgcaaggacggcacctccctcgacgacaagattcgcaacgaaatctatcaatatgagaataagtttatcgacacgctgtcggatgaagcgaagaaggtactgccgaatgtgataaagaaagaagcgacccatgacattactaaggataaacgcttcacgtctgataagttcttctttcactgcccgttgacgattaattataaagagggtgataccaagcaattcaacaatgaagtgctgagcttcttacgcggtaatccagatatcaatattattggcatcgatcgtggtgaacgtaacctgatttacgtgacagtaattaaccagaaaggagagatcctggatagtgtgagctttaatactgtaacgaacaaatctagcaagatagagcaaaccgtggactatgaagagaaactggcggtgcgtgagaaagaacgcattgaagccaagcgaagctgggattcgatttcaaagattgccacccttaaggagggctacttaagtgccattgtccacgaaatttgtctcctgatgatcaagcacaatgcaatagttgtattggagaatctcaatgctggctttaaacgtattagaggtggattgtcagagaagtcagtgtatcagaagttcgagaagatgctgattaataaactgaactacttcgtttcgaagaaggaaagcgattggaacaaaccgagcggcttactgaacggcctgcaattaagtgatcagtttgaatctttcgagaaactgggcatacagagtggctttatcttctacgttcctgctgcgtacacctccaagattgaccctacaaccggcttcgcaaatgttcttaatctgagcaaagtgcgtaatgtcgatgctattaaatccttcttcagcaacttcaacgaaatttcttattcgaagaaagaggctttgttcaaattctcgtttgacctggattctctcagcaagaaaggtttctcttctttcgttaaattcagcaagagcaaatggaacgtctatacattcggagaacgtattattaaacccaagaataagcagggttatagggaagacaaacgcattaatctgactttcgagatgaagaaactgctgaatgaatataaggtatcctttgatctggagaacaacctaatcccaaatctgacctccgcaaacctgaaagatacgttctggaaagaattattctttatatttaagaccacactgcagttgcgtaacagcgtaacgaatgggaaggaggacgtactcatatcaccggtcaagaacgcgaaaggcgagttctttgtaagcggcacccataacaagacgcttccgcaggattgtgacgccaacggcgcataccacatcgcactgaaaggccttatgattcttgaacggaacaacctcgtgcgcgaagagaaagatacgaagaaaattatggcgatctcaaacgttgactggtttgaatacgttcagaaacgtagaggtgtgctctga

SEQ ID NO: 300 - DNA, 4005 bp, Artificial Sequence
  Description of Artificial Sequence: Synthetic polynucleotide
atgagttccctaaccaagtttacaaataaatactcgaaacagctgacgattaagaatgaacttattccagtgggaaagaccctagagaatattaaggagaacggcctgatcgacggtgacgaacagcttaatgagaactaccagaaagctaagattatcgtagatgacttcctgcgtgactttattaataaagcgttaaataacacacagattggtaattggcgcgaactggccgatgctttgaataaagaagatgaagataatatcgagaaactccaggataagattcgtggcattattgtgagcaagttcgaaacgtttgatctgttctccagttattccatcaagaaagatgagaaaatcattgacgacgacaatgacgtggaggaagaagaattagatctgggtaagaagacaagttcgtttaagtacatatttaagaagaacctcttcaaactcgtgttaccgtcctatcttaagacgaccaatcaagacaaactcaagatcattagcagtttcgacaactttagcacctatttcagaggtttcttcgagaaccgaaagaatatcttcaccaagaaaccgatcagtacctccatcgcatatcgtattgtccatgataactttcccaagtttctggacaacattcgctgcttcaacgtctggcagactgaatgtccacaactgatagtcaaagcggacaactacctgaaatcaaagaacgtaatcgcgaaagacaagagcctagccaattactttaccgtcggtgcctatgactacttcttatcacagaatggtattgatttctataacaacattattggcggactgcctgcctttgccggtcatgagaagattcagggtttaaacgaattcatcaaccaggagtgccagaaggactcggaattaaagagtaagctgaagaatagacatgcattcaagatggcggtgttattcaagcagatactcagtgaccgtgagaaatctttcgttattgatgaatttgaaagtgacgcgcaggtaattgacgctgtcaagaatttctacgccgaacagtgcaaagacaacaacgtgatattcaatctgttaaacctgatcaagaatatcgcgtttctttcggatgacgaactggacggcatcttcatcgaaggaaagtacctgtcatccgtctcgcagaagttatactcagattggtcgaaattacgcaacgacattgaggactcggctaattccaaacaaggtaacaaagaactggctaagaaaatcaagaccaataaaggagacgtggagaaagcgatcagcaaatatgagttctcactgagtgaattaaacagtattgtacatgacaataccaaattcagtgatctgctgagttgcaccttacacaaagtcgcctccgagaagcttgtgaaggtcaatgagggcgactggcccaagcaccttaagaacaatgaggagaaacaaaagattaaagaaccattagatgctctactcgaaatctataataccctgctgatcttcaattgtaagagctttaataagaacggcaacttctatgtggactatgatcgctgcatcaacgagctgtcctctgtggtatatctgtataacaagacccgcaactattgtacgaagaagccatataacaccgataaattcaaactgaactttaactctccacagctgggtgagggattcagcaagtccaaggagaacgactgcctaaccttgttgttcaagaaagacgacaactactacgtgggcattattcggaaaggagccaagattaactttgacgatacgcaagcgatagccgataatacagataactgtatcttcaagatgaactatttcctgcttaaagatgcaaagaaatttatccctaaatgtagtatccaactgaaagaggtgaaagcccactttaagaagtctgaggatgactatatcctgtcagacaaagagaagtttgcttcaccgctcgtgataaagaaatcaacgttcctattggccactgcgcacgttaaagggaagaaaggtaatatcaagaagtttcagaaggagtatagcaaggagaatccgaccgagtaccgtaattctctgaacgaatggattgctttctgcaaagagtttttaaagacctataaagctgcaactatctttgacataacaacactcaagaaggccgaggaatatgccgatattgtggagttctacaaagatgtagacaacctttgctataagctcgaattctgcccgataaagacctccttcatcgagaacttgattgacaacggtgatctgtatttgtttcgcattaataataaagatttcagcagcaagtcaaccggtacaaagaatctgcacacactgtatttgcaagcgatctttgatgaacggaacctgaacaacccaacgataatgctgaatggtggcgccgaacttttctacaggaaggaatcgatcgaacaaaagaatcgaattactcataaagcaggtagtatcttggtgaataaagtctgcaaagacggcacctcgctggacgacaagatccgcaatgaaatatatcagtatgagaataagttcattgacacattgtcagacgaagccaagaaagtcttacccaacgtgataaagaaagaggccacacatgatattaccaaagataagagatttacgtctgacaagttcttctttcactgccctttgacgattaactataaagagggtgatacgaagcagttcaataacgaagtgctcagcttcctgcgtggcaatcccgacataaatattattggcatagatcgtggtgaacgcaatctgatctatgtgactgtcataaatcagaagggtgagatccttgattcagtttccttcaataccgttaccaataaatccagtaagattgaacagacggtcgactatgaagagaagctggccgttcgcgagaaagagcgcattgaagccaaacgttcgtgggattcaatctcgaagattgctactctcaaagagggttatctgtctgcaatcgtccacgaaatttgcctgctgatgatcaaacacaacgctattgtggtgctggagaacttaaatgctggtttcaagcgcattagaggaggtctgtctgagaagtcagtttaccagaagtttgagaagatgctgattaataagttgaactactttgtgtcaaagaaggaaagtgactggaataaaccttcaggcctactgaatggattgcagttaagtgaccagtttgaatcgtttgagaagttgggaattcagtccggcttcatattctatgttcctgcagcatacacgagtaagattgacccgactaccgggtttgccaacgtactcaacctgtctaaagtacgtaacgtcgacgcgatcaaatcattcttctcaaacttcaacgaaatttcctactccaagaaagaggcattatttaaattctcgttcgatctagattcactttctaagaaagggttctcctcctttgtgaagttctcaaagtctaagtggaatgtgtataccttcggtgagcgcataattaaacctaagaacaagcagggataccgcgaagacaaacgtattaacctgacattcgaaatgaagaagctgttaaatgagtacaaagttagctttgacttggagaacaacctgattccgaatttaacaagcgccaatctgaaagatactttctggaaagaactattcttcatctttaagactacgctgcaactgagaaactctgtaacgaatggcaaagaggacgtgctgatttcaccggtcaagaatgcgaagggagaattcttcgtctcaggcacgcacaataagaccctcccgcaggattgcgatgcgaatggtgcctatcatattgcactgaaaggtctgatgatccttgagaggaataacttggtgcgagaagagaaggatactaagaaaattatggccatatctaatgtcgattggttcgagtacgttcagaagcggcgtggtgtgttgtaa

SEQ ID NO: 301 - DNA, 4005 bp, Artificial Sequence
  Description of Artificial Sequence: Synthetic polynucleotide
atgagtagcctcaccaagtttactaacaaatactcgaaacaactgaccataaagaatgaacttatacccgttggcaagactctggagaatattaaagagaacggcctgattgatggcgacgaacaattaaatgagaattatcagaaggccaagattattgttgatgacttcctgcgcgactttatcaacaaagctctcaacaacacacagatcgggaattggcgtgaactagcggatgctttgaacaaagaagatgaagataatatagagaaactgcaagataagattcgcgggattattgtctcgaagtttgagacatttgacctgtttagctcatactctataaagaaggatgagaagatcattgacgacgataatgatgtggaggaggaagaactggaccttggaaagaaaacttcatcgtttaaatacatattcaagaagaacctgtttaaattagtcctgccgtcctacctgaagaccaccaaccaggataagctgaagatcattagcagcttcgacaacttctcgacatacttccgcggcttcttcgagaacagaaagaacatatttacaaagaagccgatctcgacgtcgattgcgtatcgcatcgtacacgataactttccgaaatttctggacaatattcgttgctttaatgtctggcagacggagtgccctcagttgattgtcaaggccgataattatctcaagtctaagaacgtgattgctaaggacaagagcctggccaactacttcaccgtgggcgcgtatgattatttcttatcacagaacggcatcgatttctataataatataattggaggtttacctgcatttgccgggcacgagaagattcaaggcctgaacgaatttataaatcaagaatgtcagaaagattccgagctgaagagcaagcttaagaaccgtcatgcgttcaagatggccgtgctgtttaaacaaatcctgagcgatcgtgaaaagagtttcgttatcgatgaatttgagtctgatgcgcaggtaatcgatgcggtgaagaatttctatgcggaacaatgtaaagacaataacgttatcttcaatctgttgaacctgataaagaatatcgcgttcctgagtgatgatgaattagatggtatctttatcgagggtaaatacctgagttcagtcagccagaaactgtacagtgattggagcaaacttcgtaatgatattgaagattctgcgaattccaaacaaggaaataaggaactggctaagaagatcaagacaaacaagggcgatgttgagaaagccatcagcaaatatgagtttagcctgtcggaattgaactcaattgtgcacgacaacacgaagttctcagatctgttgtcttgtactttacacaaagtggcctctgagaagctggttaaagtaaacgaaggagactggccaaagcacctaaagaacaacgaagagaaacagaagattaaagagcccttggacgccctgcttgaaatctacaacacactactgatatttaactgtaaatccttcaacaagaatgggaatttctatgtggattacgatcgctgcattaatgaattatcgtcggtagtgtacctctacaacaagacgagaaactattgtacaaagaaaccgtataacaccgataaatttaaactgaactttaacagtccgcagcttggagaaggcttctcgaaatctaaagagaacgactgtctgactttactcttcaagaaagacgataattattacgttggcatcatccgcaagggcgctaagattaatttcgacgatacacaagccatcgcggataacacggataactgtatcttcaagatgaattacttcttgcttaaagatgccaagaagtttattcccaagtgtagcatacaattgaaagaggttaaggctcactttaagaaaagtgaagatgactatattctgagcgacaaagagaagttcgcatcgccgcttgtgatcaagaaatcaacattcttactcgcaactgcgcacgttaaaggtaagaaaggtaacatcaagaaatttcagaaagagtatagtaaagagaatcctactgaatatcgcaatagcttaaatgaatggatcgccttctgtaaagaatttctaaagacttataaagctgcgacgatcttcgatataacgacgctaaagaaagcggaagagtatgcagatatcgtcgagttctataaagatgttgataacctgtgctataaactcgagttctgtcccatcaagacatcgtttatagagaatctgatagacaatggcgatttgtatctgttccgcataaataataaggatttctcttctaaatcaaccggtactaagaatctgcacaccctttatctgcaagcgatattcgacgaacgcaatctgaacaatccaaccatcatgctcaacggcggcgcagagctcttctatcgtaaggaaagtattgaacaaaagaatcgcatcacgcacaaagcagggagtatactggttaacaaagtttgcaaggatggcaccagtttggatgacaagattaggaacgaaatttaccaatatgagaacaaattcatcgatacgctcagcgatgaagcgaagaaagtgttacccaatgtcataaagaaagaagctactcatgatatcaccaaagataaacgtttcactagtgacaagttcttcttccactgcccattaacgattaactataaagagggcgatactaaacaatttaataatgaagttctgagtttcttacgcggtaacccggatattaacattattgggatcgatcgtggtgagcgcaacctgatctatgtaacggtgattaaccagaaaggtgaaattcttgatagcgttagctttaataccgtcacaaacaagagctcgaagattgagcagacagtagattacgaagagaaactcgcggttcgagagaaagaacggatcgaagccaagcgctcttgggattctatttcgaagatagctactctgaaagaaggttatcttagcgctattgtgcacgaaatttgtctgctcatgattaagcacaacgcgattgtcgtgttggagaacctgaacgcgggattcaagcgtatccgtggcggtctgagcgagaagagtgtttatcagaagtttgagaagatgttgatcaataaactgaattactttgttagcaagaaagaatccgattggaacaaacccagcggtctgttaaacggccttcagttgtctgaccagttcgaatccttcgagaagcttggcatccaaagcggctttatattttatgtccctgcggcctatacatccaagattgatccaaccaccggtttcgccaatgtacttaacctgtctaaggtcaggaacgttgatgcaattaaatcattcttttcgaacttcaacgaaatttcgtatagtaagaaggaagcactcttcaaattttcattcgatctggatagcctttcgaagaaagggttcagtagctttgtcaagttctctaagtctaaatggaatgtgtataccttcggcgaacgcatcattaaaccaaagaataaacaaggctaccgcgaagacaagcggattaacttgaccttcgaaatgaagaaactgctgaacgagtacaaggtatccttcgacctggagaacaatctgattcctaatctgaccagcgctaaccttaaggatacattctggaaagaactgttcttcatctttaagaccacgctgcagttacggaattcagtcactaacgggaaagaagatgttctaattagcccggttaagaatgcgaagggtgaattcttcgttagcggtactcataacaagaccctcccacaggactgtgatgccaacggtgcgtaccacatcgcgttgaaaggactgatgattctggaacgtaacaatcttgtgcgtgaggagaaggacacgaagaaaatcatggcgatttcgaacgtggactggttcgagtacgtacagaagcgtcgtggtgtgctttga

SEQ ID NO: 302 - DNA, 4005 bp, Artificial Sequence
  Description of Artificial Sequence: Synthetic polynucleotide
atgagcagtctgaccaaatttactaataagtattcgaaacaacttacaatcaagaatgaacttatccctgtagggaagaccctggagaacatcaaagagaatggcctaattgatggtgatgagcagttgaacgagaactaccagaaagcaaagatcatcgtggatgacttcttacgtgactttatcaataaagccctgaataatactcaaattggcaattggcgtgagctagcggatgcacttaataaagaggacgaagataacattgagaagttacaggacaagatccgcggcattattgtatcgaaattcgagacctttgacctattctctagctatagcataaagaaggacgagaagattatcgatgacgacaatgacgtggaagaagaggagctggatctgggtaagaagacaagctcatttaaatacatcttcaagaagaacctgtttaaacttgtcctaccgtcttatctgaagactactaaccaagacaagcttaagattattagctcatttgataatttctcgacttactttcgcggcttcttcgagaataggaagaatatctttacaaagaaaccaatctcgacctcgatagcataccgcatcgttcacgacaactttcccaaatttctggacaatattcggtgcttcaacgtttggcaaaccgaatgtccgcaacttattgtgaaggccgacaactacttgaagagtaagaacgtgattgcgaaagacaagagtctggcgaactatttcacagtcggcgcctatgattacttcctttcgcagaatggcatcgacttctataacaatattattggcggcctgccagcctttgccggccacgagaagattcagggcctgaacgaatttatcaaccaagaatgccagaaagactcagaacttaaatcaaagctgaagaaccgccatgcattcaagatggctgtcttgtttaaacagatcttatctgacagggagaagagctttgtaatcgatgaattcgagagcgatgcgcaggtgatcgatgctgtgaagaatttctatgccgaacagtgtaaagacaacaacgtaatatttaacctcttaaatctaataaagaatatcgcattcttgagtgacgacgaactggatggtatcttcatcgagggtaaatatctatcatcagtgagccagaaattgtattccgactggagcaaattacgtaatgatatcgaggactctgcgaactctaaacaaggaaacaaagaactggcgaaaaagatcaagaccaacaagggtgatgtggagaaggctatcagtaaatatgagttctcgttatctgaactcaatagcattgtacatgataacactaagtttagcgaccttctttcttgtactctgcataaagtggcttctgagaagctggttaaagtaaatgaaggtgattggccgaaacatctgaagaacaacgaagagaagcagaagattaaggaaccactcgacgcgttactggaaatttataatactctcctgatatttaattgtaagtcatttaataagaatgggaatttctatgtggattatgatcgctgtattaatgaactgtccagcgtcgtatatctttataacaagacccgaaattattgtactaagaaaccgtacaacactgataaatttaaactgaacttcaatagcccacaactgggtgaaggtttctctaagagcaaagagaatgactgtctgactctcctgttcaagaaagacgacaattactacgtgggcattattcgaaagggtgcaaagatcaactttgacgatacccaagccatcgcagacaatacagacaattgcatctttaagatgaattacttcctgttgaaagacgccaagaaatttattcccaagtgctcaattcagcttaaagaagtgaaagcacacttcaagaaatcagaagatgattatattctgtcggataaagagaagttcgcatctcctctggtaattaaaaagagtacgtttctcctagctaccgctcatgttaaaggaaagaaaggcaacataaagaaattccagaaagaatactctaaggagaatccaactgaataccgtaactctttaaatgaatggattgctttctgcaaagaatttttaaagacctataaagcggcgactatcttcgatatcactaccttaaagaaggccgaagaatacgccgatattgtcgagttctacaaagatgtggacaacctctgctacaagctcgagttctgcccgatcaagacgtcgttcattgagaatctgattgacaacggcgatctgtatttatttcgcattaacaataaggacttctctagcaaatcgacaggaacgaagaatctgcacaccttgtatctgcaagcgatcttcgatgaacgtaacttgaataacccaaccatcatgttaaacggcggtgccgaattattctatcggaaagaatcgatcgagcagaagaaccgcatcacgcacaaagctggctctattcttgtcaacaaggtgtgtaaagatggcacatcgctcgatgataagatacgcaacgagatctaccagtacgagaacaagttcattgacacgttgagtgatgaagctaagaaagtattaccaaatgttataaagaaagaggctacgcacgatattaccaaggataaacgcttcacttcggacaaatttttctttcattgcccgttaaccattaattataaagagggcgataccaaacagttcaataatgaagttctatcattcttacgaggcaatccggacatcaatattataggtatcgatagaggcgaaaggaatttgatctatgtgacagttatcaaccagaagggagaaatcttagatagcgtaagtttcaataccgtgacaaacaaatcgagtaagattgaacaaaccgttgactacgaagagaagctggcggtccgtgagaaggaacgaatcgaggccaagcgcagctgggatagtattagtaagattgcgactttgaaggaaggatatctgtcggcaatcgttcacgaaatctgcctcctgatgatcaaacataatgctattgtggtgctggagaatttgaatgcaggcttcaaacgaatccgcggcggtctgtcagagaagtctgtgtaccagaaatttgagaagatgctgatcaacaagctgaactacttcgtctcgaagaaggaaagtgattggaataaaccgtcgggattattaaacggtctgcagttgtcagatcagtttgaaagtttcgagaagctgggcatccaatcaggcttcatattttatgtgccagcggcttacacctcaaagattgatccgaccacgggtttcgccaacgttcttaatctttccaaggtgcggaatgtcgatgcaattaaatctttcttcagcaacttcaatgaaatctcatattccaagaaagaggcgctgtttaaatttagtttcgatctggatagtttaagtaagaagggcttctcgtccttcgttaaattctcgaaatccaaatggaatgtctacacctttggtgaacgtataataaagcccaagaacaagcagggttatcgtgaagacaaacgcattaatctgaccttcgagatgaagaagcttctcaacgaatacaaggtcagtttcgatttagagaataaccttattcccaacctgacgtcggctaacctgaaagatacgttctggaaagaacttttcttcatatttaagactacacttcagttacgcaatagcgtaacgaatggcaaagaagatgtactgattagtcccgtgaagaatgccaaaggcgagttctttgtttcgggtacccataacaagacgctcccgcaggattgcgatgctaacggtgcgtatcatattgcacttaaaggtctcatgatactcgaacgcaacaatttggtgcgtgaagagaaggatacgaagaagatcatggcaatcagcaatgtggactggttcgaatatgttcagaaacgtagaggtgtgctgtaa

SEQ ID NO: 303 - DNA, 4005 bp, Artificial Sequence
  Description of Artificial Sequence: Synthetic polynucleotide
atgtcctcactcacgaagttcactaataagtatagtaagcaactgaccattaagaatgaactcattcctgttggcaagacactggagaatatcaaggagaatggactcatcgacggagatgaacaactgaatgagaactatcagaaagcaaagatcatcgtggacgactttctcagggatttcattaacaaggctctaaacaatactcaaataggtaactggagagaacttgctgatgccttaaataaagaggatgaggataatattgagaaactccaggacaagatccggggtattatagtcagcaaatttgagacattcgatcttttctcttcttattcgattaagaaagatgagaaaatcattgatgatgacaacgacgttgaagaggaagagttggacctaggtaagaagacgagtagtttcaaatatatatttaagaagaacttatttaaacttgtccttccttcatatttgaagacgactaatcaggataagcttaagatcattagttccttcgacaacttctcaacttactttcgtggtttctttgagaatcggaagaacatcttcactaagaagcctattagcacctctattgcttatagaattgttcatgataatttcccaaagtttctcgataacatccgttgcttcaacgtatggcaaaccgaatgtcctcagctaattgttaaggccgataactatctgaagtcgaagaatgtaatcgctaaagataaatccttagctaactacttcactgtgggtgcatatgattatttcctttcacagaacggcattgacttctataacaatatcatcggtggactcccagcattcgcaggtcacgaaaagatacaaggtcttaatgaatttattaatcaggagtgtcagaaagatagcgaattaaagtccaagcttaagaacaggcacgcatttaagatggcggtgttgtttaagcagatcttatctgacagggagaaaagtttcgtcattgatgagtttgaaagtgacgcacaagtaattgatgccgtcaagaacttctatgcggaacaatgtaaggataataatgtcatctttaatttgcttaacttgatcaagaatattgccttcttatctgatgatgagcttgacggaatatttatagagggcaagtatttaagcagtgtttcccagaaactttattcagactggtctaagctccgaaatgatatcgaggactccgctaatagcaagcaaggtaataaagagctcgcaaagaagataaagacaaacaaaggagacgttgagaaggctatctccaaatacgaattcagcctttcagaactaaattctatagtgcacgacaacactaaattctcagatttgctatcatgtactctgcacaaagttgcatctgagaagcttgtcaaagtgaacgagggagattggccgaagcaccttaagaacaacgaagagaagcaaaagatcaaggagcccttagatgccctattggaaatttataatacattactaatattcaattgcaaatcatttaacaagaacggaaacttctacgttgactatgatcgatgtattaatgaactctcctctgtcgtatatttgtataataagacacggaactactgcacgaagaagccttacaatactgacaaatttaaactaaactttaacagcccgcaattaggcgaaggtttctctaagagtaaggagaatgactgtctcactttgctgttcaagaaggatgacaattactacgttggaatcattaggaaaggtgctaagatcaactttgatgatacgcaggccatagctgataatacggataattgcatattcaagatgaattacttccttcttaaggatgccaagaagttcattccaaagtgtagtatccaacttaaagaagttaaggctcactttaagaaatctgaagacgattatattctatcagataaggagaagtttgcatcaccactcgttattaagaaatcgacctttcttcttgcgactgctcatgtgaaaggtaagaaaggaaatataaagaagtttcagaaagaatacagtaaagagaatcctacagagtacaggaactctctcaacgagtggattgctttctgtaaagaattcctgaagacttataaagcagccacaatcttcgatattactacattaaagaaggctgaggagtatgctgacatcgttgaattctataaggatgtcgataatttatgttataaactcgaattctgccctataaagaccagcttcattgagaacttaattgataacggtgacctttacttattccgaattaataataaggacttctcatccaagtcgactggcacaaagaaccttcatactttgtaccttcaagccatatttgatgagcgtaatctaaacaaccctacaataatgttgaatgggggcgcagaactcttctataggaaggaatctatagaacagaagaatcgaatcactcacaaggccggcagcatccttgttaataaggtttgtaaggacggaacttctcttgacgataagataaggaacgagatctatcaatatgagaacaagtttatagacaccttgtccgacgaagcaaagaaggttctaccaaacgtcattaagaaagaggcaacgcatgatatcacgaaggataagagattcacttccgataaattcttcttccattgtcctttgactatcaattataaggaaggcgataccaaacagttcaataatgaggttctgagtttcttacgtggtaatcctgacataaacattattggaatcgatcgtggtgagaggaatctgatttacgttaccgttataaatcagaagggagaaatcctggactctgtatcattcaatacggtaacaaataagagcagtaagattgagcaaacggtcgattatgaggagaaactggctgtgagggagaaggagagaattgaagcaaagcgttcctgggactccatttccaagatagccactttgaaggaagggtacctcagtgcaatagtgcacgaaatttgcctccttatgattaaacataacgctatcgttgttctcgagaaccttaatgcgggatttaagagaatacgcggcggcctttccgagaagtcagtgtatcagaagtttgagaagatgttgatcaataagctgaattacttcgtatcaaagaaagagtctgactggaataaaccttctgggctactgaatggattacaattaagcgaccagtttgaaagcttcgagaaactgggtattcagtcaggcttcatattctatgtcccagctgcttatacatcgaagattgatccaaccacgggcttcgctaatgtgctcaatttatctaaggttcgtaacgtggacgccataaagagtttcttctctaacttcaacgaaatctcgtacagtaagaaggaagctttattcaaattctcgttcgatttagattctcttagcaagaagggcttctcatcatttgtgaaattctctaaatctaaatggaatgtatacacatttggagaaaggataatcaagcccaagaataagcaaggataccgagaggacaagagaattaatttgacattcgaaatgaagaagttgttgaacgaatacaaagtttcatttgacctcgagaacaatctcattcctaatcttacttcagctaatttgaaggatacattctggaaagaacttttctttatattcaagaccacactccaacttagaaattccgtgaccaatgggaaagaggacgtcttgataagccctgtgaagaacgcaaagggagaattctttgtttcaggtactcataataagacactgccacaagattgcgatgctaacggcgcttatcatatcgctttgaagggattaatgatcctcgagaggaataatttggtcagggaagagaaggatactaagaagatcatggccatttcgaatgttgactggtttgagtatgttcagaagcgtagaggagtattatga

SEQ ID NO: 304 - DNA, 4005 bp, Artificial Sequence
  Description of Artificial Sequence: Synthetic polynucleotide
atgtcaagccttaccaagtttactaacaaatactctaaacaactcaccatcaagaacgagctgattcctgtaggcaagacactagagaacatcaaagagaacggattgatcgatggagatgagcaactgaatgagaactaccagaaagccaagataatcgtcgacgacttccttagggactttattaataaggctctcaataacactcagattggaaattggcgcgagttagctgatgctttgaataaagaagacgaggacaatattgagaaactccaggacaagattcgaggtataatcgttagtaaatttgagacgttcgatttgttctcgtcttatagtatcaagaaggacgagaagattatcgatgacgacaacgacgtagaagaggaggaacttgaccttggtaagaagacctccagctttaaatatatcttcaagaagaacctattcaagttggtgttgcctagttatcttaagactacaaatcaagataaattaaagattatttcgtcgttcgataactttagtacctacttccgaggcttctttgagaaccgcaagaacatattcactaagaaaccaatctctacgtccattgcttataggattgttcatgataacttcccaaagttcttggataacattagatgtttcaatgtctggcaaacagagtgtccacaactgatcgttaaagctgacaattatttgaaatcaaagaatgtaattgctaaggataagtctctggccaactactttactgttggcgcctacgactatttcttgagccagaacggaattgatttctataacaacatcattggaggactgccggcgttcgctggtcatgagaagatacaaggactcaacgaatttattaatcaagaatgccagaaagattcagaacttaagtcgaagctcaagaacaggcatgcgttcaagatggctgtcttatttaaacaaatcctctcggaccgggaaaagagcttcgttatcgatgagtttgagtccgatgcgcaagtcatcgatgctgttaagaatttctacgctgagcaatgcaaagacaataacgtcatattcaacttattgaatctcatcaagaatattgcctttctctctgacgatgaattggatggtatattcattgaggggaagtacttgtcatctgtttcacagaagctatattctgactggagtaagttgagaaatgacatcgaagattcagctaactccaaacaagggaacaaagaacttgcaaagaagattaagacaaataaaggagatgttgagaaagcaatctctaagtatgaattctcgctttcagaactaaattctatcgtgcatgataatacgaaattcagcgatttgctatcctgtactcttcataaggtcgcatctgagaagttggtcaaagtcaatgagggtgactggccgaaacacctaaagaataatgaggagaagcagaagatcaaagaacctcttgacgctttacttgagatttacaatactctgctcatctttaactgcaagtctttcaataagaatggcaatttctatgtcgattatgatagatgcattaatgaactatcatccgtagtgtacctatataataagactagaaattattgcaccaagaaaccttacaatactgataagttcaaattgaacttcaactcaccacaacttggtgaaggttttagtaagtccaaggagaatgattgtttgacactattgtttaagaaggacgacaactactacgttggaatcatacgaaagggagcaaagatcaatttcgatgatacgcaggcaatagcagataatactgacaattgcatatttaagatgaactacttccttctcaaagacgcgaagaaatttattcccaagtgctctatacagcttaaggaggtaaaggcacactttaagaaatcagaggatgattatattctgtcagataaggagaaatttgcttcgccactggtgatcaaaaagagtacgttcctcctggctaccgctcatgtgaagggtaagaaaggaaacattaagaagtttcagaaagagtattctaaggagaatccgaccgagtacagaaattccctcaatgaatggatagctttctgcaaggagttcttgaagacctataaggcagccactatattcgatattacaactttaaagaaggcggaagaatacgctgatatcgttgaattctacaaagacgttgataacttatgctacaaattggagttctgtcctattaagacctcgttcattgagaacctaatagataatggagacctctacttgtttagaatcaacaacaaggatttctcatcgaaatccacaggcaccaagaatttgcatactctatatcttcaagctatcttcgatgaaagaaatcttaataacccaactataatgctcaacggcggtgctgaactcttctatcggaaggaatctattgaacagaagaaccgtatcacacacaaagctggctctattctcgtcaataaagtctgtaaagatggaacaagcctggatgataagataagaaatgaaatctaccagtacgagaacaagtttattgacacgctaagcgacgaggccaagaaagtgctccctaacgtgattaagaaagaggcgacccatgacattactaaggataagcgtttcacttccgacaagttcttctttcattgcccattgactattaattacaaagagggtgatacaaagcagtttaacaacgaagtactctcattcctcagagggaaccctgacattaacattatcggaatcgaccggggagaaagaaacctaatttacgtcactgttattaatcagaagggcgagattctagactctgtctctttcaatacggtaacaaataaatcctctaagatcgaacagactgttgattacgaagagaagcttgcggtgcgagagaaggagcgtatagaggcgaagagatcttgggatagtatcagtaagatcgcaacattgaaagaaggctatctctccgcaattgttcacgaaatttgtcttcttatgattaaacataatgccattgtcgtcttggagaaccttaatgctggattcaagagaatacgcgggggtctcagcgagaaatccgtatatcagaagtttgaaaagatgctcattaataagctgaactacttcgtgagtaagaaagagtctgattggaataaaccttctggtctgctgaacggcttacagctttccgatcaatttgaatccttcgagaagctcggtatccagagtggtttcatattctacgtgccggcggcctatacctctaagattgatccaacgactgggttcgcaaacgtacttaacttgagcaaagttagaaatgtcgatgcaattaaatctttcttctccaatttcaacgaaatttcttacagcaagaaggaagcgctcttcaaattctcattcgacttggactctcttagtaagaaaggtttctcgtcattcgttaaattctctaagagcaaatggaatgtatatactttcggtgaacgtattattaagccaaagaacaagcaaggttatcgtgaagataaacggatcaaccttacctttgaaatgaagaaattgttaaacgagtacaaagtttctttcgatttggagaacaatctgatacccaatttaacttccgctaacttgaaagatacgttctggaaggaattgttctttatcttcaagactacgcttcaattgaggaactctgttaccaacgggaaagaggacgtactaatatctccggtgaagaacgcaaagggtgaattctttgttagtgggacacataacaagaccctaccgcaggattgcgacgctaacggagcatatcatatcgcgctaaagggacttatgattcttgaaagaaataacttggtgagagaggagaaagacactaagaagattatggccatttctaacgttgattggttcgagtacgttcagaagcgccgcggagtactttaa

SEQ ID NO: 305 - DNA, 4005 bp, Artificial Sequence
  Description of Artificial Sequence: Synthetic polynucleotide
atgagttcactaactaagttcacaaacaagtactccaagcaactaacaattaagaacgaattaattccggtgggcaagacacttgagaatatcaaggagaatggtttaattgacggagacgaacaattgaatgagaactatcagaaagctaagatcattgtagatgacttcttaagagacttcattaataaagcactaaacaacactcaaatcggtaactggagagaattggctgatgctctgaacaaggaagacgaggacaatatcgagaagctacaagacaagattagaggtattattgtatctaagttcgaaaccttcgatctcttcagcagttattcaattaagaaggatgagaagatcattgatgatgataacgatgtggaggaagaagaattagacctcgggaagaagactagcagctttaaatacatattcaagaagaatttgttcaagctggtccttccgtcgtacctgaagactactaaccaggacaagttaaagatcatctcttcctttgataacttctcgacatatttccgtggtttctttgagaatcggaagaacatcttcacaaagaagcctatctcgacctctattgcttacaggatagttcacgataacttccctaagttcttagataacattcgttgcttcaatgtatggcaaacagagtgtccacaacttatagttaaggctgataattatttaaagtcgaagaacgtaatcgctaaagataaatctcttgctaactactttacggtaggtgcctacgattatttcctttcccagaatggtattgacttctataacaacattattggtggattgcctgcattcgctggacatgaaaagatccaaggtttgaatgagtttataaaccaggaatgtcagaaggattctgaacttaaatcgaaactcaagaatagacatgccttcaagatggctgtcctctttaagcagatcttgtcagaccgtgagaaaagcttcgttatcgacgaattcgaatctgatgctcaggttattgacgctgtcaagaacttctacgcagagcaatgcaaagacaataacgttatcttcaatctccttaatctgatcaagaatatagcattcctttccgatgatgagcttgatggaatcttcatagaaggtaagtacttgtcttcagtttctcagaaactttattcagattggtctaagttaaggaatgacatagaagacagtgctaactccaaacaaggaaacaaggagttagcgaagaagataaagacaaataaaggtgacgtggagaaagcaatatctaagtatgaattcagtcttagtgagttgaacagtatcgtgcacgacaacacaaagttctcagatctattaagttgcaccctgcataaggttgcttctgagaaattagttaaggtcaacgagggtgactggcctaagcatctaaagaacaatgaagagaagcagaagataaaggaacctttagacgctttacttgaaatttacaacacactccttatctttaactgtaaatccttcaacaagaatggtaatttctacgtggattatgatcgatgtattaatgaactctcttcagttgtatatctctataacaagacacgcaattactgcacgaagaagccctataacacagataagtttaagctgaacttcaattcacctcaactcggcgagggattcagtaagtctaaggagaacgattgtctcacactcctatttaagaaagatgacaattattatgtcggaataattcgtaagggcgccaagattaatttcgacgacactcaagctattgcagataacacggataattgtatcttcaagatgaactacttcctcctcaaagacgctaagaagtttatcccaaagtgttcaatacagctaaaggaagttaaggctcatttcaagaagtctgaggacgattatatccttagtgataaggagaaatttgcttctcctcttgtcattaagaagtctacatttcttcttgctacagctcatgtgaaaggtaagaaaggtaacattaagaagtttcagaaagagtatagtaaagagaacccaacggagtatagaaattccctgaacgaatggattgctttctgcaaagagttcctaaagacctacaaagccgcaacaatcttcgacattactacgctgaagaaagctgaagaatatgccgatatagtagagttctataaagatgttgataatctgtgttataagcttgagttctgtcctataaagactagcttcattgagaaccttatcgacaatggtgatttatatttgttcagaattaataacaaagatttctcttctaaatccactggaacaaagaatctgcacactctttatcttcaagcgatcttcgatgagagaaacttaaacaatccaactattatgctgaatggtggagccgagctattctacaggaaagagtcgatagagcagaagaacaggattacccataaggctggatcaatactggtaaacaaggtttgcaaagatggaactagcctggatgacaagatccgcaatgagatttatcaatacgagaacaaatttatagataccctctctgatgaggcgaagaaagtcttaccaaatgtcatcaagaaagaggctacccatgatattaccaaagacaagcgtttcacttcagataagttcttcttccattgtccactaacaatcaattataaagagggtgatacgaaacaatttaacaacgaggtcttgtctttcctgcgaggaaatccagatattaatattataggaattgatcgtggtgaacggaacttaatttacgtgacagtcataaatcagaaaggagagatattggacagtgtgtcattcaataccgtaacaaacaagagctcaaagatcgagcagacagtggactacgaagagaaacttgcagtgagagagaaagaaagaatcgaagctaagcgatcttgggattctatttcgaagatagcgacattgaaagagggatacctaagcgcaattgttcatgaaatatgtttattaatgattaagcataatgctattgtggtgttagagaatttgaatgctggttttaagagaatacgaggcggtcttagtgagaaatctgtttatcagaagtttgagaagatgcttattaacaagttgaactacttcgtttcaaagaaagaatctgattggaataaaccttccggacttcttaacggccttcagctgtctgatcaatttgagtcattcgagaaacttggtatccagtcagggtttatattctacgttccagctgcctacacgtcgaagatcgacccgaccaccggtttcgccaatgttcttaatctctcaaaggttcgtaatgtagatgctatcaaatcatttttctcaaatttcaacgaaatttcttattcgaagaaggaagctctctttaaatttagtttcgatttagactcgctctccaagaaaggtttctctagtttcgtcaagttctctaaatcgaagtggaacgtttatacattcggagaacgaattattaagcctaagaacaagcaaggctatagagaagataagaggattaatctcaccttcgagatgaagaagctcttgaacgaatataaagtctctttcgacctcgagaataatttaatccctaatttaacatcagctaatcttaaggatactttctggaaggagctattctttatattcaagacaacactgcagctcagaaattctgtgacaaatggaaaggaggacgtgcttatcagtccagtcaagaacgctaagggagagttctttgtgtctggcacacacaataagaccctgcctcaggattgcgatgcgaacggagcttatcatatcgcacttaaaggtctcatgatactcgaaagaaataatcttgttagggaagagaaagatacaaaaaagatcatggctatttctaacgtcgactggttcgaatacgttcagaagagaagaggagtgttatga

SEQ ID NO: 306 - DNA, 4005 bp, Artificial Sequence
  Description of Artificial Sequence: Synthetic polynucleotide
atgtcgtcactgacgaagtttactaacaagtactctaaacagctaacaattaagaacgaattaattcctgttggaaagacactcgagaatattaaggagaacggcctgattgacggcgatgaacagctcaatgagaattaccagaaggcgaagattatagtcgatgacttcctcagagatttcatcaataaagcattaaataacactcaaatcggcaactggagggagttggcagacgcacttaataaagaagatgaagataacatcgagaagctgcaggataagatacgtggtatcatcgtgtctaaatttgagacatttgatctattctcttcctacagcattaagaaagatgagaagattatagatgatgacaacgatgtggaagaggaggaactggaccttggtaaaaagacttctagcttcaagtatatctttaagaagaacttgttcaaattagtcttgccaagttatttgaagaccacaaaccaagataaactgaagataattagtagtttcgataactttagtacatactttagaggattcttcgagaataggaagaacatctttacgaagaagccaatctcaaccagcatcgcttatcggatcgttcatgacaactttcctaaattcttggacaatatcaggtgcttcaatgtttggcagacagagtgtcctcaactaattgtaaaggctgataactacctgaagtcaaagaacgttatcgctaaggataagtccctcgccaactacttcactgttggagcatacgattatttcttgtcacagaacggaatagacttctataacaacattatcggtggattaccagctttcgctggccatgaaaagattcagggattaaatgagtttattaatcaggagtgccagaaagacagtgagttgaaatctaaattgaagaacaggcatgcttttaagatggcagttctgttcaaacaaatcctttctgatcgtgagaaatcctttgtgattgacgaattcgaatctgacgcccaagtcatcgatgcagtcaagaatttctatgctgaacaatgtaaagataataacgtcatatttaaccttctgaacctcatcaagaatattgccttcttatcggatgatgagttagacgggatattcattgaagggaagtacctttcttccgttagtcagaagttgtattcggattggtccaagttgagaaacgatatcgaagacagtgctaattctaagcagggtaataaagagttggccaagaagatcaagactaacaaaggagatgtggagaaagcgatctcaaagtatgagtttagtctttcagagcttaattcaattgttcacgataataccaagttctcggacttattatcgtgtaccctccacaaagttgcttcggagaaactcgttaaagtaaacgaaggcgattggccgaaacatttaaagaataacgaagagaaacagaagattaaagagcctttggatgccctcctagaaatttataatacgctacttatattcaactgtaagagtttcaacaagaatggaaatttctacgttgactatgataggtgtataaacgagctatcttccgtggtttatttgtataacaagaccaggaattactgtactaagaaaccgtacaacaccgataaatttaagttgaacttcaattctcctcaattgggagagggtttctcaaagtctaaggagaacgactgtttgacattacttttcaagaaagatgataattattacgtaggaattatcagaaagggcgccaagattaatttcgacgacacacaggcaatcgctgataacaccgacaactgtatatttaagatgaactactttctcttgaaagatgcgaagaaatttatacctaagtgttccatacagttaaaggaggttaaggcacacttcaagaagagcgaggatgactatattctttcagataaggagaaatttgcttctcctctggtgatcaagaaatctactttcctcttagccacagcacacgtgaagggaaagaagggtaatatcaagaagtttcagaaggaatactccaaagagaatccaactgaataccgtaatagtctgaatgaatggattgcgttctgtaaagaattcctgaagacctacaaagccgctactatcttcgatatcacgactcttaagaaagctgaagaatacgctgatattgttgaattctataaagatgttgataacttgtgttacaaacttgagttctgtcccataaagacttccttcatcgagaaccttatagataacggagacctttatctctttagaatcaataataaggacttcagctctaaatctaccgggacgaagaacttgcatactctctatctacaagctatctttgacgaaagaaacctgaataatccgactataatgttgaatggaggcgctgagctattctacagaaaggagagcatagagcagaaaaatcggataactcataaagccggatcaatcttggttaataaggtttgcaaggatggtacatcattagatgataagatccgcaacgagatttaccagtatgagaacaaatttatcgatactttatcagacgaagctaagaaggtacttcctaatgtcataaagaaagaagccactcatgatatcaccaaggataagaggttcactagtgataaattcttctttcattgtccacttacaattaattataaggaaggagatactaagcaatttaacaacgaggtgctgagcttcttgcgtgggaatccagatatcaatattatagggatcgatcgaggagaacgtaaccttatttacgtgactgtcatcaaccagaagggagaaatcttagactcagtatcgtttaacactgttactaataaatcatctaagatcgaacagacagtggattatgaggagaagctcgcggtgagagagaaggagcggatagaggcgaagagatcttgggatagtatatcaaagatagctacactcaaggagggatatctatctgctattgtgcatgaaatctgtctactgatgattaaacataacgcaatagtcgtattagagaatcttaacgccggcttcaaacgtatccgtggtggtctttctgagaaatctgtatatcagaaattcgagaaaatgttaattaataaactaaactacttcgtctcgaagaaagagtcggattggaataagccatcgggactcctaaatggtttacagctttctgatcaattcgagtcattcgagaaattaggtatccaaagtgggttcatcttttacgttccggctgcttatacctctaagatcgatccgactacaggctttgccaatgttcttaatctctcgaaggtacggaatgtcgatgccatcaagtcattcttcagtaatttcaacgaaatttcatattcaaagaaggaggctttattcaagttttcattcgatctcgatagcttatccaagaagggtttctcaagcttcgttaaattctctaaatccaagtggaacgtgtacacattcggtgaacgtatcattaagcctaagaacaagcaaggatatagagaggataaacgtattaacttgacattcgaaatgaagaaacttctgaacgagtacaaggtatcatttgatcttgagaacaacttgatacctaatttgacatcagctaatctaaaggataccttctggaaagaactcttcttcatctttaagacaaccttgcagcttcgcaactccgtcacaaacggtaaagaagatgtacttatttctcctgttaagaacgcgaaaggcgaattctttgtgtcaggtactcataataagacactcccacaggattgtgatgctaacggtgcgtaccacattgcattgaaaggacttatgatccttgagcggaataaccttgtcagggaagagaaagatacaaaaaagattatggcaatctcaaatgtcgattggtttgaatatgttcagaagcgtcgcggagttctctaa

SEQ ID NO: 307 - DNA, 4005 bp, Artificial Sequence
  Description of Artificial Sequence: Synthetic polynucleotide
atgtcttctctgaccaagtttacgaataaatattccaaacaactcacaattaagaatgaattgatacccgtcgggaagacgctagagaacattaaagagaacggtcttattgacggtgatgagcaacttaatgagaattatcagaaagcgaagattattgtagatgatttcttacgtgatttcattaacaaggctcttaacaatactcaaattggtaattggcgggaacttgctgatgcactcaataaggaagacgaggataacatagagaagcttcaggataagattagaggaataattgtatcgaaatttgaaaccttcgacttgttctcaagttattccatcaagaaagatgagaagattattgacgacgataatgatgttgaggaagaagaattagacttggggaagaagacatcaagtttcaagtatatcttcaagaagaatctatttaagctcgtactgcccagctatttgaagaccactaaccaagataaacttaagatcatctcatcattcgataacttcagcacatatttccgcggattctttgagaataggaagaacatatttactaagaaacctattagcactagcatcgcataccgaatagttcacgataactttccgaagttccttgataatatcaggtgtttcaacgtgtggcaaacagaatgtcctcaattgatcgtcaaggctgataattatttaaagtcaaagaatgttatagccaaggataaatcccttgccaactactttactgttggtgcttacgactatttcctatcacagaatggtatcgatttctacaacaatataattggtggtctcccagcctttgcaggacacgagaagatccagggccttaatgagtttataaatcaagaatgtcagaaagatagcgaacttaagtctaagcttaagaatcgtcatgcatttaagatggctgtcttgtttaaacagattctatctgatcgagagaaatctttcgtcatcgacgagttcgaatcggacgcacaagttattgacgcagtgaagaacttctatgctgaacagtgtaaagataataatgtgatattcaacttgctgaacttgataaagaacattgccttcctttcagacgatgagcttgacgggatcttcatcgaaggtaagtacctatcgtccgtctctcagaagctttattcggattggagcaaactaaggaacgatattgaagattcagcgaatagtaagcagggtaataaggagctcgcaaagaagattaagacaaataaaggcgacgtagagaaggctatcagcaagtatgagttctccctttcagaattaaattccatcgtacatgataacaccaagttctcggatttattgtcttgtacacttcataaagttgcctccgagaaacttgtgaaggttaatgagggagattggcctaaacaccttaagaacaatgaagagaagcagaaaattaaagagccgctggacgcactgttagaaatctataatactctgttgatcttcaattgtaaatccttcaacaagaatggcaacttctacgtagattacgatcgttgtattaacgaactttcatctgtggtttacctatataacaagaccaggaattattgcacgaagaagccatacaatactgacaaatttaaacttaactttaatagccctcaactgggtgaaggtttcagcaagtccaaagagaatgattgtttgacgctcctattcaagaaagacgacaactactacgttggtatcataagaaagggtgcgaagataaacttcgacgatacccaggcaatcgcagacaacactgataattgtatcttcaagatgaattatttccttcttaaggacgccaagaaatttattccgaagtgctcaatccagttgaaagaagtgaaagcgcattttaagaagtctgaggatgattacatattgagtgacaaggagaagttcgctagtccactggtaattaagaagagcacatttctgctcgcgacagcccacgtcaaaggtaagaaaggtaatattaagaaattccagaaagaatacagcaaagagaatccaacagaataccggaacagccttaatgagtggatagctttctgcaaagagttcttgaagacttataaagcggctactatctttgacatcacaactctgaagaaggctgaggaatatgctgatattgttgagttctataaagacgtggataatttatgctataagttagagttctgtcctataaagacgtccttcatagagaatttgatagataatggcgatctgtatctgtttaggattaacaataaagacttctctagtaaatctactggaactaagaacctgcatacactttacctgcaggctatcttcgatgaacgtaatttgaacaaccctacaataatgcttaacggcggagccgaactcttctatcggaaggagtccatagaacagaagaaccggatcactcacaaagcgggttctattcttgtcaacaaggtttgtaaagatggtacttcgctcgacgataagatccgtaatgaaatctaccagtatgagaacaagtttattgacactttgagtgacgaggccaagaaggtgcttcctaatgtaattaagaaggaggctacacatgatattactaaggataagagattcaccagcgataagttcttcttccattgtccgttgaccatcaattataaagaaggagataccaagcagttcaataatgaggttctatctttcttgagaggaaatccggatattaacattatcgggatcgatcgaggtgagcgtaatctaatttacgttacagtcattaaccagaaaggcgagatcctagatagtgtatctttcaacaccgttaccaataaatcttcaaagattgagcaaactgttgactacgaggagaaactggcagtgcgggagaaggagaggatcgaagccaagaggagctgggactcgatatcaaagattgctactcttaaggagggttatttgtccgctatcgtgcacgaaatatgcctccttatgattaaacacaatgctattgttgtgttagagaacctcaacgctggatttaagagaatcagagggggattatcggagaagagtgtgtaccagaaattcgagaaaatgcttataaataagcttaactactttgtaagtaagaaagaaagtgattggaataaaccaagtggtctcctaaacggtcttcagctctctgatcaatttgagtcatttgagaagttgggtatccaaagcggattcatcttctatgtaccagccgcgtacacgtccaagattgatcctactaccggtttcgccaacgtattgaatctgagcaaggttagaaatgttgacgcgataaagagtttcttcagtaatttcaatgaaatctcctacagcaagaaagaagcgctattcaaattctccttcgatctcgatagtctatctaagaaaggattctctagtttcgtaaagtttagtaaatctaagtggaacgtctacaccttcggtgagaggattatcaaaccgaagaacaaacagggctatagagaggacaagagaattaacttgaccttcgaaatgaagaagttacttaacgaatataaagtaagtttcgatttagagaataatcttattcctaatctgacttcagcgaacctcaaggataccttctggaaggaactattcttcatattcaagacaacgttacaacttagaaactcggttacaaacggtaaggaagacgttctcatttctcctgttaagaacgctaaaggtgaattctttgtttccggcacgcataataagaccctccctcaagattgtgacgctaatggtgcatatcacatcgctcttaaaggtttgatgatccttgagaggaacaatctagtgagggaagagaaggatacgaagaaaattatggctatttctaacgtcgattggttcgaatatgttcagaaacgaagaggtgtcctttga

SEQ ID NO: 308 - DNA, 4005 bp, Artificial Sequence
  Description of Artificial Sequence: Synthetic polynucleotide
atgtcttcgcttacgaagttcactaataagtattccaaacagttgacaataaagaacgagctcatcccagtcggcaagacactagagaatattaaggagaatggattaattgatggtgacgaacaactcaatgagaactaccagaaggccaagattattgtggatgatttcctgagggacttcattaataaggctctcaataacacgcaaattggaaattggagagagctcgcggatgcgttaaataaggaggacgaggacaatattgagaagctgcaagataagatccgaggcataattgttagcaagtttgagaccttcgatctgttttcatcgtacagtattaagaaagacgagaagattatagatgatgataacgatgtcgaagaggaggagctggatctcggaaagaaaacctcttccttcaaatacatattcaagaagaatctattcaaactggtcctaccctcatatcttaagactacaaatcaagacaagttgaagattatttcgtcgttcgacaatttctctacgtacttcagaggcttcttcgagaatcgaaagaacatattcacgaagaagccaatctctacctcaatcgcttatcgaattgtgcacgataactttccgaaattcttggacaacatccgctgtttcaacgtatggcagacagaatgtccacagcttattgtgaaggccgataactacttaaagagcaagaacgtgattgccaaggataaatcactcgcaaactactttactgtaggtgcttatgattactttctttctcagaacggcattgacttctacaataatatcattggtggattgcctgcattcgctggacacgaaaagattcaagggttaaacgagtttattaatcaagaatgccagaaagatagtgaactcaaatctaaactgaagaataggcatgctttcaagatggctgttctctttaagcagatattatctgatagagagaaatcattcgttattgatgagtttgagagtgatgcacaggtcattgatgctgtgaagaatttctatgcagagcaatgtaaggataataatgttatctttaatttactgaacttaatcaagaatattgctttcttatctgacgacgaattggatgggatctttattgaaggtaagtatcttagttcagttagccagaaattgtactctgactggtcaaagctgagaaatgatatagaggattctgctaattcaaagcaaggaaataaggagttagccaagaagatcaagaccaacaaaggtgatgttgagaaagctatttcgaagtacgaattctcactgagtgaactaaactccatcgtgcatgataataccaagttcagtgatcttctttcttgtactttgcataaagtggcaagtgagaaactggtgaaagtgaatgaaggtgattggccaaagcatttgaagaacaacgaagagaagcagaagattaaggaacctttggatgcactcctcgaaatttataataccttattgatctttaactgtaagagtttcaacaagaacggtaacttctatgtcgactatgacagatgtattaatgaactttctagtgttgtctatttgtacaataagacaaggaattactgtacaaagaaaccatataatacagacaaattcaaactgaactttaacagcccacagttgggagaaggcttctccaagtctaaggagaatgattgtcttacattgctatttaagaaagatgataattattacgtcggcataatacgaaagggtgcgaagataaacttcgatgatacgcaagctattgcggacaatacggacaactgtatcttcaagatgaactacttccttcttaaagatgcaaagaagttcatccctaagtgttctatacagcttaaggaggtcaaggcacactttaagaagagcgaggacgattacatcttaagtgataaggagaaattcgctagcccgttggtgatcaaaaagagcactttcttactcgcaacagcgcacgtcaagggtaagaagggtaacatcaagaagtttcagaaggaatactccaaggagaaccctactgaatacagaaacagtttaaacgagtggatagcattctgcaaagagtttctcaagacttataaggcggcaacaatatttgacataacaactctaaagaaggccgaggagtacgcagatattgtagagttctataaggatgttgataatctctgctacaagctggaattctgcccgataaagacatcctttattgagaatctaatcgacaacggagacttgtacttgtttcgtatcaataacaaggacttctcatcgaagtctacgggtaccaagaatcttcacactttgtacctgcaagcaatatttgatgaacgtaacctcaataaccctaccattatgctgaacggaggtgctgaattgttctaccgaaaggagtctatagaacagaaaaataggatcacacacaaggcaggttcgatccttgtgaataaggtctgtaaggatggaacttcacttgatgacaagattcgaaatgaaatttatcaatacgagaacaaatttatcgatacattaagtgacgaggcgaagaaagttctgcctaatgtgataaagaaggaggctacccatgatattacaaaggataagagatttacatcagacaaatttttcttccattgcccgcttactattaactataaggaaggtgatactaagcagtttaacaatgaagtgctatcattcttgagaggaaacccggatattaacatcatcggcatagacagaggagaaaggaatttaatctatgtcacagtcattaaccagaagggtgaaatcctagattctgttagcttcaatacggtaactaacaagtcgtcgaagatagagcaaacggttgattacgaagagaagctggccgttcgagagaaggaaaggattgaggccaagcgatcgtgggattctataagcaagatcgccacacttaaggagggatatttaagcgctatcgtgcatgaaatatgccttctcatgatcaagcacaatgctattgttgtattagagaatttgaatgcaggcttcaaacgtattcgggggggactttcagagaaatcagtgtatcagaaattcgagaaaatgttaataaataagctcaactactttgtgtctaagaaagaatctgattggaataaaccttctggacttcttaacggtcttcaactatcagaccagttcgagtctttcgagaagcttggtatccagtcgggattcattttctatgtacctgctgcatatacctcaaagatcgatccgaccactggatttgctaacgtcctaaaccttagtaaggtaagaaacgttgatgcgataaagagttttttctcaaacttcaacgaaatttcttattcaaagaaagaggccttatttaagttctcgttcgatctcgacagccttagcaagaaaggtttctcgtctttcgttaagttctcaaagtcaaagtggaatgtttacacatttggtgagcgtattattaaaccaaagaataaacaaggatacagagaagataaacgcatcaatttaacctttgaaatgaagaaactgcttaatgaatataaagtttcgttcgacttagagaacaacttaataccaaatttgacatctgctaatcttaaagacaccttctggaaagaactattctttatattcaagacaacgctgcaattgaggaacagtgtgaccaacggtaaggaagatgtattgatctcgcctgtgaagaatgccaagggtgaattcttcgttagtggaactcacaataagaccttgccgcaagattgtgatgctaatggtgcatatcatatcgctttaaagggactgatgatcttagagagaaataatttggttagggaggagaaagacacgaagaaaatcatggctatatctaatgttgattggttcgaatatgttcagaagcggcgtggagtcctgtaa

SEQ ID NO: 309 - DNA, 4005 bp, Artificial Sequence
  Description of Artificial Sequence: Synthetic polynucleotide
atgagttcgttaaccaagttcacgaataagtatagtaaacagcttactataaagaatgaactaattccagtcggaaagaccctggagaacattaaggagaatggtttgattgatggtgatgaacaactgaatgagaactaccagaaggcgaagatcattgttgacgatttcttgcgcgacttcatcaacaaggcgctcaataatacacaaattggcaattggagggagttagctgatgctttaaataaagaggatgaggataatatagagaagttacaagacaagatacgtgggatcattgtttctaaattcgagacctttgatctattcagcagttactcaattaagaaggatgagaaaatcattgacgacgataatgatgtagaagaagaggagcttgatcttggcaaaaagacttcttcattcaagtacatcttcaagaagaatttgtttaaacttgtacttccttcatacctaaagacaacgaaccaggacaagcttaagatcatctcatcatttgacaacttctcaacttactttcgaggcttctttgagaaccggaagaacatctttaccaagaagcccattagcactagtatcgcttaccggatcgttcacgataacttcccaaagttcttagataacattagatgcttcaatgtttggcaaactgagtgtcctcaactcattgttaaggcggacaactatcttaagtcgaagaatgttatagctaaggacaagagccttgctaattacttcacagtaggcgcttacgattacttcctgtctcagaatggtatcgacttctataacaatatcataggagggttaccggctttcgctggtcatgaaaagatacaaggattaaacgagtttataaaccaggagtgtcagaaagatagcgaattgaagagtaaactcaagaaccggcatgcattcaagatggctgtcttgtttaagcagatcctatctgatcgcgagaaatcattcgtcattgatgaatttgagtccgatgcgcaagttatcgatgcagtaaagaacttctatgcggagcagtgcaaagataacaatgttatctttaacctactgaacctcattaagaacattgcatttctttctgatgatgaattggacggtatatttattgaaggcaagtatctcagctcagtgagtcagaaattgtactctgattggtctaaactgcggaacgacatagaagattcagctaattccaagcaaggaaataaagaacttgcgaaaaagataaagacgaataaaggagatgtagagaaggcaattagtaagtacgaattctcactcagtgagcttaattctatcgtgcacgacaacactaagttctcggatctccttagttgtacactccataaagtagctagtgagaaactcgtcaaagttaacgagggagattggcccaaacatctaaagaacaatgaggagaagcaaaagattaaagagccattagacgctttgttggagatatataatacacttctgatcttcaactgtaagtccttcaataagaatggaaacttctatgtggattacgatcgttgtattaatgagttaagttctgtggtttatctctataataagacccgaaactactgtacaaagaagccttacaacacggacaaatttaagctgaatttcaattctccgcaactaggtgaaggcttctccaagtccaaagagaatgattgtttgactttgctatttaagaaggatgacaactactacgttggtataatacgtaaaggtgctaagattaatttcgacgacactcaggctattgccgataacacagataactgtatattcaagatgaactacttcctccttaaagatgctaagaagtttattccgaagtgtagcattcaactgaaggaagttaaggcacatttcaagaagagtgaggacgattacattctgtctgacaaagagaaatttgcttctcccttagtgataaagaagtctacattcttgctagctacagcacatgttaaaggtaagaagggtaatattaagaagtttcagaaagagtattcgaaagagaatcctacagagtataggaattcattgaatgagtggatcgcattctgtaaagaatttttaaagacatataaagccgccaccatcttcgatattactacactaaagaaggcagaagagtacgctgacattgttgagttctataaggatgttgataatttgtgttacaagttggaattctgtccaatcaagacttcgttcattgagaacttgattgataatggcgacctttacctctttaggattaacaataaagacttctctagcaagtccacgggaaccaagaatctacacaccctttacctacaggctatcttcgatgagcgtaatcttaataatccaactatcatgttaaacggcggagcggaattattttaccggaaggaaagtattgagcagaagaatcgtataacccataaggctggtagtatacttgttaacaaagtctgtaaggacggaacctctctggatgacaagattcgcaacgagatttaccagtacgagaacaagtttatcgatactttgtccgatgaggcgaagaaggtgctgccaaacgttataaagaaagaggctacacacgacattaccaaagataagagattcacatcagataaattcttcttccattgtcctctgaccattaattacaaggagggtgatacgaagcaatttaataatgaagtgttgtctttcttgcgtggcaatccggatattaatattatcggaatcgatcgcggcgaacgtaatttaatctatgttaccgtgatcaaccagaagggtgagatactagattctgtgtcgttcaacactgtgacgaataagagttctaagatagaacaaactgtcgactatgaagagaagcttgcggtacgtgagaaggaaagaatcgaagcgaagagatcgtgggattctatatcgaagattgctacccttaaagaaggttacctgtcagctatcgtacacgagatatgtcttcttatgatcaaacataatgcgattgtagtgctagagaatcttaacgccggctttaagagaataagaggtggattgagtgagaaaagcgtttaccagaagttcgagaagatgttgataaacaaattaaactatttcgtttcaaagaaagagagtgactggaacaagccgtctggactcctcaacggtctgcagttaagtgaccaattcgaatcgttcgagaagttgggcattcagagtggtttcatcttctacgttccagctgcatacacatctaagattgatcctacaacgggctttgctaacgtcttaaacttgtcgaaagttagaaacgttgatgccatcaagtctttcttctctaatttcaacgagataagttacagtaagaaagaagctttgtttaagttcagtttcgatcttgattccctatcaaagaaagggttctcgagctttgtgaagttctctaagagcaaatggaatgtgtatacgtttggtgaacgtattattaaaccgaagaacaagcaaggatacagggaagataagagaatcaaccttacattcgaaatgaagaagttgttgaatgagtacaaggtatctttcgatctagagaacaacttaattccaaatcttacaagtgctaatcttaaggatactttctggaaggagttattcttcatatttaagacaactttgcaattgagaaactcagtgacgaacggaaaggaggatgttctaattagtccggttaagaatgcaaagggtgaattcttcgtgtccgggacgcataataagacactcccgcaagattgtgatgcgaatggcgcttatcatattgcattgaagggacttatgatcttggaacgcaataatctggtccgtgaagagaaggataccaagaaaatcatggcaatcagtaacgttgattggttcgagtacgttcagaagagacgcggtgtcctctag

SEQ ID NO: 310 - DNA, 4005 bp, Artificial Sequence
  Description of Artificial Sequence: Synthetic polynucleotide
atgtcaagcttaacgaagttcactaataaatactccaagcagctgacaatcaagaatgaattgattcctgtgggcaagacactcgagaatatcaaagagaatgggctaattgacggtgatgagcaacttaatgagaactatcagaaggcgaagatcattgttgacgacttcctcagggactttattaacaaggctcttaacaatacccaaattggcaactggcgtgagcttgctgacgctttgaacaaggaggatgaggacaacattgagaagttgcaggacaagatccgcgggattatcgtgtctaagtttgagacgtttgatctattcagctcctatagcattaagaaagatgaaaagatcattgacgatgataacgatgttgaggaagaggaattggatttaggcaaaaagacttcatcatttaagtacatctttaagaagaacctgtttaaattagtcctgccctcgtatcttaagacaacaaatcaagacaagttaaagataatttcctcattcgataatttctcgacttacttcagaggtttctttgagaatcgcaagaatatatttaccaagaagccaataagcacgtcgattgcataccgcatcgttcatgacaacttccctaagttcctggacaatataagatgcttcaatgtctggcaaacggagtgtccacagctaattgtgaaggctgataattaccttaagtccaagaacgttattgcgaaggataagtccctagccaattatttcaccgtgggcgcttacgattacttcctttctcagaatggaatagacttctataataatattatcggcggtttgccagcattcgcaggacatgagaaaatccaaggattaaatgagtttattaaccaggagtgccagaaagattctgaattgaagtctaaactcaagaacagacacgcctttaagatggcggtgttatttaagcagattctctcagatcgagagaaatccttcgtgattgacgaattcgaaagtgatgctcaggtgatcgatgctgttaagaatttctatgctgagcaatgtaaggataataacgtgatctttaatttgttaaacctaattaagaacattgccttcctctcggacgacgagctagatgggatattcattgagggaaagtacttgtcgtcagtatcccagaaactttattctgattggtcgaagcttagaaacgatatcgaggattcggctaactctaaacaaggaaataaggagctcgcaaagaagatcaagaccaacaaaggtgatgtcgagaaagctatttcgaaatacgaattcagcctctctgagctaaatagtatcgttcacgacaacactaagttctctgacctcctctcatgtacccttcataaagtggcgagcgagaaactagtcaaggtcaacgagggagattggcctaagcaccttaagaataacgaggagaaacaaaagatcaaagaaccacttgatgctctcttagaaatttataacacgttactgatcttcaattgcaaatctttcaacaagaatgggaacttctatgttgattatgaccgctgcatcaatgaactatctagcgtggtatatctttataataagacccgtaactactgcacgaagaaaccctataacacggataaattcaagttgaatttcaatagcccgcagctcggagagggattctctaagagtaaggagaatgattgcttgaccctgctctttaagaaagatgacaactattacgtaggcatcataaggaaaggcgcaaagattaactttgatgacacacaagctatagcggacaacactgataattgtatctttaagatgaactacttcctacttaaggatgcgaagaaattcatacctaagtgctctattcagcttaaggaggttaaagcacactttaagaaatctgaggatgactatattctgtcggataaagagaagtttgcatcgccactcgtcataaagaagtctactttcctacttgctaccgctcatgttaagggcaagaagggaaatatcaagaagttccagaaagagtacagtaaggagaacccgaccgagtataggaactctttgaacgaatggattgcattctgtaaggaattcctaaagacatataaggcagctacaatatttgatatcacaacactgaagaaggctgaagaatatgccgatatcgttgaattctataaggatgttgataacctatgttacaagcttgagttctgccctattaagacatcatttattgagaatcttattgacaacggtgatctttatttatttcgtatcaacaacaaagatttctcatctaagtctacaggaacgaagaatctacatacactttacttgcaagcaatcttcgacgagagaaacttaaacaacccgactatcatgctaaacggtggagcagagttattctacagaaaggagtccatagaacagaagaataggatcacgcacaaagctggttcgatcctcgttaataaagtttgtaaggacggaacttctctcgacgacaagattagaaatgagatctatcaatatgagaacaaattcatcgatactctaagcgacgaagcgaagaaggttctgccaaatgtgatcaagaaggaggcaacgcatgatattacgaaagataagagatttacttcagataaattcttctttcattgtccgttgacaattaactataaagaaggagatacgaagcaatttaataatgaagttctatcattcttaagaggaaacccagatatcaatattataggaattgacagaggagaacgcaatctgatctacgtgacagttatcaaccagaagggtgaaatcttggacagtgtgagtttcaacacagtaacgaataagtcctccaagattgagcaaactgtcgactatgaggagaagttagcagttagagagaaggaaagaattgaggcgaagagatcatgggactccatatcaaagattgcaacactgaaagagggatacctttctgcgattgtgcacgaaatttgcttgttgatgatcaagcacaacgcaatcgttgtcctcgagaacttgaatgcaggtttcaaacggattcgcggcggactctctgagaaatctgtgtaccagaagtttgagaagatgcttataaacaagcttaactactttgttagcaagaaggaatctgactggaacaaaccatctggcttgctaaacggtcttcaactttctgaccaatttgaatctttcgagaaattgggcattcaaagtggattcattttctacgtacctgcggcttatacttccaagatcgatcctacaacagggtttgcaaacgttctaaatctgagcaaagttagaaatgtggacgccatcaaatctttcttctcaaactttaacgagattagctattcaaagaaagaagccttgttcaaattcagtttcgatcttgacagtttgtcaaagaaaggcttctcttcattcgtcaaattctctaagagcaaatggaatgtgtacactttcggagaaagaatcattaagccaaagaacaaacagggttatagagaggataagcggattaaccttacattcgaaatgaagaagctcttgaatgagtacaaagtcagctttgatcttgagaataacctcattccaaatctgaccagtgctaatcttaaggatacattctggaaggagttattctttatcttcaagacaacattacagctacgtaacagtgttactaacggtaaggaagacgttctcatatctcctgtgaagaatgccaaaggcgaattctttgtcagtggtacccataataagaccttaccacaggattgtgatgcgaacggagcgtaccatattgcattaaagggtcttatgattcttgagagaaataatctcgtgagggaagagaaggataccaagaaaatcatggccatttctaacgttgattggttcgaatatgttcagaagaggcgtggggtgctttaa

SEQ ID NO: 311 - DNA, 4005 bp, Artificial Sequence
  Description of Artificial Sequence: Synthetic polynucleotide
atgtcgtcattgactaaatttacaaataagtattctaagcaactcactatcaagaacgaactgatccctgtaggaaagacattggagaatatcaaggagaatggactaattgacggtgatgagcaactcaacgagaactatcagaaggcaaagatcatagtcgacgatttcttgagagacttcattaacaaagcattgaataatactcagattggcaactggcgagaactagcggacgcacttaataaagaagatgaagacaatatagagaagcttcaagataagatccgcggtatcatcgttagtaagtttgaaacgtttgatttattctcatcttattctataaagaaagatgagaagattattgatgatgataatgatgttgaggaagaagagttagatcttggaaaaaagacatcatcgtttaagtacatatttaagaagaacctattcaaattagtgctaccctcatatttaaagactaccaatcaagataagcttaagatcatatcatcgttcgataatttctctacctactttagaggcttcttcgagaatagaaagaatatctttaccaagaagcctatctctacatctattgcgtaccgtattgtgcatgataactttccaaagttccttgataacattcgatgcttcaatgtttggcagacagaatgtcctcaactaattgtgaaagcagacaattaccttaaaagtaagaacgttatagcgaaggacaaatcacttgcaaattatttcactgtaggagcgtacgactactttcttagccagaacggcatagatttctacaacaacattattggtggtctcccggcgtttgctggacacgagaaaatacaaggccttaacgaattcattaaccaggagtgtcagaaggattcagagcttaagagtaaactgaagaaccgacatgcgtttaagatggctgtgctcttcaaacaaatcttatccgatcgggagaagtcattcgtcatcgatgaatttgaatctgatgctcaagtaattgacgctgttaagaacttctatgcagaacaatgtaaagataataacgttatattcaacctcctcaatttgatcaagaatattgccttcttgagtgatgatgagttggatgggatattcatagagggtaagtacttatcttctgtttcccagaaactttatagtgattggtctaaactaagaaatgatatagaagattctgctaactctaaacagggtaacaaggaattggctaagaagatcaagactaacaagggtgacgtggagaaagcgattagtaagtatgagttcagcctgtctgaactaaactccattgtgcatgacaacacgaaattctcggacctattgagttgcactcttcacaaggttgcttctgagaaattagtcaaagttaatgagggagattggcctaaacatcttaagaataacgaagagaaacagaaaatcaaggagcctctggacgctctgttggagatatataatacccttcttatatttaactgcaagtcctttaataagaacgggaacttctacgttgattacgatagatgtatcaacgagctttcatctgttgtttatttgtataataagacgcgtaattattgtaccaagaaaccgtataacaccgataaatttaagcttaacttcaactcaccgcaattgggagaaggcttcagtaagagtaaagagaatgactgtcttactctcctctttaagaaagacgacaattattatgtgggaattattaggaaaggagccaagattaatttcgacgatacacaggctatagctgataacaccgacaattgcatattcaagatgaactatttccttctcaaggacgctaagaagttcattcccaagtgcagcatacaacttaaagaggttaaagcacatttcaagaagtctgaagatgattacatcctgagtgataaagagaaattcgcttcgcctttggtcattaagaaatcaactttcttacttgctaccgcccatgttaaaggaaagaaaggtaatataaagaagtttcagaaagaatactccaaggagaatccaacggaatatagaaacagtctgaacgagtggatcgccttctgcaaggaattcctcaagacttataaggctgccacaatatttgacataacaacattaaagaaagctgaggagtatgctgacattgttgagttctacaaagatgtagataacctctgctataagcttgaattctgccctatcaagacttccttcatcgagaatctgatcgacaatggagacttgtacttattcaggataaacaacaaggacttctcatccaaatcaactgggaccaagaacctgcacacactttacttgcaggctatattcgatgaaagaaaccttaataatccaacgattatgttgaacggtggtgcagagcttttctacaggaaagagtctatcgaacaaaagaatagaatcactcataaagctggaagtatcctcgtcaataaagtttgtaaagatggaacatctctagatgataagatcagaaatgagatatatcaatacgagaataagttcattgacactcttagcgacgaagccaagaaagtcctgcccaatgtcattaagaaagaagccactcatgacatcacaaaggacaagagattcacatcagacaagtttttctttcactgtcctctgacgatcaactataaggagggcgacaccaagcaattcaataacgaggtgttaagcttcctgagaggtaatccagatataaacattatcggaattgaccgtggcgaacggaacttgatttatgtgacagtaattaatcagaaaggagagatcctggacagtgtatcgttcaatacagtgacgaataaatcgtctaagatagaacagactgtcgattatgaagagaaattggccgtgcgagagaaagaaaggattgaggcgaagagatcgtgggactccatctcgaagatagcaactctcaaggaaggttacctatctgctatagttcatgaaatttgcttgctcatgatcaagcacaatgcaattgtcgttctggagaaccttaacgcagggttcaaacgtattcgtggcgggctttcggagaaatctgtttaccagaaatttgagaagatgctcatcaataaattaaactacttcgtaagtaagaaggagtcagattggaataaaccttccggactattaaatggattgcaattgagcgatcaatttgagtcgtttgagaagttgggaattcaatctggatttatcttctacgtaccagctgcctatacgtctaagattgatccgacaacaggcttcgcgaacgtgttgaatctatcaaaggtacgaaatgttgacgctataaagtccttcttctctaacttcaatgagatttcatactcaaagaaagaagctttgttcaaattctcatttgatctagatagtctttctaagaaaggattctcatcattcgttaagttctccaagtccaaatggaatgtatacaccttcggagagcgtattatcaaacccaagaacaaacagggatatcgagaagacaagagaataaatttaacgttcgaaatgaagaaactgcttaatgagtataaggtttcgttcgatctggagaacaacctcatccctaacttgacctctgctaatctcaaagataccttctggaaagagctattcttcatctttaagactaccttgcaactccgaaattctgtaactaatggcaaggaggatgtactgattagcccggtcaagaatgctaaaggagaattcttcgttagtggaacccacaataagacattaccgcaagattgtgatgcaaatggagcttaccatattgcccttaagggactcatgatcttggagaggaataatttagtgcgcgaggagaaagacacgaagaagataatggctatttcgaacgttgattggtttgaatatgttcagaagcgccgaggcgtgctctga

SEQ ID NO: 312 - DNA, 4005 bp, Artificial Sequence
  Description of Artificial Sequence: Synthetic polynucleotide
atgagtagcttaaccaaatttaccaataaatatagtaaacaattgactataaagaatgagctaattcctgttggaaagacgttagagaatatcaaggagaatggcttgattgatggagatgaacaattgaatgagaactaccagaaggccaagattattgttgatgatttcctaagagacttcattaacaaggctctgaataatactcagatagggaattggagggagcttgccgacgcactcaataaggaagatgaagataatatcgagaagctccaggacaagattcgaggtatcatcgttagcaagtttgaaacattcgatttattctcatcttactcgataaagaaggatgagaagattatcgacgatgataatgatgtggaggaagaggaattagatctgggtaaaaagactagttctttcaaatacatcttcaagaagaatctattcaaacttgttctaccttcgtatctcaagacaacaaaccaagataagcttaagattatctcctccttcgacaacttctctacatacttcagagggttcttcgagaatagaaagaatatcttcactaagaagcccatctctacatcgatagcctacagaatcgttcatgacaactttccaaagttcctagacaatatccgatgcttcaacgtatggcaaacagagtgtcctcaactgatagttaaagcggataactacctcaagtcgaagaacgtgattgccaaagataaatctcttgctaattatttcactgtcggcgcttatgattatttcctgtcccagaatggtattgatttctataataacatcattggaggacttccagcgttcgccggtcatgaaaagatccaaggactgaatgagttcattaatcaggagtgtcagaaggattcagaactgaagtcgaagttaaagaatagacatgcattcaagatggcggtcttgtttaagcagatcttaagcgacagagaaaagagtttcgttatagatgaatttgagagcgatgcacaagtcattgatgccgtcaagaacttctatgcagagcagtgtaaagacaataatgttatctttaatttacttaatctcatcaagaatattgcattcctaagcgacgatgaactcgatggaatctttattgagggtaaatacttgtcctcggtatctcagaagctatatagtgactggagtaaactcagaaatgatattgaggactctgctaattcaaagcaaggaaataaggaactcgcgaagaaaattaagacaaataagggagatgtagagaaagcaatttctaaatacgagttctcattgtctgaattaaacagtattgttcacgataatacgaagttctctgatcttctatcatgtacgctgcataaagtggcatctgagaagctagttaaagtcaacgaaggtgattggcccaaacacctgaagaataatgaagagaagcagaaaatcaaggagcctttagatgctttactggaaatatacaatactttgctcatctttaactgtaagtcattcaataagaatggtaatttctacgttgattacgatcgctgcataaatgaattatcgagtgtagtgtatttatacaacaagacaaggaattattgtaccaagaagccgtataataccgacaaattcaagcttaactttaactcacctcaattaggtgagggattctctaagagtaaagagaacgactgccttacactcctatttaagaaggacgataactattacgttggtattatcagaaagggagcgaagatcaactttgatgatacccaagccatcgcagataatactgacaattgcatatttaagatgaactacttcctccttaaagatgctaagaaatttataccaaagtgctctatccaattgaaggaagttaaagcacacttcaagaagtccgaagatgactacatccttagcgataaagagaagtttgcttcgccactggttataaagaagtcaacattcttgctcgcaacagctcacgtaaaggggaagaagggaaacataaagaaatttcagaaggaatatagtaaggagaaccctacggagtacaggaactcgcttaacgagtggattgcattctgcaaagaattcttgaagacatataaggctgcgacgatctttgatataacaactttaaagaaagcagaggaatatgctgatattgttgaattctataaggacgtggataacctttgttacaaactcgagttctgtcctattaagactagcttcattgagaaccttattgataacggagatctttacctatttaggattaacaacaaagatttctcatccaagagcacagggactaagaaccttcatacactgtaccttcaagcaatatttgatgagaggaaccttaacaatccaacaattatgttgaatggaggtgctgaactattctatagaaaggagagtatcgaacagaaaaacagaatcacccacaaagcaggatctatactggtgaacaaagtttgtaaagatggaacctctctcgatgataagattaggaatgaaatttatcaatatgagaataaattcatcgatacacttagtgatgaagcaaagaaagtgctcccaaacgtcataaagaaagaagcaacgcacgatattaccaaagacaagaggtttacttcagacaaattcttcttccattgtcctctcacgatcaactataaagagggtgatactaaacagttcaacaatgaagtattatcattcttacgcggtaaccctgatattaacatcatagggattgacagaggagagagaaacctgatttacgttaccgttattaaccagaagggcgaaatcctcgattctgtgtctttcaacacggtcacaaataagagttctaagatagaacagactgtggactatgaagagaaacttgcagtgcgtgagaaggagagaattgaggccaagagatcatgggactctatcagcaagatagctactcttaaggaaggctatctttccgctatcgttcacgagatttgccttctaatgataaagcacaatgctatcgttgtactcgagaacctgaacgctggcttcaagagaattagaggtggtctgtctgagaagagcgtgtaccagaaatttgagaaaatgttaatcaacaaacttaattactttgtttccaagaaggagagtgactggaacaaaccatcaggactactcaacggactacagctttctgatcagttcgagtcatttgagaaacttggtattcaatcgggatttatcttctatgtgcctgctgcttacacaagtaagatagacccaactaccgggtttgcaaacgttctcaatcttagcaaagttagaaatgtagatgccattaagtctttcttctctaacttcaatgaaatctcctattccaagaaggaagctctcttcaagttcagctttgatctggattctctcagtaagaagggcttctccagctttgttaaattctccaagtcaaagtggaatgtctataccttcggagaaagaattattaagcctaagaacaaacaaggctatagggaagacaagagaatcaatttaaccttcgaaatgaagaaactcttgaacgagtataaagtcagctttgatttggagaataaccttattcctaatttaacaagtgctaatctgaaggacaccttctggaaggaactcttctttatcttcaagacaactttacagttgcgaaactccgtcacgaatggtaaagaggatgttctcatctctcctgttaagaacgccaagggtgagttcttcgttagtgggacacacaacaagacactaccacaagattgcgacgcgaatggtgcttaccatatcgctttaaagggactaatgatcctcgaaagaaacaacctagttagagaggagaaagataccaagaagattatggcaatttctaacgtcgactggtttgaatatgtccagaagcgacgtggtgtactttaa

SEQ ID NO: 313 - DNA, 4005 bp, Artificial Sequence
  Description of Artificial Sequence: Synthetic polynucleotide
atgagttctctcacgaagtttacgaacaaatactccaagcagctaactattaagaatgagcttattccagtgggcaagacactcgagaatattaaagagaatggccttatagacggagacgaacagcttaatgagaactatcagaaggctaagataatcgtcgatgatttcctcagagacttcattaataaggccttgaataacactcagattggtaactggagagaactcgcagatgcactcaataaagaggatgaagataacatagagaagctgcaagataagataagaggcattatagtttcaaagtttgaaacattcgacctattctcgtcatattctataaagaaggatgagaagattatagatgatgataatgatgttgaggaggaggaattagatctcggcaagaagacaagcagtttcaaatacatcttcaagaagaatctattcaagcttgtgctcccatcttatctcaagacaacgaaccaagataaactaaagatcattagcagtttcgacaatttctcgacttacttccggggcttcttcgagaatcgcaagaacatcttcactaagaaacccatctcgacttcaattgcatatagaatcgtccacgataatttcccaaagttccttgataatatacgctgcttcaacgtctggcagacagagtgtcctcaacttattgtgaaagcagataactacctcaagtctaagaatgtgattgctaaggacaagtcattggcaaattacttcacagtaggcgcctatgattatttcttgtcccagaacggcatagatttctataataacattatcggaggacttccagcatttgcagggcatgagaaaatccaaggactcaatgaattcataaaccaggagtgtcagaaagattcggaactcaagtctaagcttaagaataggcacgcttttaagatggcggtactctttaaacagatccttagcgatcgtgagaaatcctttgtgatcgatgagttcgaaagtgatgcacaggtcatagatgctgttaagaatttctacgcagaacaatgtaaagataacaatgtcatctttaatctcttgaatctgattaagaatatagctttcctctccgatgatgaattagatggcatattcatcgaaggcaagtatttatcttctgtgtcccagaaattatactctgactggtcaaagttgagaaatgacatagaagattcagcaaactctaaacagggtaataaggagcttgctaaaaagattaagacaaataaaggagacgtggagaaagcgatctctaagtatgagttcagcttatcggaacttaattctattgtgcacgataataccaagttctctgatttgctttcatgcacactccacaaggtcgcgtccgagaagttagtgaaagtgaacgaaggagattggccaaagcatcttaagaataatgaagagaagcagaaaattaaggaacctctcgatgctcttcttgaaatctacaatacgctacttatatttaattgcaagagcttcaacaagaacggaaatttctacgtagattatgataggtgtattaacgaactttcatctgtcgtctacctttataataagacccgaaattactgtactaagaaaccttataacactgacaaatttaagctgaactttaacagtccacaacttggtgaaggcttcagcaagagtaaagagaatgattgtctcacgctcctattcaagaaagatgataactattatgtaggaattattcgaaagggagcaaagatcaacttcgatgacactcaggctatcgcggataacacagataattgcatcttcaagatgaattactttcttctcaaagatgctaagaaatttataccgaagtgctcgattcaattgaaggaagttaaggctcactttaagaaatcggaagatgactatatactttcggataaggagaaattcgctagtcctcttgtgataaagaagtccacatttctacttgctaccgctcacgtcaaaggtaagaaagggaatatcaagaaattccagaaggagtactcgaaagagaatccaaccgagtaccgtaatagcttgaacgagtggattgccttctgcaaagaattcttgaagacatataaagcggctacaatatttgacatcacgacactcaagaaggctgaagagtatgctgatatagtagagttctataaagacgtggataacctctgttataaactagaattctgtccaatcaagaccagcttcattgagaacctcattgataatggagatctttatttgttcagaattaacaataaggacttctcgagtaagagtactggcaccaagaatttacacactctctacttgcaagcgatcttcgacgaacggaatctcaacaaccctacaattatgctcaatggaggtgctgaactcttctaccggaaagaatctatcgaacagaaaaatcgtatcactcacaaggcaggatccattcttgtaaataaggtatgcaaagatggtacatcactagatgataagataaggaatgagatatatcaatacgagaacaaatttattgatactttatcagatgaagctaagaaggtactgcccaatgtaattaagaaagaggcaactcacgacattactaaagacaaacgtttcacgtctgataaattcttcttccattgtccattaaccattaattacaaggaaggagatactaaacaatttaataacgaggtcctttcgttcttacgaggcaatccagatataaatataatcggaattgatagaggagaacggaacctcatctacgtaacagtgatcaaccagaagggagagatcctcgattctgtatcatttaacactgttacaaacaaatctagtaagattgagcaaacagttgattatgaagagaaactcgcggtccgggagaaggagagaatagaagctaagaggtcttgggatagcatctcgaagatcgcaacattgaaagaaggttacttgagcgcaattgtccatgaaatttgcttactaatgattaagcacaatgctattgtagtacttgagaaccttaatgccggtttcaagaggattcgaggcggtttatccgagaagtctgtctaccagaaattcgagaagatgttgattaacaaattaaattatttcgtgagcaagaaggaaagtgattggaataagccttcaggccttcttaatggattgcaactatctgatcagttcgagtcgttcgagaagctgggaattcagtcagggtttatattctacgtgcctgcagcctacacttcaaagattgatccaacaactggattcgctaacgtgcttaatctgagtaaagtcagaaacgttgatgctataaagtctttcttcagtaacttcaacgagatctcttactctaagaaggaggctctgtttaaattctcctttgatctcgattccttgtcgaagaaaggattctctagcttcgtgaagttcagtaagagtaagtggaacgtgtacacctttggtgagcgcatcatcaaacctaagaataagcaaggttatagggaagacaagaggattaatctgacatttgaaatgaagaaacttctaaatgagtataaggttagtttcgacttggagaataacttaattcctaaccttaccagtgccaacttaaaggacactttctggaaagagctattcttcatatttaagactaccctccagctccgtaactcggtgactaatggcaaagaagacgttctcatctcaccagttaagaatgcaaagggagaattctttgtctcgggtacccataacaagaccctaccacaggattgcgacgccaatggagcttatcatatagcccttaagggactcatgatattagaaaggaataatttagttagagaagagaaggataccaagaagattatggcaatctcaaacgtggattggttcgagtatgtgcagaagaggagaggcgttctttga

SEQ ID NO: 314 - DNA, 4005 bp, Artificial Sequence
  Description of Artificial Sequence: Synthetic polynucleotide
atgtcttctctcaccaagtttactaacaagtattcaaagcaactcactatcaagaacgagcttattccggtggggaagactttggagaatattaaggagaacggtctcatcgacggagatgaacaacttaacgagaactatcagaaggctaagatcatagttgatgatttcctccgtgacttcattaataaggcacttaataatacacagattggcaattggcgagagctggcggacgcgcttaacaaggaggatgaggataatatagagaagttacaggacaagatccgaggaattatcgtgtctaaatttgaaaccttcgatctattctcttcatattctatcaagaaagacgaaaagattattgacgacgacaatgatgttgaggaagaagagttggacttaggtaagaagacctcttccttcaagtacatctttaaaaagaacctatttaagctcgtattgccaagttacctaaagactaccaaccaagataaattaaagatcatctcttcctttgataactttagtacttacttccgaggtttcttcgagaaccgcaagaatatcttcactaagaagccaattagtacgtccattgcttacaggatcgtgcacgataattttccaaagttcttagataatattagatgtttcaatgtttggcaaacggagtgtccacaacttatcgtcaaagcagataattacctgaagtcgaagaacgtcattgcgaaggacaagtcacttgccaattacttcaccgttggtgcgtatgactatttcctttcacagaacgggatagacttctacaataatattataggaggtcttcccgcgtttgctggacatgaaaagattcaaggacttaacgagtttatcaatcaagaatgtcagaaagattctgagttgaagtcgaagcttaagaacaggcatgcgtttaagatggcagttctcttcaagcagatcctatcagacagagagaagagtttcgttatcgatgaatttgaaagtgatgctcaggtaatcgacgcagtaaagaacttctacgctgagcagtgtaaagataacaatgttatcttcaatttgttaaatttgatcaagaatatagctttcctcagtgatgatgaacttgatggtatatttattgagggcaagtatctgtcaagtgtatctcagaagttgtactcggattggagcaaactcagaaatgatattgaggattccgcaaatagtaagcaagggaacaaggagctcgcaaagaaaattaagacaaacaaaggtgatgttgagaaagcaatctccaagtacgagttctcattgagtgaactcaatagcatcgtccatgataataccaagttcagtgatttactgtcatgtacgcttcataaagtagcatccgagaaattagtgaaggttaacgaaggtgattggcctaaacatttgaagaacaacgaggagaaacagaaaattaaggagcccttggatgctcttctcgagatttataacacattactaatcttcaattgtaagtcattcaataagaacggtaacttctatgtggactacgatcggtgcatcaatgagttatcatcagttgtttatttgtataacaagactcgcaattactgtaccaagaaaccgtataacaccgataaatttaagttgaacttcaattcaccacagcttggcgaagggttcagcaagagtaaggagaacgattgccttaccctcttattcaagaaggacgataattattacgtaggaataatacggaagggagcaaagataaacttcgatgatacacaggcgatagctgataacaccgataattgcatatttaagatgaattacttccttctcaaggacgcgaagaaatttattccgaagtgctctatccaactgaaagaggttaaagcccattttaagaagagtgaagatgattatattctttctgataaagagaagttcgcgtctcctttggtaatcaagaaatctaccttcctgctggctactgctcatgttaagggaaagaaaggtaatattaagaagttccagaaggagtatagtaaggagaacccaactgaatatcgtaacagtcttaatgagtggattgccttctgcaaggaattcctgaagacttataaggcggctactatctttgacatcaccactttaaagaaagctgaagagtatgctgacatagtagagttctataaagatgtcgataatctgtgttataaactggagttctgtccaattaagacttccttcatcgagaacttgattgacaatggtgatttatacctgttcagaataaataataaggatttctcttccaagagcactggcacgaagaatcttcatacattatacctccaagcgatcttcgatgaacggaatctcaacaacccaacaatcatgctcaatggtggtgcagaattattctacaggaaagagtcgatagagcagaaaaatcggatcacccataaggctggcagcattctagtaaacaaggtctgcaaagacggaacatcccttgacgataagatcaggaatgaaatctaccagtatgagaacaagttcattgatactctgtcagatgaggcgaagaaagtcctgccaaacgtgataaagaaggaagccacccatgatattacgaaggataaacgatttacctccgataaattcttctttcactgcccactcacaattaattataaggagggagacaccaagcagtttaataatgaggttctttctttcctgcgtggaaatccggatattaacattatcggaatcgaccgaggtgaaagaaatctcatctacgttactgttattaatcagaaaggagaaatcttggatagtgttagcttcaatactgtaaccaataaatccagcaagatcgaacagactgttgactatgaggagaaacttgcggtgcgagagaaagaaagaatagaagctaagagaagttgggattccatctcaaagatagctactttgaaggagggctacctaagtgcaattgtccatgaaatatgtttactgatgataaagcacaacgcaattgtcgtgttggagaatctgaatgccggctttaagaggatacgtgggggactctcggagaagtctgtctaccagaagttcgagaagatgttgattaataaactaaactatttcgttagtaagaaggagtctgattggaataaaccttcaggcctcttaaatggtcttcaactctctgaccagttcgaatccttcgagaaattgggaatccaatctggatttatcttctacgtccctgcagcatacacatcgaagattgatccaaccacaggattcgctaacgtgctgaatttgtcgaaagttaggaatgtagatgctataaagagtttcttcagcaactttaatgagatctcctactcaaagaaagaggctctgtttaaattctcgtttgatttggactcgttgagtaagaaaggattcagtagctttgtgaagttttcaaagagtaaatggaacgtttatacatttggagaacgtataataaagcctaagaataagcagggctaccgagaagacaagcgtatcaatttgaccttcgagatgaagaagctcctcaatgagtataaggtgtcatttgatcttgagaacaacttaattcctaatctaacaagcgctaatctgaaagacactttctggaaagaattgttcttcatatttaagactactctgcagttgaggaactcagttacaaatgggaaagaggacgtgcttatatcgccagtgaagaatgctaaaggagagttctttgtgtctggtacacacaataagacgttgccgcaagattgtgatgccaacggtgcataccatatcgcactgaagggtcttatgatattagaacgaaacaaccttgttagggaggagaaggataccaagaagataatggcaatatcgaatgttgactggttcgaatatgtccagaagaggcgaggggttctttga

SEQ ID NO: 315 - DNA, 4005 bp, Artificial Sequence
  Description of Artificial Sequence: Synthetic polynucleotide
atgtcttcacttaccaagttcactaataagtacagtaagcagcttactattaagaacgaacttattccggttgggaagaccctggagaatatcaaagagaatggtctcatagatggtgacgagcagcttaacgagaactaccagaaagctaagattatcgttgatgacttcctccgtgatttcattaataaggctttgaacaacacgcagattggtaactggagagaactggcggatgctttgaacaaagaagatgaagataacatcgagaaattacaggacaagattaggggcataatagtgagtaaatttgagacattcgatttgttcagctcttacagcataaagaaggatgagaagattatcgatgatgataacgacgtggaagaggaggagttggacttgggtaagaagacatctagtttcaaatatatcttcaaaaagaatttgttcaagctcgtcctacccagttatctgaagactacaaatcaggataagctcaagataataagctcctttgataatttctctacctactttcgtggtttcttcgagaaccgcaagaatatcttcactaagaaacctatctcaacgtccatagcttatagaattgtgcatgataacttcccaaagtttcttgataacattagatgcttcaacgtttggcagaccgaatgtcctcaactcattgttaaagctgataattatttgaaatcgaagaatgtaatcgcgaaggataagtcattagcaaactacttcacggttggagcatatgattacttcttgtcacagaatggtattgatttctacaataatattataggaggattaccagcgttcgctgggcacgaaaagattcaaggattgaacgagttcataaaccaagaatgccagaaggattctgaactcaaatctaaacttaagaacagacacgcctttaagatggcagtgttatttaaacagattctctcagatagggagaagtccttcgtgatcgatgaattcgaatctgatgcgcaagttatcgacgccgtgaagaatttctacgctgagcaatgtaaggacaataacgtaatattcaatcttctcaatcttattaagaacatagcattcttatcagacgatgagttggatgggatctttatagaaggaaagtacctttcttccgttagccagaaattatattctgattggtccaaacttcgaaacgatattgaggatagtgcaaacagtaagcaaggcaacaaagaactggccaagaagatcaagactaataaaggagatgtggagaaagcaatctccaaatacgagtttagcctttcagagttaaactcaattgttcacgataacactaaattctctgatctgttgtcatgcacccttcataaagtggcttcggagaagctggtgaaagttaatgaaggagattggcccaagcacttaaagaataatgaggagaaacagaaaataaaggagccattggacgctttactcgagatttataatactttactcatctttaactgtaagagcttcaacaagaatgggaatttctatgttgattatgataggtgtattaacgagctctctagtgttgtgtacctctataacaagacacgcaattattgtacaaagaagccgtataacactgataagttcaaactcaatttcaattcaccacaattgggagagggcttctctaaatcgaaagagaacgattgtttaactctcctctttaagaaggatgataactattatgtaggtattatccgtaagggagccaagattaacttcgatgatacccaagcaatcgctgataacacagataactgtatcttcaagatgaattacttcctactgaaggatgctaagaagtttatcccgaagtgctcaattcagcttaaggaagtaaaggcccacttcaagaaatctgaggatgactacattctttcggataaagagaagttcgctagtccgctcgttattaagaagtctacgtttctacttgcgaccgcacacgtgaagggtaagaaaggaaacataaagaaattccagaaagaatactctaaagagaatcctacagaataccgaaactctcttaacgaatggattgctttctgtaaggaattcttaaagacttataaggcggcaacaatctttgatatcactactctaaagaaggccgaggaatatgctgacatcgtggaattctataaagatgttgataatttgtgttataagttggaattctgtccaatcaagacctccttcatcgagaatctcattgataatggtgacttgtacctattccggattaataataaagatttctcttctaagtcgacaggcacgaagaatctgcacaccctttatctgcaagctatctttgatgagcgtaatctcaataaccctactattatgctcaatggaggtgctgaactattctacaggaaggagtccatagaacagaagaacagaattactcacaaggctggttctatcttggttaataaggtatgcaaagacgggacttccctcgatgataagatccgaaatgagatttatcaatatgagaacaaatttatcgataccctttctgatgaagctaagaaggtgttgccgaacgtgataaagaaggaagctacacacgatatcacaaaggataagaggttcacttctgataaattcttctttcactgcccgttaacaataaactacaaagaaggagatactaaacagttcaataatgaagtactctcgttcctcagaggcaatccagacatcaacataattggaatcgatcggggtgaaaggaaccttatttatgttacagtgattaatcagaagggagaaattctggattctgtttcctttaatacagtgactaataagtcctcaaagattgaacagaccgtagattatgaggagaagctggcagtgcgtgagaaggaaagaattgaagccaaacgtagttgggatagcattagtaagatcgcaacgttaaaggaaggctatctcagcgctatcgttcatgaaatatgcctcctaatgattaagcacaacgctatagttgttcttgagaacctcaacgccggattcaagcgaattaggggcgggttaagtgagaagtctgtttatcagaaatttgagaagatgcttattaacaagttgaactactttgtgagcaagaaggagtctgactggaataagccgtccgggcttcttaacggtctccaactgtctgaccagttcgaatcatttgagaaattaggtatacagtctggctttatcttctacgtgcctgctgcatatacttctaagatcgaccctactactggattcgctaatgtactcaacctttccaaggtgcggaatgtcgatgctataaagtctttcttttcgaacttcaatgaaatttcttatagtaagaaagaagctctgtttaagttctcatttgatttagacagtctttctaagaaagggttctcgagtttcgtgaaatttagtaaatctaaatggaacgtttatactttcggtgagcgaattattaaacccaagaacaagcaaggctacagggaggataaacggattaacttaactttcgagatgaagaagttattaaacgaatataaagtttcgttcgatttggagaacaatctaattcctaatctcactagtgctaatttgaaagacacattctggaaggaattattctttatatttaagactacactccagctaaggaactccgttaccaatggcaaagaagacgtcctcatcagtccggtcaagaatgccaagggagagttcttcgtctctggaacacataataagacattaccacaggattgcgatgccaacggtgcataccatatcgcgcttaaaggattgatgatacttgagagaaacaacctcgtgcgcgaggagaaagacacgaaaaagataatggctatctctaatgttgactggttcgaatatgtgcagaaacgaagaggagtgctttga

SEQ ID NO: 316 - DNA, 4005 bp, Artificial Sequence
  Description of Artificial Sequence: Synthetic polynucleotide
atgagttcgttaactaaatttactaacaaatatagcaagcaattgacaattaagaatgaattgataccagttgggaagaccttggagaacatcaaagagaacggactaatagacggcgatgagcagcttaacgagaactatcagaaggcgaagatcattgttgacgatttcttaagagactttattaataaggcgctcaacaatactcagatcggaaactggagagaattggccgacgctcttaacaaggaagatgaagataatatcgagaagctccaggataagatcagagggattattgtatcaaagtttgaaactttcgatctattctcttcttacagcataaagaaagatgagaagatcatagatgatgacaatgacgtggaggaagaggagcttgatctcggcaagaagactagctcgtttaaatacatcttcaagaagaatctgttcaaactggtgctaccatcatatctgaagaccactaaccaagataaacttaagattatctctagcttcgacaatttctctacatacttccgcgggttcttcgagaataggaagaacatcttcactaagaaaccaatctctactagcatagcatacagaattgtgcatgacaacttcccaaagttcctagataacattcgatgcttcaacgtgtggcagactgagtgcccacaattaatcgtcaaggcagataactatcttaaatccaagaatgtgatagcgaaggacaagagcttagctaactacttcacggttggagcatacgattactttctttctcagaatgggattgacttctacaataacattattggaggcttacctgctttcgctggccatgagaagatccaaggactcaatgaattcattaatcaggaatgtcagaaggattccgagctgaagagcaaattgaagaataggcatgcctttaagatggctgttctctttaagcagatactttccgatcgggagaagagtttcgtaattgatgagttcgagtcagatgctcaagtcatagatgcagtgaagaatttctacgctgaacagtgtaaagataataacgttatattcaacttgcttaatttgatcaagaatattgctttcctctctgatgatgaattagatggtatctttatagaaggtaagtacctctcgtctgtatcacagaagttgtacagtgattggtctaaattgaggaatgatatcgaggattcagcaaatagtaagcaagggaataaggagctcgcgaagaagatcaagactaataaaggtgacgtggagaaggcaatatctaaatacgagttctctctgtctgaactaaatagtatagttcatgataatactaagttctcagacctcctctcatgtacactccataaagtcgcatctgagaaacttgttaaagtcaacgaaggagattggccgaaacatttgaagaacaacgaggagaaacagaagatcaaggagcctttggacgctttactggaaatatataatacactcttaatattcaactgcaagagcttcaacaagaatggaaacttctacgttgattatgatagatgtatcaatgagctttcttctgttgtctatttatacaacaagactcggaattattgtactaagaagccttataataccgataagttcaagctgaactttaattcaccacagcttggagagggatttagtaaatctaaggagaacgattgcctaactcttctatttaagaaggacgataactattatgttggaattattcggaaaggcgccaagattaatttcgatgatacccaggccatagctgataatacagataattgcatatttaagatgaactatttcttacttaaggatgcaaagaaatttatccctaaatgcagcatacaattgaaagaagttaaagctcacttcaagaaatcagaagatgattacatactctctgataaagagaagttcgcttctccgttggtcatcaagaagtcaacgttcctattggcaaccgcacatgttaaaggtaagaaaggtaacatcaagaaatttcagaaagaatatagcaaagagaatccaaccgaatatcgaaattctcttaacgagtggatcgcattctgtaaagaatttttaaagacctacaaggctgctacaatatttgatataacaactctcaagaaggcagaggaatacgcagatatcgttgaattctacaaggacgttgacaatctttgctataaattggaattctgcccgatcaagactagtttcatagagaacctaatagataacggagatctctatttgttccgtattaacaacaaagacttctcttctaagagtactggaacaaagaacttgcatacattatacctccaggcaatcttcgacgaacgtaatctaaataatcctaccatcatgcttaatggaggagctgaacttttctacagaaaggagtctatagagcagaaaaatagaatcacgcataaggctggatcaatcctggtcaacaaagtctgcaaggatggcacttcgttggacgataagatccgtaatgaaatttaccagtatgagaacaaatttattgatacactttctgatgaggcaaagaaggttctacccaacgtcatcaagaaagaagcaacccatgacattactaaggataaacggtttacaagtgataaattcttcttccactgtcccttaactataaattacaaggaaggagatacgaaacagttcaataacgaagtgctgtctttcttacgagggaatcctgacataaatatcattggtatagaccgaggagagcgaaatcttatttacgttactgttataaatcagaagggagagatcctggatagtgtaagcttcaatacagttaccaacaaatcttccaagatcgaacaaaccgtagattatgaggagaagttggccgttcgggagaaggagcggatagaggcaaagagaagctgggacagtatcagtaagatagcaacgcttaaggagggttacttatctgctatcgttcatgagatttgtcttcttatgatcaaacacaatgcaattgtggtcctagagaatttgaacgcgggatttaagaggattcgaggtgggctttccgagaagagtgtgtatcagaaattcgagaagatgttgattaacaagcttaattacttcgtgagtaagaaggaatcggactggaacaaaccgagtggtctccttaatggtcttcagctatctgatcaatttgaatcatttgagaaacttggaattcaaagtggcttcatcttttacgttccagctgcttacacgtctaagattgacccaactacaggcttcgcaaacgttcttaatctttcgaaggtgcgcaacgttgatgctattaagtcattcttctctaacttcaatgaaatctcatactctaagaaggaggctctattcaaattcagcttcgatctagattccctttcaaagaaaggattctcttcgttcgtgaagttcagtaagtccaaatggaacgtttacacctttggtgaacgtatcatcaagcctaagaacaagcaagggtacagagaggacaagagaataaaccttacattcgagatgaagaagctccttaatgaatataaggtttctttcgatctggagaacaatctgattccaaacttgactagtgctaacttaaaggataccttctggaaggaactattcttcatattcaagactactttgcagttaagaaattcggtgactaacggtaaagaggatgtgttaatcagtcctgttaagaacgcaaagggagaattctttgtcagtggtactcacaataagactctccctcaggattgtgatgccaacggcgcttatcatattgctttgaaagggctcatgatcttggaacgtaataacctcgtgagagaagagaaggatacaaagaagatcatggccatttctaatgtggattggtttgagtatgtccagaaacggcgaggagtgttgtga

SEQ ID NO: 317 - DNA, 4005 bp, Artificial Sequence
  Description of Artificial Sequence: Synthetic polynucleotide
atgtcctcactgactaaatttacaaacaaatactctaagcagctcactatcaagaacgaactcatcccggttggtaagactcttgagaatattaaggagaatggccttatcgatggagatgaacaactaaacgagaattatcagaaggccaagattatcgttgatgacttccttagggacttcattaacaaagctcttaacaacacacagataggtaattggcgtgaacttgcagatgcattaaataaagaggatgaagataacattgagaaactccaggacaagattagaggtataatagtgagcaagttcgagacgttcgatctgttctcgtcatattcgatcaagaaggacgaaaagatcattgacgatgataacgacgttgaagaggaagagctagacttgggaaaaaagaccagttcgtttaagtatatattcaagaagaatctgttcaagcttgtattgccgtcctaccttaagacgaccaaccaagataagctaaagatcatcagttctttcgataatttcagtacatacttccggggcttcttcgagaatcgaaagaacatattcaccaagaaaccaatcagcacatccatagcatacagaattgtacacgataattttcctaagttcttagataatatcagatgctttaacgtgtggcaaaccgaatgcccgcaactgattgtgaaagctgacaactatcttaagtccaagaatgtcattgcgaaggataagtcgttggctaactacttcaccgttggcgcctacgattactttctatctcagaacgggatcgacttctataataatattataggaggtttaccagctttcgcaggtcatgagaagatacaaggattaaatgaatttattaaccaagaatgccagaaagacagcgaacttaagtcgaaactcaagaatcgccatgcttttaagatggctgtgctgttcaaacagatcctctcagatagagagaaatcgttcgttatagacgaattcgagtctgatgcccaagtaatagatgcagtaaagaacttctatgctgaacaatgtaaggacaacaacgtgatcttcaacctgcttaatttgattaagaacatagcgttcctgagtgatgatgaactagacgggatatttattgaaggcaaatatctcagttccgtttcacagaaactctactctgattggtccaaattgagaaatgatattgaagactcggccaatagtaagcagggtaacaaagagctcgccaagaaaatcaagactaacaaaggagacgttgagaaggctattagtaaatatgaattctctctttcagagttgaactccattgttcatgataataccaaattctctgacctcctgagctgcacactgcataaggttgcttctgagaagctcgtcaaagttaatgaaggagattggccgaagcatcttaagaacaatgaggagaagcaaaagattaaggaaccactagatgcactgttagaaatttacaatacactgctaatattcaattgtaaatcattcaataagaatggaaacttctacgtagactacgatagatgtataaatgaactttcctcggtagtttacctttacaataagacacgtaactattgtacaaagaagccttacaacactgataagtttaaacttaacttcaattctcctcaattgggagaaggcttcagtaaatcaaaggagaatgactgcttaacgctgctgtttaagaaggatgataactactatgtcggaatcattaggaagggtgcaaagatcaacttcgatgatactcaggcgatagctgataatactgataactgtatcttcaagatgaactacttcctcttaaaggacgcgaagaagttcattcccaaatgttcgattcagctcaaggaggtgaaggcccattttaagaagtctgaagatgactatatactttcagataaagagaagttcgcttcgcctttggttatcaaaaagagtacattcttgctcgcgacagcacacgttaaaggaaagaaaggtaatatcaagaagtttcagaaagaatactctaaagagaatccgacagaatacagaaattctctgaacgaatggatcgccttctgcaaggaattcctaaagacgtacaaggcagctacaatcttcgacattactacacttaagaaagccgaagaatacgctgacatagttgagttctataaagacgttgacaacctttgttataagctcgagttctgtcctattaagacatcattcatagagaacctaattgataacggtgatctctatctctttcggatcaacaataaagacttctctagtaagagtacaggaacaaagaacctgcacactctttatctacaggctatattcgatgaaaggaacttaaataatccgacgattatgctgaacggtggcgctgagctcttctatcgcaaggagagtatcgaacagaaaaacagaatcactcataaggcaggatcaatcttggtaaataaggtttgtaaagacggaacttccctcgatgacaagatcagaaatgagatataccagtacgagaacaaattcattgacaccctgtcggatgaggcaaagaaagtattacctaatgttattaagaaagaggctacccacgatattactaaagataagaggttcacttcagataagttcttcttccattgtccgcttacaataaactataaagaaggagataccaagcaatttaacaatgaagttctttctttcttacgcggaaacccagatattaatattataggtatagatcgaggtgagagaaatttaatctatgtcacagtgataaatcagaaaggtgagatattggatagtgtttcgttcaatactgtgaccaataaatcatcgaagatcgaacagactgtagattacgaagagaaactagcagttagagagaaagaaagaatcgaggcgaagaggtcttgggatagcatctcgaagatcgccactcttaaagaaggatatttgtctgcaattgtccacgagatttgtctcttaatgattaaacataatgcaatcgttgtccttgagaatcttaatgctggcttcaagaggattcgtggagggcttagcgagaagtcagtttaccagaaattcgagaaaatgttgatcaataaattgaactactttgtatccaagaaggaatccgattggaacaaaccttctggtctgctcaacgggcttcaattgtcagatcagtttgagtcgttcgagaagctgggaattcagtcgggatttatcttctacgtgcccgcagcctacacgtctaagatcgatcctactacgggatttgcaaacgtcttgaatttgtctaaagtccgtaatgtcgatgccataaagagtttcttctccaacttcaacgaaatctcgtatagtaagaaagaagccttgttcaagttctctttcgatttagattccctatccaagaagggattctcttcgtttgtgaaatttagcaaatctaaatggaacgtttacacgtttggagaacgcatcattaagccgaagaacaagcaaggataccgtgaggacaagagaattaatttgacgttcgaaatgaagaaattattaaacgagtataaagtttcatttgacctggagaataatttgataccgaacttgacaagtgcgaatctcaaggacacattctggaaagaactatttttcatctttaagactactcttcaactaagaaatagtgtcacaaatgggaaagaagatgttcttatttcaccggttaagaacgcaaagggagaattcttcgttagtggcacacacaataagacacttcctcaggactgcgatgctaacggagcttaccatattgctctcaagggacttatgatattggaaagaaacaatttggtgagggaggagaaagatactaaaaagattatggcaatctctaacgttgattggtttgaatatgtccagaagcgtcgtggcgtcctttaa

SEQ ID NO: 318 - DNA, 4005 bp, Artificial Sequence
  Description of Artificial Sequence: Synthetic polynucleotide
atgtcaagtcttactaagttcaccaataaatatagtaagcaactaacgatcaagaatgagctcattccagtgggaaagactcttgagaatataaaggagaatggtttgattgatggagatgaacaacttaatgagaattatcagaaagctaagattatcgttgatgatttcttgcgagacttcattaataaagctttgaataatacacagattggaaattggagagagctcgcagatgcgttaaacaaggaggacgaggataatatcgagaaactccaagataagatccgtggaatcatcgtgtctaagttcgagaccttcgatctcttcagctcctacagcataaagaaagacgagaaaatcatagatgatgataatgatgtggaagaagaagaactcgatctaggtaagaagactagtagcttcaaatacatctttaaaaagaatttgttcaagctggtacttccatcttaccttaagactactaaccaggacaagttaaagattattagctcctttgataatttcagtacatacttccgtggattcttcgagaacaggaagaatatattcaccaagaagcctatttctacatccatagcctaccggattgtccatgataacttcccgaagtttcttgataatatccgctgctttaatgtttggcaaacagaatgtccacagctgattgttaaagctgataattatttgaagagcaagaacgttattgccaaggataagtctcttgctaactacttcacagtaggtgcttacgattacttcctttcacagaacggaatagacttctataataacataattggaggactaccggccttcgctggtcatgagaagattcaaggattgaatgaattcataaaccaggaatgccagaaagatagtgaactgaaatctaaattgaagaatagacatgcatttaagatggccgtgctcttcaaacaaatcttatcagaccgggagaagtcattcgtgatcgatgaattcgaatctgatgctcaagtaatcgatgctgttaagaatttctatgctgaacagtgtaaggataataatgtgatcttcaatctcctaaatctcataaagaacatcgccttcctgtctgacgatgaactagacggcatcttcatagaaggtaagtacttatctagtgtttcccagaaactgtattccgactggtccaagcttaggaatgatattgaagatagtgccaactcaaagcaaggaaataaagagttggcaaaaaagattaagaccaataagggcgatgttgagaaggctatttctaaatatgaattctccttgagtgagttgaactccatagtccacgataacactaagttctctgatctcctctcttgtaccttacacaaggtggcatctgagaagcttgtgaaggttaatgaaggagattggcctaaacatttgaagaataacgaagagaagcagaagattaaagaaccgttagatgcgttgttagaaatctacaatactttattgatatttaattgcaaatcgttcaacaagaatggtaatttctatgtagattatgatagatgtataaacgagttgtcttctgttgtctatttgtataataagactcggaactattgtacaaagaaaccttacaacacagacaaatttaagttaaacttcaactcgcctcaactaggcgaagggttcagtaagagcaaagagaatgattgcctcaccctgctgttcaagaaggacgataactactacgtcggaattattagaaagggagcgaagatcaacttcgacgacactcaggcaattgcagataacactgacaactgtatattcaagatgaattacttcttgctgaaagacgctaagaaatttatccctaagtgttcaatccaactgaaagaagtgaaagcacactttaagaaatcagaagatgattatattctatcagataaggagaagttcgcttcacctttagtcattaagaagagcactttcttgttagcaacagcacacgttaagggcaagaaaggtaatatcaagaagttccagaaggaatattctaaggagaaccctactgaatatagaaactcgcttaatgagtggattgccttctgtaaagaattcttaaagacatataaggctgcaacgatctttgatatcactaccttgaagaaggctgaggaatatgcggatatcgtggagttctataaagacgtggacaacctgtgctataagcttgagttctgcccaattaagacatctttcatagagaacttaatagataatggtgatttatacttgttcagaataaataacaaggacttctcatcgaagagcactggcactaagaatctccatactctttatttacaagcgatattcgatgagaggaatctaaataaccctacaataatgcttaacggtggtgctgaactattctatcggaaggaatccattgaacaaaagaacagaatcactcacaaggcgggcagtatcctggttaacaaggtttgcaaggatggtacatctctcgacgataagattcggaacgaaatctaccagtacgagaacaagtttatcgacactctctctgatgaagctaagaaggtacttcccaatgtcatcaagaaagaggctacgcatgacatcactaaggacaagagattcaccagcgacaaatttttcttccactgtcccttaactattaactataaagagggtgatacgaaacaattcaacaatgaagtgctgtctttcttgcgcggcaatcctgacataaacatcatcggtattgacagaggtgaaaggaatctaatctatgtgacggtaattaaccagaaaggtgagatactcgattcagtctccttcaatacagtaactaacaagtccagcaagattgagcagacagtcgactacgaagagaagctcgccgtccgagagaaggagagaattgaggccaagcgttcatgggattctatttcaaagatcgcaacccttaaagagggatatttgtcagctatagttcatgaaatttgtttgctcatgatcaagcacaatgcaatagtagtactagagaatttgaacgcagggttcaagaggatcagaggaggcctgtctgagaaatcagtttaccagaagttcgagaaaatgcttattaataagcttaattactttgtgtccaagaaggaatctgattggaataagccttcaggacttctgaatggtcttcagcttagtgatcaattcgaaagtttcgagaaacttggaatccaaagcggattcatcttttatgtgcctgcggcctatacctctaagatcgatcccaccacaggcttcgcgaacgttcttaatttatctaaagtcaggaacgtggatgctattaagagtttcttctctaatttcaatgaaatctcatattcgaagaaggaagcattgtttaaattcagcttcgatctcgattcgctctcgaagaaagggttctcttcatttgttaagttctcaaagagtaaatggaatgtatacaccttcggagaaagaattatcaagcctaagaataagcagggatacagggaagacaagaggatcaatctgacatttgagatgaagaaactccttaatgaatataaggtttcatttgatcttgagaacaacctaatcccaaatcttacttctgctaatctgaaagacactttctggaaagaactattctttatatttaagacgaccttgcagttgagaaacagtgttactaacggtaaggaagatgttctaatatctccggtgaagaacgccaaaggtgagttcttcgtaagtggcacacataataagacacttccacaagattgcgatgctaatggagcttaccatatagcattaaagggattgatgatactggagagaaacaatcttgtgagggaagagaaggatacaaaaaagattatggctatttcaaacgtagattggtttgaatacgtccagaaacgtagaggtgtgctgtaa

SEQ ID NO: 319 - DNA, 4005 bp, Artificial Sequence
  Description of Artificial Sequence: Synthetic polynucleotide
atgagttcacttaccaagtttacaaataaatactcaaagcagcttacgattaagaatgaattgataccggtgggcaagactcttgagaatatcaaggagaatggattaatagatggtgatgaacaattgaatgagaattaccagaaggctaagataatcgtagatgatttcttgagagacttcataaacaaggctcttaacaatacacagataggaaattggcgtgaactagctgacgcccttaataaggaagatgaagacaatatagagaagttacaagacaagataagaggtatcatcgttagtaagttcgagacgttcgatttattctcgtcctattcaataaagaaggatgagaaaatcatcgacgacgataatgatgtggaagaggaggagctcgaccttggtaaaaagacaagcagtttcaaatacatattcaagaagaacttgtttaaactggtacttccaagctatttgaagacaactaaccaagacaaacttaagatcataagctccttcgataacttcagtacttatttccgtgggttcttcgagaatcgaaagaatatctttaccaagaagcctatatcaacctctatagcttatagaatcgttcatgataacttccctaaatttctagataacattcgttgtttcaacgtttggcagactgaatgtccacagctcattgtgaaagcagataattacctcaagagtaagaacgttatagctaaggacaagtctcttgctaattacttcactgttggtgcatatgattacttcttgtcccagaacggaattgatttctacaacaacattataggaggtctacctgcgtttgctggacacgagaagatccagggtctcaatgagttcattaaccaggaatgccagaaggactcagagcttaagtcgaagttgaagaatcgacatgcttttaagatggctgtactgttcaagcaaatcttgtctgatcgtgagaaatcattcgttattgatgagttcgaatctgatgctcaagtcattgatgctgtcaagaatttctacgctgaacagtgcaaggataataacgtgatcttcaatctgttaaacctgattaagaacatagcatttctgtctgatgatgaactcgatggaatctttattgagggtaaatatttaagctcagtgagtcagaaactctatagtgattggtcaaagctccggaacgatattgaggactcagctaatagtaagcagggaaataaggagcttgcaaaaaagatcaagacgaataaaggtgatgtagagaaggctatcagcaaatacgagttctcattgtcggagttaaacagtattgtgcatgataatacgaaatttagcgatcttctaagttgcactcttcacaaggttgcttcagagaagttggttaaggtgaatgaaggagattggcctaaacaccttaagaataatgaagagaaacagaaaatcaaggaaccgcttgatgcccttctggaaatttataacacccttctcatatttaactgtaagagcttcaacaagaacggtaatttctacgttgactatgatagatgtatcaatgaattatccagtgttgtttacctttacaataagactcgaaactattgtactaagaagccttacaatactgacaaatttaagctgaactttaattcacctcagctaggagagggattcagcaagagcaaggagaacgattgtttaacacttctgtttaagaaggatgataattactatgtgggcattattaggaagggagcgaagatcaactttgatgacacccaggctatcgcagataataccgataattgtatcttcaagatgaattacttccttctgaaagatgctaagaagtttatacccaagtgttctatccaattgaaggaggtgaaggctcatttcaagaaatcagaggatgattatatcctgagtgataaagagaaatttgcttctccgttggttatcaagaaatcgactttcctcctagctacggcgcacgtcaagggaaagaagggtaacattaagaaatttcagaaagagtactccaaagagaaccctacagagtatcgaaattcgttaaacgagtggatcgccttctgcaaagagttcctcaagacgtataaggctgcaactatcttcgacataactaccctaaagaaagccgaagagtatgctgatatcgtcgagttctataaagatgtggacaatctctgctacaaactagagttctgccctattaagacttcattcattgagaatttgatcgataatggtgatctatacctctttcgaatcaacaataaagacttcagttccaagagtaccggaacgaagaacctccacacgttatatcttcaagcgatctttgatgaaagaaacctaaacaacccaaccatcatgttgaatggcggcgctgaattattctaccgtaaagaatccattgagcaaaagaacagaatcacacataaagcagggtcaatcctcgtgaataaggtatgtaaggatggaacctctcttgacgataagattcggaacgaaatctatcagtatgagaacaagttcatcgacactctatccgatgaggcaaagaaagttctacctaatgtgatcaagaaggaagctacacacgatataactaaggacaagagatttacgagtgacaaattcttcttccattgcccactcactattaactacaaagagggagataccaaacaatttaacaatgaggtcttaagtttcctcagaggtaatcctgatatcaacattatcggtatcgatcgtggtgaacgcaatcttatatacgttactgtcattaatcagaagggtgaaatactcgacagcgtttcattcaatacggtaacgaataagagttcaaagatcgagcagacagttgattatgaagagaaactcgccgtaagagagaaggagagaatagaggccaagcgtagctgggattcaatatcaaagattgccacattgaaggaagggtacctctctgctattgtgcatgaaatttgtcttctgatgattaagcacaacgcaattgttgttctagagaatctcaacgctggattcaagcggataagaggcggactttcagagaagagcgtgtatcagaaatttgaaaagatgctcattaataaattgaactatttcgtgtcaaagaaggagtcagattggaataaaccttcaggtctactcaatggattacaacttagcgatcaattcgagtcctttgagaagttgggcattcaaagcggattcatattctacgtgccagctgcatatacctccaagattgatccaacaacgggattcgctaatgtgttgaatttgtctaaggtgagaaatgtggatgccatcaagtcattctttagtaacttcaatgagatctcatatagtaagaaggaagctctatttaagtttagtttcgatctagactccctctccaagaaaggtttctcgagcttcgtaaagtttagcaagtctaagtggaacgtttataccttcggtgaacggatcattaagccgaagaataagcaaggataccgagaggataagaggataaacctcacattcgaaatgaagaagctattaaacgaatataaagttagctttgatcttgagaacaacttgatacctaatctaactagcgccaatcttaaagacaccttctggaaagagttgttcttcatattcaagacaactttgcaattgcggaatagcgtcacgaatggtaaggaggatgtattaatctcgcctgttaagaacgctaagggagagttctttgtctcgggaactcataacaagactctcccacaagattgtgatgcaaacggagcctatcatattgcgctcaagggtttgatgatattggaaagaaataatctagttagggaggagaaagatacaaagaagattatggccatctcaaacgttgattggtttgagtatgtgcaaaagagacgaggagtgttataa

SEQ ID NO: 320 - DNA, 4005 bp, Artificial Sequence
  Description of Artificial Sequence: Synthetic polynucleotide
atgtcttcactcacaaagtttacgaacaaatatagcaagcaactaactattaagaacgaattgattcccgttggaaagacattagagaacatcaaggagaacggactaattgacggagatgaacagctaaacgagaattaccagaaggcaaagattattgtggatgacttcttaagggacttcatcaacaaggctctaaataatactcaaattgggaactggcgcgaacttgctgatgccttgaataaagaggacgaggacaatatcgagaagctccaagataagataagaggaatcattgtatctaagttcgaaacattcgatttattctcttcttactctattaagaaggatgagaaaataattgatgacgataatgatgtcgaggaggaggagcttgatcttggtaagaaaacttcgagtttcaagtatatctttaagaagaatctattcaaattggttctgccttcataccttaagactactaaccaagataagttaaagattatatcctctttcgataacttctccacttactttcgcggattcttcgagaatcgtaagaatatcttcactaagaaaccaatatctacgtccatagcgtaccggatcgttcacgataactttcccaagttccttgataatatccgttgcttcaacgtctggcaaacagaatgtcctcagctgatcgtgaaggctgataactatcttaagtccaagaatgttattgctaaagataaatcgctcgctaattactttacggtgggagcttacgattatttcttgtctcagaacggaatagacttctataacaatattatcggcggtctacctgcattcgctggacatgagaaaatccaaggtttgaacgaatttatcaaccaagagtgccagaaagactcagaacttaaatctaaattgaagaatcggcatgcttttaagatggctgtattatttaaacaaatattaagtgatagggagaaaagtttcgtgattgacgagttcgaatccgacgctcaagtcattgatgcagtgaagaacttctatgctgaacaatgtaaagacaacaacgttatctttaatttactaaaccttatcaagaatattgctttcttgtcagacgatgaattagatggcatctttattgaaggaaagtacctcagctcggtgtctcagaagctctattccgactggtcgaagttgagaaacgatatagaagattccgccaactccaaacagggtaacaaggaactagcgaagaagatcaagactaacaagggagatgtagagaaggctatatctaaatatgaattcagcttgagtgaactcaattcaatagtgcatgacaacaccaagtttagtgatctactatcatgtactcttcataaggtggcttctgagaaattagttaaagtcaacgagggagattggcccaagcacttgaagaacaatgaagagaaacagaagatcaaggaacccttagatgcacttcttgaaatctacaatacgctccttatcttcaactgcaagagcttcaacaagaatggcaatttctatgtagattatgatagatgtataaatgagcttagtagtgtggtctatttgtacaataagacaagaaactactgtacaaagaagccttataacactgacaagttcaaactcaacttcaattctccgcaactaggagaaggattctcgaaatctaaggagaatgattgcctcacccttctctttaagaaagacgacaattattacgtcggcataattaggaaaggcgcgaagataaactttgatgacacgcaagcgattgccgacaatactgataattgtatcttcaagatgaactacttcctcttgaaggatgccaagaaattcataccgaagtgctctattcagttgaaggaagttaaggctcacttcaaaaagagcgaggatgattacatattgagcgataaagagaaattcgcatcacctctggttatcaagaaaagcacattcttgcttgctacagctcatgttaagggaaagaaaggcaacattaagaagttccagaaagagtattccaaggagaatccaaccgaatacaggaatagccttaatgagtggatcgcattctgtaaagagttcctaaagacgtataaggctgccacgatctttgatatcacaacattaaagaaggcagaagaatacgcggatattgttgaattctacaaagacgttgacaacctttgttataaacttgaattctgcccgattaagacgagtttcatagagaaccttatcgataatggtgatctttacctctttaggatcaataataaggacttcagttcgaagagtactggaaccaagaaccttcataccttatatctacaagctatctttgatgaaagaaacctcaataacccaactattatgcttaacggaggcgcagagctattttaccgcaaggagtctatcgagcagaagaatcgaataactcataaggctggttctattcttgtcaataaggtctgcaaggatggaacatctttggatgacaagattagaaacgagatctaccaatatgagaacaaattcattgatactctttccgacgaggccaagaaagtgctacccaatgtgattaagaaagaggcaacacatgatattactaaggataaacggttcacatccgacaagtttttcttccattgtccacttactatcaactacaaagaaggcgatacgaaacaattcaataatgaggtgcttagtttcttaagagggaatcctgatattaatattatcggtatagaccgtggggaacgtaatcttatttatgttaccgtgatcaatcagaaaggagagatccttgatagtgtgtcgttcaacactgtgaccaataaatcaagcaagatcgagcagaccgttgattatgaggagaagttggctgttagagagaaagagagaatagaggctaagagatcgtgggattcgatctcgaagattgctacgttaaaggaaggttatctgagtgcaatagtgcatgaaatttgtcttctgatgatcaaacacaatgcaattgttgttcttgagaatctgaacgctggattcaagcgtattagaggaggattaagtgagaaatctgtttaccagaagtttgagaagatgctcataaataagctgaactactttgtatctaagaaggagagcgattggaataagccctcagggttacttaacggtctgcaactctctgatcagtttgagagcttcgagaagcttggtatccaatctggatttatattttatgtacctgccgcttacactagcaagattgatccaaccacaggtttcgcgaacgtcttgaacctgagcaaggtccgaaatgttgatgccattaagtctttcttctcaaactttaatgaaatctcttactctaagaaggaagcactcttcaaattctctttcgatcttgattccttgtccaagaaaggattctcctcgttcgttaaattctccaagagtaaatggaacgtctatacatttggcgaaagaattatcaagcccaagaacaaacagggatatcgagaggataagcgtataaatttgacgtttgagatgaagaagctgttgaacgaatataaagtctcattcgatttagagaacaacctgatcccaaatcttacttctgctaatctcaaagatactttctggaaagaactattctttatcttcaagacaacgcttcagttgcgtaacagtgtgaccaacggaaaggaagatgtactgatttctcccgtcaagaatgctaaaggtgagttctttgtcagcggcacacataacaagacactccctcaggattgtgacgctaatggagcttaccacattgctcttaaaggtcttatgattcttgaaagaaacaatttagttagggaggagaaggataccaagaagatcatggctatttctaatgttgattggttcgaatacgtacagaagcggcgtggtgtgttgtaa

SEQ ID NO: 321 - DNA, 4005 bp, Artificial Sequence
  Description of Artificial Sequence: Synthetic polynucleotide
atgtcatcacttactaaatttacgaataaatattccaagcaacttacaattaagaatgaactcattcccgttggtaagacgctagagaacataaaggagaacgggttaatagatggtgacgagcagttaaatgagaactaccagaaggctaagatcattgttgatgatttcttacgggactttattaataaggcattgaacaacactcaaattggaaactggcgtgagcttgcagatgcgttgaataaagaggacgaggataacatcgagaaacttcaagacaagataagaggaataatagtcagtaagttcgagacattcgatttgttctcaagttattcgattaagaaagacgagaaaattattgatgatgataatgatgtggaagaggaagaactggatctgggtaaaaagacatcatccttcaagtatatcttcaagaagaacctctttaagctagtgttaccttcttatttaaagactactaatcaggacaagctcaagattataagctcatttgacaacttcagtacctatttccgtggtttcttcgagaacagaaagaatatctttacgaagaagccaattagtaccagtatagcctacaggatcgtacacgataacttcccaaagttccttgataacatcagatgcttcaacgtatggcagaccgagtgtccacaattaattgttaaagcggacaattatctgaaatcaaagaacgttatagctaaggataagtctctcgccaattacttcactgttggtgcatatgattacttccttagtcagaacgggatcgacttctataataatattattggcggcctacctgctttcgctggtcatgaaaagatccaaggattaaatgagttcattaaccaagagtgtcagaaagatagcgagctcaaatctaaactcaagaataggcatgcatttaagatggcggtgctgttcaagcaaatactatccgacagagagaaatctttcgtgatagacgaatttgaatccgatgcacaggttatcgacgcagtcaagaacttctatgccgaacagtgtaaagacaacaacgtcatcttcaacctcctaaacctaataaagaatattgcgttccttagtgatgatgagttagatgggatcttcattgaaggtaagtatctctctagcgtgtctcagaagctctactctgactggtctaagctccgaaacgatattgaggattctgctaatagtaaacagggaaacaaggagttggccaagaagataaagaccaacaaaggtgatgtggagaaggccatttctaaatatgagttctccctttctgaacttaattccattgtccacgacaacacgaagttctctgatctcttgtcttgtacgcttcataaagtagcatccgagaaattggtgaaggtgaatgaaggagattggccgaagcacttaaagaacaacgaagagaaacaaaagataaaggagccactcgatgcattacttgagatttacaacaccttgttgatctttaattgtaaatcattcaacaagaacggtaatttctatgtagattatgatcgttgtataaacgaactttcatcagtcgtgtacctttacaataagacccgtaattattgcactaagaagccgtacaatactgacaaattcaaactcaacttcaactcacctcaattaggcgaaggtttctcaaagtctaaggagaacgattgcctcaccttactctttaagaaagatgacaattattatgttggcattattaggaaaggtgcaaagattaacttcgacgatacgcaggctattgccgacaataccgacaactgtatcttcaagatgaattacttcctcttgaaggatgccaagaaattcatccctaagtgtagcatccaactgaaagaggttaaagcccacttcaagaagagcgaagatgattacattctatcggacaaggagaaatttgctagtccactggttataaagaagagtacattcttgttggccacggctcatgtgaaaggcaagaagggcaacataaagaagtttcagaaggagtattctaaggagaaccctactgaataccgaaactcactaaatgaatggattgcgttctgcaaagaattcctaaagacttataaagctgctactatcttcgatattactactcttaagaaggcggaggaatatgctgacattgttgaattctacaaggatgtggacaacctttgctacaaactggagttctgtcctatcaagacctcattcatcgagaaccttattgacaatggtgatttatacctcttccgtatcaataacaaagatttctcaagtaagtccacaggaactaagaacctccataccctgtatttgcaagcaatatttgacgaaaggaatctcaataaccctacgattatgttaaatggaggtgctgagcttttctacagaaaggaaagtatcgaacagaaaaatcgtattacgcataaagcaggatctatacttgttaacaaagtttgcaaggatgggacgtccctcgatgacaagatcaggaatgaaatataccaatatgagaataaattcatcgataccctttcagatgaggcgaagaaagttcttcccaacgtgatcaagaaggaggctacacatgatataaccaaagacaagagatttacaagtgataagttcttctttcattgcccgctgactattaattataaagaaggagacacaaagcaattcaacaatgaagttctctcgttcttgagagggaatcctgacattaacatcatcggtattgatcgaggtgaaagaaaccttatatatgttacagtaattaaccagaaaggtgagatattagattcggtttcatttaatacagttacaaataagagtagcaagattgagcagactgttgattacgaagagaagctggctgttagagagaaggagaggattgaagcgaagcgaagctgggattctatttcgaagatcgctactctgaaggaaggatatctttctgctattgtacacgaaatttgtttgcttatgatcaagcataatgctatcgtagtgcttgagaatttaaatgctggcttcaagcgtatacgcggggggttgtcggagaagtcggtttaccagaaattcgaaaagatgcttataaataaattaaactacttcgtctctaagaaggaatctgattggaacaaaccttccggactattgaacgggcttcaactgagtgatcagttcgaatctttcgagaaattaggaatccagagcggttttatcttctacgttccagctgcatatacctcaaagattgacccaacgactggatttgctaatgttctaaacctctctaaggtccgcaatgtcgatgctattaaatcttttttctcaaatttcaacgagatttcatattcaaagaaagaagctttatttaagttctcgttcgatttagatagcctgagcaagaaaggcttcagcagctttgttaaattctcgaaatccaagtggaatgtttacacctttggcgagcgtattattaagccgaagaacaagcagggatatcgagaagacaagcgtattaatttgacatttgaaatgaagaagcttcttaatgaatataaagtatccttcgatctggagaataacttgattcctaacttaacatcagcaaatcttaaggacactttctggaaggaattattcttcatcttcaagacgactctacagttgagaaattcagtgactaatgggaaggaggacgtccttattagccccgtaaagaacgcgaagggtgagttctttgtgtccgggacccataacaagacgttgccacaggactgcgacgcgaatggcgcatatcacattgccctaaagggtcttatgattctagaacgcaacaatttggttcgtgaagagaaagatacgaagaagatcatggcgattagtaacgttgattggtttgaatatgtgcagaagagacgtggtgtgttgtaa

SEQ ID NO: 322 - DNA, 4005 bp, Artificial Sequence
  Description of Artificial Sequence: Synthetic polynucleotide
atgtcctcattaacgaaattcacgaataaatattcaaagcaactgactataaagaatgagcttattcctgtcggcaagacactggagaatattaaggagaacggtttaattgatggtgatgagcagcttaatgagaattaccagaaagccaagattattgttgacgatttccttcgggatttcataaataaggcgcttaataacacccaaatcggcaattggagggaattagccgatgccttgaacaaggaagacgaggataatatagagaagctccaggacaagatccgtggaatcattgtctctaaatttgagacattcgatttgttctcaagctactcaataaagaaagacgagaaaattattgatgatgataacgacgttgaggaagaagaactagacctcggtaagaagacgtcaagcttcaagtatatattcaagaagaacttgttcaagcttgttctcccgtcatatctgaagactacgaaccaagataagttaaagatcatttcttcgttcgataacttctctacatacttccgaggattctttgagaacagaaagaatatcttcacgaagaagcccatttcaacttcaatcgcttaccggatagttcacgataactttcccaagttcctcgacaatattaggtgtttcaacgtctggcaaacggaatgtccacagttgattgttaaggcagacaactacttaaagtcgaagaatgtgatcgcgaaggacaagtctcttgcaaattacttcacagttggagcttatgattactttctgtcccagaacggtatcgacttctataacaacattataggtggattaccagcgttcgcgggtcacgagaaaatccagggtctcaacgaattcattaatcaagagtgccagaaagatagcgaactgaagagtaagttaaagaacaggcatgcgtttaagatggccgtgctctttaagcagattctctctgatagagagaagtccttcgtgatcgacgagttcgaaagtgatgcgcaggtgattgatgccgtcaagaacttctatgccgaacagtgtaaggataacaacgtgatcttcaacctcctcaatttgattaagaatatagcgttcctctctgatgatgaattggatggtatattcattgaagggaaatacttgagtagcgtgtctcagaaattgtattctgattggagcaagctgcgtaacgatatcgaggactcagcaaacagtaaacaaggaaacaaggaactcgccaagaagatcaagaccaacaagggcgatgtggagaaagcaattagcaagtacgagttcagtctttcagaactaaactctattgttcatgataacacaaagttctcagatttgttatcttgcacgttgcataaagtggcctcggagaagcttgttaaggtaaatgagggagactggcccaaacatttgaagaacaacgaagagaaacaaaagattaaggagccattggatgccttgttggagatttacaacaccctattaatcttcaactgtaagtcattcaataagaatggaaacttctatgtggattatgataggtgtattaatgaattatcatccgtagtttacttgtacaataagacaagaaattattgtacaaagaagccttataatactgacaagtttaaattgaactttaactctcctcagctaggtgaaggattctctaagagtaaagagaacgattgtctaactctgctctttaagaaagatgataactattatgttggaattatccggaaaggtgccaagatcaatttcgatgatactcaggccatcgcggataacactgataattgtatattcaagatgaattactttctactcaaagatgcgaagaaatttattcctaagtgtagcattcaattgaaagaagttaaggcacatttcaagaaatccgaagatgattacatcctctccgacaaggagaagtttgcatctcctcttgtgattaagaagtctaccttcctgttggcaactgctcacgtaaagggtaagaagggcaacatcaagaagttccagaaagaatactcgaaggagaatccaactgaatacagaaattcacttaacgaatggatagctttctgcaaagaattcttaaagacttataaagcggctaccatcttcgatattaccacattgaagaaagccgaagaatatgcagatatcgtagagttctataaggacgttgataacctgtgttacaagttggaattctgcccaattaagacctctttcatcgagaacctgatagacaacggtgacttatatttgtttagaataaacaacaaggacttctcaagtaagtcaaccggcactaagaacttgcatacactttatctccaggcgatctttgacgagagaaacttgaataacccaaccatcatgctaaacggaggagctgaattattctacaggaaggagtcgattgagcagaaaaaccggattacacacaaggctggttcaatccttgttaacaaagtttgcaaggacggaacatctctggatgataagatcaggaatgaaatctaccaatatgagaataaattcattgacactctttctgacgaggccaagaaggttctacctaatgtgatcaagaaggaagctactcacgacatcacaaaggacaagaggttcacatctgacaagttcttctttcattgccctctcaccatcaactataaggaaggtgatacaaagcagttcaacaatgaagtcctttcgttcttgcgcggcaatccggatataaacattattgggatcgacagaggagagcgtaacttgatatatgttacagttattaatcagaagggagaaatcctagattctgtttcattcaataccgtcactaataagagtagcaagattgaacaaacagtcgactacgaagagaaattagctgttcgtgagaaagaaaggatcgaggcgaagagatcatgggattctatctcgaagattgcaacattgaaggaaggatacttatctgcaatcgttcacgaaatatgtctattaatgattaaacataatgctatcgttgttctagagaatttgaacgcaggcttcaagaggattagaggtggactttccgagaagtcagtgtaccagaaattcgagaaaatgttgattaacaaactaaattactttgtgagcaagaaagaaagcgactggaacaaacctagtggtttacttaacggtctccaactatctgatcagttcgaaagtttcgagaaattaggaattcagagcggattcatattctacgttccagctgcttacacctccaagatagacccgactaccggcttcgcaaacgtgctcaatctttccaaggttagaaacgtagatgctataaagagttttttctccaacttcaacgaaatttcttacagcaagaaagaggcactattcaaatttagcttcgatctcgactctttgtctaagaagggattcagttcatttgtgaagttctcaaagtctaagtggaacgtttacacatttggagaacgaataattaagccgaagaataaacaaggttatagagaggacaagagaataaacctcactttcgagatgaagaaactcctaaatgagtacaaggtaagtttcgatctagagaataacctgataccaaacttaacaagcgcaaatctgaaggatacattctggaaggagctcttctttatctttaagactactcttcagcttaggaacagtgttacaaatggcaaggaagatgtgttgatatcaccggtcaagaatgcaaagggcgaattctttgtgtcaggaactcataacaagacccttccacaggattgtgatgcaaacggagcttatcatatcgctttaaagggattaatgatactcgagagaaataatttggtcagagaggagaaagacaccaaaaagattatggctatctcaaatgtagattggtttgaatatgtccagaaaagaagaggagtattgtga

SEQ ID NO: 323 - DNA, 4005 bp, Artificial Sequence
  Description of Artificial Sequence: Synthetic polynucleotide
atgtcaagtctgactaaattcacaaataagtattctaagcagctcactataaagaacgaactcatacccgtgggcaagactctggagaacattaaagagaacggattaatcgacggtgatgagcagctcaatgagaactatcagaaagccaagatcattgtggatgactttctacgagactttataaacaaagctctaaataacactcaaattggcaactggcgcgagctggcagacgcattgaataaggaagatgaggacaacatcgagaagctgcaggacaagatccggggcatcatcgtgtcaaagttcgaaacctttgatctgttcagtagttattccataaagaaagacgagaaaattattgacgacgacaacgacgtggaggaggaagaattggacctgggcaagaagaccagcagctttaagtacatcttcaaaaagaatctcttcaagctcgtgctgccatcctacttaaagactaccaaccaggataagctaaagatcatcagctccttcgacaatttcagtacttatttcagaggcttctttgagaatcgcaagaacatatttaccaagaagcccatttctacatccattgcttataggattgtccacgataacttcccaaagttccttgataacatcagatgcttcaatgtatggcagacagagtgccctcagctcatagtcaaggccgacaactatctgaagtcgaagaacgttatcgcaaaggacaaatcactggctaattatttcaccgtgggcgcatacgattatttcttaagtcagaacggaatcgacttctacaacaatattattggaggcttgcccgcgttcgcaggacatgaaaagattcagggtcttaacgaattcatcaatcaggagtgtcagaaggatagtgagctgaagagtaagcttaagaacagacatgcattcaagatggcggtgctgtttaagcagattctgtccgacagagagaaaagctttgtgattgacgagtttgagtccgatgcacaggtgattgacgccgtcaagaacttctacgccgaacagtgtaaagacaataacgtgatctttaacctgctgaacctgattaagaacatagctttcttaagtgatgatgaacttgacggcatcttcatcgaaggtaagtacctgagttcagtttcccagaagttgtacagtgattggagcaagctacgtaatgatatcgaggattccgccaactccaagcaaggcaataaagagctagcaaagaagatcaagacgaataagggagacgtagagaaggctattagcaagtatgagtttagcctgtcagagcttaactcaatcgtccatgacaacactaaattctctgatttattatcatgtacgctacacaaagtggcgtctgagaagctcgtcaaggttaatgagggcgactggcccaagcatctcaagaataatgaagagaagcagaagattaaggaacctcttgacgccctccttgaaatttacaacactctgctgatattcaattgtaagtcattcaataagaacggaaacttctatgtcgattacgatcgttgtatcaatgaactctcctctgtggtgtacctctacaataagacacgcaactactgcacgaagaaaccttacaatactgacaaattcaagctcaatttcaactctccacagctgggagaaggctttagtaagtccaaggagaacgattgcttaacactgctcttcaagaaagacgacaactactatgtaggtatcatacgaaagggcgcgaagatcaactttgatgacacccaagccattgcagacaacactgataattgtatatttaagatgaattacttccttctgaaggacgccaagaaatttatccctaagtgttctatccaattaaaggaagtgaaggcccacttcaagaagtccgaggacgactacatcctgagcgacaaagagaagttcgctagtccactcgtgattaagaagagcaccttcctccttgccacagctcacgtgaaagggaagaaaggaaacataaagaaatttcagaaagaatactctaaagagaatccaaccgagtataggaacagcctcaatgaatggatcgcattctgtaaggagttccttaagacctataaagctgcaacaatcttcgatatcaccacactgaagaaagcggaggagtacgccgatatcgtggaattctataaagacgtggataacctgtgttacaaactggagttctgtcctatcaagaccagtttcatcgagaatctcattgacaatggagacctgtatctgttccggattaataacaaggatttcagctctaagtctacgggcacaaagaacctgcatacactgtacctgcaagcaatctttgatgaacgtaacctgaacaacccaacaatcatgttgaacggaggggccgaactgttctaccgcaaagagtctattgagcagaaaaatcgcatcacacataaagccggcagcatactagttaataaagtctgcaaagatggcacttcattggacgataagattagaaacgagatatatcagtacgagaacaaatttattgacaccctgagtgacgaggccaagaaagtactcccaaacgtcataaagaaggaggcaacccatgacattactaaagacaagaggtttacttccgataagttcttcttccattgtccactcacaatcaactacaaggagggcgacacaaagcagttcaataacgaagtgctgagcttcctgagaggcaatccggacatcaacataatcggaatcgatagaggagaacgcaacctcatatatgtaactgtgataaaccagaaaggagagatcctcgattccgtgtccttcaacaccgtgaccaacaaatctagcaagatcgaacagactgtggattacgaagagaagctggcagttagagagaaggagcgtatagaagccaagcggagttgggactccatttctaagatcgctactctcaaggaaggatacctctctgctatagtccatgaaatctgcctgctgatgatcaaacacaacgctattgtggtgctagagaacctgaacgcagggtttaagaggattcggggtggcttgtctgagaaatccgtgtatcagaaatttgagaaaatgctcatcaacaaactaaactacttcgtctctaagaaagaatccgattggaacaaaccatccggtctccttaatggactgcagctctccgaccagtttgaaagctttgagaagctagggatccagtctgggtttatattctatgttcccgccgcatatactagcaagattgatccaacaactgggttcgccaatgtccttaacctgagcaaggtccgcaacgtggatgccatcaagtctttcttctcaaatttcaatgagatatcttatagtaagaaagaagcattgtttaagttctcatttgacctggattccttaagcaagaagggcttctcttcctttgttaaattctcgaaatccaagtggaatgtctataccttcggcgagcgcatcatcaaaccaaagaataaacagggctaccgagaagacaagagaataaacctgacattcgaaatgaagaagctgctgaacgagtataaagtgtccttcgatcttgagaacaacttgatcccaaacttgacctccgctaacctcaaagatactttctggaaggagcttttctttatatttaagactaccctgcaattgagaaattctgtcacaaacggcaaggaggacgtgttaatcagcccggtcaagaatgccaaaggcgaattcttcgtgtctgggacgcataacaagacactgccgcaggactgtgatgccaacggcgcgtatcacattgctctcaaaggactgatgattctcgaacgcaacaacctagtgagagaggagaaagatacgaagaagatcatggccataagtaacgtagactggttcgagtatgtccagaagaggcgaggtgtcctatag

SEQ ID NO: 324 - DNA, 4005 bp, Artificial Sequence
  Description of Artificial Sequence: Synthetic polynucleotide
atgagtagccttacaaagttcactaataagtatagcaaacagctgactatcaagaacgaactgatacctgtcggaaagaccctggagaatattaaggagaacggcctgattgacggcgacgaacagctgaatgagaactatcagaaggctaagataattgtggacgactttctgcgggacttcataaataaggcactgaacaatacacagattggaaattggagggaactcgcagatgcattaaataaagaagatgaggataacatcgagaagctacaagacaagattagaggcatcatcgtgagcaaattcgagaccttcgatttattctcctcctacagcataaagaaagatgagaagattatcgatgatgacaacgatgtggaagaagaagagctcgatctgggaaagaagacatcatctttcaaatatatatttaaaaagaacctgttcaagctggtactgccctcttatctaaagaccacgaaccaggataagttaaagatcatcagtagctttgataacttcagcacgtacttccgcggtttctttgagaaccggaagaacatctttactaagaaacctatcagcaccagcattgcctaccggatcgtgcatgacaatttccctaaattcctggacaatattcgatgtttcaacgtgtggcagaccgagtgtcctcagctcattgttaaggccgataactacctcaaatctaagaatgtaattgccaaggacaaatcgctggctaactatttcaccgttggagcctacgactacttcttgagccagaacggcattgatttctacaataatatcatcggcggcctccctgcatttgccggacatgaaaagatacagggcctgaatgaatttataaatcaagaatgtcagaaggattctgaattaaagagtaagctaaagaatcgtcacgcgtttaagatggccgtgttatttaagcagatcttgagcgaccgtgagaagagcttcgttatcgacgagtttgagagcgatgctcaagtcattgacgccgtgaagaatttctacgccgaacagtgtaaggataacaacgttatattcaaccttctgaatctcataaagaatatagcgttcttgtccgatgatgagctggacgggatctttatcgaaggtaagtacctttctagtgtgtcacagaaactttacagcgactggagcaagctcagaaacgatatcgaagacagtgccaattccaaacagggcaacaaggaattggcgaagaagataaagacaaataaaggtgatgtggagaaagcaatctccaagtacgaattctccctaagcgagctgaacagcattgtgcacgacaatacgaagttctccgaccttctatcatgcaccctgcacaaagtcgcgtccgagaaactggttaaggttaacgaaggtgactggcccaagcacctgaagaataatgaagagaagcagaagattaaggaacccttggatgcccttctggaaatttataataccctgctgatatttaactgtaagtccttcaacaagaatggcaacttctatgtggactatgacagatgtatcaacgaactctcctccgtggtttacctgtacaacaagaccaggaattattgcaccaagaagccttataacaccgacaagtttaagctgaacttcaattcaccgcaattaggcgaaggattctcgaagagcaaggagaacgattgtctgacactgctgttcaagaaggatgacaattactatgtgggcattataaggaagggcgcaaagatcaacttcgacgatactcaagcaattgccgacaacactgacaactgcatatttaagatgaattatttccttctgaaagatgccaagaagttcattcctaaatgtagtatccaattgaaagaagtgaaggctcattttaagaagagtgaagacgattacatcctgagcgataaagagaagttcgccagtcctttggtgatcaagaagtcaaccttcctgctcgcgaccgcccatgtcaagggaaagaagggcaatatcaagaagttccagaaggagtacagtaaagagaatcccacggaataccgaaacagcctcaacgaatggatagcgttctgtaaggaatttctgaagacgtacaaagccgccacgatatttgacataaccaccctgaagaaagcagaggaatatgccgacatagtcgagttctacaaggacgtagacaatttatgctataaactggaattctgccctatcaagaccagctttatagagaacctgattgataacggagatctttatctgtttcgtatcaataacaaggacttctcaagcaagagcacgggtacaaagaacctgcataccttgtaccttcaggccatatttgatgagagaaacctgaataaccctacaatcatgctgaacggcggcgcagaactattctaccggaaggagagcattgaacaaaagaatcgcatcacccacaaagcgggctccatactcgtgaacaaagtgtgtaaggacggaacctctctcgatgacaagattcgtaatgagatctatcagtatgagaacaagttcattgacacactgtcagacgaagcgaagaaggtcctgccaaacgttataaagaaggaggctacccacgatatcacgaaggacaagcgtttcacaagcgataagttcttctttcattgcccgctgacgattaactacaaagagggcgatactaaacagttcaacaacgaagtactgtctttcctgagaggcaatcccgacatcaacattatcggaatagaccgtggggagcggaaccttatttacgtgactgtgatcaatcagaagggtgagatcctggacagtgttagcttcaatactgtcaccaacaagagctcaaagattgaacaaactgtggactacgaagagaaactcgccgttcgcgagaaggagcgcatagaagcaaagcgttcgtgggactcaatctcgaagatagccacactcaaggaaggctacctgtctgcaatcgtgcacgagatttgcctgctgatgatcaaacataacgccattgtcgtgcttgagaatctgaacgcgggcttcaaacggatacgaggtggcttaagcgagaagtcagtgtaccagaagtttgagaaaatgttgattaacaagttgaactactttgtgagcaagaaagagtcagattggaacaagccctcaggccttcttaacggcctccagctctctgatcagtttgaatccttcgagaaactgggaattcaaagtggcttcatcttctacgtccctgctgcctacaccagtaagatagatcctaccacaggcttcgcgaatgtactgaatctttccaaagttcgcaatgtggacgccatcaagtctttcttctcaaactttaatgaaatctcttactcaaagaaagaggcgttgttcaagttctcattcgacttggattcattgagcaagaagggcttcagtagtttcgttaaattctcaaagtctaagtggaatgtatacaccttcggcgagaggataattaaacctaagaataagcagggctatcgggaggacaagaggattaatctcacctttgagatgaagaagctcttgaatgaatacaaggtgagtttcgatttagagaacaacttgattccgaatctaacgtccgctaatctgaaagacaccttctggaaggaactattctttatattcaagactaccctacagcttcgcaactctgttactaacggcaaggaagacgtcttaataagcccggttaagaatgccaagggtgagttctttgtttccggcacccacaataagacacttccacaggattgcgatgccaacggagcctaccacatagctctcaaaggccttatgatactcgagcgcaacaacctcgtccgagaggagaaggataccaagaagatcatggccatatccaatgtcgactggttcgaatatgttcagaaacggagaggagtcttatag

SEQ ID NO: 325 - DNA, 4005 bp, Artificial Sequence
  Description of Artificial Sequence: Synthetic polynucleotide
atgtccagcttgacgaagttcactaataagtattcaaagcagcttactatcaagaacgagctcattccagtaggtaagaccttagagaacattaaagagaatgggctgattgatggagacgagcaactgaacgagaattatcagaaggcgaagatcattgtggacgatttcctcagagacttcataaataaagccctgaacaacacacagattggaaactggcgggagttggctgatgctcttaataaagaggatgaagacaacatcgagaagctgcaggataagattcgtggcatcattgtgagcaagtttgagacgttcgatctgttcagctcatattcaataaagaaagatgagaagataatcgatgatgacaatgacgttgaagaggaagagctcgatctaggaaaaaagacaagttccttcaagtatatattcaagaagaatctgttcaagctcgtgctgccgagttatctgaagacaacaaaccaggataagcttaagattataagcagcttcgataatttctcaacctacttccgcgggttctttgagaatcggaagaatatcttcaccaagaagcccatctccacatcaatagcttacagaattgtgcacgataatttcccgaagtttctggacaacatccgctgcttcaatgtgtggcagactgaatgccctcagttaattgtcaaagcagataactatctaaagagtaagaatgttatcgctaaagacaagtctcttgcgaactacttcaccgtcggcgcatatgattatttcttgtctcagaacggaatagatttctacaacaatatcataggtggtttaccagccttcgctgggcatgagaaaatccagggacttaacgaatttattaatcaggaatgccagaaagatagtgagctaaagagcaagttaaagaacaggcatgcgtttaagatggcagtcctgttcaagcagatactgtcagaccgtgagaaatcattcgtaatcgacgagttcgaatcagatgctcaggtgatagacgccgttaagaacttctatgccgagcaatgtaaggacaacaatgtgatcttcaatttgctgaatctcatcaagaatattgcattcttatcagacgacgaattagacggcatcttcatagagggtaagtacttatcttccgtctcccagaaactgtatagcgattggtccaagctgagaaacgacatcgaagattctgccaattccaagcagggcaacaaggaactggctaagaagatcaagactaataagggcgacgtggagaaggccatatcaaagtacgaatttagcttgagcgaactgaacagtatcgtccatgacaacactaagttctccgacttattatcctgcacactgcacaaggtggcgagcgagaaattggtgaaagtgaatgagggtgattggcccaagcatcttaagaacaatgaggagaaacagaagatcaaggaacctctggatgccctactggaaatatataacaccctcctgatcttcaattgcaagtcgttcaataagaacgggaacttctatgtggattacgaccgatgtatcaacgaactgtcgagtgtagtgtatttgtataataagacgaggaattactgcaccaagaaaccttataacacggataaatttaagcttaacttcaactctccacaattaggcgaaggcttctccaagtctaaagagaatgactgcctcaccttactgtttaagaaagatgacaactactacgtcgggattataagaaagggagccaagattaacttcgacgatactcaggctatagcggacaacactgataattgtatatttaagatgaactatttcctgcttaaggacgcgaagaagttcatccctaagtgtagtatccagctaaaggaggtgaaagcacactttaagaaatcagaagacgattacatactctctgataaggagaaatttgctagtcctttggtaatcaagaaatctactttcttgctcgctactgctcacgtgaaggggaagaagggaaatatcaagaagtttcagaaagaatactccaaagagaaccctaccgaataccgcaactcactcaatgagtggatcgcgttctgtaaggaatttctaaagacctataaagccgcgacaatatttgacatcactactttaaagaaagccgaggagtatgctgatattgtagagttctataaggatgttgacaatctctgctacaaacttgaattctgcccaatcaagaccagtttcatagagaacctcattgataacggcgatctgtacttgttccgcatcaacaacaaggactttagctctaagagtacaggcaccaagaacttgcacacgctgtatctgcaggcaatcttcgatgagagaaacttgaacaatccgaccatcatgctcaatggtggtgccgaactgttctatcggaaagaatccatcgagcagaagaatcggatcactcacaaagcaggatcaatcctggtcaacaaggtgtgtaaagacggtacctcgctggacgataagattaggaacgagatttatcagtacgagaacaaatttatcgatacactctccgatgaagctaagaaggtgctccctaatgttattaagaaggaggcaactcacgacatcactaaggataagcgatttacttcagacaagttcttcttccactgccctctgaccatcaactacaaggaaggcgataccaaacagtttaacaatgaagtcctcagcttcctgagaggtaaccctgatatcaacattattggaatcgatagaggagagcgtaacctcatctatgtgaccgttattaatcagaagggagaaattctcgactccgttagctttaacaccgtgactaacaagtcttcaaagatagaacagacagtggattacgaagagaaactggcggtgagagagaaggagagaatcgaggccaaacgatcatgggattcgattagtaagatagctacgcttaaggagggctacctcagtgccatcgtacacgaaatctgtttgcttatgataaagcataacgccattgtcgtgttagagaaccttaatgccggttttaagagaattcgaggtggtctgtccgagaagtcagtataccagaaattcgagaagatgctgattaacaagttaaactacttcgtgtcgaagaaggaatcggactggaataagcctagcggactgctgaatggattgcaactgagtgaccagtttgagagctttgagaagttaggtatccagtcgggcttcatattctatgtccctgctgcctatacatctaagattgatccgactacgggattcgccaacgtcctgaatctctccaaagtacggaacgtggatgccatcaagagcttctttagcaactttaacgaaatcagctacagtaagaaggaggccctgttcaaatttagtttcgacctcgatagtttgagtaagaagggtttcagctccttcgtcaagtttagtaagtctaaatggaacgtgtacacgtttggcgaaagaattataaagcctaagaataaacagggctacagggaggataagcgcatcaacctgaccttcgagatgaagaagctgctgaacgaatataaggtgagtttcgatcttgagaataacctcattcctaacctgacgtctgctaatctcaaagacaccttctggaaggaactcttctttatcttcaagaccactctgcagttgcggaacagtgtaactaatgggaaggaagatgtgcttatcagccctgtgaagaatgccaaaggtgaattctttgttagcgggacccataacaagactctgccacaagactgcgacgctaacggcgcatatcacattgctctcaagggactgatgatcttagagcggaataatctcgtgcgagaggagaaggacactaaaaagattatggctatatctaatgtggactggtttgaatatgtccagaagaggcgaggagtgctgtga

SEQ ID NO: 326 - DNA, 4005 bp, Artificial Sequence
  Description of Artificial Sequence: Synthetic polynucleotide
atgtcgtcgctgacaaagtttactaataaatatagtaagcaactcaccattaagaatgagttgatacccgtcggaaagaccttggagaacattaaggagaatggattgatcgatggagacgagcagctgaatgagaattatcagaaggctaagattatcgtcgacgacttccttagagacttcattaacaaagctttgaataatacgcagattggaaattggagagaattggctgatgccctgaacaaggaagacgaagacaatattgagaagctgcaggataagatccgcggaatcattgtctccaaattcgagacgttcgacctcttcagttcctacagtatcaagaaagacgagaagatcatagacgacgacaacgatgtggaggaggaagaactggacctaggtaagaagacttcttccttcaaatacatattcaaaaagaatctgttcaagctggttctgccatcctatctgaagacaaccaatcaggataagctgaagatcattagttccttcgacaatttcagcacttacttccgcgggttcttcgagaacaggaagaacatattcacaaagaagccaataagtacatcaatagcctacaggatcgtgcacgataactttcctaagttccttgataatatacggtgctttaacgtctggcagacagaatgcccgcaactgattgttaaagcggacaactacctcaaatcgaagaatgtcatagccaaggataaatcgttagctaactatttcaccgtgggtgcctacgactacttcctcagccagaacggtatagatttctacaacaacatcattggcggtttgcctgcgttcgccggccacgagaaaattcagggattgaacgaatttatcaatcaagaatgccagaaagattcagagttgaagtctaaattgaagaaccggcatgcatttaagatggccgtcctgtttaagcaaatactgtcggatagagagaaaagctttgtcatcgacgagtttgagtcggacgcgcaagtaatagacgcagttaagaatttctacgccgagcagtgcaaggacaacaatgttatatttaatctattgaacttgatcaagaatatagcctttctgagcgatgacgagctagacggtatctttattgaaggaaagtatctcagcagcgttagccagaagttgtatagcgattggagtaagctgcgtaacgacatcgaagacagcgctaactcaaagcaaggcaataaggagctggcaaagaagatcaagaccaacaagggcgacgtggagaaggcaatctcgaaatatgagtttagcctctctgaattgaactctatcgtgcacgacaacacaaagttctccgacctgctttcatgtaccctgcacaaagtggccagtgagaagttagtgaaggtcaacgagggtgattggcctaagcacctaaagaataacgaagagaaacagaagattaaagaacctctcgacgccctgctggagatctacaataccctattgatcttcaattgcaagagtttcaacaagaacggcaatttctacgtggattacgacagatgtattaatgaattatcttctgtggtgtatctgtacaacaagacccgcaattactgcacaaagaagccttacaacacagacaagttcaaattaaacttcaacagcccacagcttggcgaagggtttagcaagagcaaagagaacgattgcctgaccctgctgttcaagaaggatgacaattattacgtgggtataatcaggaagggcgctaagatcaacttcgatgacactcaggccatcgcagacaacactgacaactgcatatttaagatgaactacttcctgctaaaggacgccaagaaattcattccgaagtgctccatccagcttaaagaagtgaaagctcacttcaagaaatccgaggacgactatatcctcagcgacaaggagaagtttgcgtcacctctggtgataaagaagagcaccttcctcctcgctaccgcacacgtgaaaggaaagaagggaaatattaagaagtttcagaaagaatactccaaggagaatccaacagagtatcggaattctttgaatgagtggattgccttctgtaaggagttcctgaagacctataaagctgcgaccatattcgacatcacaacattaaagaaggctgaggagtacgccgacatcgtagaattctacaaagacgttgataatctgtgctataagcttgagttctgcccaatcaagaccagcttcatagagaatctgatagacaacggagatctctacctgttccgcattaataacaaggacttctcatccaaatctacaggcaccaagaatctccacaccctgtatttgcaagcgatattcgacgaaaggaatctgaataatccaaccataatgctcaacggtggagcggagttgttttatcggaaggagtcaattgaacagaagaatcgtatcacacataaggccgggtccatcctcgtgaataaagtatgtaaggacggcaccagtctggacgataagataagaaatgagatctaccagtacgagaataagttcatcgataccctttccgatgaagcaaagaaagtactgccaaatgtgattaagaaggaagctacgcatgacattaccaaagacaagcgtttcacctctgacaaattcttcttccattgtccgctcacgatcaactacaaggagggcgacacgaagcaattcaacaatgaggtcctgtctttcctcagagggaacccagacattaacataatcggaatcgacagaggagaaagaaacttgatctacgtgacggtcattaatcagaagggcgagatcttagattccgtgtccttcaacaccgttaccaacaagtcaagcaagatcgaacaaacagtggattatgaagagaagctcgccgtgagagagaaggaacgaatagaggcaaagcgatcctgggatagcatttcgaagatcgccaccttaaaggagggctacctctcagctatcgtgcatgaaatttgcctgttaatgattaaacataacgctatagtcgtgctggagaacctgaatgctggattcaagcgcataagaggcggactttcagagaagagcgtgtatcagaaattcgagaaaatgcttatcaacaagttgaactatttcgtgagcaagaaagaaagtgattggaacaagccatccggccttctaaatgggctgcagctttctgaccagttcgagagtttcgagaagttgggcatccagagcggtttcatcttctacgttcccgcggcctatacaagcaagatagacccaactacaggattcgcgaatgtgctgaatctatctaaagtccgcaacgttgatgctatcaagtcattcttctccaactttaacgaaattagctacagcaagaaagaggctctctttaaattctcctttgacctggactcgctgagtaagaaaggattctcaagcttcgtgaaattctccaagagtaagtggaatgtgtacacctttggcgagagaattattaaacctaagaataaacagggttatcgggaagataagcggatcaatctgacctttgagatgaagaaactgctgaacgaatacaaagtttccttcgacctggagaacaacttaatacctaatctgacttccgcgaatttgaaggacaccttctggaaggaactattcttcatctttaagaccaccttacagctgcgaaattctgttactaacggcaaggaggatgtacttatcagccctgtcaagaatgctaagggcgaattcttcgtatccgggacacacaataagactctgcctcaggactgtgatgccaacggagcctatcatatcgctctcaaaggccttatgatcctggaaagaaacaacctggtgcgtgaagagaaagataccaagaagatcatggcaattagtaacgtggactggtttgagtatgtacagaaacggcgaggagtcctttaa

SEQ ID NO: 327 - DNA, 4005 bp, Artificial Sequence
  Description of Artificial Sequence: Synthetic polynucleotide
atgagtagcttaacgaaattcaccaacaaatacagcaagcagcttacaatcaagaacgagctcatcccagtgggaaagacacttgagaatatcaaagagaatggcctgatagatggcgacgaacagctgaatgagaattatcagaaagcaaagattatagtagatgacttcctcagagacttcataaataaagcccttaataacacccagattggcaattggcgtgagttggcagacgctttgaataaggaggatgaagacaatatagagaagctccaagataagatacgtggcatcattgtgtccaagtttgaaactttcgatctcttcagctcctactccatcaagaaggacgagaaaataattgacgacgataacgatgttgaggaggaagaattggacttaggaaagaagacctcttccttcaagtacatctttaaaaagaacctgtttaagctggtacttccaagctatttgaagacaaccaaccaagacaaacttaagattatttcttcattcgataacttctcaacttatttcagaggtttctttgagaatcggaagaacatctttacaaagaaaccaatctcaacatccattgcctataggattgtccatgataacttccctaaattcctggacaatattaggtgcttcaatgtttggcaaaccgaatgtcctcagctcattgtcaaggccgataactacttgaagtcaaagaacgtgatcgctaaagataaatctctggccaattactttacggtgggcgcatacgattatttcctgagccagaacggaattgacttctacaataatataataggcggcctcccagccttcgccgggcacgagaagatacagggacttaacgaatttatcaaccaggagtgccagaaggatagtgaactgaagtccaaactgaagaatagacatgcgttcaagatggccgtcctcttcaagcagattctttccgatagggagaaaagctttgtgatcgatgaatttgagtcagacgcacaggttattgacgccgtaaagaacttctatgctgagcagtgcaaagataacaatgttatatttaacctactgaacctcatcaagaacatcgccttcctctccgatgacgagctcgacgggatcttcattgaaggcaaatacttaagtagcgtatctcagaagctctattctgattggagtaagctacgcaatgacattgaggactctgcaaattcaaagcaaggtaataaggaactggccaagaagattaagacaaacaagggtgatgtagagaaagcaatttctaagtatgaattctctttgagcgagctaaacagcattgtccatgacaacaccaaatttagcgatctgttgtcatgcaccctgcacaaggtggcgtcagagaaactggtaaaggttaacgagggagactggcctaaacatttgaagaacaatgaagagaaacaaaagataaaggaacccttggacgccctcctagagatctacaataccttgctgatattcaattgtaagtctttcaataagaatggcaatttctatgtggactacgaccggtgcattaacgagctaagctccgtggtatacctttacaataagacgcggaattattgcaccaagaaaccctataatactgataaattcaagctcaacttcaacagccctcaactgggagaaggtttctctaaatcaaaggagaatgactgtctgacccttctgttcaagaaagatgacaactactatgtgggcatcatcaggaaaggcgcaaagatcaacttcgacgatacacaggccatagcagataacaccgacaactgcatcttcaagatgaactacttcctgcttaaggacgcgaagaaattcattcccaagtgctccatccagctcaaagaagttaaggctcactttaagaagagcgaagacgactacattctgagcgataaggagaaatttgcctcgcccttggtgatcaagaaatccacgttcctgctggctacagcccatgtgaaaggtaagaaaggtaatattaagaagttccagaaagaatatagtaaggagaatcccacggagtataggaatagccttaacgaatggatcgcgttctgcaaagagtttcttaagacgtacaaggccgccactatctttgatatcacaacactgaagaaagccgaggaatacgccgacatcgtggagttctataaggatgtggacaacctttgttataaattggaattctgccctatcaagacctcatttatagagaacctgattgataacggcgatttatacttgtttcgcatcaataataaggacttcagtagtaagagtaccgggaccaagaacttgcacactctgtatctgcaagccatcttcgacgagcggaatctgaataatccaacaatcatgctgaacggcggcgcagagctattctaccgcaaagagtcaatcgagcagaagaataggattacacataaggcaggcagtattctggtgaacaaagtctgtaaagacggaacctcactggacgataagattagaaacgagatctaccagtatgagaacaagttcatcgataccctgagcgatgaggccaagaaagtgctgcccaatgtgatcaagaaagaggctacacatgatatcaccaaggataaacggttcacctctgataaattcttcttccactgcccactgacgattaattataaagaaggcgacactaaacagttcaacaatgaggtcttatcattcctcagagggaatcctgatattaatattatcgggatagacagaggagaaagaaacctgatatacgtgaccgttattaatcagaaaggcgagatcctggactctgtgtctttcaacactgtcacaaataagtccagtaagatcgaacaaaccgtagactacgaagagaaactcgctgtgcgcgagaaagagcggatagaagcaaagagatcctgggatagcatctcgaagatcgccacactcaaggaaggctacctgagtgctatagtccatgagatatgtctcttgatgatcaagcacaacgcaatcgtggtcttagagaacttaaatgcgggctttaagaggattcgtggcggtttatctgagaaatctgtgtatcagaaatttgagaagatgctcatcaataagcttaactatttcgttagtaagaaagagagcgactggaacaagccatccggactgttgaatggactccagctgagtgaccaatttgaaagcttcgagaaattgggtattcagtccggattcatattctacgtgccagccgcgtacacctctaagattgaccctacaaccgggttcgctaacgtcctgaacctgagtaaggtccggaacgtggacgcaatcaagagctttttctcaaatttcaatgaaatcagttactctaagaaggaagccctgttcaagtttagcttcgatctcgacagcctgagcaagaaaggcttcagctcattcgtcaaattttctaagagcaagtggaatgtgtataccttcggcgaacggataatcaaaccaaagaacaaacaaggttatcgcgaagacaagcgcattaacctcaccttcgaaatgaagaaacttctgaatgaatataaagtgtctttcgacctggagaacaacttgatccctaacctgacttctgcaaatctgaaggatacattctggaaagagttgttctttatcttcaagactactttacagctccgcaactctgtgaccaacgggaaagaagatgtgctcatctcaccagtcaagaacgctaagggcgagttcttcgtctctggaacccacaacaagaccctaccacaagattgtgatgctaatggcgcttatcatatcgccctgaagggactgatgatcttggagagaaataatttggtaagggaggagaaagacacaaagaagattatggccatctcaaatgttgattggtttgagtatgtgcagaaacgccgcggagttctctga

SEQ ID NO: 328 - DNA, 4005 bp, Artificial Sequence
  Description of Artificial Sequence: Synthetic polynucleotide
atgtcatccttaacaaagttcactaacaagtatagcaaacagctgaccatcaagaatgagctgattcccgtcgggaagaccctcgagaacattaaggagaatggtctgatcgatggtgatgaacagctcaatgagaattaccagaaagcaaagatcatcgtggacgacttcctgcgagacttcattaataaagccctgaacaacactcaaattgggaactggagggaactggccgacgccctcaacaaagaagacgaagataacatcgagaaacttcaggataagatcagagggattatagtgtccaagttcgagacatttgatctgtttagctcttactctatcaagaaagatgaaaagataattgacgacgataacgacgttgaagaggaagaactggatctcggtaaaaagacaagttctttcaagtatatatttaagaagaatctgtttaaactggtgctgccaagctacttgaagaccactaaccaggacaaactgaagattatttcatcgtttgataactttagtacttacttccgaggcttctttgagaatcgcaagaacatctttacaaagaaacccatcagtacctctattgcatacaggatcgtgcacgacaacttccctaagtttctggacaacattaggtgcttcaacgtgtggcaaaccgagtgccctcaattgatcgtgaaggctgataattatctgaagtcgaagaacgttatcgccaaagataagagcctcgcaaactatttcaccgtgggagcatacgactacttcctgtctcagaacggcatcgacttctacaataatatcattggagggcttcccgcatttgccggccatgaaaagatccagggtttaaacgagtttataaatcaggagtgccagaaggattcagaactcaaatccaagctcaagaataggcatgctttcaagatggcagtcctgtttaaacagatcctcagcgaccgcgagaagtccttcgtgatcgacgagttcgagagtgatgcccaagtaatcgacgccgtgaagaatttctacgccgaacaatgtaaggacaacaacgtcatctttaacctcctgaacttaataaagaatatcgcatttctttctgatgacgagctggacggtatcttcatcgaaggaaagtacctgtctagcgtatcccagaagctatattcggattggtccaaattgaggaacgacatcgaagactcagccaacagtaaacagggcaacaaggaactggcaaagaaaatcaagactaacaagggagacgtcgagaaagcaatcagcaagtacgagttctctctttccgaactgaatagtatcgtgcatgataatacgaaatttagcgatctgctcagctgcaccctgcataaggtggcttctgagaagttggtgaaggttaatgagggcgattggcccaagcatctcaagaacaacgaggagaaacaaaagatcaaagaaccacttgatgccctgctggagatttacaatacgttgctgatctttaactgcaagtcattcaataagaacggaaacttctacgttgactacgacagatgtatcaacgaattgagttcagtagtgtatctgtataacaagacacgaaattattgcacaaagaagccctataacacggacaagttcaagttgaactttaactcaccacaattaggagagggcttctccaagagcaaggagaatgactgccttactctgctgtttaagaaggatgacaattattacgtaggaattatccgtaagggcgccaagatcaacttcgatgatacacaggctattgccgacaataccgacaattgtatattcaagatgaattacttcctcctgaaagatgcaaagaagttcattcctaagtgcagtatccaactgaaggaggttaaagctcacttcaagaagagcgaggacgactacatcctgtcagataaagagaagttcgcgtcgccactggttattaagaaatccaccttcctactagccaccgcccatgtgaagggtaagaaagggaacataaagaagtttcagaaagagtactccaaagagaatcctacagaatacaggaacagcctgaatgagtggatagcattctgtaaagaattcctcaagacctacaaggccgctacgatcttcgacatcaccactcttaagaaagcagaagagtacgcggatatagtggagttctacaaagacgttgacaacctgtgctacaaattagagttctgtcccattaagacctccttcatcgagaatttgatcgataacggagacctgtacttgttccgcattaacaataaagatttcagttcaaagagtaccgggacaaagaacttgcacacactgtacttgcaggcgatattcgacgagcgtaacctgaacaatcctacaatcatgcttaatggcggcgcggagctcttttatcgcaaggagagcatagagcaaaagaacagaatcacgcataaggcagggagcatattggtgaacaaagtgtgcaaagacgggacaagccttgatgataagatccggaatgaaatttaccaatacgagaataaattcatcgacactctgtcagacgaggctaagaaggtactgcccaatgttataaagaaagaagccacacacgatataacgaaagacaaacggtttacgtccgataagttcttctttcattgtcctctgaccataaactataaagagggtgatactaagcagttcaataacgaagtcctaagcttcctgcgtggcaaccctgatatcaacattattggaatcgaccgtggcgagagaaacctcatttacgtgaccgttatcaaccagaagggcgaaattctggactctgtgtccttcaatacagtcaccaataagtcttctaagatagaacaaactgtggattacgaagagaaacttgcagtgcgcgagaaggaacggatcgaggcaaagcgaagttgggacagcatctcaaagatcgctactcttaaggaaggatacctgagtgcgatcgtccacgaaatctgcctcttaatgatcaaacacaatgccatagtggtcctcgagaacctcaacgctggcttcaagaggattcggggaggtttgtccgagaagtccgtctatcagaaattcgagaaaatgctgatcaataagttaaattacttcgtgtcaaagaaagagtcagactggaataaacccagtggcttgctgaacggcctgcagttgtccgaccagtttgaaagcttcgagaaactgggcatccagagcggatttattttctacgttcctgctgcctacacaagcaagatcgatcctacaaccggcttcgccaatgtactcaaccttagcaaagtaaggaatgttgatgctatcaagtccttcttctctaacttcaacgaaatcagctactccaagaaggaagcgttgtttaagtttagcttcgacctggatagtctgtcgaagaaagggtttagctcctttgtgaaatttagcaaatccaagtggaatgtgtacacctttggtgaacggatcattaagcctaagaataagcagggatacagggaagataagcggatcaacctcacctttgaaatgaagaagctcctgaatgagtacaaagtttccttcgatctcgagaacaacctcattcccaacctgacctccgcgaacttgaaggatactttctggaaagaactgttcttcatcttcaagaccacgctccagcttcgcaactccgttaccaatggcaaagaagatgtgctcatcagcccagtcaagaacgccaagggagagttctttgtgtcaggcactcacaataagactcttccgcaggattgtgatgccaacggtgcttaccacattgctctgaagggtttgatgattctcgaacggaacaatttagtcagggaggagaaagatactaaaaagataatggccattagtaacgtggactggtttgagtacgtgcagaagcggagaggagtcctctga

SEQ ID NO: 329 - DNA, 4005 bp, Artificial Sequence
  Description of Artificial Sequence: Synthetic polynucleotide
atgtcaagcttaactaaattcacaaataagtactctaagcagctgaccataaagaatgagttaattccggtgggtaagactctcgagaacattaaagagaatggcttgatcgacggtgatgagcaattgaatgagaattaccagaaggcgaagatcattgtcgacgacttcctgagggatttcataaataaagccctgaataatacacagataggaaactggcgggagctggccgacgcccttaacaaagaggacgaggataatatcgagaagttgcaggataagattcgaggtatcatagtctcaaagttcgaaacatttgatctcttcagctcctattcgataaagaaagacgagaagatcatcgacgacgacaatgatgtggaagaagaggagctggaccttggaaagaaaacatcttccttcaaatacatcttcaagaagaacctgttcaagctagttctgccaagctacttgaagactacaaatcaggataaactcaagatcatttcgtctttcgacaatttctctacctacttccgtggtttcttcgagaacaggaagaatatctttaccaagaagccaattagcaccagcatcgcctatcgtatagttcacgataactttcctaagttcttggataatattcgctgtttcaacgtctggcagaccgagtgcccacagctcattgtgaaagccgacaactacctaaagagtaagaatgtgatagcgaaggacaagtctctagcaaattatttcaccgtcggcgcctatgactacttcctcagtcagaatggcattgacttctataataacattattggcggtctgcccgcattcgctggtcatgagaagatccaaggtctgaatgagttcatcaaccaggaatgccagaaggattctgaactcaagagcaagctaaagaaccggcatgcgttcaagatggcagtgttgtttaaacagatcctgtctgacagagagaaatcattcgtcatcgatgagttcgaatccgacgcccaggtcatagacgctgtcaagaatttctacgccgagcaatgtaaagacaataacgttatctttaacctcctaaacctcattaagaatatcgctttcctctccgacgatgagctggatggcatcttcattgagggaaagtatctgtcatctgtctcccagaagctgtactcggattggtccaagctgcgaaatgacatcgaagactcagctaatagtaagcaaggcaataaggagctcgccaagaagatcaagactaataaaggcgacgtggagaaagctataagcaaatatgaattctctctgtccgagctaaattctattgtacacgacaacactaaattctccgaccttctgtcctgtacactgcacaaagtcgcttctgagaagttggtgaaagtgaatgagggtgattggcccaagcacctcaagaacaacgaggagaaacaaaagattaaggaacctctggacgctctgttggaaatttataataccctactgatcttcaactgtaagagcttcaacaagaacggaaatttctatgtggactacgaccgctgtataaacgagctgagtagcgtagtctatctgtacaataagaccagaaattactgcaccaagaagccttacaacaccgacaaattcaaactgaacttcaactctccacagctaggtgaagggttctccaagagtaaggagaatgattgcctgacattactgtttaagaaagacgacaactactacgtcggaattatacgaaagggcgcgaagataaacttcgatgatacccaagcaatagcagacaatacagacaattgcatctttaagatgaactacttcctgctgaaagatgccaagaagtttattccgaagtgcagtatccagctgaaggaggtcaaggctcatttcaagaagagcgaggacgactatatcttatccgataaggagaaattcgccagtccactggtcataaagaaatcaaccttcctgttggcgaccgcccacgttaaagggaagaaaggcaatataaagaagttccagaaagagtacagcaaggagaatcctactgagtaccgcaacagcctgaacgagtggatcgccttctgcaaagagtttcttaagacctacaaggccgccaccatattcgatattaccaccttgaagaaggccgaggagtatgcagacatcgtcgagttctacaaggatgtagataacctttgctataaactagaattctgccctattaagacctccttcattgagaacttgatagataacggagatctttatctcttccgcattaataataaggatttcagttccaaatccacaggtacaaagaacctgcacacattgtacttgcaggctatatttgatgagagaaatttaaacaacccaactatcatgctaaatggaggtgccgaattattctatcgtaaggaaagcattgaacagaaaaatagaattacccataaagcaggaagtatactggtaaataaagtgtgcaaggacggcacttcattggacgataagatccgtaacgagatataccagtatgagaataaattcattgacacattgtcagacgaggccaagaaggtgctgcctaacgtcataaagaaggaagccacacacgatattacaaaggacaagaggtttactagcgacaaattcttctttcactgtccactgacaatcaattacaaggaaggtgataccaagcagtttaataatgaagtgctctcattccttcgcggtaatccagatatcaacattattggcatcgatagaggcgagcgcaatctgatctatgtcacagtgatcaaccagaaaggcgagatactggactcggtcagtttcaatacagtgacaaataagagctccaagatcgaacagaccgtcgactacgaagagaaactggcagtgcgcgagaaagagaggattgaggctaagcggagttgggactctatctctaagatcgccaccctgaaggaaggctacctctcagccatcgtccacgaaatttgtttgttgatgataaagcacaacgcaatagtcgtgcttgagaatctgaacgctggcttcaagaggataagaggaggactcagcgagaagagtgtttatcagaagtttgagaaaatgctgattaacaaactgaactactttgtaagtaagaaggaaagcgattggaataaaccttccggattactcaacgggttacagctatcagaccagtttgaatcatttgagaagctgggtatccaatcaggctttatcttctatgtaccagcagcttacacctcaaagatagatccgactacgggcttcgcaaatgtgcttaacctctcaaaggtgcgaaatgtggacgctatcaagtcgttcttctccaatttcaacgagattagctattctaagaaggaagctctcttcaaattcagtttcgatctagactctctgagcaagaagggtttctcttcattcgtgaaattctcaaagagtaagtggaacgtttacaccttcggcgaaagaataatcaaaccaaagaacaagcagggctatcgggaagataaacgcattaatcttacgttcgagatgaagaagctgttgaatgagtacaaggttagcttcgatctggagaataatctgattccaaacctgacgtcggccaatctgaaggacacgttctggaaagaattattttttatctttaagactactctgcagctgagaaattccgtgaccaatgggaaagaagatgtcttgattagtccagtgaagaatgccaagggcgaattctttgtcagcggcactcacaataagaccctgcctcaagattgtgatgccaatggcgcttatcacatcgccctgaaaggcttgatgattctggagcggaataacttggtcagggaagagaaggataccaaaaagatcatggctatctccaacgtagattggttcgaatacgttcagaagcgcaggggcgtgctataa

SEQ ID NO: 330 - DNA, 4005 bp, Artificial Sequence
  Description of Artificial Sequence: Synthetic polynucleotide
atgagttcattaaccaagttcacaaacaagtactcaaagcaacttaccataaagaacgagcttataccagtgggcaagaccttagagaatattaaggagaacggtctgatagatggcgacgagcagcttaacgagaattaccagaaagctaagatcattgttgacgactttcttcgagacttcatcaacaaggcgctcaataatactcagattggtaattggcgcgagctggcggacgcactcaacaaggaggacgaagacaatatcgagaaacttcaggataagattagggggatcatagtgagcaagtttgagacgttcgacctgttcagtagttactccataaagaaggatgagaagattattgacgacgacaatgatgttgaagaggaggaactagacttgggaaagaaaacaagctcgttcaaatacatatttaagaagaatctgtttaaattagtcttgccctcctatctaaagacaacgaaccaggataagctgaagatcattagctcattcgacaatttctcaacgtacttccgtggtttcttcgagaatcgtaagaatatctttaccaagaagcccatctcaacctccattgcctaccgaatcgtccacgacaactttccaaaatttctggacaatatacgctgtttcaacgtatggcaaactgaatgcccacagctgattgtcaaagctgacaattacttgaaaagcaagaatgtaatcgctaaagacaaatcccttgccaattacttcactgtgggtgcctatgactacttcttatcacagaacggaatcgacttctacaacaatatcataggcggactgccagcatttgccggccatgagaagatacagggccttaacgagttcataaaccaggaatgccagaaagactccgaattgaaatctaaactgaagaatcgacacgcttttaagatggccgtcctgttcaaacagatcctttccgaccgcgaaaagagctttgttatcgatgaattcgagagcgacgcacaggtgatagacgcagtcaagaacttctatgccgagcagtgtaaggacaacaacgtcatctttaacctgctgaatctaattaagaacattgcgtttctgtcagacgacgaactggatggaatcttcatcgaaggtaagtacctctccagcgtcagccagaagttatactccgactggagcaaattgcgtaacgacatagaggacagcgctaactcaaagcaaggtaataaagagcttgcaaagaaaataaagactaataagggtgatgtagagaaagccatctctaaatatgaattcagcctgtcagaactcaactccatcgtgcatgacaatacgaagttctccgaccttctttcctgtactctacataaagtggcgtctgagaagctggtcaaggtgaacgaaggtgactggcctaaacacctaaagaacaacgaagagaagcaaaagattaaagagccactggacgccttactcgagatttacaacacactacttatctttaactgcaagtccttcaataagaacggtaatttctacgtggattatgaccggtgtattaatgaactctcatccgtggtctatctttacaacaagacaaggaattattgtacaaagaagccctataatacagataagttcaagttaaatttcaattcacctcagctgggcgagggattctctaaatctaaagagaatgactgtctgaccttgctgttcaagaaggatgataattactatgtcggcataatacggaaaggtgccaagatcaactttgatgacacccaggccattgctgataataccgacaattgtatattcaagatgaattacttcttgttgaaagatgctaagaaattcatccctaagtgctcgatccaactgaaagaagtgaaggcacattttaagaagtccgaggacgactacatactatcagataaggagaagtttgcatctccactggtaatcaaaaagagtaccttcctgcttgctaccgcccatgtcaagggtaagaaagggaatatcaagaaatttcagaaagagtatagtaaagagaatcccactgagtacagaaactccttaaacgaatggatcgcattctgtaaggagttcttgaagacttacaaggctgcgaccatctttgatattactacgctaaagaaggcggaagagtacgccgacatcgtagaattctacaaggatgtggacaatctttgttataaactcgaattctgtccaatcaagacatcatttatcgagaacctgatcgacaacggagacttgtacctcttcagaattaacaataaggacttctcgagcaagtcgacagggacaaagaacctccataccctgtatctacaggcaatcttcgatgaaaggaacctgaacaacccaacgatcatgctgaatgggggagccgagctgttctatcgtaaagagtcaatcgaacagaagaatcgcatcacgcacaaagccggttcgatactcgtgaacaaggtgtgcaaagatggtaccagccttgacgataagattaggaatgaaatctatcagtacgagaacaagtttattgacactctctctgacgaggccaagaaggtgctgccgaacgtcattaagaaggaggccactcacgatattacgaaggacaaacgattcactagcgataagttcttcttccactgcccgctgactatcaactacaaggaaggagatacaaagcaattcaataacgaagtgctctctttcctccgcgggaatccggacattaatatcatcgggatagatagaggagagcgcaatctgatttatgtgaccgtcataaaccagaagggagaaattctggactccgtttccttcaacaccgtgacgaataagagctccaagattgagcaaaccgtggactatgaagagaaactggcggtgcgagagaaagagcgaattgaggctaagaggtcttgggactccattagtaagattgcgactctgaaagaagggtacctaagtgccatcgtacatgagatctgcctcttgatgattaagcacaatgctatagtggtgttggagaatttaaatgctggcttcaagcgaattagaggcggcctgagtgagaaatctgtataccagaagttcgagaaaatgctgatcaacaagcttaattatttcgtcagtaagaaggagtcagactggaacaaacctagcggactgctcaacggcctccagctgtccgatcagtttgagtcctttgagaaattgggtattcagagcggattcatcttctatgtcccggctgcctatacatctaagatcgatcctacaacaggattcgccaatgtgttgaatttgagtaaagtcagaaacgttgacgcgatcaagagcttcttctccaacttcaatgagatttcctattctaagaaagaggctctctttaagttctcctttgacttggacagcctcagcaagaaaggcttcagctcgtttgtgaagttctcaaagagcaagtggaacgtttacacctttggagagcggataatcaaaccaaagaataagcagggttaccgtgaagataagaggattaatctgacctttgaaatgaagaagttgctgaatgagtacaaggtttccttcgacctcgagaacaatctaattccaaacctcacctctgcgaacctcaaggacaccttctggaaagagctattcttcatatttaagactaccttgcagcttaggaactcagttacaaacggcaaggaggatgtcttgattagcccggtgaagaacgctaagggagagttctttgtctccggcacacacaacaagacgctacctcaagactgtgatgcaaatggagcatatcatatagcacttaagggtcttatgatcctggaacgaaacaacctggtgagggaagagaaggataccaagaagatcatggcgatcagcaatgtggattggtttgagtacgttcagaagcgaagaggcgttctgtga

SEQ ID NO: 331 - DNA, 4005 bp, Artificial Sequence
  Description of Artificial Sequence: Synthetic polynucleotide
atgtcttccctgaccaaatttacaaacaaatattccaaacagctgactataaagaacgagctgattccagtgggtaagacactagagaacatcaaagagaacgggttgatcgacggtgatgagcagctgaatgagaactatcagaaagccaagataatcgtcgacgacttcttacgggacttcattaataaagcactgaacaacactcaaataggaaattggagagagttggccgatgctctgaataaggaagatgaggataacattgagaaacttcaggataagattagagggatcatagtgtccaagttcgagactttcgacctgtttagctcgtacagtattaagaaggatgaaaagatcatcgacgacgacaacgatgtggaagaggaagaattagatctgggcaaaaagacatctagtttcaaatacatattcaagaagaatctgtttaaactggtgctgccaagttatctaaagaccaccaatcaggacaaattgaagatcatttcttccttcgataacttctctacgtactttagaggcttcttcgagaatcgaaagaatatcttcactaagaagcccatcagtacctccatcgcttacaggatcgtccatgacaacttcccaaagtttctggacaatattagatgctttaacgtgtggcagaccgaatgcccacagctgatcgttaaggcggacaactatctgaagtcaaagaacgtgattgcaaaggacaagagcctagccaactactttacagtgggtgcttatgactacttcttatcccagaatggaatcgacttctacaacaacattataggcggtctccctgcattcgctggacacgagaagatccaagggctcaacgagttcatcaatcaagagtgccagaaggattcggaattaaagtccaagttgaagaacagacatgcctttaagatggccgtactgttcaaacagatcctttcagatcgagagaaatcgttcgtgattgacgaatttgagagtgatgcccaggtaatcgatgctgtcaagaacttctatgccgaacagtgtaaggacaataatgttatattcaatctgctcaatcttattaagaatatcgcattcttaagtgacgacgagctggatggcatatttatcgagggtaagtatctgagttccgtctcacagaagttgtatagtgactggtctaagcttcgtaacgatatcgaagattccgcaaactctaaacagggaaacaaagagctcgctaaaaagattaagaccaacaaaggtgacgtggagaaagctatttccaaatacgagttctccctgtcggaattaaatagtatcgtccacgacaatactaaattctctgacctgctctcttgtaccttacacaaagtcgctagcgagaaactcgtcaaggtaaacgagggagactggccaaagcacctcaagaacaacgaggagaagcagaagattaaggagcctttggatgccctgctcgaaatctataatacactgctaatatttaattgcaagagtttcaacaagaacgggaacttctacgtggactatgatagatgtattaacgaactgtcgtcagtagtatacctttacaacaagaccaggaattattgcacgaagaagccttacaacacggataagtttaagcttaacttcaactctccacagctgggcgaaggcttcagcaagagcaaggagaacgattgcctgaccttgctcttcaagaaagacgataattattacgtgggaatcatccggaagggcgccaagatcaactttgacgacactcaagccatagcagataacacagataattgtatatttaagatgaactatttcctgttgaaagatgccaagaaattcataccaaagtgttcgatccaactcaaagaggtgaaggcccatttcaagaagagcgaggacgactatatcctgtcggataaagagaagtttgcctctccactcgtgataaagaagagtacattcttgctcgctactgctcatgttaagggcaagaaaggaaacattaagaaattccagaaggaatacagcaaagagaaccctactgagtacaggaactccctgaatgagtggatcgccttctgtaaagagttcttaaagacctacaaggcggctacgatcttcgacattacaacactcaagaaggcagaggaatacgccgatatcgtggaattctataaagatgtggataatctctgttacaagctggagttctgtcccataaagacaagcttcatcgagaacctgattgataatggagacctctacttgtttcgcattaacaataaagacttctcatctaagtccaccgggactaagaacctccataccctctacctgcaggctatattcgatgaacggaatctgaacaatccaaccattatgctgaatggaggagccgaactgttctatagaaaggagtcaatcgagcagaagaaccgcatcacccacaaggctgggtctattcttgtgaataaggtttgtaaggacgggacttcccttgatgataagattcggaatgaaatatatcagtatgagaataagttcatcgatacgctgagcgacgaggctaagaaggttctgcccaacgttattaagaaagaagccacacacgacatcaccaaggataagcgatttacttctgacaagtttttcttccattgtccgctgacaatcaactacaaagagggcgacaccaaacagttcaacaacgaggtgctgtcattcctgcgcggcaatccggacattaacatcattgggatagacaggggcgagagaaacctgatttatgtgactgttatcaatcagaagggcgagatactggattccgtcagctttaataccgttaccaataagtccagcaagattgagcagacagtggactacgaggagaaactggctgttagagagaaggagaggatagaagctaagcgttcttgggattcaatttctaagatcgctacactcaaagaaggctatcttagtgctatagtccatgaaatctgcctcctaatgatcaagcataatgcaattgtggtgctggagaatctgaacgccggcttcaagcgaatccgcggtggtctgtcggaaaagagcgtctaccagaagttcgaaaagatgctcatcaacaaactaaactacttcgtctctaagaaggagagcgactggaacaagccttctggacttctcaacggactccagctgtccgaccaatttgagtccttcgagaagctcggtattcagtcaggattcatcttctatgttcctgccgcttacacatcaaagatagatccaactaccggattcgcgaatgtgctcaatctctccaaagttaggaatgtggacgccatcaagagctttttctccaactttaatgagatttcctattctaagaaggaggctctgtttaaattctcattcgacttggacagcttgagcaagaaaggtttcagcagcttcgttaaattctccaaatccaagtggaatgtgtacacattcggtgagaggattattaaaccgaagaacaagcaaggctacagagaggacaagcgcattaatttgacattcgagatgaagaagctcctgaacgagtacaaggtgagctttgatctggagaacaacctgatacctaacctcactagcgccaacctcaaagatactttctggaaagaattgttctttatcttcaagacgaccctacagctgcgtaacagcgtgactaatggcaaggaagatgtgctcatttcaccagttaagaacgctaagggtgaattcttcgtatctggcacacataacaagacattaccacaggactgcgatgccaatggcgcctatcacatagctctgaagggattgatgatcctggaaaggaacaacctagtgagagaggagaaagatacaaagaagatcatggcaattagtaatgttgattggttcgaatatgtgcagaaacgacgaggagtcctgtag

SEQ ID NO: 332 - DNA, 4005 bp, Artificial Sequence
  Description of Artificial Sequence: Synthetic polynucleotide
atgtccagtctgacaaagtttaccaataagtactcaaagcagctaactatcaagaatgagctaattccagtcgggaagacgttggagaatatcaaggagaatggtttaattgatggtgacgagcaacttaatgagaactaccagaaggctaagattatagtagacgacttcctccgggacttcattaataaggcactgaataatacgcaaatcggcaattggcgcgaattagctgacgctctgaacaaagaagatgaagataacatagagaagctgcaggataagattagaggcatcattgtatccaagttcgagacctttgacctctttagttcgtactccatcaagaaggatgagaagattattgacgacgacaatgatgttgaggaggaggagctagatctaggaaaaaagacttcatcctttaagtatatcttcaagaagaacctgtttaagttagtgctgccatcttacctcaagacaactaatcaagacaagctgaagataatctccagtttcgataacttctctacgtatttccgaggtttctttgagaatcgaaagaatatattcaccaagaaacccatctctacatccatcgcttatcgaatagtgcacgacaattttcctaagtttcttgacaatattaggtgcttcaatgtgtggcagactgagtgcccgcagctgattgtgaaagccgataattatctgaagtcgaagaatgttattgccaaagataagtccttagcaaactatttcactgttggcgcctacgattacttcctgagccagaatggaatcgatttctataataacattatcggtggattgccagcgttcgccggacatgagaaaatccagggcttgaatgagtttataaaccaggagtgccagaaggatagtgaactgaaatctaaactgaagaacaggcatgcctttaagatggccgtgctgtttaaacaaatcctttccgaccgcgagaagtcgttcgtcatagatgagtttgagtcggatgcccaggtcattgacgcagttaagaatttctacgccgagcagtgcaaggacaataacgtcatatttaacttacttaatctgatcaagaacatagccttcctctctgatgacgagcttgatggtatctttatcgaaggcaagtatctttcttccgtgtcacagaagctatactctgattggagcaagttacgcaacgatatcgaggacagtgccaattccaagcaaggcaacaaggagctggcaaagaaaatcaagacaaataaaggtgatgttgagaaggcgatttcaaagtacgaattcagcctgtccgaactcaactctattgtccatgataatactaaattctcggacttgctgtcatgcaccctccataaggtggccagtgagaagcttgtcaaagtgaatgagggagattggcctaagcacctgaagaataacgaggagaagcagaaaatcaaagaaccactagacgccttgctcgaaatatacaataccctactgatcttcaactgtaagtcgttcaacaagaacgggaacttctatgtggactatgaccgttgcattaacgagctcagcagtgtagtctacttatacaacaagactcgcaattattgcacaaagaaaccgtataatacagataagttcaagctgaacttcaattcaccacaattaggagaaggtttctccaagtcaaaggagaacgactgtctgactctcctgtttaagaaagacgacaattattacgttggcatcatcaggaaaggagcgaagattaactttgacgatacacaagcaatcgcagataataccgataactgcatcttcaagatgaattatttcctgctcaaggatgcaaagaaattcataccaaaatgttctatccaactcaaggaagtcaaagctcactttaagaagtcagaggacgattatatattgagcgataaggagaaatttgcgtctccacttgtgattaagaagtccacattcctgctggcgacagcgcacgtgaagggaaagaaaggtaatataaagaagttccagaaagaatattctaaggagaatcccaccgagtatcggaatagcctcaatgagtggattgccttctgcaaagagtttctcaagacttataaggcagcgactatctttgatatcaccacccttaagaaggctgaggaatatgccgatatcgttgaattctacaaggacgtggataatctatgctacaagcttgagttctgtcccataaagactagctttatagagaacctcatcgacaatggcgatctgtacttgttccggataaataataaggactttagtagtaagagtaccggaacaaagaacctgcacacactctacctgcaggccatattcgatgagcggaatttaaacaatccaaccatcatgctaaacggaggcgcagagctcttctatagaaaggagtctattgagcagaagaacagaattacacataaggccggatccatcttggtaaataaggtgtgtaaagatgggacctccctggatgacaagattcgcaacgagatttaccagtatgagaataagtttatcgacactctctctgacgaggcaaagaaggtactgcccaacgtaatcaagaaggaagcgactcatgatattacgaaggacaagagattcacatccgacaagttcttctttcattgtccattgaccatcaattacaaggagggagacacgaaacaatttaacaacgaagtgcttagcttcctccgtggaaatcccgacatcaatataattggtatagacagaggtgagcgtaacctaatctacgtcactgtaattaaccagaaaggcgagatccttgactctgtgtccttcaacaccgtgactaataagagcagcaagattgaacagactgttgactatgaggagaaactggcagttagagagaaagagcgtatagaagcgaagcggtcctgggacagtatttccaagatcgccacccttaaagagggttacctctcagcaatcgttcacgaaatttgcctattgatgattaaacataatgccatagtggttctcgagaatctcaatgcaggatttaagaggattagagggggcctgtccgagaagagtgtttatcagaagtttgagaagatgctcataaataagttaaactatttcgtgtctaagaaagaatcagactggaataaaccatccgggctcctgaacggtctgcagctctccgaccagtttgaaagcttcgagaaacttggcattcagagcggcttcattttctatgttcccgcagcctatacttccaagatcgaccctaccaccggctttgccaacgtactgaacctttccaaagtaagaaatgtggacgctattaagtccttcttctcaaactttaacgaaatttcttactccaagaaagaggctctctttaaattctcatttgatttagactcactgagcaagaagggcttctcatcattcgtgaagttctccaagagtaagtggaatgtgtatacgttcggcgaaaggataatcaagcctaagaacaaacagggctacagggaggataagaggatcaatctgacattcgagatgaagaaactgctgaacgaatacaaggtcagctttgatctcgagaacaacttgatcccaaacctcacttcggccaatcttaaggataccttctggaaggagctgttcttcatctttaagaccactttgcagctgagaaactctgtaacaaatggcaaggaagatgtattaatatcgcctgtaaagaacgctaaaggcgaattctttgtcagtggaacgcataacaagactttgccacaggattgtgatgccaatggcgcctatcacattgccttaaaggggctaatgatcctggagcggaataacctggtacgcgaggagaaggacacaaaaaagatcatggctatctctaatgtcgactggttcgaatacgtccagaagcgccgcggagttctctga

SEQ ID NO: 333 - DNA, 4005 bp, Artificial Sequence
  Description of Artificial Sequence: Synthetic polynucleotide
atgtcttccctgacaaagttcactaacaagtactccaagcagctgaccatcaagaacgaacttattcccgtgggcaagacacttgagaacatcaaggagaatgggctgattgatggcgacgagcagctgaatgagaattaccagaaagctaagattatcgtggacgactttctgagggacttcattaacaaggcactgaacaatactcaaatcggaaattggagggaactggctgacgcacttaacaaggaagatgaggacaatatcgagaaactgcaggataagatcagaggcataatagtgtccaaatttgagaccttcgatttattcagcagttactcaatcaagaaggacgagaaaatcattgatgacgataacgatgtggaagaggaggagctggacctcggcaagaagacatcatccttcaaatatatatttaagaagaacctgtttaagctcgttctaccatcttacctgaagacgacgaatcaggacaagctgaagatcatttcaagtttcgataactttagcacatactttagaggtttcttcgagaacagaaagaatatcttcaccaagaaacccatttctacgagtatcgcatatcgtatagtacacgataactttcctaaattcctagacaatattcggtgctttaatgtctggcagacagagtgtccacagctaattgttaaagcagacaactacctaaagagtaagaatgtgattgccaaggacaagtctctagcaaactacttcaccgtgggcgcatacgattacttcttaagccagaatggaatagatttctacaacaatataataggtgggcttcccgcatttgctggccatgagaagattcagggcctgaacgagtttatcaaccaagaatgtcagaaggacagcgagttaaagagcaagctaaagaacagacacgcctttaagatggcagtcttgtttaagcagatcctctcagacagagagaagtcattcgtaatagatgagttcgagtctgatgctcaagtcattgacgctgtaaagaacttctatgccgagcagtgcaaagataataacgtgatctttaacctgttaaacctcatcaagaacattgctttcttgtctgacgatgagttagacggcatctttatcgaaggcaagtacctctccagcgtctcgcagaaattatactcagattggagcaagctgcggaatgatatcgaagatagtgccaactctaagcaaggcaacaaggagcttgcgaagaagatcaagacaaacaagggtgatgtggagaaagctatctcgaagtatgagttctcactctctgaacttaactccatagtacatgataacacgaagttctctgacctgctctcctgtaccttacataaggtcgccagcgagaaactcgtcaaggtgaatgagggtgactggcccaaacatttgaagaacaatgaagagaagcagaagatcaaggagcctctggacgccttgctggaaatctacaataccctgctgatctttaattgcaagtcgtttaataagaacgggaacttctacgtggattacgaccgctgtattaacgagctctcatccgtggtatatttatacaacaagactcggaactactgcacgaagaaaccttataatactgacaaattcaaactgaacttcaatagtccacagttgggtgagggattcagtaagagcaaagagaatgactgtctgacgctcctgttcaagaaggatgacaattactacgtgggaattattcggaagggtgccaagatcaatttcgacgacacccaggccattgcagataacactgataattgcatctttaagatgaattactttctgctgaaagatgccaagaagttcatacctaagtgcagcatccagctcaaggaagtgaaggcgcactttaagaaatcggaagacgactacatactgtctgataaagagaagttcgccagtcctctcgtgataaagaagtctacctttcttctggcaaccgcgcatgtgaagggaaagaaaggcaacattaagaagtttcagaaggaatatagcaaggagaatccaacagaataccgcaatagtctgaatgagtggatcgcattctgtaaagaatttctgaagacatacaaggccgcaaccatattcgatattactacactgaagaaggccgaagaatatgctgacatcgtggagttctataaggatgtggacaatctctgctataagctagaattctgcccaatcaagacttcatttattgagaatctcatcgacaatggcgacctgtatctctttcgaataaacaataaagacttctcatcaaagtccacaggtacgaagaacctgcacactctgtatttacaggcaatcttcgacgagcgtaacctaaacaatccaaccatcatgttgaacggaggcgccgagttgttctatagaaaggagtcgatagaacagaaaaaccgcattacgcacaaggccgggtctattctcgtaaacaaagtgtgcaaggatggaacctcccttgatgacaagatccgcaacgagatataccagtatgagaacaagttcatcgatacactgagtgatgaggctaagaaggtgttaccgaatgtgatcaagaaggaggctacacatgacattaccaaggacaagcgatttaccagcgataagtttttctttcactgtcctctaaccatcaactataaggagggcgacaccaagcagttcaataacgaagtgctgagcttcctcagaggcaatcccgacatcaacatcatcggtatagatcgcggtgagcggaatttgatctatgtaaccgtgattaatcagaaaggtgaaattctggactcagtctcctttaacactgtgacaaacaagagttctaagatcgagcagaccgtggattatgaggagaagctggccgtgcgagagaaagaaagaatcgaggcaaagaggtcttgggactcgatctcaaagatcgccacgctgaaggagggctatctgtcagccatagttcacgagatttgtttgttaatgatcaaacacaacgcgatcgtcgtccttgagaaccttaacgccgggtttaaacgcatacgagggggcttgtccgagaaatccgtataccagaaatttgagaaaatgctgataaataagctgaattacttcgtctcaaagaaagaatccgactggaataaaccaagtggcttacttaacggcctgcagctatctgaccaattcgaatcctttgagaagctgggcatccaatctgggttcatcttctatgtcccagccgcgtatacctctaagattgaccctaccacaggcttcgccaatgtcctgaacctgtctaaagttcggaatgtagacgcaatcaagagcttcttctccaacttcaatgaaataagctattctaagaaggaggcattgtttaagtttagcttcgatctcgactcgctaagcaagaaaggctttagtagcttcgtgaaattcagcaagtccaagtggaacgtctatactttcggcgaacggatcattaaaccgaagaacaagcaaggctaccgtgaagacaagcgaatcaacctcacatttgagatgaagaaactgcttaacgaatacaaggtgtccttcgacctagagaacaatctgataccaaacttaacttctgccaacctgaaggacactttctggaaggaactcttctttatcttcaagacaactctgcaactccgaaactcagtcacaaacggtaaagaagatgtgctgatctctcctgtgaagaacgcaaagggcgaattctttgtgtcaggtacccataataagacactgccacaagactgcgatgcaaacggcgcgtaccatattgccctgaaaggactgatgatattggagagaaacaacctcgttcgagaggagaaggacacgaagaagatcatggcaatctcaaatgttgactggtttgagtatgtccagaagcggagaggagtgctgtag

SEQ ID NO: 334 - DNA, 4005 bp, Artificial Sequence
  Description of Artificial Sequence: Synthetic polynucleotide
atgagctcactcaccaagttcacgaataagtattccaaacagctcaccataaagaatgagctcatacctgtaggcaagaccctggagaatattaaagagaatgggctgatcgacggcgacgaacagctgaatgagaattatcagaaggccaagatcatagtagatgatttccttcgcgacttcatcaacaaagccctgaacaacacccagattgggaactggcgagagttagcggacgcactgaacaaggaggacgaagataacatcgagaagctgcaggataagattcgcggcatcattgtgagcaaattcgagacatttgacttattcagtagctactctatcaagaaggacgaaaagattatagacgatgataacgatgtggaggaggaagaattagacttgggcaagaagacatcatctttcaaatacatctttaagaagaacctgttcaagctggtcctgcctagttaccttaagacaaccaatcaggataagctgaagattatcagctcctttgacaatttctccacatacttccgagggttcttcgagaaccgcaagaacatcttcactaagaaaccaattagcacatctatcgcctaccggattgtgcacgacaatttcccgaagtttctggataatatccggtgctttaatgtctggcaaacagagtgcccacagctaatcgtcaaggccgacaattatctcaagagtaagaacgtgattgctaaggataagagcctggcaaactacttcaccgttggcgcctatgactacttcctctctcagaatggaatcgatttctacaataatatcataggcggattaccggctttcgctggccacgagaagattcaagggctaaacgagttcattaaccaggagtgccagaaagactccgagctgaagagtaagctaaagaaccgccacgcgtttaagatggcagtcctgttcaaacagatcctcagcgacagagagaaatcctttgtgatcgacgaattcgagagcgatgcgcaggtgatagacgctgttaagaatttctatgccgagcagtgcaaggataacaacgtcatatttaatttactcaacttgataaagaacatagccttcctttcagacgacgaactcgacggcatctttattgaaggaaagtacctgtctagcgtctcgcagaaactttattctgactggtccaaactgaggaatgatatagaggatagtgccaactctaagcagggcaataaagagctggccaaaaagatcaagacgaataagggagatgtcgagaaggccatttccaaatacgaatttagtcttagcgaactgaacagtatcgttcacgacaatacgaagttctccgacctgctatcatgcactctgcacaaggtggcctctgagaaattggttaaggttaacgaaggtgattggccaaagcatttgaagaataatgaagagaaacaaaagattaaggagccattggacgctctgcttgagatttacaacactctcctgatcttcaattgtaagtcatttaataagaatggcaacttctacgttgattacgaccgctgcataaatgagctgagcagcgttgtctacctctataacaagaccagaaactattgtaccaagaagccgtacaacacagacaagttcaaactcaacttcaattctccgcaacttggcgagggtttctcgaaatccaaggagaatgactgtttaacgctgctgtttaagaaagacgacaactattacgtgggaattatccgaaagggcgctaagataaactttgatgacactcaggcgatcgctgataacactgacaactgtatcttcaagatgaactacttcctgctgaaggacgccaagaagttcatcccgaagtgttcaatccagctcaaagaggtgaaagcgcactttaagaagagtgaggatgattatatattaagcgataaggagaaattcgcaagtccattggtgatcaagaaatctacattcctactagcaaccgcacacgtcaagggcaagaagggaaacattaagaaatttcagaaggagtactctaaggagaatccaactgaatacaggaattctctcaacgagtggatagctttctgtaaggaattcctaaagacttacaaagccgcaactatatttgacatcaccacactcaagaaggcagaggagtatgccgacatcgtcgagttctacaaggacgtggacaacttgtgttacaaacttgaattctgcccaataaagacatcattcattgagaaccttattgataatggcgatctgtacctgttccgaatcaacaataaggatttctctagcaagtcaacaggcaccaagaacctccataccctctacctacaggccatattcgacgagaggaacctgaacaatcctacaattatgctcaacggcggtgcagaactcttctacaggaaggaaagcatcgagcaaaagaacagaatcacccataaagcaggaagtattctggtcaataaggtgtgtaaggacggtacatcactggacgataagatccgcaacgagatctatcagtacgagaataaatttatcgacaccctgtccgatgaagccaagaaggtcctccctaacgtcatcaagaaggaggcaacccatgatatcaccaaggataagaggttcacatcagacaagttcttctttcattgtccattaaccatcaactataaagaaggcgataccaagcaattcaacaacgaagtgctaagcttcttgcgcggcaatccagacatcaacattataggcattgaccgcggcgaacgtaacttaatctacgtgacggttataaatcagaaaggcgaaatcctggactctgtgagctttaacaccgtgacgaataaatcatctaagatcgagcagaccgtggactacgaggagaagctggctgttagagagaaggagcggattgaagctaagagatcatgggactcaatctcaaagatcgccaccctcaaggaaggttatttatcagctattgttcatgaaatatgcctgttgatgattaaacataatgctattgtggtgctcgagaatctgaacgccgggttcaaacgcatcagaggaggacttagtgagaaatctgtgtatcagaaatttgagaaaatgctgattaacaaactgaactacttcgtgagtaagaaagaaagcgattggaataaaccatcagggttgttgaacgggctacagctttctgatcagttcgagtccttcgagaaattagggattcaatctggattcatcttctacgtgcccgcagcctacacttctaagattgatccgaccaccggcttcgcaaacgttctgaatttgtccaaagtacggaacgttgacgcaataaagagcttcttcagcaactttaacgagatttcctattccaagaaggaagcgctgttcaagttctcctttgacctggatagccttagcaagaaaggtttctcctctttcgtgaagtttagcaagtctaaatggaatgtctacacatttggagaaaggataataaagcctaagaataagcagggatatcgtgaagacaaacgaatcaatctgacattcgagatgaagaaactccttaatgaatacaaagtctctttcgatctcgagaataacctcatcccaaacctgacgtccgcaaatctgaaagacaccttctggaaagagctcttctttatctttaagactacgctccagctgaggaacagcgtcactaatgggaaggaagacgtgttaatttcacctgttaagaatgccaagggtgaattcttcgtctcaggtacacacaataagactctacctcaggactgcgatgctaacggagcctatcatatagcactgaagggactaatgattctggaaaggaacaacttggtcagagaggagaaggatacaaaaaagatcatggctatctccaatgtggattggtttgagtacgtgcaaaagaggaggggtgttctttaa

SEQ ID NO: 335 - DNA, 4005 bp, Artificial Sequence
  Description of Artificial Sequence: Synthetic polynucleotide
atgtcttcccttactaaattcaccaataaatactccaaacagctcacaattaagaatgagctaatcccagtcggcaagacactggagaatatcaaagagaacggtctgatcgacggtgatgagcaattaaacgagaactatcagaaggctaagataatagtggatgactttctccgggacttcattaataaagctctgaataacacacagatcgggaactggcgagagctcgcagacgccctgaacaaggaggatgaggataatatcgagaagctgcaggataagatacgcggaatcatagtctcgaaatttgagacctttgatctgttcagctcatactctattaagaaggatgagaagattatcgacgatgataacgatgtggaggaggaggaattggacctgggtaagaagacgagttcgtttaaatatatcttcaagaagaacctattcaagttagtgttgccgtcctacctcaagacaacaaaccaggacaaactaaagattatcagctccttcgacaacttctctacctacttccgagggttcttcgagaaccgcaagaatatctttacaaagaagcctatctcaacctctatcgcctacaggattgtacatgataactttccaaagtttctcgataacatccgttgcttcaatgtgtggcaaaccgagtgcccgcagctcatcgtgaaagcagataactacttgaagtcgaagaacgtcatcgctaaagataagagcctggccaattatttcacagttggtgcctacgactacttccttagccagaatggaatcgatttctacaacaacatcattggagggttgccagcatttgcgggccatgagaagatccagggtctcaatgagtttatcaaccaggaatgccagaaagacagtgagttgaagtccaaactgaagaaccgccacgcattcaagatggcagtcctgtttaagcaaatcctctccgatagagaaaagagctttgtgatagatgaatttgaatcggacgctcaagtgatcgacgcagtgaagaacttctatgcagaacagtgcaaggataataacgtgatcttcaatctcctaaatcttataaagaacattgcattcctgtcagacgatgagcttgatggcatcttcattgaaggcaaatacttgtctagcgtcagtcagaagctgtactcggattggtccaagctgagaaatgacatcgaggatagtgccaattccaagcaaggaaacaaggaactggcaaagaaaattaagacaaacaaaggcgacgtcgagaaggctatcagcaaatacgaattctccctaagtgaattaaattctatcgtacatgacaataccaagttctccgacctgctcagttgcactctgcacaaagtagcatctgagaaactcgtgaaggtgaacgaaggagactggcctaagcatttaaagaacaatgaagagaagcagaagataaaggaacctctggatgcgctgctggagatctataatactttattaatctttaactgcaagagtttcaacaagaatggcaatttctacgtggattatgacaggtgcataaatgaactctcatccgttgtgtacctctataacaagacaaggaactactgcacaaagaagccatacaatacggacaaatttaagttgaacttcaattcacctcagttaggcgagggcttcagcaagagcaaggagaacgattgcttaacactcttgttcaagaaagacgacaactattacgtgggcataatccgaaagggagcaaagatcaactttgacgatactcaggccatcgctgacaatactgacaactgtatattcaagatgaactatttcttgctgaaggacgcaaagaaattcatcccgaaatgctcaattcaacttaaagaggtgaaggcccactttaagaagtccgaggatgattatatcctgtcagacaaagagaagttcgcgagcccactggtgatcaagaagtcaacctttctgcttgccacagcgcatgttaaaggcaagaagggaaacatcaagaagttccagaaagagtattccaaggagaatcccactgagtatcggaatagtctgaacgagtggattgctttctgcaaagagtttctgaagacatataaagccgcgacaatcttcgacattactacactgaagaaggccgaagagtacgcagacattgtggagttctataaagacgttgataatctgtgctataagttggaattctgtcccatcaagacctcatttatcgagaaccttatagacaatggtgacctatacctattccgcattaataacaaagatttcagctccaagagtactggtactaagaacctccacacactctatctacaggctatatttgatgaaaggaatcttaacaaccctactattatgctgaacggaggtgccgagctgttctaccgcaaggagtccatcgagcagaaaaataggatcactcataaggctggctctattcttgtaaataaggtatgcaaagatgggacgtccttggatgacaagattcggaatgaaatttatcaatacgagaacaagtttattgacaccctcagtgatgaggctaagaaagttctgcctaatgtcatcaagaaggaggcaacacacgacatcaccaaggataagagattcacgtccgataagttcttcttccattgccctctgactatcaattataaggaaggtgatactaagcagtttaacaatgaagtgctctcctttctgcgtgggaaccctgatattaatatcataggcattgatcgaggagaaaggaacctgatctacgtgacagtgatcaatcagaaaggagagatcctggactcggtgtcatttaatacagttacgaacaagagctccaagatagagcagactgtggattatgaagagaagctagcagtgagggagaaagagcgcatcgaggcaaagagatcttgggactcaatctcaaagatagctactctgaaagaaggctacctgagcgctatcgtacacgaaatctgtctattgatgatcaaacacaacgcaatcgtggtgctagagaatttgaacgccgggtttaagagaattagaggcggcctgtcagagaagtccgtgtaccagaagtttgagaagatgctcattaacaagcttaattatttcgtctctaagaaggagagcgactggaacaaaccatccggactgcttaatggcctccagctgagtgatcagtttgagtcattcgagaaacttggtattcagagcgggttcatattctatgtccctgcagcctacacgtcaaagattgatcccaccaccggtttcgccaatgtcctgaacttaagtaaggtccgcaatgtggatgccatcaagtccttcttcagcaatttcaacgagatcagttacagtaagaaggaggccctgttcaagtttagcttcgatctcgattctctgagtaagaagggattcagcagctttgtgaaattcagtaagtccaaatggaacgtatacacctttggagagaggatcatcaagcccaagaacaaacaaggctatagagaagataagagaattaacctcacctttgagatgaagaagctcctgaacgaatacaaagtcagtttcgacctcgagaataacttgatcccgaacttgacctctgccaatctaaaggacacgttctggaaagagttattctttatcttcaagactactcttcaacttcggaatagcgtgactaacggcaaggaggatgtattaatctctcccgtgaagaacgccaagggtgagttctttgtgtccggaacccacaataagacacttccacaggactgcgacgccaatggagcctaccatatagcactgaaaggtctgatgattctggagagaaacaacctcgtgagggaggagaaagacaccaagaagataatggcaatatcaaatgtggattggtttgaatacgtgcagaagcgtcgaggggtcttgtaa

SEQ ID NO: 336 - DNA, 4005 bp, Artificial Sequence
  Description of Artificial Sequence: Synthetic polynucleotide
atgagtagcctgacgaagtttacaaacaaatattcgaaacagctcactattaagaatgaactgatccctgtgggaaagaccctggagaacattaaggagaatggactaatagatggtgacgagcaactgaatgagaattaccagaaggcgaagatcatagtggatgactttctaagggactttataaacaaggcccttaataacacgcagattggcaattggcgtgagctggctgatgcattaaacaaggaggacgaggacaatattgagaagctacaggataagatccgcggaattatagtgtccaaatttgaaacctttgatctcttcagttcctattctattaagaaggacgagaagattatcgatgatgataatgacgtggaagaggaagaattggacttgggaaagaagacatctagctttaaatacatattcaaaaagaacctgttcaagttagtgttaccaagttacctaaagacaactaaccaagacaaacttaagataatcagctctttcgataacttctcaacttatttccgaggcttcttcgagaatcgtaagaatatcttcacgaagaaacctattagcacatcaatagcttatcggattgtgcatgataactttcctaaattcctggacaatattcgctgcttcaacgtatggcagacagaatgcccgcagttaattgtgaaagccgataattatcttaaatcgaagaatgtcatcgccaaggataaatctctagccaactatttcacagtcggtgcttatgactacttcttatcccagaacggtattgacttctacaataacatcatcggagggctcccggcgttcgccggacacgagaagatccagggactcaacgagttcatcaatcaagagtgccagaaggacagcgagttaaagagcaagctcaagaaccgccatgcgttcaagatggccgtcctgttcaaacagatcctgtcggatcgggagaaatctttcgtaatagacgagtttgagtccgatgctcaagtgatagacgccgtcaagaatttctatgctgagcagtgtaaagataacaatgttatattcaaccttctgaacctgattaagaacattgctttccttagcgacgacgaactcgacggaatatttatagagggtaagtacttgagcagcgtgagccagaagctgtattctgattggtccaagctacgtaatgacattgaggactcagcaaacagcaagcagggtaacaaagagctggccaagaagataaagacaaataagggcgatgtcgagaaggccattagtaagtacgagttctccctctctgagttaaactccatcgtgcacgacaacaccaagtttagtgatttgttgagctgcaccctgcataaggtcgcctccgagaaattagtaaaggtgaatgaaggcgactggcccaagcatctcaagaacaatgaagagaaacaaaagatcaaggagccactggatgctttacttgaaatctacaataccctgttgatattcaactgcaagagcttcaataagaacggaaacttctatgtagactatgacagatgcattaatgagcttagctctgtcgtgtatttatacaacaagacaagaaactattgcactaagaagccatataacacagataaattcaagctgaacttcaatagtccacagctgggagaaggtttctccaagagcaaagagaatgattgcctgacactcttgttcaagaaggacgacaactactacgtcggtattattcgtaaaggagctaagataaatttcgacgacactcaagcaatcgctgataatactgacaactgtatctttaagatgaactatttccttctcaaggatgccaagaaattcattcccaagtgctccattcagctgaaagaggtgaaagctcacttcaagaagtctgaagacgattacattctaagcgacaaggagaaatttgcctctcccttagtcattaagaagtccactttcttgctcgctacggctcatgtcaaaggtaagaagggcaatattaagaagttccagaaggaatactctaaggagaatccaaccgagtacagaaattcacttaacgaatggatagccttctgcaaggagtttctcaagacatacaaggctgccactatatttgacatcacaacactgaagaaagccgaggagtatgccgacatcgtggagttctacaaagacgtcgacaatctttgttacaagctggagttctgtcctatcaagacctcctttattgagaatctgatcgacaacggtgatttatatctctttcgcatcaacaacaaagacttctcctctaaatctacaggtactaagaacctgcacactctttatctacaggctatattcgacgaacggaatctgaacaatcctacaattatgctgaatggaggtgcagagctcttctacagaaaggaatctattgagcagaagaatcgcattactcataaagccggctccattcttgtcaataaggtgtgcaaagacggaacctcgttggacgacaagatccggaatgaaatctaccagtacgagaataagttcatcgataccctctctgacgaagccaagaaagtcttacctaacgtgattaagaaggaggcaacccatgacatcactaaagataaacgctttaccagcgataagttcttctttcattgtcctctgactatcaattacaaggagggtgacactaagcaattcaacaatgaagtcttaagcttcttacgcgggaacccagacataaacatcattggtattgatcgcggcgagcggaaccttatatacgtcaccgtgatcaaccagaagggagaaattcttgattctgtgagcttcaatacagttactaataaatcttctaagatcgagcagactgtggactatgaagagaaactggcagtgagggagaaggagcggatcgaggcaaagcggtcttgggactcaatatccaagattgccactctgaaagaaggatacttatctgctatagtccacgagatctgtctgctcatgattaaacataatgctattgtcgtgctggagaatctcaacgctgggttcaaacggattcgcggagggctgagcgaaaagagcgtgtaccagaaatttgagaaaatgctaataaacaagctaaactactttgtctctaagaaggaatctgactggaataagcccagtggtctgctgaatgggcttcagctgagcgaccaatttgaatcgttcgagaagcttggcatccaatccgggtttattttctatgtgccagcggcctatacttccaagatcgatccaactaccgggttcgctaacgtgctaaacttatccaaggtgcgtaatgtggatgccatcaaatctttcttctctaatttcaacgagatttcctattccaagaaggaggccctgttcaagttctcatttgacctggacagcctatccaagaagggtttctcctcattcgtcaaattctctaagagcaaatggaacgtctacacctttggcgaacgcatcattaaaccgaagaataaacaaggatatagggaagataagaggattaatctgaccttcgagatgaagaagctgctcaacgagtacaaagtatcatttgacctcgagaataatcttattccaaacctcacgagcgcaaacctgaaggacaccttctggaaggagctattctttatctttaagactactctacaattgcgtaatagcgtgacaaacggaaaggaagacgtactcataagcccggtcaagaatgctaagggagagttcttcgtgagcggcacgcacaataagaccctgccacaggattgtgacgccaatggagcttatcacatcgctttaaagggcctgatgattctggaacgtaataacctggttcgagaagagaaagatactaagaagattatggccatctccaacgtcgactggtttgaatacgtgcaaaagagaagaggcgtcctctag

SEQ ID NO: 337 - DNA, 4005 bp, Artificial Sequence
  Description of Artificial Sequence: Synthetic polynucleotide
atgtcttctcttaccaagtttacaaataagtactcgaaacagttgaccattaagaacgagcttattcccgtcgggaagacactggagaatattaaggagaacgggcttattgacggcgacgaacaacttaacgagaattaccagaaagccaagatcatcgtcgacgacttcctgagggatttcattaacaaggcacttaacaacacgcagatcggaaattggcgggagctcgcagacgccctgaataaggaagacgaggacaacattgagaaactccaagataagattcgggggatcattgtcagcaaattcgagacattcgatttatttagcagttattcaattaagaaagacgagaagattatcgacgatgacaatgatgttgaagaagaggagctggacctcggtaagaaaacttctagctttaagtatatattcaagaagaacctgttcaagctggtccttccgtcctatttaaagactaccaaccaggacaagctcaagattatttcctccttcgacaacttctctacttactttcgaggtttctttgagaaccgcaagaatatctttacgaagaagcccatctccacctccattgcttacagaatagtccatgacaactttcccaaatttctggataacattcgatgctttaacgtgtggcagacagaatgcccacaactaatcgtcaaagcagataattacctaaagagtaagaatgttattgccaaagacaagtcactcgccaattacttcactgtgggcgcctacgattacttcctgtctcagaatggaatcgacttctacaataacatcatcggtgggctgcccgcctttgcaggacatgagaaaatccagggcctcaacgaatttatcaatcaagaatgccagaaagacagcgagttgaagtcaaagcttaagaatcgacacgcattcaagatggctgtgctgtttaagcagatactgtctgatcgtgagaaatccttcgtgattgatgaattcgaatccgatgcccaggttatcgacgcggtgaagaacttctatgcagagcaatgtaaagacaacaacgtaatatttaatctcctgaatctcatcaagaatatagcattcctcagtgatgacgagttggatggtatcttcattgaaggcaaatacttaagcagcgtaagccagaagctctattctgactggagtaaacttaggaatgatattgaagacagcgcaaactctaaacagggtaataaagagctggctaagaaaattaagacgaacaaaggtgatgttgagaaagccataagtaaatacgagttctccctgagtgagttaaattcgatagtccacgataacacgaagttctccgatctcctgtcatgtaccctacataaggtcgcgtcagagaagttagtgaaggtcaacgagggtgactggccgaagcacttaaagaacaatgaggagaagcagaagatcaaagaacctctggacgccctgctagagatatacaacactttgttgatctttaattgcaagagctttaacaagaatggaaatttctatgtggactacgaccgatgcataaacgagctcagctctgtggtgtatctgtacaacaagaccaggaactattgtacgaagaagccatacaatacagacaagtttaagctcaacttcaactctcctcaattaggcgaagggttctcaaagtctaaagagaacgattgtttaaccctgttgtttaagaaggatgacaattattatgtgggtattatcaggaaaggtgctaagataaatttcgatgacactcaggccattgcggataacactgataactgtatctttaagatgaattatttcttgttgaaggacgcaaagaaattcattccaaagtgcagtattcaactgaaggaggttaaggctcactttaagaagtcagaggatgactatattctttccgacaaggagaagtttgcttctcccctcgtcatcaagaaaagcactttccttctggctaccgcacacgtgaaaggtaagaagggaaacataaagaaattccagaaagaatactctaaagagaaccctaccgaatatagaaattctcttaatgagtggattgcgttctgcaaggagtttcttaagacctataaggccgccacgatatttgacattacaacccttaagaaggctgaggagtacgcggatatcgtcgaattctataaggacgttgataacctgtgctacaagttagagttctgcccgataaagacgagtttcatagagaacctcatagacaatggtgatttgtatctgttcagaattaataataaggacttcagctctaaatcaactggcacaaagaacctgcatactttgtacctacaagccatcttcgacgagagaaacttgaataaccctacaattatgttgaacggtggcgccgaactgttctacagaaaggagtccatcgagcagaagaataggattacccacaaggccggaagcattctggtcaataaggtgtgcaaggacggaaccagtttagatgataagatcaggaacgaaatctaccagtatgagaataagttcatcgatactcttagcgacgaggctaagaaagtgcttccgaacgtgatcaagaaggaggctacccacgacatcaccaaagacaaacggtttacctccgacaaatttttctttcattgccctctgacaattaactacaaagaaggcgatacaaagcagtttaacaacgaagttctctccttcttacgcggcaaccctgacatcaacattataggtatagaccgcggtgagagaaacctgatttatgtgaccgtgatcaatcagaagggcgagatactggactcagtctccttcaacactgtgacgaataaatcatcaaagattgaacagacagtagactatgaagagaaactggcggtgagagagaaagagagaatcgaagccaagagaagctgggattcaataagcaagatcgcaacgttaaaggaaggatacctgagcgccatcgtccatgagatctgtctcctgatgatcaagcacaatgccatcgttgtcctggagaatttaaacgccggcttcaaacgcatacgtggagggctctctgaaaagagtgtgtaccagaaatttgagaagatgttgattaacaaactgaattactttgttagtaagaaggagtccgattggaacaaaccatcgggattactgaatgggcttcagctgtcagaccagtttgaaagtttcgagaaacttggcatccagagcggcttcatattctatgtacctgctgcctatacatctaagattgatccgacgactggatttgctaacgtcttaaaccttagtaaggtgcgaaacgtggatgcaatcaagtccttcttcagcaacttcaatgaaatctcatactcaaagaaggaagcactgttcaagttctcgttcgatttggattccctctcgaagaaaggattctcttcgttcgttaaattctccaagtctaagtggaatgtgtataccttcggtgaaaggattatcaaacccaagaataagcaaggctatcgggaggataagagaattaatctgacctttgaaatgaagaagctcctgaatgagtacaaggtcagctttgacctcgagaacaatctaattcccaatctgacatccgcaaatcttaaggacactttctggaaggagttgttctttatcttcaagacgacactccagttgcgcaactctgtgaccaatggcaaagaggacgttctgatctcgcccgttaagaacgctaagggcgaattctttgttagcggcacacacaataagacgctaccgcaggactgcgatgctaatggcgcctaccacatcgcgttgaagggactaatgatccttgaaagaaataatctcgttcgcgaagagaaagacacgaagaagatcatggccatatcgaacgtcgactggtttgagtacgtgcagaagagacgcggagtgctgtag

SEQ ID NO: 338 - DNA, 4005 bp, Artificial Sequence
  Description of Artificial Sequence: Synthetic polynucleotide
atgagtagccttactaagtttacaaacaagtactctaaacagctcaccataaagaacgagctaatcccagtcggcaagacactcgagaacatcaaagagaatggattgattgacggtgacgaacagctcaacgagaactaccagaaagcaaagatcatcgtcgacgactttctcagagatttcatcaataaggccctgaacaacacccaaatcgggaactggagagagctggctgacgccctgaacaaagaggatgaagataacatcgagaagctgcaagacaagattcgcggaataattgttagtaaattcgagacctttgacctgttctcttcctacagcatcaagaaagacgagaagatcatcgatgacgataatgatgttgaagaggaagagttggatctcggtaagaagacatccagtttcaagtatatcttcaagaagaacttattcaagctggtacttccatcctacctgaagacaacaaaccaggataaactcaagatcatatcctccttcgacaacttctctacctatttccgcggtttcttcgagaaccgcaagaatatcttcacaaagaagccaatctcaacatcaattgcgtacaggatcgtgcatgataacttccctaagtttctggataacattaggtgcttcaacgtgtggcagacagaatgtcctcagcttatcgtgaaggccgataactacctgaaaagcaagaacgtcatcgctaaggacaaatcactcgccaattatttcacagtcggtgcctacgactacttcctgtcacagaacgggatcgacttctacaacaacattataggaggcttgcccgcgttcgccggtcacgaaaagatccagggacttaatgagtttatcaaccaagaatgccagaaagacagcgagcttaaatcaaagttgaagaacaggcatgccttcaagatggctgtgctattcaaacagatcctttctgaccgagagaaatctttcgtcattgatgaattcgaatccgacgcccaagtgattgatgcagtgaagaatttctatgctgagcagtgcaaggacaacaacgtgatctttaatcttctgaaccttattaagaacatcgcgttccttagcgatgatgagttggatggcatctttatcgaaggtaagtacctgtcctccgttagccagaagctgtactccgattggtcaaagctgcgcaacgatatcgaagattctgcaaattcgaaacaaggcaataaagaactggctaagaaaatcaagacaaacaaaggcgatgtggagaaggctatcagcaaatacgagttctcactgtccgagctaaacagtatagtacatgataatactaaattctcagacctactatcctgtacgctccacaaggtcgcctccgagaaacttgtgaaggtgaacgagggcgactggcctaagcacctcaagaataacgaggagaaacagaagattaaagagccactggacgcccttctggagatctataataccctattgatctttaactgcaaatccttcaacaagaatggcaacttctacgtggattacgatagatgcataaatgaactgtcctcagtggtatacctgtacaataagacacgcaactattgtacgaagaagccatacaatacagacaagtttaagctgaacttcaactcaccacagttgggtgaagggttctcaaagtctaaggagaatgactgcctgacattgctattcaagaaagacgataactactacgtgggcattatcagaaagggtgctaagatcaatttcgatgatacacaggcaatcgcagataacaccgacaactgcatctttaagatgaattatttcctgctcaaggacgccaagaagtttatacctaagtgctccatccagttgaaagaggtcaaagcacactttaagaaatccgaagatgactacatcctgtctgacaaggagaaattcgccagccctctcgtgatcaagaaatcaactttcctgcttgccactgcgcacgtcaaaggaaagaaagggaatatcaagaagtttcagaaagaatactctaaagagaatccaactgagtaccgcaacagcttgaatgagtggattgccttctgcaaggaattcttgaagacatataaggcagctacaatcttcgacattactacactgaagaaggccgaggaatatgccgacatagtagaattctacaaagatgttgacaacctgtgctataaactggaattctgtccgattaagaccagtttcatcgagaatttgatcgacaacggcgatctttacctcttcagaatcaataataaggatttctcttcgaagagtactgggactaagaaccttcatacgctgtatctccaggccatcttcgatgaaagaaacctcaacaatccgaccatcatgctaaatggcggtgctgagttattttaccgcaaagaatctatcgagcagaagaataggattacccacaaagccggctcaatattggtgaataaagtatgcaaggacggcaccagcctcgatgataagatcaggaatgaaatctaccagtatgagaataaatttatcgacaccttgtcagacgaagccaagaaagtgttgcctaacgtcattaagaaagaggcaacgcacgatatcacaaaggataagcgattcacatccgacaagttcttctttcattgcccactgaccatcaattacaaggaaggagatacgaagcaattcaacaatgaagttctgtcctttctacgggggaatcctgacatcaacataattggaattgatcgcggcgagcgtaacttaatatacgtgactgtgattaaccagaagggtgagatactcgacagcgtgtccttcaacactgtgacaaacaagtccagcaagattgagcagaccgtcgattacgaagagaaactggccgttcgggagaaagagaggatagaggccaagaggagctgggatagtattagtaagatcgctaccctgaaagagggctatttaagtgccattgtgcacgagatttgtctcttaatgattaaacacaatgcgatcgtagtgctcgagaacctaaatgcaggtttcaagcgcattcgcggtggcctctctgagaaatccgtgtaccagaagtttgagaagatgctgatcaacaagctcaactatttcgtttctaagaaagagtccgactggaataagccttcagggctgttgaacggcctccaactgtccgaccagtttgagtctttcgagaaactagggattcagagcggattcatcttctacgtgcccgccgcatacacttctaagattgatcccacaaccggatttgctaatgtcctgaacctgtcaaaggtaagaaacgtggacgccatcaagtcgttcttcagcaatttcaatgaaatcagctattcaaagaaggaggcattatttaaattctcattcgacttggattccctgtctaagaagggattctctagcttcgttaagttctctaaatccaagtggaatgtatataccttcggagagcggatcatcaaacctaagaataaacaaggataccgcgaggacaagaggataaatcttacctttgaaatgaagaaactgctgaacgaatacaaagtgtccttcgatctggagaacaaccttatcccaaacttgacttctgctaacctgaaggacacgttctggaaagaactcttctttatctttaagaccactttgcagctgagaaattctgtcactaatggcaaggaggacgtcctgattagtcccgtgaagaatgctaagggcgagttctttgtttccgggacccataataagaccctccctcaagattgtgacgccaacggtgcttatcatatcgccctgaagggcctcatgatactagaacgaaacaatctggtgcgggaagagaaggatacaaaaaagatcatggctatttccaatgtagattggtttgaatatgtgcagaaacgacgaggagtgctgtga

SEQ ID NO: 339 - DNA, 4005 bp, Artificial Sequence
  Description of Artificial Sequence: Synthetic polynucleotide
atgtccagtctgacgaagtttacaaacaaatacagtaaacagctcaccatcaagaatgaattgatcccagtgggaaagaccctggagaacatcaaggagaacggtttgatagacggagacgagcagttgaatgagaattaccagaaggcgaagatcattgtagacgacttcctgcgggacttcattaacaaagccctgaataatactcagattgggaactggcgtgaactggcagacgccctcaacaaggaagacgaagataatattgagaaacttcaggataagatccgcggtatcatcgtaagtaagttcgagactttcgacctgttctctagttactcaatcaagaaggatgagaaaatcatagacgatgacaatgatgtggaagaagaggaactggatctcggaaaaaagacctcatcatttaagtatatcttcaagaagaatctcttcaagctcgtgttaccttcctatctcaagaccactaaccaggacaaattgaagatcatcagctcattcgataatttctcaacatactttcgcgggttcttcgagaacagaaagaatatattcaccaagaaacccataagcacaagcattgcctaccgtattgtccacgataactttccaaagttcctggacaatattaggtgcttcaacgtgtggcagacagagtgtcctcagcttattgtcaaagccgataactacttaaagtccaagaacgtaattgcgaaggacaagtctctggctaattatttcaccgttggagcgtatgactacttcttaagtcagaacggcattgatttctacaacaatattatcggcggattgccagccttcgctgggcacgaaaagatccagggactaaacgagttcataaaccaggagtgccagaaggattcagagctgaagtctaaacttaagaataggcacgcctttaagatggccgttctgttcaagcagatcctcagtgatcgggagaaatcgtttgtaatcgatgagttcgagtccgacgctcaggtcatcgacgccgtgaagaatttctatgccgaacagtgtaaggataacaatgttatatttaacctgctcaatttaatcaagaatattgcgtttctgtccgacgatgaactagacgggatatttatcgaaggtaagtatttgagcagcgtttcccagaagctgtatagtgattggagtaaattaagaaacgatatcgaggattcagcgaatagtaagcagggtaacaaggaactcgccaaaaagataaagactaataagggcgacgtggagaaggccattagtaaatacgagttctcccttagcgagttgaattccattgtacatgataatacaaagtttagtgatctgctgtcctgcaccctgcataaggtggcctctgagaaactggttaaggtaaacgaaggagactggcccaagcacctcaagaataatgaggagaaacagaagatcaaggagccgctggacgcactcttagagatttataatacactgttgatcttcaattgtaagagctttaacaagaatggcaatttctatgtggactatgaccggtgcattaatgaattaagtagtgtggtgtacctatataacaagacacggaactattgcacgaagaaaccctataacacagataaattcaagctgaacttcaattctccgcagctgggcgagggattcagtaagagcaaggagaatgattgcctgactctcctctttaagaaggacgacaattactacgtgggcatcatccgcaaaggcgcgaagatcaacttcgatgacacacaggcaatcgctgacaacacggataactgcatctttaagatgaactactttctcttgaaggacgccaagaaattcatacctaaatgttctatccagctcaaagaagtgaaggcacatttcaaaaagagtgaagacgactacatcctctctgataaagagaagttcgccagcccactggtcattaagaagtctaccttcctgttggccacagcacatgttaagggcaagaagggcaatatcaagaagtttcagaaagagtattccaaagagaaccctacggagtatagaaactctctgaacgagtggatcgctttctgcaaggaatttctgaagacctataaggcagctacaatctttgacatcactaccttgaagaaggccgaggagtatgcagacattgtggagttctacaaggacgtggataatctatgctacaagttggagttctgtcctattaagacgtccttcattgagaacctaattgacaacggcgatctctacctgtttagaatcaataacaaggacttctcatccaagtccaccggtacaaagaatctgcacaccttgtaccttcaggctatctttgacgaaagaaatctgaacaatccaaccattatgctcaacggaggtgccgaactgttctacagaaaggaatcgatcgagcaaaagaatagaataacccataaggcaggctcaatcctggtgaacaaagtgtgcaaagatggtacaagtctggacgataagataaggaacgagatttaccaatatgagaataaatttatagacaccctttccgatgaagcaaagaaggtcctgccaaatgttatcaagaaggaggccacacatgacataacaaaggataagagattcaccagtgataagttcttctttcactgtccactgaccatcaattacaaagagggtgacaccaagcagtttaataacgaggtgctgagcttcctgagaggtaatccggacatcaacatcatcggcatcgatcgtggcgagcgcaacctcatttatgttactgtgataaaccagaagggagagatcctggatagtgtgagcttcaacaccgtgactaataagtcatcaaagatcgagcagacggtggattacgaggagaagctggccgtgagagagaaagagaggatcgaggctaagaggtcctgggactcaattagtaagatagcaacgctgaaagagggctatctctccgctatcgttcacgaaatatgcctgttgatgatcaagcataatgccatcgtcgtcctggagaatctgaatgcaggcttcaagcgaatccgcggaggattaagtgagaagagcgtgtaccagaagttcgagaagatgttaatcaacaagctgaattatttcgtgtcaaagaaggagtccgactggaacaaacccagtggcttgctcaatggactgcagctttccgaccagtttgagtcatttgagaaattgggaatccagagtggcttcatattctatgtaccggctgcctacacaagtaagatagatcctacgaccggcttcgcaaacgtgctcaacctctccaaggtacggaatgttgacgccattaagtcatttttctccaatttcaatgagatttcatactccaagaaggaggcactgttcaagttcagtttcgatttggattctctgtctaagaagggtttctcgtcatttgtgaaattctccaagagtaagtggaacgtttacacattcggcgaaaggattattaaaccaaagaacaagcagggatacagagaagacaagagaatcaaccttactttcgagatgaagaagctgcttaatgagtacaaggttagtttcgatctggagaacaatctgatccctaatctcacctcagcgaatctgaaggacacattctggaaggagctgttcttcatcttcaagacaaccctgcagttgcgtaactccgtgacaaatggtaaggaagacgtcttaatcagcccagtcaagaatgccaaaggagaattcttcgtgagcggaacacataacaagactttaccacaagactgtgatgcaaatggagcctatcacatcgctctgaaaggactcatgattctcgaaaggaacaatctcgttcgagaggagaaggacaccaagaagatcatggccattagtaatgtagactggtttgaatatgtacagaagcggcgtggggtattataa

SEQ ID NO: 340 - DNA, 4005 bp, Artificial Sequence
  Description of Artificial Sequence: Synthetic polynucleotide
atgtcttccctaaccaaattcacaaataagtattcaaagcagcttaccatcaagaatgagctgatcccagtcggcaagaccttagagaacatcaaggagaatggcctaattgatggagatgagcaactcaatgagaactaccagaaagcgaagattatcgtcgatgacttccttcgggacttcattaacaaagccctcaacaacacgcagataggcaactggagagagttagcagacgccctaaacaaggaagatgaagataatattgagaagctccaagacaagatcagaggtattattgtgtccaaatttgagacattcgatctgttcagttcttattctatcaagaaggacgagaagattatcgatgatgacaacgacgtcgaggaggaggagctggatctcggtaaaaagacgtcctcctttaagtacatctttaagaagaacttatttaaactggtgcttccaagttacctgaagactactaatcaggacaaactcaagattatctcttccttcgacaatttctccacatactttagaggcttctttgagaacagaaagaatatattcactaagaagccaatcagtacttctattgcctataggatcgttcacgataatttccctaaattcttggataatatcagatgctttaatgtgtggcagactgaatgtccacagctgatcgtcaaggccgataattatctcaagtccaagaacgtgatagcaaaggacaagtcactcgccaattatttcaccgtcggcgcttacgactatttcctcagtcagaatggaatcgacttctacaacaacattatcggtggactcccagctttcgccgggcatgaaaagatccaaggactaaacgagttcatcaatcaggaatgtcagaaggactccgaactcaagtccaagcttaagaatcgccacgcatttaagatggccgtgctgttcaagcaaattctcagcgacagagagaaaagcttcgtcatcgatgaatttgagtctgacgcccaggtgatcgacgcagtgaagaacttctacgcagaacaatgcaaggataataacgtaatctttaacctgctcaatttgataaagaacatcgcctttctgagcgacgacgagcttgacgggatctttatagagggcaaatatctgagcagcgtgagtcagaaactctactccgattggagtaaactgagaaatgacatagaagacagtgctaactccaagcagggcaataaggagctggccaagaagataaagactaataagggcgatgtcgagaaggcgatttctaagtacgagttctctctttcagaattgaattccatcgtgcatgacaataccaaattcagcgacctgcttagctgtacgctccacaaggtggcttcagagaagctcgtaaaggtcaatgaaggagactggcccaagcatctaaagaataacgaggagaaacagaagatcaaagaacctctcgacgcactcctggaaatctataataccctgctgatcttcaattgcaagagctttaataagaatggtaatttctacgtggattacgatcgatgtatcaatgagctatcaagcgtggtgtatctgtacaataagacacggaattattgcactaagaaaccatataacacagacaagtttaaactcaactttaacagtcctcagctaggagaaggcttctcaaagtctaaagagaacgattgtctgacactgctgtttaagaaagacgacaattactacgtaggcattatccgcaagggagcaaagatcaacttcgatgacactcaggctatcgcggacaataccgacaattgtatctttaagatgaactacttcctcttgaaggacgcaaagaaatttatacctaagtgttctatacagctgaaggaggtgaaagcccactttaagaaatccgaggatgactatatcttaagtgacaaggagaagttcgcaagcccgctcgtgatcaagaaatccaccttcctcctggccacagcccatgtgaagggaaagaaaggaaacattaagaagtttcagaaagagtactccaaggagaatccgacggagtataggaattccctgaatgagtggattgccttctgcaaggagttcttaaagacctacaaggctgccacaatattcgacatcacgactttgaagaaggccgaagagtacgctgacatcgtggagttctacaaggatgtggacaatctctgttataaactcgaattctgcccaataaagacatctttcattgagaatttgatagacaatggtgacctatacctgttccggatcaacaacaaggatttctcgtctaagagcaccggaactaagaatttacacacactttacctccaggcgatatttgatgagaggaacctgaataatccaacaatcatgcttaatggcggtgccgagctgttctacagaaaggaatcgatcgaacagaagaaccgaatcactcataaggcgggtagcatcctcgtaaataaggtgtgtaaagacggtacctccctggatgataagattcgtaatgagatctaccagtatgagaataaatttatagacactttgtctgatgaggcgaagaaagtacttcccaacgtgataaagaaagaggctacccacgatattaccaaggataagcggttcacttccgataaatttttcttccattgcccactgactatcaattataaggaaggtgatacaaagcagtttaataatgaagtgctatctttcctgcgtggtaatcctgacattaacatcatcggcatagaccgtggagagaggaatctgatatacgtgaccgtaatcaatcagaaaggtgagatccttgactcagtgagtttcaatacagttacaaataagagcagcaagatcgagcagaccgtggactacgaggagaaattggcggtacgggagaaagagaggattgaagctaaacggtcctgggacagtatcagcaagatagcaaccctgaaggagggataccttagtgcaatcgtccatgagatctgcctgcttatgatcaagcataatgctattgtggttctcgagaaccttaatgccggatttaagagaattaggggcgggctgagcgagaaaagcgtgtaccagaaatttgagaagatgctgattaacaagctgaattacttcgtgtcgaagaaggaatccgattggaacaaaccaagtggactgctcaatggtctccagcttagtgaccaatttgagagctttgagaaactgggcatccaatctggctttatcttctacgtgcccgctgcctacactagtaagatcgacccaactacaggcttcgcaaacgtgcttaatttgagcaaggtaaggaacgtggatgcaattaagtctttctttagcaacttcaacgagatttcctactctaagaaagaggctctatttaaattctccttcgacctcgacagcctctctaagaaaggctttagttcctttgtcaaattctcgaagagtaaatggaacgtgtatacatttggtgaacgcatcattaagccgaagaacaaacaaggctacagagaagacaagcgcattaatctgacatttgaaatgaagaaactgctgaatgaatacaaggtgtcatttgatttagagaataaccttataccaaacctgacatcagctaatctgaaagacaccttctggaaggagttgttctttatcttcaagacaacgctccagttgcgaaattctgtgaccaatggcaaagaagatgtgctgatctctcctgtaaagaatgctaaaggcgagttctttgtgagcggcacgcataacaagactctaccacaagactgcgacgccaatggcgcctaccacatcgcactgaaagggttgatgattctggagagaaacaatctggtccgcgaggagaaggatacgaagaagattatggctattagtaatgtggactggttcgaatacgtgcagaaacgccgaggtgtcctctga

SEQ ID NO: 341 - DNA, 4005 bp, Artificial Sequence
  Description of Artificial Sequence: Synthetic polynucleotide
atgagttcgttaactaagttcaccaacaagtatagtaaacagctgacaataaagaacgagctcatacctgtgggtaagactctggagaatatcaaagagaatggtctaattgacggcgacgagcaactgaacgagaactatcagaaagctaagatcatcgtggatgatttcctgcgggacttcattaacaaagccttaaacaacacacagatcggaaactggagagaactcgctgatgccctgaacaaggaagatgaagataatatcgagaagttgcaggacaagataagaggaatcattgtctctaagttcgaaaccttcgatctgttcagcagctacagtataaagaaagacgaaaagattatagatgacgataacgacgtagaggaggaagagcttgacctgggaaaaaagacttcaagcttcaaatatatcttcaaaaagaacttgtttaagctcgtcctgccaagctatcttaagaccaccaatcaggacaagctgaagattatttccagcttcgacaactttagcacttacttccgcggattcttcgagaatagaaagaatatcttcacgaagaagcctatctcgacaagtatcgcctatcggatagtgcatgataactttcctaagtttctggacaatatcagatgtttcaacgtgtggcaaactgagtgtccacagctaattgtcaaggccgataattacctaaagagcaagaacgttattgccaaggataagagtctggcaaactacttcacagttggtgcctatgactatttcctgagtcagaacggtatcgacttctataacaacataattggagggctgcctgcattcgccggacacgagaaaatacagggactcaatgagttcattaaccaggagtgtcagaaagattctgaacttaagtctaaattgaagaaccgacacgcatttaagatggccgttctattcaaacagattctctccgaccgggaaaagagcttcgtgatcgacgaattcgagtccgacgcccaagtaatcgatgccgtgaagaacttctatgcagagcagtgcaaagataacaacgtgatattcaatctgttgaacctgataaagaacattgcatttctctccgatgacgaattggacggtatatttattgagggcaagtacctctccagcgttagtcagaagttgtactccgattggtctaagctaaggaacgatatagaggactcggctaacagcaaacagggcaacaaggagcttgctaagaagattaagaccaataagggcgatgtggagaaggctattagtaaatacgagtttagcctgtctgaactgaacagcattgtgcatgacaataccaagtttagcgacctgcttagctgcactcttcacaaggttgcaagtgagaaactggtgaaagtgaatgagggtgattggccaaagcaccttaagaacaacgaagagaagcagaagatcaaggagcctttagacgcccttctcgagatttataacactctcctgatcttcaattgtaagtctttcaataagaacggtaatttctacgttgattatgacagatgcatcaatgaactgagctctgtcgtctacctgtataataagacacggaattactgcactaagaagccttacaacactgacaagttcaagctcaacttcaacagtccgcagctgggcgagggcttctccaaatccaaggagaacgattgtctgacactactgtttaagaaggacgacaattattatgtcggtattatccggaagggagctaagatcaacttcgacgacactcaggccatcgctgacaataccgacaactgtatcttcaagatgaactatttcctcttgaaagacgcaaagaaattcatacccaagtgtagcatccagttgaaggaagttaaagcacatttcaagaagtctgaggacgattatatcctgagcgataaggagaagtttgcgtcgccgctggtgattaagaagtccacgttcctcctggcaacggcacatgttaagggtaagaagggaaatattaagaaattccagaaggagtactctaaagagaatcccaccgaatatcggaatagcctaaacgaatggattgctttctgtaaggagtttctgaagacttataaggccgcaaccatatttgacataacaacccttaagaaggctgaggagtatgccgatatcgtagaattctacaaagacgtggacaacctttgctataagctagaattctgtcctattaagacatctttcatcgagaacctgattgataatggcgatctgtacctgtttagaatcaacaacaaggacttctcctctaagagcaccggtactaagaacctccataccctgtacttacaggccatcttcgacgaaagaaatctgaataatccaacaataatgctaaacggcggcgccgaattattttataggaaggaatccatcgagcaaaagaacagaataacccacaaggccggctctattctagtcaacaaagtgtgtaaggatggaacaagtctcgacgataagatccggaacgagatctaccagtacgagaataaattcattgacaccctgtctgatgaggccaagaaggtgcttcccaatgttatcaagaaagaagcgacccacgacatcactaaagataagcgattcacctcggacaaatttttctttcactgtccactcaccataaattacaaagagggtgacacgaaacaatttaataatgaggtcctctcctttctcagaggtaatccagacatcaatatcatcgggatcgaccgaggcgagaggaatcttatctatgtaaccgtcatcaatcagaaaggtgagattctggattccgtatccttcaacacagtgactaacaagtcttccaagattgagcagaccgtggactatgaagagaagctggccgtgcgagagaaagagcggattgaagctaagaggagttgggactccatcagtaagatcgctacgttgaaagaaggctacctcagtgctatcgttcacgagatttgtcttctgatgattaagcataatgccatagtagtgctagagaatcttaatgctgggtttaagcgtataagaggtggtctgtctgaaaagagtgtgtaccagaagttcgaaaagatgctgatcaataaactgaattactttgtgtctaagaaagaaagtgattggaacaagccatcaggccttctcaacggcctgcaattaagtgaccaatttgagtctttcgagaaactgggaatccagtctggcttcatattttacgtacccgctgcgtatacctctaagattgatcctaccacaggattcgcaaacgtgctcaaccttagcaaagttcgcaacgtggacgctatcaagtcattcttcagcaacttcaacgaaatctcatacagtaagaaagaggccttatttaagtttagctttgatctggattctctatcaaagaaagggttctcttctttcgtcaaatttagcaagagtaagtggaatgtgtatacatttggtgaaagaatcatcaagcctaagaacaaacaaggataccgtgaagacaagcgcatcaatctgacgttcgaaatgaagaagttgctaaatgagtacaaagtgtcattcgacctggagaataacttaataccaaacctgaccagcgccaacctgaaggatactttctggaaggaattattcttcatctttaagaccacactccagctgagaaattcagtcacaaacggtaaggaagacgtcctgattagccctgtgaagaatgcaaagggtgaattcttcgtttccggtacccacaataagacccttcctcaggattgcgacgcaaatggcgcttaccacatcgcactgaaaggccttatgattcttgaacgcaacaacctggtgcgggaagagaaggacacgaagaagatcatggccatctccaacgtcgattggtttgagtatgtgcagaagcgccggggtgtgttgtaa

SEQ ID NO: 342 - DNA, 4005 bp, Artificial Sequence
  Description of Artificial Sequence: Synthetic polynucleotide
atgagcagtcttaccaagttcactaacaaatactctaaacagctgacaataaagaacgagttgataccagttggtaagacccttgagaacataaaggagaatgggctgattgacggagatgaacagctgaacgagaattatcagaaggccaagatcatagttgacgacttcctgagagatttcatcaataaggccttaaacaacactcagatcggcaactggcgcgaactggccgacgccttgaataaggaagacgaagataacatcgagaagctgcaggacaagattcgcgggattatcgtgtcaaagttcgagacattcgatctcttctctagctactcaatcaagaaagacgagaagataatcgacgatgataatgatgtggaggaggaagaactagacttaggcaagaagacctcttccttcaaatatatcttcaagaagaacctctttaagcttgtgctgcccagctacttaaagaccactaatcaggacaaactcaagattattagttcatttgataacttcagtacatacttccgcggcttctttgagaatcggaagaacatctttaccaagaaacctattagtactagtattgcatatcggatagtgcacgataacttcccgaagtttcttgacaacatccgctgcttcaacgtgtggcagacagagtgtcctcaactcattgtgaaggcggacaattacttgaagagtaagaacgtcattgcgaaggacaagtctctggcaaactacttcaccgttggcgcctacgattacttcctttcccagaatggaatcgacttctacaataacattataggagggttaccagcctttgcaggccatgagaagatccaaggtttgaacgagttcattaatcaagagtgccagaaggacagtgagctgaagagtaagcttaagaatcgccatgcatttaagatggccgtcttgttcaaacaaatcctctcggacagggagaaatctttcgtaattgacgaatttgagtctgatgcccaagtgattgacgctgtaaagaacttctacgccgagcagtgtaaagataacaacgtcatctttaatctcttaaacctgattaagaatatagccttcctgagcgacgacgagcttgatggcatcttcatcgaaggaaagtacttgagcagcgtgtctcagaaactgtacagtgattggagtaagctccggaacgatatcgaggatagcgccaatagtaagcagggaaacaaggagctggctaaaaagatcaagacaaataagggcgatgtagagaaagccatttccaagtatgagttctctctcagcgagttgaactctatagttcacgataacaccaagttctccgatctcctgtcgtgtactctgcacaaggtagcgtccgagaagctggtgaaggttaatgaaggcgactggcccaagcacctgaagaataacgaggagaagcaaaagattaaggagccgctagatgcactcctggagatatataacacattactgatatttaactgcaagagctttaacaagaacggtaatttctacgttgactacgaccggtgtattaacgagctgagtagcgtggtctacctctacaacaagacccggaactattgcaccaagaagccatacaataccgataagttcaagctcaacttcaatagccctcagctcggcgaaggtttctcaaagagcaaagagaacgactgcctgaccttgttatttaagaaggacgataattactatgttggcattatcaggaagggagcaaagataaactttgacgatactcaggctatagcagataataccgataactgtatcttcaagatgaattatttcttgctgaaggatgccaagaaatttattccgaagtgctctatccagcttaaagaggtgaaagcccattttaagaaatccgaagacgattacattctatccgacaaggagaagttcgcatcaccacttgtgattaagaagagcacgttcctcctggcaacagcccacgtcaagggaaagaagggaaatataaagaagttccagaaagagtattctaaagagaatcccaccgagtatcgtaactccctcaacgaatggattgcattctgtaaagagttcctgaagacctacaaggcggccaccatcttcgacataaccacacttaagaaagccgaagagtacgccgatatagttgaattctataaggacgttgataacctgtgctacaagcttgaattctgtcctatcaagacgtcctttatcgagaacttgatagataacggtgacctttacttgttccgcattaataataaggacttcagcagcaagtccacaggcacaaagaacctccatacgctgtacctgcaggctatcttcgatgaaaggaaccttaacaacccaacaatcatgttgaatggcggtgcagagttattctatcggaaggagagcatcgaacaaaagaacagaattacgcacaaggctggctcaattctggtgaataaggtctgcaaagatgggaccagccttgatgacaagattcgcaacgagatttaccagtatgagaacaagttcatcgacaccttgagcgacgaggctaagaaagttctcccaaatgttataaagaaggaagcaacccatgacatcaccaaggacaaacggtttaccagtgataaattcttctttcactgcccgctgaccattaactataaggagggcgacaccaagcagttcaacaacgaagtgctgtccttcctgcggggcaacccagacattaatattattggtatagataggggcgagcggaacctcatatacgtcactgtgatcaaccagaagggagaaatactggattcagtctccttcaacacagtgaccaataagagtagtaagatcgagcaaacagtggactacgaggagaaactggctgttagagagaaagaaagaattgaggcgaaacgttcttgggattctataagcaagattgccaccctgaaagaaggctacctttccgcaatcgtgcatgaaatttgcttactcatgattaaacacaatgctattgtcgtgctggagaatttaaacgctggatttaagaggatcagaggtgggctctctgagaaatctgtgtaccagaagtttgagaagatgctgatcaacaagctgaattactttgtgtccaagaaagagtcagattggaacaagcccagtgggcttctcaatggcctacagcttagcgaccagtttgagagcttcgagaaacttgggatccagtcagggtttattttctacgtaccagctgcttatacatcaaagatcgacccgaccactggtttcgcaaatgtattaaacctgtccaaggtgaggaacgtggacgccattaagagcttcttcagcaacttcaacgaaatctcttatagcaagaaagaggccttattcaaattctcctttgatttagactccctgtctaagaagggcttctcatcattcgttaagttctctaagagcaaatggaatgtctacacctttggcgagcgcatcatcaaaccgaagaataaacagggttatagggaggacaaacgaattaacctgactttcgagatgaagaagctacttaatgaatataaggtttccttcgacctggagaataatcttattcccaatttgactagcgccaatctaaaggacacattctggaaggagttgttctttatctttaagacaactctgcagctgagaaacagcgtgacaaatgggaaagaggacgtccttatttcgcctgtaaagaatgcaaagggcgaattctttgtgagcggaacccataataagaccctcccacaggattgtgatgctaacggcgcctaccacatagctctcaaaggtttaatgatcctagagagaaacaacttagtacgcgaagagaaggatacaaagaaaatcatggctatttcaaatgtggattggttcgaatatgtgcagaagagacgtggagtcctgtga

SEQ ID NO: 343 - DNA, 4077 bp, Artificial Sequence
  Description of Artificial Sequence: Synthetic polynucleotide
atgggaaagatgtactatttaggcctcgacattggaacgaatagtgtcggctatgctgttactgatccaagctaccacctcctcaagtttaaaggtgagccgatgtggggggcgcatgtattcgcagccggaaaccagagtgcggagagaaggtccttcaggacatctagacgcaggttggataggcgacagcaacgggtgaaattagtacaagagatattcgctcccgtcattagtcctattgatcctcgattctttattagactccatgagagtgctctatggagagatgatgtcgctgagactgataaacatattttctttaatgatccgacctatactgacaaggaatattattcagattatcctacaatccatcacttgatcgtcgatctgatggagtccagtgagaaacatgatcctcgtttggtgtatttggcagtggcatggcttgtagcgcatcgaggtcacttcttgaacgaagttgataaggataacataggagatgtgctatcctttgacgcattctatcccgaatttctcgcattccttagcgataatggagtctcgccatgggtatgtgaatcgaaggccttacaagcgacccttctttctcgcaactcagtaaatgataaatacaaagcattaaagtctctcatcttcggatcccagaagcccgaagataactttgatgctaatatctcagaggatggtctcattcaattactcgctggcaagaaggtaaaggttaacaagttgttccctcaggaatctaacgatgcgagtttcactctaaacgacaaggaggacgctattgaggaaatccttggaactttaactcctgatgaatgcgaatggatagctcacatcaggaggctgttcgattgggctattatgaaacacgcattgaaggatggtcgaactatatctgaaagtaaggtgaagctgtatgaacaacatcatcatgacttgactcagcttaagtatttcgttaagacttatcttgctaaggaatatgatgacatcttccgtaatgtcgattccgaaacaaccaagaactatgttgcttattcatatcatgtgaaggaggttaaaggaacacttcctaagaacaaagcaacccaagaggagttctgcaagtatgtactcggtaaggttaagaatattgagtgctcagaagccgataaagttgacttcgatgagatgatacaaagactcacagacaattcctttatgccgaagcaagtgtctggtgagaatagagtaattccataccaactctactactacgagcttaagacgatccttaataaggctgcttcatacctaccattccttactcagtgtgggaaagatgcgatttctaaccaggataagctgctctcaattatgacgttcagaataccatacttcgtcgggcctctgaggaaggataattctgaacatgcctggcttgagcggaaagctggaaagatctatccgtggaacttcaacgataaagtggatttagataagtcagaagaggccttcatcaggagaatgaccaatacatgcacctactatccaggtgaagacgtgctgccgttagatagtttgatttacgagaagttcatgatactgaacgagataaataatattagaattgatggataccctatctcagtcgatgtgaagcaacaggtgttcggattgtttgaaaagaaaaggcgagtcactgtgaaagatatacagaatttgttgttatctttaggcgcacttgacaaacacgggaaattaactggtattgatacgactatccacagtaattacaacacctatcatcactttaagtctcttatggagcgcggagtcctgacacgtgacgatgtcgagaggatagtggaacgaatgacctactcggatgatactaaacgggtgaggttatggctaaataataattatggcacccttacagctgatgacgttaagcacatcagccgtctacggaagcatgactttggtcgactgtcaaagatgtttcttacaggattgaaaggagtccataaggagactggtgaaagggcctcgatcttggatttcatgtggaacacaaacgacaatttgatgcagcttctttcggaatgctatacatttagcgatgaaattactaagttacaagaagcctactacgctaaagctcaactgagtttaaatgatttcttggacagtatgtatatttcaaacgccgttaagagaccaatctaccgtactttagcagtcgtgaatgatattcgtaaggcatgcggtactgctcccaagcgcatattcatagaaatggctagagatggcgagagtaagaagaagaggtccgttactagacgagagcagattaagaacctatataggtcgatccgcaaggacttccagcaggaggtcgactttcttgagaagatcctggagaacaagtctgatggacagttgcagagcgacgccctttacctttactttgctcaacttggtcgtgacatgtacacaggcgacccaatcaaattagaacatattaaagatcagtcattctataatatcgatcacatttaccctcaatccatggtgaaagatgacagtcttgataataaggttctagtgcaatccgaaatcaatggtgagaagtccagtcgttatccactcgatgccgctataagaaacaagatgaaacctctttgggacgcttattataaccatgggctaatatcattaaagaagtaccagcgtttaactaggtctacacccttcacagatgacgagaagtgggacttcattaataggcaacttgttgaaaccagacaatccaccaaggctcttgctattcttctcaagcgaaagtttcccgacactgagatagtctacagtaaggccggtttgtccagcgatttccgtcacgagttcggtttggttaagagcagaaatattaacgacttgcaccatgctaaggacgctttcttagctattgtcactggcaatgtctatcatgagagattcaatagaagatggttcatggtcaaccaaccttactctgtaaagacgaagacactattcacacatagtataaagaacggaaatttcgttgcatggaatggagaggaggaccttggtcgaattgtcaagatgctcaaacagaataagaacacaatccatttcacgcggttctcattcgataggaaagagggattatttgacatacaacctctcaaagcttcgaccggactagtgcctaggaaagcgggtctagatgttgtgaagtacggtggttacgataaatctactgctgcttattatttactagttaggttcacattagaagataaaaagacccaacacaaattgatgatgatcccagtagagggtctatataaggctcgcattgaccatgacaaggagttcttgaccgattatgctcaaactaccatatcggaaatattacagaaagataaacagaaagtaattaacattatgttccctatgggtaccagacacataaagcttaatagtatgatcagcatcgatggtttctatttgtctattggtggtaagtcttctaaagggaaatcagtgctttgtcatgcaatggtacctctaattgttccgcacaagattgaatgttatattaaggctatggaaagctttgctaggaagttcaaggagaataacaagttacgcatcgtagagaaatttgataagattactgtcgaagataatttgaatctttacgagctattcttacagaaactccaacataatccgtacaacaagtttttctcgacccaatttgacgtccttacaaacggacgttctacgttcacgaaattaagtccggaggagcaggttcagaccttacttaatatcctgtccatcttcaagacatgccggtcatctggttgcgatctcaagagtattaatggttctgcccaggcagctcgaattatgatcagcgcagacttgacaggtttatcaaagaagtacagtgatattagattagtggagcaatccgcctccggactgtttgtttccaagtctcagaatttgcttgaatacctatga

SEQ ID NO: 344 - DNA, 3717 bp, Artificial Sequence
  Description of Artificial Sequence: Synthetic polynucleotide
atgaacaattacgatgaatttactaagctttatcctatccagaagaccataaggttcgaattgaagccgcagggacgaacaatggaacatctcgagacattcaatttctttgaggaagaccgtgatcgtgccgagaaatacaagatcctcaaagaagccattgacgaatatcataagaagtttatagatgagcacctaactaacatgtcacttgattggaattcgcttaagcagatttccgagaaatattacaaatcccgtgaagagaaggacaagaaggtcttcctttccgaacagaaaaggatgaggcaagaaatcgtttcagagttcaagaaagatgacagatttaaggatttgttcagtaagaaactcttctcggaattgctcaaggaggagatctataagaaagggaatcatcaggaaatcgatgcactcaaatcgtttgataaattctccggttactttattgggttacatgagaaccgaaagaacatgtattccgacggagatgaaattacggctatttcaaatagaattgtgaatgagaatttccctaaattccttgataacttacagaagtaccaagaagcacgaaagaagtatcctgagtggattatcaaagctgagagcgcactggtggcccataacattaagatggacgaggtcttcagcttggaatacttcaataaggtgttaaatcaggagggaatacaaagatataatttagcacttggcggctatgttactaagagtggagagaagatgatgggattgaacgatgcgctgaacttagcccaccaatcagaaaagagtagcaaaggccgtatccatatgactccactctttaaacagatactgtctgagaaggaaagtttctcttatattcctgatgtattcacggaagattctcagcttctaccatccataggtgggttctttgcccaaatagagaatgataaggatggtaatatcttcgatcgagctttagagttgattagttcttatgccgagtacgacacagagagaatctatatccgacaggcggatatcaacagggtgagcaatgtaatctttggtgaatgggggactctgggcggtcttatgcgtgagtacaaggctgattctatcaatgatattaacctagaaagaacttgtaagaaggtcgacaagtggctggatagcaaagagtttgcattgtccgatgtcttggaggctatcaagcgtactggcaataacgacgccttcaacgaatatatatccaagatgcgtacagccagagaaaagatcgatgccgcgcgtaaagagatgaaatttatctctgagaagatcagtggagacgaagagtccatccacattataaagactcttcttgactctgtgcagcagttcttacatttctttaacttgttcaaggcacggcaagacattcctctcgatggcgcgttctacgctgagttcgatgaggtgcatagcaaactgtttgccattgtgcctctatataataaggttagaaattacctaacaaagaataatctcaatacaaagaaaatcaaactgaattttaagaatcctacattagccaatggttgggaccagaacaaagtgtacgactatgcgtcgctcatctttcttcgcgacggaaactattacttaggaattatcaatccgaagcgcaagaagaacattaaatttgagcaaggcagcggtaatggacctttctacaggaagatggtctataagcaaattccgggaccaaataagaacctacccagagtattcttgacttcaacgaaagggaagaaagaatacaaaccttccaaagaaatcatagagggttacgaggccgacaagcacatccgtggtgataagttcgatctcgatttctgccacaagttgattgatttctttaaagagtccatcgagaagcataaagactggagcaagttcaacttctacttctcgcctactgagagttacggagacataagcgagttctatttagatgttgagaagcaaggttacagaatgcacttcgagaacatctcggctgaaactatagatgaatacgtcgagaagggtgatttgttcctatttcaaatatataataaggactttgttaaagctgctaccggtaagaaagatatgcatacgatatattggaatgcagcgttcagtcccgagaacctccaagatgttgttgttaagcttaatggagaggcggaattgttctacagagacaagtctgatattaaagaaattgtgcatagagagggagagatcctggttaatagaacgtacaacggtagaacgcctgtccctgacaagattcataagaagcttacagactaccataatggacgaaccaaggaccttggagaagctaaggaatatttggacaaagtgcggtatttcaaagctcactacgacatcacgaaggatcgacgttatttaaacgacaagatctactttcatgtacctctcactttgaactttaaggccaatggcaagaagaatttgaataagatggttatagagaaattcctgtcggatgagaaagcacacattattggaatagatcggggcgagcgtaatttgctgtactattcaattatagatcgttcgggtaagatcatcgatcagcagtcattgaatgtaatcgatggctttgattatagagagaaactcaaccagagagaaattgagatgaaagacgctaggcaatcgtggaacgcaattggcaagattaaagatttgaaggaaggttatctcagcaaggccgtccacgagattactaagatggccatacagtataacgctattgtcgtgatggaagaacttaactacggattcaagcgcgggcgattcaaagtcgagaaacaaatctaccagaaattcgagaacatgcttatagataagatgaattatttagtgttcaaagatgctcctgatgagtcaccaggtggagtacttaatgcttatcagctgacaaacccgctggaatcctttgccaagctaggtaagcaaacagggatcttattctatgttcctgctgcttacactagcaagatcgacccaacgacaggattcgtcaacttattcaacacgtcttccaagacgaatgctcaggaaagaaaggagttcttgcagaagtttgaatctatttcttactcagctaaggacggtggaatatttgctttcgcctttgactatcgtaaatttggtacaagcaagacagatcataagaacgtgtggacagcttacacgaatggagagagaatgcgttatattaaggaaaagaagagaaatgagttgttcgatcccagcaaggagattaaggaggctcttacatcttctggcatcaaatacgatggaggacagaatatcctgccagacatccttcgttctaacaacaacggattaatatatacgatgtactctagcttcatagctgcaattcagatgcgggtctatgatgggaaggaggattacatcatatcacccatcaagaacagcaaaggtgaattctttcgtacggatccaaagagaagagagctcccaatcgacgcagacgccaatggagcttataacattgcacttcgaggtgagttgactatgcgggccatcgccgagaaattcgatcctgatagcgagaagatggcgaagttagaactcaagcataaggactggttcgaattcatgcaaacacgtggagattaa

SEQ ID NO: 345 - DNA, 3708 bp, Artificial Sequence
  Description of Artificial Sequence: Synthetic polynucleotide
atgcatacaggaggtcttctttcaatggatgctaaagagttcaccggacaataccctttgtctaagacactccggttcgaattacgcccaatcggacgcacgtgggataatttggaggcttctggatatctcgcagaggatagacatagagctgaatgttatcctagggcaaaggaattgttggacgataatcatagggcatttctcaatagagtgttgccacagattgacatggattggcacccaatagctgaggcattctgcaaagttcacaagaacccgggtaataaggaattagcacaggattacaacttgcagcttagcaagcgacgaaaggagatttcggcttatttacaagacgctgatgggtataaaggcctatttgccaagcctgctctggatgaggccatgaagattgctaaggagaacggaaacgaaagcgatatagaggtgttggaagccttcaacggattctctgtttacttcacgggatatcatgaatcacgagagaatatttactctgatgaggatatggtatctgtagcttacaggatcaccgaagataacttcccaaggttcgttagcaatgcgcttatatttgataagctgaacgaatcacatcctgacattatttctgaagtttctggtaatcttggagtagatgacattggaaagtacttcgatgtaagcaactataacaactttctgtctcaagctggaatcgatgattataatcacataattggaggacatacaactgaagacggcttgatacaagctttcaatgtggttctgaacctgcgccaccagaaagatccgggcttcgagaaaatccaattcaagcaactttataaacaaattctttcagttagaacttccaagagttacattcccaaacaattcgataacagtaaggaaatggtggattgtatctgtgattacgtgtccaagattgagaagagcgagaccgttgaaagggcacttaaattggtgagaaatatctcctcgttcgaccttcgaggtatcttcgtaaataaaaagaatttgcgaatcttatcaaataagcttattggagactgggacgccattgaaaccgctctaatgcattcttcttcttctgagaacgacaagaagtcagtatatgactcagcagaggcattcaccttggatgacattttctcttcagtcaagaaattctcagatgcgagtgctgaagatatcgggaaccgggctgaagacatctgtagggtcatctcggaaactgcacccttcattaatgacttgagagctgttgatcttgattccttgaacgatgatgggtatgaagccgctgtttcgaagattcgcgaaagcttggagccttatatggatctctttcatgaacttgagatattcagtgttggtgatgaatttccgaaatgcgcggccttctattcggagctcgaagaagtatcggaacagttgattgagataattccactattcaataaagctcggagtttctgcactcgtaagagatattcgacagataagatcaaggtgaatttaaagtttcccaccctggctgatggatgggacctgaacaaagagcgcgataacaaagcggcaatactccgtaaagatgggaagtattatttagctattctcgatatgaagaaagatctctcttcaatccggacatcagatgaagacgagtcttcattcgagaagatggaatacaaactattaccgtcgcctgtaaagatgctcccaaagatcttcgtcaaatccaaagcagcgaaggagaaatacgggctcacagatagaatgttggagtgctacgataagggtatgcacaaatcaggtagtgctttcgatctgggattctgtcacgagttgattgattattataagagatgtattgcggaatatcctgggtgggacgtgtttgatttcaagtttcgtgaaacctccgactacggcagcatgaaagagttcaacgaggatgttgctggtgctggctattatatgtctcttaggaagatcccttgttccgaggtttaccgacttcttgatgagaagagtatatacctattccagatttataacaaggactattctgagaatgctcatggaaacaagaatatgcatactatgtactgggaaggactcttctccccacagaacctcgaatccccagtcttcaaactttccggaggcgcagaactcttcttcagaaagagttctattccaaatgatgcgaagaccgttcatcctaagggcagcgtgttagttcctcgaaatgatgttaatggaagacgaatccctgacagtatatacagagaactaaccagatatttcaatcgaggtgattgcagaattagcgatgaagctaaatcttatttggacaaagttaagactaagaaagcagatcacgatatagttaaggatagacgcttcacggttgataagatgatgtttcacgtacctatcgcaatgaacttcaaagccatatccaaaccaaatttgaataagaaggtaatcgatggaataatcgatgatcaagatttaaagattataggtattgatcgtggtgagagaaaccttatctatgttactatggtggaccgcaagggaaacattctttaccaggattcactgaatatcctaaacggttacgattatcgcaaagcccttgacgtgagagaatatgataataaagaagctagacggaactggactaaagtcgaaggtattagaaagatgaaggaaggatacctcagccttgctgtttctaagttggcggacatgattattgagaacaacgcaatcatagttatggaggacctgaatcatggattcaaagctggaaggtctaagattgagaagcaagtctaccagaagttcgaatctatgttgatcaataagctcggttatatggtgttgaaggacaagagtatagatcagagcgggggagctcttcatggctatcaattggccaaccacgtgactactttagctagtgtgggaaagcagtgcggagtcatattctacatcccagcagcgttcacgtcaaagattgacccgactactggtttcgctgatttatttgcacttagtaatgttaagaacgtggcttcaatgagagaattctttagtaagatgaaatcagtgatttatgacaaagctgagggtaaatttgcatttacgttcgattaccttgattacaatgtgaaatctgaatgcggtcgtaccctttggactgtatacacagttggtgagagattcacgtactcacgggtgaatagggagtacgtgcgtaaggttcctacagatataatttatgatgctctacagaaggctggcatatcagttgaaggtgatttgcgcgaccgtattgcagagtccgatggagataccttaaagtccatattctatgcattcaagtacgcactagacatgcgagttgagaatagagaagaggactacattcagtcgcctgtgaagaatgcatcaggtgagttcttctgctctaagaatgctggaaagagtctcccacaggatagtgatgcaaatggtgcatataatatcgctttaaagggtatactgcagttacgcatgttaagtgaacaatacgatccaaatgcagaatctatcaggctcccactaatcactaacaaagcttggttgacattcatgcaatctggcatgaagacttggaagaattaa

SEQ ID NO: 346 - DNA, 3783 bp, Artificial Sequence
  Description of Artificial Sequence: Synthetic polynucleotide
atggattctcttaaggatttcaccaacctttatccagtatctaagacactaaggttcgagttaaagcctgtggggaagacactggagaacatagagaaagctggaattctgaaagaggatgaacatagagcagaatcttacagaagagtcaagaagatcattgatacatatcacaaagtcttcattgactcgagccttgagaacatggctaagatgggaattgagaacgagattaaggctatgctccaatcattctgcgaattatataagaaggatcataggaccgaaggtgaggataaggctttagataagatccgtgcagttcttcgtgggcttattgtgggagctttcactggagtctgtggaaggagggagaatacggtgcagaatgagaagtacgaatcgctcttcaaagagaaactcattaaagaaatcttaccagatttcgttcttagtaccgaggctgaaagccttccattctctgttgaagaggcaactcggtctcttaaggaatttgattccttcacctcatacttcgcgggcttctatgagaatcgcaagaacatatacagtaccaaacctcaaagtacggctattgcgtaccgattgatccacgagaatctcccgaagttcatagataacatactggtattccagaaaataaaggagccaatagctaaagaattggagcatatccgagccgatttctcagccggtggttatataaagaaggatgaacgcttagaggacatattttccctcaattactacatacatgtactaagtcaggctggaattgagaagtataatgctctcatcggcaagatcgtcacagaaggagacggtgaaatgaagggtttgaatgaacatattaacttgtacaatcaacagcgtggtagggaagataggttgccattatttagaccgctctacaaacaaatactcagcgatagagagcaacttagttatttaccagaatctttcgagaaagatgaagaattattgagagccttgaaggaattctatgatcacatcgcagaagatatacttggtagaacacaacagctgatgacgagtatttcggaatatgatctgagtcgcatctacgtcaggaatgactcacaattgacggatatttcaaagaagatgttgggtgattggaatgctatctacatggcaagggaacgtgcatatgatcacgaacaagctcctaagcgtattacagctaagtacgagagggatagaattaaggctctcaagggagaagaatctatctcattggcaaatttgaactcatgtatcgccttcttagacaacgtaagggactgtcgtgttgacacatatctttccactcttggtcagaaggaggggccacatggattatcgaatttggttgagaacgtcttcgcttcataccatgaagctgaacaactactaagtttcccatacccggaagagaataacttgatccaagataaggataatgtcgtgttgatcaagaacttgctagataatataagcgatcttcagaggttccttaaacctctctgggggatgggcgacgaacctgataaggatgaaaggttctatggagaatacaattatattagaggtgcattggatcaagttatacctctttacaacaaagttcgaaattacctcactcgtaaaccatatagcacacgtaaagtcaagttaaacttcggtaattcacagttgctttcgggatgggaccgaaacaaggagaaggataatagctgcgtgatcctgaggaaaggccagaatttctacttggccataatgaataacagacataagagatcctttgagaataaagtgctccctgagtataaggaaggagaaccatatttcgagaaaatggactacaaatttctccctgatcctaacaagatgttgcccaaggtattccttagcaagaaaggaattgagatctataagccaagtcccaagctactggaacaatacggacatggtacacataagaaaggcgatacatttagtatggacgatctgcacgaacttatcgacttcttcaagcactctattgaggcgcatgaggattggaaacagttcggattcaaattctcagatactgctacgtacgagaatgtttcttccttctacagggaagttgaggatcaaggttacaaactgtccttcaggaaggtgagcgaatcttacgtttattctttgattgatcagggtaagctttatttgttccaaatttataataaagacttctctccttgttccaaaggtacaccaaacctccatacgctatactggagaatgctatttgatgagagaaacctcgctgatgttatctataagctcgacggcaaggcagagatcttcttccgtgagaaatcattaaagaacgatcatccaacccatccagctggtaagccaatcaagaagaaatcacggcagaaaaaaggagaggaatctctattcgagtacgatttagttaaggatcgccattataccatggataagtttcaatttcacgttcctataactatgaacttcaaatgctctgctggctccaaagtcaatgatatggtgaatgcacatattagagaggccaaggatatgcatgttataggaattgatagaggagagcgtaacctgctatatatctgcgttattgattccagagggactatactagatcagatttcactgaatacgatcaatgacattgattaccatgatcttctcgagtctagagataaggatagacagcaggaaaggcgtaattggcaaactatcgaagggattaaagaactaaagcagggatatcttagccaggcggtgcatcgcattgcagaattaatggttgcctacaaggccgttgttgctttggaagaccttaacatgggattcaagcgcgggagacagaaagttgaatcttctgtctatcagcaattcgagaagcaacttattgataaactgaactatctcgtagataaaaagaaaaggccagaggatatcggtggtctattacgggcataccagttcactgcacctttcaagtcctttaaagagatgggtaaacagaacggctttctcttttacattccagcgtggaacacatccaatatcgatccaacgaccggatttgtaaacctgtttcatgctcaatatgagaatgtagacaaggcgaaatcattctttcagaagttcgatagtatatcctataaccctaagaaggattggttcgagtttgcgtttgattataagaacttcaccaagaaagctgaagggtcacgatcgatgtggattctctgtactcacggaagtagaattaagaactttcgcaattcccagaaaaacgggcaatgggattctgaggaatttgcgcttaccgaggcattcaaatcattgttcgtgagatacgagatcgattacactgcggatttgaagactgcaatagtcgatgagaaacagaaggatttcttcgtggatctccttaagttatttaaactcaccgttcagatgcgcaattcatggaaggagaaagatttggattatctaatctctccagtggcaggtgcggatggacggttcttcgacactcgtgaaggtaacaaatccctccctaaagatgcagatgctaacggtgcttacaatattgcactaaagggactgtgggcattgaggcaaatcagacagacttccgaaggaggtaaacttaagcttgctattagcaacaaggaatggcttcagttcgttcaggaacgatcatacgagaaggattag

SEQ ID NO: 347 - DNA, 3957 bp, Artificial Sequence
  Description of Artificial Sequence: Synthetic polynucleotide
atgaccaacaaattcactaaccagtattcactatcgaagaccttaaggttcgaactcataccacaaggaaagacattggagttcattcaggagaagggtttactatcacaggacaaacagcgtgccgaaagctaccaagagatgaagaagaccatcgataagtttcataagtactttatcgatttggcactttctaacgcgaaactcactcatctagagacctacctggaactttataataagagcgctgagacaaagaaggagcagaagttcaaggatgacttgaagaaggtgcaggataacttgaggaaagaaatagtgaagagcttctctgatggagacgccaaatcgatcttcgccattctggacaagaaggaacttataaccgtggagctcgagaaatggtttgagaacaatgagcagaaagatatttacttcgacgagaaatttaagacgttcactacttatttcactggattccatcagaaccgcaagaacatgtattccgttgaacctaatagtaccgccatcgcttataggttaatacacgagaatctcccgaaatttctggagaacgcaaaggcatttgagaaaattaagcaggttgaatcactacaagtcaacttcagagaactcatgggtgaattcggtgatgaagggctaatattcgtgaacgagttggaggaaatgttccagattaattactacaacgatgttctatcccagaacgggattacaatttacaatagtataatctctggatttacaaagaacgacattaaatataagggacttaatgaatacatcaacaattataatcaaactaaggacaagaaagacagattacctaagctgaagcaattgtataaacaaatcctctcagaccgtatcagtctctcgttcttgcctgatgcatttacagatgggaaacaggttcttaaagcaatattcgatttctataagattaacttgttgagctacaccatagaaggtcaagaagaatctcagaacctcttgcttcttatcagacagacaattgagaacctctctagctttgatactcagaaaatttacctcaagaatgatacacacttgacaactatttcccaacaagtgttcggcgacttctctgtgttctctacagcattgaactattggtacgagacaaaggtcaatcccaaattcgaaactgaatacagtaaggctaatgagaagaagagagaaatccttgataaggccaaggccgtcttcactaagcaagattacttcagtattgctttccttcaggaagtcctctcagagtatattctcaccttggatcacacctctgatatcgtcaagaaacatagtagtaattgtatagcggattactttaagaatcacttcgtagcaaagaaagagaatgaaactgataagacgttcgatttcattgcgaatattactgcgaagtatcagtgtatccagggaatccttgagaatgccgatcagtacgaggatgagcttaaacaagaccagaaactcatcgataaccttaaattctttcttgacgccatccttgagctgcttcactttatcaaaccactgcatcttaaatctgaatctattacagagaaggacacagcgttctatgatgtattcgagaactactatgaggcgctatccctcttgacgcctctgtataacatggttcgtaactacgtaacccagaagccatattctactgagaagattaaactaaactttgagaacgcacagctgctgaacgggtgggacgcaaataaggagggtgattatctgacaacgattctgaagaaagacggaaattactttctagcaattatggacaagaagcacaacaaggcattccagaaattcccggaaggcaaggagaactatgagaagatggtatacaaattgctgcctggcgtcaacaagatgttgccaaaggtattcttttcgaataagaacatagcttatttcaacccttctaaagaattattggagaattacaagaaggagacgcacaagaagggagataccttcaatcttgagcattgccacactttgattgatttctttaaggattctttgaacaaacacgaggattggaaatactttgacttccagttctctgagacaaagtcttatcaagatctatccggattctacagagaagttgagcaccagggatacaagattaactttaagaacattgattctgaatacattgatggtcttgtcaacgaaggtaaactgtttttattccaaatttacagtaaagatttctcgcctttctctaagggtaagcctaacatgcataccctctactggaaagcgctattcgaagagcagaacctccagaatgtgatatataagcttaatggtcaggctgagattttctttcgaaaggcctcaattaagcccaagaatatcattcttcataagaaaaagatcaagatcgctaagaagcacttcatagacaagaaaactaagactagtgagattgttccagtacaaaccataaagaacttgaacatgtactatcagggtaagatatcagagaaagaactaacccaggacgacttgcgttacattgacaacttcagtatatttaatgagaagaacaagaccatcgacataattaaggataaacgtttcactgtggataagtttcaatttcatgtgccgatcacaatgaacttcaaagctactggcggttcctacattaaccagaccgtactcgaatatcttcagaacaacccagaagttaagataatcggattagaccgtggagagcgacatcttgtctacctgacattaattgatcaacaaggtaacatcctcaagcaggaatctcttaataccataactgattctaagatttctactccatatcataagcttcttgataacaaagagaatgagcgagaccttgcgcgtaagaattggggaacggttgagaacataaaggagcttaaagagggttatatcagccaggtggtgcacaagattgctacattaatgttggaggagaatgctattgtggtgatggaagatctcaacttcggatttaagagaggtaggttcaaggtagagaagcaaatttatcagaagttggaaaagatgctgatcgataagttgaactatcttgtcttgaaagataagcaaccgcaagagcttggaggactctataacgctctgcaattaacaaacaagttcgagtccttccagaaaatgggtaagcagtcagggttcttgttctacgtaccggcatggaatacgtctaagatagatccaactacaggctttgttaattacttctataccaagtacgagaacgtggataaggccaaggctttctttgagaaattcgaggctatccgcttcaacgcagagaaaaagtatttcgaatttgaagtcaagaagtactctgatttcaatcctaaagcggaaggaacgcaacaagcttggactatatgtacatatggagaacgcatagagaccaagaggcagaaagatcagaacaacaaatttgtctctacgcccataaaccttaccgaaaagatcgaagatttccttgggaagaaccagattgtttacggtgatggtaactgcatcaagtcacaaattgcttccaaggacgataaggcattcttcgaaactctgctatactggttcaagatgacactacaaatgcgtaattcagaaacacgaaccgatatagattacctcatatcaccagtgatgaatgacaatgggacattctacaattctcgtgattacgagaagttggagaatcctaccctacctaaggatgctgacgctaacggtgcctatcatattgccaagaaaggattgatgctcctgaataagatcgaccaagcagacctaacaaagaaggtggatctttcaatttcaaacagggattggttacaattcgttcagaagaataagtga

SEQ ID NO: 348 - DNA, 4023 bp, Artificial Sequence
  Description of Artificial Sequence: Synthetic polynucleotide
atggagcaagagtactatctgggtcttgatatgggtacagggtctgttgggtgggcagtcaccgattcggagtaccatgtattgcggaaacatggaaaggcgctttggggggtcaggttgttcgagtccgcatcgaccgctgaggaacgccgtatgtttcggacaagtagacgtagacttgataggcgaaactggaggatcgaaatattgcaggagatattcgccgaggagataagcaagaaagatccagggttcttcctacgtatgaaagagtctaagtactaccctgaggataagcgtgatataaatggaaactgtccagagctgccttacgcgctctttgttgatgatgacttcactgataaagattatcataagaagtttcctaccatctaccatttgcggaagatgttaatgaacacggaagagactcctgatattcgacttgtgtaccttgcgatacaccacatgatgaagcatcgtggacatttcttgctgtcgggtgacatcaacgaaattaaagagttcggaaccactttctccaagctcctggagaatataaagaacgaagagttagattggaatttggaattgggcaaggaagaatatgcggttgtggagtctatactcaaggataatatgctcaatcgctccaccaagaagacgcgtttaattaaggctctcaaagctaagtcgatttgcgagaaggcggtgcttaacttactggccggaggaacggttaagttgagcgacatctttggcctggaagaactgaatgagacagagcgacctaagatctctttcgctgacaacggttacgatgattatattggtgaggtggagaacgagcttggcgagcagttctacatcatagaaacagctaaagcagtttatgactgggctgtacttgtcgaaatattgggtaaatatacttcgattagcgaggcaaaggttgcaacatatgagaagcacaagagcgacttgcaattcctgaagaaaatagtaagaaagtatctcactaaggaagagtataaagacatattcgtcagcacgtccgataagctcaagaattatagtgcttatatcggcatgactaagattaatggaaagaaggtcgatcttcagtcaaagcgttgtagtaaagaagagttctatgacttcatcaaaaagaatgtgctgaagaagctggaaggtcagccggagtatgagtatttgaaggaagaactggaaagggagacgttcttgccgaagcaagttaatagagataacggcgttattccttatcaaatccacctctacgaactcaagaagatactcgggaatttgcgtgacaagattgatctaattaaagagaacgaggataaactggtgcaattatttgagtttagaattccatactatgttgggcctttgaataagatagacgatggaaaggaagggaagtttacttgggctgtccgtaagagtaacgagaaaatttacccgtggaatttcgagaatgttgtcgatatcgaagcttctgcagagaaattcatccgtagaatgacaaataaatgtacctaccttatgggtgaagacgtgctgccaaaggattctctgctctatagcaaatacatggttctaaacgaactgaataatgttaaactcgacggagagaaactgtcagtagaattgaagcaacgattgtatactgatgtgttctgcaaatatagaaaggtaactgttaagaagattaagaattaccttaagtgcgagggaataattagtggaaacgttgagatcacgggtattgatggagatttcaaggcgtctcttactgcctatcacgacttcaaggagatcttaacagggacagagttagcgaagaaagataaggagaacatcattactaacattgttctatttggtgatgacaagaaactcttgaagaaacgacttaaccggctatacccacaaattacacctaatcagttaaagaagatttgtgctttaagctacactgggtggggacgattcagcaagaagtttcttgaggaaataaccgctccagatccggaaacaggtgaagtctggaatataattacggcactgtgggaaagtaacaacaacttaatgcaactcttatccaatgaatatcgatttatggaagaggttgaaacatataatatgggtaagcaaacaaagacgctttcgtatgaaaccgttgagaacatgtacgtttctccctccgtcaagagacagatttggcagacacttaagatagtcaaggaattagagaaggtgatgaaggagagtccaaagcgggtgttcatagagatggcaagagagaaacaagaatcaaagagaacagagagtaggaagaagcaacttatcgatttgtataaggcttgtaagaacgaagagaaagattgggttaaggaactaggtgatcaggaggaacagaaactgagatctgacaaattatacttgtattacacacagaagggaaggtgcatgtacagtggtgaagttatcgaacttaaggatctctgggacaacacaaagtatgatattgatcatatttacccacaatccaagacgatggatgactcattaaacaaccgagtattagttaagaagaagtataatgctactaagtcagacaagtatccacttaatgagaacattaggcacgaacgtaaagggttctggaaatccttgcttgacggcggatttatctctaaggagaagtacgaacgactcattagaaatacagaactttctcccgaggagctcgcgggtttcatcgagagacaaatagttgagacgcgtcagtcaactaaggccgtggctgagattcttaaacaggtgttccctgagtccgagatcgtttatgttaaagctggtaccgtttctagatttagaaaggatttcgaactcttgaaagtacgtgaggtcaatgatctccaccatgctaaggatgcatacctcaatattgtggtcggaaactcgtactatgttaaatttacgaagaatgctagctggtttatcaaggagaacccaggaaggacttataacttgaagaagatgtttacatccggttggaacattgaacggaatggtgaggttgcctgggaggtcggtaagaagggaacaatagtgactgtcaaacagatcatgaataagaataacatccttgtgacacgtcaagttcatgaggcaaagggagggttgttcgaccaacagattatgaagaagggtaagggacaaatcgcaatcaaagagacagatgaaagacttgcgagcatagagaagtacggaggctataacaaagccgccggtgcatatttcatgctcgttgagtctaaggacaagaaaggaaagacgatcaggaccattgaatttatcccgctttacttaaagaataagattgagagtgatgagagtattgctttgaatttcttagagaagggacgtggacttaaggagcctaagatccttctgaaaaagattaagatagatactctgtttgatgttgacggatttaagatgtggttgtcaggtaggacgggagatcgtcttctcttcaaatgcgctaaccagttaatcttagatgagaagataatcgttaccatgaagaaaattgttaagttcatacagaggcgtcaagagaatagagagttgaagttgtctgacaaggatggaatagataacgaggtgcttatggagatatacaatactttcgtcgataaacttgagaataccgtttatagaattagactttccgagcaggcaaagactttaatcgataaacagaaagaatttgagcggttaagccttgaggataagagtagtacactattcgaaatcctccatatcttccagtgtcagtcttccgctgctaatttgaagatgataggcggaccaggtaaggctggaattctcgttatgaataacaatatcagcaaatgcaataagattagtattattaaccagagccctaccgggatcttcgagaatgagattgatttgctgaagatctga

SEQ ID NO: 349 - DNA, 3831 bp, Artificial Sequence
  Description of Artificial Sequence: Synthetic polynucleotide
atgtctttcgactctttcaccaatctatactccctctcaaagactctaaagttcgaaatgcgcccggttggaaacacacagaagatgcttgacaatgctggagtgtttgagaaggataagctcatacaaaagaagtatggtaagactaaaccctacttcgatagattacatcgtgagttcattgaagaggctcttacaggtgttgaactaataggactcgacgagaactttagaactttggtggattggcagaaagacaagaagaacaacgtggctatgaaagcttatgagaattctctgcagagacttagaaccgaaattggcaagatatttaatctgaaggccgaagattgggttaagaataaatatccgattctaggattgaagaataagaataccgacattctattcgaagaggcggtcttcggaatactcaaggctaggtatggtgaagagaaggatacattcatagaagtagaggaaattgacaagacaggaaagtccaagataaatcagatttctatctttgattcttggaaaggattcactggttattttaagaaattctttgagactaggaagaacttctataagaatgatggaaccagtactgctattgctactaggatcatagaccagaatcttaaacgtttcatcgataatttatcaattgtggaatctgtccgacagaaggtggacttagcagaaacagagaagtcatttagtatctctttgtcacagttcttctccatagacttctataataagtgtctgttacaagatggcattgactactacaataagatcataggtggagaaaccttgaagaacggagagaagctaatcgggttgaatgaacttataaatcaatatagacagaataacaaggatcagaagataccattcttcaagttgctggataaacaaatcttaagcgagaaaatactctttctagatgagataaagaatgatactgaactaattgaagctctctcacagttcgccaagaccgctgaagagaagaccaagattgtgaagaaactgttcgcagatttcgtggagaacaactctaaatacgacctagctcagatctacatatcccaagaagcattcaacacaatttctaataagtggacctccgagaccgagacattcgccaaatacttgttcgaagctatgaagagtggtaagcttgctaagtatgagaagaaggacaattcatacaagtttccggacttcattgcattaagtcagatgaagagtgctttgctctcaatcagtcttgaaggacatttctggaaggagaagtattataagatctcgaagtttcaggagaagactaattgggaacaattcctggctatcttcctttatgaatttaacagtctgttctctgacaagataaatactaaggatggtgaaactaagcaggttggttattacttattcgcgaaggatctccacaacttaatattgagtgagcagattgatattccgaaagactctaaggtgaccattaaagatttcgctgatagtgtgttgacaatataccaaatggcgaagtatttcgcagttgaaaagaagagggcttggcttgcagaatacgaactggatagcttctacactcaacccgacactgggtatctacaattctatgataacgcgtatgaggatattgttcaggtttacaataaacttaggaactacctaactaagaagccctactctgaagagaaatggaaactaaatttcgagaactctactctggccaacggatgggacaagaacaaggaaagtgataactctgctgtcatactccagaagggcggaaagtactatttagggctaattactaaaggccacaataagatatttgatgaccgattccaagagaagttcatcgtcgggattgaaggaggaaagtatgagaagatcgtttataagttcttcccggatcaggctaagatgtttccaaaggtctgcttcagtgcgaagggattggaattctttcgacctagtgaggagattctcaggatatacaacaatgccgagtttaagaaaggagagacctacagtattgacagcatgcagaaactgatagatttctacaaagattgtctcacgaaatacgaaggatgggcttgttacacattcagacacctcaagcccacggaagagtaccagaataatatcggagagttcttcagagacgtggccgaagatggatatagaatcgacttccaaggaatctccgatcagtatatacatgaaaagaacgagaagggagagctgcatttattcgagatacataacaaggattggaatttagataaggctagagatggaaagagtaagacaactcagaagaaccttcacacattgtacttcgaatccttattcagtaacgataatgttgttcagaatttccctattaagttgaatggccaagcagagatattttatagaccaaagacagagaaagacaagttggagtctaagaaggacaagaagggaaataaagttattgatcacaagagatattctgagaataagatcttctttcatgtgcctctgacactgaaccgaacaaagaacgacagttatcgcttcaacgcccagataaataactttctcgctaataacaaagatataaacatcataggtgttgacagaggcgagaaacatttggtttactacagtgtcatcacccaagcaagcgatatattggagtcaggctcattgaacgagctgaacggtgttaattatgctgagaagctgggcaagaaagctgagaatagagagcaggcaaggagagattggcaagacgtccaaggtataaaggaccttaagaaaggttacatctctcaagtagtccgaaagttggctgatttagccatcaaacataacgcaattatcatcctggaagatttaaatatgcgtttcaagcaagttcgaggaggcatcgagaaatccatctatcaacaattggagaaggcacttattgataagcttagcttcctcgtggacaaaggtgagaaaaaccctgaacaggcaggtcatctcctcaaagcgtatcaattatctgcgccctttgaaacgttccagaaaatgggtaaacagactggtataatcttctatacccaggcctcttacacttccaagagcgatccagtgactggttggcgccctcatctatatcttaagtatttcagcgccaagaaggctaaggatgatatcgcgaaatttactaagatagaatttgtcaacgatagatttgagctgacctatgatattaaggatttccagcaggccaaagaataccctaataagactgtctggaaggtttgctcaaatgtcgagaggtttcgctgggacaagaatttgaaccagaataagggtggatacactcattatactaatatcacggagaatatccaggaactgtttactaaatatggtatagacattaccaaagacttattaacccagattagcactatcgatgagaagcagaatacctctttctttagagacttcatcttctacttcaatttgatctgccaaatacgtaatactgacgattccgagatagccaagaagaacggcaaggatgatttcatcttaagcccagtagaaccgttctttgattcccgcaaagacaacgggaacaagttgccagagaatggagatgacaacggtgcgtataacattgctcgtaagggtatagttatcctcaacaagatatcacaatattctgagaagaacgagaattgtgagaagatgaagtggggcgatctttacgtgagcaacatcgactgggataatttcgtc

SEQ ID NO: 350 - DNA, 3465 bp, Artificial Sequence
  Description of Artificial Sequence: Synthetic polynucleotide
atggagaacttcaagaacttatatcctataaataagaccctcagatttgagcttagaccctatggaaagaccttggagaacttcaagaagtctggactcttagagaaagatgcgttcaaagccaattctaggagatccatgcaggctataattgatgagaaattcaaggaaacaatcgaagagcggttgaagtatacagaattcagtgagtgtgatctaggcaatatgactagcaaagacaagaaaattacagataaagcagcgaccaatttgaagaaacaggtgattctttctttcgatgatgagatctttaataactatttgaagcctgacaagaacatcgatgctttattcaagaatgatccttctaaccctgtcatttctacattcaaaggattcaccacatactttgtaaacttctttgaaattagaaagcacatattcaagggtgaaagttctgggagtatggcataccgaattattgatgagaatctgactacgtacttaaacaatatcgagaagattaagaaacttcctgaagagttaaagagtcaactcgaagggattgatcagattgataaacttaataactacaacgaatttatcacacagagcggaataacacactacaatgagatcatcggaggtatttctaagagtgagaatgtgaagatccagggaataaatgagggtatcaatctttactgtcagaagaataaggtcaaattgccaaggttaacgcccttgtataagatgatcctctcagatcgggtgagtaattcatttgtgcttgatacgattgagaacgacaccgagctaatagagatgatttcagatttaattaacaagactgagattagccaagatgttattatgagtgacatccagaatatattcatcaagtacaaacaacttggaaaccttccaggaatatcttattcgtcaattgtaaacgccatctgctctgattatgacaacaattttggagatggtaagaggaagaagtcatatgagaatgacaggaagaaacatcttgagactaatgtttattctataaactacatttcagaactccttactgatacagatgtctcctcaaacatcaagatgcgatacaaagagttggaacagaactatcaagtttgcaaggagaactttaatgctactaactggatgaatattaagaatattaagcaatccgaaaagacaaacttgatcaaggatctattggacatcctcaaatcaattcagcgattctacgacctctttgatatcgtcgacgaggataagaatccatccgcagaattctacacgtggctctcgaagaacgcagagaaattggacttcgaatttaactcagtttacaacaaatcaagaaactacctcactagaaagcaatactcagacaaaaagattaagttgaacttcgattcgcctactctagctaaaggatgggatgctaacaaggagattgataattccactatcataatgaggaagtttaataacgatcggggagactatgattacttcttagggatttggaacaaatctacaccagcaaatgaaaagatcatcccattagaagacaacggtctctttgaaaagatgcaatataaactttacccagatccgagtaagatgttacctaagcagttcctctcaaagatctggaaagcaaagcatccaacaactccagaatttgataagaaatacaaagaaggcaggcataagaaaggtccagatttcgagaaggaatttctacatgagcttatcgattgcttcaaacacggccttgttaaccacgacgagaagtatcaggacgtatttgggtttaacttgagaaacacagaggactacaatagttacacagagtttctagaagatgtagagaggtgtaattataatttatccttcaataagatagccgatacttctaatcttataaatgatggtaaattatatgtgttccagatctggtcgaaagacttctcaatcgactctaaagggaccaagaatcttaacacgatatacttcgagtcgctcttctcagaggagaatatgatcgagaagatgttcaagctctctggtgaagcagaaatcttctatagaccagcaagtttgaattattgcgaagatataattaagaagggacatcaccatgcagagttgaaagataagtttgactatccgatcattaaagacaagcggtatagtcaagataaattcttcttccatgtgccgatggttataaactacaagtcagagaagctgaactcgaaatcattgaataatcgtacaaatgagaatctcgggcaattcacccatatcatcggtattgatcgcggtgaaagacacctgatttatctcactgtggtcgatgtctcaaccggcgaaattgtagaacagaagcatctcgacgaaattattaatactgatacgaagggtgttgagcataagacccattatcttaataagctggaagagaagtctaagacacgagataacgagcgcaagtcttgggaggccatagagactattaaagaattgaaagaaggctacatatcgcatgtgatcaatgagattcagaagctccaagagaaatataacgctctcatcgttatggagaaccttaattacgggtttaagaactctagaatcaaggttgagaagcaggtttatcagaaatttgaaaccgctttaataaagaagttcaactacataatagataagaaggatccagaaacctacatacacgggtatcaactcacaaaccctataaccacgctagataagatcggaaatcagtctggcatcgtgttatacatcccggcatggaatactagcaagattgatccagtaacagggttcgtcaacttgctttatgctgatgatcttaagtacaagaatcaagaacaagcgaaatcatttattcaaaagattgataacatatatttcgagaacggagagttcaaattcgatattgacttcagtaagtggaataacagatactcgatctcaaagacaaagtggactctgacatcttacggcactcgaattcagacattcagaaaccctcaaaagaataataagtgggacagtgctgagtacgatctcaccgaagagttcaaacttatccttaatattgatggtacattaaagtcacaggatgtagagacttataagaaatttatgtcactatttaagttgatgctacaattgaggaactctgttacaggaaccgacatcgattacatgatttcgccagttacggataagacaggcacacacttcgatagtcgggagaacattaagaacctccctgctgatgctgatgctaacggagcttataatatcgcgcggaaaggaattatggcaatcgagaacatcatgaatgggatatctgatcctcttaagattagtaacgaagattaccttaaatacatccagaaccagcaagagtag

SEQ ID NO: 351 - DNA, 3924 bp, Artificial Sequence
  Description of Artificial Sequence: Synthetic polynucleotide
atgacacaatttgaagggtttacaaacctctaccaagtttcaaagactcttagatttgaattgattccacaagggaagaccttgaaacacattcaggaacaagggttcatcgaagaggacaaggctaggaacgatcattacaaagaactcaaaccgatcattgataggatatacaagacttatgctgatcagtgcttacaacttgtgcaactcgattgggagaacctatcagctgctatcgattcctaccggaaagagaagactgaagagacaagaaatgcactgatcgaagaacaagcgacataccgaaatgctatccacgattatttcatcggtcgaacagataatcttactgacgctatcaataagagacatgcagaaatatataaaggattatttaaagcggagttgttcaatggtaaagtattgaagcagctaggaacagttaccacaactgagcatgagaatgcactcctgagatctttcgataaatttactacctacttctcaggattctacgagaacaggaagaacgtgttctctgctgaggatatatcaacggcaattccacatcggatcgttcaagacaacttcccgaaatttaaagagaactgtcatatctttacaagacttatcaccgcagtacccagcctgagggagcacttcgagaacgtgaagaaagcgataggtatcttcgtaagtacctcgatcgaagaagtattctcgtttccgttctataatcaactactgacacagactcaaatcgacctatacaatcagttgcttggaggcatcagtagggaggccgggacagagaaaatcaaaggattaaatgaggtactgaacctcgcgattcagaagaatgatgaaactgcacatatcattgcttctctaccacatagattcatacctctattcaaacaaattctttcagataggaacacattgtcctttatattggaagaattcaaatcggatgaagaggttatccagtcattctgtaaatataagaccctgctaagaaatgagaacgtgctcgaaactgcagaagctctattcaacgaattaaactccattgaccttacccacatctttatttcccataagaagttggaaacaatctcttctgctctttgtgatcactgggacacccttagaaacgcactgtacgaaaggagaatttcggaacttaccggcaagattactaaatctgccaaagagaaggtgcaaagatcattgaaacatgaggatatcaacctccaagagattatatctgctgctgggaaggagctttcagaagctttcaaacagaaaacttcggaaatcctatctcatgctcatgcggcccttgatcagcctcttccaacgacactgaagaaacaagaggagaaagagatcttgaaatctcagctagattcactcctaggcttgtaccacttacttgattggtttgccgttgatgagtcaaacgaagtagacccagaattctcagcaagactgacaggtattaagcttgaaatggaaccttccttgagtttctacaacaaggctcgaaattacgctaccaagaagccctactctgtagagaagtttaagctgaacttccagatgccaacacttgcttctggttgggacgtcaacaaagagaaaaataatggagcaatattattcgttaagaacggtttgtactacttaggaatcatgcctaaacagaaagggagatacaaggcgctctcattcgaaccgacggagaagacttcagaaggctttgacaagatgtactatgattactttcccgatgctgcaaagatgattcccaagtgcagtactcagctcaaggctgtgaccgcgcactttcagacacacaccacacctattcttctatcaaacaacttcattgagccattagagataacgaaggaaatctatgatctcaataatccggagaaagagcctaagaagttccaaactgcttacgccaagaagactggtgaccagaagggctacagagaggccctgtgtaagtggatcgacttcacccgggacttcttgtccaaatacactaagacgacttcaattgatctttcttcgctgagaccatcatcacagtataaggatttaggtgaatattatgctgagcttaacccactactgtatcatatttcattccaacggatcgctgagaaagaaataatggatgcagttgaaacagggaagttgtatttgtttcagatttacaacaaagacttcgccaagggacatcatggtaaacctaacttacacacgttgtattggacaggtctattctctccggagaacttggcaaagactagcatcaagttaaatggtcaggccgagcttttctatcgtccgaagtctcgcatgaagagaatggctcataggcttggtgagaaaatgctcaataagaagttgaaagaccagaagacacctatacctgatactctttatcaagagttatacgattatgttaatcacagattatcccacgacctctctgatgaagctcgtgctcttcttccaaatgtaataactaaggaagtatcacacgaaatcattaaagatcgtaggttcacatcggataaatttttctttcacgtgcctattacccttaattatcaggccgctaactcaccatctaaattcaatcagcgggttaatgcctacctgaaggaacatccagagacacctatcataggaatcgaccgtggggaacgtaatttaatttatattacagtgattgatagcacagggaagatcttggaacagagatcactgaacacaattcaacaatttgattatcagaagaagttagataatagggagaaagagagagttgctgcaaggcaggcatggtcagtggttgggacaattaaagaccttaagcagggatacttaagtcaggttatccatgaaatagttgatttaatgattcattaccaagccgttgtcgttctggagaatcttaacttcggcttcaagagcaaacgcactgggatcgcagagaaggctgtttaccaacaattcgaaaagatgctgatcgacaaactaaactgtctcgtgttgaaggactaccctgcggagaaagtgggaggagtgcttaatccatatcaattgacagatcaatttacgtccttcgccaagatgggaacacaatcaggattcctcttctatgttccagcaccatatactagtaagatcgatccacttacaggcttcgtagaccctttcgtatggaagacgataaagaaccacgaaagtaggaagcacttccttgagggtttcgacttcctacattatgatgttaagactggtgacttcattctccactttaagatgaataggaatttatcctttcaacgcggtttgccaggatttatgcctgcttgggacatagtattcgagaaaaatgagacccaattcgacgccaagggtacacctttcattgctggcaagcgaatcgtacctgttatcgagaatcacagatttactggtagatacagggacctatacccagctaatgagctcatagcgttactagaggagaaaggcatcgtatttagagatggaagtaatatcctccctaagctactggagaacgatgattctcacgcgattgatacaatggttgcgttgattcgatcagtccttcagatgcggaattcaaacgcagccaccggagaagactatatcaattcaccggttcgagatctcaatggtgtctgctttgactcacgattccagaacccggaatggccaatggatgctgatgcgaacggcgcctaccatatcgcactcaaaggccagctactgctcaaccacctcaaagagagtaaggaccttaaactacagaatggaatttcaaatcaggattggttagcctacatccaagagctccgcaattga

SEQ ID NO: 352 - DNA, 3390 bp, Artificial Sequence
  Description of Artificial Sequence: Synthetic polynucleotide
atggccgttaaatctattaaggtcaagcttcgtctcgacgatatgccagaaattcgggctggtctctggaaattgcataaggaagtgaacgcaggtgtgcggtattacacagagtggcttagtcttcttaggcaggagaacttataccgaagatcaccaaatggtgatggtgagcaagaatgtgataagactgctgaggaatgcaaagctgagttgctagagaggcttcgtgctaggcaggttgagaatggtcatcgagggcctgcgggtagcgacgacgaactactccagcttgcacgtcagctctatgagttgcttgttccacaggctatcggtgcgaaaggagatgcacagcaaatcgcaaggaagttcctcagtccacttgcggataaggatgcggtcggcggattaggtattgctaaagcaggtaacaagcctagatgggtcagaatgagagaagcaggagaacccggttgggaggaagagaaagagaaggccgaaactcgcaagagtgctgatcggacggctgatgtgctcagagctcttgcagatttcggattgaagccacttatgagagtatatactgatagcgagatgagttctgtcgagtggaagccactgaggaagggccaggctgtcaggacttgggaccgtgatatgttccagcaagctatcgaaaggatgatgtcatgggagagctggaaccagagagtcggtcaggagtatgctaagctcgttgaacagaagaataggtttgagcaaaagaactttgtgggtcaagaacacttagtgcacctagtaaatcaactgcaacaagatatgaaagaagctagcccgggtcttgaatctaaggagcagacagcccattatgttactggacgagcccttagaggaagcgataaggtctttgagaaatgggggaagcttgcaccggacgctcccttcgatttatacgatgctgagattaagaacgtacaacgacgaaacactcgtcgattcggatcccatgacctgtttgcaaagctagccgaacctgaataccaggctctttggcgagaagatgcctcgttcctaacgcgatacgcggtatataatagcatattgcgtaaacttaaccacgcaaagatgttcgccacatttaccctcccggacgcgactgctcatccaatctggacacgattcgacaagttgggaggtaatttacaccagtatacgttcttattcaatgagttcggagaacgacgtcatgcaatcaggttccacaagctgttgaaagtagagaacggagttgctagagaagtggatgacgttactgttccaatctcgatgagtgaacaattagataaccttctacctcgtgatcctaatgaacccatagcattatacttcagggattatggtgcggaacaacacttcacaggagagttcggcggagctaagatccagtgtaggcgtgatcaattggcacatatgcacagaagacgtggggcccgggatgtatacctcaatgtgtctgtacgagtccaatctcaatctgaggcccgtggtgagcgtcgtccaccttatgcagcggtctttcgattggtcggagataaccatcgtgctttcgttcacttcgacaaattgtcagattatcttgccgagcaccctgatgatggtaaactaggttctgaaggtcttcttagtggactccgagttatgtccgtggatctagggcttcgtacttctgcgtctatttctgtattcagagttgcacggaaggatgagcttaaacccaattctaaaggaagagttcctttcttcttcccaatcaaaggaaacgacaacctcgtcgctgtccacgaaaggtcgcaactgcttaagttgcctggtgagaccgagagtaaggatttgcgggcaatccgggaagaaaggcaacgtacattgagacaattaaggacgcaactcgcctatcttagactgcttgtcagatgcgggtcggaggatgtgggaagaagagagcgttcgtgggctaagctcattgaacaaccggtggatgctgctaatcatatgactcctgattggagggaagcattcgagaacgagctacagaagctaaagtcacttcatggaatctgttcagacaaagagtggatggacgcagtgtatgaatctgtcagaagagtttggcggcatatgggaaagcaggtacgagattggaggaaagatgttagaagtggagaaaggccaaagatccgtggctacgctaaggacgtcgttggtgggaactctatagaacaaatcgagtacctcgagcgccagtataagtttcttaaatcttggtccttcttcggaaaggtttcgggtcaggtcataagggctgagaaaggctcaaggttcgctatcacattgcgggagcatatagatcatgctaaagaagatagacttaagaagctagctgatagaattatcatggaggctcttggttacgtgtacgcattagatgagagaggcaagggcaagtgggtcgcaaagtatcctccttgtcagttgattctgttagaagaacttagcgaataccagttcaataacgacagaccacctagcgagaacaaccagttgatgcaatggtcccatagaggagtgtttcaggaacttataaaccaagcacaagttcatgatcttcttgttggtactatgtatgctgctttctcgtctcgattcgacgctcgcaccggtgctccaggtatccgatgtagaagagttcctgctagatgtacccaggaacacaacccagaacccttcccttggtggctcaataagttcgtcgttgaacatactctggatgcttgtcctttgagagcagatgatctgataccgaccggagaaggagaaatcttcgtgtcaccattctcagctgaagagggagacttccaccagattcacgctgatcttaatgctgctcagaacctccagcaacgcttatggtcggacttcgatatctcacaaatccgactccgttgtgactggggagaagtcgacggtgaactcgtcttgattccgcgactaacagggaagagaacggccgatagttatagtaacaaagttttctatacgaacacaggcgtgacgtactatgagagagagcgcggtaagaagagaaggaaggtatttgctcaagagaaattatcggaagaggaggctgagttgttggtcgaagcagatgaagcaagagagaaatcggtagtactgatgagagatccaagtggaataatcaaccgcggcaactggacaagacagaaggaattctggtctatggtgaaccagcgtattgagggctaccttgtgaagcagattaggtccagagttccgctgcaagatagcgcttgtgagaatactggagatatttga

SEQ ID NO: 353 - DNA, 3327 bp, Artificial Sequence
  Description of Artificial Sequence: Synthetic polynucleotide
atggccacgagatcatttattcttaagattgagcctaatgaagaggtgaagaaaggtttatggaagacgcatgaggtcctcaatcatggaatcgcttattatatgaatatcctcaaactcataagacaagaggcgatatatgaacaccatgagcaagatcctaagaatcccaagaaggttagtaaggcagaaattcaagctgagttatgggatttcgtgctaaagatgcagaagtgtaactctttcactcatgaggtggataaggatgtcgtatttaacatccttagagaactctatgaggagttagttccctcttctgttgaaaagaagggcgaggcaaatcaattgtcaaataagttcctttacccgttggttgacccaaattcccaatctggtaagggtacggcttcctcagggcgaaagccacgttggtataatcttaagatcgctggtgatccatcctgggaggaggagaagaagaagtgggaggaggataagaagaaagatccattggcgaagatcttgggaaagctagcagagtacggtttgatccctctgttcatcccatttacggactccaacgagccgatagttaaggaaatcaagtggatggagaagtcacgaaaccagtcagtccgccggctcgacaaggatatgtttattcaagctcttgagcgtttcttatcttgggaaagctggaacctcaaagttaaggaggagtacgagaaagtggagaaagaacataagacgcttgaagagaggatcaaagaagatattcaagcatttaagtcactagaacaatacgagaaagaaaggcaagagcaattgttgcgtgataccttaaacacgaatgaatacagactatctaaacgtgggcttcggggttggcgagaaataatccagaaatggcttaagatggatgagaacgagccgagcgagaagtacctagaggtgtttaaagattaccaaaggaaacatccaagagaagctggcgactattccgtctacgagtttctcagcaagaaagagaatcacttcatctggcgtaatcaccctgaatacccatatctttatgctacattctgcgagattgataagaagaaaaaagatgcaaagcagcaggctacatttactctagcagatccgattaatcatccactctgggtgcgatttgaagagaggtccggaagtaatttgaacaagtaccgaatattgacagagcaacttcatactgagaaattaaagaagaagttgactgttcagttagacagactgatttaccctacagagagtggtggttgggaagagaaaggcaaggttgatattgttcttcttccatctcgtcagttctacaatcaaatattcttggatatcgaagagaagggaaagcatgcctttacctacaaagatgaatcgattaaatttccgctaaagggaacattaggtggagctagggtacaatttgatcgagatcatctgcgtaggtacccacataaggtcgagagcgggaatgtcggcagaatttactttaacatgactgtaaatatagaaccaactgaatctcctgtctcgaagtcgttgaagatccaccgagatgattttccgaagttcgtgaacttcaaaccaaaggagcttacagagtggattaaggatagtaaaggtaagaaattgaagtctggaattgagtctctggagatagggttacgagttatgtctatagatcttggtcagcgtcaggcagcagcggcgtcgatctttgaagttgtagatcagaaaccagacatcgaaggtaagttgtttttcccaatcaagggaactgagctttacgcggttcatcgagcatctttcaacataaagttgcccggagaaaccctcgttaagagtagagaagtgctgcgcaaagctagagaagataaccttaaactgatgaatcagaagttgaatttcttgaggaacgtactccactttcaacaattcgaagacatcactgaacgagagaagagagtaacgaaatggatctcccgccaggagaactcggatgttccgttagtatatcaagatgaactcattcagataagggagctaatgtataagccttataaggactgggtcgctttccttaagcagcttcataagagactcgaagtagaaatcggtaaggaagttaaacactggaggaagagtttatccgacggccgtaagggactttatggcattagcctaaagaatattgatgagatcgatcgtacgaggaaattcttgctcagatggtcattgaggccaaccgagcctggagaggtgagacgcttagaacctggacagagatttgctattgatcagcttaaccacctcaacgcgcttaaggaggatagactcaagaagatggcaaatacgataatcatgcatgcccttggttactgctacgatgtgagaaagaagaagtggcaggcgaagaatccggcttgtcagattatccttttcgaagatctttcaaactacaatccctatgaggaacgttctcggttcgagaactcgaagctcatgaagtggtcaagacgggaaatccctagacaggttgctcttcaaggcgagatttatgggcttcaagttggcgaagtgggagcacaattctcgtcccgtttccacgcaaagacaggcagtccaggcataaggtgtagcgttgtcacgaaggagaaattgcaagacaacaggttcttcaagaaccttcaacgcgaagggagattaaccctcgataagatcgccgtactaaaggaaggtgatttgtacccagataagggtggcgagaaattcatctctttatccaaggacagaaagctagtgacaacccacgctgatattaacgctgctcagaatctacagaaacgtttctggaccaggactcacggtttctataaagtttactgtaaagcttatcaagttgacggacagacggtttatatcccggaaagtaaggaccagaagcagaagattattgaagaatttggagaaggttacttcatattgaaagatggcgtttacgaatggggaaacgctggtaagctgaagattaagaaaggttcttcgaagcagtcatcatctgagttagttgatagcgatatactgaaggattcattcgaccttgcatcggagcttaagggagagaaattgatgttgtacagagatccttccggtaacgtgttcccaagcgataaatggatggctgcgggtgtattcttcgggaagcttgaacgcatcctaatttctaaattgactaatcaatactctatttcgacaatagaagatgatagctcaaagcaatctatgtaa

SEQ ID NO: 354 - DNA, 3450 bp, Artificial Sequence
  Description of Artificial Sequence: Synthetic polynucleotide
atgccaacaagaacgattaaccttaaactagtccttggtaagaatccggagaacgctaccttaagacgtgctttgttctctacacatagactcgtgaaccaggctaccaagaggattgaagaattccttctactttgccgaggagaggcataccgtaccgtcgataatgagggtaaggaggctgaaatccctcgtcatgcagtacaggaggaggcgcttgcgtttgctaaggccgctcaacggcataacggatgtataagtacatatgaggatcaagaaatcctagatgttctgcggcaactttatgaaagacttgttccttcagtcaacgagaataacgaagctggcgatgcgcaagcagctaacgcttgggtctcaccattaatgtccgcagagagcgaaggtggtctttctgtctatgataaagtacttgatccaccaccggtctggatgaagttgaaagaggagaaagcaccaggttgggaggccgccagccaaatttggatacaatccgacgagggtcagtcacttctcaataagccgggttctccaccgaggtggataagaaagctgagatcagggcaaccgtggcaggatgacttcgtatccgaccagaaaaagaagcaagatgaacttaccaaaggaaatgctcctcttataaagcagctcaaggagatgggactccttccactcgtgaacccattctttagacaccttctcgatccggaaggtaagggtgttagtccctgggatagactcgctgtgagagctgccgttgcccacttcatttcatgggaaagctggaaccatagaactagagctgaatataactcccttaagctccgtagagatgaattcgaagctgccagtgatgagtttaaggacgacttcaccttgctccgtcaatatgaagcaaagaggcattccacattgaagagcattgcacttgcagacgattctaatccttaccgtattggtgtccggtccctcagagcatggaacagagtgcgtgaagaatggatcgataagggtgccacagaggagcagagagtcacaatcttgtcgaaactccaaacacaactccgtggcaagtttggagatcctgacctcttcaattggctcgcacaagaccggcatgttcacctgtggtcacctcgggactccgtcacacctttggtgagaataaatgcagttgataaagtccttaggcgtagaaagccttacgcattgatgacattcgctcaccctagatttcaccctaggtggatattgtacgaggctcctggtgggagcaatctgaggcaatacgcactcgattgtactgagaatgctttgcacatcacattaccactgttagttgatgacgcccacggaacttggattgagaaaaagatcagagtcccgttggctcctagtggacaaattcaggatttgactcttgagaaactggagaaaaaaaagaaccgcttatactacagatccgggtttcaacaattcgctgggttagctggaggagcggaggtcttattccaccgtccctacatggagcatgatgagagaagtgaggagagtctacttgaacgtccaggcgcagtctggttcaaacttacacttgatgttgctactcaagctcctcccaattggttagatggcaagggcagggtaagaacacctcctgaagtgcatcactttaagaccgcactctcaaacaagagtaagcatacaagaacactccagccaggactcagagtactgtctgtggatcttggaatgcgaactttcgcctcatgttctgtgttcgaactcattgaaggtaagccggaaacaggaagggcgtttccagtggctgatgagcgctcaatggattcgcctaataaattgtgggctaagcatgaaaggtcattcaagctcaccctgcccggcgagacgcctagtcgtaaggaagaggaggagagatcaattgcaagagcggaaatatacgcgcttaaacgcgatattcagcgacttaagagtctgttacgactcggagaggaggacaacgacaacagaagagatgccctattggaacagttctttaaaggatggggagaggaagacgttgtcccaggacaagcatttccaagatctttgtttcaaggactgggagcagctccattcaggtcaacgcctgaattatggcgacagcactgccagacgtattatgataaggctgaggcatgccttgcgaagcatatctctgattggcgcaaacgtacacggccaagacccacctcgcgggagatgtggtataagacacgatcctatcacggaggcaagtcaatttggatgctggagtatctagatgctgtcagaaagctacttctaagctggagccttcgggggcgtacttacggcgctataaacagacaagatacggcccgcttcggcagcttggcaagcagactactccatcacattaactccctcaaggaggaccgaattaagaccggtgccgacagtatcgttcaagcagctcgcggctatataccgctgccgcatggaaagggatgggaacagcgttacgagccctgccaactaattttgtttgaagatcttgcgaggtacaggttcagagtggatcgcccgcgccgtgagaacagtcagcttatgcaatggaatcacagagctattgtggctgagacgacaatgcaggctgaactctacggacagatagttgagaacactgcagccggattctcctctagatttcatgctgctacaggtgcacccggtgttaggtgccgatttctcctggaacgtgactttgacaacgatcttcctaagccttacctgctcagagaattgagttggatgctcgggaatacgaaggttgagtcagaagaagagaagttaaggttgctctcagagaaaattcgtccgggatctttagttccatgggatggtggtgagcagtttgctactctacaccctaagaggcagacgttgtgcgttatccatgctgatatgaacgcagctcagaacctgcaacggaggttcttcggtcggtgtggtgaagcgttcagactggtgtgtcagccacatggcgacgatgtgttgaggttggcaagcacgccgggagcaagactactgggagcattgcagcaacttgagaatggacaaggagcatttgagctagtccgagatatgggatccacatcgcaaatgaacagattcgtcatgaagtccttggggaagaaaaagatcaaacctcttcaagacaacaatggcgatgacgagctcgaagatgtcttgagcgttcttcccgaggaggatgataccggtcgaatcactgtgtttagagattctagtggtatcttcttcccttgtaacgtgtggattcccgccaagcaattctggcctgccgtaagagctatgatatggaaagtgatggcttcacattcgttaggttag

SEQ ID NO: 355 - DNA, 3759 bp, Artificial Sequence
  Description of Artificial Sequence: Synthetic polynucleotide
atgacaaagctccggcatcgtcagaaaaagcttacacacgactgggctggatcaaaaaagagagaagtgttaggctctaatggaaagttgcagaacccactccttatgccggttaagaagggtcaagttacagagttcagaaaggcattctcagcgtatgctagagcaacgaagggtgaaatgaccgatggtagaaagaacatgtttacgcacagcttcgaaccattcaagacgaagccatctctccaccagtgtgaactggctgataaggcctaccagtctttacactcttaccttccgggtagtttggctcacttccttctaagtgctcacgctctcggcttcagaatatttagtaaatctggtgaagcaactgcattccaggcttcctcaaagatagaggcgtatgagtctaaacttgcatcagaactcgcttgcgtggatctttcaattcagaacctaactatttcgacattatttaatgcacttaccacaagtgtgagaggcaagggagaggaaacatccgctgatccactaatagctcgcttctatactctcctaacagggaagccactctctcgagatacacagggacctgaaagagatcttgccgaggttatatctcgaaagatcgcgtctagtttcggtacatggaaagaaatgactgctaatcctctacaatccttacagttcttcgaagaggaattgcacgcgttagatgctaacgtttcgctttctccggctttcgatgtgctcatcaagatgaatgatcttcagggtgatctcaagaatcgaaccatcgtattcgatccggatgctcctgtatttgagtacaacgcggaagatccggccgatattatcatcaaattaacagcaagatacgccaaggaagcagttattaagaatcagaacgtgggtaattatgtcaagaacgctatcactactacgaacgccaacggtctcggatggcttcttaataagggtctgtcgttattgcctgtatccactgatgatgagctgcttgagtttatcggtgttgaaagatcgcacccatcatgccacgctctgattgaactgatagcacaactagaagctccggaattattcgagaagaatgtgttcagtgacaccagatccgaagtccagggaatgatagacagcgctgtgtctaatcacatcgcgagattgtccagctctagaaattcccttagtatggactctgaggaactcgagcgtctcatcaagtcattccagatccatactccacactgtagtttatttataggtgctcaaagcctcagccaacagttagaatcgctgccagaagcgctgcaatctggagtaaattccgctgatatcctactaggctcaacgcaatatatgcttacaaactcgttagttgaagaatctattgcgacttatcaacgcaccttgaaccgaattaattacctatctggcgtggcaggtcaaataaatggtgccatcaagaggaaagccatagatggtgagaagatacatcttcccgctgcatggtccgagctaatctcactaccgtttataggacaaccagtgatagatgtggagtctgatcttgctcatttgaagaaccagtaccaaacattgagtaatgaatttgatactcttatcagcgctttacagaaaaatttcgatctgaacttcaataaagcgctgcttaatcggactcagcactttgaagcaatgtgtagaagtacgaagaagaacgcgctaagcaagcctgaaattgtttcatacagggatcttcttgctcgtctaacttcttgcctttaccgcggatctcttgtcctcaggagggcgggaattgaggtgcttaagaaacataagatattcgaaagtaatagcgagcttagagagcatgtccacgagagaaagcatttcgtgtttgtttcgccacttgacaggaaagctaagaaactgttgaggcttaccgattcgcgaccagacctcctccatgttattgatgagatcttgcaacacgataatctggagaacaaagatagagaatccctttggttagtgagatccgggtaccttctcgcaggacttcctgaccagctgagctcgagcttcatcaaccttccgatcattacacagaagggtgatagacgacttattgacttgatccagtacgaccaaattaatagggatgcctttgtgatgcttgttacatccgcattcaagtccaacttatcaggtctccaataccgtgctaataagcaatccttcgtcgttaccaggactctcagtccttacctaggttctaaactagtgtacgttcctaaagacaaagattggttggtaccaagtcaaatgttcgaaggtagatttgcagatatacttcagagtgactacatggtttggaaagatgccggcaggttatgcgtgattgacactgctaagcacctgtcaaatatcaagaagtctgtattctcttctgaagaggtccttgcctttcttagggaattaccgcatcgcacatttatccagaccgaggttcgtggacttggtgttaacgttgacggaatagctttcaataatggtgatatcccttctttaaagacgttctccaattgcgtgcaagtcaaagtttctcgaacaaacacaagcttggttcagaccctgaatagatggtttgagggaggtaaggtctctccacccagcatacaattcgaacgtgcttactacaagaaagacgatcagatccatgaggatgccgcaaagcgaaagataagattccaaatgcctgccacagagctagttcatgcttctgacgatgctggttggacaccttcttacctgttaggtattgatcctggagagtatggtatgggtttgagtttagtgtcaattaacaacggtgaagtgttggactcaggattcatccatataaattcactaataaacttcgcttctaagaagagtaaccaccaaaccaaggtcgtcccaaggcaacagtataaatcaccgtatgctaattatctggaacaatctaaagattctgctgctggtgacatagcacatatacttgacagacttatctacaaattgaatgcattgccggtcttcgaagcgttgagcggaaactctcaatccgcggcagaccaagtttggacaaaggtacttagcttctatacctggggcgataatgatgcacagaactctattaggaagcagcactggtttggtgcatcccactgggacatcaagggcatgttgaggcaacctcctactgagaagaagcctaagccatatatagccttccctggatcccaagtttcaagttacgggaatagtcaaaggtgcagctgctgtggacggaatccgatcgagcagctcagagagatggctaaggatacaagcattaaggagttgaagatcagaaactcggagatacaactctttgatgggacgattaagctgttcaacccagatcctagtacagtcattgagagacgtcgacacaaccttggaccttccaggattccagttgcggatcgcacattcaagaatatttcgccttcaagcttggagttcaaagaactcatcaccattgtttctagatctataagacactcgcctgaattcatagctaagaagcgtggaatcggcagcgagtacttctgtgcatacagtgattgcaattcttcattaaactctgaagctaacgccgctgccaatgtcgctcagaaatttcagaaacaactgttcttcgagctttag

SEQ ID NO: 356 - DNA, 3864 bp, Artificial Sequence
  Description of Artificial Sequence: Synthetic polynucleotide
atgaaacgtatcctcaactctctgaaggtcgctgctctcagactgttgttcagaggcaagggttcagagcttgtaaagacggttaaatatcctcttgtttcaccagtgcaaggagctgtggaggagctagcagaagctataagacacgataatcttcacttattcggacagaaggaaattgtagacctgatggagaaagatgaaggtactcaggtttattcagttgttgacttctggctcgacactcttcgtctgggcatgttcttcagcccctctgccaatgctctgaagattaccctgggtaaatttaattctgatcaggtaagtcccttccgcaaggtgcttgaacaaagccctttctttctcgcaggaaggttgaaagtggagcctgctgagagaatcttaagtgtggagatccgtaagatcggtaagagggagaacagggtggagaattacgctgcagatgttgagacttgctttataggtcagctgtcatctgatgagaagcagtcaattcagaagcttgctaacgatatatgggatagcaaggatcatgaagagcaacgtatgttaaaggctgatttctttgctattccacttattaaggatcctaaagcagtgacagaagaggatccggagaatgaaacagccggtaagcagaaacctctggagttgtgtgtgtgtctcgttcctgagctttacacccgtggatttggatcaatagctgactttctagtccagaggctaacattattgcgggataagatgagcaccgatacagctgaggattgcttggagtatgttggtattgaggaagagaagggaaacggaatgaattcattgttgggcaccttcttgaagaacctccagggtgatggattcgaacagatatttcagttcatgttaggttcttatgtcggctggcagggtaaggaggatgtcttaagagaaagactcgatttgcttgctgagaaagtgaagagattgccgaagccgaagttcgcgggcgaatggtctggtcatcggatgttcctgcacggtcagctgaagagctggtcttctaatttcttccgcttgtttaatgaaactcgagaattactagaatctatcaaatcagatattcaacacgcaacaatgttaatctcgtacgttgaggagaagggtggctatcatcctcagctattatcccaatacaggaagttaatggaacaattgcctgcactcaggactaaggtacttgacccagaaattgagatgactcacatgagcgaggctgtaagatcatacattatgattcacaagagtgtcgccggattcttgccagatctcttagagtcccttgatagagataaggaccgagaattcttgctttcaatatttcctagaatacctaagatagataagaagaccaaggaaatcgttgcttgggaattgccgggtgagccagaggaaggttatctctttacagctaataacttgtttcgtaatttcctcgagaatccgaaacacgtcccacgtttcatggctgaaagaatccctgaagattggacaaggttacgctcggcgcccgtatggttcgatggaatggttaaacagtggcagaaagtggtcaaccaactcgttgagtcgccaggtgctctctaccagtttaatgaatcgttcttaagacaacgactgcaggctatgctgaccgtttacaagcgcgaccttcaaactgagaagtttcttaagcttcttgcagacgtatgcagacctcttgtcgatttctttggtcttggtggaaacgacataatctttaagagttgtcaagacccacgtaaacagtggcagacagtcataccattaagtgttccggctgatgtttacacagcctgtgaaggactggccatcagactaagggagacgcttggcttcgaatggaagaaccttaagggccacgaaagagaggatttcttacggctacaccagttgcttggaaacctgttgttctggatcagggatgctaagctggttgttaagttggaggattggatgaacaacccttgcgttcaagagtatgtcgaagctcgtaaagcgattgaccttccgctcgagatattcggtttcgaagtcccaatcttccttaatgggtacttattctctgagttgagacagttggagttgctgttaaggcgtaagtcggtgatgacgagttactccgtcaagaccactggttcaccgaaccgattgttccaattagtatacttgccgctcaacccttctgatccggagaaaaagaattcaaacaacttccaagaaagactggatactccaaccgggttatctagacggttcttggaccttactcttgacgcatttgcaggaaagctgttaacagatcctgtaacacaagaacttaagacaatggccggcttctatgatcatctattcggtttcaaattgccatgtaaactggcggcaatgagtaatcatccagggagttccagcaagatggttgtcctagctaaacccaagaagggcgtcgcctcgaatattggattcgaacctatacctgatcctgcgcatcccgtgtttcgggttcgctcttcatggccagagttgaagtacttagaaggccttctttatctccctgaagatactccattaacgatagagcttgctgaaacctccgtttcatgtcaaagcgtgtcttctgttgcattcgatttaaagaacctcactacaatactcggccgtgtaggtgagttcagagttaccgccgaccagccattcaagcttactccaattattcctgagaaggaggaatcatttatcgggaagacatatctgggattggatgctggagaaaggtcaggtgttgggttcgcgattgtcacagttgacggtgatggttatgaggtacagcgcctcggtgtccatgaagatactcagctcatggcccttcaacaagttgcttctaagtccctgaaagaacctgtgttccaacctttgcgtaagggtacgtttagacaacaagagaggatccgcaagagtctcagaggttgttactggaatttctatcatgctttaatgatcaaatacagagcaaaggttgttcatgaggagtcagttggatcaagcggtttggtcggccaatggttacgggcatttcagaaggatttgaagaaggctgacgtcttgcccaagaagggcggcaagaatggtgtagacaagaagaagagggagtctagtgcccaggacactctttgggggggtgcgttctcaaagaaggaggaacagcaaattgcctttgaggtgcaggctgctggtagttcccaattctgcctgaaatgcggttggtggttccaactaggaatgagagaagtgaatagagttcaagaatctggtgtcgtcttggattggaacagatcgatagttaccttcctaatcgagagctctggcgagaaggtttatggtttctcacctcagcaattggagaagggattccgaccagacatcgaaacgttcaagaagatggttagggactttatgcggccgcctatgttcgaccgaaagggtcgtcctgctgctgcatatgagcgatttgtccttgggcggaggcatcgaagatatcggttcgacaaagtgttcgaggagcggttcggtagatcagccctctttatttgtccacgtgtcggttgcggtaatttcgatcattcctctgaacaaagtgccgtagtcttggcactaattgggtatatagccgataaagagggtatgtccgggaagaagcttgtgtacgttcgactcgctgagttgatggctgagtggaaactcaagaaattggaacgcagcagggttgaagagcagtcttccgcacaatag

SEQ ID NO: 357 - DNA, 3579 bp, Artificial Sequence
  Description of Artificial Sequence: Synthetic polynucleotide
atggccgaatcaaagcaaatgcagtgcagaaagtgtggagcttctatgaaatatgaggtgatcgggttaggtaagaagagttgtaggtacatgtgcccagattgcggcaaccatacaagtgcacgtaagatccagaataagaagaagcgagataagaaatacggctctgcgagtaaagctcagagtcagagaatcgctgtagccggtgctctatatccagataagaaggtgcaaactattaagacctacaagtatcctgcagatttaaatggtgaggtacatgatagcggagtggcagaaaagattgctcaagctatacaagaggatgaaattggcttactcgggcctagttccgaatacgcttgctggatcgctagtcagaaacagagcgaaccctactccgtggtagatttctggtttgatgctgtttgtgctggtggtgtatttgcttattcgggagctcgtttgttatcgactgttcttcaattatctggagaagagtctgtgttgcgggcagcactcgcttcctcacccttcgttgatgatataaaccttgctcaagcggagaagtttcttgcggtctctaggagaacgggacaagacaagttaggaaagcgtattggcgagtgtttcgcagaagggagactcgaggctttaggcatcaaagatcgtatgcgggagtttgttcaggctattgatgtggctcaaaccgccgggcagcgattcgcagctaaactcaagatctttggtatttcgcagatgcccgaagctaagcagtggaataacgactctgggctcacagtttgcatcctaccagactactacgtcccagaagagaaccgggcggatcagctagttgtgctgttgagaagactccgcgagattgcctattgcatgggtattgaggatgaggcaggctttgaacatctaggtattgatcccggagccctctctaatttctcgaatgggaacccgaagagagggtttctcggccgattgctcaataatgatataatcgcgcttgctaacaacatgtctgcaatgacgccatattgggaaggccgcaagggagaattgatcgaaagactggcttggttgaagcatcgtgctgagggactctaccttaaggaaccacatttcggtaactcatgggccgatcaccggtctcgaattttctctaggatagccggttggcttagtggttgcgctgggaaactcaagatcgcgaaggatcaaataagcggagtgaggactgatttgtttctattgaaacgccttctcgatgcggttcctcagagtgctccatctccagatttcatcgctagtatctcggcacttgatagattcctcgaggccgcagagtcatcccaagatccggccgaacaagtcagggcactttacgctttccatctcaacgctccggcagtaagaagtatagcaaacaaggctgttcaacgatccgactcccaggagtggttaatcaaagaattggatgctgtggatcatctagaattcaataaagcattcccattcttctcagatacgggcaagaagaagaagaaaggagcgaactctaacggcgcgccttctgaggaggaatacacagagactgaatctatccagcagccggaggatgctgaacaagaggtaaacggtcaagagggtaatggagcatctaagaaccagaagaagtttcagagaattccaaggttcttcggagagggctctcgttccgagtacagaatcttgaccgaggctccacaatacttcgatatgttctgcaacaacatgagggcgatctttatgcaactcgaatcccaaccacgtaaagctcctagggactttaaatgctttctacagaataggcttcagaagctttacaagcagacattcttgaacgctaggagcaacaagtgtcgtgctttacttgaaagtgttctcatctcctggggtgagttctacacatacggtgcaaacgaaaagaaattcaggcttcgtcacgaagcaagtgaacgttcttcagaccctgattatgtcgtacagcaggcactggagattgctagaagacttttcttgtttggcttcgaatggcgggattgtagcgccggtgagagagttgatctcgtagagattcataagaaggctatctccttcctacttgccataacgcaggccgaggtgtctgtcgggagttataattggttgggaaattcaacagtatcgcgctatcttagtgttgcgggaactgatactctgtatgggacacaactagaagagttcctcaacgctactgtcctatctcagatgagaggtctggctattcgtttgagctctcaagagcttaaggatggcttcgacgtacaacttgaatcatcgtgtcaagataacttgcaacatttgttggtgtatagagcgtcccgcgatctcgcagcttgtaagcgtgctacttgtcctgctgagttagatccgaagattctcgtgctgcccgtcggcgcattcatcgctagtgttatgaagatgattgaaagaggtgatgaaccattggcaggcgcatacttgcgtcatcgtccgcattcatttgggtggcaaatccgtgttcgtggggtagcggaagtgggtatggatcagggtacagcactcgccttccagaaacctaccgaatcggaaccattcaagattaaaccattctcagctcaatatggtccagttctttggctgaactcaagttcgtactcgcagtcccagtacttggatggattcttgtcccagcctaagaattggtctatgagagttctgcctcaagcaggtagtgtccgagtcgaacagagggtggcccttatatggaatctccaagcaggaaagatgagacttgaacgttctggcgctcgtgcattctttatgcctgtccctttctctttccgtccatctggatcaggtgacgaagccgtactggctcctaatagatatctaggactctttccacactcaggagggatagagtatgccgttgtagatgtgttggattcagctgggttcaagatattggaacgtgggacaattgctgttaatggattctcgcagaaaagaggagaacgtcaagaggaggcccatcgtgagaaacaacgccgcggcatttcagatatcggtaggaagaagcctgtccaagctgaagttgacgcagcgaatgagctgcaccgaaagtacacagatgtagcaacgagactaggttgccgaattgttgtccaatgggcaccacaaccgaagcctggtacggcgccaactgcacaaacggtgtacgctcgagctgtaaggacagaagcgcctcgtagcggcaatcaggaggatcatgctcggatgaagagttcgtggggctacacctggggtacttactgggagaagcgtaagccggaagatatcttgggtatttccactcaggtgtattggactggcggcattggtgaatcatgtccggcggtcgctgtcgcattactcggacatattagagctacttcaactcaaacagaatgggagaaggaggaagtggtgtttggaaggctgaagaagttctttccgtcctga

SEQ ID NO: 358 - DNA, 2958 bp, Artificial Sequence
  Description of Artificial Sequence: Synthetic polynucleotide
atggagaaaagaatcaacaagattcgcaagaagctaagtgctgataatgctactaaacccgtgtcacgcagtgggccaatgaagactctattggttagagtgatgacggacgatctcaagaagaggcttgagaagagacggaagaagcccgaggtcatgccgcaagttatttctaacaatgcagccaacaatcttagaatgctgcttgacgattataccaagatgaaggaggcgatattacaagtttattggcaagagtttaaggacgaccacgttggtttgatgtgcaagtttgctcagccggcctcaaaaaagattgatcagaataaacttaaacctgaaatggatgagaagggaaaccttaccacagcaggcttcgcttgttctcaatgtggacaacctctatttgtgtacaagctcgagcaagtcagcgagaagggtaaagcctacacaaactactttggaagatgcaacgttgctgagcatgagaagctaatacttctcgcacagttgaaacctgagaaagattctgatgaagccgttacatattcattaggtaagtttggccaaagggctctagatttctacagtattcatgtaaccaaagaatcgacgcaccctgttaagccacttgcacaaatagctggaaatagatatgctagtgggccagtagggaaagctttatcagacgcttgcatgggtactatcgcttctttcctatctaagtatcaggatattataatcgagcatcagaaggttgtcaaaggtaatcagaaacgtctggagagcctcagagagttagcaggaaaggagaaccttgaatatcctagtgtaacccttcctcctcagcctcataccaaggagggagtagatgcttacaatgaggtgatcgctagagttaggatgtgggttaatttaaatctgtggcagaaattgaagctatccagggacgacgctaaaccattgctgcgtcttaaaggattcccttctttcccagtcgttgagagacgtgagaatgaagtcgattggtggaatactatcaacgaagtaaagaagcttattgatgcaaagcgagatatgggaagggtcttttggagtggtgttactgcagagaagcgtaatacaatattagaaggatacaattacctgccaaacgagaatgatcacaagaagagggagggatcacttgagaatcccaagaagcctgcaaagagacagtttggtgacttattgttgtatctagagaagaaatatgctggagattggggtaaggtcttcgacgaagcatgggaaagaattgataagaagatcgccggcctgacaagtcatatcgagagagaagaagctcgtaacgcggaagatgctcagagtaaagccgtgttgactgattggttaagggctaaagcgtctttcgtcttggaacgacttaaagagatggatgagaaggagttctacgcttgcgagattcaactccagaaatggtatggagatttgcgaggtaatccgttcgcggtagaggcggagaaccgggttgtagacatctcagggttctcgattggttcggatgggcactccatacaatataggaacctcctggcttggaaatatcttgagaatggtaaacgtgaattctacctgctaatgaactatggtaagaagggccgcattcgattcacagatgggacagatataaagaaaagtggaaagtggcagggacttctgtatggaggtggtaaggctaaagtcattgatctaaccttcgatccagacgacgagcagcttattatcttaccgttggcgtttggtacaagacaaggcagagaattcatctggaacgacctgctttcgttggaaacaggacttatcaaactcgcgaacgggagagtcattgagaagacaatttacaacaagaaaattggtagggatgagccggctctcttcgttgctctcacattcgagaggcgggaggttgttgatccttctaatatcaaaccagtcaacttgattggagtcgaccgaggcgagaacatccctgctgttatcgctttgacagatccagaaggatgcccgttacctgagttcaaagactctagtggaggtccaacggacatcttacgtattggagagggatataaggagaaacaacgggccatacaagctgctaaggaggtggaacaaaggagagcgggagggtacagtagaaagtttgcaagtaaatctagaaatttggctgacgacatggtgagaaactcagctagggacttgttctaccacgctgttactcacgatgccgtattggtattcgagaacttgtcacgaggcttcggaagacaaggtaagcgtactttcatgacagagagacagtatactaagatggaagattggttaactgccaaattggcctacgaagggctcaccagtaagacttatttatctaagactttggctcagtacaccagcaagacatgttcgaattgcgggttcactataaccacggcagactatgatggtatgttggttagattaaagaagactagcgatggctgggctactacattgaacaataaggagttgaaggctgaagggcaaatcacctattataatcgttataagagacagactgtcgagaaggagttgtctgctgagttggatcgtctctctgaggagtctgggaacaacgacatttcaaagtggactaagggacgtcgagatgaggctctgtttttgctcaagaagaggttctctcatcgtcccgtccaagaacaatttgtctgtctggattgtggccatgaggtccatgctgatgaacaagctgctcttaacattgcacgaagttggctcttcttgaatagtaattctaccgaattcaaatcctataagagtggaaagcaacctttcgtcggagcttggcaggcattctataagaggaggctgaaggaagtttggaagcccaacgct

SEQ ID NO: 359 - DNA, 2919 bp, Artificial Sequence
  Description of Artificial Sequence: Synthetic polynucleotide
atgaagagaatcaataagatccggcgcagactggttaaggattctaacacgaagaaggcaggaaagacgggtccaatgaagacgcttctcgtgcgggtgatgactcctgacctccgtgaaagactggagaacttgcgtaagaagccggagaatattcctcaacccatctcaaacacgagtagagctaacttaaacaagttattgacagactacacagaaatgaagaaggcaatcctgcacgtttattgggaagaattccagaaggaccctgtaggattgatgtcaagagtcgcacaaccagcacccaagaatattgaccaaaggaagttaattccagtcaaggacggaaacgaaaggctcactagctcgggatttgcatgttctcagtgttgtcaacctttgtatgtgtacaagttggagcaggttaacgacaaagggaaacctcacactaattacttcgggaggtgtaacgtgtcagagcacgagcgactcatccttctcagccctcacaaaccagaggcaaatgatgagcttgtgacttattcacttggcaagttcggtcagcgggcgcttgacttctatagtattcacgtgacaagagaatctaatcatccagtcaaacctttggagcaaataggaggaaattcttgtgcatctggtccagtcggcaaggctctctccgacgcatgcatgggagcagtagcttccttcttaaccaaatatcaggatataatcctagagcaccagaaggtcattaagaagaatgagaaaaggctcgctaatttaaaggatatagcatcggctaatggacttgctttccctaagattactttgcctcctcagcctcatacgaaagagggtatcgaagcctataataacgttgttgcgcaaatagtgatttgggtgaatttaaatttatggcagaagttgaagattggacgtgacgaagctaagccgctacagcgccttaaaggattccctagctttcctctcgttgaaagacaagccaacgaggttgactggtgggatatggtgtgtaatgttaagaagttaatcaacgagaaaaaggaagatggaaaggtgttctggcagaaccttgctgggtataaacgtcaagaagctttacttccatacttgtcatcagaggaagacagaaagaagggaaagaaatttgctagatatcaattcggcgatctgctcttacatctggagaagaagcatggtgaagactgggggaaagtctatgatgaagcctgggagcgaattgataagaaagtcgaaggattgtcgaagcatattaagctggaggaagagagacgtagtgaagatgctcaatctaaggcggctttgaccgattggttacgagctaaagctagtttcgttatcgaaggactcaaggaggctgacaaggatgagttctgtagatgtgaattgaaactccagaaatggtacggagaccttagaggaaagccattcgccattgaagctgagaacagtatattggatataagcggattctcgaagcagtacaactgtgcattcatctggcagaaagatggtgttaagaagctgaatttatatctcattattaactatttcaagggagggaagctgaggtttaagaagattaagccagaagcctttgaagccaatcggttctacacggtgattaataaaaagagcggagaaatcgtgccgatggaggttaacttcaatttcgatgatcctaacttaatcatcctcccacttgctttcggtaagagacaaggacgtgaatttatctggaacgacctactgtccctggagacgggatcactgaagttagcgaacggacgtgttatcgaaaagaccctttataatagacgaacccgccaggatgaacctgctttattcgtcgccctgacgttcgagcgtcgcgaggttcttgattcttctaatatcaagcctatgaacctcattggtatagatcgcggagagaacatccctgctgtgattgccttgaccgatcccgaaggatgccctctaagtaggtttaaggatagtcttggtaatccaactcatatacttaggattggagaatcatacaaggagaagcagagaacaatacaggctgcgaaagaggttgagcagcgtagagctggtggatacagtcgtaaatacgcgagtaaggcaaagaatctggctgatgatatggtaagaaatactgcgagagatttgttatattacgcagttacacaagatgctatgcttatattcgagaatctttcacgaggatttgggaggcaagggaagaggacattcatggctgaacgtcagtacactcgtatggaggattggcttactgctaaacttgcttacgaaggattacctagcaagacatacctaagcaagacattggctcaatatacgtctaagacttgctcgaactgcggattcacgatcacctctgcagactacgatcgcgtgcttgagaagctgaaaaagaccgccacaggttggatgacaaccataaacggaaaggaacttaaggtggaaggacagatcacatattataacagatataagaggcagaatgtcgttaaggatctctctgtcgagctcgatagacttagtgaagagtcagtaaataatgatatttcatcatggactaagggacgctcaggcgaggctctttcacttcttaaaaagagattctcccaccgtcctgtccaggagaagtttgtttgtttgaattgcggtttcgaaacccatgctgatgagcaagctgcactcaatatagcgaggtcttggctatttctcagaagccaggagtacaagaaatatcaaaccaacaagactactggaaatactgacaagagggcattcgttgaaacatggcaatcgttctatcgcaagaagcttaaggaggtgtggaaacct

SEQ ID NO: 360 - DNA, 25 bp, Artificial Sequence
  Description of Artificial Sequence: Synthetic oligonucleotide
tttcttaggtccagcagatacacgt

SEQ ID NO: 361 - DNA, 25 bp, Artificial Sequence
  Description of Artificial Sequence: Synthetic oligonucleotide
tttgcaagctccctacaggccattc

SEQ ID NO: 362 - DNA, 25 bp, Artificial Sequence
  Description of Artificial Sequence: Synthetic oligonucleotide
tttaggggattggatagcgtgaccc

SEQ ID NO: 363 - DNA, 25 bp, Artificial Sequence
  Description of Artificial Sequence: Synthetic oligonucleotide
tttatgttatcgtgcttcccatgcc

SEQ ID NO: 364 - DNA, 124 bp, Artificial Sequence
  Description of Artificial Sequence: Synthetic polynucleotide
ccgaagcattggccgtaaccttaacaagaaattgggaagagacgtgtatctgttagatctgcgtaaccatggatcctcaccacacagttcagtccataactacgaagtcatgtcggaagacgtg

SEQ ID NO: 365 - DNA, 124 bp, Artificial Sequence
  Description of Artificial Sequence: Synthetic polynucleotide
ttcgaaaaaccaagttttacaacgacgtccattagaatcgactaacagtaatcatgggttcgcgtctagcctgcaggccattccggaaaacacgatgagtggcagtgataatgcttcttttcaa

SEQ ID NO: 366 - DNA, 124 bp, Artificial Sequence
  Description of Artificial Sequence: Synthetic polynucleotide
attttgctaacgataaatggtgacatcaagttggcagactggggtcacgctattcagagcccgaagtctaacgacttccagattggtaccgataattacagggcgccagaaactttctctggcc

SEQ ID NO: 367 - DNA, 124 bp, Artificial Sequence
  Description of Artificial Sequence: Synthetic polynucleotide
agaacgccttttagagacgtttatttcaaatacacttcgcttatgggttcccacatgttctacgtgattgttcttcccatgcctgtgtggcttggataccgcgatttaacacgggacatgatct

SEQ ID NO: 368 - DNA, 124 bp, Artificial Sequence
  Description of Artificial Sequence: Synthetic polynucleotide
ccgaagcattggccgtaaccttaacaagaaattgggaagagacgtgtatctgctggacctaagaaatcatggatcctcaccacacagttcagtccataactacgaagtcatgtcggaagacgtg

SEQ ID NO: 369 - DNA, 124 bp, Artificial Sequence
  Description of Artificial Sequence: Synthetic polynucleotide
ttcgaaaaaccaagttttacaacgacgtccattagaatcgactaacagtaatcatgggtttgcaagctccctacaggccattccggaaaacacgatgagtggcagtgataatgcttcttttcaa

SEQ ID NO: 370 - DNA, 124 bp, Artificial Sequence
  Description of Artificial Sequence: Synthetic polynucleotide
attttgctaacgataaatggtgacatcaagttggcagactggggtcacgctatccaatcccctaaatctaacgacttccagattggtaccgataattacagggcgccagaaactttctctggcc

SEQ ID NO: 371 - DNA, 124 bp, Artificial Sequence
  Description of Artificial Sequence: Synthetic polynucleotide
agaacgccttttagagacgtttatttcaaatacacttcgcttatgggttcccacatgttttatgttatcgtgcttcccatgcctgtgtggcttggataccgcgatttaacacgggacatgatct

SEQ ID NO: 372 - DNA, 197 bp, Artificial Sequence
  Description of Artificial Sequence: Synthetic polynucleotide
ggccccaaattctaatttctactgttgtagatttaggtccagcagatacacgtccgaagcattggccgtaaccttaacaagaaattgggaagagacgtgtatctgttagatctgcgtaaccatggatcctcaccacacagttcagtccataactacgaagtcatgtcggaagacgtgctcgcacggctaacgtgaga

SEQ ID NO: 373 - DNA, 197 bp, Artificial Sequence
  Description of Artificial Sequence: Synthetic polynucleotide
ggccccaaattctaatttctactgttgtagatcaagctccctacaggccattcttcgaaaaaccaagttttacaacgacgtccattagaatcgactaacagtaatcatgggttcgcgtctagcctgcaggccattccggaaaacacgatgagtggcagtgataatgcttcttttcaactcgcacggctaacgtgaga

SEQ ID NO: 374 - DNA, 197 bp, Artificial Sequence
  Description of Artificial Sequence: Synthetic polynucleotide
ggccccaaattctaatttctactgttgtagatggggattggatagcgtgacccattttgctaacgataaatggtgacatcaagttggcagactggggtcacgctattcagagcccgaagtctaacgacttccagattggtaccgataattacagggcgccagaaactttctctggccctcgcacggctaacgtgaga

SEQ ID NO: 375 - DNA, 197 bp, Artificial Sequence
  Description of Artificial Sequence: Synthetic polynucleotide
ggccccaaattctaatttctactgttgtagattgttatcgtgcttcccatgccagaacgccttttagagacgtttatttcaaatacacttcgcttatgggttcccacatgttctacgtgattgttcttcccatgcctgtgtggcttggataccgcgatttaacacgggacatgatctctcgcacggctaacgtgaga

SEQ ID NO: 376 - protein, 6 aa, Artificial Sequence
  Description of Artificial Sequence: Synthetic peptide
HHHHHH

SEQ ID NO: 377 - DNA, 27 bp, Artificial Sequence
  Description of Artificial Sequence: Synthetic oligonucleotide
  modified_base (4)..(25): a, c, t or g
yttnnnnnnnnnnnnnnnnnnnnnngg

SEQ ID NO: 378 - DNA, 27 bp, Artificial Sequence
  Description of Artificial Sequence: Synthetic oligonucleotide
  modified_base (5)..(24): a, c, t or g
tttannnnnnnnnnnnnnnnnnnnagg

SEQ ID NO: 379 - DNA, 27 bp, Artificial Sequence
  Description of Artificial Sequence: Synthetic oligonucleotide
  modified_base (5)..(24): a, c, t or g
tttcnnnnnnnnnnnnnnnnnnnncgg

SEQ ID NO: 380 - DNA, 27 bp, Artificial Sequence
  Description of Artificial Sequence: Synthetic oligonucleotide
  modified_base (5)..(24): a, c, t or g
tttgnnnnnnnnnnnnnnnnnnnnggg

SEQ ID NO: 381 - DNA, 27 bp, Artificial Sequence
  Description of Artificial Sequence: Synthetic oligonucleotide
  modified_base (5)..(24): a, c, t or g
ttttnnnnnnnnnnnnnnnnnnnntgg

SEQ ID NO: 382 - DNA, 27 bp, Artificial Sequence
  Description of Artificial Sequence: Synthetic oligonucleotide
  modified_base (5)..(24): a, c, t or g
cttannnnnnnnnnnnnnnnnnnnagg

SEQ ID NO: 383 - DNA, 27 bp, Artificial Sequence
  Description of Artificial Sequence: Synthetic oligonucleotide
  modified_base (5)..(24): a, c, t or g
cttcnnnnnnnnnnnnnnnnnnnncgg

SEQ ID NO: 384 - DNA, 27 bp, Artificial Sequence
  Description of Artificial Sequence: Synthetic oligonucleotide
  modified_base (5)..(24): a, c, t or g
cttgnnnnnnnnnnnnnnnnnnnnggg

SEQ ID NO: 385 - DNA, 27 bp, Artificial Sequence
  Description of Artificial Sequence: Synthetic oligonucleotide
  modified_base (5)..(24): a, c, t or g
ctttnnnnnnnnnnnnnnnnnnnntgg

SEQ ID NO: 386 - DNA, 16 bp, Artificial Sequence
  Description of Artificial Sequence: Synthetic oligonucleotide
gtcaaaagaccttttt

SEQ ID NO: 387 - DNA, 19 bp, Artificial Sequence
  Description of Artificial Sequence: Synthetic oligonucleotide
aatttctactcttgtagat

SEQ ID NO: 388 - DNA, 17 bp, Artificial Sequence
  Description of Artificial Sequence: Synthetic oligonucleotide
gtctggccccaaatttt

SEQ ID NO: 389 - DNA, 19 bp, Artificial Sequence
  Description of Artificial Sequence: Synthetic oligonucleotide
aatttctactgttgtagat

SEQ ID NO: 390 - DNA, 16 bp, Artificial Sequence
  Description of Artificial Sequence: Synthetic oligonucleotide
gtcaaaagacctgtgt

SEQ ID NO: 391 - DNA, 17 bp, Artificial Sequence
  Description of Artificial Sequence: Synthetic oligonucleotide
gtctggccccaaattct

SEQ ID NO: 392 - DNA, 19 bp, Artificial Sequence
  Description of Artificial Sequence: Synthetic oligonucleotide
aatttctactagtgtagat

SEQ ID NO: 393 - DNA, 19 bp, Artificial Sequence
  Description of Artificial Sequence: Synthetic oligonucleotide
aatttctacttttgtagat

SEQ ID NO: 394 - DNA, 19 bp, Artificial Sequence
  Description of Artificial Sequence: Synthetic oligonucleotide
aatttctactattgtagat

SEQ ID NO: 395 - protein, 5 aa, Artificial Sequence
  Description of Artificial Sequence: Synthetic peptide
KMFPK

SEQ ID NO: 396 - DNA, 20 bp, Artificial Sequence
  Description of Artificial Sequence: Synthetic oligonucleotide
agcagctttatcatctgccg

SEQ ID NO: 397 - protein, 7 aa, Artificial Sequence
  Description of Artificial Sequence: Synthetic peptide
QQLYHLP

SEQ ID NO: 398 - DNA, 20 bp, Artificial Sequence
  Description of Artificial Sequence: Synthetic oligonucleotide
agcagttataataactgccg

SEQ ID NO: 399 - DNA, 70 bp, Artificial Sequence
  Description of Artificial Sequence: Synthetic oligonucleotide
accgtaaagttcgcgtgatggcagccgattatgaaaatcagctcgacgagttttccctcgatgcgcccat

SEQ ID NO: 400 - DNA, 70 bp, Artificial Sequence
  Description of Artificial Sequence: Synthetic oligonucleotide
accgtaaagttcgcgtgatggcagcctaataagagaatcagctcgacgagttttccctcgatgcgcccat

SEQ ID NO: 401 - DNA, 70 bp, Artificial Sequence
  Description of Artificial Sequence: Synthetic oligonucleotide
accgtaaagttcccgtgatggcagccgattatgaaaatcagctcgacgagttttccctcgatgcgcccat

SEQ ID NO: 402 - DNA, 62 bp, Artificial Sequence
  Description of Artificial Sequence: Synthetic oligonucleotide
accgtaaagttcgcagccgattatgaaaatcagctcgacgagttttccctcgatgcgcccat

SEQ ID NO: 403 - DNA, 38 bp, Artificial Sequence
  Description of Artificial Sequence: Synthetic oligonucleotide
ccgtctaamwacmhtttwkaatttctactrttgtagat

SEQ ID NO: 404 - protein, 11 aa, Artificial Sequence
  Description of Artificial Sequence: Synthetic peptide
  MOD_RES (3)..(3): Lys or Asn
  MOD_RES (4)..(4): Asn or Tyr
  MOD_RES (5)..(5): Asn, Thr, Ile, His, Pro or Leu
  MOD_RES (6)..(6): Leu or Phe
  MOD_RES (7)..(7): Glu or absent
  See specification as filed for detailed description of substitutions and preferred embodiments
PSXXXXXFLLL

SEQ ID NO: 405 - DNA, 36 bp, Artificial Sequence
  Description of Artificial Sequence: Synthetic oligonucleotide
gtttgattatcctttgaatttacatatctctcaaac

SEQ ID NO: 406 - DNA, 29 bp, Artificial Sequence
  Description of Artificial Sequence: Synthetic oligonucleotide
actacattttttaagacctaattttgagt

SEQ ID NO: 407 - DNA, 35 bp, Artificial Sequence; identical to SEQ ID NO: 86
  Description of Artificial Sequence: Synthetic oligonucleotide

SEQ ID NO: 408 - DNA, 36 bp, Artificial Sequence; identical to SEQ ID NO: 87
  Description of Artificial Sequence: Synthetic oligonucleotide

SEQ ID NO: 409 - DNA, 38 bp, Artificial Sequence; identical to SEQ ID NO: 88
  Description of Artificial Sequence: Synthetic oligonucleotide

SEQ ID NO: 410 - DNA, 32 bp, Artificial Sequence; identical to SEQ ID NO: 89
  Description of Artificial Sequence: Synthetic oligonucleotide

SEQ ID NO: 411 - DNA, 35 bp, Artificial Sequence; identical to SEQ ID NO: 90
  Description of Artificial Sequence: Synthetic oligonucleotide

SEQ ID NO: 412 - DNA, 33 bp, Artificial Sequence; identical to SEQ ID NO: 91
  Description of Artificial Sequence: Synthetic oligonucleotide

SEQ ID NO: 413 - DNA, 36 bp, Artificial Sequence; identical to SEQ ID NO: 93
  Description of Artificial Sequence: Synthetic oligonucleotide

SEQ ID NO: 414 - DNA, 36 bp, Artificial Sequence; identical to SEQ ID NO: 94
  Description of Artificial Sequence: Synthetic oligonucleotide

SEQ ID NO: 415 - DNA, 35 bp, Artificial Sequence; identical to SEQ ID NO: 95
  Description of Artificial Sequence: Synthetic oligonucleotide

SEQ ID NO: 416 - DNA, 52 bp, Artificial Sequence
  Description of Artificial Sequence: Synthetic oligonucleotide
  modified_base (19)..(33): a, c, t, g, unknown or other
actatcaatgggctaactnnnnnnnnnnnnnnntgaaacatctgcaactgcg

SEQ ID NO: 417 - DNA, 52 bp, Artificial Sequence
  Description of Artificial Sequence: Synthetic oligonucleotide
actatcaatgggctaactacgttcgtggcgtggtgaaacatctgcaactgcg

SEQ ID NO: 418 - skipped

SEQ ID NO: 419 - DNA, 28 bp, Escherichia coli
gtaacttcaaacgtaccctggttggcag

SEQ ID NO: 420 - DNA, 28 bp, Escherichia coli
aactcttcaatggtgacatcacgcaggg

SEQ ID NO: 421 - DNA, 28 bp, Escherichia coli
tccgcttcactggaagtcgcggtcggaa

SEQ ID NO: 422 - DNA, 28 bp, Escherichia coli
cgaactttacggtcatcgcgtggtgcac

SEQ ID NO: 423 - DNA, 28 bp, Escherichia coli
gcagctttatcatctgccgctggacggc

SEQ ID NO: 424-638 - skipped (215 entries)

SEQ ID NO: 639 - RNA, 35 nt, Artificial Sequence
  Description of Artificial Sequence: Synthetic oligonucleotide
gucaaaagaccuuuuuaauuucuacucuuguagau

SEQ ID NO: 640 - RNA, 36 nt, Artificial Sequence
  Description of Artificial Sequence: Synthetic oligonucleotide
gucaauaagacucauuuaauuucuacuucgguagau

SEQ ID NO: 641 - RNA, 36 nt, Artificial Sequence
  Description of Artificial Sequence: Synthetic oligonucleotide
gucuggccccaaauuuuaauuucuacuguuguagau

SEQ ID NO: 642 - RNA, 36 nt, Artificial Sequence
  Description of Artificial Sequence: Synthetic oligonucleotide
gucuagguacucucuuuaauuucuacuauuguagau

SEQ ID NO: 643 - RNA, 37 nt, Artificial Sequence
  Description of Artificial Sequence: Synthetic oligonucleotide
ggucuagguacucucuuuaauuucuacuauuguagau

SEQ ID NO: 644 - RNA, 36 nt, Artificial Sequence
  Description of Artificial Sequence: Synthetic oligonucleotide
gucuaagaacuuuaaauaauuucuacuguuguagau

SEQ ID NO: 645 - RNA, 36 nt, Artificial Sequence
  Description of Artificial Sequence: Synthetic oligonucleotide
guugaguaaccuuaaauaauuucuacuguuguagau

SEQ ID NO: 646 - RNA, 36 nt, Artificial Sequence
  Description of Artificial Sequence: Synthetic oligonucleotide
gucaaaucguuuuuaaaaauuucuacuauuguagau

SEQ ID NO: 647 - RNA, 36 nt, Artificial Sequence
  Description of Artificial Sequence: Synthetic oligonucleotide
guuaaguuauauagaauaauuucuacuguuguagau

SEQ ID NO: 648 - RNA, 36 nt, Artificial Sequence
  Description of Artificial Sequence: Synthetic oligonucleotide
guuaaguaauauaaaagaauuucuacuauuguagau

SEQ ID NO: 649 - RNA, 36 nt, Artificial Sequence
  Description of Artificial Sequence: Synthetic oligonucleotide
gcuuaagacuuagaaauaauuucuacuauuguagau

SEQ ID NO: 650 - RNA, 36 nt, Artificial Sequence
  Description of Artificial Sequence: Synthetic oligonucleotide
cucuacaacugauaaagaauuucuacuuuuguagau

SEQ ID NO: 651 - RNA, 36 nt, Artificial Sequence
  Description of Artificial Sequence: Synthetic oligonucleotide
guuuaauccauauauaaaauuucuacuuuuguagau

SEQ ID NO: 652 - RNA, 36 nt, Artificial Sequence
  Description of Artificial Sequence: Synthetic oligonucleotide
gucuaauacccauauaaaauuucuacuuuuguagau

SEQ ID NO: 653 - RNA, 36 nt, Artificial Sequence
  Description of Artificial Sequence: Synthetic oligonucleotide
cucuaauaccucuauaagauuucuacuuuuguagau

SEQ ID NO: 654 - RNA, 36 nt, Artificial Sequence
  Description of Artificial Sequence: Synthetic oligonucleotide
cucuaaaacccccaacaaauuucuacuuuuguagau

SEQ ID NO: 655 - RNA, 36 nt, Artificial Sequence
  Description of Artificial Sequence: Synthetic oligonucleotide
gucuaaaacucauucagaauuucuacuaguguagau

SEQ ID NO: 656 - RNA, 36 nt, Artificial Sequence
  Description of Artificial Sequence: Synthetic oligonucleotide
guuuaaaaccacuuuaaaauuucuacuauuguagau

SEQ ID NO: 657 - RNA, 36 nt, Artificial Sequence
  Description of Artificial Sequence: Synthetic oligonucleotide
guucugcauccauauuggauuucuacuuuuguagau

SEQ ID NO: 658 - RNA, 36 nt, Artificial Sequence
  Description of Artificial Sequence: Synthetic oligonucleotide
guuuaaaaguccuauuggauuucuacuuuuguagau

SEQ ID NO: 659 - RNA, 36 nt, Artificial Sequence
  Description of Artificial Sequence: Synthetic oligonucleotide
cucuagcaggccuggcaaauuucuacuguuguagau

SEQ ID NO: 660 - RNA, 36 nt, Artificial Sequence
  Description of Artificial Sequence: Synthetic oligonucleotide
aucgaacagacucauaaaauuucuacuguuguagau

SEQ ID NO: 661 - RNA, 36 nt, Artificial Sequence
  Description of Artificial Sequence: Synthetic oligonucleotide
guuaaguaaccuaaauaauuucuacuguguguagau

SEQ ID NO: 662 - RNA, 36 nt, Artificial Sequence
  Description of Artificial Sequence: Synthetic oligonucleotide
guuaaguaaccuaaauaauuucugcuguguguagau

SEQ ID NO: 663 - RNA, 37 nt, Artificial Sequence
  Description of Artificial Sequence: Synthetic oligonucleotide
aguuugaauaaccuuaaauaauuucuacuuuguagau

SEQ ID NO: 664 - RNA, 37 nt, Artificial Sequence
  Description of Artificial Sequence: Synthetic oligonucleotide
guuaaauaauaagaaaaaauuucuacuaguguagauu

SEQ ID NO: 665 - RNA, 36 nt, Artificial Sequence
  Description of Artificial Sequence: Synthetic oligonucleotide
gucuaagacuuaaagauaauuucuauacuauuagau

SEQ ID NO: 666 - RNA, 35 nt, Artificial Sequence
  Description of Artificial Sequence: Synthetic oligonucleotide
cucaaaacucauucgaaucucuacucuuuguagau

SEQ ID NO: 667 - RNA, 21 nt, Artificial Sequence
  Description of Artificial Sequence: Synthetic oligonucleotide
gaaucucuacucuuuguagau

SEQ ID NO: 668 - RNA, 21 nt, Artificial Sequence
  Description of Artificial Sequence: Synthetic oligonucleotide
caaauuucuacuguuguagau

SEQ ID NO: 669 - RNA, 21 nt, Artificial Sequence
  Description of Artificial Sequence: Synthetic oligonucleotide
agaauuucuacuaguguagau

SEQ ID NO: 670 - RNA, 22 nt, Artificial Sequence
  Description of Artificial Sequence: Synthetic oligonucleotide
aauaauuucuacuguuguagau

SEQ ID NO: 671 - RNA, 21 nt, Artificial Sequence
  Description of Artificial Sequence: Synthetic oligonucleotide
agaauuucuacuuuuguagau

SEQ ID NO: 672 - RNA, 21 nt, Artificial Sequence
  Description of Artificial Sequence: Synthetic oligonucleotide
uuaauuucuacuguuguagau

SEQ ID NO: 673 - RNA, 21 nt, Artificial Sequence
  Description of Artificial Sequence: Synthetic oligonucleotide
uuaauuucuacucuuguagau

SEQ ID NO: 674 - RNA, 21 nt, Artificial Sequence
  Description of Artificial Sequence: Synthetic oligonucleotide
uuaauuucuacuauuguagau

SEQ ID NO: 675 - RNA, 19 nt, Artificial Sequence
  Description of Artificial Sequence: Synthetic oligonucleotide
aauuucuacuauuguagau

SEQ ID NO: 676 - skipped

SEQ ID NO: 677 - RNA, 42 nt, Artificial Sequence
  Description of Artificial Sequence: Synthetic oligonucleotide
  modified_base (22)..(42): a, c, u, g, unknown or other
uuaauuucuacucuuguagaunnnnnnnnnnnnnnnnnnnnn

SEQ ID NO: 678 - RNA, 56 nt, Artificial Sequence
  Description of Artificial Sequence: Synthetic oligonucleotide
  modified_base (36)..(56): a, c, u, g, unknown or other
gucaaaagaccuuuuuaauuucuacucuuguagaunnnnnnnnnnnnnnnnnnnnn

SEQ ID NO: 679 - DNA, 25 bp, Unknown
  Description of Unknown: Target sequence
cttagctacaggagaggtaagtggc

SEQ ID NO: 680 - DNA, 25 bp, Unknown
  Description of Unknown: Target sequence
gggtgatctttggtctcttcggaaa

SEQ ID NO: 681 - DNA, 25 bp, Unknown
  Description of Unknown: Target sequence
gggtccattagctgtttagagcaaa

SEQ ID NO: 682 - DNA, 25 bp, Unknown
  Description of Unknown: Target sequence
gtagtccaaggagggtatagataag

SEQ ID NO: 683 - DNA, 25 bp, Unknown
  Description of Unknown: Target sequence
tttaccgtcaccaaaatcagattca

SEQ ID NO: 684 - DNA, 25 bp, Unknown
  Description of Unknown: Target sequence
tttgacctacgaattggagatgaag

SEQ ID NO: 685 - DNA, 25 bp, Unknown
  Description of Unknown: Target sequence
tcagattcagaaccacttctctaaa

SEQ ID NO: 686 - DNA, 25 bp, Unknown
  Description of Unknown: Target sequence
tttaaagaagctaagttggaaatgg

SEQ ID NO: 687 - DNA, 25 bp, Unknown
  Description of Unknown: Target sequence
ccctttaaagaagctaagttggaaa

SEQ ID NO: 688 - DNA, 25 bp, Unknown
  Description of Unknown: Target sequence
tttgacctacgaattggagatgaag

SEQ ID NO: 689 - DNA, 25 bp, Unknown
  Description of Unknown: Target sequence
ggtgggttgggctggaggtttcaaa

SEQ ID NO: 690 - DNA, 25 bp, Unknown
  Description of Unknown: Target sequence
cctgctgaattactcacgccccaag

SEQ ID NO: 691 - DNA, 25 bp, Unknown
  Description of Unknown: Target sequence
tttaccacctgctgaattactcacg

SEQ ID NO: 692 - DNA, 25 bp, Unknown
  Description of Unknown: Target sequence
gtaaatcctcagcccacaagggaaa

SEQ ID NO: 693 - DNA, 25 bp, Unknown
  Description of Unknown: Target sequence
ggtgctgcctacgctccatagtaaa

SEQ ID NO: 694 - DNA, 25 bp, Unknown
  Description of Unknown: Target sequence
tttcaaatgaaccctgcgctgtcat

SEQ ID NO: 695 - DNA, 25 bp, Unknown
  Description of Unknown: Target sequence
ccatagtaaatcctcagcccacaag

SEQ ID NO: 696 - DNA, 25 bp, Unknown
  Description of Unknown: Target sequence
cttcttcgaattttaccacctgctg

SEQ ID NO: 697 - DNA, 25 bp, Unknown
  Description of Unknown: Target sequence
tttgagaatgttgtagccatgaagg

SEQ ID NO: 698 - DNA, 25 bp, Unknown
  Description of Unknown: Target sequence
gtttgagaatgttgtagccatgaag

SEQ ID NO: 699-720 - skipped (22 entries)

SEQ ID NO: 721 - protein, 5 aa, Artificial Sequence
  Description of Artificial Sequence: Synthetic peptide
KMLPK

SEQ ID NO: 722 - DNA, 3897 bp, Artificial Sequence
  Description of Artificial Sequence: Synthetic polynucleotide
atgacaaagaccttcgattcggaattcttcaatctatattccctacagaaaaccgtacgtttcgaactgaaaccggtgggtgagacggcgtcctttgtggaagactttaagaatgaaggtctcaaacgcgtcgtgtcggaagatgagcgccgcgccgtggattaccagaaagtgaaagagattatagatgactaccatcgagatttcatcgaagaaagtttgaactacttcccggaacaggtgtcgaaggatgcattggagcaggcatttcacctgtatcagaaactcaaagctgccaaagtggaggaacgcgagaaggcactcaaagagtgggaggccctgcaaaagaaacttcgcgagaaggtggtaaagtgcttcagtgactcaaataaggcacgctttagtcgcatagacaagaaagaactgattaaagaagatctgatcaattggctggtggcgcagaatcgtgaggacgacatcccaaccgttgaaacgttcaacaacttcacaacctactttaccggatttcacgagaacagaaagaatatttacagtaaagatgatcatgcaacggctatcagtttccgcctgatccatgagaacctgccgaagttcttcgataacgtgatttcgttcaataaactcaaagaagggtttcctgaactgaaattcgataaagtcaaagaagacttagaagtcgattacgatctcaaacacgcgtttgaaattgagtacttcgtgaacttcgttacccaagctggtattgatcagtacaattacctgcttggtggtaagactctggaagatgggacaaagaaacagggcatgaacgaacagattaacttgtttaaacagcaacaaacacgcgataaagctcgtcaaatacccaaactgattccgctgttcaagcaaatcctaagcgaacggaccgaatcgcagtcgttcattcctaaacagttcgaaagcgaccaagagttattcgactccttacagaaactgcataacaactgtcaagataagttcacagtcctgcaacaagcaatcctgggcctggctgaagccgaccttaagaaagtattcatcaagacctccgatctgaacgcgctcagtaacacaatatttgggaattacagtgtcttttctgatgcactcaacctctacaaggaatctttaaagacaaagaaagcgcaagaggcgtttgagaagttaccagcgcacagcatacatgaccttatccaatatcttgaacagttcaattcttcattggacgctgagaaacagcagtcaaccgatacagtactgaactacttcatcaagaccgatgaactgtattcaagattcattaaatctacatccgaagcgtttacgcaagtccagccgctgttcgaattggaagcgttaagctcgaagcggaggccgccggaaagtgaggatgagggtgctaaaggtcaggaaggctttgaacaaattaaacgcatcaaggcttatctggatacccttatggaagcggtgcactttgcgaaaccgctgtatttggtgaagggtaggaagatgatcgaaggtctggataaagatcaaagtttctatgaagcctttgagatggcttatcaggaactggaatcgctgattatcccgatttacaacaaagccagaagctaccttagtcgtaaaccgtttaaagcggataaattcaagattaacttcgataacaatacgctcttgagtgggtgggatgcaaacaaagagactgcgaacgcaagtattctatttaagaaagacggtctttattatctgggaatcatgcctaaagggaagactttcttgttcgattatttcgtttcatcagaagatagcgagaaactaaagcaacgtcgtcaaaagactgcagaagaagcgctggcccaggatggcgaatcgtacttcgagaagattcgttataaactactgcctggtgcatcgaagatgctgcctaaggtcttcttctcaaataagaatattgggttctacaatccgagtgacgatatattaagaattcgtaataccgcaagccatacgaagaacggcacaccgcagaaaggtcatagcaaagtcgaatttaacctcaacgactgtcataagatgattgatttctttaaatcatctatccagaagcatccagaatggggcagctttggattcacatttagtgataccagcgacttcgaagatatgtccgccttctatcgcgaagttgagaaccagggttatgttatctcattcgacaagatcaaagaaacgtatatacaatcacaggtagagcagggaaatctatatctctttcaaatttataacaaagacttctctccgtattcgaaaggtaaacctaatctgcacactttatattggaaagctttgtttgaagaagccaacctgaacaatgttgttgccaagttaaatggagaggccgaaatcttctttcgccgccactctatcaaagccagtgataaagtcgtgcatccagcgaaccaggcaatcgataataagaatcctcataccgaaaagacgcaaagcacgtttgaatatgatctggtgaaagacaaacgttacacacaagacaagtttttcttccatgtcccgatttctctcaacttcaaagcccagggtgtgtccaaatttaatgataaagttaacggcttcctcaaaggcaaccctgatgtaaacataataggcatagacaggggtgaaagacatttactgtacttcactgtggttaaccagaagggcgaaattctcgtgcaggaatcacttaacactctgatgtcggataaaggccatgttaacgactatcagcagaaactcgacaagaaagagcaggagagagacgcggcgcgcaaatcatggaccacggtcgagaacatcaaagagctcaaagaaggctacctgagtcacgtcgttcataagctggcacacctgattattaaatataacgcgattgtgtgcttagaagatctgaactttggattcaaacgcggcagattcaaagtcgagaagcaggtttaccagaaattcgagaaagccctcatcgacaaactgaactacttagtgtttaaagagaaggaattaggcgaagtaggtcattacctgacggcataccaactgacggcgccgttcgagagcttcaagaaactgggtaagcagagtggcattcttttctacgtgccggcggattatacgagcaagatcgatccgaccacagggttcgtcaacttcctggacctgcgctaccagagtgttgagaaagccaaacagctgcttagtgactttaatgcaatacgcttcaatagtgttcagaattatttcgaattcgaaatcgattataagaaattaacgccgaagcgaaaggtcggcacccagagtaaatgggtaatatgcacttacggcgacgtccgttatcagaaccgccgcaatcagaaaggacattgggagacggaagaagtgaacgtcacggagaaactgaaagcactgtttgcttctgattctaagacgacgaccgtgattgattatgccaacgatgacaacttgattgatgtcatcctcgaacaggataaggcgtcattcttcaaggaactgctttggctgttgaagctcaccatgactttgcgtcatagcaagatcaagtctgaagatgacttcattctgtcacccgtcaagaacgagcaaggcgagttctacgattccaggaaggccggtgaagtttggccgaaagacgcagatgccaatggtgcataccacattgctttgaaaggattatggaatcttcaacagatcaatcaatgggagaagggcaagacgctgaatctggcaataaagaaccaggattggtttagctttattcaagagaaaccttaccaggagtaa

SEQ ID NO: 723 - DNA, 3897 bp, Artificial Sequence
  Description of Artificial Sequence: Synthetic polynucleotide
atgacgaagacgtttgattcggagttctttaatctgtactctttgcaaaagaccgttcgctttgaactcaagccggtcggcgaaactgcatcctttgttgaagactttaagaacgaaggcctgaaacgtgtagtgtcggaggatgaacgacgcgccgtcgactaccagaaggttaaggaaattattgatgattaccaccgtgacttcattgaagaatcgctgaactattttcctgaacaggtaagcaaggatgcgcttgaacaagcgtttcatttataccagaagctgaaggctgcgaaagttgaagaacgtgagaaggccctgaaagaatgggaagctttgcagaagaaactgagggagaaagttgtcaagtgcttcagcgacagcaacaaggcaagattctcgcggatcgacaagaaagagcttatcaaagaagatctgatcaattggttagttgcacagaaccgcgaagatgacattccaactgtcgaaacatttaataatttcacgacatacttcaccggtttccacgagaacagaaagaatatttattcgaaagatgatcacgcgacagcgattagcttccgactgatccacgagaatctgccgaagttcttcgacaacgtcatctcattcaataaattgaaagaaggcttccctgaactcaagtttgataaagtcaaagaagatttagaagttgactatgatctcaagcatgcattcgaaattgaatacttcgtcaactttgtgactcaggccggcattgatcagtataattatctgctgggtggcaagaccctggaagacggtactaagaaacagggcatgaacgagcagataaatctgtttaaacagcagcagactcgtgataaagcgcgccagatccctaagctgatcccgctgtttaaacagatcctgtcagagagaacagagagccagtcatttattccgaaacagttcgagtcggaccaggagttatttgattcgcttcagaagcttcacaacaactgtcaggataaattcaccgtgctacagcaggccattctgggcttagcggaagcggatcttaagaaagtgtttatcaagacaagcgacctgaacgctctgagcaacacgatctttgggaactattccgtcttctccgatgcccttaatctgtacaaggaaagccttaagaccaagaaagctcaggaggcgttcgagaaactgccggcgcattcaattcatgatttgatccagtatttagaacaattcaattcgtccctggatgcggagaagcagcagtcgactgacaccgtgctgaactacttcattaagactgacgaactgtacagcaggtttattaagagcacgtctgaagccttcacacaggtgcaacccttgtttgaattagaggcgctgtctagcaaacgtcgcccgccggaaagcgaagatgaaggagccaagggccaggagggtttcgagcagatcaagcggattaaagcgtatttggacacattaatggaagctgttcactttgcgaaaccgttgtatttagtaaagggtcgtaagatgattgagggccttgataaagatcagtcattctatgaagcgttcgaaatggcttatcaggaactcgaatcactgattattccaatttacaataaagcccgctcttacctgtctcgcaagccgttcaaagccgataaattcaagatcaacttcgataataatacactgctgtctggctgggatgctaacaaggaaacggcaaatgcgtcaatactcttcaagaaagacggtctctattaccttggcatcatgcctaagggtaagacgttcttatttgactactttgtctcatcggaagattcagagaaactgaagcagcgaaggcaaaagacagcagaagaggccttggcccaagatggcgaaagttatttcgagaagatccgctataagctgctgccaggcgcgtctaagatgctgcctaaagtcttcttcagcaacaagaacatcgggttctataacccttcagatgatattctgcgcatccgcaacacggcgagtcatacgaagaatggtactcctcagaagggacattctaaggtcgaattcaacttaaatgactgccataagatgatagatttctttaaatcttccatacagaaacatccggaatggggcagcttcggtttcactttctctgacaccagcgatttcgaagatatgtcagctttctatcgtgaggtggagaatcagggctatgttatctcgttcgataagatcaaagaaacctacatccagagtcaagtggaacaaggtaatctatatttatttcaaatctataataaggacttctctccgtacagcaaaggcaaaccgaacctccatactttgtattggaaggcgttgtttgaggaggccaacctgaacaacgttgtcgcgaaattaaacggagaggcggaaattttctttcgtcgtcattcaatcaaggccagcgacaaagtagtgcacccggcgaaccaagcgatagataataagaacccgcatacggagaaaactcaatcaacatttgagtatgatttggtaaaggataagcggtatacccaagacaagttcttcttccacgtgccgattagtctgaacttcaaagctcaaggtgtgtctaagtttaatgataaggttaatggcttcttgaagggaaatccggatgtgaatattattggcatcgaccgtggtgaacgccacctgctgtatttcaccgtagtgaatcagaagggtgaaattctggtccaagagtctttgaacaccttaatgtctgacaaaggacacgtgaatgattatcagcagaagctggacaagaaagaacaggagcgagacgccgctcgcaaatcatggacgacggtggagaatatcaaagaattgaaggaaggttatctgagtcatgttgtgcataaattggcgcacctcattattaaatacaacgccatagtgtgcctggaggatctgaacttcggtttcaaacgaggtcgctttaaagtcgagaaacaggtgtatcagaaatttgagaaagccttaatcgacaaattaaactatctggtgttcaaagagaaggaacttggtgaagtgggacattatttaacagcatatcagctgaccgcaccgtttgaatcttttaagaaacttggcaaacaatctggtattctattctatgtcccggccgactatacctctaagattgatccgactaccggattcgttaacttcctggatctccggtatcagtctgtggagaaagctaagcaacttctgagcgactttaacgcgattagattcaattcagttcagaactacttcgaatttgaaatagactataagaaactcacgccaaagaggaaggttggaacccagagcaaatgggtgatttgcacctacggagacgtgcgttatcagaatcgtcggaatcagaaaggacactgggaaacagaagaagtgaacgttaccgagaaattgaaggcactatttgcatctgacagtaagactactactgtaattgattatgctaatgacgacaacctgatcgatgtgatcttggaacaggataaggcatctttctttaaagaattgttgtggcttcttaaactgaccatgactctgcgccattcaaagattaaatccgaagacgatttcatattatctcctgtcaagaatgaacaaggtgaattctatgattcacgtaaagcaggtgaagtatggccgaaggatgcggatgctaatggagcttatcatattgccctgaagggactgtggaatctccagcagataaaccaatgggagaagggaaagacacttaacctggcaattaagaatcaagactggtttagctttattcaggagaaaccatatcaggagtaa

SEQ ID NO: 724 - DNA, 3897 bp, Artificial Sequence
  Description of Artificial Sequence: Synthetic polynucleotide
atgacgaagacctttgattctgagttcttcaatctctatagcttgcagaagacagtacgtttcgaactgaaaccggtaggcgaaaccgcctctttcgtagaagactttaagaatgaaggcctgaaacgggtcgtgagtgaagacgagcgccgtgcagtggattaccagaaggtgaaagaaatcattgatgattatcatcgcgactttatcgaagaatcactgaattatttcccggaacaggttagcaaagatgcgctggaacaagcctttcatctctatcagaaactgaaagctgctaaggttgaagaacgggagaaggcattaaaggaatgggaggctttgcagaagaagttgcgtgagaaggttgtcaaatgcttcagcgatagtaacaaagcgcggttcagtagaatcgacaagaaagaactgatcaaggaagacttgattaactggctggtagctcagaatcgtgaagacgatattcctaccgtggaaacattcaacaactttaccacatactttacaggtttccatgagaatcgaaagaatatctactccaaagacgaccacgccacggcgattagctttagactcattcatgagaatctgccaaagttcttcgataacgtcattagtttcaataaacttaaagaaggcttcccagaacttaaatttgataaagttaaggaggatctggaagtggactacgatctgaaacatgcatttgaaattgaatatttcgttaacttcgtcacgcaggcgggcatcgatcagtataactatctattaggcggtaagacactagaggatggaactaagaaacaaggcatgaatgaacagatcaacttattcaagcaacagcagacgcgtgacaaagcgagacagatcccgaaacttataccactgtttaaacagatcctatcggaaaggactgaaagccaatcgttcatcccgaaacagtttgaatctgatcaagaactgtttgatagtctgcagaaacttcacaataattgccaagataagtttacggtgcttcagcaagccatcctgggcttagcagaagctgacttaaagaaggtatttattaagacgtcagatttgaacgcgttatcaaataccatcttcggcaattatagcgtgtttagcgacgcgctcaatttatataaggagtccttgaagacgaagaaggcgcaggaagctttcgagaaactgccggcccatagtatccacgatctgattcaatatctggagcagttcaatagttctcttgatgcagagaagcagcagtctacagataccgttctgaactactttataaagactgatgaactgtatagcagattcattaaatcgacctccgaggccttcacccaggttcagccactgttcgagctggaggcattaagcagtaaacggcgtccgcctgagagcgaagacgaaggagctaagggccaagagggcttcgaacagattaagcgcatcaaggcctacttagacacgctgatggaggcagtacacttcgccaagccattgtatctcgttaaaggtagaaagatgatcgaagggctggacaaagatcagtctttctacgaggcattcgaaatggcctaccaggaactggaaagcctgattattccgatttataataaagcccgtagttatctgtcacggaagccgttcaaagcggacaaatttaagattaacttcgacaacaacaccttactgtcgggctgggacgctaacaaggaaaccgccaacgctagtatactattcaagaaggacggtctgtattatcttggcatcatgccgaaaggaaagacgttcttatttgactactttgtaagcagtgaggactctgagaaactgaaacagcgccgacagaagaccgcagaagaagccctcgcgcaggacggagagtcatactttgagaagattcgatataaactgttaccgggtgccagcaagatgttgccgaaggtatttttctccaacaagaacattggattctacaatcccagcgatgatattctgcgtatccgtaataccgcgtctcataccaagaatggtacgccgcagaagggacactcgaaagtcgaattcaatcttaacgattgtcacaagatgattgacttcttcaaatcgtcgatacagaaacatccagaatggggaagctttgggttcacattcagcgacaccagcgatttcgaagatatgtctgcgttctacagagaagtcgagaatcagggctacgttatcagcttcgacaagatcaaggaaacctatatccagtcgcaagtcgagcagggcaatctgtatttattccagatctataataaggacttcagtccgtactccaaaggtaaaccgaacctgcacacactgtattggaaagcgctgttcgaagaagcgaacctgaataatgtggtggctaaactaaatggcgaagccgaaatattcttcagacgccactccatcaaagcgtcagataaagttgtacatccggcgaaccaggcgatcgataataagaaccctcacaccgagaagacccagtctacgttcgagtatgatttagtcaaagacaagagatatacccaagataagttcttcttccacgttccgatctccctgaacttcaaggcacagggcgtgtcgaagtttaatgataaagtcaatggattcttgaaggggaacccggacgttaatataattggaattgatcgcggtgaacgtcacttattatatttcacggttgttaaccagaaaggagaaattcttgtgcaggaatctttgaatacgctcatgtcggacaagggtcacgtgaacgactatcagcagaagctggacaagaaagagcaggaacgtgacgctgcgcgtaagtcttggaccaccgtggagaacattaaagagttgaaggagggttatctgtctcacgtcgtacataaactggcgcacttgattattaaatataatgcaattgtgtgcctggaggacctgaactttggctttaaacgcggtcgtttcaaagtagagaaacaggtgtatcagaaattcgagaaggcgttgatagacaaactgaattatcttgtatttaaagagaaagaactgggtgaggtaggtcattatttgactgcatatcaactcactgctccattcgagtcctttaagaaactaggcaaacaatcaggcattttattctatgttccggcggattacactagcaagatcgatcccactactggtttcgttaacttcctggatctgcggtatcaatcggtggagaaggccaaacagttattatcagacttcaatgccatccgatttaatagtgtccagaactacttcgagtttgagatcgactataagaaattaactcctaaacggaaggtcggtacccaaagtaaatgggtgatctgcacgtatggcgacgtccgttatcagaatcgtcgcaatcagaagggtcactgggaaaccgaggaagtaaacgtcactgagaaattaaaggccttatttgcgagtgattcaaagaccacgaccgttatagattacgccaacgacgacaacctgatagatgtgattctggagcaagataaggcaagcttcttcaaagaattgttatggctgctgaaactaacaatgacgctgaggcacagcaagattaaatcggaagatgacttcatcttatcacccgtgaagaatgagcagggagagttctatgattcgcgcaaagcgggtgaagtatggccgaaagatgccgatgccaacggagcttaccacattgctctgaaaggtctgtggaatctgcagcaaattaatcagtgggagaaggggaagacgctgaatctggcaataaagaaccaggattggttctcatttatccaggagaaaccgtatcaggaatag

SEQ ID NO: 725 - DNA, 3897 bp, Artificial Sequence
  Description of Artificial Sequence: Synthetic polynucleotide
atgaccaagacattcgattcagaattctttaacctgtacagcctgcaaaagactgttcggtttgaactcaaacccgtcggcgaaaccgcgtcatttgttgaagactttaagaacgaaggcctgaaacgcgtggtgagtgaagacgagcggcgggccgtggactatcagaaggttaaagaaatcatagacgattaccaccgagacttcatcgaagagagcctaaattacttcccggaacaggtgagcaaagatgcgctcgagcaagccttccacctgtaccagaaactgaaagcagctaaagtagaagagcgtgagaaggcgttgaaagaatgggaagcactgcaaaagaaactgagagagaaagttgtcaaatgtttctcggattcgaacaaagctagattctcgcgcatcgataagaaggaactgatcaaagaagatttaatcaattggttagtggcccagaatcgagaagatgatataccaaccgttgagactttcaataacttcaccacctacttcactggctttcatgagaaccgcaagaacatttatagtaaagatgaccacgcaacggctatcagctttcgcctgattcatgagaacttgcccaagttcttcgataacgtgattagcttcaataaactgaaagaaggctttccagaactgaagttcgataaagttaaagaggatctggaggtcgattatgatttgaagcatgccttcgagattgagtatttcgtgaacttcgtaactcaggcgggcattgatcaatacaattatctacttggcggaaagacactcgaagatgggacgaagaagcagggtatgaatgaacaaatcaacctgttcaaacagcagcagactcgcgacaaagctcggcagattccgaagctgatcccactgtttaaacagattctgtcggagcgtaccgaatcccagagctttatcccgaaacagtttgaatctgaccaggaactattcgattctctgcagaaattacacaacaattgccaagataaatttactgtacttcagcaagctatccttggtctggcggaggccgatttaaagaaggtctttattaagacgagcgatttaaacgcactctctaacaccatctttggtaattatagtgtattcagtgatgcgctgaatctgtataaagaatcacttaagaccaagaaggcgcaggaagcattcgagaagctgccggcccattctatccacgatttgattcagtatctggaacagtttaactcatccctggatgcagagaaacagcaaagtaccgatacggtgctgaactatttcataaagaccgacgaactgtatagccgctttattaaatcaacgtcagaagccttcacacaagtgcagccgctgttcgaactggaagcgctgtctagcaaacgtagaccgccggaatctgaggatgaaggcgcgaagggccaggaaggtttcgagcaaattaagcggattaaagcgtatctggataccttaatggaagctgttcactttgcgaagcctctatatctggtcaaaggaagaaagatgattgagggtctggataaagatcagtcgttctatgaagcgtttgagatggcctatcaggaacttgaaagtcttatcattccgatctacaacaaagcgcgtagttatctaagccggaagccattcaaagccgataaattcaagatcaactttgacaataacaccctgttaagcggttgggacgcaaataaagagaccgccaacgcttccatcttgtttaagaaagatggtttgtattatctgggcattatgcctaagggtaagacctttctgttcgactacttcgtttcatctgaggacagtgagaagctaaagcaacgcagacagaagactgctgaggaagccctggcccaagacggcgagtcatatttcgagaagatacgttacaaactgctgcccggtgccagtaagatgttaccaaaggtctttttcagcaataagaatatcgggttctacaatccgagcgacgatatcctgcgaatccgcaacactgcctcgcacacgaagaacggcacaccccagaaggggcattctaaagttgaattcaatctcaatgactgccacaagatgatcgacttctttaagtcttcaattcagaaacatccggaatgggggagcttcggctttacctttagcgatacgtcggacttcgaagatatgtccgcattctaccgcgaagtggagaaccagggctacgtgatttcgttcgacaagattaaagagacatacatccagtcgcaagtggagcagggcaatctgtatctgtttcagatttacaacaaagacttcagcccttattctaaaggtaaaccgaacttacatacgctgtattggaaagccctgtttgaagaagccaatttaaacaacgttgtcgcgaagctgaacggagaagccgaaattttcttccgccgccactcgattaaagcgagtgataaagtggtgcacccagctaatcaggcaattgataacaagaacccgcacacagaaaagactcagtctactttcgagtatgacctggtgaaagataaacgttatacgcaagataagttcttcttccatgtgcccatttccctgaacttcaaagcacagggtgtatccaaattcaacgataaagtcaatggcttccttaaagggaatccagacgtgaacattatcggcattgacagaggggagcgccacctactgtacttcaccgttgtaaaccagaaaggcgagatcctagttcaggaatcgttaaacaccctgatgtctgataaaggtcatgtcaatgactatcagcagaagctggacaagaaagaacaggaacgggatgcagcccgcaaatcgtggacgaccgttgagaacatcaaggaacttaaagaaggctatctctcgcacgtggttcataaattagcacacttaattattaagtacaatgccattgtgtgtttggaggatcttaacttcggtttcaaacgcggtcgtttcaaagtcgagaagcaagtgtatcagaagtttgagaaagctttgattgacaaactgaattatctggtatttaaggagaaggaacttggtgaggtgggacattacttaacagcctaccaactgaccgctccgtttgaaagctttaagaagcttggcaaacaatctggtattctattctatgttcctgccgattatacgtcgaagattgatcccaccaccgggttcgtgaacttcctcgacttgagatatcagagtgtagagaaagctaaacagctcctaagcgatttcaacgcaattcgatttaattcagtccagaattacttcgagtttgaaattgactacaagaaattgacgccgaaacggaaggtaggcacacagagcaaatgggtcatatgtacctacggcgatgtgaggtatcagaaccgcagaaaccagaagggacactgggaaacagaagaagttaatgtgaccgagaagttgaaagccttgtttgcgagtgattccaagaccaccacagttattgattatgctaatgacgacaatctgattgatgtgattctcgaacaggataaagcgagcttcttcaaagaactgctctggcttctgaaactgacgatgaccctcagacactcaaagataaagagcgaagatgacttcattctgagcccggtcaagaacgagcaaggagaattctatgactcgcgcaaagcaggagaggtatggccgaaagacgcggatgcgaacggcgcctatcacatcgcactgaaaggattatggaacctgcaacaaattaaccagtgggagaagggaaagaccttaaacttagcaataaagaatcaggattggttcagtttcatccaggagaagccgtatcaggaatga

SEQ ID NO: 726 - DNA, 3897 bp, Artificial Sequence
  Description of Artificial Sequence: Synthetic polynucleotide
atgactaagaccttcgattcggagttcttcaatctgtatagcctgcaaaagacagtgcgcttcgagttgaaaccggtgggtgaaaccgcatctttcgtggaagactttaagaatgaaggactgaaacgtgtggtgtcggaagatgaacgccgtgctgtcgattatcagaaagttaaggaaatcattgacgactaccatcgagacttcattgaagaaagtctgaattactttccagagcaagtcagtaaagatgccctagaacaggccttccacctttatcagaagttgaaagctgcgaaggtcgaagagcgtgagaaggcgctgaaagaatgggaagccctgcaaaagaagctgcgtgagaaagtagtcaagtgcttcagcgactcaaacaaagcccgcttctcgcgtattgataagaaagaattgatcaaagaggacctgataaattggttagtagctcagaatcgcgaagatgacattcctacggtagaaacctttaacaactttactacctacttcacgggctttcacgagaataggaagaacatatattcaaaggatgatcacgctaccgcgatctcgtttagacttattcatgagaacctgccgaagttcttcgacaacgtcattagtttcaacaaactgaaagaaggctttccggaactaaagttcgacaaagttaaagaggacttggaggtggattatgatctgaagcatgcatttgaaatcgagtatttcgtcaacttcgtcactcaggccggcattgatcagtataattacttacttggcggaaagacgttggaggacggtaccaagaaacagggcatgaacgaacagataaatctgtttaagcagcaacaaacgcgggacaaagcgcgccagataccaaagctgattccgctcttcaaacagatcctcagcgaaagaactgaaagccaaagcttcattccaaagcagtttgaatcggaccaggagctgtttgatagccttcagaaactgcataataactgccaagataaattcaccgtattgcaacaagcaattctgggtttggcagaagcagatttgaagaaagtattcataaagacgagcgatctgaatgctctgtctaataccatctttggtaattattctgtgttctcagacgcgctcaatttatacaaggagtctttaaagactaagaaggcacaggaagcgtttgagaagctgccagcgcacagtattcacgatctgatccagtatctcgagcagttcaattctagcttggatgcggagaagcagcaaagcaccgacactgttctgaattactttatcaagaccgacgagttgtactcgcgattcataaagagcaccagcgaggcctttacacaggtgcagccgttatttgaacttgaagctctaagcagcaaacgtcggccaccggagtcggaagatgaaggcgctaagggtcaagaaggcttcgaacagatcaagagaattaaagcgtatctagataccttgatggaagctgttcactttgcgaaacctctgtatttagtgaagggtcggaagatgatcgaaggcttagacaaggatcaaagcttctatgaggcgtttgaaatggcataccaggaacttgagagcctcattattcctatctataataaagctagatcgtacttgtctcgtaagccgttcaaagcggataaatttaagattaatttcgataataacacactgctatctggttgggatgccaacaaggaaaccgcaaatgcgtcaattctctttaagaaggatggcctctattatcttgggattatgccgaaaggaaagaccttcctgtttgactatttcgtttcgagcgaggactcagagaaactgaagcaacgcagacagaaaaccgccgaagaagcgctagcgcaggacggtgagtcatatttcgagaagattcgttataaattgttaccaggcgcgagcaagatgttgccaaaggtcttcttctcgaacaagaacatcggcttctataacccaagcgatgacatactgcgaattcgaaacaccgccagccatacaaagaacggcacgccgcagaagggacacagcaaagtagaattcaacctgaacgactgtcacaagatgattgacttctttaaatcatccatacagaagcatccagaatggggttcgttcggcttcacgttctctgatacgagtgatttcgaagatatgtcagcgttctatagggaagtagagaaccagggctacgtcatttcattcgacaagattaaagaaacgtatatccagtcccaagtcgaacagggcaatctatatctgtttcagatctataataaagatttctcaccctatagcaaaggtaagccaaacctgcataccctgtactggaaagctttgtttgaggaagccaatttaaacaatgtggtcgctaagctgaacggtgaagccgagatattctttcgtcgtcatagtataaaggcgtcggacaaggtagtccatccagccaatcaagccattgataacaagaacccgcacacggagaagacccagtctaccttcgagtacgatcttgttaaggacaagagatacacacaggataagttcttctttcacgtgcccatcagtcttaacttcaaagcacaaggtgtcagcaagtttaacgacaaagttaacggctttctgaagggtaatccggacgttaatattatcggcattgatcggggtgaacggcacctgctgtacttcacggtcgttaatcagaagggcgagatcctcgtccaagagtcactgaataccttaatgtcggataaaggccatgtaaacgattatcaacagaagttggacaagaaagaacaggagcgcgatgctgcgcgcaagtcatggaccactgtcgagaatatcaaggagctgaaagaagggtacttatcgcacgttgtacataaattagcacatctgatcattaaatacaatgcaatagtttgcttggaggacctgaacttcggattcaaacgcgggcgcttcaaagtagagaaacaggtttatcagaaatttgagaaggctttgatcgataagcttaattatctcgtattcaaagagaaggagcttggcgaagtgggccattatctcacagcctatcaattaaccgcaccattcgaatcgttcaagaagctgggcaaacaaagtggcattctgttctatgttcctgccgattatacctccaagatcgacccgaccacaggctttgttaacttccttgacctgcgatatcagagcgtcgagaaggctaaacagctgttgagtgactttaatgccatccgcttcaacagtgttcagaactatttcgagttcgaaatcgattacaagaagctgacgccgaagcgaaaggtcggcacccagtctaaatgggtgatctgcacgtacggcgacgtacgttatcagaatcgtagaaatcagaaaggtcattgggaaaccgaagaggtgaatgtgaccgagaaactgaaagcgctgtttgctagtgattccaagacaaccacggtgatcgattatgccaacgacgataacctgattgacgtcatcctagaacaggataaggcctccttcttcaaagagctgctatggttgctgaagcttactatgacgctgaggcacagcaagattaaatcggaagatgatttcatattgtcgccggtgaagaatgagcagggagaattctatgattcgcgtaaagccggcgaagtctggcccaaagatgctgatgcaaacggtgcataccatattgctctgaaaggcttatggaacctgcagcaaatcaaccaatgggagaaggggaagacccttaacctggctattaagaaccaagattggtttagctttatccaggagaagccataccaggagtaa

SEQ ID NO: 727 - DNA, 3897 bp, Artificial Sequence
  Description of Artificial Sequence: Synthetic polynucleotide
atgactaagacgtttgatagtgagttcttcaatctgtatagtttgcagaaaacggttcgctttgagctgaagccggtgggagagacggctagtttcgtggaggatttcaagaacgaaggtctcaagcgcgtcgtcagtgaagatgaacgtcgagcggtggattaccagaaggttaaagaaattattgacgattatcatagagacttcatagaggaaagcttgaattactttcccgaacaggtgagcaaagatgcgctggaacaggcattccatctataccagaagctgaaagcggcgaaagttgaggaacgcgagaaggcactgaaggaatgggaggcattacagaaaaaactgcgagagaaggttgtgaaatgctttagcgatagtaacaaagcgcgcttcagtcggattgataagaaagaacttattaaggaagaccttattaactggcttgtagcgcagaatcgcgaggacgacattcccaccgtagaaacattcaacaatttcacaacatactttactggtttccatgagaaccggaagaacatctattcgaaagacgatcacgctactgccattagtttccgtttaatccatgagaatcttccgaagttctttgataatgtaatttcgttcaataaactgaaagaaggcttcccagaactgaagtttgataaagtgaaggaagacctggaagtggattatgatttaaagcacgcatttgaaattgagtactttgtcaactttgtaactcaggcaggcatcgatcaatataattaccttctgggaggtaagacattagaggatggtacaaagaagcaagggatgaatgaacagattaatctgtttaaacagcagcagactcgtgacaaagcccgccagattccgaagctgatcccgctgtttaagcaaatcctgtcggaacgcacagagtcccaatcgtttattccgaaacaatttgaaagcgaccaggaactgttcgatagcttgcagaaactgcacaacaactgtcaggacaaattcacagtccttcaacaagcgatcctgggtctggccgaagcagacctgaagaaagtctttataaagactagcgacctgaatgctctgtccaacaccatatttggcaactatagtgtcttcagcgacgcattaaatctctataaagaatcgttaaagactaagaaagcgcaggaggcgtttgagaaacttccggcgcattccattcacgatctgattcaatatctggaacagtttaactcgtccctggacgcagagaagcaacagtcaactgataccgtattaaattatttcatcaagactgacgagctttacagtcgctttattaaatcaacctctgaagcgtttacccaggtccagcctctgttcgagttagaagcattaagttccaagaggcgaccgccggagtccgaagatgaaggagccaaaggccaggaaggcttcgaacaaattaaacgtattaaagcgtacttagataccctgatggaagccgtgcatttcgcgaaaccactgtatctggtcaagggcagaaagatgatcgaaggtttggacaaagatcagtccttctatgaagcgttcgagatggcctatcaagagctagagagcctgattatccctatatataataaagcgcgcagctatctgtcacgcaagccgttcaaagcagataaatttaagattaacttcgataacaataccctgctgtccgggtgggacgccaataaagagactgcgaatgcgtccatactatttaagaaagatggcctgtactatctcgggattatgcctaagggaaagacctttctgtttgattactttgtctcaagcgaggattcagagaagctgaaacaacgtcgccagaagacagctgaagaggcgcttgcccaagacggcgaatcgtacttcgagaagatccgctacaagctgctgcccggcgcctccaagatgctacctaaagtgttctttagtaataagaacattggtttctacaacccatcggatgatattctgcgtattcgcaacacagcgagccatacgaagaacggcacgccgcagaaaggccactcgaaagtagagttcaacttaaatgattgtcataagatgatcgatttcttcaagagctctattcagaagcacccggaatggggttcgtttggtttcacattctctgatactagcgacttcgaggacatgagcgcgttctatcgtgaagttgagaatcagggttatgtgatttcctttgacaagattaaagaaacctatatccaatcgcaggtagaacagggcaatctgtatctcttccagatctataataaagatttcagcccgtactctaaagggaagccgaacctgcataccctgtactggaaagctttattcgaggaagcgaacctgaacaacgtggtagcaaagttgaatggcgaggctgaaatcttctttcgtcgtcatagtattaaggcctctgataaagtagttcacccagcaaatcaagcaattgataataagaacccgcacacggagaagacacagtcaacctttgaatacgacttagtcaaagacaaacgctatacgcaggataaatttttctttcatgtcccgatctcgcttaacttcaaagcgcagggcgtttctaaatttaacgataaagtgaacggctttctgaaagggaatccggatgtgaacattattggtatcgatcgcggagaacgccatctgctgtacttcactgtagtcaatcagaaaggagaaatactggtacaggaaagcttgaatactctgatgtctgacaaaggtcatgtcaatgattaccagcagaagctggataagaaagaacaggaacgtgacgccgctcgtaagagttggaccaccgttgagaacattaaggagttgaaagagggctatctgtcgcacgtggttcataaactggcccatctgatcattaagtacaacgcgatagtttgtctggaagatttaaacttcggcttcaaacgcggccgctttaaagtggagaagcaggtgtaccagaagtttgagaaagcattaattgataagctgaactacctggtcttcaaagagaaggagcttggcgaagtgggccactaccttacggcgtatcagttaacagcaccgtttgaaagcttcaagaagttaggtaagcaatcgggtatactcttctacgtgccggcagattacacaagtaagattgatcctaccacgggtttcgttaatttcctggatctgcgctaccaatcggtggagaaagccaaacaactgctaagcgatttcaacgctattcgcttcaactcggtgcagaattactttgaatttgaaatcgactacaagaagctgacgccaaaacgcaaagtaggtacacagtccaagtgggtgatttgcacatatggcgatgtccgttatcagaaccgccgtaaccagaaaggccactgggaaaccgaagaagtcaacgttacggagaaactcaaagcgctgtttgcgtctgattcaaagaccaccacggtgattgattatgctaatgatgataacttaattgatgtcatactagaacaggataaggctagcttcttcaaggaattgctgtggcttctgaagctcacaatgacgttacgtcacagcaagataaagtccgaagatgacttcatattatcgccggtcaagaatgagcagggtgaattctatgattctcgtaaggcgggcgaagtgtggcctaaagatgcggacgcaaatggagcgtaccacattgcgctgaaaggcttatggaacctgcagcagatcaaccagtgggagaaggggaagaccttgaatttggccataaagaatcaggactggtttagctttatacaagagaaaccgtatcaggagtaa

SEQ ID NO: 728 - DNA, 3897 bp, Artificial Sequence
  Description of Artificial Sequence: Synthetic polynucleotide
atgaccaagacctttgatagtgaattcttcaatttgtattctttgcagaagaccgtgcgctttgagctcaaacctgttggagagacagcgagctttgtggaagactttaagaatgaaggtctgaaacgggttgtatcggaggatgagcgtagggcagtagactatcagaaagtcaaagaaatcatcgacgattatcatcgggacttcattgaagaatctctgaattacttccctgagcaagtgagtaaggatgcgttggaacaggcgtttcatttataccagaagcttaaagccgccaaggtggaagaacgtgagaaagctttgaaagaatgggaagctctgcaaaagaagctgcgtgagaaagttgtgaagtgtttctcagactcgaacaaagcgaggtttagccgcattgacaagaaagagctgatcaaagaagatctgattaactggctggttgcacagaaccgggaagatgacatccctacggtcgagacattcaacaacttcacgacatatttcacgggtttccacgagaatcgcaagaatatctacagtaaagacgatcacgcaacagcaatttcctttcgcctgattcatgagaatctgccaaagttctttgataacgtgatctcctttaataagctcaaagaaggtttcccggagcttaaatttgataaagtgaaagaggacctagaagtggattatgacctgaaacacgcattcgagattgaatactttgtaaacttcgtcacacaggcgggtattgatcagtacaattatctgctgggtggtaagacccttgaagatggcaccaagaaacagggcatgaatgagcaaattaatttatttaaacagcagcaaacccgtgataaggcccgccagattccaaaactgatcccgctcttcaaacagatcctttccgaacgtaccgaatctcagagcttcatcccgaaacagttcgagtctgaccaggagttatttgactctctgcagaaattgcataacaattgccaggacaaatttacggtactacagcaagcgatcctgggtctggcggaggcggatcttaagaaagtgttcatcaagacctcagatttaaatgccctctcaaacaccatcttcggtaactactctgtcttttctgatgcattgaacctgtataaagaatctttgaagacgaagaaagcgcaggaagcgttcgagaagctgccggctcattcgattcatgaccttattcaatatctcgaacagtttaattcatcactggacgcggagaaacagcagtcaaccgacaccgttctaaattactttatcaagacggatgaattgtactctcgattcattaaatcgacctcagaggcgttcacgcaggttcaaccactgttcgaactggaagccttgtcgagcaagcgtagaccgccggaaagtgaagacgaaggtgctaagggtcaagagggctttgaacagatcaaacgcattaaggcgtacttagacaccctgatggaggcagtacatttcgcgaaaccattatatctggttaaaggtcggaagatgatcgaaggccttgataaagatcagtccttctacgaagccttcgaaatggcatatcaggagttagaaagcctgatcatcccgatttataacaaggctcggtcttatctgagtcgcaagccgtttaaggcagataaattcaagattaacttcgataataatacccttctgtccggctgggacgccaataaagaaacagcgaacgcgagtattctgttcaagaaagacggtctgtattacctgggtatcatgcccaaggggaagacattcttatttgattatttcgtttccagcgaggattccgagaagcttaaacagcgccgccagaagaccgcagaagaagcgttggcccaggatggcgaatcgtatttcgaaaagattcgctataagctgctgccgggcgcgagcaagatgctcccgaaagtgttcttctcgaacaagaatattggattctataatccgtcagatgatattcttcgtatacggaacacggcctcccatacgaagaacgggactcctcagaagggccatagcaaagtggaatttaatcttaatgactgccacaagatgattgacttctttaaatcctcgatccagaaacacccggaatggggcagcttcggcttcacgtttagcgatacctctgacttcgaagatatgagtgccttctatcgagaagttgagaatcaaggttacgtgatctcctttgataagatcaaagaaacatatattcagtctcaagttgaacagggtaacctatatctgttccaaatctataacaaagacttctctccatatagcaaaggtaaaccaaatcttcacaccctgtattggaaagctctgtttgaggaggctaatctgaataacgtggtggcgaaactgaacggagaggcagaaatcttttttcggcgacatagtatcaaagcgagtgataaagtggtgcatccagcaaaccaggcgatcgataataagaatccgcacaccgaaaagacccagtcaacattcgaatatgacctggtcaaggacaaacgctatacccaggataagtttttcttccatgtgccaatctctttaaactttaaagcgcaaggagtgagcaagttcaacgacaaggtaaatggcttcctgaaaggaaatccggacgtaaatatcattgggatcgaccggggggaacgacatctgctttacttcacggtggtgaaccagaaaggagaaatactcgtgcaagaatcattaaacaccctgatgtctgataaaggccatgtcaacgattatcaacagaaacttgacaagaaagaacaagagcgcgatgcggctcgcaaatcttggacgactgtggagaatattaaggaattgaaggaaggctacttatcgcatgttgtgcataaattagcccatctgattatcaagtacaatgcgatcgtgtgcctggaagatttaaactttggttttaagagaggtcgctttaaagtagagaaacaagtgtaccagaagtttgagaaagcgcttatagacaagctgaattatctagtattcaaggagaaggagcttggcgaagtcggccattatttgactgcatatcagttaaccgcacccttcgaatcctttaagaaacttggcaaacagtccgggattttattctacgttccagccgattatacgtcgaagattgatccaacgaccggtttcgtgaacttccttgatttgcggtatcagagcgtggagaaagcgaaacaattgctgtctgacttcaacgcaattcgattcaattctgtgcagaattacttcgaattcgagattgattataagaaactgacaccgaagcgtaaagtgggtactcagagtaaatgggttatctgtacctacggcgacgtccgttatcagaatcgccgcaaccagaagggccattgggaaaccgaagaggtgaacgtcacggagaagctgaaagcgctgtttgccagcgactctaagaccactacggttatagattacgcaaatgatgacaatttaattgatgtaatactcgagcaagataaagcctcgttctttaaagaactcctgtggttacttaagctgaccatgacgcttcgtcacagtaagataaagagcgaagatgacttcattctgagcccggtgaagaatgaacaaggcgaattctacgattctcgtaaggcgggcgaagtttggcctaaagatgctgacgcgaatggcgcatatcacattgcgctgaagggcttatggaacttacagcaaataaaccagtgggagaagggaaagaccctgaaccttgcaatcaagaaccaagactggttttcgttcatccaagagaagccgtatcaagagtga

SEQ ID NO: 729 - DNA, 3897 bp, Artificial Sequence
  Description of Artificial Sequence: Synthetic polynucleotide
atgaccaagacattcgatagtgagttctttaatctgtactctctgcagaagaccgttagatttgaacttaagccggtgggcgaaactgcgtcctttgtagaagactttaagaatgaaggtctgaagcgtgtggtgagcgaagacgaacgtcgagccgtggattatcagaaagtcaaagagattattgatgactatcaccgagacttcatcgaagaaagcttaaattactttccggaacaagtcagtaaggatgccctggaacaggcgtttcatctttatcagaaactgaaagccgcaaaggtcgaagaacgcgagaaagcactgaaggagtgggaagcactgcagaagaagctgcgggagaaagttgttaagtgtttctcagattcaaacaaagcccgtttctcccgcattgataagaaggaactgatcaaggaagatcttattaattggctggtggcgcagaaccgcgaagacgacattcctactgttgaaacattcaacaactttacgacatactttactggattccacgagaaccgtaagaatatctattcaaaggatgatcacgccaccgcgattagtttccgcttgattcatgagaatttaccaaagttcttcgacaacgttataagcttcaacaaactgaaagagggctttccggaactgaaatttgataaagtgaaagaagatcttgaagtggactatgatcttaaacacgcctttgaaatagaatacttcgtcaactttgtaacccaagctggtattgatcaatataactatctgctgggcggaaagacgttggaagatgggacaaagaaacagggtatgaatgaacaaatcaacttgttcaaacaacagcagactagagataaagcgcgtcaaattcctaaacttataccgctatttaaacaaatcttaagcgaacgtaccgaatcgcagtcgttcattccgaaacaatttgaatcggatcaagaattgtttgattcacttcagaaactgcacaacaattgccaggacaaatttacagtacttcagcaagccatcctgggtctggcagaagccgacttaaagaaagtcttcattaagacgtctgatctgaatgcattatcgaatacaatattcggaaactactctgtgttctcagacgccttgaacctgtacaaggaatcgctgaagacgaagaaagcgcaagaagcctttgagaagctgccagcccactctattcatgatctcattcagtacctggaacagttcaacagttcgctggatgcggagaagcaacagagcacggacaccgtcttaaattacttcataaagacggacgaactttactcccgtttcattaagtcaactagtgaggcctttactcaggtgcaaccactgttcgaactggaagccctatcttcgaaacgtcgcccaccggagagcgaagatgaaggtgccaagggtcaagagggctttgagcaaattaagcgcattaaagcgtatctggacacgcttatggaagcggtacacttcgccaaaccgttgtacttagtgaaaggtcgtaagatgatcgaaggtctggacaaagatcagagtttctatgaagcgttcgaaatggcctatcaagagctggagtctctgattatcccgatttataataaagcacgtagctatctgtcacgtaaaccgtttaaggcagacaagttcaagatcaactttgataacaacaccctgctaagcggttgggacgcgaataaagaaacggccaacgcgagcattctgttcaagaaagacggtttatactatttgggtattatgccgaaaggtaagacgttcttatttgattacttcgtgagcagtgaagattcggagaaactgaaacagcgccgtcaaaagacagccgaggaggcgttggcgcaggatggtgagtcttacttcgaaaagattcggtacaagctgctgccgggtgcgagtaagatgctgccgaaagttttctttagcaataagaacatcgggttctataacccatctgatgatatccttcggattcgcaataccgcctctcatactaagaacggtacgccgcagaaaggtcacagcaaagttgaatttaatttaaacgattgtcacaagatgattgacttcttcaagagttcaattcagaaacacccggaatggggatcgtttggatttacattcagtgatacttcggacttcgaagacatgtcagcattctatcgcgaagtagagaaccaaggctacgtgatctccttcgacaagatcaaagaaacatatatccagagccaagtcgagcagggcaatctgtacttattccaaatttataataaagactttagtccttattcgaaagggaagcctaacttacataccctttattggaaggcactctttgaagaagcgaacctcaacaatgttgtagccaagctgaacggcgaagcggaaatcttcttcagacgccactctattaaggcgagcgacaaagtggtgcatccagctaaccaggctattgacaacaagaacccgcatactgagaagacacagtcaacgtttgaatatgatctagtgaaagataaacgttatacccaggataaattcttcttccatgtgccgatttcattgaacttcaaagctcaaggcgtctctaaatttaatgataaggtgaacggcttcctaaagggaaatccggacgtgaatattattggaatcgatagaggtgagcgtcacctgctgtacttcactgtggtgaatcagaaaggagagatcttagttcaagaaagcctgaataccctgatgagtgacaaaggccatgttaatgactatcagcagaaattggacaagaaggaacaggaacgtgacgctgcaaggaagagttggaccactgttgagaacatcaaagagcttaaagaaggttatttatctcacgttgtacataaactggcgcatttgattatcaagtacaacgcaatcgtgtgtctcgaagatttgaactttggattcaaacgtggccgcttcaaggtcgagaagcaggtgtatcagaagtttgagaaagcccttattgataaattgaactatttggtcttcaaagagaaggaactaggcgaggtgggtcattatctgacggcatatcaactgaccgctccgttcgaatcgttcaagaagctcggcaaacagtctggtatcctcttctacgttccagcggactatacctcgaagatcgacccgacaaccggattcgtcaacttcctggatctgcgctaccaatccgttgagaaagctaagcaactgctgagcgacttcaacgcaattagattcaactcagtgcagaactatttcgaatttgaaatagactacaagaagctgacgcctaaacgcaaagtgggtacacagtctaaatgggtgatatgtacctatggtgacgtacgctaccagaatcgacgcaaccagaaaggccattgggaaacggaagaagtcaatgtcaccgagaagttgaaagcactgtttgcatcagactccaagactaccaccgtcattgactatgcgaacgatgataatttgatcgatgttatactcgaacaggacaaagccagcttcttcaaagaactcctttggctgctgaaactgaccatgactctgcgccactctaagataaagagcgaggacgatttcatactaagcccggtaaagaatgaacagggtgagttctatgacagccgtaaggcgggagaagtctggccgaaagatgctgatgcgaatggcgcttatcacattgcgctgaaaggcttatggaatcttcagcagatcaatcagtgggagaagggaaagacccttaacctagctattaagaatcaagattggttctcgttcatccaagagaaaccgtatcaggagtaa

SEQ ID NO: 730 - DNA, 3897 bp, Artificial Sequence
  Description of Artificial Sequence: Synthetic polynucleotide
atgacgaagactttcgactcggagttctttaatctgtacagtctgcaaaagactgttcgtttcgaattaaagccggtgggtgaaacagcttccttcgtggaggacttcaagaacgaaggtctgaagcgcgtagtctcggaagacgaacgacgagcagtggattatcagaaagtcaaagaaattattgacgattatcatcgcgacttcatcgaagaaagccttaattactttccggaacaggtttctaaggatgcccttgaacaggcattccacttatatcagaagctcaaagccgccaaggtagaagaacgtgagaaggcgcttaaagagtgggaggcgttgcaaaagaaacttcgcgagaaagtggtgaaatgtttctcagattcgaacaaggctaggttctcccgtattgataagaaagagttaattaaagaggatttgattaattggctggttgctcagaaccgtgaagacgatattccgaccgtggagaccttcaataacttcaccacctatttcaccggtttccatgagaataggaagaacatctactccaaagacgaccacgcgaccgcgatttcgtttcgtctgattcacgagaatctacctaaattctttgataacgtgattagctttaacaagcttaaggaaggcttcccggaactgaagtttgataaagtgaaggaggatctcgaagttgattatgacctgaaacatgccttcgaaattgaatatttcgtcaatttcgtgacgcaggccgggatcgatcaatacaattacctgctgggcggaaagacgcttgaggatgggacaaagaaacagggcatgaatgagcagatcaatttattcaagcaacagcagactagggacaaggcacgtcagatcccgaaactcattcctctgtttaaacaaatcctgtccgaacgtaccgaatcacagtctttcattcccaaacaatttgagagtgatcaggagctgttcgatagtctgcagaaactgcataacaattgccaagataaattcactgttcttcaacaggcgatccttggtctggctgaagccgacttaaagaaggtattcatcaagacctcagacttgaatgccttgtctaacaccatcttcggaaactactcagttttctcggatgcgctgaacctgtataaagaaagtcttaagaccaagaaagcgcaggaggcgtttgagaaattgccggcgcatagcatccatgatttaattcaatatctggagcaatttaatagtagtttggatgcagagaagcaacagtccaccgacacagtactgaattacttcatcaagactgatgaactgtactcacgctttattaagagtactagcgaagcgtttacccaagtacaaccgctgtttgagctggaagcactgtcctctaaacgtcgaccgccggaaagcgaagatgagggcgccaagggccaggaaggcttcgagcagattaagcgtattaaagcatatttagataccctcatggaggccgtccatttcgcgaagccgctgtacttggttaaaggacgaaagatgatcgagggcttggataaagatcaatcattctacgaagcatttgaaatggcgtatcaggaactggaaagcttgatcatcccgatttataacaaagcccgttcgtacctgtcccgtaaacctttcaaggcagataagtttaagataaactttgacaacaatacgctgctgtccgggtgggacgccaataaggagacggcaaatgcgtcaattctgtttaagaaagatggcctgtactatctcgggatcatgccgaagggaaagaccttcttattcgattatttcgtcagttccgaagactcagagaaattaaagcagcgacgacaaaagaccgcagaagaagcacttgcgcaggacggtgaaagctactttgagaagattcgctacaaattgctccctggcgcctcgaagatgctgccgaaagtatttttctcaaataagaacatcggtttctacaacccgtctgatgacatcttacgtatccgtaacactgcgtcccacaccaagaacggtactccgcagaagggtcactccaaggtagagtttaatctgaacgattgtcataagatgatagacttctttaagagcagtattcagaagcatccggaatgggggtcattcggctttacattctccgatactagtgacttcgaagatatgtcagccttctatcgcgaagttgagaatcaaggctacgttatctcgttcgacaagatcaaagagacgtatatccagtcccaggtagaacaagggaacttgtatctgttccagatctataacaaagatttctcaccgtatagtaaaggtaaaccaaaccttcataccttatattggaaagcgttgtttgaagaagccaacttaaataacgttgtggccaaattgaacggcgaagccgagattttctttaggcgtcatagcattaaagctagcgataaagttgtacacccggcgaatcaggcgattgataacaagaatccacacaccgagaaaacgcagtcaaccttcgaatatgacctggtcaaggacaagcgctacacccaggataaattcttctttcatgtacctatatcgctgaactttaaggctcagggcgtgtcgaaatttaatgataaagttaatggcttccttaaaggtaacccagatgttaatataattggaattgatcgtggagaacgccacttgctgtatttcaccgttgtaaatcagaagggcgagatcctggtgcaagaatcgttgaacaccttaatgtctgacaagggccatgttaacgactaccagcagaagctagataagaaggaacaggaacgtgatgctgcaaggaagagttggaccactgtagagaatatcaaagaactcaaggagggatatcttagtcatgtagttcacaaactggctcatctgatcattaagtacaacgccattgtgtgcctcgaagacctgaactttgggtttaaacgcgggaggttcaaagtggagaaacaagtataccagaagtttgagaaagccctgattgataaactgaactacctggtattcaaggagaaggaattaggcgaagtgggtcattacctgaccgcatatcaattaacggcaccatttgagagctttaagaagctgggtaagcagtctggtatcttattctacgttccagcggattacacgtctaagattgatccgacgacaggatttgtgaactttctcgatttgcgctaccagagtgtagagaaggctaaacaattgctgtccgatttcaatgcaattcgcttcaatagcgtacagaactactttgaatttgagatcgactataagaagctcacacctaaacgcaaagtgggcactcagtctaaatgggtcatttgtacttacggcgacgtgcgttatcagaatcgtcgcaatcagaagggacattgggaaacagaggaagtaaacgtcaccgagaagctgaaggcgctattcgcgtcggattcaaagacgacaacagtgatcgattatgcgaatgacgataacctgatcgatgtgatcctcgaacaagataaggcatccttctttaaagagttgctttggttgctcaagttgaccatgaccctgcgccacagtaagatcaagagcgaggatgacttcatcttgagcccagttaagaatgagcagggtgagttctatgatagccgtaaagccggcgaggtgtggcccaaggatgcggatgcgaacggcgcgtatcatattgcgttgaaaggtctgtggaacctccaacagattaatcagtgggagaagggaaagactcttaatttagccatcaagaatcaagattggttctctttcatccaggagaagccgtatcaagaataa

SEQ ID NO: 731 - DNA, 3897 bp, Artificial Sequence
  Description of Artificial Sequence: Synthetic polynucleotide
atgacaaagacctttgacagtgagttctttaatctgtattcactccaaaagacggtgcggttcgaacttaaacctgttggagaaacagcatctttcgtcgaagactttaagaacgaaggcctgaaacgagtagtaagtgaagatgagcgtcgcgcggtggattaccagaaggtcaaggagatcattgatgactatcatcgcgactttatagaagaatctctgaattacttcccggagcaggtcagcaaagatgcgctagaacaagcattccatttgtaccagaagctcaaagcagctaaagtggaagaaagagagaaagcactaaaggaatgggaagctctccagaaaaaacttcgtgagaaagtggtcaagtgcttcagcgactctaataaagcccgctttagccgtatcgacaagaaagaactgatcaaagaagacctgatcaattggttagttgcgcagaatagggaagatgatattccaacggtagaaacctttaataacttcaccacgtatttcaccgggttccacgagaaccgcaagaacatctacagcaaggatgatcatgcaaccgccatcagtttccgcctgattcacgagaatctaccgaagttctttgacaacgtgatcagcttcaataaactgaaggagggctttcccgaattgaagttcgataaagtcaaagaagatctggaagtggattatgatttgaaacacgcctttgagatcgaatactttgtcaacttcgtcacccaggccggcattgatcagtacaattatctactcggtggcaagactttagaagatggcacgaagaaacaaggcatgaatgaacagatcaatctgttcaaacagcagcaaacccgtgataaagcccgtcagatcccgaagcttattcccttgttcaaacagatactcagtgaacgcacggagtctcaaagcttcattccgaaacagtttgaatctgaccaggagttgttcgacagcttacagaaactgcataataactgtcaagataaattcactgtgttgcaacaagctatccttggcctggccgaagccgacttgaagaaagtatttataaagacgtcagatcttaacgccctgtctaacactatcttcggcaactatagcgtattcagtgacgcgctgaatctttacaaagaatctttgaagacaaagaaggctcaggaagcgtttgagaagctgcccgcccactccattcacgatctgatccagtatctggaacagttcaactcaagtctcgatgcggagaaacagcagagcacagacaccgtacttaactacttcataaagactgacgaactgtactcaagattcataaagagtacatcagaggctttcacccaggtgcaaccactcttcgaactagaagccctgtctagcaagcgacggccgccagagagcgaggatgagggtgccaaaggccaggaaggcttcgaacagattaaacgcatcaaggcctatctcgatacgctaatggaagctgtccactttgcgaagcctctttatctggtgaaaggtagaaagatgattgaaggcctggacaaagatcagtctttctatgaagccttcgaaatggcgtatcaggaactggaatcgcttattatcccaatttacaacaaggcgcgatcatacctgagccgcaaaccgtttaaagcagataaattcaagatcaactttgataataatacactgctgtcgggttgggatgccaataaagaaaccgcgaacgcgagcatattatttaagaaagacggcttatattatcttgggattatgcctaaaggcaagacctttctgttcgattatttcgtgagcagcgaggactctgagaaacttaaacaaaggcgccaaaagactgccgaagaagccctggcacaggatggcgaaagttacttcgaaaagatacgttataaactgttgcctggtgcaagtaagatgctgcccaaagtcttcttctcaaataagaatatcggcttctacaatccttccgatgacatccttcgcatccgcaacaccgctagccatacaaagaacggcacgccccagaagggccattctaaagtggagtttaatctgaacgattgtcataagatgattgacttcttcaagtcttctattcagaaacacccagaatgggggagcttcggattcacattctctgacacttcagatttcgaggacatgtccgccttctatcgtgaagtcgagaaccagggttatgtaatctcgttcgacaagatcaaggagacatacattcagtctcaggtagagcagggcaatttgtatctgtttcagatttataataaagacttcagcccatattcgaaaggtaagcctaacttgcataccctttattggaaagcgttattcgaagaagcgaaccttaataatgtggttgctaaattgaatggcgaagctgaaatcttctttcgtcgtcatagcatcaaagcgtctgataaagtagtgcatccggcgaaccaggccatcgataataagaatcctcacaccgaaaagacccaatctaccttcgaatacgatctggtgaaagacaaacgctatacccaggataagttcttcttccacgttccgatatccctgaactttaaagcccagggtgtgtccaagttcaatgacaaggtgaacggtttcctgaaagggaacccggacgtaaatattatcgggatcgatcgcggtgaacgtcatctgttgtactttacggtggtaaatcagaaaggcgaaatcttagtgcaggaatctctgaataccctcatgagtgataaaggtcatgtgaatgactaccagcagaagttggacaagaaagaacaggaaagagatgcagcaaggaagtcctggaccacggtggagaatatcaaagaactgaaagaaggttacctgagccatgttgtccataagctggcgcacctgattatcaaatataacgctattgtttgcctggaagacctaaactttggcttcaagagaggtcggtttaaagttgagaagcaagtatatcagaaatttgagaaggctctgattgataaattaaattacctggtgttcaaagagaaagaacttggagaggtcggccattacttaactgcttaccaattaacggctccgttcgaatccttcaagaaattaggtaagcagagcggcattctattctatgtacctgcggattacacgtcaaagattgacccaacaacgggatttgttaacttcttagatttgcgttatcagtcggtggagaaagccaaacagctgcttagcgacttcaatgctattcgattcaatagtgtccagaattacttcgaatttgaaattgattacaagaaattgactcctaagcgtaaggtgggcacacagagcaaatgggtgatatgcacctatggcgacgtgcgttatcagaaccgtcgtaaccagaaaggtcattgggaaacagaagaagtgaatgtgaccgagaagctcaaggcgctgtttgccagcgattccaagaccacgacggtcattgattatgctaatgatgataatttaatagatgtcatcttggagcaggataaagcatccttcttcaaagaattgctatggttattaaagctgaccatgacgctccgccatagtaagatcaagagcgaagacgactttatcctgtctccggtcaagaacgaacagggtgagttctacgattcacgtaaggctggcgaagtttggccgaaagacgcagacgcgaatggcgcctaccatatcgccctgaaaggtctgtggaacctgcagcagattaaccaatgggagaagggtaagaccctgaatctcgccatcaagaatcaggactggttctctttcattcaagagaaaccgtatcaggaatag

SEQ ID NO: 732 - DNA, 3897 bp, Artificial Sequence
  Description of Artificial Sequence: Synthetic polynucleotide
atgacaaagacgttcgactccgagttcttcaatctctacagtctgcaaaagaccgtacggtttgaactgaaaccggtgggtgagaccgcaagctttgtcgaggactttaagaatgaaggcctgaaacgagtggttagtgaagatgaacgccgtgcggtcgattatcagaaagttaaagagattatcgatgactaccatcgcgactttatcgaggaaagcctaaattacttccctgagcaggtttcgaaggatgcgctcgaacaagcctttcatctgtatcagaaattgaaggccgcgaaagttgaagagcgcgagaaggcactgaaagaatgggaggcactgcagaagaaactgcgggagaaggttgttaaatgtttctctgacagtaacaaagcgcgtttctcaaggattgacaagaaagaactgatcaaagaggatctgatcaactggctggtagctcagaatcgtgaggatgatattccaacggttgagacgtttaacaatttcactacctatttcacaggtttccatgagaatcgaaagaacatatattctaaggacgatcatgccacggcaatctcgtttcgcctgattcatgagaatctgcccaagttcttcgacaatgttattagcttcaacaaactcaaggaaggattcccggaactgaaattcgataaggttaaagaggatctggaagtcgattatgacctaaagcatgcgttcgaaatcgaatactttgtcaatttcgtaactcaagcgggtatcgatcagtataactatctgctcggagggaagactttggaagacggcacgaagaaacagggtatgaatgaacagattaatctgtttaaacaacagcagactcgcgataaggcaagacagattccgaaactgattccactgttcaaacaaattctgagcgaacgtactgagagccagagctttattcctaagcagtttgaatcagatcaggagctgttcgacagcctgcagaaactgcataacaattgccaagacaaatttaccgtattacagcaggctatcttaggtttggctgaagctgatctcaagaaagtattcattaagacatctgaccttaacgccttgtcaaacacgatcttcggaaattacagcgtcttcagcgatgcgttgaacctatacaaagagtcattaaagactaagaaagctcaggaagccttcgagaagttaccggcccattccatccacgacctgatccaatatttggagcaatttaactcgagcctggatgcggagaaacagcagtcgacagatactgtgctgaactatttcataaagacggacgaactttattcgcgctttattaaatctacaagcgaagcgtttacccaagtgcagccgctctttgagttagaggcattgtctagtaagagacgtccacctgaatctgaggatgagggtgctaaaggtcaagaaggattcgagcaaattaaacgtattaaagcatatctggatacccttatggaagcagttcatttcgcgaaaccgctgtacttggtcaaaggaaggaagatgatagaaggtctcgacaaggatcagagcttctacgaggcatttgaaatggcctatcaagagctggaaagcctaattattcctatttataataaagcccgtagttacctgtcgcggaaaccgtttaaagcggataaattcaagatcaacttcgataataataccctgctgagcggttgggatgcaaacaaggagactgcaaatgcaagtatcctcttcaagaaagacggactgtactatctgggcatcatgcctaaaggtaagactttcttgttcgactacttcgtgtctagcgaagactctgagaaactcaaacagcggcgtcagaaaaccgcagaagaagccctcgcccaggatggcgaatcttatttcgagaagatccgctataaactgctgccgggtgcctctaagatgttgcctaaagttttcttttcaaataagaatatcgggttctataatccgtcagatgacatcctgcgaattcgcaataccgcttctcacactaagaatggcacgccccagaaaggacactcgaaggtggagtttaatttaaatgattgccataagatgattgacttcttcaaatcgtcaatccagaaacatccagaatggggtagctttggctttacattctcggacacaagcgatttcgaagatatgtctgccttctaccgtgaagtcgagaaccaaggctatgtgatttcgtttgacaagattaaggaaacctacattcaaagccaagtcgaacaaggtaatctgtacctgttccagatttacaataaagatttcagcccgtattctaaaggcaaaccgaatctgcataccctgtattggaaagctctctttgaagaagcaaacttgaataacgtggtggctaagttgaatggtgaagcggaaatattctttcgtagacactctatcaaagccagtgataaggtagtccatccggcgaatcaggctatagataataagaacccgcacactgagaaaactcagagcacattcgaatatgatctggtgaaagacaaacgttatacacaagataaattcttcttccatgtgccaattagtttaaatttcaaggctcagggcgtctcgaaatttaacgacaaagttaatggctttctgaagggaaacccggatgtcaatattattgggattgatcgcggagaacgccatctgttatactttacagtggttaatcagaagggcgagattctggttcaggaaagcctgaatactttaatgagcgacaaaggccatgtaaatgattatcaacagaaactggacaagaaggaacaggagagggacgccgcccgcaagtcatggactaccgtggagaatattaaggaattgaaagaaggctacttgagtcacgtcgtgcataaactggctcatctgattattaaatacaatgcgatcgtctgcttagaagatttaaatttcgggttcaagcgagggcgattcaaggtcgagaagcaggtttaccagaaattcgagaaggcgttaattgacaagttgaactatttagtgttcaaggagaaagaacttggtgaggtgggtcattacctgacggcatatcagttgacggcacccttcgaatcatttaagaaactgggaaagcagtcgggcattcttttctatgtgccagcggattacactagtaagatcgatccgacaaccgggttcgttaatttccttgatcttcgctaccaatcagtagagaaagccaagcaactgctgtcagacttcaatgcaattcgctttaatagcgtacagaactacttcgaatttgagattgactacaagaaactgacacctaagcgaaaggttggcacccagagcaagtgggtaatctgtacctacggcgacgtccgttatcagaaccgtcgtaaccagaaaggtcattgggaaactgaagaagttaatgtaaccgagaaacttaaagcgttgtttgccagcgactccaagacgacgacggtgatcgactacgctaatgacgacaatctgattgatgtgattctggaacaagataaagcgagcttctttaaagaactattatggctgctgaaacttaccatgacgctgcgccacagtaagatcaaatcggaagatgacttcatactatcaccggtaaagaacgagcagggagagttctatgacagtaggaaagcaggtgaagtatggccgaaggacgcggatgccaacggcgcgtatcacattgcgctaaagggtttatggaacttacaacagattaaccagtgggagaaagggaagacgcttaacttggcgataaagaaccaagactggttctcatttattcaagagaagccgtatcaagagtga

SEQ ID NO: 733 - DNA, 3897 bp, Artificial Sequence
  Description of Artificial Sequence: Synthetic polynucleotide
atgacaaagaccttcgattccgagttcttcaatctgtactctcttcagaagacggttcgtttcgaactgaagcccgttggtgaaactgcgtcatttgttgaagacttcaagaatgaaggtttgaaacgcgtggtgtcagaggacgagcgtcgggcagttgattatcagaaagtgaaggaaattatcgatgattaccatcgagacttcattgaggaaagcttaaattacttcccggaacaggtcagcaaagatgccctcgaacaggcctttcacctgtatcagaaactgaaggcggccaaagtcgaagaacgtgagaaggctttgaaggaatgggaagccctgcaaaagaaactgcgcgagaaagtcgtgaagtgtttctctgattctaataaagcaaggttctcacgtatcgataagaaggaactgatcaaagaggatctgattaattggttagttgcacagaatcgtgaagatgatatcccgactgttgaaacctttaacaacttcactacgtacttcacgggtttccacgagaatagaaagaacatttatagcaaggatgatcacgcaaccgcgatttcctttcgcttaattcacgagaatttaccgaagttctttgacaacgttatttccttcaacaaactgaaagagggctttccggaactcaaattcgataaggtcaaggaggatctggaggttgattacgatttgaagcacgcctttgaaatagagtactttgtgaacttcgttacacaggcaggcattgatcagtacaactatctgcttggagggaagaccctggaggatggtaccaagaaacagggtatgaacgaacagatcaatttgtttaagcagcagcagactcgtgacaaagctcgtcaaatcccgaaactgatccctttgtttaagcagatcttaagcgaacggaccgaatctcagtctttcataccaaaacagttcgagagcgatcaggaattgtttgatagcttgcagaaactgcataacaattgtcaagacaaatttaccgtcctccagcaggcaatcctcggtctggcggaagctgacctaaagaaagtgtttattaagacctctgatttaaatgcactttctaacacgatatttggcaactatagtgtattctcagacgccctgaacctgtataaagagtctttgaagacgaagaaagcccaagaagcgtttgagaaacttccggcgcattcgatccacgatctgattcagtatctcgaacagtttaactcaagcctggacgcggagaagcagcagtctaccgatacagttctgaattacttcattaagaccgatgaattgtattcgcgcttcatcaagtcgacctctgaagcgtttacccaggttcagccactcttcgaacttgaagcattaagttccaagcgcagaccgccggaatccgaagatgaaggagcgaaaggtcaggagggattcgaacagataaagagaatcaaagcttatctggataccctaatggaagcagttcactttgctaagcccttatatcttgttaaaggtcggaagatgattgagggcctggataaagatcagagtttctatgaagcgtttgagatggcctatcaggaactggaaagtttaattattccgatttataacaaagctcgtagctacctcagtcgtaagcctttcaaagcagataaattcaagatcaatttcgataacaatacgctgctgagtggctgggatgcaaacaaggaaacggctaatgcatcaattctgtttaagaaagacggcctttattatttgggcatcatgcccaaagggaagacattcttattcgactacttcgttagcagcgaagatagtgagaaactgaaacagcgccgccagaaaaccgccgaggaagcactggcccaagatggagaatcatatttcgagaagatccgttataaactgttgccgggcgcttcgaagatgctgcctaaggtcttcttcagtaataagaatataggcttctataacccgtctgacgatatacttcgcattcgtaatactgcgagccataccaagaatggcactccgcagaaaggtcactccaaagttgaattcaatctgaacgactgccataagatgattgatttcttcaaatcatcaattcagaagcatccggaatggggatctttcggattcacgttcagcgacaccagcgactttgaggatatgagcgccttctatcgggaagtggagaaccaaggctatgttatctctttcgacaagatcaaagaaacctatatacagagccaggtagagcaaggtaacttgtatctgtttcaaatctacaacaaagatttctcgccgtatagtaagggtaaaccgaatctacatacgctctactggaaagctctgttcgaagaagccaacctcaacaacgtggttgctaagctgaatggagaggcggaaattttctttcgcagacactcgatcaaagcatccgacaaggtagtacacccggccaaccaggccatcgataataagaatccgcacacagaaaagactcagagcacctttgaatatgacttggtgaaagataaacgttacactcaggataagttcttcttccacgtacctatttctctgaacttcaaagctcagggtgttagcaaatttaacgacaaagtcaatggattcctgaagggaaacccggacgtaaatataatcggtatcgaccgtggtgagcggcatctgctgtacttcacggttgttaaccagaaaggcgaaatactggttcaggaatccctcaatacgttaatgtctgataagggccatgttaatgactaccagcagaaactggacaagaaggaacaagaacgtgacgccgcccggaagtcgtggacaacggttgagaacattaaggaacttaaagagggttacttgtcacacgtggtacacaaacttgcacacctgattatcaaatataacgctattgtatgcttagaagatttaaactttgggttcaaacgcggtaggttcaaagtcgagaaacaagtatatcagaagtttgagaaggctctcattgataaactgaattacctagtgttcaaagagaaagaactcggtgaagtaggacattatcttacggcgtatcagcttactgcacccttcgaatccttcaagaaactgggcaaacaatccggaatcttattctatgtaccggcagattatacctctaagattgatccgaccacaggctttgtgaatttcctcgatcttaggtatcagtcagttgagaaagcgaaacagctgttgagtgatttcaacgcgatccgcttcaacagtgtccagaactactttgaatttgagatcgattataagaaactgacgcctaaacgcaaagtgggtacgcaatccaagtgggtcatttgcacatatggagatgtacgttatcagaatcgccgaaatcagaaaggccactgggaaacagaagaagtgaacgtaacagagaagctgaaagcgctgttcgcgagcgattctaagacaacgacggtaattgactatgccaatgatgacaacctgatcgatgtaattctagaacaggataaagccagcttcttcaaggaactgctttggctgcttaagttaacgatgactttacgtcatagtaagatcaagagtgaggacgatttcatcctgtcgcctgttaagaatgagcagggcgagttctatgattctcgaaaggcaggagaagtgtggccgaaagatgccgatgccaatggagcgtaccacatcgcattgaaaggcctgtggaacttgcaacagatcaatcagtgggagaaggggaagaccctgaatctagcgataaagaatcaagattggttctcatttattcaagagaagccctaccaggaataa

SEQ ID NO: 734 - DNA, 3897 bp, Artificial Sequence
  Description of Artificial Sequence: Synthetic polynucleotide
atgactaagacatttgattctgaattctttaacctgtattcacttcagaagacagttaggtttgaattgaaaccagtgggcgagacggcttcattcgtagaagacttcaagaacgaaggcctgaaacgcgttgtgtcggaagatgaacgacgtgctgtagattatcagaaagtgaaagaaattattgatgattatcaccgtgatttcatagaagaatcacttaattacttccctgagcaggtgagcaaagacgcacttgaacaggcattccatttgtatcagaaactgaaagcggccaaagtggaagaacgggagaaagcgttaaaggagtgggaggcacttcagaagaaactgcgcgagaaggtcgttaaatgtttctcggactctaacaaagcacgcttctctcgcattgacaagaaagaactcatcaaagaagacctgatcaattggctggtggcgcagaatcgtgaggatgacatcccgactgttgaaacattcaacaactttacgacgtactttaccggatttcatgagaaccgaaagaacatatatagtaaagatgatcatgcgacagctatcagctttcgactgattcatgagaatctgcctaaattcttcgataatgttatctccttcaataaactgaaggaaggctttcccgaactaaagtttgataaagtaaaggaggatcttgaggtggactatgatctgaagcatgcgtttgagattgaatatttcgttaactttgtgacgcaagccggcatcgatcagtataattacctgctgggcggcaagactctggaggatggtaccaagaagcagggtatgaatgaacagattaacctgttcaagcaacagcagacacgggataaagcccgccagatcccgaagctgattccgctgtttaaacaaatcctctccgagcggaccgaatcacaatcgtttatcccgaagcaatttgagtctgatcaagaactgtttgattcattgcagaaacttcataataactgccaagacaaattcaccgtattacaacaagctattctcggtctggcggaggccgatttgaagaaagtctttatcaagacctctgatttgaacgctttatcaaacactatcttcggaaactacagcgtgttttccgacgctttgaatctctacaaagagagtctcaagacaaagaaggcccaagaggcgtttgagaagctgccggcacacagtatacatgatttgattcagtatctcgaacagttcaacagtagcctggacgccgagaagcagcaatccacggataccgtgctgaactacttcattaagacagatgaactgtatagtagatttatcaagagcacctcggaagccttcacgcaagtgcagccactgtttgaactcgaagccttaagtagtaaacgccgtccgccggagagcgaggatgagggtgccaaaggtcaggagggtttcgaacagattaagagaatcaaggcttatttagacaccctgatggaggctgtacacttcgcgaaaccactgtacctcgttaagggccgaaagatgattgagggtctagataaagaccagtcgttctatgaagcattcgaaatggcctatcaagaactggagtctctgatcatcccgatatacaacaaagcacgcagttacctctcccgtaagccgttcaaagcggacaaatttaagattaactttgataataatacattgctgtcgggttgggatgcgaataaggagaccgccaatgcctcgatcctctttaagaaagatggtctgtattacttagggatcatgccgaaagggaagacgttcctcttcgattactttgtaagcagcgaagactctgagaagctgaaacagcgtcgccagaagacagccgaagaagccctcgctcaagacggcgaaagctacttcgagaagattcgttataagttgctcccgggtgcaagcaagatgctgccgaaagtctttttctcaaataagaatataggtttctacaatccaagtgatgacattcttcgtatccgcaataccgcgtcacacactaagaatgggactccgcagaaaggccatagcaaagtggagttcaacctgaatgattgccataagatgattgatttcttcaagagctcaattcagaagcatcctgaatggggaagctttggatttacgttctcagacacctcggacttcgaagatatgagcgctttctaccgagaggtagagaatcagggctacgttatttcgttcgacaagataaaggaaacatatattcagtctcaggttgaacagggcaatctgtatctgtttcaaatttataataaggatttcagcccgtatagtaaagggaaaccgaatttacacacactgtattggaaagctctgtttgaggaggcgaacctgaacaacgtagttgccaaactcaatggagaggcagaaatattcttccggcgtcacagtattaaagcatcggataaagtcgtgcacccggcgaatcaggccattgacaacaagaacccgcataccgagaagacccaatcaaccttcgagtatgacttagtcaaagacaaacgatatacccaggataaattcttcttccatgtaccgatttctctgaacttcaaggcacaaggcgtaagcaaatttaatgacaaggtcaacggattcttgaaaggtaatccagatgtcaacattattggtatagaccgtggcgagcgacatctgttgtatttcacagtggtaaatcagaaaggcgagattctggtccaggaaagcttgaataccctgatgtcggataaaggtcatgtaaatgattatcagcagaaactggataagaaagagcaagaaagggatgccgcacgtaaatcctggaccaccgtcgagaacattaaagaacttaaggagggttatctgtcgcatgtggtccataagctggcgcatcttattatcaaatataatgccatagtgtgcctcgaagacctgaacttcggatttaaacgtggtaggttcaaagtcgagaaacaggtgtatcagaagtttgagaaagcactgattgataagctcaactatctcgtatttaaagagaaggaattaggcgaggtcggccactatctgaccgcataccagttaacggcaccatttgaaagcttcaagaaattgggcaagcagagtggcatcttgttctacgtgccggcggattacaccagcaagatcgaccctacaacaggcttcgtgaatttcctggatctgcgttatcaatctgtggagaaggctaaacaactgttaagtgacttcaacgccattcgctttaacagcgtgcagaactacttcgaattcgaaattgattataagaagttaacgccaaagcgcaaggtcggcacgcaatctaaatgggtcatttgtacttacggagatgtacgttaccagaatcgccgtaaccagaagggccactgggaaacagaagaagttaatgtcaccgagaagctgaaagcgttgttcgccagcgattctaagacgaccaccgttattgattacgcgaacgatgataatctgattgacgtaattctggaacaagataaagcctcattctttaaagagttactctggctgctgaaactcacaatgacgttacggcatagtaagatcaaatcggaagatgacttcatcttatctcctgtcaagaacgagcagggtgaattctacgattccaggaaagcgggtgaggtttggccgaaggacgccgatgcgaacggcgcgtaccatatcgcactgaaaggtttatggaatctgcagcagattaaccagtgggagaaaggtaagactctcaacctggccatcaagaatcaggattggtttagctttatccaggagaaaccgtaccaggaataa

SEQ ID NO: 735 - DNA, 3897 bp, Artificial Sequence
  Description of Artificial Sequence: Synthetic polynucleotide
atgacgaagacattcgattcggagttcttcaatctgtacagcctccagaagaccgtgcggttcgaacttaagccagtgggcgaaaccgcttcgttcgttgaagactttaagaatgaaggcctgaaacgtgtcgttagcgaggatgaaaggcgcgcggtggattatcagaaagttaaagaaattatcgatgattatcatagggatttcattgaagaatccctgaattatttccctgagcaggttagcaaagacgccctggaacaagcgttccacctgtatcagaagttgaaagctgcgaaagtcgaggaacgcgagaaggccttgaaggaatgggaagcacttcagaaaaaactgcgcgagaaggttgtgaaatgcttcagtgattctaacaaggcacgattcagtcgtattgacaagaaagaattgattaaagaagatctgataaattggctggtggctcagaatcgtgaagacgatattcctaccgtagaaaccttcaataacttcacaacatacttcacaggctttcatgagaacagaaagaatatttactcgaaggatgatcacgccactgcaattagctttcgcctgattcacgagaatctgccgaaattcttcgacaacgttatcagtttcaataagctgaaggaaggctttccggaactgaagtttgataaagtcaaggaagacttagaagttgactacgatctgaaacacgcctttgagattgaatacttcgtgaacttcgtcacgcaggccggcatcgatcaatacaattacctgttaggcgggaagacgctagaagacggcaccaagaaacagggcatgaatgaacagattaatttattcaaacaacaacagacgcgcgacaaagcaagacagatcccgaaacttattcctctgttcaaacaaattctgtctgagcggaccgaaagccagagctttatccctaaacaattcgaaagcgaccaagaactgttcgatagcctgcagaaattacataataactgccaagacaagtttacagtgttgcagcaagcgatcctgggcttggcggaggctgatctcaagaaagtctttatcaagacaagtgatctgaatgctctgagcaatacgatctttggaaactactcggtgttctctgatgcgcttaatctgtataaagaatcgctcaagactaagaaagcccaagaagccttcgagaagctgccggcgcactccatccacgatctcattcagtacttggaacagttcaatagtagtctggatgccgagaagcagcagtcaacggacaccgttcttaactacttcattaagactgacgagctgtatagtcgctttattaaatcaacgagtgaggcattcacgcaggtgcagccgttgtttgaactcgaggctctgagcagcaagaggcggccaccggagtcagaagatgagggcgcgaaaggccaagaagggtttgaacaaattaagcgtattaaagcgtatctggatactctgatggaagccgtgcactttgctaaaccgctgtacctggtgaaaggccgaaagatgattgaagggctggataaagatcagagtttctatgaagcgttcgaaatggcgtatcaggaactggaaagtttaatcattccgatatacaacaaagcacggagctacctgtctcgtaagccatttaaagcagacaaatttaagattaactttgataataacacgttactatctggctgggatgccaacaaggaaactgcaaatgccagtatactgttcaagaaagatgggctttattacctgggcattatgcctaaagggaagacattcctattcgattacttcgtgagctcggaggatagcgagaaactaaagcagcgccgtcagaagaccgctgaagaagccttagcgcaggacggcgaatcgtacttcgaaaagattcggtataaactgctgccgggcgcctcaaagatgctgcccaaggtattcttcagtaacaagaacataggtttctacaatccatctgatgatattctccggattcgcaacacggctagtcacacaaagaatggtactccacagaagggccacagcaaagtcgagttcaatctgaatgactgtcataagatgattgacttctttaaatcctccatacagaagcacccggaatgggggagctttggcttcacctttagcgataccagtgatttcgaagatatgagtgcattctatcgtgaggttgagaaccagggctacgtcatcagtttcgataagattaaagaaacttacattcagtcgcaggttgagcagggcaacctgtatttgttccagatttataataaagatttctcgccgtacagcaagggcaagcctaaccttcatacactctactggaaggccctgtttgaagaagcaaatttgaacaacgttgttgcgaagctgaacggcgaagccgaaatattctttagaagacatagcataaaggccagcgataaagtggtgcacccggctaaccaggcgattgacaataagaacccgcatactgagaagactcaatccacctttgaatacgatctcgtcaaggataagcgctatactcaagataagttcttcttccatgtcccaattagcttaaactttaaagcgcagggcgtttctaaattcaacgataaagtgaatggctttctgaaaggtaatccggacgtgaacattatcgggatcgatcgcggagaacgtcacctgttgtactttactgttgtaaatcagaagggcgagatattagttcaggagtctcttaatactttgatgtcggacaaaggtcacgtcaatgattatcagcagaaactggataagaaagaacaagagcgtgatgccgctcgtaagtcatggaccacggtcgagaatattaaagaactgaaagaaggctatctgtcccacgtcgtgcataaactggcgcacctgataatcaaatacaatgccatagtttgtctggaagatctgaacttcggctttaagagaggacgcttcaaagttgagaaacaggtgtaccagaaattcgagaaggccctgatcgataaactgaattatctggtcttcaaagagaaggaattgggcgaagttggtcattacttgactgcctaccagctgacagcgccgttcgagtcgttcaagaaactaggcaaacaaagcggaatacttttctacgtacctgctgattacacctcgaagattgacccgacaactggtttcgtgaactttctggatttacgctatcagtctgtggagaaggccaagcaactgttaagcgacttcaatgccattcgcttcaacagtgtacagaattactttgagttcgaaatcgactataagaaactgacgcctaaacgtaaggtcggcacgcagtccaaatgggtgatctgtacgtatggtgatgtacgctatcagaaccgccgtaatcagaaaggtcactgggaaaccgaagaggtcaacgtgaccgagaagttgaaagccttattcgcttctgattccaagacgaccacggtgattgactatgcaaacgacgataacctgatagacgttatcctcgagcaagacaaagcgtctttcttcaaagaactgctgtggctcctgaagcttaccatgaccctgcgccacagtaagatcaaatcagaagacgatttcatcctatcgccggtgaagaacgagcagggcgaattctatgattcgagaaaggcaggagaggtgtggccgaaagacgccgatgccaatggcgcatatcatattgccctgaagggtctgtggaacttacagcaaattaatcagtgggagaagggtaagaccctcaatctggccattaagaaccaggactggttttccttcattcaggagaagccataccaggagtag

SEQ ID NO: 736 - DNA, 3897 bp, Artificial Sequence
  Description of Artificial Sequence: Synthetic polynucleotide
atgactaagacgttcgactctgagttctttaacctttattcactacagaagacagtgaggtttgagctcaaaccagtgggtgaaacagcgagtttcgtggaagacttcaagaacgaagggctcaaacgcgtggtaagtgaagacgaacgccgggcggtggattatcagaaggtaaaggagattattgatgactatcatcgtgatttcattgaggaatcactgaactactttcctgaacaggtgtcaaaggatgcactggaacaggcgtttcatctttatcagaaactgaaggctgctaaggttgaagagcgggagaaagcactaaaggaatgggaagcactgcagaagaagctgcgtgagaaggtcgtgaaatgcttcagcgactccaacaaggccaggttctctcgcatcgacaagaaagaactaatcaaggaagatctgatcaattggctcgtcgcacagaaccgcgaagatgatattccgaccgtagagacctttaataacttcaccacctacttcaccggcttccatgagaatcggaagaacatatattcgaaagatgatcatgcgacggccatttcgtttcggctgattcacgagaacctgcccaagttctttgacaacgttatttctttcaacaaattgaaggaaggcttccctgagcttaagtttgataaggtaaaggaagacctcgaagtcgattatgatctgaaacacgccttcgaaatcgaatatttcgttaacttcgtcacacaggccggtatcgatcagtataattatctgcttggtggcaagacactagaggatgggaccaagaagcaaggtatgaacgaacagattaatctgtttaaacaacagcagacgcgcgataaagcaagacagatccctaaactgattccgttattcaaacagatactgagcgagcgcaccgagagccagtcgtttatcccgaagcaattcgaatccgaccaggaattgttcgatagtctccagaaattacacaataactgccaagataaattcaccgtactgcagcaagcgattcttggcttggcggaagcggatctcaagaaagtctttattaagaccagcgatctcaacgcgttatcgaataccatcttcgggaattatagcgtgttcagcgatgccttaaatttatataaagaatcattaaagactaagaaagctcaagaggcgttcgagaagctgccggcgcacagtatacacgatctgatacaatacctggagcagtttaatagttctctggatgcggagaagcagcagtctaccgatactgttctgaattatttcattaagaccgacgagctgtattctcgtttcattaagtcaacgtcagaagcattcacccaagtgcaacctctgttcgaacttgaagctctgagctcgaagcggcgcccgcccgaatctgaagacgaaggagcgaaaggacaggaaggctttgagcaaatcaaacgtattaaagcatacctggatacccttatggaggcggtacactttgcgaagccgctctacttagtcaaaggccgcaagatgatagagggtctggataaggatcagagcttctacgaagcgttcgaaatggcctatcaggaattagaatctctgatcatcccaatttataacaaggcgcgctcatatctgtcacgtaaaccatttaaagcagacaaatttaagatcaatttcgataataacaccttactgtcgggctgggacgccaacaaagaaaccgccaatgcatcgatcctgttcaagaaagatggcctgtactacctcgggatcatgcctaaggggaagacgttcttattcgattactttgtatctagcgaggattcggagaaactcaagcagcgccgtcaaaagacagccgaagaggcccttgcgcaggatggcgaatcgtactttgagaagatccgctacaaactgcttccgggtgcaagtaagatgctgcccaaggtattcttcagcaataagaacatcggtttctataacccttctgacgatatcctgcgtattagaaacactgccagccacaccaagaacggcacgccgcagaagggtcattcgaaagtagaatttaatctcaatgactgtcacaagatgattgacttcttcaagagctcgatacagaagcatcctgaatggggatctttcggctttacattctcagacacttcagacttcgaggacatgtctgccttctaccgagaggtcgagaaccagggatatgttataagcttcgataagattaaggaaacctatatccagtctcaagtggagcagggcaatctctatctcttccaaatttataataaagactttagcccgtatagcaaaggcaaaccgaacttgcacaccctgtactggaaagccttattcgaggaggctaaccttaacaacgtggtcgccaaactgaacggagaagctgagatattcttccgccgccatagtattaaagcttcagataaagtggtccatcctgcgaaccaggcgattgacaataagaacccgcacacagagaagacgcagagcacgttcgaatatgatctggtgaaggataaacgctatacacaagataaattcttcttccatgtccctatctctctgaacttcaaagcacagggcgtgagtaaattcaacgataaagtcaacggtttcttaaagggtaatccggatgttaatataattggtattgaccgtggcgaacgccatctgctctacttcaccgtggtgaatcagaaaggcgaaattctggttcaggaaagtctcaacacactgatgtcggataaaggtcacgtgaatgattatcaacagaaactggataagaaagaacaggaacgcgatgctgcacgaaagagctggacgactgtcgagaacatcaaggagcttaaggaaggctatttgagccatgtcgtgcacaaattggcgcatttgattatcaagtacaatgcaatcgtgtgtctggaggatctgaactttggcttcaaacgcggtcgcttcaaagtcgagaaacaggtctaccagaaattcgagaaggctttaattgacaaactcaactacttagtgtttaaagagaaagaactaggtgaagtaggtcattacctgaccgcataccagttaacagcgccgtttgagagttttaagaaactcggcaagcaatcgggcatccttttctacgtccctgcagattatacgagtaagattgaccctacgactggcttcgttaatttcctcgacttacgctaccagagcgtggagaaggcgaaacagctcctaagcgactttaatgcgatacgtttcaattctgtgcagaactatttcgaatttgaaatcgattataagaagttgacaccgaagcgcaaagttggcacccagtctaaatgggttatttgcacatatggtgacgtcagatatcagaaccgccgcaaccagaaaggccattgggaaaccgaagaagtcaacgtaactgagaaattaaaggccctgttcgcatcagattcgaagacgaccaccgttatcgattatgctaacgacgataacctgatagacgtcattctggaacaggacaaagcttcgttcttcaaagaactgttgtggcttctgaaactgactatgaccctgcgtcactctaagataaagagtgaggatgacttcatacttagtccggttaagaatgaacagggcgagttctatgactcacgtaaagcaggcgaagtgtggcctaaggatgccgacgccaatggagcctatcacattgcgctgaagggcctttggaacctgcagcaaattaaccagtgggagaaggggaagactttaaacctggccattaagaaccaagattggttctcatttattcaggagaaaccgtaccaagaataa

SEQ ID NO: 737 - DNA, 3897 bp, Artificial Sequence
  Description of Artificial Sequence: Synthetic polynucleotide
atgacgaagacgtttgatagcgaattctttaatctgtactccttgcaaaagaccgtgagattcgaacttaaaccggtaggcgaaacggccagcttcgtggaggacttcaagaatgaagggttgaaacgggtagtttctgaggatgaacgtcgtgccgttgattatcagaaagtcaaagagatcatcgatgactatcatcgtgactttattgaagaatccctcaactatttcccggagcaagtgtctaaagatgcccttgaacaggccttccacttataccagaagcttaaagcggccaaagtggaagaacgtgagaaggcattaaaggagtgggaagcattgcagaagaagctgcgggagaaagttgtcaaatgtttcagcgattcgaacaaagcccgcttcagccgcatcgacaagaaagaattgattaaagaagacctgatcaattggcttgtggcgcagaatcgcgaagatgacattccaactgtagaaacctttaacaactttaccacttacttcactggcttccatgagaacagaaagaacatttactccaaagatgatcacgccaccgccataagcttccgtctgatccatgagaacctgccgaaattcttcgataatgttatcagctttaacaaattgaaagaaggcttcccagagctgaaatttgataaagtcaaggaagacctggaagtagattatgacctcaaacatgctttcgaaattgagtactttgtaaacttcgttactcaagcaggaattgatcaatataattacctgctgggtgggaagaccttggaggatggtactaagaaacaaggtatgaatgagcagatcaatttgttcaagcagcaacagacccgagataaggcgcgccagattccgaaactgatcccgttattcaaacagattctgtcagagcggactgaatctcagtcattcatcccgaaacaattcgaaagcgaccaggagctgttcgacagtttacagaagttacacaacaactgccaagacaaatttactgtcctacaacaggccatcttgggtttggccgaggccgacttaaagaaagtattcataaagactagcgaccttaacgctctgagcaacaccatcttcggaaattatagtgttttctcagatgcccttaatctgtataaagaatcgttgaagaccaagaaagcgcaggaggcatttgagaagctgccggctcatagcattcacgatctgatccagtacctggaacagttcaatagcagcttagatgcagagaagcagcaatctacagatacagtgttaaactactttattaagaccgatgaattgtattcccgctttattaaatcaacgtcggaagccttcacccaagtccaaccgctgtttgagttagaagcgctgtcaagcaaacgtcgtccgccagaatcagaagatgagggcgctaaggggcaggagggcttcgaacagattaaacgcattaaagcctacctagataccctgatggaagcagttcactttgcgaagccgttgtatttagttaaaggtaggaagatgatcgaaggtttagacaaagatcagtctttctatgaagcgtttgagatggcctatcaagaattagaatccctcattattccgatttacaacaaggcacgcagctacctgagtcgcaagccattcaaagcagacaaatttaagatcaacttcgataataacacattgctgtctggttgggatgcaaataaggaaacggcaaacgcgtctattctgtttaagaaagatgggttgtattatctgggtattatgccgaaaggcaagaccttcctgtttgattatttcgtgtctagcgaggacagtgagaagctcaagcagcggagacagaagactgcagaagaagctctcgcacaggatggcgaatcgtacttcgagaagatccgttacaagctgctgccgggagcgagcaagatgctgcccaaggtctttttctctaacaagaacatcggtttctataacccgagtgacgatatacttagaattcgcaacacagccagtcataccaagaacggtactccgcagaaggggcacagcaaggttgaatttaatttgaacgactgccacaagatgattgatttcttcaagagctccattcagaaacacccggaatggggttcatttggctttacgttctctgatacatctgatttcgaagacatgtccgcgttctatcgggaagtggagaatcaaggttacgttatctctttcgacaagattaaggaaacctacattcaatcgcaggtcgagcaaggtaatctgtatctctttcagatctataataaggacttcagcccatactccaaagggaagccgaatctgcataccctatattggaaagctttatttgaagaagcaaacctgaacaacgttgtagccaagctgaacggcgaggctgaaatattttttcgcagacattcgattaaagcttcggacaaagttgttcatccagccaaccaagccatcgataataagaacccgcacactgagaagacccagtctacatttgaatacgatcttgttaaagataaacgctatacgcaggataagttcttctttcacgttccgatttctctgaacttcaaggctcagggcgtcagtaagtttaacgataaggtgaatggtttccttaagggcaatcccgatgttaatattatcggtattgatcgtggggagcggcatctgctctatttcaccgtggtgaaccagaaaggtgagatcctggttcaggagtcactgaatacgctcatgtcagataaaggccatgtgaacgattatcaacagaagcttgacaagaaagaacaggagcgcgatgcggctcgtaaatcgtggacgaccgtggagaatatcaaagaactcaaggaagggtacctgagccacgtggtgcacaagttggcgcatctgatcatcaagtataacgccattgtgtgcttggaggatcttaacttcggattcaaacgtgggcggtttaaagttgagaagcaggtgtatcagaaattcgagaaggccctgattgataaattaaattacctggtcttcaaagagaaggaattaggagaagttggacattacctgacggcatatcaacttaccgctccgtttgagagcttcaagaaactaggcaaacagtcaggaatcctgttctatgtgccggccgattataccagcaagattgatccgacaacaggcttcgtgaactttcttgatctccggtatcagtcagtggagaaagcaaagcagctgttgagtgacttcaacgcgattcgtttcaacagtgttcagaattacttcgaatttgaaattgattataagaaactgactcctaagcgcaaagttggtacacaaagcaaatgggtgatctgtacctatggtgacgtacgttaccagaaccgccgcaatcagaaaggccattgggaaacggaagaagtcaatgtgacagagaagctcaaagccctctttgcatcggactccaagacgacaaccgttattgactatgcgaatgatgataatttgatcgatgtgattctggaacaagataaagcgagtttctttaaggagttattgtggcttcttaaactaaccatgaccctgcgacacagcaagatcaagagcgaagacgacttcattctgtcaccagtgaagaacgaacagggagaattctacgatagccgtaaggcaggtgaggtgtggcccaaagatgccgatgccaacggtgcataccatattgcgcttaaaggtctctggaatctgcaacagatcaatcagtgggagaagggcaagaccctcaaccttgcgattaagaaccaggattggttctctttcatccaagagaagccgtaccaagaatga

SEQ ID NO: 738 - DNA, 3897 bp, Artificial Sequence
  Description of Artificial Sequence: Synthetic polynucleotide
atgactaagacctttgattcagagttcttcaatctgtacagtctacagaaaacagtccgattcgaactgaaaccggttggtgagaccgcaagcttcgtggaagattttaagaacgaaggtctgaagcgtgtcgtgtcggaggacgagcgccgtgcagtagattatcagaaagtgaaagaaataatcgatgattaccatcgtgacttcattgaagaaagtctgaactactttcctgaacaggtgagtaaggatgcactggagcaggcatttcatctttatcagaagctgaaagcggcgaaggtggaggagcgtgagaaagcactgaaagagtgggaagcgttacaaaagaagctgcgtgagaaagttgtgaaatgctttagtgacagcaacaaagctcggtttagtcgcatcgataagaaagagctgattaaagaagatctgatcaactggctggtggcccagaaccgggaagatgatataccaaccgtggaaacgtttaataactttaccacgtacttcaccggctttcacgagaaccggaagaacatttattccaaggatgatcatgctacggcaatttcctttagacttatacatgagaacctccctaaattcttcgataatgtcatcagctttaataagctgaaagaaggattcccggaacttaaattcgataaagttaaagaggatctggaagtcgattatgatctgaagcatgccttcgaaatcgaatacttcgttaatttcgtcacacaggctggaatcgaccagtataactacctgttaggcggcaagactctggaagacggtacgaagaaacagggtatgaacgaacaaattaacttgttcaaacaacagcagactcgtgataaggcccgccaaattcccaaattgattcccttgtttaagcagatattgtcagaacgcacggagtcgcagagcttcatcccgaaacagtttgaatctgaccaggaactgttcgactctctgcagaaattgcataataactgccaagacaaatttactgtacttcaacaagcaatcttgggcctggcagaagcggaccttaagaaggtattcatcaagacaagcgatttgaatgcgttgtcgaacacgatattcgggaactatagcgttttctccgacgcccttaacctctataaagaatcactgaagaccaagaaagcgcaagaggcgtttgagaagctgccggctcactctattcatgatctgattcagtacctggagcagtttaactcgagcctggatgcggagaagcagcagtctactgatacggtgcttaattatttcatcaagacagatgagctctatagccgctttattaaatcgaccagtgaagcgttcacccaggtccagccactgtttgaactcgaggccctgtcatcgaagagacgtcctccagagtccgaagatgagggagccaaaggccaagaagggtttgagcagattaagcgtattaaagcctacctggacaccttgatggaagcggtgcatttcgctaagccgctgtatttagtcaagggtcgcaagatgatcgaaggtctggacaaagatcagagtttctacgaagcctttgagatggcttatcaagaactggaatccttgatcatcccgatctataacaaagcgagaagctatctgtcacggaaaccatttaaggccgataaattcaagatcaacttcgataacaacacactgctctcgggttgggatgctaacaaagaaacggctaatgcgtctatcctgtttaagaaggatggcttgtattacttagggataatgcccaaaggcaagacattcctgtttgactactttgtctctagcgaagatagtgagaagctgaaacagcgtcgccagaagacagccgaagaggcacttgcacaggatggtgaaagttatttcgagaagattcgctataaattactgcccggcgcttcgaagatgctcccgaaggtgtttttctcaaacaagaacattggtttctataatccgtcggatgacatcttacggattcgcaatactgcttctcatacgaagaatgggactcctcagaagggtcatagcaaggttgagtttaatcttaatgattgccacaagatgatcgacttctttaagtcatccatccagaagcacccggaatgggggagtttcggctttactttctcggatacctcggacttcgaagatatgtctgcgttctatcgcgaagttgagaaccaagggtatgtgatctcatttgataagattaaagaaacgtacattcaatcacaggtggaacaaggtaatttatatctgttccaaatctacaacaaggatttcagcccgtactcgaaagggaaaccgaacctgcacacgctgtactggaaggctctgtttgaggaggcaaacctgaacaacgttgtggcgaaactaaacggtgaggcagaaatcttttttcgccgtcatagtattaaagcgtcggataaagtggtgcatccagccaatcaggccattgacaataagaacccgcatacagaaaagacccaatcaacattcgaatacgatctggtcaaagacaaacggtacacccaggataagttcttctttcacgttccaatctctctgaatttcaaagcccaaggcgttagtaaatttaacgacaaagttaatggatttctgaaaggcaacccagacgtaaatattattggtattgatcgcggagaacggcatctgttgtacttcactgtggtaaaccagaagggagaaatcctggttcaggagtcattaaatacccttatgagtgacaaaggccatgtaaacgattaccaacagaagctggacaagaaagagcaggaacgtgatgccgcgaggaagagctggaccaccgtagagaacattaaagaattgaaagagggctacctttcccacgttgtccacaagttagctcacctcatcattaaatacaacgcaattgtgtgtctggaggacctaaacttcggctttaaacgcgggcgtttcaaagtcgagaaacaggtatatcagaagtttgagaaagccttaattgacaaactaaattatctggtatttaaagagaaggaattgggagaagttgggcattatcttaccgcttatcagctgactgctcctttcgagagcttcaagaaacttggtaaacagagcgggatattgttctacgtgccggcagattacacttctaagattgacccgaccacaggcttcgtgaacttccttgacctgcgctaccagagcgtcgagaaagctaagcaactgttatcggatttcaatgctattcgctttaactctgtgcagaattacttcgaattcgaaattgattacaagaagcttacgccaaagcgtaaagttggtacacagtctaagtgggtaatctgcacctatggcgacgtgcgttaccagaatcgccggaaccagaaaggccattgggagactgaagaagtgaatgttacagagaaactcaaggccctgtttgcaagcgatagtaagacaacgacggtaatagactatgcgaacgatgataatttgatcgatgtgatactcgaacaagataaggcgtctttctttaaagaactcttatggctcctgaaactgacaatgaccctgaggcattcgaagattaaatctgaagacgacttcatcctgtcgcctgtaaagaatgaacagggtgaattctatgattcacggaaagccggtgaggtgtggcctaaggatgcggatgcaaacggtgcgtaccatattgcattgaagggactgtggaacctccaacaaattaatcagtgggagaagggaaagaccctgaatttggcaatcaagaaccaggattggttctcattcatccaggagaaaccttatcaggagtaa

SEQ ID NO: 739 - DNA, 3897 bp, Artificial Sequence
  Description of Artificial Sequence: Synthetic polynucleotide
atgacaaagacctttgatagtgagttctttaacctgtacagcttacagaagaccgtacgattcgaattgaagccggtcggcgaaactgcctctttcgtggaagacttcaagaatgagggcctgaaacgtgtggtctcggaagatgaacgtcgagcggtggattatcagaaggtgaaggagattatcgacgattatcatcgtgacttcattgaggaatctcttaattacttcccggaacaggttagcaaagacgccctggagcaggcctttcatctgtatcagaaactcaaggcagcgaaagttgaggagcgtgagaaagccttgaaagaatgggaagcactgcaaaagaaactgcgggagaaagtagtgaaatgcttctccgattctaacaaagcacgcttctcacggatcgacaagaaagaactgattaaagaagatctgatcaactggcttgtggctcagaatcgtgaagacgatataccaacggtagaaacctttaacaactttactacctacttcacgggctttcatgagaatcgcaagaatatttacagcaaagatgatcacgcgactgctatttcctttcgtttaatacacgagaacctgccgaagttctttgacaatgtgatcagtttcaataagctgaaagagggattccctgaacttaagttcgataaagtcaaggaagaccttgaagtcgattatgatcttaagcatgcattcgaaatcgaatatttcgttaacttcgtcacccaggccggcattgaccaatataattatctcctgggcgggaagactttagaggatggaacaaagaagcagggtatgaacgagcagatcaacttgttcaaacagcagcagacccgtgacaaagcccgccaaattcctaagctgatcccattgttcaaacagattctttcagaacgtacggaaagccagtccttcattcccaaacagtttgaatccgatcaggaactgtttgactctctgcagaagctgcataacaactgtcaggacaaatttactgtgttgcagcaggctattctgggcttggctgaagctgacctcaagaaagtcttcattaagacatccgacttgaacgcgctgagtaatactatatttggtaactatagcgtcttctctgatgcactcaacttatataaggaaagcctcaagacgaagaaggcgcaggaagcgttcgagaaattgccggctcactctatccatgatctcattcagtacttagaacagtttaacagcagcctggacgcggagaagcaacaatccactgatactgtgctgaactatttcattaagacggacgaactttattctagatttattaagagcacgtcggaagctttcacgcaagtgcagcctctctttgagctggaagcgctgtcttctaagagacggccaccggaaagcgaagatgaaggtgcaaagggccaagaaggcttcgagcagattaaacgcattaaggcctatttggataccctgatggaagcggtccacttcgccaaaccgctgtatttggttaaaggacgaaagatgatagaaggtttagataaagaccagagtttctatgaagcgttcgagatggcgtaccaggaactagaaagtcttatcatcccaatttataataaagctcgctcatatctgagtcgcaaaccctttaaagccgataaatttaagattaacttcgacaataataccctcctgtcgggctgggatgcgaataaagaaacagcaaatgcgtcaatcttattcaagaaagatggcctgtattaccttggcatcatgccgaagggcaagactttcttgtttgattatttcgtgtcgagcgaggactccgagaaacttaagcagcgcagacagaagactgcagaagaagccttagcacaagacggcgaatcgtacttcgagaagatacgttacaagctgcttccaggcgcttctaagatgttaccgaaagtatttttcagcaacaagaacattggcttctacaacccttctgatgatattctacgtattcggaatactgcaagtcacaccaagaacggcactccgcagaaagggcatagtaaagtcgaatttaacctgaacgactgtcataagatgatcgatttcttcaaatctagtatccagaaacacccggagtggggttcatttggatttacattctcggatacctctgacttcgaagatatgagtgccttctaccgcgaagtggagaaccagggctatgtgatttcattcgataagatcaaagaaacctatatccagtcacaagttgagcagggtaacctttatctgttccaaatttacaataaggatttctcaccgtattcgaaaggtaaacccaacctgcatacgctttactggaaagctttatttgaggaagctaatttaaacaatgtggtggccaaactgaatggcgaagcagaaatattttttagacgtcattcaatcaaagcgtctgacaaagtggtgcatcctgcaaatcaggcgatagataacaagaacccgcatacggagaagacccaaagtacctttgaatatgacttggtcaaagataagcgttatactcaagataagtttttctttcacgtgccgatttctctgaatttcaaagcgcagggtgttagtaaattcaacgataaggtcaatggatttcttaaaggcaacccggatgtgaatattattggtattgatcgcggagagcgtcatctcctgtatttcacggtcgttaatcagaagggcgaaattctggtccaggagtccctgaacaccctgatgagtgataaaggccacgtcaacgattaccagcagaagttagacaagaaagaacaagaacgggacgccgctcgtaaatcctggaccacggtagagaatattaaagaactgaaagagggatatctgtcacatgtagtgcacaaactggcgcatctcataatcaaatataatgcaatcgtctgcctggaggatctgaacttcggcttcaaacgaggcagatttaaggttgagaaacaggtctatcagaaatttgagaaggcattgattgacaagctgaactatttggtgttcaaggagaaggagctgggcgaggtgggccattacctgacagcttaccagctgacggcgccttttgaatcgttcaagaaactcggtaaacaatctgggatcctattctatgtgccggctgattatacctcgaagatcgacccgaccactgggtttgttaactttctggacctgcgttatcagagtgtggagaaagcgaaacagctgctgtctgacttcaacgccattcgcttcaatagcgtgcagaactatttcgagttcgaaatcgattataagaaactcactcctaagcgcaaagttggaacgcagtcgaaatgggtaatttgcacgtacggtgacgtacgttatcagaatcgcaggaatcagaaaggacattgggaaaccgaagaggttaatgttaccgagaagttaaaggccctgtttgccagcgacagtaagaccacgaccgtaattgactacgcgaacgatgataatctgatagacgttattctcgaacaggacaaggcatcattctttaaagaattattatggttacttaaacttaccatgaccttgcgccattcaaagatcaagagtgaagatgactttatactgagccctgttaagaatgaacaaggagagttctacgactctcgaaaggccggcgaagtgtggccgaaagacgccgatgccaatggagcctaccacatcgcgcttaagggtctttggaacctgcagcagattaatcagtgggagaaagggaagaccctgaatttggcgatcaagaaccaggattggttcagctttattcaggagaagccgtatcaggaataa

SEQ ID NO: 740 - DNA, 3897 bp, Artificial Sequence
  Description of Artificial Sequence: Synthetic polynucleotide
atgacgaagaccttcgatagtgagttcttcaatttatacagcctccaaaagacggtgaggttcgaactcaagccggttggcgaaaccgcgtcgtttgtcgaagattttaagaacgaaggtctaaagagggtcgtgtcggaagatgagcgccgagctgttgattatcagaaggtcaaagagatcattgacgattaccaccgcgacttcatcgaagaaagcttgaactatttcccggaacaggttagcaaggacgcattagagcaggcatttcatctgtaccagaagctgaaggccgcaaaggtcgaggaacgggagaaggcgctgaaagaatgggaagcgctgcagaaaaagcttagggagaaggttgtgaaatgtttcagtgactctaataaagcacggttctctcgaatagacaagaaggagctgataaaggaagatctcatcaattggcttgtcgcgcagaatcgtgaggatgacattccgacagtagaaacatttaacaatttcaccacgtacttcacgggctttcacgagaatcgtaagaatatttactcgaaagacgaccatgccactgcaattagctttcgactgattcacgagaacctcccgaagttctttgataacgttatctcgttcaataagctgaaagagggctttccagaactgaaattcgataaagtgaaagaagatctggaagtggattatgacctgaaacacgcatttgagatcgaatacttcgtaaacttcgtaacgcaggcgggcattgaccagtacaattatcttctgggtggtaagacgctggaagacggtacgaagaaacagggtatgaatgaacaaattaacctgttcaaacaacaacagacccgggataaagcgaggcaaatcccgaaacttattccgctattcaagcagattctgtcagaacgtacagagtcgcagtcattcattccgaaacagtttgaaagtgatcaagagttgtttgattcattacagaagttgcacaataattgccaggacaaattcaccgtcctgcaacaagcaattctgggcttagccgaggcagatcttaagaaggtgtttatcaagacgagcgatctaaatgccctatctaataccatctttgggaattattcggtgttctctgacgcgctgaatctgtataaagaaagtttgaagacgaagaaagcacaggaagccttcgagaagctgccggcgcattcaatccatgatttaatacaatacctggaacagtttaactcatcgctggatgctgagaagcagcagtccactgacactgtcctgaattacttcataaagactgacgaattgtattctcgtttcattaaatctaccagcgaagccttcacgcaggttcagccgttgtttgagttggaagcactgagttcgaaacgtcggcctccggaaagcgaagatgaaggcgcaaagggacaggagggctttgagcaaattaaacgcattaaagcctacctggacacactgatggaggcagtgcactttgcgaagccactgtacctggttaaagggagaaagatgattgagggcctggataaggaccaatcgttctatgaagcattcgaaatggcgtaccaagaactagagtctttgatcataccgatttacaacaaagcccgtagctatctgtcgcgtaaaccctttaaagccgataagtttaagatcaatttcgacaataacaccctactttccggctgggatgctaacaaagagacagccaacgcgagtattctgtttaagaaggatgggctgtattacttgggcattatgcccaaaggcaagaccttcctgtttgattacttcgtcagctctgaagacagcgagaagctgaagcagcgccgccagaagacagcagaagaagctctggcgcaagacggcgaatcgtacttcgagaagatccgctataaactgctgccgggtgcatccaagatgctgccgaaagtattttttagcaacaagaacattggtttctacaatccgtcagacgatatcttacgcatccgcaacactgcctcccacactaagaatggcacaccgcagaagggtcatagcaaggtcgaatttaatctgaatgactgtcataagatgatcgacttctttaagagttcgatccagaagcatccggaatgggggtcatttggcttcacctttagcgatacatcggactttgaggacatgagcgcgttctatcgcgaagtagagaaccaaggttatgttatttctttcgataagatcaaggaaacctatatccaaagccaggtggagcagggcaacctctacctctttcagatctacaataaagatttcagcccgtatagcaagggcaaaccgaatttacatacactgtattggaaggctctcttcgaggaagcgaatttaaacaacgtcgtggcgaagcttaacggcgaagccgaaatcttcttccgtcgtcatagtattaaagcatcggataaggtagtgcatccggcaaaccaagcgatcgacaacaagaacccgcatacggagaagacccaatccacattcgagtatgatctggtcaaagataaacgatacacgcaggacaagttcttcttccacgtaccgatcagtctgaatttcaaagcgcagggcgtgagcaaatttaacgataaagtgaatggcttcctgaaaggtaacccagatgtgaacataataggaattgaccgtggtgaacgccacctgctgtactttaccgtcgttaatcagaaaggcgagattctggtccaggaatctctgaacacgctgatgagtgataagggccatgttaacgactaccagcagaagttagacaagaaagaacaggagcgggacgccgcgcgtaagtcatggaccacggtcgagaatattaaagaactgaaagaaggctatttgtcgcatgttgtgcataaactggcccacttgattattaaatacaatgccattgtgtgtttagaagatcttaacttcggatttaaacgtggccgctttaaggtcgagaagcaagtttatcagaagtttgagaaggctctcatcgataaactgaactatctggtctttaaagagaaggagttaggtgaagttgggcactatctgacggcctatcagctgaccgcaccattcgagtcatttaagaagttaggtaaacagagcggcatcttgttctatgttcctgcagattatacatctaagatcgatccaacgaccggctttgttaatttcctggacctgcgttatcaatctgtcgagaaagctaagcaactgctgagtgactttaacgctatccgctttaactcggttcagaactatttcgaatttgaaattgactacaagaaactgactccgaaacgcaaggttggcacgcagtcgaaatgggtcatttgcacttatggagacgttcgctatcagaatcggcgaaaccagaaaggccattgggaaactgaagaagttaatgttacggagaagttgaaagcactattcgcatctgatagtaagacaaccaccgtaattgactacgcaaacgacgacaacctaattgacgtgatcttggaacaagacaaagcgagcttcttcaaagagcttctgtggctactaaagctcacgatgacattacggcattcgaagattaaatcggaagatgatttcattctcagcccggttaagaacgaacagggcgagttctatgattcacggaaagctggagaagtttggcctaaggacgccgacgccaacggcgcttatcatattgcgcttaagggcctgtggaacttacagcagatcaatcagtgggagaaaggcaagacacttaacctggcgattaagaaccaagattggttctcgttcattcaggagaagccgtaccaggaataa

SEQ ID NO: 741 - DNA, 3897 bp, Artificial Sequence
  Description of Artificial Sequence: Synthetic polynucleotide
atgacaaagacatttgacagcgaattctttaacctgtattctctgcagaagacggtacgcttcgagctgaagcctgtgggcgaaactgcttctttcgtcgaggatttcaagaacgagggtctgaaacgggtggtttcggaagatgaacgtcgagcggtggattatcagaaagttaaagagatcattgacgactaccaccgtgacttcatcgaggaatcactgaattacttcccggagcaggtctccaaggatgcgctagagcaggcctttcatctgtatcagaagctgaaagccgctaaggtcgaggagagagagaaggcccttaaggagtgggaagctctgcagaagaaactcagagagaaagtggtcaaatgtttctcagatagcaataaagcccgcttcagtcgtatcgacaagaaagaactgatcaaagaggatctgattaattggctggtggcgcagaatcgtgaggatgacattcctaccgtggaaactttcaacaacttcactacatacttcaccggtttccatgagaatcgcaagaacatttatagcaaagatgatcacgcgaccgcaatttctttccgtctgattcacgagaacctacctaagttctttgataatgttattagctttaataaactgaaagagggtttcccagaactcaagtttgataaagtgaaagaagatttagaagtagactacgatctcaaacatgccttcgagatcgagtacttcgttaatttcgttacccaggcaggcattgaccaatataactatctgctgggcgggaagacgctggaagacggcaccaagaagcagggtatgaatgaacagatcaatttgtttaagcaacagcagacccgtgacaaggcacgccagatacccaaattgatcccgctattcaaacagattctgtctgaacggaccgagtcccagagcttcatacctaagcaattcgaatctgaccaagaattatttgacagtctgcagaagctccataataattgccaagacaaatttaccgttctgcaacaggccattctcggcttggccgaagccgacctgaagaaagtcttcattaagacctcggatctgaacgcgctgagcaacacaatatttggaaattattcagtcttcagcgatgccctgaacctgtacaaggaaagtttgaagaccaagaaggcccaagaagcattcgagaaactgcccgcgcattctatacacgacttgattcagtaccttgagcagtttaattctagtttggatgcagagaagcagcagtctaccgacactgttctgaactactttataaagactgatgaactttactcacgctttataaagtcgactagtgaagcatttacgcaagtgcagccgctgtttgaactagaggccctatcgagcaagcgtaggccgccggaatccgaagatgaaggtgctaagggtcaggaaggtttcgaacagattaaacgcatcaaagcgtatttagacaccctaatggaagcggtgcacttcgcgaagcctctctacctggttaaagggcgaaagatgatagaaggtctggacaaagatcagagtttctatgaagcgtttgaaatggcatatcaggaactggaaagcttaatcattccaatttataataaagcgcgctcttatttgagtaggaaacccttcaaggccgataagttcaagattaactttgataataatactctgctttctggttgggacgccaataaagaaactgcaaacgcctccatcctctttaagaaagacgggttgtattacttaggcattatgcccaaagggaagaccttcctgttcgattatttcgtctccagcgaagattcagagaaactgaagcagcgtaggcaaaagacggccgaggaagcactggcccaggatggcgagagctacttcgagaagattcggtataaactgctgccaggtgcgagcaagatgttaccgaaagtcttcttctctaacaagaatatcgggttctataacccatctgacgacattcttagaattcgtaacacggcctctcacaccaagaacggcacgccgcagaaagggcactctaaggtagaattcaatctgaatgactgtcataagatgattgatttctttaagagtagcattcagaaacacccggaatgggggtcattcggattcaccttctcagacacgagcgacttcgaggatatgagcgccttctaccgagaagtggagaaccagggttacgtcataagctttgataagatcaaagaaacgtacatccagagtcaggtggaacaaggcaacctgtacctgtttcagatctataataaagacttctcaccgtactccaaggggaaaccgaatctccacacgttgtactggaaagccttattcgaggaagccaatttaaacaacgtggttgcgaagctcaacggcgaagctgaaatcttcttccgccgtcatagtattaaagcatccgacaaagtcgtgcatccagcgaatcaggccattgataacaagaatcctcataccgagaagacacagagcacatttgaatacgatctcgtcaaagataaacgttacactcaagacaaattcttctttcatgtgccgattagtctcaacttcaaagctcagggagtaagcaagttcaacgataaggttaacggcttcctcaagggtaacccggatgtcaatatcataggcatcgaccgcggcgagagacacttgctgtacttcacggttgtaaaccagaaaggtgaaatcttagtacaagaatctttgaacacgctgatgtctgataaagggcatgttaatgattaccaacagaaattggacaagaaagagcaagagcgtgatgccgcgcggaagagttggacaacggtggagaacattaaagaactaaaggagggttacctgtctcatgtggtacacaaattggcacatctgatcatcaaatataacgccattgtatgtcttgaagacctgaatttcggattcaaacgcggaaggtttaaagttgagaagcaggtctatcagaaattcgagaaggcgctgattgataagctgaactacctggtgtttaaggagaaggaactgggcgaagtaggacattatcttacagcgtatcagctgacagcacctttcgaaagcttcaagaaattaggcaaacaaagcggtatactgttctatgtgccggcggattatacttctaagatcgatccgacgaccggctttgttaactttctggatctgcggtatcagtctgttgagaaagctaagcaactgctctctgatttcaacgcgattcgtttcaacagtgttcagaactatttcgaatttgagatcgactacaagaaattaacgcccaaacgtaaggtcgggacgcaaagcaaatgggtgatatgtacctatggcgatgtccgctatcagaaccgtcgtaaccagaaaggtcactgggagactgaggaagttaatgttacggagaaactgaaagccctgttcgcgtctgacagtaagactaccaccgtcatcgattacgctaacgacgataacctgatcgatgtcatcttggagcaggacaaagccagtttcttcaaagagctgctctggttactgaaactgactatgacgttacgccatagtaagattaagtctgaagatgacttcattctttcacccgtaaagaacgaacagggcgagttctatgatagtcgcaaagcgggagaagtctggcccaaggatgcggatgcgaatggcgcataccacatagcgctgaaaggcctgtggaacctccagcaaattaatcagtgggagaaggggaagacgttaaacctggcaatcaagaatcaggactggttttcattcattcaggagaagccataccaggaataa

SEQ ID NO: 742 - DNA, 3897 bp, Artificial Sequence
  Description of Artificial Sequence: Synthetic polynucleotide
atgactaagaccttcgattccgaattctttaatttatattcactacagaagacagtcagattcgaattgaaaccagtgggtgaaactgcaagcttcgtcgaggattttaagaacgaaggtctgaagcgtgtcgtcagtgaggatgaaaggcgagctgtagattatcagaaagttaaggaaataattgatgattatcaccgtgacttcattgaagaatcactcaattactttccggaacaagtatccaaagatgcgttagaacaggcgtttcacctatatcagaagttgaaagcggccaaggttgaggaacgtgagaaggctctcaaggaatgggaagcacttcagaagaagttgcgagagaaggtagttaagtgtttctcggactcgaataaagctagatttagtagaattgacaagaaggagctaattaaagaggatttgataaattggttagttgcacagaatagagaggacgacatcccaacagtagaaactttcaataatttcactacctatttcacaggcttccacgagaatcgaaagaatatttactcaaaggacgatcatgcaacggctatttcgttcaggcttatacatgagaatttgcccaagttctttgacaatgttatatcattcaacaagctgaaagaaggctttccggagttgaagttcgacaaagttaaggaagatttagaggttgactatgatttgaaacatgcgttcgaaatcgagtactttgtaaatttcgtaactcaagccggtatcgatcaatataattatctgctaggaggtaagacattggaagatgggactaagaagcaaggaatgaatgaacaaataaacctgtttaagcagcaacaaacaagagacaaagccagacaaatacccaaactgatcccgctcttcaaacaaatcctgtcagaaagaactgaatcacagtcgtttattccaaagcaattcgaatcggaccaagagctatttgatagtcttcagaaacttcataacaattgtcaggacaaatttaccgtattacagcaagcaatcctgggactagctgaggccgatttgaagaaagtatttatcaagacttctgatttaaacgccctttctaataccatcttcggtaattattccgtcttcagtgatgccttgaatttatataaagaaagcttgaagacgaagaaggctcaagaagcgtttgagaagttaccggcgcatagcatacatgacttaattcagtatctggaacaatttaattcttccctcgatgcagagaaacaacaaagtacagatacggttcttaattacttcatcaagaccgacgaattatattcccgctttatcaagagtactagtgaagctttcactcaagttcaaccgttatttgaactggaagctttatcatctaagagaagaccaccagaatcggaggatgaaggcgctaaaggtcaagagggctttgagcagattaagagaatcaaggcttatttagatacattaatggaggctgtccactttgcgaaacctctctacctagtgaagggacgtaagatgattgaaggcctagataaggatcaatctttctacgaggcgttcgagatggcttaccaagaattagaatcccttatcataccaatttataataaagcaagaagttatttgtcaagaaagcctttcaaagcagataaattcaagatcaacttcgataataacacactactttctggctgggatgcaaacaaagagactgctaatgcctcgatcttatttaagaaagatggtttatattatttaggtattatgccgaagggtaagaccttcctcttcgattatttcgtatcttccgaagattccgagaaattgaaacaacgaagacagaaaaccgcggaagaagcactagctcaagacggtgagagctacttcgagaagatccgatataagttgctacctggagcttccaagatgttgcctaaagtcttcttctctaataagaatattggattctacaatccatcagatgacattctcagaatcagaaatacagcatcacacacaaagaacggtacgccacagaaaggtcattcaaaggttgagtttaaccttaacgattgccacaagatgatagatttctttaagagttcaatacagaaacacccagagtggggttcattcggctttacattctctgataccagtgatttcgaagatatgtcagctttctacagagaagtagagaaccagggctacgtaatatcattcgataagattaaggaaacttatattcaatcccaagttgaacaaggtaacttatacctgtttcaaatatacaacaaagacttctcaccttactcgaaaggcaaacctaacttacacactctatattggaaagccctctttgaggaagctaacttgaacaacgtcgttgctaaattaaatggcgaagcagagatattctttaggagacattcaattaaggcatcagacaaagtggtacaccctgctaaccaagctatagataataagaatccacacacagagaaaacacaatctacattcgaatatgacctcgttaaggataagagatacacgcaggataagtttttcttccatgttccgatatctcttaacttcaaagcccaaggtgtaagcaagtttaatgataaggtcaatggcttcctaaagggaaatccggatgtgaacataattggaattgatagaggtgaaagacatcttctgtatttcacagtagtcaatcagaaaggtgaaatcctcgttcaagaatctttgaacacattaatgtcagacaaaggtcatgttaacgactaccaacagaagcttgacaagaaagaacaggagcgcgatgccgccagaaagtcctggactacagtcgagaatattaaagaactaaaggagggatacctctcccacgtggtacataaattggctcatttaattattaaatacaatgccattgtatgtttagaggacttgaatttcggatttaagagaggcagattcaaagttgagaagcaagtttatcagaagtttgagaaggccttaatagataagttgaattacttagtattcaaagagaaggaactaggtgaagtaggtcactatcttacagcttatcaactgactgctcctttcgaatccttcaagaaattgggtaagcaatccggaatcctgttctatgtccctgctgattacacctcaaagattgatccaacgactggtttcgtgaacttcttggatctgagataccaatccgttgagaaggccaaacaattgctgtcggatttcaacgctataagatttaactctgttcagaattacttcgaatttgaaatagactacaagaagctaacacctaaacgtaaagttggtactcagagtaagtgggtaatttgtacttatggcgatgttagatatcagaacagaagaaaccagaagggtcattgggaaacagaggaagtaaatgtcacggagaagttgaaagcattatttgcgagcgattctaagacgactactgttatcgattacgcaaatgacgataaccttatagatgtaattctagaacaggataaagcttctttctttaaagaattgttgtggcttcttaaactaacaatgactttacgtcattccaagataaagagcgaggacgactttatattaagccctgtcaagaatgaacaaggagaattctatgattctaggaaagcgggtgaagtctggcctaaagatgctgatgctaacggcgcttatcatatcgcacttaagggtctttggaaccttcaacagattaaccaatgggagaaaggtaagactctgaacttggccatcaagaatcaagattggttctcctttattcaagagaaaccataccaagaatga

SEQ ID NO: 743 - DNA, 3897 bp, Artificial Sequence
  Description of Artificial Sequence: Synthetic polynucleotide
atgacgaagaccttcgactctgaattctttaacttgtactcattgcaaaagactgtgagatttgagcttaaacctgtaggtgaaactgcctccttcgtcgaggacttcaagaacgagggattaaagagagttgttagtgaggatgaaagaagagctgttgattaccagaaagttaaagaaattattgacgattaccatagggacttcattgaggagtcactaaactactttcccgaacaagtatcgaaagatgccttagaacaagcgttccatctatatcagaagttaaaggcggccaaagtggaagaaagggagaaggcgttgaaagaatgggaagcattacagaagaagttgagagagaaggtcgtcaagtgcttctcagacagtaataaagcgcgcttctcccgtatagacaagaaggaacttatcaaagaagacttaattaactggttggtcgcgcagaaccgtgaagatgatatcccaacagtggaaacatttaataatttcacgacttacttcactggattccatgagaacagaaagaatatttactcgaaagatgatcacgccactgctattagtttcaggctaatacatgagaaccttcctaaattctttgataatgtaattagtttcaacaagctcaaggaaggatttcctgaattgaaatttgataaagttaaggaagatttagaagtggattacgatctgaagcacgctttcgaaatagaatacttcgtcaacttcgttactcaagcaggtattgatcagtacaactatttactgggtgggaagaccttagaagatggtactaagaaacaaggtatgaacgaacagattaatttatttaagcagcagcagacaagggataaagccagacagatacccaagttaatcccactctttaaacagatcctaagtgaacgcactgaatcacaatcattcattcctaaacaatttgaatccgatcaagagttgttcgatagcttgcagaaattacataacaattgccaggataaatttacagttctccaacaagctatcctgggtttggcagaggctgacttgaagaaagtattcattaagacctccgatttaaacgcattaagtaacaccatcttcggcaactattcggtgttctcagacgctttaaatttgtataaggagtctctgaagacaaagaaagctcaggaggcctttgagaaattgcctgcacacagtatacatgatctaatccagtatcttgagcaatttaactcatctttagacgctgagaagcaacaatctacggatacagttctcaactacttcatcaagacagatgaattgtactcaagattcatcaaatctacttccgaagcctttacacaggtgcaaccattgtttgaattggaggctttatcctcaaagaggagaccacctgagtctgaagatgagggtgctaagggtcaagagggtttcgaacagataaagagaattaaagcttacttggatacgctgatggaggctgttcacttcgccaagccattgtatttagtcaagggtagaaagatgatagaaggcctagataaagatcaatcgttctatgaagctttcgaaatggcttaccaggagttggaatctttgataataccaatttataataaagcaagatcatatttaagtcgcaagccgtttaaggcggacaaatttaagatcaatttcgacaataacactttattaagcggatgggatgcaaataaagaaactgctaatgcttcgatactattcaagaaggatggtttgtattatttaggtataatgccaaaggggaagactttcttattcgattatttcgtcagctcagaagatagtgagaaactcaagcagagacgccaaaagacagcggaagaagcattagcacaagatggcgaatcttactttgagaagatcagatataaactgttgccaggagcgagtaagatgctcccgaaagtcttcttctccaacaagaatattggtttctacaatccaagtgatgacatcttaagaattcgaaataccgcatcccataccaagaatggtactcctcagaaaggacattccaaagtcgaatttaacttaaacgactgtcataagatgatcgatttcttcaaatcctcaatccagaaacaccctgaatggggttcattcggtttcacgttctctgacacgtccgactttgaagatatgtccgcgttctatagagaagttgagaatcaaggctacgttatttcattcgataagattaaggagacctatattcagagccaagttgaacaagggaatttatacttattccagatttataataaggatttctcgccatattctaaggggaagcctaacttgcacactctgtactggaaagcgttattcgaagaagcgaatcttaataatgttgtcgctaagttgaatggtgaagccgaaatcttcttccgacgccacagcatcaaagcttcagataaggttgtacacccagctaaccaggctatcgataataagaatccacacacagagaaaacccaaagtaccttcgagtacgatctagttaaggataagagatacacgcaggacaaattcttctttcatgtgcctatatcactgaacttcaaggcgcaaggcgtttccaagtttaacgataaggtgaatggtttcttgaaaggtaatcctgacgtaaatattatagggatagacagaggagagagacacttgctttacttcacagtagtaaatcagaaaggtgaaatactagtgcaagagtccctaaatacattaatgtccgataaaggccatgtaaatgattaccaacagaagcttgacaagaaagaacaggaacgagacgccgcgaggaagtcgtggactactgtagagaacatcaaagaacttaaggaaggttatctcagtcatgttgtgcataaactcgcccacttaatcattaaatataatgcaattgtctgtttagaagatttaaacttcggatttaagagaggtaggttcaaagttgagaaacaagtatatcagaaatttgagaaagctcttatagacaagttgaattacctggtatttaaggagaaggaattaggagaggttggccactatctaactgcgtatcaattaactgctccttttgaatcattcaagaagctaggcaaacaatcaggaatcctcttctacgtccctgccgattatacttctaagatagacccaaccacaggatttgtcaacttcttggatcttagatatcagtccgtagagaaggccaaacaactgctctctgacttcaatgcaattagattcaacagtgtacagaactatttcgaatttgaaattgactataagaaactaactccaaagaggaaggtgggaacccagtcgaaatgggtgatatgcacatacggcgacgtacgttatcagaataggagaaatcagaagggtcattgggaaactgaagaggttaacgttaccgagaaattgaaggcactattcgcatcggacagtaagacaacaacagtcatcgattacgccaatgacgataatttaattgatgttatactcgagcaagacaaggctagcttctttaaagaattattatggcttcttaagttgactatgactttacgtcacagtaagattaagtccgaagatgacttcatattatcaccagtaaagaatgagcaaggtgaattctatgattcgagaaaggcaggtgaagtttggccaaaggatgctgacgccaacggagcgtaccatattgccttgaagggactatggaatcttcaacaaattaatcaatgggagaagggtaagactttaaacttagctattaagaaccaggattggttctcgttcatccaagagaagccatatcaagaataa

SEQ ID NO: 744 - DNA, 3897 bp, Artificial Sequence
  Description of Artificial Sequence: Synthetic polynucleotide
atgacgaagacgttcgattctgagttcttcaatctctatagcctacagaagactgttagattcgagttgaagcctgtaggtgaaaccgcttctttcgttgaggactttaagaatgaaggtctgaagagggttgtttctgaagacgaaagaagagctgtggattatcagaaggtaaaggaaataatagatgactaccatagagacttcatcgaagaaagtttgaattacttcccagaacaggtcagcaaggacgccctggaacaagccttccacctatatcagaagttgaaagctgccaaggttgaagaaagagagaaggccctcaaggaatgggaagcgttgcaaaagaaattaagagagaaagtcgttaaatgcttctcagactccaataaagcaaggttctctaggattgataagaaagaattgatcaaagaggatttaataaattggctcgttgctcagaacagagaagatgatatcccgacagtcgaaactttcaacaatttcacgacttacttcacaggattccatgagaaccggaagaatatttactctaaagatgatcatgctacagcaattagtttcaggctaattcacgagaacttgcctaaattctttgacaatgtgatatcgttcaataagttgaaggaaggcttccctgaattgaaatttgataaagtgaaggaggatttggaagtggactatgatctgaaacatgcctttgaaattgaatacttcgtaaacttcgtcactcaggcaggtattgatcagtataactatctattaggcggtaagacactagaagatggtacgaagaaacaaggtatgaacgagcaaatcaatttgtttaagcaacagcaaactagggacaaagcaagacaaattcccaagctaataccattattcaaacaaatcttgagtgaaagaacagaatctcaaagcttcatccctaaacaatttgaaagtgatcaggagttgttcgatagtttgcagaagctacataacaattgtcaggataagtttacagtattacagcaagctatactaggtttggcggaagctgatttgaagaaagtgtttataaagacttcggatttaaacgctttgagcaacacaatatttggaaattatagcgtgttctcggatgcacttaatttgtataaggaatcactaaagacaaagaaagctcaggaagcgtttgagaaattaccagcacattcgattcacgacctgattcaatacctggaacaattcaactcatccttggacgcagagaaacagcagtcaaccgacactgttctaaactacttcatcaagacggacgaattatactccagattcataaagtcaacctcggaagctttcacccaagtacaaccgttatttgaactagaagcgttgtcctctaaacgtagaccaccagaatccgaagatgaaggagctaaaggacaagaaggattcgaacaaatcaagaggattaaggcttatcttgatacattgatggaagccgtacatttcgcgaagccgctatacttagtcaagggacggaagatgattgaaggtctagataaggaccaaagtttctatgaggcatttgagatggcataccaagagcttgaaagcttgattattccaatctataacaaggcgcgctcatatttatctaggaaaccctttaaggctgataagtttaagattaactttgataacaatacattgttgtccggctgggatgcaaacaaggagacagccaacgcctccatcctatttaagaaggacggtctgtactacttgggtatcatgcccaaaggcaagactttcttattcgattactttgtctcctccgaagatagtgagaagttaaagcaaaggcgacagaagacagcggaagaagctctggcgcaagacggtgaatcttatttcgagaagataagatataagttgttaccaggtgcttccaagatgttgcctaaggtattcttcagcaataagaatattggcttctacaacccaagcgacgatatcctcagaattagaaatacggcctcacacacgaagaatggaacgccacagaaaggtcattcaaaggttgagttcaacctaaacgactgccacaagatgatagacttcttcaaatcatccatacagaagcatccggaatggggctcgttcgggttcactttctctgatactagcgacttcgaagatatgtctgctttctacagagaagtcgagaatcaaggctatgtgatctctttcgacaagattaaggaaacctacatccaaagtcaagttgaacaaggtaacctttacttattccaaatttataacaaagacttctctccatattctaagggtaagcctaacctacatacattgtattggaaagcattattcgaagaagccaatttaaataatgtcgtcgcgaaattaaatggtgaagccgaaattttctttaggaggcacagtattaaggcatcagataaagttgtacatccagctaatcaagcaattgataacaagaatcctcataccgagaaaacccaatccacatttgaatatgatttggtcaaagataagagatatactcaagataaattcttcttccatgttccaatatccttgaacttcaaagcgcaaggtgtgtccaagtttaatgataaagtgaatggattcctaaagggtaatcccgatgttaatattatcggtatagatcgtggcgaaagacatttgttgtatttcacagttgtgaatcagaaaggagaaatattggtgcaagagtcactaaatacattgatgtccgataaaggccacgttaatgattatcaacagaagcttgacaagaaggaacaagagagagatgctgcacgtaaatcttggaccactgtcgagaacatcaaggaactgaaagaaggttatttaagccatgttgtccataagttagcgcatttgataatcaagtacaatgcaattgtctgtttagaagacctaaacttcggctttaaacgtggaagatttaaggtggagaagcaggtgtatcagaagttcgagaaggcactaattgataaattaaattacttagtcttcaaggagaaagaattaggtgaggtgggtcattacttaaccgcttaccaactaacagcgccgtttgaatcctttaagaaactaggtaagcagtctggtatcttgttctacgtgccagcagattacaccagcaagattgacccaaccacaggattcgttaacttccttgacttgagatatcaatctgtagagaaagcaaagcaacttctatccgactttaacgcgattaggttcaatagtgttcagaactactttgagtttgaaattgactacaagaaattaacaccgaagagaaaggttggcactcaatcgaagtgggtcatttgtacatatggtgatgttaggtaccagaataggcgtaatcagaaaggacactgggagacagaagaagttaatgttactgagaagcttaaggctctcttcgcctcagactcaaagactactactgtcattgattatgctaatgatgataacttgatagatgtcatcctggagcaggataaagctagcttctttaaagaactattgtggttgttgaagttaactatgactcttcgacatagcaagataaagagtgaagacgatttcatcctctcaccagttaagaacgaacagggtgaattctacgacagccgcaaggcaggtgaagtatggcctaaagatgcggacgcaaatggagcttaccatattgcactgaagggtctttggaatttacaacagattaaccagtgggagaaaggaaagactttgaacctcgcaataaagaatcaagactggttcagctttatacaagagaagccataccaggaataa

SEQ ID NO: 745 - DNA, 3897 bp, Artificial Sequence
  Description of Artificial Sequence: Synthetic polynucleotide
atgactaagaccttcgactccgaattcttcaatctctactctcttcagaagaccgtcagatttgaactaaagcctgtcggtgagacagcaagctttgtagaagactttaagaacgagggcctgaagagagttgtttcggaggatgaaagaagagcagttgactaccagaaagtaaaggaaattatcgacgactaccatagagacttcatcgaggaatcactgaattacttcccggagcaagtttctaaggacgccctcgagcaagctttccatctttatcagaagttgaaagccgctaaggtcgaagaaagagagaaggcactcaaagaatgggaagcactacaaaagaagttaagggagaaggttgttaagtgtttctctgatagtaataaggcaaggtttagtagaattgacaagaaagaattaattaaggaagacttaattaactggttggtggctcagaacagagaagatgatatacctacagttgaaacatttaacaatttcactacttacttcaccggattccatgagaatagaaagaatatttactcgaaggatgaccatgctacagcaatctcatttcgtttaatccatgagaacctacccaagttctttgataatgtgatttcgttcaacaaacttaaagagggtttcccagaattgaagttcgataaggttaaggaagacctggaagttgattatgatctcaagcatgcctttgaaattgaatactttgttaactttgtcactcaagctggtatagatcaatataattatctactaggcggcaagacacttgaagatgggacaaagaaacagggaatgaatgaacaaattaacttatttaaacaacaacagacaagggataaggcccgtcagattcccaagttgattccattgttcaagcaaatactttccgaacggacagaatcacaaagctttattcctaaacaatttgagtccgatcaggaactgtttgattcattgcagaaattgcacaataactgtcaagataaattcacagtattacagcaagcaattctgggcctagctgaagccgatctgaagaaggtgtttatcaagacttcagatttaaatgccctgtcaaataccatcttcggaaattactctgtcttctctgatgccttaaacctgtataaggagtccctaaagaccaagaaagcccaagaagcgttcgagaaattgccagcacattccatacacgacttaatccaatacctcgagcagttcaatagttcacttgatgctgagaagcaacaatcaacagataccgtcttgaattactttattaagacagatgagttgtattctagattcattaaatcaacatctgaagcctttacacaagttcagcctctcttcgaattagaggccttatcttcaaagagacgtccacctgaatccgaggacgaaggtgccaagggtcaagaagggttcgagcaaatcaagagaattaaggcatatctagatacgctaatggaagccgtgcacttcgctaaaccactatacttagtaaagggtagaaagatgattgaaggtctagataaagaccaatcattctacgaagcgtttgaaatggcctatcaggagttagagtctttgatcattcctatctataataaagcaaggtcttatctaagtcggaagcccttcaaggctgacaaatttaagatcaacttcgacaacaatactctcttatccggttgggacgcgaacaaagagacagcaaatgctagtattctctttaagaaggatggtttatactatctaggtatcatgcctaaaggaaagacctttctatttgattatttcgtttcatcagaagatagtgagaaattaaagcaacgtcgtcagaagaccgcggaagaagctttagctcaggatggcgaaagctacttcgagaaaattagatataagttgttgccaggcgcctctaagatgctaccaaaggtattcttttctaacaagaacattggcttctacaatccgtctgatgatatacttagaattagaaacactgcatcgcatacaaagaacggaactcctcagaaaggccatagcaaggtagaatttaacctaaacgattgtcacaagatgattgatttcttcaagagttctatccagaaacatccagaatggggaagctttggatttacattcagtgacacttcagacttcgaagatatgtccgcgttctacagggaagtggagaatcaaggatatgtgatcagctttgataagattaaagaaacatatatccaatcacaggttgaacaaggtaatctttacttgttccaaatctataacaaagatttctctccgtatagtaaagggaaaccaaacctacatactttgtactggaaggcattattcgaagaagccaatttgaataacgtggtggctaagttgaacggtgaagctgaaatattctttaggagacactctatcaaggcctctgacaaggttgtccacccagctaaccaagctatcgacaataagaacccacacacagagaagactcaatctacatttgaatacgatctggtaaaggacaaacgatacacgcaggataagttcttctttcatgtgccaatttcattaaatttcaaagcccagggagtatctaagtttaatgataaggttaatggcttccttaaaggcaatcctgatgtgaatattatagggattgatcgcggagaaagacatttactatactttaccgtcgtcaaccagaagggtgaaatcttagtgcaagagtccttaaatacgctgatgtctgacaaaggacatgtgaacgattaccaacagaagttggacaagaaagagcaagaaagagacgcggcacgaaagagctggacaactgtagagaacataaaggaactgaaggagggttatttgtcgcatgttgtacataaattagcacatttaattattaaatataacgcaattgtttgtttggaggatctgaacttcggattcaagcgtggaaggttcaaagtagagaaacaagtttaccagaaatttgagaaggccttaattgacaaattgaactacttagtctttaaggagaaggaattgggtgaagtcggtcattatctaactgcataccaactcacagctccgttcgaaagtttcaagaagctgggtaaacaatccggaatattgttctatgtacctgcggattacacaagtaagattgatccaactactgggttcgttaacttcttagacttacgatatcaatcggttgagaaggcaaagcagctgttgtcggacttcaatgcaattagatttaatagcgtccagaactatttcgaattcgaaattgattataagaagttgacgccgaagcgtaaggtgggtacgcaatcaaagtgggtaatctgcacatatggtgatgtcaggtaccagaacaggagaaatcagaagggacactgggaaactgaggaggttaatgtcactgagaagctgaaggctctctttgcaagtgatagcaagactactactgttatagattatgcaaatgacgacaatctgatagatgtcattctggaacaagataaagcctctttctttaaagaacttctttggctgttgaaactgacgatgacattacgtcatagcaagattaaatccgaagacgacttcatcttgtctccagtaaagaatgaacaaggagaattctatgattctaggaaggccggtgaagtttggccaaaggatgctgatgcaaatggtgcttatcacattgctcttaagggcttatggaacttacaacaaattaatcaatgggagaaaggaaagactttgaacttggccattaagaaccaagattggttttccttcatacaagagaaaccatatcaagaataa

SEQ ID NO: 746 - DNA, 3897 bp, Artificial Sequence
  Description of Artificial Sequence: Synthetic polynucleotide
atgactaagacgtttgatagcgaattctttaatctatattctttgcagaagactgttaggttcgagcttaaacctgtgggtgaaaccgcttcatttgtcgaagactttaagaatgagggcttaaagagagttgtgtccgaagacgaaagaagggctgtagattatcagaaggtcaaagaaattattgacgattatcatagggatttcattgaagagtctttgaattactttccagagcaagttagtaaggatgcattagaacaggcatttcacctatatcagaagctgaaggcggcgaaagttgaagagagagagaaagctttgaaggaatgggaagccctccagaagaagctacgtgagaaagttgttaagtgcttctccgattcaaataaagctagattcagtagaattgataagaaagagttgataaaggaagatctcattaattggttggtagctcagaacagggaggacgatattcctaccgtagaaacatttaacaacttcactacttactttactggatttcacgagaatcgcaagaatatttattctaaggatgatcatgctaccgctatttcgttcagattaattcatgagaatttacctaaattctttgacaatgtaatttcatttaacaagttgaaggaaggattcccggaacttaagtttgacaaggtaaaggaagacctggaagttgactacgatcttaaacacgcatttgaaatcgaatatttcgttaacttcgttacacaagcgggtattgatcaatataactatttattgggaggcaagacattagaggacggaacgaagaaacagggtatgaatgaacagataaatttgtttaaacaacaacaaacacgtgacaaagctcgccagattccaaagttgattccactgttcaagcaaatattgtcagaacgtactgaatctcaaagcttcatacctaagcaatttgaatcagaccaagagctgtttgactctttacagaagctgcacaataattgccaagataaatttacggtcctacagcaggctatattaggtcttgctgaagccgatttaaagaaagtatttattaagacctcagacttaaacgcactaagtaatacaatattcggtaactattctgtgttctctgatgcattgaatttgtataaggaatctctaaagaccaagaaagcccaagaagccttcgagaaattgccggctcactctatccatgaccttatccaatatttggaacagttcaatagctccctcgacgctgagaaacaacagagtaccgatactgtattgaattacttcattaagacagatgaattgtattctaggtttatcaagtcaacgtctgaagccttcactcaagtgcaaccgctgttcgaacttgaagctttaagtagcaagcgtagaccacccgaatcggaagacgagggcgccaagggacaggaaggcttcgaacaaattaagcgaattaaagcatatctagacactttaatggaggccgttcacttcgccaaacccttatatcttgttaagggtcgtaagatgatagaagggttggataaagatcagtcgttctatgaggcattcgaaatggcgtaccaagaattagagtcattaataattcctatatataataaagcaagatcctacttgtcccgtaagccgttcaaagctgacaaatttaagataaacttcgataataatactttactgtctggatgggatgcgaacaaggaaactgcgaatgcttcgatcttattcaagaaagacggcctatattatttaggcattatgccaaagggcaagacattcctatttgattacttcgtgtctagtgaggattctgagaagctaaagcaaaggcgtcagaaaacagcagaagaagccctagcccaagatggtgaatcctacttcgagaagattaggtataaattgctgcctggtgcctctaagatgttacctaaagtgttcttctccaataagaatattgggttctataatccatctgatgacatattacgaattagaaatactgcttcacatacgaagaacggaactccccagaagggacactctaaagtcgaattcaatctaaatgattgtcataagatgatcgatttctttaagtcttctatccagaaacaccctgaatggggttcgtttggtttcacattctcagatacatcggactttgaagatatgagcgctttctatagagaagttgagaatcaaggttacgtaatatcatttgacaagattaaggagacatatatacagtctcaagtggagcaagggaatttgtatttattccaaatttacaataaagacttctctccgtactccaagggtaaacctaacttgcacactctgtactggaaagctttatttgaggaggctaacttaaataatgttgtcgctaagcttaatggtgaagcagaaatattcttcagaagacattccattaaggcgtctgataaagtcgtacatccagcaaatcaagctatagacaataagaatccgcatactgagaaaactcaaagtacattcgaatacgatttagtcaaagacaagaggtatacccaggataaattcttcttccatgtgcctattagcctaaactttaaggcccaaggcgtgtcgaagttcaatgataaggttaacggattccttaagggcaaccctgatgttaacattattggaattgacagaggtgaacgacatttattgtactttacagttgttaaccagaaaggagaaatacttgttcaggaatctctgaatacgttaatgtctgataagggtcacgtcaacgactaccagcagaaactagacaagaaagagcaagaaagggacgctgctagaaagtcctggaccacagttgagaatattaaggaattgaaagaaggttatttaagtcatgtagttcataaattggcccaccttattataaagtacaatgcgattgtgtgtttagaagatttgaatttcggctttaagagaggcaggttcaaagttgagaagcaagtttaccagaagtttgagaaggccctaatagacaaattaaattacttagtattcaaggagaaggaactcggcgaagtaggacattatcttactgcgtaccaattgaccgcaccctttgaatcgtttaagaagttgggtaaacagtcgggtatactgttctatgttccggcagattatacgtccaagatagatccaactactggctttgtaaactttctggatttaaggtaccagtccgttgagaaagcaaagcagctcctgtctgactttaacgctattcgcttcaatagtgttcagaactacttcgaatttgagatcgactacaagaaattaacgcccaagaggaaagttggaactcaatctaagtgggtaatttgtacctatggtgatgttagataccagaatagaaggaaccagaaaggtcactgggagaccgaggaggtcaacgtcaccgagaaattgaaagctttatttgcttctgattctaagacgacaactgttattgattatgctaatgatgataatttgatcgatgtaatcctggaacaagataaagcttctttcttcaaagagttattgtggctgctaaagcttacgatgactctgaggcattctaagataaagagtgaagatgactttatcttatcaccggtaaagaacgaacaaggtgagttctacgattctcgaaaggcaggagaagtgtggccgaaggatgcggatgcaaatggtgcttatcacattgccttaaagggactgtggaatttgcaacaaattaatcagtgggagaagggaaagacacttaacttagcgattaagaatcaggattggttctccttcatacaagagaagccataccaagaatga

SEQ ID NO: 747 - DNA, 3897 bp, Artificial Sequence
  Description of Artificial Sequence: Synthetic polynucleotide
atgaccaagacatttgattctgaattctttaatttatattcactgcagaaaactgttaggtttgaactaaagccagtgggtgaaacggcgtcattcgtggaagacttcaagaacgaaggattgaagagggtcgtatcagaagatgaacgcagagcagtcgattaccagaaggttaaggaaatcatcgacgattatcatagagacttcatagaagaaagtctgaactactttcctgaacaagtgagtaaggatgcccttgagcaagcatttcatttgtaccagaagttaaaggctgctaaagtagaggagagagagaaagccttgaaagaatgggaagctcttcaaaagaaattgagagagaaagtagtcaagtgcttctccgattctaacaaagcgcgattcagtagaatagacaagaaggaattgatcaaagaagacttgattaactggctcgttgcgcagaatagggaagatgatatacccaccgtcgaaacctttaacaacttcactacatacttcacagggtttcacgagaatagaaagaatatatatagcaaagacgaccatgctactgctatttcatttagactgatacatgagaatctccctaaattctttgataacgtaatttcgttcaacaagcttaaggaaggctttcctgaattgaagttcgataaggttaaggaagatttagaagtggactacgatttgaaacatgcgttcgaaattgagtacttcgttaatttcgttactcaggctggcatagatcaatataattatttactaggaggtaagacactcgaagacggcactaagaaacaaggtatgaacgaacaaatcaatttattcaaacaacaacagacgagggataaagctcgtcaaatcccaaagttaattccgttgtttaagcaaatcctgtccgagagaactgaatcacaatcatttattcctaagcaattcgaatctgatcaagaattatttgactcgctacagaaattgcacaataattgccaagataagtttacagtcttgcagcaagcaatactgggccttgcagaagcagacttgaagaaagtatttataaagacttctgacttaaatgctttgagtaacactatattcggcaattattcagtattctccgatgcgttgaatttatacaaggaatctctgaagacaaagaaagctcaagaagcatttgagaagttgccagcacattcaattcatgacctaattcagtatctggagcaattcaattcgtcgttggatgccgagaaacaacaatcaactgataccgtactgaattactttatcaagaccgacgaactctattcaaggtttattaaatcaactagcgaagctttcacacaagttcaaccgttgtttgaacttgaagctctatcctcgaagaggaggccaccggaatccgaagatgaaggtgcaaagggtcaagaaggctttgaacaaataaagagaattaaagcgtatttggatacattgatggaagccgttcacttcgcaaagccattgtacttagtgaagggtagaaagatgattgaaggcttggataaagaccagagtttctatgaagccttcgaaatggcctatcaagaattagagtcccttattattccaatctataataaagcgcgcagctatttaagtcgaaagccgttcaaggccgataaattcaagatcaacttcgataataacaccttattgtccggatgggatgccaacaaagaaacagcaaacgctagtatattattcaagaaagatggattatactatcttgggatcatgcctaaagggaagactttcctgttcgactactttgttagtagcgaagactctgagaaattaaagcaaagaagacagaagactgctgaagaagcattggcccaagacggagaatcttacttcgagaagataagatacaaactattaccaggtgctagtaagatgctgcctaaagtatttttctctaataagaacataggtttctacaatcccagtgatgacatcttgagaattaggaatactgcgtcgcataccaagaatgggacaccacagaagggtcactccaaggtagagtttaacttgaacgactgtcacaagatgattgatttctttaaatctagtatccagaagcaccctgaatggggttcattcggctttacattcagcgatacgagtgacttcgaggatatgtcagccttctaccgtgaagtcgagaaccaaggttacgtcattagcttcgacaagattaaagaaacatacattcaatcacaggtggaacaaggtaatctttatctattccaaatctacaataaagacttctcaccctattcgaaaggtaagcctaatttgcatacattgtattggaaagccctatttgaagaggctaatttaaacaacgtcgtggctaaattaaacggcgaagctgaaatcttctttagacgtcattccattaaggcaagtgataaagttgttcatcctgcgaaccaagctatcgataacaagaatcctcatacagagaaaactcaatcgaccttcgaatacgatttggttaaggataaacgctacactcaagacaaatttttctttcacgttccaatctcacttaactttaaggctcaaggtgtatctaaattcaatgataaggttaacggcttcttaaagggcaatccggacgtgaacattataggaattgatagaggagagagacacttgctgtacttcaccgttgttaaccagaaaggtgaaatattggttcaagaatctctgaacacactaatgagcgataaaggtcacgtgaatgactatcaacagaagctcgataagaaagaacaagaacgtgacgcagcacggaagtcgtggacaactgtagagaatataaaggaattgaaggaaggatatttgtcacatgttgttcacaaacttgcacacttgataatcaaatataatgcaattgtctgtcttgaggacttaaacttcggtttcaagcgcggtcgcttcaaagtggagaagcaggtctatcagaagttcgagaaagcactaatcgataagctgaattatcttgtctttaaggagaaagaattgggtgaagtgggacattatttgactgcatatcaattaacagcaccatttgaatcattcaagaaactaggaaagcaaagtggtatcttattctatgtgcccgcagattacacgagcaagatagatccaactaccggcttcgttaatttcttagatttacggtatcagtcagtggagaaagccaaacagctattgtctgatttcaatgccatccgtttcaatagtgtacagaactactttgaatttgaaattgattacaagaagctaactccaaagcgcaaggttgggacacaatccaagtgggttatatgcacctacggtgatgtcagatatcagaatcgtagaaaccagaagggccattgggagacagaggaggtgaacgttaccgagaaactgaaggcattgttcgcttctgactctaagactaccacagtgatagactacgccaatgacgataatttgattgatgtaatactcgagcaggacaaagcctcattctttaaggagttgttatggctgctgaagctgacaatgacgttacgccactctaagattaagtctgaggacgacttcatcttgtctcctgtaaagaacgaacaaggtgagttctatgattcacgtaaggctggcgaagtatggcccaaagacgcagatgccaatggagcctatcatatagctcttaaaggcctctggaatttacaacaaattaatcaatgggagaagggcaagacactaaatctcgcaattaagaatcaagactggttcagtttcatacaagagaagccttaccaagaataa

SEQ ID NO: 748 - DNA, 3897 bp, Artificial Sequence
  Description of Artificial Sequence: Synthetic polynucleotide
atgaccaagaccttcgattccgagttcttcaatttgtattccttgcaaaagacagttagattcgagttgaagccagtaggagaaactgcatccttcgttgaggactttaagaatgaagggttgaagagagtggtatccgaagatgagagaagagcagtggactatcagaaagtcaaagaaataatagatgattatcaccgcgactttatcgaagaatctttgaattactttcctgaacaagtctccaaagacgccctggagcaagcattccatctatatcagaagttaaaggctgcaaaggtcgaagagagagagaaggctttgaaggaatgggaagctttgcaaaagaagttgagagagaaagtagttaagtgtttctccgactctaacaaagcccgattctcaaggatagacaagaaggaattgataaaggaagatttgattaattggttggtggcacagaaccgagaagacgacattcccacagttgagaccttcaataatttcacaacgtatttcactggattccatgagaaccgcaagaatatctacagtaaagatgatcacgctactgctatatcatttcgattgatccacgagaacttacctaagttctttgacaatgttattagtttcaataaattgaaagaagggttcccagaattaaagtttgacaaagttaaagaagatttggaagttgattatgacttgaagcacgccttcgaaatagaatacttcgtaaactttgtaacccaagcgggtatcgaccagtacaattatttgttaggtgggaagactttagaagacggcaccaagaaacagggtatgaacgaacaaattaatctattcaaacaacaacagactagagacaaggcccgtcaaattccaaagctaataccgttgttcaaacagatccttagcgaaagaacagaatcgcaaagcttcattcctaagcagttcgagagcgatcaggagctatttgatagtctccagaagttacataataattgccaggataaattcacagttctccaacaagcaatactaggtttagccgaggcagatttaaagaaggtgtttataaagacttcagacttgaatgcgctcagtaataccatatttggtaattactccgtgttcagtgatgctttaaatttgtataaggagtccttaaagaccaagaaggcacaggaagctttcgagaagttgccggcacattcaatacatgacttaattcaatacttggagcaatttaattctagcttagatgcggagaaacagcagtctacagacactgtgcttaattatttcattaagactgatgagctgtattcgcgatttattaagtctacctctgaagccttcactcaggtccaacctttgtttgaattggaagcgttatcttcgaagagaagaccacctgagtctgaagatgaaggtgccaaaggccaagaaggattcgaacaaattaagagaattaaggcctacttagatacgttgatggaagccgtccactttgctaagccattgtatttagttaagggccgaaagatgatcgaaggtttggataaggaccaatcattctatgaagccttcgaaatggcgtatcaagaattggaatccctgattatacctatatataacaaggctcgctcttacctttctcgtaagccatttaaggcagataagttcaagatcaactttgataataacactttattatcaggctgggacgcaaataaagagacggctaatgccagcatattgtttaagaaagacggtttgtattacctaggtattatgcctaagggaaagacattcctctttgattatttcgtctcatcggaagatagtgagaaacttaagcaacgtagacagaagactgccgaagaagctttagctcaggacggtgagtcatacttcgaaaagattaggtataaacttctaccaggcgcaagcaagatgttgccaaaggtgttcttctcaaacaagaatattggcttctataatccatctgacgatatattgagaatcagaaatactgcatcccatacgaagaatggtactccacagaaaggtcattctaaagtggaattcaatcttaacgactgtcacaagatgattgatttcttcaaatcctccattcagaagcatccagaatggggctcgttcggctttaccttctccgatacgtcagatttcgaagatatgtccgccttctatagggaagtagagaatcaaggctacgtaatttccttcgacaagatcaaggaaacttatatacaatcccaggtggaacaaggtaacttatacttatttcaaatctacaataaggatttctcaccatatagtaaaggaaagcctaatctacacacattatattggaaagctttgttcgaagaagccaatctaaacaacgtggtggcgaagttgaatggtgaagctgagatcttctttaggagacactctattaaagcctcagacaaagtcgtccacccagcaaaccaggctattgacaacaagaatcctcacactgagaagacacaatctacgttcgagtacgatttagttaaagataaacgttatacgcaagataagttcttctttcatgtgcctatctctctaaatttcaaagctcaaggtgtctccaagtttaatgataaagtgaatggattcctgaagggcaatccagatgttaatattataggtatcgatagaggtgagcggcatctattatacttcactgtagttaaccagaagggtgagatcttagtccaagagagtttaaatacgttaatgagcgacaagggtcatgttaacgattaccagcagaaattggataagaaggaacaagaaagggatgcggctcgcaaatcttggacgactgttgagaatatcaaggaactgaaggagggttatttgtcgcacgtagtccataagcttgcacacctaattattaagtacaacgctattgtttgtcttgaggacctaaatttcggattcaaacgaggcagattcaaagttgagaagcaagtttatcagaaatttgagaaagctttgatagataaactgaactatttagtatttaaagagaaggaacttggagaggttggtcactatctaacggcttatcaattgactgctcctttcgagtctttcaagaagttaggtaaacaaagtggtatattgttctatgtgcccgcggattatacttctaagattgatccaactactggattcgtcaacttcttggatctacgatatcaatcagttgagaaggcaaagcaattactctcagactttaatgcaataagatttaacagtgtgcagaattatttcgaatttgaaattgactataagaaacttacgcctaagagaaaggttggaacacagagcaagtgggttatatgtacatatggagatgttcgttaccagaacagacggaatcagaaaggacattgggagactgaagaagtcaatgtcactgagaaattgaaggcactatttgcctcagattctaagacaacaacggttattgattacgcaaacgacgataacttaatcgatgtcattcttgagcaagataaagcctctttcttcaaggaattgttgtggttgttgaaattgactatgacgcttaggcactccaagatcaagagcgaagatgatttcattctgtcgccggtcaagaatgaacaaggtgagttctatgattcccggaaggctggtgaggtttggcctaaagatgcagatgccaacggtgcttatcatattgccttgaaaggattatggaatcttcagcaaattaatcaatgggagaagggtaagactttaaacctggccataaagaatcaagattggttctctttcattcaagagaagccttatcaagaataa

SEQ ID NO: 749 - DNA, 3897 bp, Artificial Sequence
  Description of Artificial Sequence: Synthetic polynucleotide
atgaccaagacattcgattcagagttctttaacctatatagtctacagaagaccgttagattcgaacttaagccagtgggagaaactgcaagcttcgttgaagacttcaagaatgagggtttaaagagagttgtttcagaagatgaaagaagagccgtggactaccagaaggttaaagaaataatagatgattatcatagagactttatagaagaaagtttgaactacttcccagaacaagtgagcaaagacgcattagaacaggcatttcatctatatcagaagttgaaggccgctaaagttgaagagcgcgagaaagctctgaaggaatgggaggctttacagaagaagcttagagagaaagttgtcaagtgtttcagtgactcgaacaaagctagattcagtagaattgataagaaggaattgattaaagaagacttgatcaattggttggtagcgcagaacagagaagatgatataccaaccgttgagaccttcaacaactttactacctacttcaccgggtttcatgagaatcgaaagaatatttactccaaggacgaccatgccacggctatatctttcaggctaatccacgagaatctacctaagttcttcgataacgttatctcatttaataaacttaaggaaggattccctgaactgaagtttgataaggttaaagaagatttagaagtcgactacgaccttaagcatgctttcgaaattgaatacttcgtcaacttcgtaacgcaggctggcattgaccaatacaattatttattaggtggaaagactttggaagacggtaccaagaaacaaggtatgaacgagcaaatcaatctgttcaagcaacaacaaacacgtgacaaggctagacaaataccgaaattgatcccactgttcaaacaaatactaagcgaaagaacggaaagccaaagctttattcccaagcaatttgaaagcgaccaagaattgtttgactctcttcagaagctgcataacaactgccaagataagtttacggtgttacaacaagcgatccttggtctcgctgaagctgatcttaagaaagtattcattaagacgtcagatttaaacgcactgtccaacactatatttggaaattactccgtattcagcgatgcattaaatctgtataaagaatcattaaagacaaagaaagcccaggaagcatttgagaagctacccgcccactccatacacgacctgatacaatatttagaacaattcaattcatcattggatgccgagaagcaacaatcaacagacacagtgttaaattatttcataaagaccgatgaattgtacagcagattcatcaagtctacctctgaagcatttacacaggttcaaccgctgttcgagctagaggctttgagttcaaagagaagaccaccagaatctgaagatgaaggagctaaaggtcaagaaggcttcgaacagattaagaggataaaggcttatttagataccctaatggaggccgtgcacttcgctaagccattgtacttggttaaaggtcgtaagatgatagaaggtttggataaggatcaatccttctatgaggcatttgaaatggcctaccaggaactagaatcgttaatcatacccatatataataaagctaggagctacctatctcgcaagccctttaaggccgataaattcaagatcaacttcgataataatacactccttagtggttgggacgctaacaaagaaactgcaaacgcaagtatattgttcaagaaagatggtctatactacttgggtattatgccgaagggaaagacgttcttgtttgattacttcgttagttccgaagatagtgagaagttaaagcaaaggagacagaagactgcagaagaagcacttgcacaggacggtgaatcttacttcgaaaagattaggtataagttgctgccgggtgcatcgaagatgctgcctaaggtcttcttctctaataagaacataggcttctataaccctagtgatgatatacttcggatcaggaacactgccagccacacaaagaacggaacaccacagaaaggtcatagcaaggtagaattcaatcttaatgattgtcataagatgatagatttctttaagtcatctattcagaaacacccagagtgggggtctttcggctttacattctccgatacttcagacttcgaagacatgtctgctttctaccgggaagttgagaaccaaggttatgtaatttcgttcgataagattaaggagacctatatacagtctcaggttgaacagggaaatttatacttgtttcagatatataataaggacttctcaccgtattccaaggggaaaccgaatctccacaccttatactggaaagcattatttgaagaggccaacctcaataacgtggttgctaagttgaacggagaagcggaaatattctttagacgtcactctattaaggccagcgataaggtagtacacccagccaaccaagcaattgacaacaagaacccgcatacagaaaagacacaatctacatttgaatatgacttggttaaagacaagaggtatacacaagataagtttttctttcatgtccctatctctctaaacttcaaagcccagggcgtaagtaagtttaatgacaaagttaatggtttcttgaaaggaaatccagacgttaatataattggtattgacagaggagaaagacacttgctatacttcacggtagttaatcagaaaggcgaaatcttagtccaagaatcattaaatactctcatgagcgataaaggtcatgtaaacgattaccagcagaagcttgataagaaagaacaagaaagagatgcagctagaaagtcctggactacggtggagaacattaaagaacttaaagaaggatacttatctcacgtagtgcataagctggcccatctcattatcaaatataatgcaattgtctgcctagaagatctaaacttcggatttaagagagggcggttcaaggtggagaagcaagtttaccagaagtttgagaaagctttaattgacaaattgaattatcttgtattcaaagagaaagaattaggtgaagtaggtcactacttgactgcttatcagcttaccgctcccttcgaatcattcaagaaattaggcaagcaatcaggcatcttgttctacgtacccgccgattatacatcgaagattgatccaactacaggcttcgtcaatttcttagacctgagatatcaatctgttgagaaggctaaacagttattgagtgatttcaatgctatcagatttaactctgtacagaattactttgaatttgaaatcgattacaagaaattgactcctaagcgcaaggttggtacgcaatctaagtgggtgatatgtacttacggagacgtcagatatcagaatagacgtaatcagaagggccactgggaaactgaagaagtaaatgtcaccgagaaattaaaggcattatttgcatcggattcgaagactacaactgtaatcgactacgcaaatgatgataacttgattgatgtcatcctggaacaagataaggcctcattctttaaagaattgctctggttattgaagttaacgatgacattaaggcactcaaagattaagtctgaagatgatttcatcttatcacccgtcaagaacgaacagggtgaattctacgatagtcgaaaggctggtgaagtctggcctaaagacgccgatgcaaacggtgcttatcatatcgccctcaagggactctggaatctccagcaaataaatcaatgggagaagggaaagacgcttaatttagctataaagaatcaggattggttctcgtttatccaagagaaaccatatcaagaataa

SEQ ID NO: 750 - DNA, 3897 bp, Artificial Sequence
  Description of Artificial Sequence: Synthetic polynucleotide
atgacaaagacgttcgattcagagttctttaacctatactcacttcagaagactgtacgcttcgaactcaaaccggttggtgaaactgccagctttgtggaagactttaagaacgagggcttgaagcgggttgtcagcgaagatgagcgtagagccgtagattatcagaaggttaaagagattattgacgattaccatagggacttcatagaagagagtttgaattatttcccagagcaagtgtctaaggatgccctagaacaggctttccatttgtaccagaaactgaaagctgcaaaggtggaggaacgggagaaagcattgaaagagtgggaagcattgcagaagaagcttagagagaaggtagttaaatgtttctctgatagtaacaaggctcgcttctcaagaattgacaagaaggagctgatcaaggaagatttaataaattggctggtagctcagaacagggaggatgatataccgactgtagaaacattcaataacttcacaacctactttactggattccatgagaacagaaagaacatttattctaaagatgaccatgccacggccatttccttccgtctaatccacgagaatcttccgaagttctttgataatgtaatatcatttaataaacttaaagagggatttccagaattaaagtttgataaggtcaaggaggacttggaagtggattacgatttgaagcatgcgttcgagatagaatacttcgtgaacttcgttacacaagccggcatcgatcaatacaattacctattgggtggaaagacattggaggacggaactaagaagcagggtatgaatgaacaaataaatctgtttaaacagcaacaaactagggataaggcgcggcagattcctaagttgattccgttgttcaagcaaatactgtctgaaaggactgaatcgcagtctttcattcccaaacagtttgaatcagatcaagaattatttgactcattacagaagttgcacaacaactgccaagataagtttacagtcttacaacaagcgatattaggtttggcagaggctgatcttaagaaagtatttattaagacgagtgatttaaatgccttatctaacactatctttggtaactactctgtattctcagatgcattaaatttatataaagagtcactcaagacgaagaaagcacaggaagcgttcgagaaattacctgctcactcaatccacgacttaatccaatacctggaacagttcaattcctcgcttgatgcagagaaacaacaatctacggatacggtattgaattatttcattaagacagatgagttatatagtagatttattaagtcaacatcagaggcctttacacaagttcaacccttgtttgaattggaggctctttcgagtaagcgaaggccaccagagtcagaagacgaaggtgccaaaggtcaggaaggtttcgagcaaattaaacgtatcaaggcctatctagatactctaatggaggccgttcatttcgccaaacctctgtatttagttaaagggcgcaagatgatagaaggattggacaaagatcaatcattctacgaagctttcgagatggcttaccaggaacttgaaagtcttattattccaatatataacaaggctagaagctatctttcacgtaagccatttaaggccgataaatttaagattaacttcgataacaacactttgctaagtggttgggatgcgaacaaggagaccgcgaatgcttccattctatttaagaaagatggactgtattatttaggtattatgcctaaaggaaagacattcttattcgactacttcgtttcttcggaggatagtgagaagcttaagcaaaggagacaaaagactgctgaagaggcattagcccaggatggtgaatcctacttcgagaagatcaggtacaagctgttaccgggtgcaagtaagatgctaccaaaggtctttttctctaataagaatatcggcttctacaatccgtcggatgatatattaaggattcggaacacagcctctcatacgaagaacgggacaccacagaagggccatagcaaggtagaatttaatttaaacgattgccacaagatgattgacttcttcaagtcttcgattcagaaacatcccgagtggggctcgttcggatttacattcagtgacaccagtgacttcgaagatatgtctgcattctacagagaagttgagaaccaaggttacgttatatcctttgataagatcaaggagacatacattcaatctcaagtggagcaaggaaatttatatctatttcaaatttacaacaaagatttctcaccatatagtaaaggaaagcccaatctgcataccctatactggaaggctctattcgaagaagcaaacttgaacaacgttgttgcgaagttaaatggtgaggcagaaatattctttcgccgtcactctattaaagcttcggacaaggtggtgcatcctgctaaccaagcgatagataataagaacccacatactgagaaaacacagagtacatttgaatatgatttagtcaaagataagaggtatacacaggacaagttcttctttcatgtcccaatctccttaaacttcaaagcccaaggtgttagcaaatttaatgacaaagttaatggcttcttgaagggcaaccctgatgtaaatattatagggattgatcgaggcgaaaggcatttactctatttcactgttgtgaatcagaaaggtgaaatccttgttcaagagtctttgaatacactaatgtccgataagggtcacgtcaacgattaccaacagaaattagataagaaggaacaagaaagggatgcagccaggaaatcgtggacaactgtggagaacatcaaggaacttaaagaaggctatctgagccatgttgttcataaattggcacatttgataattaaatataatgctattgtgtgcctcgaagaccttaacttcggatttaagagaggtcgtttcaaggtagagaaacaagtttatcagaagtttgagaaggctttaatcgataagttgaattacttggtcttcaaggagaaagaactaggcgaggtcggtcattatttaactgcttatcagctgactgcacccttcgaatcatttaagaaattgggtaaacaaagtggtattctgttctacgtgccagcggattacacgtcaaagatcgatccaacaacaggattcgtgaacttccttgatttgagatatcagagcgttgagaaagcgaagcagctattatccgacttcaacgctattagatttaactcagttcagaattatttcgaatttgagatcgattacaagaaattgactcctaagcggaaggtgggcacgcagtcgaagtgggtgatctgtacttacggtgacgtaagatatcagaacagaaggaatcagaaaggtcattgggaaactgaagaagttaatgtaaccgagaagttaaaggccttattcgcaagtgactccaagactacaacggtgatagattacgctaatgacgacaatcttattgatgttatccttgagcaagataaggcttcgttcttcaaagagttactatggttgctaaagcttactatgaccctgcgccattctaagatcaagtctgaagacgacttcatcctgtcaccggtaaagaacgaacaaggtgagttctatgattctaggaaagccggcgaagtatggccaaaggatgccgatgccaatggcgcgtatcatattgccttgaagggactatggaacttgcaacagataaaccaatgggagaaaggtaagacactaaacttggctataaagaatcaagattggttctcgtttattcaggagaagccttatcaggaataa

SEQ ID NO: 751 - DNA, 3897 bp, Artificial Sequence
  Description of Artificial Sequence: Synthetic polynucleotide
atgaccaagaccttcgatagcgaattctttaacttgtattcccttcagaagacagttagatttgaattgaaacctgttggtgaaacggcttcattcgtagaggattttaagaatgaaggccttaagcgagtcgtatctgaagacgaaagaagagctgtggactaccagaaggttaaagaaatcattgatgactaccatcgtgacttcattgaagaatcactgaattactttcccgaacaagtcagtaaggatgcgttagagcaagcattccatttatatcagaaattaaaggctgccaaagttgaagaacgcgagaaggcacttaaggaatgggaagccttgcagaagaagctaagggagaaggtagtcaaatgcttctcggattcaaacaaggctaggttctcccgtatcgacaagaaagaacttatcaaggaggatttgatcaattggttagtggcccagaaccgtgaagacgatatcccaaccgtcgaaacgttcaacaacttcactacctacttcacaggcttccatgagaatagaaagaacatttacagcaaagacgatcatgcgacagctatatcatttagattgattcatgagaaccttcccaagttctttgacaacgtcatttcctttaataagcttaaggagggatttcccgaattgaaattcgataaagtcaaggaagatctggaagtagattatgatttaaagcatgccttcgaaattgaatactttgttaatttcgtaacacaggcagggattgaccaatataactatttgttgggcggcaagactttagaggatggaacaaagaaacaaggtatgaatgaacaaattaacttattcaaacagcaacagactcgggataaggcaaggcaaattcctaagctaatcccactattcaaacaaattctctcggaaagaacagaatcccaatcctttatacctaagcaatttgagtccgaccaagagttattcgactccttgcagaaactgcacaacaactgccaagataaatttaccgtgttgcaacaagctattctcggccttgcagaagcagaccttaagaaagtgtttatcaagacaagcgatttgaatgcattatctaatactatctttggcaattatagtgtcttctctgatgcacttaatctgtacaaggaatcgttaaagacaaagaaagcacaggaggcctttgagaaactaccagcacactctatccatgaccttatccaatatctggagcaattcaattcgtctctggacgccgagaagcagcagtcaactgatacagttctcaattactttattaagaccgatgagttgtattctcgattcattaagagcacttctgaagcgtttacgcaagtgcaacctctatttgaacttgaggcattatcttcaaagcgtagacctcctgaaagtgaggacgaaggtgctaaaggtcaggaagggttcgagcaaattaagcgtattaaagcatatttagatacactgatggaagctgtacacttcgctaaaccactttatttggtcaaaggcagaaagatgattgagggtctagacaaggatcaaagtttctatgaagcgttcgagatggcctaccaagaattagaatcgttgattattccgatatataataaagctcgctcttatttgtctcgtaagccatttaaagctgataagttcaagattaactttgataacaacaccttactgtctggatgggatgcaaacaaagaaacggctaacgctagtatcctattcaagaaagacggattgtattacctgggtatcatgcctaaaggaaagaccttcttattcgattactttgtctcgagtgaagatagtgagaaacttaagcaacgcagacagaagacagctgaagaggctctagctcaagacggagaatcttacttcgagaagatcagatataaactgctacctggtgcaagtaagatgttgccgaaagtgttcttttccaacaagaacattgggttctataacccatcggatgatatcttgcgtatcagaaacacagcgtcacatacaaagaatggtacaccgcagaaaggtcactccaaagtggaatttaatttgaatgattgccacaagatgattgatttcttcaagtcctctatacagaaacatccagagtggggatcctttggattcacatttagcgacacaagtgatttcgaggacatgtctgcattctacagagaagtagagaaccaaggttatgtcatttctttcgataagattaaggaaacgtacattcagtctcaggtggaacaaggtaacctttatttgtttcagatatacaacaaggatttctctccttatagtaagggtaaaccgaatcttcatactctctattggaaagcattgttcgaggaggccaatcttaataatgttgttgctaagttaaatggagaggctgaaatcttttttagaagacatagcataaaggcatctgataaggtcgttcatcctgctaatcaggcgatagataacaagaatcctcatacggagaaaacacaatctacattcgagtatgatttagtaaaggacaagagatatactcaagataagttcttctttcatgtgcccataagcctaaacttcaaagcccagggtgtcagtaaatttaacgacaaagttaatggcttccttaaaggtaatcctgatgttaatatcattggaatcgaccgcggtgaaagacatttgttgtacttcacggtcgtcaatcagaaaggcgaaattcttgtacaggaatctttgaatacacttatgtcagataagggacatgtaaacgattaccagcagaagctagacaagaaggaacaggaacgcgatgctgctcggaagtcctggactacggtggagaatataaaggaattaaaggaagggtacttgtcacacgtcgttcacaaactagctcatttgatcataaagtacaatgctatcgtgtgtttagaggatttaaactttggatttaagagaggcaggttcaaagttgagaagcaagtttaccagaagtttgagaaggcacttattgacaaacttaattacttggtattcaaagagaaggagctgggagaagttggtcattatttgaccgcttatcaattaactgcacccttcgaatcgtttaagaaactgggtaaacaatcaggtatcctattctatgttccggcagattacacctccaagattgatccaacgactggtttcgtgaacttcctggatttgagataccagtcagtcgagaaagccaaacagctactctcagacttcaatgcaattaggtttaatagtgtacagaattactttgaatttgaaattgattacaagaagctaacgccaaagcgaaaggttggcacccaatccaaatgggtaatttgcacctacggagatgtgaggtatcagaacagaagaaaccagaaaggacattgggaaactgaagaagtaaatgtcaccgagaaactgaaggcattgttcgcaagcgattcaaagaccacgacagtcattgattacgcaaatgacgacaatctaatagatgtgatcctcgaacaagataaagcgagtttctttaaggaactcctgtggttactaaagttgacaatgacccttcgtcattcaaagattaagagcgaagacgactttatattatcaccggttaagaacgaacaaggtgagttctacgattcaaggaaggcaggagaggtgtggcccaaggacgccgacgcgaatggcgcttaccacattgctcttaaaggattatggaacttacagcaaatcaatcagtgggagaaggggaagaccttgaaccttgcaataaagaaccaggattggttctcgttcatccaggagaagccctaccaagaatag

SEQ ID NO: 752 - DNA, 3897 bp, Artificial Sequence
  Description of Artificial Sequence: Synthetic polynucleotide
atgaccaagactttcgatagtgagttcttcaacctatactccttacagaagactgttcggtttgaactaaagcccgtcggtgagacagcttccttcgtagaagacttcaagaatgaaggtcttaagcgagtggtctcagaagacgagcgacgggccgttgactatcagaaagtgaaggaaattattgatgattaccatagggactttatagaagaatctttaaattacttccctgaacaagtttctaaggacgcccttgagcaggctttccatctgtaccagaagttgaaggccgcgaaagtcgaagaacgggagaaagctcttaaagaatgggaggcgttacagaagaagttaagagagaaggttgtcaaatgcttctcagactccaacaaagcacgtttctctaggattgataagaaagaacttattaaggaagatctcattaattggcttgtcgcccagaatcgtgaagacgatataccaaccgtagaaacgtttaataacttcacaacttacttcactgggttccatgagaaccgtaagaatatttattctaaagatgatcacgcaaccgccatttcgtttagactgattcacgagaacttacctaagttctttgataacgttatttcctttaataaacttaaggaaggttttcctgaactcaagttcgacaaggtgaaggaagatttagaagttgattacgatttaaagcacgcgtttgaaatagaatacttcgttaactttgtgactcaagccggaattgaccaatataactacctgctgggtgggaagacgcttgaggatggaaccaagaaacaaggtatgaatgaacaaattaatctatttaaacagcaacagacgagagataaagcccgacagatacctaagcttatcccattgttcaagcaaattctttctgaacgcaccgagtcacaatccttcattcctaagcaatttgaatcagatcaagaattattcgattctctacagaagctacataataactgtcaagataaatttacagtgctccaacaagctatattaggactagccgaagcagatttaaagaaagtctttataaagactagtgatctaaatgcactgtcgaacacgatattcggtaactatagcgtctttagtgatgccctaaacttgtataaagaaagtttgaagaccaagaaagctcaagaagccttcgagaaactaccagctcattcaatccatgatttaatccagtacctagaacagttcaatagctctctagacgcggagaagcagcagtctacggacactgttcttaactatttcataaagaccgatgaactttactctcgtttcattaaatctactagtgaggccttcacacaagtgcaacctttgtttgagttggaagctcttagtagtaagaggcgtccaccagaatctgaagatgaaggtgccaaaggacaagaaggcttcgaacaaattaagcgtatcaaggcttacctggacactctaatggaagccgttcacttcgctaaacccttgtatttagtgaaaggtcggaagatgatcgaaggtttagacaaagatcaatcattctatgaagctttcgaaatggcctatcaggaactggagagcctaataattccaatctacaataaagctagaagctatttatctcgcaagccattcaaggccgataagttcaagataaatttcgataataataccttacttagtggttgggacgctaataaagaaactgctaatgcgtccattctgttcaagaaagatggtttgtattacctaggtattatgcccaaaggaaagacattcttatttgattacttcgtgtcgagtgaagattcagagaagctgaaacaacgtcgtcagaaaacagctgaagaagctcttgcgcaagatggtgaatcatacttcgagaaaatccgttataagctgctcccgggtgcgtcaaagatgttacctaaagtatttttctcaaataagaatattggcttctataatccatcagacgatatacttaggattcgaaatacggcgtcacatacaaagaatggtactccacagaagggtcatagcaaggtggaattcaacctgaatgattgtcataagatgatagacttcttcaaatcatcgatacagaaacatccagaatggggcagtttcggattcacattctctgatactagtgactttgaggacatgtcagccttctatagagaagtcgagaaccaaggttatgttatttcattcgataagataaaggagacctatatacaatcacaagtcgagcaaggtaatttatatctatttcaaatttataataaagatttcagtccttatagcaaaggtaagccaaatttacacaccctttattggaaggcattgttcgaagaagcaaatctgaataacgttgttgctaaattaaatggtgaagcagagatattcttccgacggcattccattaaagcgtcagacaaggttgttcaccctgcaaaccaagccattgacaataagaatccacacaccgagaagacccaatctacattcgaatacgacttagtcaaggataaacgttatacacaggataaatttttctttcatgttccgatctccctcaactttaaggcacaaggagtgtcgaagttcaacgacaaagtcaacggtttccttaagggcaacccagatgtcaacatcatcggaatagacagaggtgaaagacatttgctgtacttcactgtcgtgaaccagaaaggtgaaatcctagtgcaagaaagtttaaacactctaatgagtgacaaaggacatgtaaacgattaccaacagaagcttgataagaaagaacaagagagagatgccgcccggaaatcttggactactgtggagaatattaaggagttgaaggagggttacttgagtcatgtcgtgcataaattggctcatttaatcattaaatataatgcaatcgtatgtctcgaagatctgaactttggtttcaaacgtggacgatttaaagtcgagaagcaggtttatcagaaatttgagaaagccctaattgataaacttaactatttggtatttaaggagaaagagctaggtgaagttggccactatctcacagcttatcaattaacagcaccattcgaaagttttaagaaacttggtaaacaatctgggatcctattctacgttcctgctgactacacaagcaagattgatccaacgacaggtttcgtcaacttcttagatctgagataccaatctgtagagaaggctaagcaattactttctgacttcaacgctattaggttcaattcagttcagaactatttcgagttcgagattgactacaagaagttaactcccaagaggaaggtaggtactcaaagtaaatgggttatttgcacctatggcgacgttaggtaccagaatcggagaaatcagaaaggccattgggaaacagaagaagttaacgttaccgagaagctcaaagcattattcgcctctgactccaagaccacaacggttatagactatgccaatgacgataatctgattgacgttatcttagaacaagacaaggcttctttctttaaggaacttctttggctgctcaaactgactatgacattaagacattctaagatcaaatccgaagatgacttcatactgtctccggttaagaacgagcagggtgaattctatgatagtagaaaggctggtgaggtttggcccaaggatgctgacgctaacggtgcataccatatagcacttaagggattgtggaatttgcaacaaattaaccaatgggagaagggcaagacattgaaccttgcaattaagaaccaagattggtttagctttatccaggagaagccttaccaagaataa

SEQ ID NO: 753 - DNA, 3897 bp, Artificial Sequence
  Description of Artificial Sequence: Synthetic polynucleotide
atgaccaagaccttcgatagcgaattctttaatttgtattctctccagaagacagttagatttgaattaaagcctgtaggcgaaacagcaagctttgttgaagattttaagaatgaaggattgaagagagtagttagcgaggacgaaagaagagcagttgattatcagaaggtcaaggaaataattgacgactatcacagagacttcattgaagaatcattgaactactttcctgaacaagtctcgaaggatgctttggaacaagcatttcacttgtaccagaagctgaaggccgctaaggtggaagagagggagaaggcgctgaaggagtgggaagcattgcagaaaaaactacgtgagaaggtagtgaagtgcttcagcgacagtaataaagcacgattctctagaatagacaagaaagaactgattaaggaagatttgataaactggttagtagcgcagaacagggaagatgacattccaacagtggaaaccttcaataacttcacgacgtacttcacaggattccatgagaatcgaaagaatatctatagtaaggatgaccacgcaactgcgatctcgttcagactcattcacgagaacttaccaaagttctttgacaatgtcattagcttcaacaaattgaaggaaggatttccagaactgaaatttgataaagtcaaggaggatctggaagtggactatgacctgaaacatgctttcgaaattgaatatttcgtcaatttcgtcacccaagcaggtatcgaccaatataactatctcctcggtggtaagacgttggaagatggtactaagaaacaaggcatgaatgaacagataaacctattcaaacaacaacaaactagggacaaggctaggcaaatacctaagttaatcccattattcaaacaaatacttagtgaaagaacggaatcacagagcttcataccaaagcagtttgaaagcgatcaagaactgttcgactcattgcagaaattacacaacaattgccaagataagttcaccgtgttacagcaggctattctgggtttggcggaggcagatttaaagaaagtgttcatcaagactagtgatcttaatgccttgtctaacacaatcttcgggaattactcagtgttctcagatgccttgaatttatacaaggaaagtctcaagacaaagaaagcacaggaagccttcgagaaattgcccgcccattcaattcatgacctcatacaatatttggagcagtttaactcatccttagatgccgagaaacaacaatctacagacacagtattgaactactttatcaagactgatgaactctactcgagatttataaagtcaacatctgaagctttcactcaagttcagccactgttcgagttagaagcgttgtcctccaagaggagaccacctgaatcagaggacgaaggagctaagggccaagaaggcttcgagcagatcaagagaattaaggcttatctagatacattaatggaagctgttcacttcgctaagcctctatatctggttaaaggtaggaagatgatagaaggtctagataaagaccaatcattctatgaagcattcgaaatggcctaccaagaacttgaatctctaataattccaatatacaataaggcacgttcttatctttcaagaaagccattcaaggcggataagtttaagattaacttcgacaataacactttattgtccggctgggatgccaacaaggaaacagccaatgccagtatcttgttcaagaaggacggtttgtattacttgggaattatgcctaagggtaagacgttcttgttcgattactttgtcagttctgaggattcagagaagctaaagcaacgtaggcaaaagacagctgaagaagctttggcccaggatggtgagtcttacttcgagaagattcgttataagttattaccgggtgccagtaagatgttacctaaagtgttcttctctaacaagaatatcggcttctataatccgtcagacgacatccttcgtatccgtaatacagcttcgcataccaagaatggtacgcctcagaaaggacatagtaaggttgaatttaatctaaacgattgccataagatgattgacttctttaagtcgtccatacagaaacatccagagtgggggtcgttcggatttacattcagcgacacttctgacttcgaagacatgagtgctttctacagagaggtcgagaaccaaggttacgtaataagtttcgataagataaaggagacgtatatccagagccaagttgagcaaggcaacctatatttgtttcagatatataacaaagatttctctccatactccaaggggaagcctaacctgcacactctttactggaaagctttattcgaggaggctaatctcaacaatgttgttgctaaattgaacggtgaggctgaaattttctttagaagacattcaatcaaggcctctgataaagttgtgcatccagcaaatcaagccattgacaataagaacccacatacagagaaaactcaatccacatttgaatatgaccttgtcaaggacaagagatacacccaggacaagttcttctttcatgttcctatttctttaaacttcaaagctcaaggtgtctctaaattcaacgataaagtcaatggcttcttgaagggcaatcctgatgtgaatataatcggtatagatagaggagagaggcatttgttgtacttcacagttgttaaccagaaaggtgagatattggtacaggaaagtctaaatacattaatgtcggataaaggccatgttaatgattaccaacagaaattagataagaaagagcaagaacgggatgctgcgcgtaagtcttggaccaccgttgagaacattaaagaacttaaagaaggatacttgtcacatgtggtccataagttggctcatttgatcatcaagtataatgcgatcgtatgcctggaagatttaaacttcggtttcaagagaggaagattcaaggttgagaagcaagtttatcagaagtttgagaaagccctgattgataagttgaattatttagtatttaaggagaaagagctgggcgaggtgggtcattatctaacagcataccaattaactgctcccttcgaaagcttcaagaagttagggaaacaatcaggtattttattttacgtcccagctgattatacatccaagatagatcctaccacagggttcgtaaactttctagacctaagataccaaagtgtcgagaaggcaaagcaactgttaagtgatttcaatgccataagattcaattctgtccagaactacttcgagtttgaaatagactacaagaagctaacaccgaaacggaaagtaggcactcaatccaagtgggttatatgtacatatggagatgtgagatatcagaacagaagaaatcagaaggggcattgggagacagaagaggtaaatgttactgagaagttaaaggcgttattcgcatccgatagcaagacaacaacagtaattgattatgcgaacgatgataatctaatagatgtaatccttgaacaagataaagcttcattctttaaggaattattgtggttgttgaagttaacgatgacgttacgtcatagcaagattaagtcggaagatgacttcatcttaagtcccgtgaagaacgaacagggtgagttctatgattctagaaaggccggtgaagtttggcctaaggacgcagatgctaacggtgcctaccacattgctctaaagggtctttggaatttacaacaaataaaccaatgggagaaaggcaagactttgaacttggccataaagaatcaagactggttctcattcatccaagagaaaccttatcaagagtag

SEQ ID NO: 754 - DNA, 3897 bp, Artificial Sequence
  Description of Artificial Sequence: Synthetic polynucleotide
atgacaaagaccttcgattcagagttcttcaacttgtacagtttgcagaaaactgttcgatttgaactcaaaccagttggagagactgcatcctttgttgaagacttcaagaatgaagggctgaagcgggtagttagcgaagatgagcgccgtgctgtagattatcagaaagtcaaggagataatagatgattaccacagagatttcattgaagaatcccttaactactttccagaacaggtcagtaaagatgcattggaacaagcatttcatttgtaccagaaattaaaggcagctaaagttgaagaaagagagaaagccctaaaggaatgggaggccttacagaaaaaattgcgggagaaagttgttaaatgcttctccgactcaaacaaggcccgattctctcgtatcgataagaaggaacttattaaagaagatctaatcaactggttggttgcgcagaatcgtgaagacgatatcccaacagtagagacgttcaataacttcactacatacttcacaggtttccacgagaaccgtaagaatatatattcgaaagacgatcatgctactgctatctcctttcgtctaattcatgagaatttacctaagttcttcgataacgttataagctttaacaaattaaaggaaggctttccagaattaaagttcgataaggtcaaagaagatcttgaagttgattatgatttgaaacatgctttcgagatcgagtatttcgttaactttgtaacacaagctggtatagatcagtacaactacctgttgggaggtaagactctggaagatggtacgaagaaacaaggtatgaacgaacaaataaacttattcaaacaacaacaaactagagataaggcccgacagattccaaagcttattccgttgttcaaacaaatactgtctgaaaggactgaatctcaatcatttattccaaagcagtttgaatcggaccaagaattatttgacagcctccagaagttgcacaacaattgccaggataagttcacggtactgcaacaagcaattctcggcttagcagaagcagacttaaagaaggtattcataaagacaagtgatcttaatgctctaagtaatacaatatttggcaactacagtgtcttctcagatgcactcaacctgtacaaagaatcattaaagactaagaaagctcaagaggcattcgagaaattaccagcccactctattcatgatcttattcaataccttgaacaatttaactcatcactagacgcggagaaacaacaaagcactgatacagtgttgaattatttcataaagactgacgagttatattcaaggtttataaagtcaacatctgaagctttcacgcaggttcagccactcttcgaattagaagctctcagttcgaaacgaagaccacctgaatcagaagacgaaggtgcgaagggacaagaaggattcgaacaaatcaagagaatcaaggcttacttagatactttgatggaagctgttcatttcgccaagccattgtacctagttaagggtcggaagatgatcgagggtttggacaaggatcaaagtttctacgaagcattcgaaatggcctatcaagaacttgagtcattgatcattcctatatataataaggccaggtcataccttagcagaaagccgtttaaagctgataagttcaagattaacttcgataacaacaccttattatccggatgggatgcaaataaagaaaccgccaatgcatccatattatttaagaaagatggtttgtattatttaggcattatgcccaagggcaagaccttcttatttgactactttgtgagttctgaggattcggagaagttgaagcagcgaaggcagaagaccgccgaggaagctttggctcaagatggagagtcctatttcgagaagatcagatataaactattaccaggagccagtaagatgctccctaaggtcttcttcagcaacaagaatatagggttctacaatccttccgatgatatattgagaattcgtaatacagcatcgcatacgaagaacggcactccacagaaaggtcattccaaggtcgaattcaatcttaatgattgtcataagatgatcgacttcttcaaatcctctattcagaagcatcccgaatggggcagtttcggctttaccttctcagataccagcgacttcgaggatatgtcggccttctaccgtgaagttgagaaccaaggctatgtaatcagtttcgacaagatcaaagaaacctatatccaatctcaagtcgaacaaggtaatttgtatttatttcaaatctacaataaagacttctctccttactctaagggtaaaccgaatttacatacgttgtattggaaggcattgtttgaggaagctaatttaaataatgtggtggctaagttaaatggagaagcagaaatcttctttagaagacattctatcaaagcctcggataaagtggtacatcctgcaaaccaggcgattgataataagaacccacatacagagaagactcaaagtacctttgaatacgacttggttaaggataagcgttacacccaagacaaattcttcttccatgtacctatctccctaaactttaaggctcaaggtgtcagcaaatttaacgataaagtgaatggattcctaaagggaaatcctgatgtgaatatcatcggtattgatagaggagaaagacacctgttatacttcaccgtagtcaatcagaagggtgagattctagtacaagaatcgttaaatacactaatgtctgacaaaggtcatgtgaacgactatcaacagaaattggataagaaggaacaggaacgtgatgccgctcggaagtcgtggaccacagttgagaatatcaaggagctgaaagaaggctatttgagccatgttgtgcacaagctagctcatctaattattaaatataatgcgattgtttgtcttgaagaccttaatttcggctttaagagaggtagatttaaagtcgagaagcaagtgtaccagaagttcgagaaggccttgatcgataaattgaactacttagtatttaaagagaaagaattgggtgaagtcggccattatctaaccgcatatcaactaacagctccatttgagtctttcaagaaattaggaaagcaaagtggaattctattctatgttcctgccgactatacttcaaagatagaccctaccaccggtttcgtaaacttcttagatcttcgctatcaatctgttgagaaggcgaagcaattgctatctgacttcaatgcaattcgctttaactctgttcagaattacttcgaatttgagattgattataagaaattgactccaaagaggaaagttggtactcaaagtaagtgggtgatctgtacttacggagacgtgagatatcagaacaggcgcaatcagaaaggccattgggaaactgaggaagtcaatgttaccgagaagctcaaggccttatttgcttccgacagtaagaccacaaccgtgatagattacgctaatgatgataacttgatagatgtgatactcgaacaggataaggcctccttcttcaaggaattgttatggttgttgaagttaacaatgaccctgagacattccaagatcaagagcgaagatgacttcatcctgtcacctgtaaagaatgaacaaggagaattctacgactctaggaaagcgggtgaagtttggccaaaggacgctgatgccaatggtgcgtatcatattgctttgaaaggcttgtggaatttacaacaaatcaatcaatgggagaagggcaagactctcaacttggccataaagaatcaagattggtttagctttatccaagagaaaccatatcaggaataa

SEQ ID NO: 755 - DNA, 3897 bp, Artificial Sequence
  Description of Artificial Sequence: Synthetic polynucleotide
atgaccaagacgtttgactccgaattctttaatttatactccttgcaaaagactgtgcgctttgagcttaagccagtaggtgagactgcttcgtttgtagaagacttcaagaatgaaggtttgaagagggttgttagcgaagatgaacggagagcagttgactaccagaaagtcaaggaaattattgatgactatcatagagacttcatagaagaatctttgaactacttccctgaacaagtttcgaaggatgcattagaacaagcattccacttataccagaaacttaaggctgccaaggtagaggaaagagagaaagccttgaaagaatgggaggccctacagaaaaagttaagagagaaggtcgtcaagtgcttctcagatagcaacaaagctagattctctagaatagacaagaaagaactgattaaggaagatttgatcaactggctagtggcacagaacagggaagatgatatcccgactgttgaaacattcaacaatttcaccacttacttcactgggttccacgagaatagaaagaacatatattctaaagatgaccacgcgaccgctatctcgtttaggttaatacatgagaacctaccaaagttctttgacaatgtcatctcatttaataagctgaaagaaggatttccggaattgaaatttgataaggtcaaggaggatttagaagtggactacgacctgaagcatgcattcgaaattgagtacttcgttaacttcgtgacacaagcgggaattgatcaatataattacttgctaggtgggaagacattggaggatggtacgaagaaacaaggaatgaatgaacaaatcaatctattcaagcaacagcaaaccagagataaggctagacaaattcctaaactgataccattatttaagcagatcttgagcgagagaacagagtcgcaatctttcattcccaaacagttcgagtcagatcaggaactattcgacagtttgcagaaactacataataattgtcaagataagtttacagtgttacaacaggcaatattgggcttggcagaagctgatctaaagaaagtgtttataaagacatctgacttgaacgctctatcaaacacgatattcggtaactactccgtcttctccgatgccttgaatttatataaagagagcctgaagacaaagaaagcacaagaagcgtttgagaaactgcctgcccacagtatacatgatttaattcaatatcttgaacaattcaactcgtctctagacgctgagaaacagcaatccactgacacagttctgaattactttataaagacagacgagctgtattcacgtttcataaagtcaacctcagaagctttcacacaagtacaacctttgttcgaattggaagcgctgagctcaaagagaagaccgccagaatctgaggacgaaggtgctaaaggtcaggaaggcttcgaacagattaaacgcattaaagcttatttagataccctgatggaggcagtacacttcgccaagccattgtatttggtcaaaggacgtaagatgattgaaggtcttgacaaggatcaaagtttctacgaagctttcgagatggcgtatcaagagttagagtcgcttattatcccaatctataataaagcaaggtcctatttgagcagaaagcccttcaaggccgacaaatttaagattaatttcgataacaataccctacttagcggctgggatgctaacaaagaaacagctaatgcatcaatactatttaagaaagacggcttgtattacctaggcattatgcccaagggaaagacgttcttatttgattatttcgtttcttcagaagattcggagaaattgaaacagagacgacagaaaaccgctgaagaagcactcgcccaggacggtgaatcgtactttgaaaagatcaggtacaagttattaccaggagcctccaagatgttgccgaaagtctttttctcaaacaagaacatagggttctacaacccttcagatgatattctaagaatacgtaatactgcttctcacactaagaatgggacgccccagaagggccattccaaggttgagttcaacttgaatgattgtcataagatgatagatttctttaagtcaagtatacagaaacatccagaatggggttcatttggatttaccttctcagatacttccgacttcgaggatatgtcagctttctatcgtgaggttgagaatcagggttacgttatctcatttgacaagattaaggaaacttatattcaaagccaggttgaacaaggcaacctctacttatttcaaatctacaataaggacttcagcccttactctaaaggtaaacccaatctacacaccttgtattggaaggcattgtttgaggaggctaatcttaataatgttgttgcaaagttgaatggtgaagccgaaatattctttagaaggcattccatcaaggcttcagataaagtcgtacatccggctaatcaagctatagataataagaatcctcacacagagaaaactcagagcacatttgagtatgatttagtcaaggacaagcgttatactcaagataaattcttctttcatgtaccaattagtcttaacttcaaggctcagggcgtcagcaaatttaacgataaggtaaacgggttcttgaaaggcaatccagatgttaatattatcggtatagaccgaggagaacggcatttactatacttcactgttgtgaatcagaagggagaaatactggtgcaagaatctttgaacactcttatgagcgataagggacacgtgaatgactatcaacagaaattggacaagaaagaacaagaaagagacgcagcgagaaagagttggactactgttgagaacatcaaggaactaaaggagggttatttgtcacacgtagtccataaacttgcacatttaattattaagtataacgctatcgtctgcttggaggatctcaacttcggatttaagagagggagattcaaagtagagaagcaggtttatcagaaattcgagaaggcattaattgataagttgaattacttagtcttcaaagagaaggaactgggtgaagtcgggcactatcttaccgcttatcagctaacagcgccattcgagtctttcaagaaattgggtaaacaatctggtatactattctacgttcctgctgactacaccagtaagatcgatccgactactgggttcgtcaactttctagatttgagataccaatcagtagagaaggctaaacaactattgtctgacttcaacgccattagatttaatagtgtacagaattactttgaatttgagattgattataagaaactcactcccaagcgtaaagttggaactcaatctaaatgggtgatttgtacatatggtgatgttcgttatcagaacagaaggaatcagaaaggtcactgggaaaccgaagaagtaaatgtcactgagaagttgaaagcattatttgcgtcagattctaagactaccactgttatcgattatgcaaatgatgataatttgatcgatgttatattggagcaagataaagcgagcttcttcaaagaattgctttggcttcttaagctaacgatgactttaagacatagcaagatcaagtctgaggacgacttcatactaagcccagttaagaacgaacaaggagagttctatgatagtcgtaaggcaggtgaggtctggcccaaagacgctgatgctaatggagcttatcatattgctcttaagggattatggaatcttcagcaaattaaccaatgggagaagggtaagacattaaatcttgctataaagaatcaagattggttctcgtttattcaggagaaaccttaccaagagtag

SEQ ID NO: 756 - DNA, 3897 bp, Artificial Sequence
  Description of Artificial Sequence: Synthetic polynucleotide
atgacgaagacctttgatagtgaattctttaatttatactcgttgcagaagactgtgagattcgagttaaagccagtcggcgagacagcttcattcgttgaagacttcaagaacgaaggcctcaaacgggtagttagcgaagacgaaagaagagctgttgactatcagaaggttaaagagattatagacgactatcatagagacttcattgaggaaagtctaaattactttcctgaacaagtatccaaagatgcattagagcaagcattccatctataccagaaattgaaggccgccaaggtcgaagagagagagaaggcattgaaagagtgggaagccttacaaaagaaattaagagagaaggttgttaagtgcttcagtgacagcaataaggccaggttctcgagaattgacaagaaggagttgatcaaagaagatttgataaattggctcgttgcacagaatcgagaagatgatattccgacagttgagacctttaataactttacaacctactttaccggattccatgagaaccgcaagaatatatattctaaggatgatcatgcaacagcgatatctttcaggcttatccacgagaacctgcctaagttctttgataacgttatatcattcaataaattgaaggaaggttttccggaattgaagtttgataaggtcaaagaagatttggaggtggattacgacttaaagcacgcatttgagattgaatacttcgtaaacttcgtgactcaagcgggaattgatcaatacaattatctactcggtggtaagacattagaagatggtactaagaaacaaggtatgaatgaacagatcaatctattcaagcaacaacagacccgagataaggctagacaaattccaaagctaatccctctattcaaacagatactcagtgaaagaaccgaaagccaatctttcattccgaaacaatttgaatcagaccaagaattgtttgattcattgcagaaattacataacaattgccaagataaattcaccgttctccaacaggcaatattaggcctagctgaggccgacttaaagaaagtatttatcaagacatccgatctgaatgccctgtctaacacaatatttgggaattacagtgtattctccgacgcgttgaacctatataaagaatccttaaagacaaagaaagcacaagaagctttcgagaagttgccagctcatagtattcatgacttgattcaatatttggaacaattcaattcatctctggacgccgagaagcaacaatcaactgatactgttcttaactacttcataaagacggatgagttgtactcgagattcattaaatcgacctccgaggcattcactcaagtgcagcccttgtttgaactggaagcactatcaagcaagaggcgccctcccgagtcggaagacgaaggtgctaaaggtcaagagggtttcgaacagataaagagaatcaaagcttacctggatacccttatggaagcagttcatttcgctaaacctctatacctagttaagggacgcaagatgatcgaaggattggacaaggaccagtcattctatgaggcgtttgaaatggcttaccaagaactggaatcacttatcattcctatttataacaaagcgagatcctatctatcacgtaaaccctttaaagccgataagtttaagattaactttgacaacaatacattattaagcggttgggatgctaataaggaaaccgcaaacgcttccatcctattcaagaaagatggtctttactatttgggcattatgcctaagggaaagaccttcttattcgactactttgtttcttcagaagattcagagaagcttaagcagagaaggcaaaagacggcggaagaagcattagcgcaagacggagaatcatacttcgagaagatccgttataagttactaccaggtgcctccaagatgttgccgaaggttttcttttcgaataagaatataggtttctataatccatctgacgatatcttgcgaattaggaacactgcctcccacacgaagaatggtactccacagaagggacactctaaggttgaattcaacttgaatgattgtcacaagatgatcgacttcttcaagtcctcgatccagaaacatcctgagtggggcagtttcggatttacattctctgacacttctgatttcgaagatatgtccgccttctatagagaagttgagaatcaaggttacgttatttcattcgataagataaaggaaacttatattcaatctcaggtcgagcaaggcaacttgtatctattccaaatttataacaaagatttcagcccttattctaagggcaagccaaatttacatacactatattggaaagcattattcgaagaggcgaacttgaataacgttgtcgctaagttgaatggtgaggccgaaattttctttagaaggcattccatcaaggcttctgacaaggttgttcatcctgcaaatcaagcaattgataataagaaccctcacaccgagaagacccaatcgacctttgaatatgacctagttaaagataaacggtatacccaggataagttcttctttcatgtaccaatttcactcaatttcaaagctcaaggtgtgtcgaagttcaacgacaaggtcaacggcttcttgaaaggtaatcctgatgttaatatcataggaatagatagaggtgaaagacatttgctatactttactgtcgtcaaccagaaaggtgaaatactggtgcaggaatcattaaatactttaatgtccgacaaaggtcatgttaatgattatcaacagaagctggacaagaaggaacaagaaagagatgcagctagaaagtcgtggacgaccgttgagaatattaaggaattgaaggaaggttacctttcacatgtagtccataagttagctcacttaattataaagtacaacgccattgtatgcttggaagatcttaacttcgggttcaagagaggtagattcaaagttgagaaacaagtttaccagaaatttgagaaggcattgattgacaaactaaactatctggtcttcaaagagaaagaactgggcgaggtagggcattatttgactgcttatcaactaaccgctccgttcgaatcctttaagaagctaggtaaacaatcaggcatattattctatgttccagcagattatacatcgaagatagacccaactactggcttcgttaatttcttggatttacgataccagtccgtagagaaggctaagcagctgctatcagactttaatgctattaggtttaattcggtccagaattacttcgaatttgaaatcgattacaagaaactgactcctaagcgcaaggtaggtactcaaagtaaatgggttatctgtacttacggtgatgtgaggtatcagaacagacgaaatcagaagggtcattgggagactgaggaagtcaacgttactgagaaattgaaagccctgtttgcttctgattcaaagaccacaactgttatagattatgcaaatgatgataatttaattgatgtaatactggaacaagataaggcctccttctttaaagaattgttgtggttactgaagcttacgatgaccctaagacactccaagattaagtcagaagatgactttatactatcacctgttaagaatgagcaaggtgagttctatgattcacgcaaagctggtgaagtttggcctaaggacgctgatgccaacggcgcttatcatatcgctttaaagggcctatggaacttacagcaaattaatcagtgggagaaaggcaagacgctaaacctcgcgatcaagaaccaagattggttcagtttcatccaagagaaaccctatcaagaatga

SEQ ID NO: 757 - DNA, 3897 bp, Artificial Sequence
  Description of Artificial Sequence: Synthetic polynucleotide
atgacaaagaccttcgattcagaattctttaatctatactccttacagaaaacagttaggtttgagcttaaacccgttggcgaaaccgcatcgtttgttgaagacttcaagaatgaaggtctaaagagagttgtgtcggaggatgaaaggagagcagttgattatcagaaggtaaaggaaattattgatgactatcatcgtgacttcatcgaagaatctttaaattacttcccagaacaagttagcaaggatgccttggagcaagcgttccatttgtaccagaagttgaaggcagctaaagttgaagaacgagagaaagcgctaaaggaatgggaagctttgcagaagaagttaagagagaaggttgtcaaatgcttctctgattctaataaagctcggttctctcgcatagacaagaaggaactcattaaagaagacctaatcaactggttagtcgcccagaacagagaggatgatattcctaccgtggaaacgttcaataatttcaccacatacttcaccggcttccacgagaaccgcaagaatatttactccaaagatgatcatgctaccgctatcagcttcagattaattcatgagaacttgcctaaattcttcgataatgttatatcattcaataagttgaaagaaggattcccagagttgaaatttgacaaagtcaaggaagacttggaagttgactacgatctaaagcatgctttcgaaatagaatacttcgtaaatttcgtcacccaagctggtattgaccaatacaactatttattgggcggcaagacattagaagacggtacgaagaagcaagggatgaacgaacaaattaatttattcaaacaacaacaaacccgtgacaaggccagacaaattccaaagctaatacccttattcaaacagatcttgtccgaaagaaccgaatcacagtcgtttattcccaagcagttcgagtccgatcaagaactattcgacagtctccagaaattgcacaacaattgtcaagataagtttactgtgttacaacaagcaatccttggtttggccgaagcagatctgaagaaggtatttattaagacttccgatttaaacgctctctctaacactatattcggtaattactctgttttctctgacgcgttaaatctgtacaaagagtctttaaagaccaagaaagctcaagaggccttcgagaagcttccagctcattctattcatgacctcatccaatatctcgagcaatttaattcgtccttggatgctgagaagcagcaaagcaccgacaccgtgttaaattacttcattaagacagacgagttgtactcgagatttatcaagtcaacgtctgaagcgtttacacaggtccaaccattatttgagttagaagctttatcttccaaacgccggccgcccgagagcgaagatgaaggtgctaagggccaagagggattcgaacagattaaacgcatcaaggcttatctagatacactgatggaagcagttcacttcgctaagccactttatttagtcaagggcaggaagatgatagaaggcttggacaaagatcaatcgttctatgaagctttcgaaatggcctaccaagagttggagtcactaattattccaatctacaacaaagctaggtcctatttgtccaggaaaccattcaaagctgataaattcaagatcaactttgataacaacaccttactaagtggttgggatgccaacaaagaaacggcaaatgctagcattctgtttaagaaagatggcttatattacttaggtataatgcccaaaggaaagacgttcctatttgactactttgtatcttcagaagattcagagaaactcaaacagagaagacagaagactgcggaagaagcacttgcccaagatggtgagagctactttgagaagataagatataaacttctacctggcgccagtaagatgttgcccaaggtctttttctcaaacaagaacatcgggttctacaacccttccgatgatattctgcgaattagaaacaccgcatcccatacaaagaacggaactcctcagaaaggtcactctaaagttgaatttaaccttaacgactgccacaagatgatagatttctttaagtcttctatacagaaacatccggaatggggctcctttggatttaccttcagtgatacgtccgacttcgaagacatgtctgcgttctatagagaagtcgagaaccagggatacgtcattagcttcgataagataaaggagacttatattcaatcccaagtggaacaaggtaatctatatttattccagatttataacaaggatttcagcccgtactcgaagggtaaacccaatttgcataccttgtattggaaggcattgtttgaagaagccaatcttaataacgttgtcgcaaagttaaacggtgaagccgagatattctttagaagacattcgatcaaggccagtgataaggtagtccacccagctaaccaagcgattgataataagaatcctcatacggagaagacgcaaagcacatttgaatacgatcttgttaaagacaagcggtacactcaagacaagttcttcttccatgtaccaatttctctgaactttaaagctcaaggagtaagtaaatttaatgataaggtaaacggcttcttgaaaggaaacccagatgttaacattatcggtatcgatcgtggcgaaagacatctactctacttcacagttgttaaccagaagggtgaaatactcgtacaagaatcgttgaatacattgatgagcgataaagggcatgtaaatgattatcagcagaaattagacaagaaagaacaagagagggacgccgccagaaagtcctggacaacagttgagaatattaaagaactcaaggaaggttatctgtcgcatgtagtccataagcttgcgcatctaattattaagtacaacgcaatagtttgtttggaggatttgaacttcggattcaagcgaggccgtttcaaggttgagaaacaagtctaccagaagtttgagaaagccttaattgataagctaaattacttggtatttaaagagaaggaattgggtgaggtcggtcactacttgacagcttaccaattgacggctcccttcgaatcatttaagaaactagggaagcaatccggtatcttgttctatgttcccgcagattatactagtaagatcgatcctacgactggatttgtaaactttctggacttgagatatcagagcgtggagaaagccaagcaattattgagtgatttcaacgctataaggtttaattctgttcagaattacttcgagtttgaaattgactacaagaaattgacgcccaagcgtaaggttggtacacaaagtaagtgggttatctgtacatatggtgacgttaggtatcagaatcgtaggaatcagaagggccattgggaaacggaggaagtgaatgtcaccgagaaattaaaggctttgtttgcatcggactcaaagactaccacagttatcgactatgctaatgacgataacttgatcgacgtcatccttgaacaagataaggctagcttcttcaaggagttactatggctccttaagcttacaatgacattaagacatagcaagattaagtcagaggatgacttcatcctgtcgcctgtcaagaacgagcaaggcgaattctacgactcacgtaaggctggcgaagtgtggcctaaggatgctgatgccaacggcgcgtaccacattgctttaaagggtttgtggaatctgcaacaaattaatcaatgggagaaaggaaagactttaaacctagccattaagaaccaggattggttctcattcattcaggagaagccatatcaagaataa

SEQ ID NO: 758 - DNA, 3897 bp, Artificial Sequence
  Description of Artificial Sequence: Synthetic polynucleotide
atgacaaagacgttcgactctgagttctttaacctctactccctccagaaaactgtgagatttgaactcaagccagtaggtgaaactgcttcatttgtagaagatttcaagaatgaaggtctaaagagggtagttagcgaggatgaaaggagagctgtcgattatcagaaggttaaggaaattattgatgattatcaccgcgacttcattgaagaaagtcttaactactttccggagcaagtatccaaggacgcattagagcaggcgtttcatttatatcagaagttgaaggcagctaaggtcgaggaaagagagaaggcgttaaaggaatgggaagctcttcaaaagaaactaagagagaaagttgtgaagtgcttcagcgactcgaacaaagccagatttagtcgaatagataagaaagaattgataaaggaggatttgattaattggttagttgcacagaacagagaagacgacattccaactgtcgaaaccttcaataacttcaccacttacttcacgggattccatgagaacagaaagaatatttattctaaggatgaccacgccacggcaatttccttcaggctaatccacgagaacctgcctaagttcttcgataacgtaataagcttcaacaagttgaaagagggtttccctgaattgaagttcgataaggtgaaggaagacttggaggtcgactacgatctaaagcatgctttcgaaatagagtacttcgtaaacttcgtaacccaagccggaattgatcagtataactatttgttaggtggaaagacattagaagatggtactaagaagcagggtatgaacgaacaaataaacttgttcaaacaacaacagacgagggataaagccagacaaatacctaagttgattccattgttcaaacaaatcttgtcagaaagaacggaatctcaatcgttcatcccgaagcaattcgaatcagaccaagagctgtttgattctctacagaagcttcacaataattgtcaagataaattcactgtgcttcaacaagcgatcttagggctagctgaagccgatcttaagaaagtcttcattaagacctcggatttgaatgcactttccaatacaatattcggtaactacagtgtgttctctgatgcattaaatctatataaagaatctttaaagaccaagaaagctcaggaagccttcgagaagcttccagcgcattccattcatgacctaatacaatatcttgagcagtttaattcatcactggatgcagagaagcagcaaagtactgacacggtactgaattactttataaagacggatgagttatattctagatttattaaatctacttcagaagcgtttactcaggtacaacctttattcgagttggaagctttgagtagcaagagaagaccacctgagagcgaagatgagggcgctaaaggacaagaaggcttcgagcaaattaagagaattaaggcatatttggatactcttatggaggctgtccacttcgcaaagcctttatacctggtcaaaggacgaaagatgattgaaggtttggacaaggatcaaagtttctacgaagcctttgaaatggcatatcaggaactagaatccctcataattcctatttataacaaagcccgtagctacttgtctaggaagccgttcaaggccgataaattcaagataaatttcgacaacaataccctcctttcgggctgggatgctaataaagagacagcgaatgcttccatactgttcaagaaagatggtttatattacctcgggattatgccgaagggtaagacattcttgtttgactacttcgtatccagcgaagattcagagaaattgaaacaacgtaggcagaaaactgctgaagaagccttggcacaagatggagaaagctacttcgagaagattcgttacaagttgctacctggcgcttccaagatgctcccgaaggtattctttagtaataagaatatcgggttctataatccttctgacgacattctaagaatcagaaatacagcctcccatactaagaatggtactccacagaaaggtcattcgaaggtcgaatttaatttaaatgattgtcacaagatgatagacttctttaagtcttccatacagaagcacccagaatggggctccttcggattcacgttctccgacacttcggacttcgaggacatgagtgctttctatcgtgaagtcgagaaccagggctacgttatatccttcgataagattaaagaaacttatattcaaagtcaggttgaacaaggtaacctttatctatttcaaatttataataaagacttctctccctattcgaaaggtaaaccaaacctgcatactctttattggaaagccttgtttgaagaagctaacctgaataacgttgtagcgaagttaaacggcgaagctgaaatattcttccggagacatagtatcaaagcctctgataaagtagtccatcccgctaatcaagctattgataacaagaatccacatactgagaaaactcaatcaacattcgaatatgatctggttaaagataaacggtatactcaagacaagttcttctttcacgttcctatttcattaaacttcaaggctcagggagtttctaagttcaatgataaggtaaatggtttcttgaaaggcaacccagatgttaacattattggtatcgatagaggagaaagacatctactctacttcactgttgttaatcagaagggtgaaatcctggtacaagaatcattgaacacgctaatgtcggataagggtcatgtcaatgactaccagcagaaactagacaagaaagaacaggaaagggacgctgcgagaaagagttggacaaccgtcgagaatattaaggaattgaaagagggataccttagtcatgtcgttcacaaattagctcacttaataattaagtataacgccatcgtttgtttagaggatttaaatttcggctttaagcgcgggaggttcaaagttgagaaacaagtttatcagaaatttgagaaggcattaatcgacaaattgaactacttagtgtttaaggagaaagaattgggcgaggttggtcactacctaacggcctatcaattaacagcacccttcgaatcattcaagaaattgggaaagcaatccggtattctattctatgtcccagctgattatacatcaaagattgatccaacgacagggttcgtaaactttctggatcttcggtatcaatccgtagagaaagccaagcaactcttgtcagatttcaacgcaattcgatttaattcagtgcagaactacttcgagttcgaaatagactacaagaaactcacgcctaaacgtaaagtcggaactcaatcgaaatgggtgatatgcacatatggtgatgttaggtaccagaatagaagaaatcagaaaggtcactgggaaacagaagaagttaacgttactgagaaattgaaggctttgtttgcatcggactccaagacgaccactgtaattgattatgcgaatgacgataatttaatcgatgtcattctcgaacaggataaggcttctttctttaaagaactattgtggttgctcaagctaacaatgaccctaagacattcgaagattaagtctgaggacgacttcatcttaagtccagtcaagaacgagcaaggtgagttctatgattctaggaaggctggcgaggtttggcctaaggatgctgacgcaaatggagcatatcatattgccttgaaaggtttatggaatctacagcaaataaatcagtgggagaaagggaagactttaaacttggccataaagaaccaagactggttctcatttattcaagagaaaccttaccaggaatag

SEQ ID NO: 759 - DNA, 3897 bp, Artificial Sequence
  Description of Artificial Sequence: Synthetic polynucleotide
atgaccaagacattcgattcggagttcttcaatttatatagcctacagaaaaccgtgagatttgaacttaaaccggttggtgagaccgcatcattcgtcgaggactttaagaacgaaggtctgaagagggttgtaagcgaggatgaaagaagggctgttgactatcagaaggtcaaagagataatcgatgattaccatagagacttcatcgaagaaagcctcaattactttccagaacaagtttctaaagacgccttggaacaagcctttcatctgtaccagaaactgaaagcagcgaaagttgaggaacgagagaaggctttgaaggaatgggaagcattgcaaaagaaattaagagagaaggtcgtcaaatgtttctcggactcaaataaagcaaggttctctcgtatagataagaaggagctaataaaggaagacctaataaattggttggttgcacagaatagggaagacgatatacctactgtcgaaacatttaacaacttcactacttatttcacgggattccatgagaataggaagaacatttattccaaggatgatcatgcgactgctatcagcttcaggttgattcacgagaatttaccaaagttctttgataatgtaatctcgttcaataaattaaaggaaggcttcccagaactcaaattcgataaggtcaaagaagatttagaagtcgattacgaccttaaacatgcatttgaaattgaatactttgtgaacttcgtcacccaagctgggattgatcaatacaattatttattgggaggcaagactttggaagatggtactaagaaacagggcatgaatgaacaaattaatctatttaaacaacagcaaactagagataaggctaggcagataccgaaattaataccattattcaagcaaatactttcagaaagaacagaaagccagtctttcataccaaagcagtttgaaagcgatcaagaactgtttgatagtttgcagaaactacacaacaactgccaagataaattcaccgttctacagcaggctatcctgggcttggcagaagcagacttaaagaaggtcttcataaagacgagcgatctcaacgccctatcgaatacaatcttcggtaactattctgtattcagtgacgccctgaatctgtataaagaatccctcaagacgaagaaggcacaagaagcattcgagaagctaccagcacattccattcacgatttaatccaatacctggagcaatttaactcatcacttgatgctgagaaacaacagagtacagatacagtcctaaattactttatcaagacagacgaattgtactctagatttataaagtctactagcgaagctttcacgcaggttcaaccattgtttgagttagaagcactatcatctaagcgaagacctccagaatccgaagatgaaggtgctaaaggtcaagaagggttcgaacaaatcaagcgaataaaggcatatctagataccttgatggaggccgtacacttcgctaagccgctttatctggtaaagggcaggaagatgatagagggtttggataaggatcagagtttctacgaagcatttgaaatggcttatcaggaactggaatcactcatcattccaatctataataaggccagatcatatttatcacgaaagccctttaaggctgataaattcaagattaatttcgacaataacacgctattatcaggttgggatgcaaataaagaaaccgcgaacgctagtatcttgtttaagaaagatggtctgtattacttaggtataatgccaaagggtaagactttcttgtttgattacttcgtaagtagtgaagactctgagaaactaaagcaaagacgtcagaagactgcagaggaagcgctagcacaagacggtgaaagctacttcgagaagattcgttataagctgcttcctggtgcgagcaagatgttgcctaaagtcttcttctccaacaagaatatcgggttctataatcccagcgacgacatactgcgaatcagaaacaccgcatcacatacaaagaatggaacaccgcagaaaggtcattcaaaggttgaatttaacttaaatgattgtcacaagatgattgacttctttaaatcttctattcagaaacacccagagtggggatcgtttgggttcacgttctcagatacctctgatttcgaggacatgtccgccttctatcgggaagtggagaaccaaggttacgttatatcattcgataagatcaaggagacctatatacaatcccaagtcgaacagggcaacctttatttattccaaatttataacaaagacttcagcccctactcgaagggtaagccaaaccttcataccttgtactggaaagctctattcgaggaagctaacttgaataatgtggttgccaagttgaacggagaggccgaaatattctttcgtagacacagtattaaagcttcagacaaggttgtgcacccagccaaccaggcaattgataacaagaatcctcacaccgagaaaacacagtccactttcgaatatgatcttgtcaaggacaagcgatacacccaggataaatttttctttcacgttccaatctctcttaacttcaaggcgcagggtgtttcgaagttcaacgataaagtcaatggattcttgaaaggaaatcctgacgtgaacattattggtattgatcgaggcgaacgtcacttgttatatttcaccgttgttaatcagaaaggtgaaatcctagttcaagaatctctcaacaccctaatgtctgataaaggtcacgttaatgattatcaacagaagctagataagaaagaacaagaacgagatgccgcgcgaaagtcgtggaccactgtagagaatatcaaggaattgaaagaagggtacctttcacatgttgtgcacaagttagcccacttaattatcaagtacaatgctattgtatgcttagaagacttaaacttcggatttaagcgcggaagatttaaagtggagaagcaggtgtatcagaaatttgagaaggcattaatagacaaattgaactatttagtctttaaggagaaggaacttggtgaagtaggtcattacttaacagcctatcaactgacagcacccttcgaatctttcaagaaattgggcaagcaatctggtatacttttctatgtaccagcagactatacttcgaagattgatccgacaactggtttcgttaacttcctagacttgcgatatcaaagtgttgagaaagctaaacaattattatctgatttcaacgctattcgctttaattctgtccagaactatttcgagttcgaaattgattacaagaaactaacaccgaagaggaaagttggcacgcaatcaaagtgggttatttgtacatatggtgatgtaaggtaccagaatcgaagaaatcagaaaggccattgggaaaccgaagaagttaatgttactgagaagcttaaagcattgtttgctagtgacagtaagacaacaacagttatcgattatgcaaatgatgataatctcattgatgttatattggagcaagataaggcgtctttcttcaaagaattgctttggctacttaaattaactatgacattgagacatagtaagattaagtctgaagatgacttcatcctgagccccgtgaagaacgaacaaggcgagttctatgactcgaggaaggccggtgaagtatggcctaaagacgcagacgcgaatggcgcttatcacattgccttaaagggcttatggaatttacaacaaatcaaccaatgggagaagggcaagactctaaacttggcgattaagaatcaagattggttctcgttcatacaagagaagccataccaggaataa

SEQ ID NO: 760 - DNA, 3897 bp, Artificial Sequence
  Description of Artificial Sequence: Synthetic polynucleotide
atgacgaagacattcgatagtgagttcttcaatctctattccctacaaaagactgttagattcgaactaaagccagtgggcgaaactgcctcattcgtcgaggacttcaagaacgaaggtctcaagagagtcgtttccgaggacgaacgcagagcggtcgactaccagaaggtcaaagaaattattgatgattatcacagagacttcatcgaagaatcattgaattacttccctgaacaagtcagcaaagatgcactggaacaagcgtttcacttatatcagaaactgaaggcagccaaggtcgaggagagagagaaggctttgaaggaatgggaagcattacagaagaagttgagggagaaagtcgtgaaatgcttctccgattctaacaaagctcgcttcagcaggatcgacaagaaagaattgataaaggaggatttaattaactggttggtcgctcagaatcgtgaggatgatattcccacagtggaaaccttcaacaatttcacaacttactttaccggtttccacgagaatcgtaagaacatttactccaaagatgatcacgctaccgctatatcatttaggttgatccatgagaatctacctaagttctttgacaatgttatatcattcaacaagttgaaggaagggttcccagaactgaaatttgacaaggttaaagaagatttagaagtggactacgatctcaagcatgcgttcgaaatcgaatactttgtgaactttgttactcaggccggtattgaccaatataactatctgttgggtgggaagactctggaagatggaacgaagaaacaaggtatgaacgaacaaatcaatctctttaaacaacaacagacccgtgataaagccagacagattccaaagcttattccgctcttcaagcaaattctttcagaacgtacagagtcccagtcattcattcctaagcagtttgaatcggatcaagaattattcgatagtttacagaaactgcataataattgtcaggacaagttcactgtactgcaacaagcgattctagggctggctgaagccgatctgaagaaagtgttcatcaagacttccgatcttaatgcattgagcaataccatatttggtaactattcagtcttcagtgatgctctaaatttgtataaagagtcgctaaagacaaagaaagcacaagaggcattcgagaagctcccggcacatagtatccatgatctcatccaatatcttgaacagtttaactcatctttggatgcagagaagcaacaatcaaccgatactgtcttaaactatttcataaagacagatgaattgtatagccgatttataaagtccacttcagaagctttcactcaggtacagccactatttgaattggaagctctgtcttctaaacgaagaccgccagaaagtgaagatgaaggtgctaagggacaagaaggattcgagcaaataaagagaattaaagcatatttggatacactgatggaggcggtacactttgcgaagccattgtacttggtaaagggtcgtaagatgattgaaggcttagataaagatcaaagcttctacgaagcattcgaaatggcgtatcaagagttggaatcgctgattataccgatttataataaggccaggtcttatttgtctcgaaagccatttaaagccgacaaattcaagattaacttcgataataacactttgttatcaggttgggatgcaaacaaagagactgctaatgctagtatcttatttaagaaagacggtctttactatttgggtattatgcccaagggtaagactttcttatttgactacttcgtgtcctctgaagattctgagaagctgaaacaacggagacaaaagactgctgaggaagctttggcacaagacggtgaatcttatttcgagaagattcggtacaaactgcttcctggagcgtctaagatgttacccaaagtcttcttctctaataagaatataggcttctacaatccatcagatgacatattaagaattcgtaacacggctagtcataccaagaatggcacgccgcagaaaggacatagtaaggtagaatttaatctcaacgattgtcacaagatgattgatttctttaaatcttcgatacagaagcatccagaatgggggtcgttcggcttcactttcagcgatacctccgacttcgaagatatgtctgctttctaccgtgaagttgagaaccaaggttatgtcatatcgtttgataagattaaggagacatatatacaatcacaagtcgaacagggtaacttatatttgtttcaaatctataataaagatttctcaccatatagcaaaggaaagcctaatctacacacgttgtattggaaagcattatttgaagaagccaacttaaataatgtagtggctaagctgaatggagaagcagaaatattcttcagacggcatagtatcaaggcttcggacaaggtagtccacccagccaatcaggcgattgataataagaacccacatacagagaagacacaatccacgttcgagtatgatttagttaaagacaagagatatacacaagataaattcttcttccatgttcctatctcgctgaatttcaaggcccaaggtgtctccaagtttaacgataaagtgaatggtttcctaaagggcaaccctgatgtaaacataattggaattgatcgtggagaaagacatctcctttatttcactgtagtgaatcagaaaggtgagatactggtgcaggaatctcttaatacattaatgagtgacaaaggtcatgttaatgattatcaacagaagttggataagaaagaacaagaaagagatgccgcacgcaagtcatggactactgttgagaacattaaggagttgaaggagggttatctgagccatgttgttcataagctcgctcacttgataattaaatacaatgctattgtttgcttggaggatctaaatttcggcttcaagcgtgggaggtttaaagtagagaaacaagtttatcagaaatttgagaaagccctgatagataagttaaattacttagtattcaaagagaaggaattgggcgaggtgggtcattatttaacagcataccaattgacagcacccttcgaatccttcaagaaattgggtaaacaatctggtatactgttctatgttcccgcggattatacttcaaagattgatccaacgaccgggttcgtgaacttcctagatttgcgttatcagtctgttgagaaagctaagcaactcctgtcagatttcaacgctattagattcaattctgtccagaattactttgaattcgaaattgactacaagaagttgactccaaagcgcaaggtaggaacccagtctaagtgggtgatatgcacgtacggtgacgttcgatatcagaataggagaaaccagaaaggtcactgggaaacagaggaagtcaatgttacagagaaacttaaagctctcttcgcctcagatagtaagaccaccacagttattgattatgctaatgacgataatctaattgatgtcatcctagaacaagataaggcgtctttcttcaaagaattactttggttgctgaaactgaccatgactttaagacactcgaagatcaaatcggaggatgatttcatattatcaccagttaagaatgagcagggtgaattctacgactcccgcaaagcaggtgaagtctggccaaaggatgcagatgcaaatggagcctatcatatcgcgcttaaaggtctttggaacctgcaacagattaatcaatgggagaaagggaagactttgaatcttgcaataaagaaccaggactggttcagctttatacaggagaagccttatcaagaataa

SEQ ID NO: 761 - DNA, 3897 bp, Artificial Sequence
  Description of Artificial Sequence: Synthetic polynucleotide
atgacaaagacattcgactccgaattctttaatttatatagtcttcagaagacagtcaggttcgagcttaagccagtgggagaaactgcttctttcgtagaggatttcaagaatgaaggcctgaagagagttgtctctgaagatgagagaagagctgttgattatcagaaggttaaggagataatcgacgattatcacagggacttcatagaggaatcactaaactactttccggaacaggtcagtaaagacgcccttgaacaagcctttcatttgtaccagaagttgaaggctgcgaaggtagaagaacgtgagaaagctttgaaagaatgggaagctttgcagaagaagttgcgggagaaagtggttaaatgtttcagcgattcaaataaggcaagattctctagaattgacaagaaagaattaatcaaagaagatttaattaattggttggttgctcagaatcgagaggatgatattccaacagtagagaccttcaacaacttcaccacatacttcacaggattccatgagaaccgcaagaacatctacagtaaagacgatcacgccactgcaataagtttccgattaatacatgagaatttgccgaaattcttcgataatgttatttccttcaataagttgaaggaaggatttcctgaattgaagtttgataaagtgaaagaagaccttgaagtcgactatgacctgaaacatgcgtttgagatagaatacttcgtgaacttcgtaactcaggccggtatagatcaatataattatttattgggcggtaagactctagaagatggtacaaagaagcaaggtatgaatgagcagatcaatttgttcaagcaacaacaaaccagagacaaggcccgtcaaataccaaagttgattcccttatttaaacagattctatccgaaagaaccgaatcacagagcttcattcctaaacaattcgagtcggaccaggaattgtttgattccttgcagaagcttcacaacaactgtcaagataaattcacggtgctacaacaagcgattctaggtttagcagaagcagacttgaagaaagtgtttataaagacttccgatttgaacgcgctaagtaacactatctttggtaattatagcgtgttcagcgatgccctaaatttgtataaagaaagtttaaagactaagaaggcacaggaggctttcgagaaattaccagctcactctatccatgatctaattcaatatctggaacaattcaatagttctttggatgcagagaagcaacaaagtacagatactgttctgaattacttcataaagaccgatgaactgtacagccgctttatcaagtctacctctgaagcgtttacccaagtacaacctttgtttgaattggaagcgttgtcctcaaagagaagacctccagaatctgaggacgaaggagcgaaaggacaagaaggtttcgaacaaattaaacggattaaagcgtatttggatacacttatggaggctgtgcacttcgcgaaacctttgtatttagtcaagggtcgaaagatgattgaaggactagataaggaccagtcattctacgaagcatttgaaatggcttatcaagagctcgaatcactaataatccctatttacaacaaagctagatcatatctttctcgtaaaccatttaaagctgataaatttaagatcaatttcgacaataatactttattaagtggttgggatgcgaacaaggagactgccaatgctagcatactatttaagaaagatggtctttattatctgggtattatgcctaaaggtaagacctttctcttcgactatttcgtctcatcagaggatagcgagaaactgaagcaaagacgacagaagaccgccgaagaagcacttgcacaagatggagaatcctactttgagaagattcgttataaattattaccaggagccagcaagatgttaccgaaggtattctttagcaataagaatataggcttctacaatccaagcgatgatattctaagaatccgtaatactgcctcgcacactaagaacggcacacctcagaaaggtcattcgaaagttgaattcaacctaaacgattgtcacaagatgatagatttctttaagtccagtatacagaagcatccggagtgggggtcgttcggctttacattctcagacacgagcgactttgaggatatgagtgccttctacagggaagttgagaatcaaggttatgtaatatctttcgataagattaaggagacctatattcaaagccaagtggaacaaggtaacctatacttattccaaatttacaacaaggacttctctccttactccaaaggtaaacctaatttgcacaccttatattggaaagcattatttgaagaagccaacttgaacaatgtagtagctaaattgaatggagaagccgaaatattcttcaggagacatagcattaaagcatcagacaaggtagtccacccagcgaaccaagcaatcgataataagaatcctcatacagagaaaacacaatcaaccttcgaatacgatttagtaaaggataagaggtatactcaggacaagttcttctttcatgttcctatctcattgaatttcaaagcccaaggtgttagtaagttcaatgataaagtcaatgggttcctaaagggtaatcctgatgttaatattatcggtattgaccgcggagagagacatttgttgtactttacagtggttaatcagaagggtgaaatacttgtacaggaaagccttaacactttgatgtccgataagggacatgttaatgattatcaacagaaattagataagaaagaacaagaaagagacgctgccaggaagagctggactactgtagagaacatcaaagaattgaaggagggctacttgagtcacgttgttcataagctcgctcatttaattatcaaatataatgcaattgtttgtttagaagacctgaacttcggattcaaacgtggtcgtttcaaagttgagaagcaggtttaccagaagttcgagaaagcattaattgataagctcaattatttagtgttcaaagagaaggaattaggcgaggttggtcattatctgacagcctaccaactaacagctccgttcgaatccttcaagaagcttgggaagcaatcaggtattctattctacgtaccagccgactatacatcaaagattgatccaactaccgggttcgtgaatttcttggatctgagataccaatctgtggagaaagctaaacagctgttgtctgacttcaacgcaatccggttcaacagtgtccagaattatttcgaatttgagatcgattacaagaagttgacacctaaacgtaaggttggtactcaatccaagtgggttatttgtacttatggtgacgttagatatcagaatcgtcgtaaccagaaggggcactgggagacagaggaggttaatgttactgagaaacttaaagctttgtttgcatcagactctaagacaacaacagtcattgactatgccaatgacgataatctaatagatgtcattcttgaacaggataaagctagcttctttaaagaactcctttggttacttaaactaacgatgaccttgcggcacagtaagatcaagtccgaagatgacttcatattgtcgcccgtaaagaatgaacagggagagttctacgattcccggaaggccggtgaagtatggccaaaggatgcggatgcaaatggtgcttatcacattgctctcaaaggtttatggaatttgcaacaaattaatcaatgggagaaaggaaagacattaaatttggccatcaagaaccaagattggttctccttcattcaagagaaaccatatcaagagtga

SEQ ID NO: 762 - DNA, 3897 bp, Artificial Sequence
  Description of Artificial Sequence: Synthetic polynucleotide
atgacgaagacatttgattccgaattctttaacctatatagcctgcagaagaccgtgcgcttcgagcttaaaccggttggagagactgcctcattcgtggaggactttaagaacgagggtttaaagagagtggtgagcgaggatgaaaggcgtgcggtggattatcagaaggttaaggagatcatcgatgactatcaccgcgatttcatagaagaaagcctgaactactttcccgaacaagtttctaaggatgcactggagcaggcctttcacctgtatcagaaactcaaggcagccaaggtggaagaaagagagaaggcgttaaaggagtgggaggcgctgcaaaagaaattgcgcgagaaggttgtgaagtgtttcagcgattcaaacaaggcccgcttctctaggattgataagaaggaacttataaaggaagatctgattaattggctcgtggcccagaatcgagaggacgatattccaacagttgagacatttaataactttacgacctactttacaggcttccacgagaacagaaagaacatctactccaaggacgatcatgccactgccatcagcttcagactgattcatgagaatctaccaaagttcttcgataacgtgatttcatttaataagcttaaggaaggctttcctgaactgaagttcgacaaggtaaaggaggatcttgaagtggactatgatttgaagcatgccttcgagatcgagtactttgtaaactttgtgacccaagctgggatagatcagtacaactacctgctgggcggaaagacactggaggacgggacgaagaagcaaggcatgaacgaacagatcaatctgttcaagcagcagcagacacgggataaggctcggcagatacctaaactcattccactgtttaagcaaattctaagtgagcgtacagagtcccagagcttcatcccaaagcagttcgagtccgaccaggaattgttcgattccctccagaagttacataataattgtcaggataagtttacggtcctgcaacaggctatcctgggactagctgaggcggacttgaagaaagtcttcattaagaccagcgatctgaacgcactgagtaacacaatatttgggaactattcggttttctccgatgctctgaacttgtacaaggagtcattaaagaccaagaaagcccaggaagcattcgagaaactgcccgctcactcgatccatgatctgatccagtacctggaacagttcaacagctctctcgatgcggagaagcaacagtcgacagacaccgtgctcaattatttcatcaagaccgatgagctttattcacggtttatcaagagtacttctgaagccttcacgcaggtccagccactcttcgaactggaagccctatcctccaaacgaagaccaccagagagcgaagatgagggagccaaaggacaagagggattcgagcaaatcaagagaatcaaggcatacctcgataccctcatggaagcagtccacttcgccaaaccactctacctggtcaagggacgtaagatgatcgagggcctggacaaagatcagtcattctacgaagcatttgagatggcctatcaagaactggaatcactcattataccgatctacaacaaggcacgcagctacctgtcacggaagccattcaaggcggataaattcaagatcaacttcgacaacaatacactgctgagtggttgggacgccaataaagagaccgctaatgcatccatcctcttcaagaaggacggtctctattaccttggaataatgcctaaggggaagacctttctgtttgactacttcgtcagttctgaggactccgagaaacttaagcagaggcgtcaaaagactgccgaagaggccctggcccaggacggtgaaagctatttcgagaagatcagatataagctgctgcccggtgctagtaagatgcttcctaaagtattcttctccaataagaatattggcttctataatccatccgatgacatcctgcgcatcagaaacacagcatcacatacgaagaatggtaccccgcagaaaggacattctaaagtggagttcaacttgaatgactgccacaagatgatcgacttctttaaatcttcgattcagaagcatcccgaatgggggtctttcggctttaccttcagtgatacaagtgactttgaagatatgtccgcgttctacagagaggtggagaatcagggttatgtgatctcattcgataagattaaggaaacgtatattcagtcccaagtcgaacaaggtaatttgtacctattccagatctataacaaagacttctctccgtacagcaagggaaagcctaatctgcacaccctctattggaaggctctctttgaagaggctaacttaaacaacgtagtggccaagcttaatggagaagccgaaatattctttaggcgccactcaatcaaagcctctgataaagtggtacacccagccaatcaggcgattgacaacaagaaccctcacacagagaaaacgcaatcgacctttgaatatgacctggtgaaggataagcggtacacgcaggacaagtttttcttccatgtgcccatcagcctgaacttcaaagctcaaggtgtctctaaatttaatgacaaggtgaatggattcctgaaaggtaatccagacgtcaacataataggaatcgatagaggggagcgccatttactctacttcacagtggttaaccagaaaggcgagatcttagtgcaagagagtcttaatacacttatgtctgataaaggacacgtgaacgactaccagcagaagttggacaagaaagaacaggaacgggatgctgctagaaagtcttggactacagtggagaacattaaagaactgaaagagggatatctgtctcatgtagtgcacaaactggctcacctgattattaagtataacgcaatcgtgtgcctcgaagacctcaatttcggctttaaacgagggagattcaaggtggagaagcaggtctaccagaagtttgagaaagctttgatcgacaagctgaactacttggtcttcaaagagaaagaactcggagaggttggccactatcttactgcttaccagttgactgctccattcgagtcctttaagaaacttggcaagcaaagcggaatccttttctacgtgccggcagattataccagtaagattgaccctactacgggatttgtgaatttcctggaccttaggtatcagagtgtggagaaagcgaagcagctcttaagcgatttcaatgccatcaggtttaactctgttcagaattacttcgagttcgaaattgactacaagaagctaacacctaagagaaaggttggcacccagtccaagtgggtcatctgtacatatggcgatgtccgctaccagaatcggaggaaccagaaaggccactgggagactgaggaggtgaatgtaaccgagaagctcaaagccttatttgcctctgattccaagactactacagttatcgattacgccaacgacgataacttaattgatgtcatcctagaacaggataaggcttctttcttcaaagaactcctgtggctcctcaaattaacaatgaccctgcgtcacagtaagatcaaatctgaggacgactttatcctgtctcctgttaagaacgagcaaggcgaattctatgactcacgtaaggcaggagaggtttggcctaaagacgcggacgctaatggtgcttatcatattgctctcaaaggcctgtggaacctgcagcagataaatcaatgggagaagggcaagacccttaatctcgcaatcaagaaccaggactggttctcatttatccaggagaagccataccaggaatag

SEQ ID NO: 763 - DNA, 3897 bp, Artificial Sequence
  Description of Artificial Sequence: Synthetic polynucleotide
atgaccaagacattcgattcagaattcttcaatctgtattccctccagaagaccgttagattcgaattgaaacctgttggagaaaccgcctcctttgtggaagactttaagaacgagggattgaagagagttgtgagtgaggacgagcgccgggccgtagactaccagaaagttaaggaaatcattgacgattaccatcgggacttcatcgaggagtcactcaattactttccagagcaagtgagtaaggatgcacttgagcaggcgttccatctctaccagaaactcaaggcagctaaggttgaagaaagggagaaggccctgaaggagtgggaggctctgcagaaaaagctgcgtgagaaagtagttaagtgtttctccgatagcaacaaggctaggttctctagaattgataagaaggaactcatcaaagaagacctgataaattggttagtagcgcagaatcgcgaggacgacattcctacagtagaaacattcaataacttcactacctacttcacaggcttccatgagaacagaaagaacatctactccaaggacgaccatgcgacggcaatcagcttccggttgatacatgagaacctgccaaaattcttcgataacgtcatttccttcaacaaactcaaggagggcttcccagaattgaagttcgataaagtcaaggaggatttggaggtggactacgatctcaagcacgcattcgaaattgaatatttcgtgaacttcgttacgcaagcaggcattgaccagtacaactatctgcttggcggcaagaccttagaagacgggactaagaaacaaggcatgaatgagcaaatcaatctcttcaaacagcagcagactcgagacaaagcccgacagatccctaaactcattccactgtttaaacaaatcctcagtgagcgcacagaatctcaatcgttcattcctaagcaatttgagtctgaccaggagctgtttgattccttgcagaaattacataataactgccaagacaagtttaccgtcctgcagcaggctatcctcgggcttgcagaagctgatttgaagaaagtcttcatcaagacctctgatctcaacgccctttcaaatactatcttcggtaattacagcgtctttagtgatgctctgaatctgtacaaagagagtctgaagacgaagaaggctcaggaggcatttgagaaactgcctgctcactcgatccacgatcttatacaatatctggaacagttcaatagttcactggatgccgagaagcagcaatcaacagatacagtgctgaactatttcattaagactgatgaattgtacagccgctttatcaaatctacatccgaggcgttcacccaggtacagccgctgtttgaactggaagccctcagctctaagagacgccctccagaatccgaagacgaaggcgccaaggggcaagaaggtttcgaacagataaagagaattaaagcctatctcgacactctgatggaagcggtccacttcgctaaaccgctgtatctcgtgaagggccggaagatgatcgaaggactggacaaggaccaatctttctatgaagcgtttgagatggcctatcaggaactggagtccctgatcatccctatctataacaaggcacgaagttatttgagccgtaagccgttcaaggctgataagttcaagatcaacttcgataataataccttgctctcaggctgggacgctaacaaggagaccgctaacgctagcatcctattcaagaaggacggtctttactaccttggaattatgcctaagggaaagacctttctatttgactacttcgtatcaagcgaggatagcgagaaacttaagcagagaagacagaagaccgccgaggaggccctggcacaggacggtgagagctacttcgagaagattaggtataagctgctgcctggagcttccaagatgcttcctaaagtattcttcagcaataagaacattggattctataacccttccgacgatattctcaggatcagaaataccgcttcacataccaagaacggcaccccacagaaaggacattcgaaggttgagtttaacttaaatgattgccacaagatgatcgatttctttaaatcttctatccagaagcatccagagtgggggtcgttcggtttcaccttctcagacacttccgatttcgaggacatgagcgcattctaccgggaagtggagaaccaaggctacgtgatttcattcgacaagatcaaggagacctatatacaatctcaggttgaacaaggcaacctctacttatttcaaatctacaacaaagacttcagcccatacagtaaagggaagccaaatcttcacactctgtattggaaggctctctttgaagaagcaaacttaaacaacgtggtggccaagttgaatggcgaagctgagatattcttcagacgacatagcatcaaggcctctgacaaagtagtacacccggccaaccaggcaattgacaacaagaatcctcatactgaaaagacccagagcacctttgagtacgatctcgtcaaggacaagcgctacacccaggataagtttttcttccacgttcctatcagtctaaatttcaaggcacagggcgtttcaaagtttaacgacaaagttaatggtttcttgaagggtaaccctgacgttaacattattggaattgaccgaggggaacgccacttgctctacttcacagtggtcaatcagaaaggcgaaatattggtgcaggagagccttaatacacttatgtccgacaagggccacgttaatgattaccagcagaagctggacaagaaggagcaggagcgagacgcggcccggaagagctggactaccgtcgagaatattaaagagttgaaggagggatacctttcccatgtggtgcacaagttagcccacctcatcattaagtataacgccatagtgtgtctcgaggacctgaatttcggattcaagcgcggcaggttcaaagtcgagaaacaggtgtaccagaagttcgagaaagccctaattgataagctgaactacttagtcttcaaagagaaggaactgggagaagttgggcattacctgacagcataccagctcaccgctcccttcgagagtttcaagaagttgggcaagcagtccggcatcctcttctatgttccggccgattatacctctaagattgaccctactactggctttgtgaactttctggacctgaggtatcagagcgtggagaaagctaagcagttgctttccgactttaacgctatcaggtttaatagtgtccagaattacttcgagtttgaaattgattacaagaagttgacgcctaaacggaaggtgggtacgcagagcaagtgggttatatgtacatacggtgacgtccgataccagaatcggcgaaaccagaaagggcactgggaaaccgaagaagtgaatgtgaccgagaagcttaaagccctgtttgccagcgatagcaagacgactaccgttattgactacgccaacgatgacaatttaatcgatgtgatcctagagcaggataaagctagcttctttaaggagctgttgtggctgctcaaacttacaatgaccctgaggcattcgaagataaagagcgaagacgactttatactgagcccagttaagaatgaacagggcgaattctacgattcaaggaaggctggtgaagtatggcccaaggatgccgatgctaatggtgcgtatcatatcgcactgaaaggtctctggaatttgcagcagattaaccagtgggagaagggaaagactctgaacttagccatcaagaatcaggactggtttagcttcattcaggagaaaccgtatcaggaataa

SEQ ID NO: 764 - DNA, 3897 bp, Artificial Sequence
  Description of Artificial Sequence: Synthetic polynucleotide
atgaccaagacctttgactccgagttcttcaatttatactccctccaaaagaccgtccgctttgagcttaagccagtgggtgaaaccgcctctttcgtagaggactttaagaacgaaggcttaaagcgggtggtaagtgaggacgagagacgggcagtggactaccagaaggtgaaagagattattgatgactaccacagagatttcatcgaagagtcactgaattacttcccggagcaggtgagtaaagatgcattagaacaggctttccacctgtatcagaagctgaaggctgcgaaggtagaggagagagagaaagcccttaaggagtgggaagcattgcagaaaaagctgagggagaaagtagtgaaatgtttctccgactcgaataaggcgcgcttcagtcgtatcgataagaaagagctgattaaagaagatcttatcaattggttagtagcccagaaccgagaagacgacattccgacagtggaaacattcaataactttactacttatttcacaggctttcacgagaatcgcaagaatatttattcaaaggacgatcatgcaaccgctattagcttccggttaattcacgagaacctccctaagttctttgacaatgtgatctcattcaacaagctgaaagaagggttcccagagttgaaattcgataaggtcaaggaggatctggaggtcgattatgacctgaagcatgcctttgagattgagtacttcgtcaacttcgtcacccaggctgggatcgatcaatacaactatctgctcggcggtaagacactggaggatggtacaaagaagcagggtatgaacgaacagataaatctctttaaacagcagcaaacaagggacaaggcccgacaaattcccaagctcattcctctgtttaagcaaatactgagtgaacgtacagagtcccagtcattcattccgaagcagttcgaatcagaccaggagttatttgattcgttacagaaattgcacaacaactgtcaggacaagtttacagtgttgcagcaggcaatactcgggctggcagaggctgatctcaagaaggtgtttatcaagaccagtgacttgaatgcactgtccaataccatctttggtaattacagtgttttctctgacgctcttaatctgtacaaagagtccctaaagacaaagaaagctcaggaagcgttcgagaagctgccagcgcatagcatccatgatttgatacagtacctggaacagttcaattcctccttagacgcggagaagcagcagtccactgataccgtgctgaactacttcatcaagacggatgaattgtactccagattcataaagagcacctcggaggcattcactcaggtccaaccactgttcgagttggaggctctgtcaagtaagagacggccgcccgagtcggaggatgaaggcgctaagggtcaggagggcttcgagcagattaagagaataaaggcctatttggacactctaatggaagctgtccacttcgccaaacctctgtatcttgttaaaggacgaaagatgatagaaggacttgacaaggatcagagcttctatgaggccttcgagatggcctaccaggaactggagtccctcatcattcctatctacaataaggcccgttcatatctcagtcgcaagcctttcaaggccgacaaattcaagattaacttcgataacaacacactactgtccggctgggacgccaataaagagacggccaacgcctcaatcctgtttaagaaagacggcctgtattacctaggaataatgcccaagggaaagacgttcctatttgattacttcgtctcctccgaagattctgagaagctgaagcagagaagacagaagacagcggaagaggcgctggcccaggacggcgagtcttactttgagaagattaggtacaagcttttaccgggcgccagcaagatgctgcctaaagtattcttctctaacaagaatattggcttctacaacccaagtgacgacattctcagaatccgcaacacagcctcccacacgaagaatggcactccgcagaaaggtcattctaaggtggaatttaatctcaacgactgtcataagatgatcgatttcttcaaatcttcaatccagaaacatcctgagtggggttcctttgggtttaccttctcagatacttctgatttcgaggacatgtctgcattctaccgggaggtggagaatcaaggatatgttatttcctttgataagatcaaagagacttatattcaatctcaggtggagcagggaaatctgtacttattccaaatctataataaagacttcagtccttattccaagggcaagcctaatcttcacactctgtactggaaggcgttgtttgaggaggctaatctgaacaatgttgtggccaaacttaatggagaagctgaaattttctttcggcggcactctatcaaggcctcagacaaagtagtgcacccagcgaatcaggccatagacaacaagaaccctcacactgagaaaacgcagtcaacctttgaatatgacctggtcaaagataagcggtacacccaggacaagttcttctttcacgtgcccatctctctgaacttcaaagcccaaggtgtgtccaaatttaatgacaaggtgaacggctttcttaaaggcaaccctgacgtgaacatcataggcattgatcgtggtgagagacacctattatacttcaccgtggtgaaccagaagggagagatcctggtgcaggagagcctaaatactcttatgtccgacaagggacacgtgaacgattaccagcagaagctcgataagaaagaacaagaacgtgacgccgctcggaaatcttggactacagtagagaacataaaggagcttaaggaaggttacctgagccatgtcgttcataagctggcacacctgatcattaaatacaacgccattgtttgcctggaggacctaaacttcggctttaaacgagggagattcaaagtggagaagcaggtctaccagaagtttgagaaggctctcattgacaagttgaactacctcgtgttcaaggagaaggagctgggagaagtgggccactacttaactgcttaccagctcacagcacctttcgaatctttcaagaagctcggaaagcagtcaggcatcctgttctacgttcctgccgattacacctcaaagattgatccaacgacagggtttgttaatttcttggatctgcgatatcagtcggtggagaaggctaaacaactgttaagtgactttaatgccatacgattcaactccgtgcagaattacttcgagttcgaaatcgattataagaagctgacgcctaaacggaaggtcggcactcagtccaagtgggttatttgcacctatggcgatgttaggtaccagaatagacgcaaccagaaaggacattgggagacagaagaagtgaatgttacggagaagcttaaggccctgttcgccagcgacagcaagaccacaactgttatcgattatgccaatgatgataatctcattgacgttatcctcgaacaagacaaagcgtccttctttaaggagctgctctggttgctgaagctcaccatgacgctgagacattccaagataaagagcgaggacgacttcatattgtctccagtgaagaatgagcaaggcgagttctatgatagccggaaagcaggtgaagtctggcctaaggacgctgatgctaatggagcgtatcatatcgccctgaaaggcctgtggaacttgcaacagatcaaccagtgggagaagggaaagacccttaatcttgccattaagaaccaggactggttctccttcatccaagagaagccatatcaggaatga

SEQ ID NO: 765 - DNA, 3897 bp, Artificial Sequence
  Description of Artificial Sequence: Synthetic polynucleotide
atgaccaagacatttgatagcgagttcttcaatctctattcgcttcagaagacagtgcgctttgagttgaagcccgtgggcgaaacagccagtttcgttgaggattttaagaacgagggattgaagcgtgtggtatcggaggatgagaggagggccgtcgactatcagaaggtgaaggaaatcattgatgactaccatagggatttcatcgaagaatcattgaattattttcctgagcaggtgagcaaggatgccctggaacaggctttccacctttatcagaagttgaaggccgccaaggtagaagaaagggagaaggcattgaaggaatgggaagccctgcaaaagaaactgcgtgagaaagtggtgaagtgcttctccgacagcaataaagcaaggttcagccgaatagataagaaagagcttattaaggaggatcttatcaattggcttgtcgcccagaacagggaagacgatatccctacagttgagactttcaacaacttcaccacatatttcacaggatttcacgagaaccggaagaatatttactcaaaggacgaccacgctactgcaatttcattccggcttatccatgagaatttgccgaagttctttgacaatgtcatatcatttaacaaacttaaggagggctttcctgagttaaagttcgacaaagtgaaagaagacctggaggtggattacgacctgaagcatgccttcgaaatcgagtacttcgtgaactttgttacacaggcaggcatcgatcagtataactatctactgggtggaaagactctggaggacggaaccaagaagcaaggaatgaacgagcagatcaatctgtttaagcagcaacagacgagagacaaggcacgacagattcccaagcttatccctttgtttaagcagattctgtccgagagaaccgagtcccagtctttcatccctaaacagttcgaatctgatcaggaattgtttgactccctccagaagctgcacaataactgtcaggacaagttcactgtccttcagcaggctatactgggtctcgccgaggccgacttgaagaaggtgtttattaagacctccgatctgaacgcgttgtcaaacacaatatttggcaactactcagtatttagcgatgcgctgaatctatacaaggagagtctgaagaccaagaaggcacaggaggcattcgagaaacttcctgcccactccattcatgacctgattcagtatttagagcagtttaactccagtctcgatgctgagaagcagcagtcaaccgacactgtgttaaactatttcataaagaccgacgagctgtacagcagattcattaagagtaccagtgaggcctttacacaggtccagccactcttcgaattagaagccttatctagtaagagacgcccgcccgagagtgaggacgaaggcgcaaagggccaggaagggttcgagcagataaagaggatcaaagcctatttggacaccttgatggaggccgttcactttgctaagccgctgtatctagttaaaggtcggaagatgattgagggcttggacaaggatcagtcattctacgaggcctttgaaatggcatatcaggaactggaatccctgattataccaatctacaataaagcccgatcatatctgtctcggaagcccttcaaggccgacaaattcaagattaactttgataacaacactctgctctccggctgggacgctaataaggaaaccgccaacgccagcatcctgttcaagaaggatggattgtattaccttggcatcatgcccaaaggcaagacctttttattcgattacttcgtctcgtcggaagacagtgagaaactcaagcaacgacggcaaaagacagccgaagaagccttggcccaagatggcgagagctacttcgagaagattcgatacaagctgctgccaggagccagtaagatgcttcctaaggtgttcttctctaataagaacattggtttctataatccaagcgatgacatcctgaggattcgtaatacagcctcgcatactaagaacggaacaccgcagaaaggacactctaaagtggagttcaatttgaatgattgccacaagatgatagacttcttcaagagcagtatccagaaacatcccgagtggggctctttcggcttcaccttctccgacacaagtgatttcgaagacatgagcgctttctaccgggaagtagagaatcagggatatgtgatttcctttgacaagatcaaagagacatatattcagtcccaggtggaacaaggcaacttatacctcttccaaatctacaacaaggatttctcaccctacagtaaaggcaaacccaatctccacaccttgtattggaaggctctgttcgaggaagcgaaccttaataacgttgtagccaagctcaatggtgaggccgagatcttcttccgacgtcatagcatcaaggcctcagataaggtcgttcaccctgctaatcaggctattgacaataagaacccgcacaccgagaagacccaaagtacctttgaatacgacctcgtgaaggacaagaggtatacacaggacaaattcttctttcatgtaccaatctcccttaatttcaaggcacaaggcgtgtcaaagttcaacgacaaggtgaatggattcttaaagggaaatccagatgtcaacatcatcggaattgatagaggtgagcggcacctcctgtacttcactgtggttaaccagaagggagaaatactcgtacaggagtcgctgaacacacttatgagcgataaaggacacgtgaatgactatcaacagaaactcgataagaaagagcaagaaagagatgcggcccgcaagtcctggaccacggtcgagaatatcaaagagctgaaagagggctacctgagccatgtcgtgcacaagttagctcacctgattattaagtacaatgctatcgtgtgtctcgaagatctgaatttcggctttaaacgcggaagatttaaggttgagaagcaagtgtatcagaagttcgagaaagccctcatcgataagttgaactacttagtattcaaagagaaagaattaggcgaagtcggccactacctgacggcgtaccagcttaccgctccattcgagtctttcaagaaacttgggaaacagtccggcatcctattctatgtaccagccgactacacctctaagattgaccctaccacaggatttgtgaacttcctagacttgcgctatcagagcgtggagaaggccaaacagctgctttccgactttaacgctattagattcaactctgtccagaattacttcgagtttgagattgattacaagaaattgacgcctaaacggaaagtgggaactcaaagcaagtgggttatttgtacatacggtgatgtgagataccagaatcgaaggaaccagaaaggtcattgggagacagaagaggtcaatgtcacagagaagctgaaggccctgttcgcttctgacagcaagacaacaactgtgatcgattacgccaacgatgacaatttaattgatgttatcctcgaacaagataaggcttcgttcttcaaggaactactttggcttctaaagctgactatgaccctgcgccattcgaagatcaagagcgaggatgacttcattctcagtcctgtaaagaatgaacagggcgaattctatgattcgagaaaggctggcgaggtgtggccgaaagacgcagacgccaatggcgcataccacattgctctgaaaggtttatggaacctgcaacagattaaccagtgggagaagggtaagacccttaaccttgctatcaagaaccaagactggttcagctttatccaggagaagccttaccaggaatga

SEQ ID NO: 766 - DNA, 3897 bp, Artificial Sequence
  Description of Artificial Sequence: Synthetic polynucleotide
atgaccaagaccttcgattccgagttcttcaacttgtattccctgcagaagaccgttcgctttgaactgaaacctgtcggtgagactgcctccttcgtcgaggatttcaagaatgagggactgaagagggtcgtgtccgaagacgagagacgagcggttgactatcagaaagtaaaggaaattatagatgactaccaccgcgacttcatagaagaatctcttaactactttcccgagcaggtaagtaaagatgctctggagcaggcatttcatctgtaccagaagctgaaagccgctaaggtggaggaaagagagaaggcactgaaggagtgggaggccctccagaagaagctccgtgagaaggtggttaagtgtttcagtgattctaataaagcgcggttctcgagaatcgataagaaggaactcattaaagaagatctcattaactggctggtcgcccagaatcgtgaggatgacatcccaacagtggagactttcaataacttcaccacctactttacaggcttccatgagaacaggaagaatatctactccaaggacgatcacgccactgcaatctctttcaggcttattcatgagaaccttcccaagttcttcgataacgtgatctcctttaacaaactgaaagagggattcccagagcttaagttcgataaagtcaaagaggatctggaggttgattatgatctcaaacatgcgttcgagattgaatactttgtcaacttcgtcacgcaggctggaatcgatcagtacaattatttgctgggcggaaagacgttggaagatggcacgaagaagcagggtatgaacgagcagattaacctgttcaagcagcagcagacaagagacaaagcccggcagatacccaaactgatccctctgtttaagcagatcctctcagaaagaaccgaaagccagagcttcatccctaaacagtttgagtcagaccaagagctgttcgacagcctgcagaaattgcacaataactgtcaggataagttcaccgtcctccaacaagcgattctgggtctcgcagaagctgacctgaagaaagtattcattaagacctcagatctgaacgctctaagcaataccatatttgggaactacagcgtgtttagtgacgccttgaatctctataaagaaagcctgaagacaaagaaagctcaggaagcattcgagaaacttccagcccactcaatccacgatctgatacagtaccttgagcagttcaattcttctctggatgccgagaagcagcagtctacagataccgttctgaactacttcattaagactgacgagttgtatagtcgattcattaagtctacctccgaggcattcactcaagtccaaccgctgtttgaactcgaggctctgagctctaagaggaggcctcctgaaagcgaggacgagggcgcaaagggacaggagggattcgagcagattaagcggatcaaggcctatctggatactctcatggaggccgtacatttcgctaagcccttgtatctggtgaagggccgtaagatgatagagggcctcgacaaggaccaatctttctatgaagccttcgagatggcgtatcaggaacttgaatcattgataatccctatttataacaaggccagatcttacttaagtaggaagccctttaaagccgacaaatttaagatcaatttcgataacaacacactattatctggttgggatgcgaacaaagaaaccgcaaatgctagcatactgtttaagaaggacggactgtattatctgggaatcatgcccaaaggtaagacctttctcttcgactatttcgtgagctctgaagactctgagaagctgaaacagaggaggcaaaagactgccgaagaggccctcgcccaggatggagaatcctacttcgagaagattaggtacaagcttctgcccggtgcctcaaagatgttaccaaaagtatttttctctaacaagaatataggcttctacaatccctctgacgacatactgaggatccgcaacactgcctctcacacgaagaacgggacgcctcagaagggtcactctaaggtggagtttaacctcaatgactgccataagatgatagacttctttaagagctccatccagaaacacccggagtggggaagcttcggctttactttctcggatacatccgacttcgaagacatgagcgcattctacagagaggtcgagaaccaaggctacgttatcagctttgacaagataaaggaaacctacatccagagccaagtggagcaagggaacttgtatctcttccagatttacaacaaagatttctctccctattccaaaggcaagcctaacctgcatacactgtattggaaagcgttatttgaggaggcaaacctgaataacgtcgtggccaagctcaacggagaagcagagatcttcttccgacgccacagcattaaagcatcagacaaagtggtacatcccgcaaatcaagcaatcgataacaagaaccctcacactgagaagacccagtccacattcgaatatgatctggtgaaagacaagcgatacacccaggataagttcttctttcatgtacctatatccctgaacttcaaggcccaaggcgtgtcaaagttcaacgataaagttaatggattccttaagggcaatcccgacgtaaacattatcggcatagatcgaggcgaaaggcacctgctgtacttcacagtggtgaaccagaaaggagaaattctcgttcaggagtctctcaacacactgatgtctgataagggtcacgtgaatgattatcagcagaagctcgataagaaggaacaggagcgcgacgcagcgcgtaagtcatggacaaccgttgagaatatcaaggaactcaaggagggttaccttagtcatgtcgtccataagctggcccatctgatcattaagtacaatgctatcgtctgtttagaggacttgaatttcgggtttaaacgcgggaggttcaaggtcgagaaacaggtgtaccagaagttcgagaaagcgctgatagacaaacttaactatctggtctttaaagagaaagagctgggagaggtgggccactatttgaccgcatatcagttgactgctcccttcgagtcctttaagaagctgggaaagcagagcggcattttgttctatgtgcccgccgactatactagtaagatcgatcctactactggcttcgtgaactttctggatctccggtatcagtccgtggagaaggccaaacagctgctgtctgacttcaatgcgattaggtttaactctgttcagaattacttcgagttcgagatcgactataagaaacttacacctaagcgcaaagtcggtactcaaagcaagtgggtgatatgtacctatggagatgtgaggtatcagaatcggcggaatcagaaaggccattgggagaccgaggaggttaatgtgaccgagaagttgaaggccttgtttgctagtgactcaaagactaccacggttatcgactacgctaatgatgataaccttatagacgttatcctcgaacaagataaggcatccttcttcaaggagttgctctggctcctcaaattgaccatgacactccggcacagtaagattaagtcagaggatgatttcatcctaagtcccgtgaagaacgaacaaggtgaattctatgattcccggaaggcgggtgaggtatggccaaaggacgcagatgcaaacggcgcataccatatagcattaaagggactatggaatttgcagcagatcaaccaatgggagaagggcaagacattaaatctagccatcaagaatcaggattggttcagcttcatacaggagaaaccataccaggagtaa

SEQ ID NO: 767 - DNA, 3897 bp, Artificial Sequence
  Description of Artificial Sequence: Synthetic polynucleotide
atgacgaagacgtttgacagcgagttcttcaatttatactctctccaaaagacagtccgattcgaactgaagccagtaggtgagaccgcgagtttcgtagaggacttcaagaacgaaggccttaagcgggtcgtttcagaggatgagcgccgcgctgtggactaccagaaagtgaaggagatcatagacgactatcaccgcgacttcatcgaggaatctttgaactattttcctgagcaggtgtccaaagacgcactcgagcaggctttccatctgtatcagaaactcaaggccgctaaggtggaagagcgggagaaagcccttaaggaatgggaggccctccaaaagaaactgcgagagaaagtggtgaagtgcttcagcgattccaacaaggccaggttctctcgcatcgataagaaggaactgatcaaagaggacctgattaactggcttgtggctcagaaccgggaagacgacattccaacggtcgagacattcaacaacttcactacatacttcacaggctttcacgagaatcgaaagaacatctattctaaagatgatcatgcaactgccatatccttccgtctcatacacgagaacctacctaagttctttgacaacgtgatttcctttaataagctgaaggaaggcttcccagagcttaagttcgacaaagttaaagaggatctggaagtagactatgaccttaaacatgccttcgaaattgaatatttcgtgaacttcgtaacgcaggcaggcattgatcaatataattacctcctgggtgggaagactctcgaagatggcacgaagaagcaaggaatgaacgaacaaataaacttgtttaaacagcagcagacgagagacaaagcaagacagatcccaaagctgatccctctatttaagcaaattctctccgaacgcactgaatcccaaagtttcataccgaagcagtttgagagcgaccaggagctgtttgacagtcttcagaagcttcacaacaactgccaagataaattcacagtgttgcaacaagcaattctagggctggctgaggccgatctgaagaaggtgttcattaagacttccgatcttaatgcactctcaaacactatcttcgggaactactctgtgttctccgacgctttgaatctctataaagagagcctcaagacgaagaaggcccaggaagcatttgagaagctgcccgctcatagtattcacgatctaattcagtacttggagcagtttaactcttccctggacgccgagaagcagcagtcaaccgacacagtgctgaattacttcatcaagactgacgagttgtacagtcgcttcattaaatctactagcgaggcctttactcaagtgcaaccactgtttgagctggaagcgctgagctctaagagacggcctcctgagagtgaggatgagggtgccaaaggacaggaaggtttcgaacaaattaaacgaattaaggcttatctggatactcttatggaggcagtccactttgccaagcctctgtatttagtgaagggtcggaagatgattgagggcctggataaagaccagagcttctacgaggccttcgagatggcgtaccaggagctcgagtcactcatcatacccatttataataaggcacgcagttacctaagtagaaagccgttcaaagctgataaattcaagataaatttcgataacaataccctgctcagcggctgggacgcgaacaaggagactgctaatgcaagcatattgtttaagaaagatggactgtattacctcgggattatgcctaagggtaagaccttcctgttcgactactttgtaagttctgaagattctgagaaacttaagcagcgtagacaaaagacagccgaggaagccttagcccaggacggagaatcctactttgagaagatccggtacaagttgctacctggcgcttcgaagatgctgccgaaggtgttcttcagtaataagaacatcggtttctataatccatccgacgacatcctccggattcgcaataccgccagtcatacaaagaacgggacgcctcagaaaggacactccaaagtggagttcaacttgaacgactgccataagatgatcgacttctttaagtcatcgatacagaaacatcctgagtggggctcatttgggttcactttcagcgacacttctgacttcgaagacatgagcgcattctacagagaagtagagaatcagggatacgttatttctttcgataagatcaaggagacatacattcagagccaagtggaacagggcaacctgtacctattccaaatatacaacaaggatttctctccttatagcaagggaaagcctaatctccacacactttactggaaggcactattcgaggaagccaacctgaataacgtcgtcgcgaaacttaacggtgaggccgagatatttttccgacggcacagtatcaaagccagcgataaggtcgttcatccggccaatcaggccattgacaacaagaatccacacaccgagaagacacaatcgaccttcgaatatgacctggtcaaagacaagaggtacactcaggataagttcttctttcatgtgccaatttcattgaatttcaaggcccagggagtatctaagtttaacgataaggtgaacgggtttctcaagggtaaccctgacgttaatatcattgggatcgaccgaggcgaacgtcacctgctctactttactgtcgtgaatcagaagggagaaatcctggtgcaggaatccctcaacacgctaatgtccgacaaaggtcatgtgaatgactaccagcagaaattggataagaaggagcaggaacgggatgccgctaggaaatcctggactaccgtggagaatatcaaagagctgaaggaaggctatctgtcccacgtggttcataagctcgcacatctcatcattaaatacaacgcaatcgtctgcctcgaagacctgaacttcggattcaaacgtggacgtttcaaggtagagaaacaagtctatcagaagtttgagaaagcccttatcgacaagctgaattacctagtgtttaaggagaaagagctgggagaagtgggacattacttgacagcctatcagctgacagctcctttcgagtcatttaagaaactcgggaagcagagcggaattttattctacgttcccgccgactacacttcgaagattgatcccacaactggattcgtgaatttcttagatctcagataccagagcgtggagaaggcaaagcagctcctgtccgacttcaacgccatccgctttaactcggtccagaactacttcgagtttgagatcgattacaagaagctcacaccaaagcggaaggttggcacccagagtaaatgggttatctgtacttacggcgacgtccggtatcagaatcggaggaatcagaagggtcactgggagaccgaggaggtgaatgtcacagagaagctcaaggcgctgttcgcatctgattcgaagaccacgactgtgatcgactatgccaatgatgataatcttattgacgtcatcctggagcaggacaaagcttctttcttcaaggaactgctgtggctgctgaagttgacaatgaccttgaggcactcaaagattaaatcagaagacgatttcattcttagtccggttaagaacgaacagggcgaattctacgatagcaggaaagccggagaagtgtggcccaaagacgccgatgcaaatggtgcttatcatattgcgctgaagggcttgtggaacttgcagcaaattaaccagtgggagaaaggaaagactttgaacctcgccattaagaaccaagattggttctcattcattcaggagaaaccttaccaagagtag

SEQ ID NO: 768 - DNA, 3897 bp, Artificial Sequence
  Description of Artificial Sequence: Synthetic polynucleotide
atgaccaagactttcgattcagagttcttcaacttgtactcattgcagaagaccgtgcgcttcgaactgaaacccgtgggcgagacagcctccttcgtggaagactttaagaacgaagggttaaagagggttgtgtctgaggatgagcgtagagcggttgattaccagaaggtgaaggaaatcattgatgattaccacagggacttcatcgaggaatcattgaattacttccctgaacaggtttctaaggatgccttggaacaggcgtttcacctgtaccagaagctgaaggccgcaaaggttgaagagagagagaaagcactgaaggagtgggaggcactccagaagaagctgcgcgagaaggtagtgaagtgcttctctgatagcaacaaggcccggttctcccgtatcgataagaaagaacttattaaagaggatctgatcaattggttggtggctcagaaccgagaggacgacattccaactgtggagaccttcaataacttcacaacctatttcaccggattccacgagaatagaaagaacatctattctaaagatgatcatgcaaccgcaatcagctttcggctcatccacgagaacttacccaaattctttgacaatgtgatctcatttaataagctcaaggagggcttcccggagttaaagtttgacaaggtgaaggaggacctggaggtagattacgatctgaagcacgccttcgaaattgagtacttcgtcaactttgtgacacaggccggaatcgaccaatacaattacttgctgggtgggaagacactggaggacggtactaagaaacaagggatgaatgagcagataaatctgttcaaacagcagcaaactagggataaggccagacagatcccaaagctgatcccattgtttaaacagatcctctcagagagaacagaaagccagtctttcatcccaaagcagtttgagtcagatcaagagctattcgactccctacagaagcttcataataattgtcaggataaatttacggtgctgcagcaagcaattctgggattggcagaagcagaccttaagaaggtattcataaagaccagtgatttaaacgctttatccaacactatatttgggaactactcggtcttctctgacgctctgaacctgtataaggagtcgctcaagactaagaaggcccaggaagctttcgagaagctaccagctcattctattcatgaccttatccagtacctggagcagtttaattcttcattagacgccgagaagcagcaatccacagatactgtgctaaattatttcattaagactgatgaactgtatagcagatttatcaaatccacttcagaggccttcacacaggttcagccgctctttgagttagaggcgctttctagcaagaggcggccgcccgaaagtgaggacgaaggcgcgaaaggacaggagggctttgagcagatcaagcgaattaaggcttatctggacactcttatggaggctgtgcacttcgcgaagccactgtatctcgtcaagggtagaaagatgatcgaaggacttgataaggaccagagtttctatgaggcgttcgagatggcttaccaggaattagaatctctgatcattccgatctacaacaaggcccgtagctatctcagtaggaaacccttcaaggccgataaattcaagatcaactttgataacaacaccttgttgagcggctgggacgccaataaggagaccgccaacgccagtatcctattcaagaaggatgggctgtactatttagggattatgcctaaaggaaagacattcctgttcgattactttgtcagctctgaggattccgagaaactcaagcagcggaggcagaagacagccgaagaagctcttgcccaggatggagagtcctatttcgagaaaataaggtataagctgctgccaggtgcttctaagatgcttccgaaggtcttcttcagcaacaagaatattggattctacaatccgtcagacgatatcctccgaatccgcaacacagcatcccacacgaagaatgggacgccccagaaaggacattcaaaggtggagttcaatctcaatgattgccataagatgattgacttctttaagtcctccatccagaagcacccagagtggggttccttcgggtttacgtttagtgatacctccgactttgaggatatgtccgccttctaccgtgaagttgagaaccagggctatgtgataagcttcgacaagattaaagagacatacatccagtctcaagttgaacaaggaaacctttatttgttccagatctacaacaaggatttctcgccatactctaagggcaaacccaacctccacaccctctattggaaagccctctttgaggaggcaaacctcaacaacgttgtcgcgaaattgaatggcgaagctgaaattttcttcaggaggcatagtattaaggcttccgataaggtcgtgcatccggctaaccaggccatcgacaacaagaatcctcacacagaaaagacacagagtactttcgaatatgatctggtcaaagataaacgatacacacaagacaagttcttctttcacgttcccatcagtctgaactttaaagcgcaaggagtgagcaagtttaatgataaagtgaatgggttcctaaagggcaatcccgacgtcaacatcatagggatagacagaggagagaggcacctgttgtatttcactgttgtgaatcagaagggcgagatactggttcaagagtcactgaacaccctgatgtctgataaaggtcacgtgaatgactaccagcagaagctcgataagaaagagcaggaaagagatgccgcgcgtaagagctggaccactgtcgagaacattaaggagctcaaggagggttatttgtctcatgtggtgcacaaattagcccacctcattattaaatataacgccatcgtatgtctcgaagacctgaacttcggcttcaaacgcggtcgctttaaggtcgagaagcaggtttatcagaaatttgagaaggctctgattgacaagctgaactacttagtatttaaggagaaagagttaggtgaagtcggtcattatttaaccgcctatcagctgacggctcctttcgaaagctttaagaaattaggtaagcagagcggtatcttattttatgtacctgcggattacacttctaagattgatcctacaactggcttcgtcaacttcctggatttacggtaccagtctgtggagaaggccaaacaactccttagcgactttaacgcgatacggtttaactctgtgcagaactatttcgagtttgagatcgactacaagaaactgacgcccaaacggaaggttggcacacagtcaaagtgggtgatctgcacatacggcgacgtgagataccagaataggcgcaatcagaaaggtcattgggagaccgaggaagtaaacgtgacagagaagctgaaagccctctttgccagtgattctaagaccactacagtcatcgactatgccaacgacgacaacctgatcgacgtgatactggagcaggacaaggcatcgttcttcaaggaactgctgtggctcttaaagctcactatgactcttcgacacagtaagattaagagcgaggatgacttcattctgagccctgtaaagaatgaacaaggtgagttctatgattcaaggaaggccggagaggtgtggcctaaagatgccgacgcgaacggcgcctaccacatcgctttgaagggactatggaatctgcagcagattaaccagtgggagaaaggaaagacactgaacctggccatcaagaatcaggattggttctcatttatccaagagaagccttaccaagaataa

SEQ ID NO: 769 - DNA, 3897 bp, Artificial Sequence
  Description of Artificial Sequence: Synthetic polynucleotide
atgactaagaccttcgactccgagttctttaatctgtacagtcttcagaagacagtaaggtttgagctgaaaccagttggtgaaaccgctagtttcgtcgaggacttcaagaacgagggcctgaaacgcgtagtgagtgaggacgagagaagagccgttgactaccagaaagtcaaggagataatagatgactaccaccgtgactttatcgaggaaagtctcaattattttccagagcaggtatccaaggatgcactcgaacaagcgttccacctctatcagaagttaaaggcagcgaaagtggaagagcgtgagaaggccttaaaggagtgggaagcgctgcaaaagaaattgcgtgagaaagtcgttaagtgctttagcgacagcaataaagcccgcttctcccgaattgataagaaagagctcatcaaggaagacctgattaactggctagtcgcacagaatcgagaagatgatattccaacagttgaaacctttaacaacttcacaacatacttcacaggcttccatgagaaccgtaagaatatctacagtaaagacgaccatgcaacagcaatttcattcagattaatacatgagaacttgcccaaattctttgacaacgtcattagcttcaataagttgaaggaaggatttccggaactgaagttcgacaaggtgaaagaggacctcgaggttgactacgacctgaaacacgcatttgagatcgagtactttgtaaacttcgtcactcaggcgggcattgaccagtacaattatctacttggcggcaagaccctcgaggacgggacaaagaaacaaggaatgaatgaacagatcaacctctttaaacaacaacagacaagagacaaggcacgccagatccctaagttaatccctctatttaaacaaattctgtccgagcggactgagtctcaatcctttataccaaagcaattcgagtccgatcaggaactgttcgattcgctacagaaattgcataacaactgtcaggacaagttcactgtgctgcagcaagctatactcgggttggctgaagccgatctaaagaaggtctttatcaagactagcgacttgaacgcgctgagtaacacaatctttgggaactatagtgtattcagtgacgctctcaacctgtacaaagaatctctgaagacaaagaaggctcaagaggcgttcgagaagctgcctgcacactccatacatgacttgatacagtatctcgaacaattcaacagctcactcgacgccgagaaacagcagtccactgacactgtactgaactatttcattaagactgatgagttatatagtaggttcatcaagtccacttctgaggcgttcactcaggttcagccactgtttgagctcgaggcactatcttctaagcgcaggccaccggagagcgaggacgagggtgctaaaggtcaggagggctttgaacagattaaacgaattaaagcctacctggacacacttatggaggctgtgcacttcgctaaaccactctacctggtaaagggtcggaagatgattgagggactggataaggaccaatcattctacgaagcattcgaaatggcctatcaggaattggagagtctgatcattcctatatataataaagcccgctcatatctgagccggaaaccgtttaaggctgacaagttcaagattaactttgataacaatacattactgagcgggtgggacgccaataaggagacagctaatgccagcatcctgtttaagaaggacggcctctattatctaggaattatgcccaagggaaagacctttctcttcgattactttgtatcctctgaagattcagagaaactaaagcagcgaagacagaagacagctgaggaggcgttggcacaggacggtgagagctatttcgaaaagatccggtataaactgctgccgggagcaagtaagatgttgcctaaggtgttcttcagcaacaagaacatagggttctacaacccgagtgatgatatccttcggattcgcaataccgcctctcacaccaagaatgggactccacagaaaggccactcgaaggtagagtttaaccttaatgactgtcataagatgatcgacttcttcaagagctcgatccagaagcatccggagtggggcagctttgggtttacattcagcgacacctccgacttcgaggatatgtccgccttctatagggaagttgagaatcaaggctatgtcatttcattcgacaagatcaaggagacttatattcagtcacaggtggagcaagggaacctgtacctatttcagatatacaacaaggacttcagcccttactctaagggcaaacccaacctgcacacactgtattggaaggcattattcgaagaggccaatctcaataatgtcgtagcaaagctgaatggagaagcggagatcttcttccgaaggcactccatcaaagccagcgataaagtggtgcatcctgccaatcaggcaattgataataagaacccacacactgaaaagacacagtctacatttgaatacgacctagtgaaggacaagcggtacacccaggacaagttcttcttccacgtaccaatctcactcaacttcaaggctcagggtgtgagcaaatttaatgataaggtgaacgggttcctgaaaggtaatccggacgttaacatcattgggattgatagaggcgaacggcatctgctttactttacagtggtcaatcagaagggagagattctggtgcaagagagtcttaataccctcatgtcagataagggccatgtcaacgattatcagcagaagctcgacaagaaagaacaggaacgtgacgctgcccgcaagtcttggaccaccgtggagaatatcaaggagctgaaagaaggctatctctcgcacgtcgtgcacaagctagcccacttaatcattaaatataatgctattgtgtgcctggaggatcttaatttcgggttcaagagagggcgatttaaggtggagaaacaggtgtaccagaagtttgagaaggctctcattgataagttgaactacttggtcttcaaggagaaagaactgggagaagtcggacactacttaacagcttatcagttaacggcaccctttgagtctttcaagaagctcggtaaacagagcggtattctcttctacgtgccagccgactacacctcgaagatcgacccaaccactgggtttgtgaatttcttagatctgcggtatcagagtgtcgagaaagcaaagcagctcctttcagacttcaacgccatccggttcaatagcgtccagaattacttcgagtttgagatcgattacaagaaactcacgcccaaacggaaagttggcacgcaaagtaagtgggtgatctgcacatacggcgatgttagataccagaaccggaggaatcagaagggacactgggaaaccgaggaggtgaacgtgaccgagaagcttaaagctttatttgctagcgattccaagactacaaccgttatcgattatgccaacgatgacaacttgattgacgtcattctggagcaggacaaagcttcattcttcaaggagctgctgtggctgcttaaattaactatgactctaaggcactctaagattaagagcgaagacgacttcatactgtctccagtaaagaacgagcagggcgagttctatgattctcgaaaggcgggagaagtatggccaaaggacgccgatgccaatggcgcataccacatcgcacttaaaggactgtggaatctgcagcagattaaccagtgggagaaggggaagacattgaatttagctattaagaatcaggattggttcagtttcatccaagagaagccatatcaggaatag

SEQ ID NO: 770 - DNA, 3897 bp, Artificial Sequence
  Description of Artificial Sequence: Synthetic polynucleotide
atgactaagacattcgatagcgaattctttaacctctactcactgcagaagacggtgaggttcgaactaaagcctgtgggcgagaccgcatcatttgtagaagactttaagaacgagggtctcaagagagtggttagcgaagacgaaagaagagcggtggactaccagaaggtgaaggaaattatcgacgactatcaccgagactttatagaggagtcactcaactactttcccgaacaggtctcaaaggacgctctcgagcaggcgttccatctctaccagaaactcaaggccgccaaggtggaggaaagggagaaggcacttaaggaatgggaggcattacagaagaagctgcgtgagaaagttgtaaagtgtttctctgatagtaacaaggctaggttctcacgtattgacaagaaggagctaatcaaagaagatctaattaactggctcgtagctcagaatcgggaagatgatattcccaccgtggagacctttaacaactttacaacgtacttcacaggatttcatgagaatcggaagaacatttacagcaaagacgatcacgcaacagccatatcatttaggctgatccatgagaatctgcccaagttcttcgacaacgtgatcagctttaataaacttaaagagggatttccggagctgaaattcgataaggtgaaagaagacctggaagtcgattacgaccttaaacacgctttcgagattgagtacttcgtcaacttcgtcacacaggctggcatagatcagtacaattaccttctcggaggtaagacgctcgaggacggcaccaagaagcaaggcatgaatgagcaaatcaacctgtttaagcagcaacagacacgggacaaggcgcggcagatacccaagttaattccactatttaagcagattctcagcgagcggactgagagccagtctttcattccgaaacagttcgaaagcgaccaggagctcttcgacagcctgcagaaattgcacaataattgccaagacaagttcacagttctgcagcaggctatactgggtcttgccgaggctgacttaaagaaggtcttcataaagacctctgatctgaacgccctgtctaatactatattcgggaattatagtgtcttctcagatgctctaaatctttacaaggaaagcctgaagactaagaaggctcaggaggcattcgagaaattgcccgctcattccattcatgacttaatccagtatctggaacagtttaattcctcactggacgccgagaaacagcaaagcacagatacagtcctgaactatttcattaagactgatgagctgtatagcaggtttatcaagtccacctcggaggcgtttactcaggtgcagccactgtttgaactggaggccctttcatccaaacggcggccaccggaaagcgaggacgagggtgctaaaggtcaggaaggattcgagcaaataaagcgcatcaaggcctatctggatactctgatggaggcagtccactttgctaaacccttgtacttggtgaagggccgaaagatgatcgaaggattagataaggaccaatcattctatgaagcatttgagatggcctatcaggagttggagtcgctgattatcccgatctacaacaaggcccgttcttacctgtcgaggaaacccttcaaagccgataagtttaagataaacttcgataacaatactttactctcaggctgggatgccaacaaagaaaccgccaatgcctccatcctgttcaagaaagatggactatattatctgggaataatgcctaagggaaagaccttcctctttgattatttcgtgtcttcagaggactctgagaagctaaagcagcgacgccagaagaccgctgaggaggccttagcccaagacggagaaagctacttcgagaaaatccgatacaagctgttacctggcgccagcaagatgcttccaaaggtcttcttctccaataagaacatcggtttctacaaccctagcgatgatattctgcgaatccggaacaccgccagtcataccaagaatggtactcctcagaaggggcacagcaaagtggagtttaacctcaatgactgtcataagatgatcgatttcttcaaatcatcgatccagaaacacccagagtggggtagcttcggattcactttcagcgataccagcgatttcgaggatatgagcgccttctaccgggaggtggagaaccaaggatatgtaatatccttcgataagattaaagagacttacatccagagccaggtggagcaaggcaatctgtacctgtttcagatctacaacaaggatttctcgccatattctaaaggcaaacccaacttgcatactctgtactggaaggctctgttcgaagaggccaacttaaataatgtggtcgcgaagttaaatggcgaagccgaaatattttttcgtcggcactctattaaggcttcggataaggtggtgcatccggctaatcaggccatcgacaacaagaatccacacaccgagaagacgcagtcaacgttcgaatatgatctggtcaaggacaagcgctatacccaagataagtttttcttccatgttccaatcagtttgaactttaaggctcagggagtgtctaagttcaatgataaggttaatggattcctgaaaggcaatcccgacgtaaatatcattgggatagatagaggtgagcgccacttgctgtacttcaccgtggtgaaccagaagggagaaatccttgttcaggaatctttaaacaccctcatgagtgacaagggacacgtaaacgattaccagcagaaattagacaagaaagagcaggaacgcgacgctgctaggaagagttggacaacagtagagaatatcaaggaactcaaagagggctatctgtctcacgtcgtccataaactggcccatctgatcattaaatataatgccatagtctgcctggaagatctgaactttggattcaagcggggtagattcaaggtagagaaacaggtctatcagaagttcgagaaggcccttatcgacaaattgaactatctcgtgtttaaggagaaagaactcggagaagtcgggcactacttaaccgcctatcagctgacggcacccttcgagtcgttcaagaaactcgggaaacagtcaggaatcctcttctatgttccagcagactacacaagtaagatagatcctaccaccggatttgttaatttcttagacctgcgctaccagagcgtggagaaagctaaacagctgctctctgactttaatgccattaggtttaactcagtccagaactatttcgagttcgaaatcgactacaagaaactgacacccaagcgcaaggttgggacccagtctaagtgggtcatctgcacctatggtgatgtgaggtaccagaatagaagaaaccagaaagggcattgggagaccgaagaggtgaacgtgacagagaaacttaaagcattatttgcgtcagatagcaagaccactacagttatagactatgcaaacgatgataacctgattgacgtcatcttagagcaggacaaagcttcattcttcaaagaactgctttggctgctaaagcttaccatgaccctgcgacactcaaagataaagtcagaagatgatttcatcctgtcacctgtcaagaatgagcagggagaattctatgattcacggaaagcaggagaagtttggccaaaggatgctgacgccaacggcgcctaccatatagcgctcaaaggcctctggaatctgcagcagatcaaccagtgggagaagggcaagaccttgaacctcgcaataaagaaccaggactggtttagtttcatacaggagaagccataccaggaatga

SEQ ID NO: 771 - DNA, 3897 bp, Artificial Sequence
  Description of Artificial Sequence: Synthetic polynucleotide
atgacgaagactttcgacagcgagttctttaacctatactctctgcagaagactgtcagattcgaactgaaacctgtgggagaaaccgcgtccttcgtggaggatttcaagaacgagggactgaaacgggtcgtgtctgaggatgagcggagggctgtcgactaccagaaggttaaagagattatcgacgactaccaccgggacttcatcgaggagagtctgaattatttcccggagcaagtgtccaaagatgctttggaacaagccttccacctttaccagaagcttaaggctgcaaaggtggaggaacgcgagaaagcgttaaaggaatgggaggcactccagaagaaactcagagagaaagtggtgaaatgcttctctgattcaaataaggcccgcttcagtcggatcgacaagaaggagctaatcaaggaagatctgataaattggctcgttgctcagaacagggaggacgacatcccaacggttgagacatttaacaacttcactacctactttaccgggttccatgagaacagaaagaatatttattccaaagacgaccacgcaacagccatcagctttcgcctgattcacgagaacctcccgaaattcttcgacaacgtaatatcatttaataagctgaaggaaggctttccagagctcaagttcgacaaggtgaaggaggatcttgaagttgattacgatctgaagcatgcatttgagattgaatatttcgtaaatttcgtgactcaggccggtatcgatcagtacaattacctgttgggtggcaagacccttgaggacggtacaaagaaacaagggatgaacgaacagatcaatctatttaaacagcagcagacccgggataaggctcggcagatcccgaagctaatccctttgtttaagcagattctgtccgagcgcaccgagtctcagtcattcatcccaaagcagttcgagagcgaccaagaactgtttgactccctgcagaaactccacaacaattgccaggataaattcacggtgcttcagcaagctatactgggactggcagaggccgacctcaagaaggtcttcattaagacgtctgacctaaatgccctgtcaaatacaatctttgggaattattctgtgtttagtgatgctctgaacctgtataaggagagcctcaagacaaagaaagctcaagaggccttcgagaagctgcccgcgcattccattcacgatcttatccagtacttggagcagttcaactcaagtctcgatgccgagaaacagcagagcaccgatacagtcttgaattacttcataaagacagatgagctctattcgcggttcattaagtctacttcagaggctttcacccaggttcagcccttgttcgagctggaggccctttcctctaaacggcgaccgcccgagtctgaggacgagggagcgaagggacaggagggcttcgagcagatcaaacgcatcaaagcatacctggatacactcatggaagctgtgcacttcgccaagcctttgtacctggtgaaaggtcgtaagatgatcgagggccttgacaaggaccagtcgttctatgaggcattcgagatggcctaccaggagctggagtccttgattatcccaatatacaacaaggccagatcctacctcagcagaaagccattcaaggcggataagttcaagattaactttgataataacactttgctctccgggtgggatgccaataaagaaaccgccaacgcttccatcctctttaagaaagacgggctttactacctgggcattatgcccaaaggaaagaccttcctcttcgattacttcgtgtcttcggaggactctgagaaactgaaacaacggaggcagaagaccgccgaggaggctcttgcacaagatggtgaatcctacttcgagaagataaggtacaagctgctccctggcgctagcaagatgctcccaaaggtcttcttcagtaataagaatatcgggttctataacccgtccgacgatatactgagaattcggaatacagcaagtcacaccaagaacggcacgccacagaaaggacacagtaaggtcgagttcaatctgaacgattgtcacaagatgattgatttcttcaaatcgtccattcagaaacatccagaatggggcagctttggattcacattcagcgacaccagtgactttgaggatatgtcagccttctatagggaggtagagaatcagggttatgtgataagcttcgacaagataaaggaaacctacattcagagccaggttgaacaaggaaatctctatttgttccagatctacaacaaggacttctctccatatagcaagggcaagcccaacctacacactctctattggaaggctctatttgaagaagctaacttgaacaatgtggtggctaaactgaatggcgaggccgagattttctttcgacgacacagcataaaggcctccgataaggtggttcatcccgcgaatcaggcgatcgataataagaaccctcatacagagaaaacgcagtctacatttgagtacgacctggttaaggacaagcggtacacccaggacaaattcttctttcacgtccctatttcgctgaatttcaaggctcaaggagtgagcaaattcaacgataaggtgaatgggttcctgaaaggcaacccagatgtcaacatcatcggcatcgaccgtggagaacggcacctcctgtacttcaccgtggtgaaccagaaaggcgaaatcctggtgcaggaaagtttaaatactctcatgtcagataagggacacgtaaatgactaccagcagaaactggataagaaagagcaggaaagagacgccgctaggaaatcctggaccacagtggagaatatcaaagagctcaaggagggttacctgtctcatgtggtgcacaagttggctcatctgattattaagtataatgccattgtatgcttggaagatttgaacttcggattcaagcgcggtcggtttaaagttgagaagcaagtgtaccagaaatttgagaaggcactgattgacaagctgaactatctggtgttcaaagagaaagaactgggcgaagtaggccactacttaacagcctatcagctgaccgctcccttcgagtctttcaagaaacttgggaaacagagtggtatcctattttatgtgccggccgactacaccagtaagatcgacccaaccaccggtttcgtgaacttcctggatctgagataccagtcggtcgagaaagccaagcaactgttgagcgacttcaacgccatacgtttcaacagcgtccagaactacttcgagttcgagatagactacaagaagctgacacctaagagaaaggtgggtacacagtccaagtgggtgatttgcacatacggagacgtgcgataccagaaccgacgcaatcagaaagggcactgggaaactgaagaggtgaacgtcacggagaaactcaaagccctgtttgcctcagactcgaagacgactaccgtcatcgactacgcaaatgatgacaaccttatcgatgtcatactggaacaggacaaggcctctttctttaaggaactgctgtggctgcttaagttgaccatgacactgaggcatagcaagattaagagtgaggacgacttcatcctgtccccggtcaagaacgagcagggagaattctatgattctagaaaggcaggcgaagtgtggccaaaggacgcagacgccaatggagcttaccatatagcactgaaaggcttgtggaacctgcagcagatcaaccagtgggagaaaggtaagacattgaatctggctataaagaatcaggactggttctcattcatccaagagaagccttatcaggaatga

SEQ ID NO: 772 - DNA, 3897 bp, Artificial Sequence
  Description of Artificial Sequence: Synthetic polynucleotide
atgaccaagacattcgattctgagttcttcaatctttattccctgcagaaaaccgtccgcttcgaactaaagcctgtgggagagaccgcatccttcgttgaagacttcaagaacgaagggttgaagcgtgtggtgtcggaggacgaaaggagggcggtcgattaccagaaggtgaaagagattattgatgattaccatcgggacttcatcgaagaaagccttaactactttccagagcaagtttcgaaagatgccctcgagcaggcatttcacctctaccagaaactgaaagcagccaaagttgaagaaagagagaaagccttgaaggagtgggaagcgctgcagaagaagctacgagagaaagtggtgaaatgtttctccgactccaataaagcaaggtttagtcgcatcgacaagaaggaacttattaaggaagatctgatcaattggctggtcgctcagaatagagaagatgacattcctaccgtagagacctttaataacttcacaacatacttcacgggatttcacgagaatcgcaagaatatctattctaaagacgaccacgccaccgccatctccttccggctgatccacgagaacctccctaaattcttcgacaacgtgatcagcttcaataaactaaaggagggcttcccagagctgaagttcgataaagttaaggaggacctggaagtcgattatgatctaaagcacgccttcgaaatagagtacttcgtgaatttcgtgacacaagccggcattgaccagtataactatctgttaggcgggaagaccctggaggacgggacaaagaagcaaggaatgaatgagcagatcaacctgttcaagcagcagcagacccgcgacaaagcaaggcaaattccgaagctgatccctctcttcaaacagatactctccgagcggactgaatcgcagtcatttattcccaagcaatttgaaagcgaccaggagttgtttgacagcctccagaagctccacaataactgtcaagataagttcactgttcttcaacaggcgatcctcggattagctgaagcagatcttaagaaagtgtttatcaagaccagtgaccttaatgctctttccaacactatattcggaaactactcagtgttctcggatgccctgaatctgtataaggagtcactcaagacgaagaaggcacaagaggccttcgagaagctgcccgctcattctattcatgacctgatacagtacctggagcagttcaattctagcctggacgcagagaagcaacagtcaaccgatacggtgctgaactatttcataaagacagacgagctttatagtcgattcattaagtctaccagtgaggcatttactcaggtacagcctctgtttgagcttgaagccctgtcctccaagcgaaggcctcctgagagcgaggatgagggagccaagggacaggagggattcgaacagattaagcgaattaaggcctatctggacacgctcatggaggctgttcatttcgccaagccgctgtacctggtgaagggacggaagatgatcgaaggcctggacaaagatcagtctttctatgaggcgttcgagatggcctatcaggagctggagtccttaatcatccctatatataacaaggcccgtagttatttaagtaggaaacctttcaaagcagataaatttaagatcaacttcgacaacaacactttgctgtctggttgggacgctaacaaagagaccgctaatgcaagcattctgttcaagaaagatggcctctattacctcggaatcatgccgaagggcaagacattcctcttcgactactttgtgtcttctgaagatagcgagaagcttaagcagcgccggcagaagaccgcggaggaggctcttgcccaggacggagagtcgtactttgagaagattcgctacaagctcttaccaggagcttctaagatgctgcctaaggtattcttctctaataagaacattggtttctataatcctagtgatgatatcttacgtatcagaaatacggcctcgcatacaaagaacggcacgcctcagaaaggccacagcaaggtggagttcaacctgaacgattgtcataagatgatcgatttcttcaaatcgtcaattcagaagcacccagagtgggggtccttcggtttcaccttctctgacacatctgactttgaggatatgagcgcgttctaccgcgaggtggagaatcagggttacgtgatttccttcgacaagatcaaagaaacttacattcagtctcaggtggagcagggcaacttatacctcttccaaatctacaacaaagatttctctccctatagtaagggcaaacctaacctccatacactgtattggaaggctctctttgaagaagccaatcttaataatgtcgtcgctaaactgaacggcgaggctgagatattctttcgacggcacagcataaaggctagtgataaggtggtacaccctgccaatcaagctatcgataataagaatccgcatacagagaagacccaaagcacgttcgaatacgacctcgtgaaggataagaggtatacacaggataaattcttcttccacgtgcccatctctcttaatttcaaggcacagggcgtgtcaaagttcaacgataaggtgaacgggttcctgaaaggaaacccagatgtaaatattataggaattgatagaggggagaggcacttgctttactttaccgtggtcaaccagaaaggagaaatcctggtgcaggaatcactgaatactctaatgtcagataagggccacgtcaacgactatcaacagaaattggacaagaaggagcaggagcgggatgccgctagaaagagttggaccacagttgagaacataaaggagcttaaggaaggttacttgtcacatgtggtccataagctggcccatctgattatcaaatataacgccatcgtttgcttagaggaccttaatttcggctttaaacgcggccggttcaaggtggagaaacaggtgtaccagaagttcgagaaggctttgatcgacaagctgaattatcttgtattcaaggagaaagagctcggtgaagtaggccattacctaaccgcctaccagctgaccgctccgttcgaatccttcaagaagctaggcaagcaatctggcatcctgttctatgtgcccgctgattacacatctaagattgatcctacgactggtttcgtcaacttcctggatttgcggtatcagtccgtcgagaaagcgaagcagctgttgagcgatttcaatgctatcaggttcaattctgtgcagaattacttcgaatttgagatcgactataagaaattaactccaaagcgtaaggtgggaacgcagagtaagtgggtcatctgcacctatggcgacgttcggtatcagaatcggcgcaatcagaagggacactgggaaacagaggaggtcaatgtcaccgagaagctgaaggccctattcgccagcgacagtaagaccacaaccgtcatcgattatgctaatgatgataacctgattgatgtaattctcgaacaggacaaggcgtctttctttaaggaattgttgtggttgctgaaactaacaatgactttgcgtcacagcaagattaagtctgaggatgactttatcctgtctcctgtgaagaacgagcagggagaattctacgatagcaggaaagcaggtgaagtctggccaaaggacgcagatgccaacggtgcctatcatatcgctcttaaaggtctttggaacctccagcagattaatcaatgggagaaaggcaagactctaaaccttgccatcaagaatcaggactggttctccttcattcaggagaaaccttaccaagagtga

SEQ ID NO: 773 - DNA, 3897 bp, Artificial Sequence
  Description of Artificial Sequence: Synthetic polynucleotide
atgacgaagaccttcgacagcgaattctttaacctgtattctctgcagaagaccgtgagattcgagctgaaacccgtgggagaaactgcgtctttcgtcgaggacttcaagaacgagggtttgaagagggttgtgtcagaagacgaaaggagggccgttgattatcagaaagtgaaggagatcattgacgactatcaccgcgacttcatagaggagtcgttgaactactttcctgaacaggtctcgaaggatgccctggaacaggcgttccatttgtatcagaagctcaaggccgctaaggtggaagagcgggagaaagctctgaaagagtgggaggcgctacagaagaaattacgcgagaaggtggtgaaatgcttcagtgactcaaataaagcccgctttagtcgcattgataagaaagagctgatcaaagaggacctcattaactggctcgtcgcgcagaatagggaggatgacattccaactgttgagacctttaataatttcactacatactttaccggcttccacgagaaccgaaagaacatctacagcaaggatgatcatgccaccgcaatttctttccggctgatccacgagaaccttcctaaattctttgacaacgtgattagctttaacaagttgaaagaaggttttcctgaacttaagtttgataaggtgaaggaagatctggaggtggactacgacctcaagcacgccttcgaaatcgaatactttgttaactttgttacgcaggctggcattgaccaatacaattacctgctgggtggaaagactctagaggacggtacgaagaagcaaggcatgaacgaacaaataaacctgtttaaacagcagcagacccgggacaaggccaggcagataccgaagctcattcctttattcaagcagatcctgagcgagagaacagaaagccagtctttcatccctaaacaattcgagagcgaccaggagctcttcgactcactccagaaattacacaacaactgccaggacaagtttactgtgctgcagcaagccatcttaggtcttgccgaggcagacctcaagaaggtcttcataaagacctctgacctcaacgcactctcaaataccatatttggaaactattcagtcttctccgacgcattgaacctgtacaaggaatctttaaagacaaagaaggcgcaagaagccttcgagaagttgccggcccattccattcacgatctcatccagtatttagaacagtttaacagctctctggacgccgagaagcagcagtcaaccgacacagtgttgaactactttatcaagaccgacgagctgtattcccggtttattaagtcgacttccgaggccttcacgcaagttcagcctctcttcgagctggaagccctgagctccaagagacgacctcccgagagtgaggacgaaggtgctaagggacaggagggcttcgaacagatcaagcgaatcaaagcatatctggatacactaatggaagccgtgcactttgccaaaccgctgtacctcgtgaagggaaggaagatgatcgaaggactcgacaaagaccaaagtttctatgaggcgttcgagatggcgtaccaggagctcgaaagcctaattatcccaatctacaacaaggccagatcctatctttctaggaaacctttcaaggccgataagttcaagattaacttcgataacaataccttgctgagcggctgggatgccaacaaggagactgcgaatgccagcatactgtttaagaaagatggcctatattaccttggtatcatgccaaagggaaagacctttctgtttgattacttcgtctcatcggaagatagcgagaagctgaaacagcggaggcagaaaaccgccgaagaggctctggctcaggatggcgaatcgtacttcgagaagattcggtacaaactgctgcccggagcatcaaagatgctaccaaaggtcttctttagcaacaagaatatcggcttctataatccaagcgatgacatccttagaattcggaacactgcaagccataccaagaatggtactccacagaaaggacatagcaaagtcgagttcaatctgaatgactgccataagatgatagatttcttcaagtcttctatccagaagcaccctgagtggggatctttcggtttcacattctcagacacctccgatttcgaagacatgagcgcattctatagagaggtggagaatcagggttacgttatatccttcgacaagataaaggagacctacatacagtcacaggttgaacaaggcaacctttatttattccagatatacaataaggacttctctccatactccaagggtaaacctaacctgcacactctctactggaaagcactatttgaagaggccaatctgaacaacgtcgttgccaagcttaacggtgaagcagagatattctttcggaggcatagcattaaagctagcgacaaagtggtgcatcctgccaatcaggccatcgacaacaagaacccacatacagagaagactcagagtacctttgaatacgatctggtgaaagataagaggtacacccaggataaattcttcttccacgtccctatcagcttgaacttcaaggcacagggcgtaagcaaattcaacgataaggtgaatgggtttctgaagggcaacccagatgtgaatatcataggtatagatcgaggtgagagacacctgctctacttcaccgttgtgaatcagaaaggcgagatcctcgtccaagagagcctaaacaccctcatgtccgataagggtcacgttaatgattaccaacagaaactggacaagaaggagcaggaaagagatgcagcccggaagagctggacgaccgtcgagaacattaaggagcttaaggagggctatctttcccacgtcgtacacaagctggcccacttgatcattaagtataatgcaatcgtgtgtctcgaagaccttaacttcgggtttaagcgcggacggtttaaggtggagaagcaggtgtatcagaagtttgagaaggctttgatcgacaagcttaactacctggtgttcaaggagaaggagctgggagaagtgggacattatttaaccgcctatcagctgacagcgccatttgaaagcttcaagaaattgggcaagcagtcgggaatactgttctacgttccggccgattatacttctaagatcgacccaacaaccggcttcgttaatttcttagacctgaggtatcagtccgttgagaaggcgaagcagttgctgtcagacttcaacgccatccggtttaatagcgtgcagaactatttcgagttcgagatcgattacaagaaactgacaccaaagaggaaagttggaacgcagagcaagtgggtgatatgcacctatggagacgtccgctaccagaatagacgcaatcagaaaggtcattgggagaccgaggaagtcaatgttaccgagaaactcaaggctttgttcgctagtgacagcaagaccactacggtgatcgactacgctaatgacgataacctgatagacgtcatactggagcaggataaggccagcttctttaaggaacttctgtggctcctcaagctgaccatgacactgagacactcaaagataaagagcgaagacgatttcatcttgtcaccagtcaagaatgagcaaggcgaattctatgacagccggaaggctggtgaagtctggccgaaggacgccgacgctaatggcgcctaccatattgcattgaagggactttggaacttgcaacagatcaaccagtgggagaaagggaagacgctgaacctggctatcaagaaccaggactggttctcatttatccaggagaagccataccaagagtga

SEQ ID NO: 774 - DNA, 3897 bp, Artificial Sequence
  Description of Artificial Sequence: Synthetic polynucleotide
atgacgaagacatttgatagcgagttctttaatctttattcattacaaaagacagtgagattcgaactgaaacctgtgggtgagacagcttctttcgtcgaggactttaagaacgaaggccttaagagggtggtgtcagaggatgagcgtcgggccgtggactatcagaaggttaaggaaatcattgatgactatcatagggacttcatcgaggaaagcctcaactacttccctgagcaggttagcaaggatgcccttgagcaggcattccatctgtaccagaagctgaaggcagctaaagtcgaagaacgagagaaagctctgaaggagtgggaggcgttgcagaagaaacttcgggagaaagtggtgaagtgcttctctgatagtaataaggccaggttctcccgaatcgacaagaaagagctcataaaggaggacttgatcaactggcttgtggcacagaatcgggaggacgatattcctactgtggagacctttaacaacttcaccacctactttacaggcttccacgagaatcggaagaacatctatagcaaagatgaccacgctacagcaatctcatttaggctaattcatgagaacttgcccaagttcttcgacaatgtgatctctttcaataagctgaaggaaggttttccggaacttaaattcgacaaagtgaaagaggatctggaggtggattacgacctcaagcatgccttcgagatagaatacttcgtgaactttgtaacacaggccggcattgatcagtacaattaccttctcggcgggaagacccttgaagacggaaccaagaagcaaggaatgaatgagcaaattaacttatttaaacagcagcaaacccgagataaggccaggcagattcccaaactcatcccactatttaaacagatcctgtcagaacgcaccgagtcacagagtttcattccaaagcagtttgagtcagaccaggagctgtttgacagcctacagaagctgcataataactgtcaggataaatttaccgtacttcaacaggccatcctgggcctagctgaggctgatttaaagaaagtgtttataaagaccagcgatctcaatgcactgagtaataccatcttcgggaactactccgtgttcagcgacgccttgaatctgtacaaggagtcactgaagaccaagaaggcccaggaggcatttgagaagctccctgcacatagcatccacgacctcatccagtaccttgaacagtttaactcttcacttgacgctgagaaacagcagtctactgacacagtgctgaattacttcattaagactgacgagctatatagccggttcatcaaatctacctcggaagcctttacccaggtgcaaccattgtttgagctggaggccctgagctctaagcgtcgtcctccagagtccgaagacgaaggcgccaaaggccaggagggcttcgagcaaataaagcgcattaaagcatacttggatacactgatggaagccgtgcatttcgcaaaacctctgtaccttgtcaaagggaggaagatgatcgagggtcttgataaagaccagagcttctacgaggcgtttgagatggcctaccaggagctggagtccctgatcataccgatatacaataaggccagaagctacctgtcccgaaagcccttcaaggccgacaagtttaagatcaatttcgacaataatactctgttatccgggtgggatgctaataaggaaacagcaaatgccagtattttattcaagaaagatgggttatactatctcggcattatgcctaaggggaagaccttcctcttcgactacttcgtcagcagtgaggacagcgagaagcttaagcagcgtcggcagaagacagcagaggaggctctggcacaagacggcgagagttatttcgagaagatacggtataagctgctgcctggcgcctctaagatgcttcctaaagtgtttttctccaacaagaatatcgggttctacaatccaagcgacgacatcctaagaattcggaacactgccagccataccaagaatggaacacctcagaaaggacactccaaagtggaatttaaccttaatgactgtcacaagatgatcgacttctttaagagcagcattcagaaacatcctgagtggggttcattcgggtttacattctctgatacctctgacttcgaagatatgagtgcgttctatcgggaggtggagaatcagggttacgtaatctcgttcgataagataaaggagacgtacatccaatcacaagttgaacagggaaacttatacctgttccagatttataacaaagatttctcgccctatagcaaaggcaaacccaacctgcacacactttattggaaggcattatttgaggaagccaatcttaacaacgtagtggccaagcttaatggtgaagctgagatcttttttcgtcgacactccatcaaggcatcagataaagtagttcaccctgctaaccaagccatagataacaagaatcctcataccgaaaagactcagtccaccttcgaatacgacttagtgaaggacaagcgctatactcaggacaaatttttcttccacgtcccaatcagccttaacttcaaggctcagggcgtgtctaaattcaacgacaaagtcaatggattccttaaaggaaacccagacgtgaatattataggtatcgatcgaggagagagacatctgctgtacttcaccgtcgttaatcagaaaggcgaaatcctggttcaggaatcccttaatacgcttatgtctgacaaaggccatgttaacgattaccagcagaagctcgacaagaaggaacaggaacgtgacgccgccagaaagtcctggaccaccgttgagaatattaaggaactcaaagaaggctacctgtcccacgtagtccataagcttgcccatctgattattaagtataacgccattgtttgtttggaagatctgaacttcgggttcaaacgcggtcggtttaaggtggagaagcaagtttaccagaagttcgagaaagccctaatagataagctcaattatctcgtgttcaaagagaaggaattgggagaggtgggacactatcttaccgcatatcaactcaccgcgccgttcgaatctttcaagaaactgggtaaacaatccgggattctcttctacgttcctgcagactacactagtaagatagatcctacgactggcttcgtgaacttccttgatcttaggtaccaaagcgttgagaaggccaaacagctcctgtccgacttcaatgctatcagatttaacagtgtccagaattatttcgaatttgagatagactacaagaaactcactcctaagcgtaaggtagggacacagagcaagtgggtcatttgcacatatggtgatgtgcggtatcagaatcggcgtaatcagaagggccattgggagaccgaagaggtgaatgtgaccgagaaacttaaagccctgttcgcctcagactctaagactacgaccgtcatcgactatgccaacgatgacaatttgatcgacgtcatcttggagcaggataaagcctcgttctttaaggagcttctatggctgttaaagctcaccatgacccttcggcactccaagataaagtctgaggatgactttattctgtctccggttaagaacgaacaaggcgaattctacgactctcggaaggccggagaggtgtggccaaaggacgccgatgctaatggagcctaccatattgctctgaaaggcctttggaacttacagcagattaatcagtgggagaaagggaagaccctcaatctggcaataaagaatcaagactggttctcgttcattcaggagaagccgtaccaggaatga

SEQ ID NO: 775 - DNA, 3897 bp, Artificial Sequence
  Description of Artificial Sequence: Synthetic polynucleotide
atgactaagacctttgactctgagttcttcaatctgtactctctccagaaaaccgtacgatttgaacttaagccagtgggcgaaaccgcctcctttgtggaagattttaagaatgaaggactcaaacgagtggtgtctgaggacgagcggagggctgttgactaccagaaggtgaaggagataatcgatgactaccatcgcgactttatcgaggaatcactgaactactttcccgagcaagtctctaaggacgcgttggagcaggcctttcacctgtaccagaaactgaaagcagctaaggtagaggagagagagaaggctctcaaagaatgggaggcactgcagaagaaacttcgtgagaaggtggtgaagtgtttctcagacagcaataaagcgaggtttagcaggattgacaagaaagaattgatcaaggaggacctgatcaactggctcgtggcgcagaacagggaggatgatataccgaccgtcgagactttcaataacttcactacctatttcaccgggttccatgagaatcgaaagaacatctacagcaaagacgatcacgctacagctatttccttccgcttgatccacgagaatctgcccaaattctttgataacgtgatcagcttcaacaagctgaaagagggcttcccagagcttaagtttgacaaggttaaagaagacctcgaggtggactacgatctgaagcatgcattcgaaatcgagtatttcgtgaatttcgtgacccaagccggaatcgatcagtacaattacctgttgggcgggaagactctcgaggatggtaccaagaagcaaggtatgaacgaacaaataaacctattcaagcaacaacagactagagataaagccaggcagatccctaagctcattccactctttaagcagatcctgtcagagagaacagagagccaatccttcatcccgaaacagtttgagtcggaccaggaactcttcgatagcttgcagaaattgcacaataactgtcaggataaattcacggtcctgcagcaagcgattctcggactcgccgaggctgaccttaagaaggtgttcatcaagacaagcgatctcaatgcactgagcaataccatcttcgggaattactcagttttctccgatgccttaaatctttataaggaatccttgaagactaagaaagcgcaggaggcctttgagaaactgcctgcacattccatccatgatcttatccagtatcttgagcagttcaacagttccctggatgccgagaagcagcagagcaccgacactgtcttaaattacttcatcaagaccgatgaactctacagccggtttatcaagtcaacctccgaggcgtttacacaggtccaacctctgttcgagcttgaggcgctaagcagtaagaggcgcccacctgagtctgaggatgagggcgccaaagggcaggaaggcttcgaacagatcaagcgcatcaaggcctacctcgatactctgatggaggctgtccacttcgccaagcctctctatctggtcaagggccggaagatgatcgagggtctcgacaaggaccagagcttctatgaggcctttgagatggcctatcaggaattagaatctctgattattcctatttacaataaggctcggagctacctttcgcgcaagccattcaaggcagacaaatttaagatcaatttcgacaataatacactgctaagcggctgggacgcaaataaagagactgcaaatgcgtccatcctcttcaagaaggacggcctgtactacctagggatcatgcccaaaggtaagacatttctcttcgattacttcgtatcttctgaagacagtgagaagctcaaacaacggaggcaaaagactgctgaagaggccctcgcccaggatggcgaaagttacttcgagaagatccgttacaaactgcttcctggcgccagtaagatgctgcccaaggtgtttttctccaacaagaacattggcttctataatccctctgacgatattctgcggatacgcaacacagcctcacataccaagaatggaactcctcagaaaggtcatagtaaggtagagtttaatcttaacgactgccataagatgatagacttcttcaaatcctctatacagaaacacccagaatgggggtcgttcgggtttacctttagcgatacatcagacttcgaggacatgagcgcattctacagagaggtcgagaaccagggctacgtgatcagtttcgacaagatcaaagagacatacattcagagtcaggtggagcaagggaacctctacctcttccagatctacaacaaagatttctctccatatagcaaaggtaaacccaacttacatacgctttactggaaggccttatttgaggaagccaatctcaataatgtggtcgccaagttaaacggcgaagctgaaatattcttcaggcgacatagcattaaggccagcgataaggtcgttcacccagccaaccaggctatcgacaacaagaatcctcacacggagaagacccagtccaccttcgaatatgacctggtcaaggacaagagatatacacaggataaattcttcttccacgtcccaatctccttaaactttaaagcacagggagtttcgaagtttaacgataaggtcaacggcttcctcaaaggaaaccctgacgttaacattatcggcatcgaccgtggcgaacgacacttactgtatttcaccgtggtcaaccagaaaggcgagattctggtgcaagagtctctgaacaccctgatgagcgataagggtcacgtgaatgattatcagcagaagctggataagaaggaacaggaacgggacgccgcgcggaagagctggacaacagtagagaacatcaaagaactgaaggaaggttatctatcccatgttgtccataagctcgcacacttgataattaaatataacgcgattgtgtgcctcgaggacctgaacttcggcttcaagagagggcggttcaaggtggagaagcaggtgtaccagaaatttgagaaggctttaattgataaacttaattatttggtcttcaaggagaaggagcttggcgaagtcggccattacctgacagcttaccagctgacagcaccgttcgagtccttcaagaagctgggcaaacaatccggcatcttattctacgtgcctgccgactatacctcgaagatcgacccgaccaccggctttgtgaacttcctggatctgcgctaccaatcagttgagaaggccaaacagctcctgagtgatttcaatgcgatccgtttcaattcagttcagaactacttcgagttcgagattgactacaagaagctgacgccaaagcggaaggtcggaacccagtctaagtgggttatctgcacatacggtgacgtgcgctaccagaatagaaggaatcagaagggccattgggaaacagaggaagtgaacgtgacagagaaattgaaggcgttattcgcatcagatagtaagaccacgaccgttatagactatgcaaacgacgataacctgatcgacgtcatcctggagcaagacaaggcctcattcttcaaagaactgctatggttactaaagctcaccatgacgttgcgacactcaaagattaagtccgaagatgatttcatactctcaccggtcaagaacgagcagggagaattctacgattccagaaaggcaggcgaagtctggcccaaggatgctgacgcaaatggcgcttaccatatcgcactgaaaggactgtggaacctgcagcagattaaccagtgggagaaaggcaagaccctgaatctggctattaagaaccaggattggttcagcttcattcaggagaagccctatcaggaataa

SEQ ID NO: 776 - DNA, 3897 bp, Artificial Sequence
  Description of Artificial Sequence: Synthetic polynucleotide
atgacgaagacattcgacagtgaattctttaacctgtatagcctccaaaagactgttcggtttgagctgaaacccgtgggcgaaactgcaagctttgtggaggattttaagaatgaaggcctgaaacgggtggtgtccgaggacgaacgacgcgccgtcgactaccagaaggtcaaagagattatcgatgactatcacagagatttcatcgaggaatctcttaattactttcctgagcaggtttccaaggatgccttggaacaggcgttccacttataccagaaactcaaggctgcaaaggtggaggagcgtgagaaggcactgaaggagtgggaggccctgcagaagaagcttagagagaaagtggtgaagtgcttctctgactcgaataaagcccggttcagtagaatcgataagaaggaattaatcaaagaggacctgattaactggctggtggcccagaacagggaggacgacatcccgacagtggagacatttaacaacttcactacgtacttcaccggctttcatgagaatcgcaagaacatctacagtaaggatgatcacgccacggcaatctcctttcggctcatccacgagaacctgcctaagttctttgacaacgtaatttcctttaataaacttaaggagggattcccggagttgaagtttgataaagtgaaagaggacttggaagtcgactacgacctgaagcacgcattcgagatcgaatatttcgtcaactttgtgactcaggctggtatcgatcagtataactaccttctcggcggtaagactcttgaggacggaacaaagaagcaaggcatgaacgaacaaattaacctatttaagcagcagcagacacgtgacaaggcccgacaaattccaaagctgattcctctcttcaagcagattctgagcgagcgaactgaatctcagtcattcatacctaagcagtttgaatcagaccaagaactgtttgactcactgcagaagctccacaataactgccaggataaatttaccgtgctgcagcaggccattcttgggctcgccgaggctgatcttaagaaagtcttcatcaagacaagtgaccttaacgctctctccaatacaatctttgggaattactcagtcttctcagatgccctgaatctgtacaaggagtcactgaagaccaagaaagcccaagaggcattcgagaagttaccagcgcacagcatacatgatctgatccaatacctggaacaatttaattctagtttggacgccgagaagcagcagtcaaccgatactgtactgaactacttcatcaagactgacgaattgtacagtcggttcattaagagcacctctgaggcctttacccaggttcagccactgttcgagctggaagctctgagtagcaaacgcaggcctcccgagtctgaagatgagggcgccaagggccaggaaggatttgaacagataaagcgcattaaagcctacctcgataccttaatggaagctgtgcatttcgcaaagcccttgtatcttgtaaagggacgtaagatgatcgaaggtctggacaaggaccagtctttctacgaggcctttgaaatggcttaccaagagctagagagcctgatcattccaatctataataaggcccgcagttatttatcccggaagcctttcaaagctgacaagtttaagatcaacttcgataataatacgctgctgagtgggtgggacgctaataaggagacggcgaacgcaagtattctgttcaagaaagatggcctttattatcttggaattatgcctaagggtaagactttcctgttcgattacttcgtgtcctcagaggacagcgagaagctgaaacagcggcggcagaaaaccgctgaagaagccttagcacaggatggagaatcttactttgagaagattcggtataagctcctgccaggcgcctccaagatgctgcccaaggtgttcttcagcaacaagaatatcgggttctacaatccaagtgacgacatccttaggatccgcaacacggcgagtcacactaagaatggaacacctcagaagggacacagcaaagtcgaattcaacctgaacgactgtcataagatgattgatttctttaaatccagcattcagaaacatcctgagtgggggagcttcgggtttacattctccgatacatccgactttgaagacatgtccgctttctaccgggaggtagagaaccagggatatgtcatcagtttcgataagattaaagaaacctacatccagtcccaggtagagcagggaaacctgtatctctttcaaatctataataaagatttctctccctattcgaagggtaaaccgaaccttcataccttgtactggaaggccctcttcgaagaagcgaatcttaataatgtggtcgctaagcttaatggtgaagcggagatcttcttcagacgccattctattaaagcttccgacaaagtagtgcatcccgccaaccaggccatagacaacaagaatccacataccgaaaagacacagtccactttcgagtacgacctggtcaaggataagaggtatacacaggacaagtttttcttccacgtacccatttctctgaatttcaaggcccagggagtgagtaaattcaacgacaaggtgaatgggttcctgaaaggcaaccctgacgtgaatataatagggattgaccgcggagagcgccatcttctctatttcacagtggtcaatcagaaaggcgagattctagtgcaggaatctctcaacacgttgatgtccgataagggccatgtgaatgactatcaacagaaattggataagaaggaacaggagcgcgacgccgccagaaagagctggaccacggttgagaatattaaggaactgaaggaaggttacctctcacatgtagtacataagctcgcacatctgatcatcaagtacaacgctattgtgtgtcttgaggacctgaactttggtttcaagcgagggcgattcaaagtggagaaacaggtctatcagaaatttgagaaggctctgatcgacaagcttaactacctcgtattcaaagagaaagagctcggcgaagtgggtcactacctgaccgcatatcagctcacagcgcctttcgagagttttaagaaactagggaaacagagcggcatactattctacgttcctgctgattatacgtccaagatcgatcccacaacaggtttcgtgaacttcctagatcttagataccagtcagttgagaaggcaaagcagctcttgtcagatttcaacgcaatacggtttaactctgttcagaattacttcgagtttgaaattgactacaagaagcttacacccaagagaaaggtagggacacaaagcaagtgggtcatctgcacttatggagacgtcagatatcagaaccgcaggaatcagaaaggccattgggagacagaggaggtgaacgtcaccgagaagttaaaggccctcttcgcatcagattcaaagaccactaccgtcattgactatgctaacgatgacaacctgattgatgtgatcctggagcaagacaaggcctcgttctttaaggagcttctctggttgttgaaattgactatgaccctgcgccattcaaagataaagagtgaggacgactttattctgtctccagtgaagaatgagcagggagaattctacgacagtaggaaggccggcgaagtgtggcctaaggatgctgatgctaatggagcctatcatattgcgctcaagggcctgtggaatctgcagcaaataaaccaatgggagaagggcaagacgcttaatctggcgataaagaaccaggactggttctcattcatccaagagaagccatatcaggagtga

SEQ ID NO: 777 - DNA, 3897 bp, Artificial Sequence
  Description of Artificial Sequence: Synthetic polynucleotide
atgaccaagactttcgattcagaattcttcaatctgtattctctgcagaaaaccgtgcgctttgagcttaaacctgttggcgagaccgctagcttcgtcgaggatttcaagaacgaaggactcaagcgtgttgtgtcagaagacgagcggagggctgttgactaccagaaggtcaaggagataatcgacgactaccacagagacttcatcgaggagtcactgaactactttcccgagcaagtctctaaagacgccctggagcaggcgttccatctgtaccagaaactgaaagcagctaaggtggaggagagagagaaggccctgaaggagtgggaagccctccagaagaaattgcgagagaaggtcgtcaagtgctttagtgactcaaataaggctcgcttctcccgaatcgacaagaaagagttaatcaaggaggacctcattaactggctggtggctcagaatcgagaggacgatatacctactgtggagaccttcaacaacttcactacatacttcacaggtttccatgagaaccggaagaacatttatagtaaagacgatcacgcaactgccattagtttccgcctcatccacgagaaccttcccaagttcttcgataatgtcattagctttaacaaactcaaagaagggttcccagagctgaaattcgataaggtgaaggaggatctagaggtggactatgatctcaagcacgccttcgagatcgaatatttcgtcaactttgtcacccaagctggcattgaccagtacaattatctgctgggtgggaagaccctcgaagacggcaccaagaagcagggcatgaacgagcaaatcaacctgtttaaacagcagcagacccgggacaaggcgcgccaaattccaaagcttattcccttgtttaagcaaatcctctccgagcgcaccgagtcacagtcgttcataccaaagcagttcgaatccgaccaggagttgttcgattccctccagaagctacacaacaactgtcaggataaattcacagtcctgcaacaggcaattctgggtttagctgaagccgatctcaagaaggtgtttataaagactagcgacttaaatgccctttcaaatacgatcttcggcaattactctgttttctccgatgccttgaatctatacaaggaatccctgaagacgaagaaggctcaggaagccttcgagaagctgcccgctcactcaatccacgacctgatccaatacttggaacagttcaattctagcctggatgctgagaaacagcaaagcaccgataccgttcttaattactttataaagaccgatgagctctactctcgctttattaagagcacgtctgaggccttcactcaggtccagcccttatttgaattggaagccctgtcctctaagcggcgaccgcccgagagcgaagacgagggagccaaaggccaggaagggttcgaacaaatcaaacgcatcaaggcatacctcgataccctgatggaggccgtgcacttcgccaagcctctgtacctcgtgaaagggcggaagatgatcgaaggactggacaaagatcagtcgttctatgaggctttcgagatggcctaccaggagctcgaatctctaataattccgatctataataaagcacggagttatctgagcaggaagccattcaaggcagataaatttaagataaacttcgataataacaccctcctgtcgggatgggatgccaacaaagaaacagccaatgcaagcattctatttaagaaagatggtctatattatctgggtatcatgccgaaggggaagaccttcttgtttgactactttgtgagcagtgaggattccgagaagctgaagcagcggcggcagaaaaccgcggaagaggctcttgcccaggatggtgagtcctacttcgagaagattcgatataagttactgcctggtgcgagcaagatgctgcccaaggtgttcttcagcaataagaatataggcttctataatccttcggatgatatccttcggatccggaatactgcctcccacactaagaacggcactccgcagaagggccacagcaaggtcgagttcaacctgaatgattgtcacaagatgatcgatttctttaaatcctcgattcagaagcatcccgaatgggggtcctttggatttaccttctccgacacatctgactttgaggacatgtcagcattctacagggaggtagagaatcagggatatgtgattagcttcgacaagattaaagagacatacatacagtcacaggtggaacaaggaaatttgtatttgttccaaatttacaacaaggacttcagcccatatagcaagggcaagcctaatctgcataccctgtactggaaggcactctttgaagaggctaacctcaacaacgttgtggcgaagctgaacggcgaggctgaaatattcttcagacgtcactctatcaaagcttccgacaaggtcgtccacccagctaaccaagccattgacaataagaatcctcatactgagaagactcagtcaacattcgaatacgacctcgtgaaggacaaacgctacacacaggacaagttcttcttccacgtgccaattagtttgaatttcaaagcccaaggagtatccaagttcaatgacaaagtgaacggattccttaaggggaacccggatgtgaacattatcggcatagacagaggcgagagacatctgttgtactttaccgtggtcaaccagaagggagagatactggttcaggaatccctgaatacacttatgtccgacaaaggccacgtaaatgattaccagcagaagctcgataagaaggaacaagaaagagatgccgcccgtaagtcatggacgaccgttgagaacataaaggaactcaaagaaggttatctgagccacgtcgttcacaagctggctcatctcataataaagtacaatgctatagtgtgtctcgaagatctcaatttcggcttcaagagaggaaggtttaaggtggagaagcaggtttatcagaagttcgagaaagcccttatcgacaaactcaattacttggtattcaaggagaaagagctgggagaggtgggacactatctcactgcataccagctgacagcgcccttcgaaagcttcaagaagttgggaaagcaatctggcattctgttctatgtaccagctgattacacgtcaaagatcgatcctacaactgggttcgtgaacttcctggacctgaggtatcagagcgtggagaaggcaaagcaactcctgtccgacttcaacgcgatccgctttaactccgtgcagaactacttcgaatttgaaattgactataagaagcttactcctaagagaaaggtaggaacacagagcaagtgggtaatttgcacttacggagacgtaagatatcagaatcgtcgcaatcagaaaggccactgggagaccgaagaggtgaatgtgaccgagaaactgaaagccctcttcgcttcggacagtaagactaccacagtgattgactatgctaatgacgataatctgatcgacgtcatcctagagcaggataaagcatccttcttcaaggaattactgtggctgctgaagctgacaatgaccctgagacattcaaagatcaagagcgaggatgacttcatcctgagtcccgtgaagaatgagcagggagaattctacgactcccgaaaggcgggtgaagtatggcccaaggacgccgacgctaatggcgcataccacatcgcacttaaaggactttggaatctgcagcagataaaccagtgggagaagggaaagactctaaatctcgcaatcaagaatcaggactggttctcattcattcaggagaagccataccaggagtaa

SEQ ID NO: 778 - DNA, 3897 bp, Artificial Sequence
  Description of Artificial Sequence: Synthetic polynucleotide
atgacaaagacatttgattccgagttctttaatctgtactctcttcagaagactgtcagattcgaattaaagcccgtcggtgaaacggcgtccttcgtggaagacttcaagaatgaaggacttaagcgcgtcgtgagcgaggatgagcggagggctgtggactatcagaaggtaaaggaaatcatcgatgattatcaccgcgacttcatcgaagagagtctgaactacttccctgagcaggtgtccaaggatgctctggaacaggcatttcacctctaccagaagctcaaagcggctaaggtggaagagcgggagaaggcacttaaggagtgggaggccttacaaaagaagctccgtgagaaagtggtgaagtgcttctctgactccaataaggcccgcttctctagaattgacaagaaagagctgatcaaagaagatctcattaactggctagtagcccagaatcgggaagacgacattccaaccgtcgagacctttaataacttcaccacctactttaccgggttccatgagaaccgcaagaatatctacagtaaggatgaccacgcaacggctatctcgttccgactgatccacgagaacctgccgaagttctttgacaacgtcatctccttcaacaagctcaaggagggatttccagagttgaaattcgacaaagttaaggaagacctggaggtcgactatgacttgaaacacgcgtttgaaatcgagtatttcgtcaacttcgtcacacaggctggcatagaccaatataactatctcctgggaggaaagaccctggaagatggcacgaagaaacaaggaatgaacgaacagatcaacctgttcaaacagcagcagacccgtgataaggcacgccaaattcctaaactgatcccactctttaaacagatactgtccgaacgcaccgaatcccagtctttcattccaaagcagttcgagagtgaccaggagctgtttgactcactacagaagctgcacaataattgccaggacaaattcacagtgttacagcaggccatactgggcttggcggaagccgaccttaagaaggtgtttataaagacatcggaccttaatgctctcagcaacaccatctttggcaactacagcgtcttctccgatgcactgaacttgtacaaagaaagccttaagactaagaaagcccaggaggcctttgagaagcttccagcccactcaatccacgatctgattcagtacttggagcagtttaattcaagcctcgatgctgagaagcagcagagcacagatacggttctgaactatttcataaagacagatgagctttactccagattcattaagagcacgtccgaggccttcactcaggtgcagcccttgtttgagctcgaggcccttagtagcaagaggcggccaccagagtcagaggatgagggagctaaaggtcaggagggctttgagcaaataaagcgaataaaggcatacctggacaccttgatggaggccgtgcacttcgctaaaccattgtacctcgtgaaggggcgtaagatgattgagggtttggacaaggaccaaagcttctatgaagcgtttgaaatggcttatcaggagctggagtccctcatcattcctatctacaataaagccaggagctacctcagccggaagccgttcaaagccgacaagtttaagattaatttcgataataacacccttctgtcagggtgggatgccaataaagagacagctaacgcaagcatcttgttcaagaaggatggcctttactatcttgggataatgcccaagggcaagactttcctctttgattatttcgtatcatccgaggattctgagaagttgaaacagcggcgccagaagactgcggaggaagccctcgcacaggacggtgaaagctacttcgagaagatccggtacaaactactgcccggagccagcaagatgcttcctaaagtctttttctctaataagaatattggattctacaacccaagcgatgacatactgaggatcagaaacacagcctcacatacaaagaacgggacgccacagaaaggacattctaaggtcgaattcaacctgaacgattgtcacaagatgattgacttcttcaagtcaagcattcagaagcaccctgagtgggggtctttcggcttcactttctctgacacctctgactttgaagacatgagtgctttctatagagaagtggagaatcagggctacgtcatttcattcgacaagattaaagagacttacattcaatcacaggtagaacaaggcaatctctacctgttccagatatacaacaaggacttcagcccttatagcaaagggaaaccgaacctacacacattgtattggaaggccctgtttgaggaagccaacctaaacaatgtggtggccaagctgaacggagaggccgaaatatttttccgacgccattccatcaaggcttctgataaagtggtccacccagcaaatcaggcaatcgataacaagaatccacatacggaaaagacccagagcactttcgagtacgacctcgtgaaggacaagaggtatacgcaggataaattcttcttccatgttccgatctccctgaatttcaaagcgcaaggagttagcaagttcaacgacaaggtcaacggattcctgaagggaaatcctgatgttaatattattggcatcgatagaggtgaaaggcatttgctgtacttcacagtggtcaaccagaagggagaaatacttgttcaggagtccctgaatactctcatgagcgacaaaggacatgtcaatgattatcagcagaagctggataagaaggagcaagaacgcgacgccgctcgcaagagctggacaactgttgagaatattaaggaactcaaagagggctatctgtcacatgtagttcataagctcgcgcaccttattatcaagtacaacgctatcgtatgtcttgaggatctgaatttcggctttaaacggggacgcttcaaagttgagaagcaggtataccagaagtttgagaaagctctgatcgacaagctgaactatctggtatttaaagagaaagagctcggcgaggtcggccactatctgactgcttaccagctgacagcaccgtttgaatcatttaagaagctaggaaagcagtccggtatcctgttctacgtgccagccgattatacttccaagatcgatccaactacaggatttgtgaacttcctggaccttaggtatcagagcgtcgagaaagctaaacagctattatccgactttaatgcaatccgctttaacagtgtccagaattacttcgaatttgagatcgactacaagaaattgacaccaaagaggaaagtcggaacccagagcaagtgggtgatctgtacatacggcgatgtccggtaccagaacagacggaatcagaaaggtcattgggagacagaggaggtcaatgtcactgagaaactcaaagctctctttgctagtgattccaagaccactacagttatagactatgcaaacgacgataatttaatcgacgtgattctggagcaggacaaagcttcgttctttaaggaattgctgtggctcctcaagttgaccatgaccctaaggcactccaagataaagagcgaagatgacttcatcctgagtccagtcaagaacgagcagggtgaattctacgatagccggaaggccggtgaagtatggcccaaagacgctgatgcaaacggagcttaccacatcgccctcaagggtttatggaatctccagcagattaaccagtgggagaagggaaagaccctcaatctggccattaagaaccaggactggttctccttcattcaagagaaaccttaccaggagtaa

SEQ ID NO: 779 - DNA, 3897 bp, Artificial Sequence
  Description of Artificial Sequence: Synthetic polynucleotide
atgacaaagactttcgacagtgagttcttcaacctttacagtttgcagaagacagtgagattcgaacttaaacccgtgggtgaaacagcctctttcgtcgaagactttaagaacgaaggcctgaagagggtcgtatccgaagacgagcgacgggcagtggattaccagaaggtgaaggaaataatcgacgattaccaccgcgatttcatcgaagagagcttgaattactttcctgagcaagtgagtaaggacgccctggaacaggctttccacctttatcagaagctgaaggcagccaaggtcgaagaaagagagaaagctttgaaagaatgggaggcactgcagaagaaactgcgcgagaaagtcgtcaagtgctttagtgacagtaacaaggctcgtttctcccgaattgataagaaagaactgatcaaggaggacttaatcaactggctggtggcacagaatagagaggacgacatacccaccgtggaaacctttaacaatttcaccacctactttaccggctttcatgagaaccgaaagaatatttactctaaagacgatcacgctactgccatctcgtttaggttgatacacgagaacttgcctaagttcttcgataacgtgatctcattcaataagttaaaggagggcttcccagagctaaagtttgataaggtgaaagaggatctggaggttgactacgacctcaaacacgcgtttgaaatagagtatttcgtaaatttcgtgactcaagccgggattgaccagtataattacctcctcggaggcaagacgcttgaagatgggacgaagaagcagggaatgaatgagcaaatcaatctctttaagcaacaacagacaagagataaggcccgacagatacctaagctgataccactctttaaacagatcttatcggagcggaccgagtcccagagtttcatacccaaacagtttgaatctgatcaagagctgttcgactcattacagaaactgcataataattgccaggacaaattcaccgtgcttcagcaagctatcctgggattggcagaagctgatttgaagaaggtgtttattaagacaagtgatctgaacgcattgtcaaatacaatatttggcaattattctgttttctcagatgcattgaatctttataaggagtcgctgaagactaagaaagcacaggaggcattcgagaaattgccggctcactccattcacgacctaattcaatatttggaacagttcaactcaagtctggacgctgagaaacagcagtcgacagatactgtcctgaactactttataaagaccgacgagctctactccaggtttatcaaatccacctccgaagcctttacccaagtgcagccgctgttcgagctggaggccttatcttctaaacggcggccacccgaatctgaggacgagggcgctaagggacaggagggctttgaacaaatcaaacgcattaaagcttacctcgatacacttatggaagctgtgcacttcgccaagccactgtatctagtgaaaggaaggaagatgatcgagggtttggacaaagaccagtcattctacgaggccttcgaaatggcttaccaggaactcgagtccttgattatcccgatctacaacaaggctcgaagctatctcagtcggaaaccattcaaggcggataaatttaagattaacttcgataataacacactcctcagcggatgggatgcaaacaaagagactgcgaacgcatccatattatttaagaaggacggcttgtattacctgggtattatgccgaaaggcaagacattcctcttcgactactttgtttcctctgaggactcggagaagcttaagcagaggaggcagaagactgcagaggaagcacttgcacaggacggcgagtcttacttcgagaagatccgatataaactcctgcctggcgcaagtaagatgctgccaaaggtcttcttctccaataagaacatcgggttctacaacccgagcgacgacattctgcggattcggaacaccgctagccataccaagaacggtactccacagaaaggtcactcaaaggtggaatttaacttaaatgattgtcataagatgatagatttctttaaatcctctatccagaagcatcccgagtggggttcctttggtttcactttctcagatacatcagacttcgaggacatgagcgcattctatagggaggttgagaatcaaggctatgtcatttcattcgataagatcaaggagacttatattcagagtcaagtggaacagggcaatttgtatttgtttcagatctataacaaagatttcagcccgtactccaagggcaagccgaacctccatacgctgtactggaaagccctatttgaagaagcaaacctaaataatgtggtcgcaaagctcaatggagaggctgagatattctttagaagacatagtataaaggcgtccgacaaagtggtgcatcctgcaaatcaagctatcgataataagaatcctcatacggagaagacacagagcaccttcgaatacgacctggtgaaagacaaacgatatacccaggacaagttcttcttccacgtcccaatctctcttaactttaaagcgcagggtgtctccaagttcaacgacaaagtgaacgggttcttgaaaggcaatccggacgtgaatatcattgggatcgaccgtggtgaacgccatctattgtatttcacagtggtgaaccagaaaggtgaaattctcgtgcaggagtccctgaacaccctgatgagcgacaaagggcacgtgaatgattatcagcagaaattggataagaaggagcaagaaagagacgccgctaggaagtcatggactactgtagagaacattaaggaactgaaggagggctacctgagccacgtggtacataagctcgcccatctgatcattaagtataatgccattgtgtgcttagaggatctgaacttcggttttaagagagggcggttcaaggtcgagaagcaggtttaccagaagttcgagaaggcactgattgacaagctgaattacctggtgttcaaggagaaggagctgggagaagtgggacattaccttaccgcgtaccagctgaccgcgcccttcgagagcttcaagaagctcgggaagcagtctggtatcttgttctacgtcccggctgactatacctccaagattgacccaactacgggctttgtcaatttcttggatctgagataccaatcagtggagaaggccaagcagcttctttctgatttcaatgcaatcagatttaatagcgtgcagaactatttcgaatttgaaattgattataagaaactaacacctaagagaaaggttggaactcagagtaaatgggtcatatgcacctacggcgacgttcgttatcagaaccgtcgaaaccagaaaggtcattgggagacagaggaagtgaatgtgacagagaaactcaaggctctgttcgcctctgatagtaagactaccacagtaattgactacgccaacgacgacaacctgatcgacgtaattctggagcaggataaggcaagcttcttcaaagagttattatggctgctcaagctgaccatgacactgaggcatagcaagatcaagagtgaggacgatttcatactcagcccagtgaagaatgaacagggcgagttctatgatagccgcaaagcaggagaggtgtggccaaaggatgccgatgcgaatggcgcttaccacatagcactgaaaggtctgtggaacctacaacaaatcaatcagtgggagaaggggaagactctgaatctggctatcaagaatcaggattggttctcctttattcaagagaagccctatcaggaataa

SEQ ID NO: 780 - DNA, 3897 bp, Artificial Sequence
  Description of Artificial Sequence: Synthetic polynucleotide
atgaccaagaccttcgacagcgagttctttaatctgtactccctgcagaagacagtgcgctttgagttgaaacccgtcggagagacagcttcattcgtagaggattttaagaacgagggcctgaagagagtggttagtgaggatgagcgaagggcagtggactaccagaaagttaaggagatcattgacgattatcaccgtgactttattgaggaaagcctgaactacttcccggaacaggtaagcaaggatgccctcgaacaggcctttcacctctaccagaaactcaaagccgccaaagttgaggaaagagagaaagcactgaaagaatgggaggctctgcagaaaaagttgcgcgagaaggtggtgaagtgtttctcagactcaaacaaggctaggttctctcgcattgataagaaagaactcatcaaggaagatttgattaactggctggtggcgcagaaccgtgaagatgacataccaacagtggagacgtttaataatttcaccacttactttaccggtttccacgagaacagaaagaacatctatagtaaagatgaccacgcgacagcaatctcctttcgactcattcacgagaacctgcccaaattctttgataacgtaatttcgttcaacaagctgaaagaaggattcccggagcttaaatttgacaaggtcaaggaagatctggaagtcgattatgacctaaagcacgccttcgagattgagtacttcgtgaactttgtgacgcaagctggtattgatcagtacaactatctgcttggcggtaagaccctggaggatggcacgaagaaacaagggatgaatgaacaaatcaacctgtttaaacagcagcagacaagagacaaagctcgccagattcccaaacttattccactctttaagcagatcttatccgaaagaacagaatcccagtccttcattcccaaacagtttgaaagcgaccaagaactgttcgacagtttacagaaactccacaacaattgccaggataagtttactgtcctgcagcaggcaatcctaggcctggccgaggctgatctgaagaaagtgttcataaagacctccgacctgaacgcgttgagcaatacaatattcgggaactatagcgtctttagcgatgccctgaatctgtacaaagagtctctcaagacgaagaaagctcaggaagcatttgagaaactgcccgcccactccattcatgatctaatacagtatctagagcagttcaacagtagtctcgacgccgagaaacaacaatctaccgacactgtactaaactacttcataaagaccgatgagttgtatagcagatttattaagtctacttctgaagccttcacccaggtgcaaccgctgtttgaactggaggctctgtccagcaagagaaggcctccggagagtgaagacgaaggcgccaaagggcaagaaggattcgagcagatcaagcgcattaaggcctaccttgataccctgatggaagctgtgcacttcgctaagccactgtatttggtgaaaggcaggaagatgattgagggactagacaaagatcagtctttctacgaggcatttgagatggcctatcaggagttggaaagcctgataattccaatttacaataaagctcgtagttatttgtcaagaaagccgttcaaagcagataagtttaagatcaacttcgataataatacactccttagtgggtgggacgccaataaagaaacagcaaacgcctctattctctttaagaaagatggcctgtactacctcggcatcatgcccaaaggaaagacatttctgtttgactactttgtgagctcagaagattccgagaagctgaagcagcggcgccagaagaccgccgaagaagctcttgcccaggacggcgaatcttacttcgagaagattcgatataagttgctaccgggtgcttcaaagatgctgcctaaggtgttcttctctaataagaacataggattctataatccttccgacgacatactcagaatcaggaatacagcaagtcacacgaagaacggaactccgcagaaaggtcactcaaaggtggaattcaatctgaacgattgccacaagatgatcgacttcttcaaatcttccatacagaagcatcctgagtggggatccttcggctttactttcagcgacaccagtgactttgaggacatgagcgcattctatcgcgaggttgagaatcagggatatgtaatctccttcgacaagattaaggagacatacatccagagtcaggtggagcagggcaatctatatctgttccagatttataataaggatttctctccctacagtaagggtaaaccaaatcttcatacactgtactggaaggctctgttcgaggaggccaatcttaacaatgtcgtagcaaagcttaatggcgaggcagaaatcttttttagaagacacagtattaaggcatccgacaaagtcgtacatccagcgaatcaagctattgacaataagaaccctcatactgagaagactcagtcaacatttgagtatgacctggtgaaggataagaggtacacacaggacaaattcttctttcatgtacctatctcccttaatttcaaagcccaaggcgtctccaagtttaacgacaaggtgaacggatttttaaagggtaatcccgacgtaaatattattggcattgaccgtggtgagcgtcatctgctctatttcactgtagtcaatcagaaaggcgaaatcctggtacaggagtccctcaataccctgatgagcgacaaaggccacgtcaacgattatcagcagaagctagacaagaaagagcaggaacgcgacgccgcccgaaagagctggaccacagtagagaacattaaagagctgaaggaaggatacttgagccatgtagtccataagctggctcatctgattatcaagtacaatgccattgtgtgcctcgaggatctcaactttggatttaaacgcggtcgattcaaggttgagaaacaagtctatcagaagttcgagaaggcgctcatcgataagctcaattacctggtattcaaagagaaggagctgggtgaagttggacattatctgaccgcctatcagctgaccgcgcctttcgagagttttaagaaactcggcaaacagagtgggatcctcttctacgtgcccgctgactacacttccaagatcgatccaaccactggcttcgtcaacttcctggaccttcgatatcagtccgtggagaaggccaagcagctgctttccgactttaacgccatcagattcaactcggtgcagaactatttcgaattcgagattgattacaagaaactgacaccaaagaggaaagtcggaacgcaatccaagtgggttatatgcacatatggcgacgttaggtatcagaacagaagaaaccagaagggccattgggaaaccgaggaagtcaatgtgaccgagaaactcaaggcactcttcgcctccgatagtaagacgaccacggtgatagactatgccaacgatgataatcttatcgatgtgattctggaacaggataaagccagtttcttcaaggagctattgtggttgctcaaactgacgatgaccctgcgtcactcgaagattaagtccgaggatgactttattctgtcacctgtgaagaacgagcagggtgagttctacgactcccgcaaggccggcgaggtgtggcccaaggacgcagacgctaatggagcctaccatatcgccctgaaaggactgtggaatctgcaacaaattaatcaatgggagaagggcaagacactcaacctggcaataaagaatcaggattggttctcgttcatccaggagaagccctaccaggagtaa

SEQ ID NO: 781 - DNA, 3897 bp, Artificial Sequence
  Description of Artificial Sequence: Synthetic polynucleotide
atgacaaagacattcgactccgaattctttaatctatatagcctgcaaaagactgtgcgtttcgagcttaagccagttggagagacggcttcctttgtcgaagatttcaagaacgagggccttaagagagtggtctcagaggatgagcggagagctgttgactatcagaaggtgaaggaaatcatagacgactaccacagagacttcattgaggagagtttgaactactttcctgagcaagtgtctaaagacgccttagaacaggcctttcatctgtatcagaagctgaaagctgctaaggtggaagaaagagagaaagccttgaaggagtgggaggccttgcagaagaagctgagggagaaggtcgttaagtgtttctccgacagcaacaaagccaggttctcaaggattgataagaaggagctgattaaggaagacctgataaactggctcgtggcacagaatagagaggacgatatcccaactgtggaaactttcaacaactttaccacttacttcactgggttccacgagaatcgtaagaatatctactccaaagatgaccacgcgactgctatctccttcaggctcattcacgagaatcttcctaaattcttcgataacgtcattagtttcaacaagctgaaggaaggattccctgagcttaagttcgacaaagttaaagaagatctggaggtagactacgatctgaaacacgccttcgaaatcgaatatttcgtaaacttcgtcacacaagctggaatcgaccaatataactatctactgggagggaagacactagaggacggtacaaagaagcaaggaatgaacgaacagatcaacctgttcaagcagcagcaaaccagagacaaggccaggcagattcccaagctgataccgttattcaagcagattctatccgaaagaaccgagtcacagagcttcatccctaagcaattcgaatcagatcaggaattatttgactccctgcagaagcttcataacaactgtcaggacaaatttacagtgctacagcaggccatcctgggacttgcagaagccgatctgaagaaggtgtttataaagacatccgatcttaatgccctatccaacacaatcttcggcaactactcagtcttctccgatgccctcaacctgtacaaagagtcattaaagaccaagaaggcccaagaagcattcgagaagttgcctgctcattctatccatgacctcattcagtatctggagcagttcaacagctctcttgacgcagagaaacagcagtccacagacaccgttctgaattacttcattaagaccgatgaactctacagccgtttcattaagagcacctccgaggcgttcactcaagtacaaccgctgttcgagctagaggccctgagcagtaagagaagacctcccgagagcgaagatgagggagctaaagggcaagagggtttcgaacagatcaagaggattaaagcctacctggacactcttatggaagccgtgcactttgcgaagccgctgtatctggtcaaaggacggaagatgatcgaaggcctggataaggatcaatctttctatgaagcctttgaaatggcctaccaggagttggagtctcttatcatcccaatctataataaggcaaggagttacctttcgcggaagccatttaaagccgataaattcaagattaacttcgataataacacgcttctcagcgggtgggatgctaataaggaaactgctaatgcctccattttgtttaagaaagacgggctgtactatctgggcattatgcctaagggaaagaccttcctgttcgactatttcgtgtcatcagaggacagtgagaaactgaagcagcgacgccagaagaccgctgaggaggccctagcacaggatggcgagtcgtatttcgagaaaatacggtataaactgttgccaggagcatccaagatgctacctaaagtattctttagcaataagaatatagggttctacaatccatccgacgacatcctgagaataaggaataccgctagtcatacgaagaatggcacgccgcagaagggccattccaaagttgagttcaatctgaacgattgccacaagatgattgatttctttaagagcagcatccagaagcatcccgagtggggttcgtttggctttaccttctccgacacctctgactttgaagacatgagtgccttctaccgggaggtggagaaccaaggatatgtaattagctttgacaagattaaggaaacttatatccaatcccaggtcgagcagggaaacctgtatttgtttcagatttacaacaaagacttctctccctattcaaagggaaagccaaacctccacacgctgtattggaaagctttgttcgaagaggctaatctgaacaacgtcgtcgctaagttgaatggcgaagctgagatcttcttccggcggcatagtatcaaagcgagtgataaggtggtgcaccctgccaaccaggctattgacaataagaaccctcataccgagaagacccaatcaaccttcgaatacgatcttgtgaaagataagaggtatacacaggacaaattcttcttccatgtgccaattagtctgaacttcaaagcgcaaggcgtgtccaaattcaacgacaaggtgaatggctttcttaaaggcaatccggatgttaacatcattgggatcgaccgtggcgagagacacctgctgtacttcactgtcgttaaccagaaaggcgagatcctggttcaagagagcctgaacaccctgatgtcagacaaagggcatgtgaatgactatcagcagaaactagataagaaggagcaagagagagatgccgcgcgcaagagttggacaaccgtggagaatatcaaagagcttaaggagggctacttgagccacgtggttcataaactcgcacacctaattatcaagtacaatgccattgtctgcctggaggacctgaacttcggcttcaaacgcggaaggttcaaggtggagaaacaggtatatcagaaattcgagaaagcattgattgacaaattaaattacctcgtgtttaaagagaaggagctcggtgaggtcggccattatctgacagcttaccaactaaccgcaccattcgaatcctttaagaagctcgggaagcagtctggtatcctattctacgttcctgcggactatacttcgaagatcgaccctaccactggctttgtgaatttcctggaccttcgataccaatcggtcgagaaagcaaagcagctgctaagcgactttaacgccatccggttcaacagtgtccagaattacttcgagtttgagatagactataagaaactgacgccgaaacggaaagtcggtacacagtcgaaatgggttatctgcacctatggcgacgtgaggtaccagaatagacgcaatcagaaaggccattgggaaaccgaggaagtgaatgtaacggagaaactgaaagctttgtttgcaagtgattcgaagaccacaaccgtgattgattacgccaacgacgacaacctgatcgatgtgatcctggaacaagacaaggcgtccttctttaaagaattgctctggcttctgaagctgactatgaccctgcggcactcgaagatcaagagcgaggatgatttcatcctaagcccggtcaagaatgaacagggcgaattctacgatagccgcaaggcaggcgaggtttggccgaaggatgccgatgccaatggagcctaccacatcgccctgaaagggttatggaacctacagcagattaatcaatgggagaaaggcaagacacttaatctggccataaagaatcaggactggttctcgttcatccaggagaaaccttatcaggaataa

SEQ ID NO: 782 - DNA, 3897 bp, Artificial Sequence
  Description of Artificial Sequence: Synthetic polynucleotide
atgacaaagacctttgattctgagttcttcaatctctacagtctgcagaaaacagttaggtttgaattgaagccggtgggtgagactgcctcattcgtggaggacttcaagaatgaagggttgaaacgagtagtaagtgaggatgagaggcgcgccgtcgactaccagaaggtcaaggaaataatcgatgattatcacagagatttcatcgaagaatcccttaactacttcccagaacaagtgtctaaagacgctttagagcaagcatttcatttataccagaagcttaaagcggccaaagtcgaggaaagagagaaagcacttaaggaatgggaagctctccagaagaagttacgtgagaaagtcgttaaatgcttctcagattcaaacaaagcgaggttctctcgcattgataagaaggagttgattaaagaagatcttataaactggttagtggcacagaaccgagaggatgatatacctacagtcgagacatttaataactttactacgtacttcacaggatttcatgagaaccgtaagaatatatatagtaaagatgaccacgctaccgccatatcctttagactcatacacgagaatctgccaaagttctttgataatgtcattagtttcaataaacttaaggaagggttcccagagttaaagttcgataaggtgaaagaggatttagaggttgattatgatttaaagcacgctttcgagattgagtacttcgtaaatttcgttacccaggcaggcatagaccaatataattacttgctgggaggtaagactctagaagacggcacaaagaaacaaggtatgaatgaacagatcaacctgttcaagcaacagcaaacgagggataaagcccgacaaatccctaagttgataccgctgttcaaacaaatactatcagagagaactgaatctcagagctttatacctaagcagttcgagagcgaccaggaactattcgatagtctgcagaaactacacaacaattgtcaagataagttcaccgttctgcaacaagcaattcttggattagctgaagcagatttgaagaaggtatttattaagacttctgatctcaatgcactttcaaatacaatcttcggtaattattcagtcttttcagatgcgcttaatttgtataaagagtcactaaagacaaagaaagctcaggaagcctttgagaagttgccagcacactctatacacgatctgatccagtacttggaacagtttaactcctcacttgatgcagagaagcagcagtcaacagatacagtcctcaactacttcataaagacggatgaactatatagtcgatttatcaaatctacttccgaggcatttacacaagtccaaccattgtttgaattagaagctctcagttcgaagaggagacctccagagagcgaggatgaaggtgctaagggacaagagggatttgaacagattaaacgtattaaagcttaccttgacacactcatggaagctgttcacttcgcgaagcctctttacttagttaagggtagaaagatgatagaaggcttagataaggatcaatctttctacgaggcatttgaaatggcataccaggagttggagagtctaattataccaatctacaataaagctcgctcgtatctatcgaggaagcctttcaaagccgataaatttaagattaatttcgataataacaccttactatctggatgggatgcaaacaaagaaaccgctaatgcgtcaatcctatttaagaaggacggcctctactatctaggaattatgcctaagggtaagactttcttatttgattacttcgttagttcagaggatagtgagaagcttaagcaaaggagacaaaagacagctgaagaggccttggcgcaggatggagagtcttacttcgagaagataagatacaaactactgcctggagcttcaaagatgcttcccaaagtattcttcagtaacaagaacattggtttctacaatccatcagatgatattctacgcataagaaatactgcaagtcatactaagaacggaacgccacagaagggacatagcaaagtcgaatttaacctgaacgattgccacaagatgattgatttcttcaaatcatctatccagaaacaccctgagtggggcagtttcggattcacgtttagtgatacatctgactttgaagacatgtctgccttctacagagaggttgagaaccaaggttacgtcatctcattcgataagattaaggagacgtacatacagtcacaagtggaacagggcaacctttatctcttccaaatatacaataaggactttagtccatatagtaagggtaagccgaatctccatactctctactggaaggcgttgtttgaggaggcaaatttaaacaatgttgtagcaaagctcaacggtgaggcagagatattctttagaaggcactctattaaagcttccgataaggtggtgcacccagcgaaccaggctattgacaataagaacccacatactgagaaaacacagtccaccttcgaatacgatctagtgaaagataaacgttatactcaagataagttcttcttccacgtgccaatatcgcttaatttcaaagcccagggcgtttctaagttcaatgataaagtcaacgggttcctaaagggaaatcctgacgttaacatcataggtattgatcgcggcgagcggcatctcctttacttcaccgtggtcaaccagaagggagagattctagtgcaagaatcacttaacacgttgatgagcgataaagggcatgttaatgattatcaacagaagttagacaagaaagagcaagagagagatgccgccaggaagagttggaccacagtggagaatattaaagaattgaaggaaggttatttatctcatgtggttcataaattggcccacttaattattaaatataatgctatcgtctgtttggaagacctaaactttggctttaagagaggtcgattcaaggtggagaagcaagtgtatcagaaatttgagaaggcccttatcgacaaattaaactatcttgtgtttaaggagaaagagctaggcgaggtgggacattatcttacagcttatcagcttacagctccttttgaatcattcaagaagcttggcaagcagtctggaatactattctacgttcctgcagattatacatctaagatagatcctacaacaggcttcgttaacttcctagacctacggtaccaatctgttgagaaagccaaacaactacttagtgacttcaatgctatccggttcaattctgtgcagaactatttcgagttcgagattgactacaagaagcttacgcctaagaggaaagttggtactcaaagcaaatgggttatttgcacatacggtgatgtgcggtaccagaatcgtcgtaatcagaagggtcattgggaaactgaagaggttaatgtcactgagaaactaaaggcactatttgcctcagattccaagacgactaccgtgattgattatgctaatgacgataacctcattgatgtcatactcgagcaagataaggcttcgttctttaaagaattgctctggttactcaagctcactatgactcttaggcattcgaagatcaaatccgaagacgacttcattctttctcccgtgaagaacgaacaaggagaattctacgattcccgtaaggcaggagaagtttggccgaaagatgcagatgctaatggtgcataccacattgctcttaaaggcttgtggaatttacagcaaattaatcaatgggagaaaggaaagactcttaacctggcgattaagaaccaagactggttctctttcattcaggagaagccttaccaagaatga

SEQ ID NO: 783 - DNA, 3897 bp, Artificial Sequence
  Description of Artificial Sequence: Synthetic polynucleotide
atgacaaagacattcgatagtgaattctttaatttgtattctctacagaagacagttcgatttgaacttaaaccagttggagaaaccgcctcatttgtggaggacttcaagaacgaaggtctcaagagagtggtttctgaggatgaaagaagagctgtagattaccagaaggttaaagaaataatcgacgattaccaccgagacttcattgaggagagcctaaattactttccagaacaagtttcgaaggatgcactggagcaagccttccacctctatcagaagttgaaagcagcaaaggttgaggaaagagagaaagctcttaaggagtgggaagcattacagaagaaactacgtgagaaagtcgttaagtgtttctcggattcaaacaaggctagattcagccgaatagataagaaagaactgattaaggaagatttgatcaactggttggttgctcagaaccgagaggatgatatacctacggtcgagacgttcaataacttcacaacatacttcacaggattccatgagaaccggaagaatatttatagcaaggatgatcatgcaactgccatcagcttccgtttaatacatgagaacttacctaaattctttgataacgtgatatcgttcaataaacttaaagaaggattccctgagttgaagtttgataaagttaaagaggatcttgaggtggattatgatttgaaacatgccttcgaaatagaatacttcgtaaatttcgtaactcaagctggcattgatcagtacaattatctcctaggaggcaagaccctagaggatggcacgaagaagcagggtatgaatgaacagataaatttgtttaaacagcaacagacacgagataaggcgcggcaaatccctaaattgataccgttgtttaaacagatactctctgaacgtactgaatcgcaatcatttatccctaaacagtttgaatctgatcaggagctcttcgattctttgcagaagctccataataattgccaagataagtttaccgtccttcaacaagcaatccttggcttagcggaagctgatctcaagaaggtatttatcaagacttcagatttgaatgctctatccaatacaatctttgggaactattcagtcttctctgatgccctgaacctttataaggaatcattaaagaccaagaaggctcaggaggcgtttgagaaacttcctgcacattctatccacgatctgatccaatatctagaacagtttaactcatctcttgacgcggagaaacaacaaagtaccgacactgtccttaattacttcattaagacggatgaactgtatagtagattcataaagtcaacttctgaagcctttacacaagtgcaaccgctcttcgaactagaagcactatcaagtaagcgaaggccacctgagtctgaagatgaaggagccaagggtcaagaaggcttcgagcaaattaagcgcattaaagcatatctcgatacacttatggaagcagtgcacttcgccaaaccattatatctcgttaaaggccgtaagatgatcgagggacttgataaagatcaaagtttctacgaagctttcgaaatggcgtaccaagaacttgaaagccttattatcccaatttataataaagctcgtagttaccttagtaggaaaccattcaaagcggataaatttaagattaactttgataataacacactcttgtctggctgggatgcaaacaaggaaactgctaacgcttctatcttgttcaagaaggatggtttatactatctgggaattatgccgaaaggtaagacattcttattcgattatttcgtttcttccgaggattcagagaaattgaaacaacgtcgacaaaagactgcagaggaggcgctagctcaggatggagagtcttatttcgaaaagatccgctataaacttctgccaggcgcaagtaagatgctccctaaagtcttctttagcaataagaatatcggtttctataacccttccgatgatatccttcggataaggaatactgcctcgcatacaaagaatggtacaccacagaaaggccattcgaaagtggagtttaatttaaatgattgtcacaagatgattgatttcttcaagagttctattcagaaacatccagagtggggttctttcgggtttacattcagtgatacaagcgactttgaagacatgagtgcattctatagagaggtagagaatcaagggtatgtgatctcgttcgataagatcaaggagacctatatccaaagccaagtggaacaaggaaatctttacttattccagatttataataaggatttcagcccatacagtaaaggtaagcccaaccttcataccctctactggaaagccttatttgaagaggctaacctaaataatgttgttgctaaacttaatggtgaagcagagatattctttagacgtcattcaataaaggcttccgataaagttgtccatcctgctaaccaggccattgacaacaagaatccgcacaccgaaaagacccaatcgacatttgagtacgatcttgtgaaggataaacggtatacacaagacaaattcttctttcatgtgcctatctcactaaactttaaggcgcaaggcgtttctaagttcaatgataaagtgaatgggttcctgaaaggaaatcctgacgttaacattataggaatagaccgaggggaaagacacctcttatatttcactgttgtgaatcagaaaggtgagattctagtacaggaatcactcaatacactcatgtcagataaaggccatgtgaacgactaccagcagaaattggacaagaaggaacaagagagagatgcagcgaggaagtcttggactacagttgagaacattaaagaactgaaagaagggtacctctcacacgttgttcataagcttgcccatcttatcatcaagtacaatgcaatagtatgtctggaggatttgaacttcgggtttaagagaggaagatttaaagttgagaaacaggtttatcagaaattcgagaaagctctaatagataaattgaactatcttgtatttaaggagaaagagctcggagaggttggccactaccttactgcttatcaactcacagcgccgttcgaaagcttcaagaaactgggaaagcaatctggaatattgttctacgttcctgctgattacaccagtaagattgatcctactacgggctttgtaaactttctcgatctccggtatcaatccgtcgagaaagctaaacaacttctttcggactttaatgctataaggtttaatagtgtacagaattatttcgagttcgagatagactataagaaacttactccaaagaggaaagtaggcacacagagcaagtgggtgatctgcacatacggagatgtccggtaccagaatcggcgaaaccagaagggacattgggaaactgaagaggtcaacgttacggagaaattgaaggctttgttcgcttcggattccaagacaaccacagttatcgattacgccaatgatgacaacctcattgatgttattcttgaacaagacaaagcgagcttctttaaagaattgctgtggcttctcaagttaactatgaccctacgtcactcaaagattaagagtgaagatgatttcattctgagcccagttaagaacgagcaaggcgaattctatgactcacggaaagctggtgaagtgtggccaaaggatgctgatgcaaatggcgcttaccacattgctcttaaaggactttggaatctgcaacaaataaaccagtgggagaagggaaagactcttaaccttgcaattaagaaccaggattggtttagtttcatccaagagaaaccatatcaagaataa

SEQ ID NO: 784 - DNA, 3897 bp, Artificial Sequence
  Description of Artificial Sequence: Synthetic polynucleotide
atgacaaagactttcgatagcgaattctttaatctttactctttgcagaagacagtacgtttcgaactcaagcctgttggtgagactgcaagctttgtggaggatttcaagaatgaaggattgaagagggtcgtgtctgaagatgagaggagggcggtggattatcagaaagtaaaggaaattatcgatgattatcacagggatttcatcgaagagtctttaaattacttcccggaacaagtttccaaagatgctcttgaacaggccttccacttgtatcagaaattgaaggctgctaaagtagaggaacgggagaaggcattgaaggaatgggaagccctccagaaaaaactcagagagaaggtcgttaagtgcttctcagatagcaacaaggcacggttctcgagaatagataagaaggaactgatcaaagaggatctgataaactggcttgtggctcagaacagggaagatgacattccgacggtagagactttcaataatttcacaacctactttactggctttcacgagaatcgtaagaatatatacagtaaagatgatcatgcaaccgcaatctctttcagattaattcacgagaatcttcctaagttctttgataatgtcatttctttcaacaagcttaaggagggattcccagaactgaaatttgataaagtcaaggaagacctcgaagtggattatgatctcaaacatgccttcgaaattgagtacttcgtcaactttgtgacacaggccggcattgaccagtataactatctcctcggcgggaagactttagaggacgggacgaagaagcaaggtatgaacgagcagattaacctattcaaacaacaacaaacgcgtgataaggcccgacagatccctaaactcataccgctgtttaaacagatactcagcgagagaaccgagtcacaaagtttcattccgaaacagtttgaatctgatcaagaattgtttgattcacttcagaaactgcataataactgccaggataagtttaccgtacttcagcaggcaatactgggtttggccgaagccgatttgaagaaggtgttcattaagacttcagatcttaatgctttgtccaatacaatattcggcaactactcggtgttctctgacgctctaaatttatataaagagtcgctcaagactaagaaggctcaggaggctttcgagaaattgcccgctcactccatccacgatttgattcaatatttggagcaatttaactccagtctggatgcagagaaacaacagtccacagatacagtgctcaattacttcatcaagaccgatgaattatacagtagatttattaaatcaacgtctgaagcctttacgcaagtccagcctctatttgaactcgaagctctatcgtctaagagacgtcctccagagtccgaggatgagggagctaaaggacaggaaggctttgagcagataaagagaattaaggcatatcttgacacgctaatggaagctgttcacttcgctaaacctctctaccttgtcaagggacgtaagatgatcgaaggattagacaaagaccagtccttctacgaagcattcgaaatggcctatcaggaattggaatccctcattatacctatctataataaggcccgttcttacttatcgcgtaagccattcaaggctgataaatttaagattaactttgacaataatacacttctttctggatgggatgccaataaggagactgcaaacgcttctatcctgttcaagaaggacggcctgtattatttgggaatcatgccgaagggaaagacgttcttgttcgattatttcgtctcttcagaggattctgagaagcttaaacaaagaagacagaaaacagcagaggaggccttggcacaggatggagagtcgtacttcgagaagattaggtataagctcttaccgggagctagcaagatgttacctaaggtattctttagtaataagaatatcgggttctacaatccgtctgatgatattcttcgaattcgaaacacagctagccataccaagaacgggacgccacagaaaggccattctaaggttgaatttaaccttaatgattgccacaagatgattgatttcttcaagagttccattcagaagcacccagaatgggggtcctttggtttcacattctccgatacaagcgacttcgaagatatgtctgctttctaccgtgaagttgagaaccaaggttatgtgatctcatttgataagattaaagaaacatacattcagtctcaagttgagcaaggaaacctgtatctcttccagatatataataaagatttctcgccatactcgaagggaaagccgaatcttcatactctgtactggaaagcgctcttcgaagaggctaatctgaataatgtagtagcgaagttgaatggagaagccgagatcttctttaggaggcattccataaaggctagtgataaggttgtacatccagcgaatcaagctatcgataataagaatccacacactgagaagactcaaagtacattcgaatatgacttggtcaaggataaacgttacactcaagataagttcttctttcatgtcccgataagtcttaacttcaaggcgcaaggtgtatccaaattcaatgacaaagttaatggtttccttaagggaaatcctgatgttaatatcatcggtatcgatcgcggagagcggcatttgttatacttcactgtcgttaatcagaagggtgagatactcgttcaggagagcctcaatactcttatgtcagataaaggtcatgtcaacgactatcagcagaagcttgacaagaaagagcaggaacgcgatgccgctcggaagagttggacaaccgttgagaacatcaaagaattgaaagagggatatctaagccacgtggttcataagctagctcaccttataattaagtataacgctattgtttgcctggaagaccttaacttcggattcaagcgcggacgatttaaagttgagaaacaggtataccagaaattcgagaaggctcttattgataaattgaactatctagtatttaaagagaaggagctcggagaggttggacattacctcactgcgtaccaattgaccgctcccttcgagtcttttaagaaactcggtaaacaatcaggtattctcttctacgttcctgcggactatacatctaagattgatccaaccactgggttcgtgaactttcttgatcttaggtaccagtccgtagagaaagctaagcaacttcttagtgacttcaacgcgatcagatttaactctgtccagaactatttcgagtttgagatcgactacaagaagcttactcctaaacggaaagtcggcacacagagcaaatgggtcatatgtacgtatggagacgtcagataccagaaccgtaggaatcagaaaggtcattgggaaactgaggaggtcaacgttacagagaagctcaaggcattgtttgcttcggattcaaagaccactacagtaattgactacgctaatgatgataacttgatcgatgttatattggaacaggacaaagcgtcattcttcaaggagttgctttggttactaaagcttaccatgacgctccggcatagtaagatcaagagtgaagacgatttcatcctctctcctgtaaagaacgaacaaggcgaattctacgatagtcgaaaggcaggcgaggtgtggccaaaggatgctgatgcaaacggcgcataccatatcgctttgaagggactgtggaatttgcaacaaatcaatcaatgggagaagggaaagacactaaatctcgcgataaagaatcaggattggttcagtttcattcaggagaaaccctaccaagaatga

SEQ ID NO: 785 - DNA, 3897 bp, Artificial Sequence
  Description of Artificial Sequence: Synthetic polynucleotide
atgaccaagaccttcgattctgaattcttcaacctatattctttacagaagacagttcggttcgagcttaagcctgttggtgaaacagcttcgttcgtagaagactttaagaatgaaggattgaagcgagttgtttctgaagatgagaggagggctgttgattatcagaaagttaaagaaattatcgatgactatcatagagacttcattgaagaatctctaaactacttcccggagcaagtgtctaaggatgcgttggagcaggctttccatctttatcagaagcttaaagctgctaaagtagaggaaagagagaaggctctgaaagaatgggaggccttacaaaagaagttaagggagaaggtggtcaaatgcttctctgattctaacaaggctagattctctagaatagataagaaggaactaattaaggaagacttaatcaattggcttgtggcacagaaccgtgaagatgacataccaactgttgaaacatttaacaatttcaccacttacttcactgggttccatgagaataggaagaatatatattccaaagacgaccacgctacagctattagtttccgtttgattcatgagaatttgcctaagttcttcgataacgttatcagcttcaacaagttgaaggaaggattccctgagcttaagtttgataaagtgaaggaggatcttgaggtggattatgacttgaagcatgccttcgaaatcgagtactttgtaaacttcgttactcaggcaggaatagatcagtataactatttgctcggtggcaagaccctagaagatggaaccaagaagcaaggcatgaatgagcaaatcaacttgtttaaacagcaacaaactagggacaaggctagacaaattcccaaattgattcctttgttcaaacagatactgagtgagaggacagaatctcaaagtttcattcctaaacaatttgaatctgaccaggaactatttgacagtctgcagaagcttcataacaattgtcaggataagtttacagtgctgcagcaagctatcttgggtctagctgaggctgatctcaagaaggtgtttatcaagacttctgatcttaatgcattgagtaataccatcttcgggaattattctgtgttttcagatgcattgaacctctacaaagagtcccttaagacgaagaaagcacaagaagcattcgagaaacttccagcccattccatccatgatcttatacagtacttggagcaatttaacagttctttggacgcagagaaacaacagtctactgatactgtgcttaactacttcataaagacagatgaattatatagtagatttataaagtccacgtccgaagcattcacacaagttcaacctttgtttgaacttgaggcattatcgagcaagcgtagaccgccagaatcagaggacgaaggagctaaaggtcaggagggatttgagcagataaagagaattaaagcgtacctagatacactcatggaagccgtacatttcgctaagcctttgtacttggttaaaggtaggaagatgattgagggacttgacaaggatcagtctttctatgaagcatttgagatggcatatcaagagctggagtccctcattataccaatttataataaggcacgatcctacttatcgcggaaacctttcaaagctgataaattcaagataaatttcgacaacaacaccctactatcaggatgggacgctaacaaagaaaccgctaatgcgagtatcctctttaagaaagacggcctttattacttaggcattatgcctaaaggcaagactttcttgtttgattatttcgtgtctagtgaggattctgagaaactcaagcaacggaggcagaagactgctgaggaggctctggcacaagatggagaatcttatttcgagaaaattagatacaagttattgccaggagcttcaaagatgctgccgaaggttttcttttccaacaagaatattggcttctataacccatccgacgatattcttcgaattcgaaacaccgcctctcatacaaagaatggtacgcctcagaagggtcactctaaagtggaattcaacctcaacgattgtcataagatgatcgatttcttcaaatcaagcatccagaagcacccagagtggggcagctttggctttactttctcagacacttccgactttgaggatatgtctgcattctacagagaagtggagaaccaaggatacgttataagcttcgataagattaaagaaacatacatccagtcacaggttgagcagggtaatttatatctattccaaatctataacaaggacttctcgccttattcgaagggtaagccaaatctccacaccctctattggaaagccctcttcgaagaagcaaacctaaacaacgtcgttgccaagctaaacggagaagctgaaatattttttcgccgtcactctatcaaggcaagcgataaagtggtccacccggcaaatcaagcaatcgataataagaatcctcataccgagaaaacgcagagtactttcgagtatgacttggtgaaggataagagatacacgcaagataagtttttcttccacgtgcctatctcactcaacttcaaagcacaaggcgtgtcaaagtttaatgataaagttaacggcttcttgaagggaaatccagatgttaacatcatcggtatcgatcgaggagaacgacatttgctttacttcacggtggtgaatcagaagggtgagatactagtgcaggagtccttgaacacgcttatgtctgacaaaggacatgttaacgattaccaacagaagttagacaagaaagagcaagagcgtgatgctgctaggaagtcttggacgacagtggagaacataaaggaacttaaggaaggttacctgtcccacgttgtgcacaagttagctcacctaatcattaagtacaatgctattgtttgtcttgaggatcttaatttcggatttaagagaggaaggttcaaggttgagaagcaagtctaccagaaatttgagaaagctctgatagataagcttaactaccttgtgttcaaggagaaggagcttggcgaggtaggacattacttaactgcatatcagttaaccgctcctttcgaatcatttaagaagctaggtaaacagtctggtatcctattctatgttcctgctgactacacttctaagatagatccaacaactggattcgtaaacttcctagatttacgttatcaatcggttgagaaggcaaagcaattactttcggatttcaatgcaattaggtttaattcagtgcagaactacttcgagttcgaaattgattataagaaactcacgccaaagcgcaaagttggaacacaaagcaaatgggtaatttgcacatatggtgatgttcgatatcagaatagacgaaatcagaaaggacattgggaaacggaagaagtgaacgttactgagaaacttaaagctttattcgcgagcgactcgaagacaactactgttatcgattacgcaaacgatgataatctaattgacgttatccttgaacaagataaggcttcattctttaaggaactcctttggcttcttaagttaaccatgacactccggcattctaagatcaagtccgaggatgacttcatcttatcacccgttaagaacgaacaaggtgagttctacgattctcgcaaggccggtgaggtgtggccgaaggacgcagatgctaatggagcttaccatattgctttgaaagggttgtggaacctccagcagatcaatcaatgggagaagggtaagacgctgaacctagctattaagaatcaggactggtttagtttcatccaagagaagccttatcaagagtga

SEQ ID NO: 786 - DNA, 3897 bp, Artificial Sequence
  Description of Artificial Sequence: Synthetic polynucleotide
atgaccaagacattcgactccgagttctttaatctttatagtctacagaagactgtgagatttgagcttaagcctgttggagaaaccgctagtttcgtggaagactttaagaacgagggattgaagagggtcgtctccgaggacgaacggagagccgtggattaccagaaagtcaaagaaattattgatgactaccaccgtgacttcattgaggagagcctcaactacttccctgaacaagtgagcaaggatgcgctcgagcaggcattccatctttaccagaagcttaaagctgctaaagtcgaagagagggagaaggcattgaaggagtgggaagcattacaaaagaaattacgagagaaagttgtaaagtgcttctccgatagcaataaagcccggttctctcgaatcgataagaaggaactaatcaaagaggatttgatcaattggctcgttgctcagaatagagaagatgacattccgaccgttgaaacctttaataatttcacgacttactttacgggtttccatgagaatcgtaagaacatctattctaaggatgatcatgcaaccgctatatccttcagactaattcacgagaatttgcctaaattctttgataacgtgatttcattcaataagcttaaagagggctttcctgaattgaagtttgataaagtcaaggaagatttggaagtcgattacgacctgaagcacgccttcgaaattgaatacttcgtgaatttcgtgacacaagcgggaatagatcagtataattacctacttggtggaaagactcttgaggatggtacaaagaagcaaggtatgaacgaacaaatcaacttattcaaacagcagcaaacgcgtgacaaagctagacaaatccctaagttgatacctttgtttaagcagatactttctgagcggaccgagagtcaaagcttcatccctaagcagtttgaatcggatcaggagctgttcgatagcctccagaaattacataacaattgccaagacaaattcactgttctgcaacaagcgattcttggacttgccgaggcggatctaaagaaagtattcataaagacctcggatctcaacgctctcagtaatactatctttggtaactatagcgtgttctccgatgccctcaatctctacaaggaaagtttgaagacgaagaaggcacaggaagcatttgagaaacttcccgctcacagtatccacgatttgattcagtacctggaacagtttaacagttcgcttgacgcagagaagcaacagtcaactgacactgttctaaactacttcattaagaccgatgaattgtattctagatttatcaaatctacatccgaggccttcactcaagtgcaaccgttgtttgaattagaagcattgagttcaaagagacgaccgcccgagtctgaagatgaaggagctaaaggtcaagaaggattcgaacagattaaacggattaaggcttacttagatactttgatggaggctgtgcactttgctaaaccactatatctcgttaaaggtagaaagatgatcgaaggtttggataaagaccaatcattctatgaggcgttcgaaatggcataccaggaactggaatccctaattatacctatttataataaagctagatcctatctatctaggaaaccctttaaggcagataaatttaagatcaacttcgacaacaatacattgctcagtggctgggatgccaacaaggaaacggcgaacgcttctattttgtttaagaaggacggactttattacttgggcattatgccgaaaggaaagactttcttatttgattacttcgtctcatccgaagattctgagaaactaaagcagagacgtcagaaaactgcagaggaagcacttgcacaggatggagagagttacttcgagaagatccgttataagttacttcctggagcatcgaagatgctacctaaggtctttttctcaaataagaatataggattctataacccttctgacgatatcttaaggattcgcaacacagcatctcacacaaagaacggaacgcctcagaagggccacagtaaagtggagtttaatctcaacgactgccacaagatgatagatttcttcaagagctccatccagaaacatcccgagtggggctcgtttggattcaccttctctgatacatctgacttcgaggatatgagtgccttctatagagaagttgagaaccagggatacgtcatttctttcgataagattaaggaaacatacatacaatcacaagtagaacaaggtaacctgtacttgtttcaaatatacaataaggacttctcaccttactccaagggcaagcctaatctgcacactctgtactggaaagctctgtttgaggaggctaatcttaataatgtggtggctaaattaaacggtgaagcagaaattttctttaggaggcatagtattaaagcttcagataaggttgtccatccggctaaccaagcgattgataataagaatccacacactgaaaagacccagtctacgttcgagtacgatctcgtgaaggacaagagatacacacaggataaattcttctttcatgttccaattagtcttaacttcaaggcacaaggagtctctaaatttaatgataaggttaacggatttcttaaaggtaatcctgatgtaaacatcataggtattgatagaggtgagagacatttattatatttcactgttgttaaccagaaaggcgaaatccttgtacaagagagtttgaatacactcatgtcagacaaagggcatgtcaatgattatcaacagaaactcgacaagaaagaacaagaacgggacgctgcacggaaatcatggaccacggtagagaacattaaggaacttaaagaaggttatctatcacatgtggtccacaaattggctcacctaatcataaagtataacgctatcgtatgccttgaggacctcaacttcggctttaagagaggcagattcaaagttgagaagcaggtctaccagaaatttgagaaagccttaattgataaactgaattacttggtatttaaggagaaagagttaggcgaggtgggacactatttgactgcgtaccaattaacggcaccattcgagtcattcaagaaactgggtaaacagtcgggtatcctgttctacgttcctgcagactatacatcaaagattgatcccactaccgggtttgttaatttcctcgatctaagataccaaagtgttgagaaggctaagcaattgctttcggatttcaatgctatccgctttaattcagttcagaactacttcgagttcgaaatcgactacaagaaacttacgccaaagcggaaggtcggaacacagtccaaatgggttatctgtacatatggcgacgtaagataccagaacaggagaaaccagaagggccactgggagaccgaggaggtcaacgtcactgagaaattaaaggcattattcgcttccgactctaagaccactactgtgatcgattatgcaaacgatgataatttgatagatgtcatactggaacaagacaaggcgtccttcttcaaagagttgctttggctgcttaaattgacaatgactttgagacattcgaagatcaagtctgaggacgatttcatcctgtcacccgtaaagaatgagcaaggtgaattctacgactccagaaaggcaggagaagtctggccaaaggacgcagatgctaatggagcataccacattgcccttaaaggtctgtggaatcttcaacaaattaaccaatgggagaagggtaagacacttaaccttgcaattaagaatcaagactggttctcattcattcaggagaaaccctatcaagaatag

SEQ ID NO: 787 - DNA, 3897 bp, Artificial Sequence
  Description of Artificial Sequence: Synthetic polynucleotide
atgactaagaccttcgattctgagttctttaacctttactcccttcagaagactgtcaggtttgagttgaagcctgtgggcgaaacagcatctttcgttgaagactttaagaatgagggactaaagagagtcgtaagcgaagatgaaagaagggcagtggattatcagaaggtgaaggagattatcgacgattatcacagggatttcattgaggagagtctaaattacttcccagaacaggtcagcaaggatgcgctcgaacaagccttccatctttatcagaaattaaaggctgctaaggtggaagaacgtgagaaggcattaaaggaatgggaggcacttcaaaagaagctcagggagaaggttgtcaagtgcttctcagactccaacaaggctcggttctcgcggatcgataagaaggaactgattaaagaggatctgattaattggttagttgcgcagaatcgggaggatgatattcctaccgtagaaaccttcaacaacttcacaacgtatttcacaggattccacgagaaccgaaagaatatatattctaaagatgaccatgctactgcaatctcattcaggttaattcatgagaacttgcccaaattctttgataacgtcatttcattcaacaagctcaaggaaggtttccctgaacttaaatttgataaagtcaaggaggatcttgaagttgattatgatcttaagcatgctttcgaaattgagtatttcgtgaacttcgttacacaagccggaatagatcaatacaattacctattaggtggaaagaccctagaagacggtactaagaaacagggcatgaacgagcaaattaacctgtttaaacagcaacagactagagacaaggctagacagattccgaagttgatcccattgttcaagcaaatacttagtgagagaactgaatcccagagcttcatcccaaagcagtttgaatctgatcaagagctatttgatagcttacagaagctccataataattgtcaagataagtttacagttcttcagcaagcaatcttaggattagctgaagcagatttaaagaaagtattcattaagacgtctgatcttaatgccttgagtaacaccatattcgggaattactctgtcttcagtgacgctctcaatctttataaggagtcattgaagacgaagaaggctcaagaggctttcgagaagttaccagctcattcgattcacgatcttatacagtacttggaacagttcaattcttcactagacgcagagaagcagcagagtactgacacagttcttaattatttcatcaagactgacgaattgtatagccgatttatcaagagtacatcagaagcattcacgcaggtacaacctctgtttgagctggaagcactatcctctaagagacgaccacctgaatcagaagatgagggtgccaagggtcaggaagggtttgaacagattaaacgtataaaggcttacttggatactcttatggaagcagtccactttgctaaacctctctatttggtcaagggacgtaagatgattgaaggtctcgataaagatcagtccttctatgaagctttcgaaatggcttaccaagagctagaaagtttaatcatccctatttataacaaagcgcggagctacctctcacggaaacctttcaaagctgacaagtttaagattaacttcgacaacaatacgctcctttctggatgggacgcaaataaagagacggctaacgcctctatactcttcaagaaagatggtctttactatctgggtattatgccgaaaggaaagacatttctctttgactatttcgtatcttcagaagacagcgagaagctcaagcaaagaagacagaagaccgctgaggaagcactggcacaagacggagagagttactttgagaagatccggtataagctactgccaggtgcctcaaagatgctcccgaaagtattcttctcgaataagaacataggcttctacaacccaagcgatgatatcctgagaattagaaatacggcttcgcataccaagaacggtacaccgcagaagggtcacagcaaggttgaatttaacttaaatgattgccacaagatgatcgatttctttaaatcaagcattcagaagcatccagaatggggttccttcggcttcaccttctctgatacatctgactttgaggatatgagcgcgttctaccgagaggtagagaatcaaggttacgttattagcttcgataagataaaggaaacttacatccagtctcaagttgagcaaggtaacctgtacttgtttcaaatctataataaagatttctctccttactccaaagggaagcctaatttgcataccctatactggaaagctttgttcgaagaagctaacttaaacaacgtggttgcgaagctcaatggagaagcagagatattttttagacgtcactcgatcaaggcgtccgataaagtcgtacatcctgctaaccaggcaatcgataacaagaatccacataccgagaagacacaaagtacatttgaatatgacttagttaaagataagcgatacactcaagacaagttcttcttccatgttccgatttctcttaacttcaaagcgcagggcgtcagtaagtttaatgataaggtgaatggatttcttaaaggaaaccctgatgttaatattatcgggatcgaccgcggtgaaagacatcttctttactttaccgtagtgaaccagaagggtgagattcttgtccaggagtcactgaataccctaatgtcggataaaggtcacgttaatgattatcaacagaagctagataagaaagaacaagaaagggatgctgctcggaagagttggactacggtcgagaacattaaagaactcaaggagggttatttgtctcatgtggtacacaagttggcacatcttataattaagtacaatgctatagtttgtctggaggatttgaacttcggatttaagcgcggcaggtttaaggtcgagaagcaagtgtaccagaagttcgagaaagcccttatagataaactgaattatcttgtgtttaaggagaaggagctcggcgaggttggacattacttgactgcatatcagctcactgcaccattcgaaagctttaagaagcttggaaagcagagtggaatcttattctatgttccggcggattatacttcgaagatagatccgaccacgggtttcgttaacttcttagacttgcggtaccaatccgtagagaaagctaagcaattgttgagtgactttaacgccatccggtttaatagtgtacagaattatttcgagttcgagatcgattataagaaactgacgcccaaacgtaaggtgggtacgcaatccaagtgggtaatctgtacatatggagatgtcagataccagaatagaaggaaccagaagggtcattgggagactgaagaagttaacgttaccgagaagctcaaggctttgttcgccagtgattcaaagacaacaactgttatagactacgctaatgatgataatttaatagacgtcatactcgagcaagacaaagcatctttctttaaggaattgctgtggctacttaaactgacaatgacgttgcgacactctaagattaagagcgaagatgatttcattctttctccggttaagaacgaacaaggtgaattctatgattctcgtaaagcaggtgaagtgtggcctaaagacgctgatgctaatggtgcttaccacatagcattgaaaggactctggaatctccaacaaatcaaccagtgggagaaagggaagacgttaaaccttgctatcaagaatcaagattggttctctttcatccaagagaaaccttatcaggaatga

SEQ ID NO: 788 - DNA, 3897 bp, Artificial Sequence
  Description of Artificial Sequence: Synthetic polynucleotide
atgacgaagactttcgacagcgaattcttcaacctttattctcttcaaaagacggtgcgtttcgagttgaaaccggtaggcgagaccgcttctttcgttgaggactttaagaatgagggactaaagcgggtggttagcgaagatgaaagacgggcagtcgactatcagaaggttaaggaaattatagatgattatcatcgagatttcattgaagaaagtcttaactacttccctgagcaggtttcaaaggatgctttggaacaggcatttcatctgtaccagaaattgaaagctgctaaggtcgaggagagggagaaagctcttaaggagtgggaagcgttgcagaaaaagctgagagagaaggtggttaagtgcttcagcgattcgaacaaggcgcgcttctctaggatagataagaaggagctaatcaaggaggatctgattaattggctcgtcgcccagaatcgagaggatgatatcccaactgtcgagacatttaataactttaccacttacttcacaggattccatgagaataggaagaatatatatagtaaagacgaccatgccactgctatttctttccgattgatccatgagaacctccctaagttctttgataatgtaatctctttcaataagttgaaggaaggctttccggagcttaaattcgataaggttaaggaagatcttgaagtggattatgacctcaagcatgcatttgaaatcgaatacttcgtgaatttcgttactcaagcaggtatagatcaatataactatctgctgggtggcaagacactagaggacggcactaagaaacaaggcatgaatgagcaaattaatttgttcaagcagcaacagactagagacaaggcgagacaaattcctaaattgataccattgttcaaacagatcctttcggaacgtacggaatctcaatctttcattcctaaacagtttgaaagtgaccaggaactgttcgatagtttacagaagcttcacaataattgtcaagataagtttactgttctccaacaagcaattctcggcctggcagaggcagatcttaagaaggtatttatcaagactagtgacctgaatgctttgagtaacacaatctttggcaattatagtgtattctcagatgctttgaatctctacaaagaaagtcttaagacaaagaaggctcaagaggcgttcgagaagctcccagctcatagtattcatgacttgattcagtatctcgaacagtttaattcctctcttgatgctgagaaacagcagagtaccgataccgtactaaattacttcattaagaccgatgaattgtattcaagatttattaaatctaccagcgaagcattcacacaagtgcaaccactctttgaattggaggcgctttcatcgaagagacgtccaccggaatcagaggatgagggtgccaagggacaagaagggtttgaacagatcaagagaattaaggcatatctagatacacttatggaggcagtacacttcgctaaaccactttacctagtgaaaggaaggaagatgattgaaggattagataaggatcagagcttctatgaggcatttgaaatggcttaccaagagttagaaagtttaatcattccgatatataacaaagctagaagctatcttagtcgtaagccatttaaggctgataagtttaagattaactttgataacaacactctattgtctggatgggatgctaacaaagagaccgcaaatgcaagcatcctgtttaagaaggacggattgtactacttgggtatcatgcctaaaggtaagactttcttatttgactactttgtttcatcagaagactccgagaaacttaaacaacgtcgacagaaaacagctgaagaagctcttgcgcaagacggtgaatcatactttgagaagatcagatacaaattgctacctggtgcttctaagatgctacctaaagtgttcttcagcaacaagaatattgggttctacaacccttctgatgacatattacgaattcgtaatacagcttctcataccaagaatggcacaccgcagaaaggacactctaaggttgagttcaatctgaacgattgtcacaagatgattgatttcttcaagagcagcatccagaaacaccctgagtgggggtcgttcgggttcaccttctctgatacttcggacttcgaggatatgagcgctttctatagagaagttgagaatcaaggttacgtgataagcttcgacaagatcaaggaaacgtacatccaatctcaagttgaacaaggcaatttatatttattccaaatttataataaagatttcagtccttattctaagggaaagcctaacctgcacactttgtattggaaggcactgtttgaagaggcaaatttaaataacgttgttgcgaagttgaacggagaggcagaaatcttcttcagacggcacagtatcaaagcgtcggataaagttgttcaccctgcaaaccaggctattgataacaagaatcctcatactgagaaaacacaatctacattcgagtacgatcttgtcaaagataagcgttacacccaagataagtttttctttcatgtaccaataagtctgaactttaaagcacagggtgtgtctaagttcaacgacaaagttaacggattcctcaagggtaacccagatgttaatattatcgggatagatcgaggcgaaagacatctactctacttcactgttgtaaatcagaagggagagatactggtacaagaatcactaaacaccctcatgagtgacaaaggacatgtcaacgactaccagcagaagctcgataagaaggaacaagagcgtgacgctgcacggaagtcttggacgacggttgagaacattaaagagcttaaagagggatatttatcacatgtggtgcataagctcgcacatcttattatcaagtataatgctattgtgtgtctagaggatctcaactttggatttaagcgaggcagattcaaagttgagaagcaagtgtaccagaaattcgagaaagctcttattgataagctcaattatttagtcttcaaagagaaggaattaggagaggttggtcattaccttactgcgtaccagttaacagctcctttcgaatccttcaagaaacttggaaagcagagtggtattttattttacgttcctgctgattatacttcaaagattgatcctacaacaggctttgtaaacttcttggatttgcgttaccaaagtgtagagaaggctaaacaactactcagcgactttaacgccattcggttcaacagtgtgcagaactacttcgaatttgaaattgattacaagaagctcactccgaagcggaaggtcggtacacaatcaaagtgggtcatctgtacctatggtgatgtgcgttaccagaaccgccgaaaccagaagggacactgggaaacagaagaagtcaatgtgactgagaaattaaaggcattattcgcaagcgattctaagacaactactgttattgattacgcaaacgatgataacttaattgatgttatcctggagcaagacaaggcctctttctttaaagaactactatggctgctaaagcttacaatgactcttagacattctaagattaagagcgaggatgacttcatactttctccagtaaagaacgaacagggagagttctacgattccagaaaggccggtgaggtgtggcctaaagatgcggatgccaacggtgcgtatcatattgctcttaaaggtttgtggaatctgcaacagatcaaccaatgggagaagggtaagactctgaatcttgctataaagaaccaagattggttctcgttcattcaagagaagccttaccaagagtga

SEQ ID NO: 789 - DNA, 3897 bp, Artificial Sequence
  Description of Artificial Sequence: Synthetic polynucleotide
atgactaagacattcgacagcgagttctttaacctgtattccttacagaaaactgtccggttcgagctaaagccagtcggagagactgcttctttcgttgaggattttaagaacgagggtcttaagagggttgtgtcagaagatgaaagacgggcggtggattaccagaaggtcaaagaaatcatagatgattatcaccgcgactttattgaagaaagcctcaattatttcccagagcaggtttccaaagacgccttagaacaagcctttcatttataccagaagcttaaagctgcaaaggtagaagagagagagaaggctctcaaagagtgggaagcacttcagaagaagttacgggagaaagtggtcaaatgcttctcagactcaaataaagcgcgcttctctagaatagacaagaaggaattgatcaaagaagatcttattaactggctagtagctcagaatcgtgaagatgatattcctacagtagaaaccttcaacaactttacaacatatttcacgggattccacgagaataggaagaatatctattctaaagatgaccacgccactgctatttcctttagactcattcatgagaatttgcccaagttcttcgacaatgttatctccttcaacaaactcaaggagggcttccctgaacttaaatttgataaagttaaagaggatctcgaagttgattatgatctgaagcatgcgttcgaaatcgaatacttcgtgaacttcgttacccaggctggaatcgaccagtacaactacttgctcggtggaaagactttagaagacggaactaagaaacagggtatgaatgaacaaataaatttgttcaagcaacaacagacaagagataaggctagacagattcctaagctgatacctttattcaaacagatccttagtgagagaactgagtcccaatcattcatccctaaacagtttgaatcagatcaagaattgtttgattctttacagaaattgcacaacaactgtcaagataagttcacggtccttcagcaagctatacttggactcgcagaggcggatctaaagaaagtgtttattaagacgtccgatttgaatgctctttctaacacgatctttggtaattattccgttttctctgatgcgttgaacttatataaagaatcactcaagactaagaaagctcaggaggcattcgagaaactgccggcacactctattcatgacctaatacaataccttgagcaatttaattcctctctcgacgctgagaaacagcaatcgacggacacagtactgaattatttcataaagaccgatgagctctatagtaggttcatcaagtctacctcagaggctttcacgcaagtacagccattgtttgaacttgaagccctttcgagtaagagaagacctcctgaaagtgaagacgagggagccaaaggtcaagaaggatttgagcaaattaagaggatcaaggcttacctggacacactcatggaagctgtgcacttcgctaagccattatacttagttaagggtcgcaagatgattgaaggattggacaaggatcaatcattctacgaggcgtttgaaatggcgtatcaggaacttgaatcgctcattatccctatctataataaggctcgatcatacttgagccgtaagccatttaaagctgataagttcaagattaactttgacaacaacactttgctcagcggatgggacgcaaacaaggagactgcgaatgcttcaatcttgttcaagaaggatggactttattatctcggtatcatgccaaagggaaagacattcttgtttgattacttcgtatcttcagaggatagtgagaaacttaagcagaggagacagaagacagctgaggaggctttggctcaggacggagaatcctatttcgagaaaattagatacaagttgttacctggcgcttctaagatgttacctaaggttttcttttcaaacaagaatataggattctataatccgtcggatgacatccttcgcatcaggaataccgcatcacatacgaagaacggaactcctcagaaagggcactccaaggttgagttcaatcttaatgattgtcacaagatgatcgacttctttaagtcatcaattcagaagcacccggagtggggctcgttcggctttacattctctgatactagtgatttcgaagatatgagtgcgttctacagggaagtggagaatcagggttacgttattagctttgacaagattaaggagacgtacatacaaagtcaagtggagcaaggtaacttgtatctgtttcagatctacaataaggatttctcaccgtattcaaagggaaagcccaatttacatacactatactggaaagctctctttgaggaagcgaaccttaacaatgttgtggctaaactcaatggtgaggctgagatcttcttccgaaggcattcaataaaggcatccgacaaagttgtccatccggctaatcaggcaatcgacaataagaaccctcataccgagaagacacaaagcacatttgaatatgatctagttaaggataagcggtatactcaagataaatttttcttccatgtccctatctcacttaacttcaaggctcaaggcgtgtcaaagtttaatgacaaggttaatggtttccttaaaggtaatccagatgtcaatatcattggcatcgaccgtggcgagaggcacttgttgtacttcacagtcgttaatcagaagggtgaaatactagtccaagaaagtcttaatacactcatgtcagataaaggacacgtaaatgactatcaacagaaattagataagaaagagcaggaaagggacgcggcacgaaagagctggacgacagtggagaacataaaggaactcaaggaaggatatcttagtcatgtggtccataagctagctcaccttatcatcaagtataatgctatcgtgtgtttagaggaccttaacttcggattcaagagaggtagatttaaagtagagaagcaggtttatcagaagtttgagaaagcattgatagataagttgaattatctggtatttaaagagaaagagttaggcgaagttggtcattatctcaccgcttaccaattaaccgcaccctttgagtcattcaagaaactgggtaagcagtctggaatcctcttctatgtccctgcagactacacatctaagatagacccaaccacaggcttcgttaatttcttggatctccgctatcagtcggtcgagaaggctaaacaattactgagtgatttcaatgccattagattcaatagcgtccagaactacttcgagtttgagatcgactataagaagctaactccaaagaggaaagtgggaactcaatccaaatgggttatttgcacctatggcgatgtacgttaccagaaccgtcgaaatcagaagggtcattgggaaacagaggaggtaaacgtcaccgagaagttgaaagccctatttgcttcagattcaaagacgacgactgtcattgattacgccaacgacgacaatcttatcgatgttatacttgaacaagataaggctagtttcttcaaggaactattatggcttcttaagctcacaatgacacttcgtcactctaagataaagtctgaagatgacttcatcctcagtccggtgaagaacgaacaaggagaattctacgactcgagaaaggcaggagaggtttggcctaaggatgctgatgcgaatggcgcatatcacattgcattgaagggattgtggaacctacaacaaataaaccagtgggagaaagggaagactctaaatttggcaattaagaatcaagactggtttagctttatccaagagaagccatatcaagagtaa

SEQ ID NO: 790 - DNA, 3897 bp, Artificial Sequence
  Description of Artificial Sequence: Synthetic polynucleotide
atgaccaagaccttcgattcggagttcttcaacttgtactcacttcaaaagactgtgcgctttgagcttaagccagtaggagagactgccagtttcgtcgaagatttcaagaacgaaggtcttaagcgtgtcgtgtctgaagatgagcggagagctgttgattaccagaaagtgaaagaaattattgatgattatcacagagatttcatcgaagagagtctaaactactttcctgagcaagtgtcaaaggatgcactagagcaagcattccatctttaccagaagttaaaggcggcgaaagttgaggagagagagaaggcacttaaagagtgggaggcgcttcagaaaaagttgagagagaaggttgttaagtgtttctctgatagcaacaaggcacgtttcagccgtatcgacaagaaagaactcattaaggaagatctaattaactggctcgtcgctcagaatagggaggatgatatacctaccgtagagacatttaataacttcacaacttatttcacagggttccatgagaatcgaaagaacatttatagtaaggatgatcatgccaccgcgataagcttcaggctgatccacgagaacctccctaagttcttcgataatgttatcagctttaacaaactcaaggagggattcccggagctcaagttcgataaggtcaaagaagatttagaagttgattacgacctgaagcatgcgtttgaaattgaatacttcgtaaacttcgtcacgcaggccggtatagaccaatacaactatctactaggtggcaagacactagaagatgggacaaagaaacagggaatgaacgagcaaattaatttgtttaagcaacaacagacgagagacaaggcaagacagatccctaaattgatcccactattcaaacaaatactatctgaaagaactgaatctcaatcattcatccctaagcagttcgagtctgatcaggaactctttgattctttgcagaagctccataataactgtcaggataagtttactgtgttacagcaggcgattcttggattggcagaggctgacttgaagaaggtgtttattaagacatctgatcttaacgctttgagtaatacaatatttggaaactattcggtcttctctgatgccctgaatctctacaaggaaagcttaaagaccaagaaagcccaagaagccttcgagaagcttccagcccattctattcacgacttgattcaatacttggaacaatttaattccagtcttgatgcggagaagcaacagtctaccgacaccgtattgaattactttattaagactgatgaactttattctcggttcataaagtcaacgtcggaagctttcacgcaagttcaacctctctttgaacttgaggcattaagctcaaagcgacgaccaccagaatctgaggacgaaggagctaaaggccaggaagggtttgagcaaatcaagagaatcaaggcttatttggatacccttatggaggccgttcacttcgctaagcctctgtatcttgttaaaggaagaaagatgattgaaggcttggataaagatcagagtttctacgaggcgttcgaaatggcttaccaggaacttgagtctttaattatcccaatatataataaggcccgcagctacttatcgcgcaaacccttcaaggcagacaagtttaagatcaacttcgataacaacactctcctgtcaggttgggacgcaaataaggagacagcaaatgctagcatcctgttcaagaaagacggactatactatctcggtattatgccgaagggtaagacgttcttatttgattacttcgtttcctctgaggattccgagaaacttaaacaacgtaggcagaagacagcagaggaagctctcgctcaagatggtgaaagttatttcgagaagatacggtataagctgttgcccggcgcgtcgaagatgttgcctaaggtcttctttagcaacaagaatataggtttctataacccttccgatgatatccttagaattagaaacacagcatcgcatacgaagaatggtacaccacagaaaggtcacagtaaggttgagtttaacctaaacgattgtcacaagatgatagatttctttaagtcctccatacagaaacatccagaatgggggtcctttggattcacattctcagatacatcagacttcgaggacatgtcagcattctatagggaggttgagaatcaaggttatgtgatatcgtttgacaagatcaaggagacttatatacaatcgcaggtcgaacagggaaacttgtatttgtttcagatctacaataaagacttcagcccatactccaaaggcaagccgaatcttcataccctttactggaaagccttgtttgaggaagcaaacctcaataatgtcgtcgcaaagttgaatggcgaagctgaaatcttcttccgaagacactcaatcaaggctagtgataaggtggtgcatccggctaaccaggctattgataacaagaatccgcacacagaaaagactcagtccacatttgagtacgacctggtgaaggacaagagatatacccaagataagttcttctttcatgttccaatcagtttaaacttcaaagctcagggagtcagtaagtttaacgacaaagtcaacggattcctcaaaggtaatcctgatgtgaacattataggtattgaccgaggagaacggcacctactatacttcacagtcgttaaccagaagggtgagatattggttcaggaatccctgaacactttaatgtctgataagggtcatgtgaacgattaccaacagaagcttgacaagaaagaacaggagcgtgatgctgctagaaagtcgtggactaccgtggagaacatcaaggagttaaaggagggttatctcagtcacgttgtgcataagctggctcatctgatcattaaatacaacgcgatcgtgtgcctagaggatcttaatttcggctttaagagaggtcggttcaaagtagagaagcaggtgtatcagaaatttgagaaagcactgatcgataaattgaactacttggtcttcaaagagaaggagttgggtgaagtcggtcattaccttactgcttaccaattaaccgcgccgttcgaatctttcaagaaattaggtaagcaatccggaatattgttctacgttcccgctgattacacctctaagatcgatcctacaacaggtttcgttaatttcctcgaccttagatatcaatcagtggagaaggcaaagcagcttcttagtgactttaacgcaattagatttaattctgtccagaattactttgaatttgagattgactacaagaaactcactcccaagagaaaggtgggtacacagagtaagtgggtgatctgtacttacggcgatgtcagatatcagaacagaagaaaccagaaggggcattgggagaccgaggaagttaacgttacagagaagttgaaagctctgttcgcatctgatagcaagacaactactgttatagactatgcgaacgatgacaatctcatagacgttatcctagagcaggataaagcttccttcttcaaagaacttctatggctattgaagcttacgatgacgcttaggcactccaagattaagtctgaggatgacttcatactaagtcccgttaagaatgagcaaggtgaattctatgattctcgtaaagctggagaggtttggccgaaggatgctgacgctaatggagcttaccacatagcacttaagggcttgtggaatcttcaacaaattaaccaatgggagaagggaaagacgcttaatttagctattaagaatcaggactggttcagtttcattcaagagaagccttatcaagaataa

SEQ ID NO: 791 - DNA, 3897 bp, Artificial Sequence
  Description of Artificial Sequence: Synthetic polynucleotide
atgactaagacctttgattccgaattctttaatctatacagcttgcagaagaccgtaaggttcgagctaaagcccgtgggagaaacagcaagcttcgttgaggattttaagaatgagggcctgaagagagttgtaagcgaagatgagcgtcgagctgttgattaccagaaggtgaaagagataattgatgattaccatcgagactttattgaagagagtttaaactacttcccggaacaggtgtcaaaggatgctttagaacaggccttccacctctaccagaagctgaaggccgcaaaggtggaagagagggagaaggcacttaaggaatgggaagccctccagaaaaagctgagagagaaggttgttaagtgtttctcagactcgaataaggctaggttctcgcgtatagataagaaggaacttatcaaggaagacttaataaactggttggtcgcccagaacagggaggacgatatcccaacggtggagactttcaataacttcaccacttacttcactggctttcacgagaatcgcaagaacatctactctaaagatgatcatgcaaccgctatcagcttccgcctcatacatgagaatctcccaaagttctttgataatgtaatatcgtttaacaagttgaaagagggattcccagaactcaaatttgataaagttaaggaggaccttgaggtagattacgatctaaagcacgctttcgagattgagtactttgtaaactttgtgacccaggcagggatcgaccagtataattaccttctaggtggcaagacacttgaagacggtacgaagaagcagggtatgaatgaacaaatcaacttgtttaaacagcagcagacaagggataaagctcgtcagatcccgaagttaatacctttattcaaacaaatcctttccgaaagaactgaaagccagagtttcatcccgaaacagtttgaatctgatcaagaactgtttgattcacttcagaagctccataacaattgccaggataagttcacggtccttcaacaagcaattcttggtttggcggaagcagatctaaagaaggtattcattaagacgtcggatcttaatgctctctcaaatactatattcggaaattactccgtgttcagtgatgctcttaacctctataaggaatctctgaagacgaagaaagcccaagaggcctttgagaaattaccagctcattctatccacgatttgatacagtacttggaacaatttaactcttctctcgacgccgagaagcaacagagtaccgataccgtgcttaattacttcataaagacggatgagctttattcacgatttatcaaatctacctcagaggcattcacgcaagttcagcctctctttgaactcgaggcactttccagcaagcgtaggccgccagagagcgaagacgagggtgctaagggtcaggagggatttgagcagattaaacgtattaaagcttacctggacacccttatggaagcagttcacttcgcgaaacctctttacctggtgaagggaagaaagatgattgaaggactggataaagaccaatcattctacgaagcattcgagatggcctaccaagaattagagagcctaatcatccctatttataataaagctcggagctatcttagtagaaagccgttcaaagccgataagtttaagatcaacttcgataataatactttgttgtcaggttgggatgcaaacaaagaaacagcgaatgcttctatcttattcaagaaagatggattgtattatctcggtattatgcctaaaggaaagacgttcctctttgattacttcgtttctagtgaggactcagagaaattgaaacagaggcgacagaagaccgcggaagaggcgttagcccaggatggtgagagctatttcgagaagattcgatataaattgttgcctggtgcctccaagatgctccctaaggtcttttttagtaataagaacattggcttctataacccgtcggacgacatcttgagaatcagaaatactgcttcacatactaagaatggaactcctcagaaaggacacagcaaggttgaatttaaccttaacgattgtcataagatgatcgacttctttaaatcttcaatacagaaacatccagaatggggtagtttcggtttcactttcagtgacacgtcggacttcgaggatatgagcgcattctatagagaggtcgagaaccaaggctatgtgatttccttcgataagatcaaggagacatatatccaaagccaggtagaacaaggaaatctttacctgttccagatatataacaaggatttctcaccatactctaagggtaaacctaacctccacacactctactggaaagcactattcgaagaagctaacttgaacaatgtggttgctaaactaaacggagaagctgaaatcttcttcagaagacattctatcaaggcatctgataaagttgtgcatccggcaaatcaggcgatagataataagaatcctcatacggaaaagacacaatccactttcgagtatgatcttgtaaaggataaacgttacactcaggataaattcttcttccatgtaccaatatctctgaacttcaaggctcaaggagtgagtaagtttaacgataaagttaatggctttctaaagggaaacccagacgttaacatcataggtattgatcgaggggagcgtcatttgctttatttcacagtggtcaatcagaagggtgaaatccttgtgcaggagtctttgaacacattaatgtcagataagggacacgttaatgattatcagcagaaattggataagaaggagcaggaacgggatgctgctcgtaagtcatggacaacagtggagaatataaaggaacttaaggaaggatatttgtctcacgtagtgcataaattggcccacctcatcattaagtacaacgctatcgtctgtctcgaagacctaaactttggtttcaaacgcggaagatttaaagttgagaagcaagtttaccagaaatttgagaaagctttgatcgataagcttaattacctggtcttcaaagagaaagaattgggagaggtaggacattatttaactgcttaccagttaactgcgccattcgagtcgttcaagaaactcgggaagcagtctggtattttattctatgttccggctgattatacgtctaagattgaccctacaactggcttcgtcaatttccttgatcttagataccaatctgttgagaaggcgaaacagctactcagtgacttcaatgcgattagattcaattctgttcagaattacttcgaattcgaaatcgattacaagaaattgactccaaagcggaaggttggaacccaatcgaaatgggtcatctgtacttacggagacgtcagataccagaaccgaagaaatcagaagggacattgggagacagaagaggtgaatgttactgagaaacttaaggcattgtttgctagcgacagcaagaccacgactgtgattgactacgccaatgacgacaacttaatagatgttattcttgagcaggataaagcaagcttctttaaagaactcctgtggctccttaagcttaccatgacccttagacactctaagatcaagtctgaagacgacttcatcctatcgcctgttaagaacgaacaaggtgaattctacgactcacgcaaggcaggtgaggtatggccaaaggacgctgatgccaatggcgcttaccacatcgctcttaaaggactctggaatctgcagcagattaaccaatgggagaaagggaagactcttaatctcgctataaagaatcaggattggtttagcttcatccaggagaagccgtaccaggaataa

SEQ ID NO: 792 - DNA, 3897 bp, Artificial Sequence
  Description of Artificial Sequence: Synthetic polynucleotide
atgacgaagacattcgatagcgagttcttcaacctgtactcacttcagaaaacagtgcgatttgaactcaaacctgttggcgaaactgcctcgtttgttgaagacttcaagaatgagggtctaaagcgggtggtgtctgaggacgagagaagagctgtcgactaccagaaggtgaaggagatcatagatgactatcatcgtgacttcatagaggaatcattgaattacttccctgagcaagttagcaaggatgctttagaacaagcgtttcacttgtaccagaaacttaaggcagctaaggttgaagaaagagagaaggcattgaaggaatgggaggctttgcaaaagaaactcagagagaaagtggtcaagtgtttcagtgattcaaacaaagctaggttctccagaattgacaagaaagagttgatcaaggaggacttaatcaattggttggtggcgcagaaccgggaggatgatataccaacggttgagacctttaacaacttcactacgtatttcacaggattccatgagaacagaaagaacatatattccaaagatgatcatgcaacggcaatctcatttcggttaattcacgagaatctaccgaagttcttcgacaatgttatctcgttcaacaaactcaaagagggcttcccagagttgaagttcgacaaagttaaagaggatttggaagtggattatgatttgaaacacgccttcgagattgaatacttcgttaacttcgttacacaagccggtattgatcaatacaattatctgcttggtggaaagactctcgaagatggaaccaagaagcaagggatgaacgagcaaatcaacttgtttaagcaacagcagaccagagataaggcccgacagatccctaagttaattccgctgtttaagcaaattctttccgaacgaacagaatctcagtcattcattcccaagcagttcgaatctgatcaagaactgtttgactcattgcagaagcttcataacaactgccaagataaattcactgttctgcaacaggcaattcttggtttggcagaagcagatttaaagaaggtcttcataaagacttctgatcttaacgcattgagcaatacaatattcggtaactactccgtgttcagtgatgctcttaatttatacaaggaatcattgaagactaagaaagcgcaagaagcgtttgagaagctccctgcacatagtattcatgaccttatacaatatttagagcagttcaactcttctcttgatgcggagaaacaacaatcaacagacactgtcctaaactacttcatcaagaccgatgagctatactctcggttcattaagtcaacttcagaggcattcactcaggttcaacctctcttcgagttagaagcactatcgtccaagagacgccctccggagtctgaagacgaaggagctaaagggcaggaaggttttgagcaaattaagagaattaaggcttacttggataccctcatggaggcggttcactttgcgaaaccattatatcttgttaaaggacggaagatgattgaaggcctagacaaggatcagagtttctatgaagcatttgagatggcatatcaagaattggaatcactcatcattccaatctataacaaagctagatcatatctttcgcgcaagccgttcaaagcggacaagtttaagattaatttcgataacaatacattgcttagtggttgggatgctaacaaggaaacagccaacgcaagcatactcttcaagaaggacgggttgtattatctagggatcatgcctaaaggtaagaccttcctatttgattacttcgtgtcaagcgaagattccgagaaattgaagcaaagaagacagaagaccgcagaggaagcacttgcgcaggatggcgaaagctactttgagaaaatacggtacaagctgttgccaggagctagtaagatgcttccgaaagtctttttctctaacaagaacattggattctacaacccttctgatgatattctcagaatacgcaacacagcttcacatacaaagaatggaactcctcagaaaggacatagtaaagttgagttcaacctaaacgattgccataagatgatagatttctttaagtcttccatccagaagcatccggaatggggttcattcgggttcacattctctgatacttctgatttcgaagatatgagtgcattctatagagaagttgagaaccaaggatacgttatctctttcgacaagattaaggaaacatacatacagtcacaagttgaacaaggcaatttatacctcttccaaatctacaacaaagacttcagtccttatagcaagggtaagccaaacttgcatactctttattggaaagctctatttgaagaggctaacttgaataatgtggttgccaaattgaacggagaagcagaaattttctttcgtaggcattccatcaaagcttccgacaaggttgtacatccggccaatcaggctattgataacaagaatccacatactgaaaagacccagtccacatttgaatatgacctcgtgaaggacaagagatatacgcaggataaattcttctttcatgtgccgatatctcttaacttcaaggcgcagggagtttcgaaattcaacgacaaagtgaatggtttcctgaaaggtaatcctgatgtaaatattatcggtattgatagaggagagaggcacttgctttacttcacggttgttaaccagaaaggagagatactcgttcaagagtctctaaacacgctcatgagcgacaagggtcacgtcaatgactatcagcagaagctagataagaaagagcaggaaagagatgcagcaagaaagtcatggactacggtggagaacattaaggaactcaaggaagggtatctgtcccacgttgtgcataaacttgctcatctcatcattaaatataatgctatcgtgtgtcttgaggacttgaacttcggtttcaaacgaggtaggttcaaagttgagaaacaagtttatcagaagtttgagaaagctcttatcgataagctgaactaccttgtgttcaaggagaaggaactcggcgaagtaggccactacctgacggcttaccaattaacagcacctttcgaatcatttaagaagttaggtaaacagtcagggatcttattttacgttccggctgactatacctcgaagatcgatcctaccactggattcgtcaatttcttagatttacgatatcaatcagttgagaaggccaaacagttgcttagtgatttcaatgctattagatttaatagcgtccagaactacttcgagttcgaaatagattacaagaagctgactcccaagaggaaggttggtacacagagtaagtgggttatctgcacatacggagatgttagataccagaatcggagaaaccagaagggtcactgggagactgaagaagttaacgtaaccgagaagcttaaggccctcttcgctagcgattctaagaccactacggtgattgattatgctaatgacgataacttaatagatgtaatactggagcaggacaaggcatcattcttcaaggagctcctctggttattgaaactcacgatgacattgcgccatagtaagattaaatccgaagacgactttatcttatctccagtaaagaacgaacagggagagttctacgactcacggaaagcgggtgaggtatggcccaaggatgctgatgccaatggagcttaccacatcgcacttaagggactttggaatttgcaacaaattaaccagtgggagaaaggtaagacgcttaatctagcgataaagaatcaggattggttctcgttcatccaggagaaaccatatcaagagtga

SEQ ID NO: 793 - DNA, 3897 bp, Artificial Sequence
  Description of Artificial Sequence: Synthetic polynucleotide
atgacgaagaccttcgattccgaattcttcaatctctactcattgcaaaagacagtgcgtttcgaattaaagccagtaggagaaaccgctagcttcgtcgaagattttaagaatgagggcctgaagcgtgtcgtctcagaagacgagagaagagcagtggattatcagaaagttaaggagatcattgatgactatcatagagacttcattgaggaatcccttaactatttccctgagcaggtttctaaggacgcattggagcaagcgttccatctttatcagaaattgaaagctgccaaggttgaggagagagagaaagctttgaaagagtgggaagctttgcagaagaagttaagagagaaagtcgtcaagtgctttagcgactctaataaggctcgcttctctcgtattgacaagaaagaactaatcaaagaggacctcatcaattggctagtcgctcagaaccgtgaagatgatatcccaactgttgagactttcaataactttacgacatacttcacaggtttccatgagaaccggaagaatatctattccaaagacgaccacgctacagcaatctcattccgtttgatccatgagaatctacctaaattctttgataatgttatttctttcaacaagttgaaagaaggttttccagaactgaagtttgacaaggtaaaggaggaccttgaagtagactacgatttgaaacatgcctttgagattgagtactttgtaaacttcgtcactcaagcaggaatagatcaatacaattatctgcttggcggtaagacacttgaggacgggactaagaagcagggtatgaatgaacagataaacttgtttaagcaacaacaaacacgggataaagctcgacagattcctaagttaattcctctattcaaacagatcctttctgagagaacagagtcgcaatcctttattcctaagcagtttgagagcgaccaagagttgtttgacagtctacagaagcttcataataattgccaggataagtttactgtactgcagcaggctatcttaggactcgccgaggctgatctcaagaaagtgtttataaagacctctgacctcaatgcgttgtctaacaccatctttggtaattattccgtattctctgatgctttgaacttatacaaggaaagtctgaagacaaagaaggctcaagaggcgtttgagaaattaccggctcattctattcacgatcttattcagtatctcgaacagtttaatagcagtttggatgcagagaaacagcagagcactgatacggtgcttaattacttcattaagacagatgaactctacagcaggtttataaagtcgacatctgaggcgttcacacaggttcaaccattgttcgaactcgaagcgttatcatcaaagaggaggccacccgaaagtgaggacgagggagccaagggtcaagagggatttgaacagattaagagaattaaggcatatttggacactctcatggaggcagttcactttgcgaagcctctatatctagttaagggccgcaagatgattgagggactcgataaggatcaatccttctatgaggctttcgaaatggcttatcaagaacttgagtcactaatcatacccatttacaacaaagcgcgttcttaccttagccgaaagccattcaaagcagacaaattcaagataaacttcgataataacactttgctttccggatgggatgcgaacaaggagaccgcgaacgcctcgatcctgttcaagaaggacggcctttattatttaggaattatgccgaaagggaagactttcctctttgactacttcgtctcctctgaagactcagagaaactcaaacaaaggagacagaagacggctgaagaagcgctggcacaagacggagagtcatatttcgaaaagattagatacaagctgttgccaggcgcgtcaaagatgttgcctaaagtgtttttctcgaacaagaatatcggtttctataaccctagtgatgacatattaaggatccgaaatactgctagccacactaagaacggaacaccgcagaaaggtcatagtaaagtcgagttcaaccttaatgactgtcacaagatgatagacttctttaagagctcgatccagaaacatcccgagtggggtagcttcggctttaccttctcagatacatcagactttgaagatatgtcagctttctacagggaggtggagaatcaaggatatgttatatcatttgataagatcaaggaaacttatatacagagccaagtggaacaaggtaacctgtatctgtttcaaatttataataaggacttcagtccctactctaaggggaagcctaacctccatactctatactggaaagcgctatttgaggaagctaatttgaataacgtcgttgctaagctcaacggagaggcagagattttctttagaagacatagcatcaaagcttccgataaagttgttcatccagcgaaccaggcaattgataataagaaccctcacactgagaagacccaatctacctttgaatatgatcttgttaaagacaagagatacactcaggataaattcttctttcacgtccctatatcgttaaactttaaagcccagggagtttccaaatttaacgacaaagttaatggtttcctcaagggtaatcctgatgttaatataattggaattgatagaggcgaacggcatttgctatacttcacagttgtgaatcagaaaggtgagatactggttcaagaatctttaaatactctcatgagcgataaaggacatgttaacgattatcagcagaaattagacaagaaagaacaagagagagatgccgctcggaagtcttggactactgtggagaatatcaaggagttgaaggaaggctatctatctcatgttgtgcataagttggctcatctgatcattaaatataacgcaattgtttgtttggaagatttgaacttcggattcaaacgaggcagattcaaggtcgagaagcaagtataccagaaattcgagaaggccttaattgataaattgaactatcttgtctttaaagagaaagagctgggagaagtagggcattacttgaccgcgtaccaactcacggcaccgttcgaaagctttaagaagctaggcaaacaatcaggcattctcttctacgttccggcggattacacatcaaagatcgaccctaccactgggttcgtgaatttcttggacttaagatatcagtctgttgagaaagcaaagcaattgctttcagacttcaacgccataagatttaattctgtgcagaactacttcgagtttgagattgattacaagaaattgacacctaaacgcaaggtgggaacccaaagtaaatgggtaatttgtacatatggagacgttcgttaccagaataggaggaatcagaaagggcactgggaaacagaggaggttaatgtcacagagaagcttaaagcattgtttgcttccgatagtaagacaacaacagtaatagattacgctaatgatgataatttgatcgatgtgatacttgagcaggacaaggcttctttctttaaagagcttctttggctattgaaactgactatgactcttcgacattctaagataaagagtgaagatgacttcatcctctctccagtcaagaatgagcaaggtgaattctatgattcacgcaaggcaggtgaagtatggcctaaggacgccgatgccaatggtgcgtatcatatcgccttgaagggtctctggaatttacaacaaattaaccaatgggagaaaggaaagacattgaacctcgctataaagaaccaagattggttctccttcatacaagagaaaccctatcaggagtga

SEQ ID NO: 794 - DNA, 3897 bp, Artificial Sequence
  Description of Artificial Sequence: Synthetic polynucleotide
atgactaagaccttcgattctgagttcttcaatctgtactcattgcagaaaactgtcaggtttgaattgaagcctgttggcgaaacagcctccttcgttgaagattttaagaacgaaggcttgaagagagtcgttagcgaggatgaaaggagagctgttgactatcagaaagtgaaggagattatcgatgactaccacagagacttcattgaagaatctctgaattactttcccgagcaggtaagtaaggatgccttggaacaagctttccatttgtatcagaaacttaaggcagctaaggttgaggaaagagagaaggctttgaaagagtgggaagcactacaaaagaagttgagggagaaggttgtgaagtgcttcagcgatagtaataaggctcggttctcaaggatcgataagaaagagttgatcaaagaagatttaataaattggctcgtggctcagaatcgggaggacgacattcctactgtggagacgttcaataacttcacgacatatttcacaggattccacgagaaccgaaagaacatatactcaaaggatgatcacgctactgccatctcattccgactcattcatgagaaccttcctaagttctttgacaacgttatttcattcaacaaactgaaggaaggtttcccagagctgaaatttgataaagtcaaagaggatctagaggtagactacgatctcaagcacgcatttgagattgaatactttgtgaatttcgttacacaggccggtattgatcaatacaattacttattaggtggcaagactttggaggacgggacgaagaagcaaggtatgaatgaacagattaatttgtttaagcagcagcagacccgagataaagcccgtcagatcccgaaacttattccgctgttcaaacaaattctttcagagagaaccgagtctcagtcattcattcctaagcaattcgaatcagaccaagaactattcgactctttgcagaagctccataacaactgtcaagacaagttcaccgtgctgcagcaagctatactagggttggccgaggctgatctaaagaaggtctttataaagactagtgatttgaatgctctctctaatacaatctttggaaattacagtgtgttttctgatgctttgaacctctataaggagagtctcaagacaaagaaggcgcaagaggccttcgagaaattgcctgctcacagcattcatgatctgatccaatacctagaacaattcaactcttccttggatgcagagaaacaacaatcgacggatacagttctaaattacttcataaagactgatgagctttactcacgtttcattaaatcgacttctgaagcatttactcaggtgcagccactctttgaactggaagcattgagttccaagagaagaccacctgaatcagaagatgagggtgccaaaggtcaagaaggcttcgagcagattaagcgtataaaggcctatctcgatacactaatggaagctgttcacttcgctaagcctttatacctcgtgaaaggtcgcaagatgatcgaaggcctagacaaagaccaaagtttctacgaggcatttgagatggcatatcaggaactcgagagtctaattattcccatttacaataaggccagatcctatttgtcacggaagccatttaaagctgataagttcaagattaactttgataacaatactcttctgtctggttgggatgcaaataaggaaacggctaacgccagcatactcttcaagaaggatggattgtactacctgggcatcatgcctaaggggaagacgttcctattcgattacttcgtcagctctgaagattcggagaagctcaagcagcgcagacaaaagacggcagaggaagcccttgcccaagacggtgaatcttatttcgaaaagatcagatacaaattgcttccaggtgcatctaagatgcttcccaaagttttcttttccaacaagaacattgggttctataacccaagtgatgacatcttaaggataaggaacaccgcatcacacactaagaacggaactccacagaagggtcattccaaggttgagtttaatctaaatgattgtcacaagatgattgatttctttaagtcttctattcagaaacatccagaatggggttcatttggtttcactttcagcgatactagcgatttcgaggacatgtctgccttctatagagaggttgagaatcagggttatgtgatttcatttgacaagataaaggaaacctacatacagagccaagttgagcaaggaaatttatatttattccaaatatataataaggacttcagtccctattctaaaggtaagccaaacttgcacaccctctactggaaagcgttgttcgaggaggctaatcttaacaacgtggtggctaagttaaatggtgaggcagaaatattcttcagaagacactctataaaggccagtgataaggtcgtccatcccgctaatcaggctatcgataataagaaccctcatactgagaagactcagtctacatttgagtacgacttagtcaaggataaacgttatacacaggataagttcttcttccatgtacccatatcactaaatttcaaagcacaaggtgttagtaaatttaacgataaggttaatggatttcttaaaggaaaccctgatgtcaacattattggtatagatcggggcgaacgtcacctactttacttcactgtagtgaatcagaaaggtgagatactagttcaagagtcattaaacaccttgatgtcagataagggtcatgttaacgattaccagcagaagttggataagaaagagcaagagcgcgatgctgcgagaaagagctggactacggtggagaatattaaggaacttaaagaagggtatctcagccacgtggttcataaattggcacatctaattataaagtacaatgcaattgtctgcctggaggatttgaacttcggattcaagcgagggagatttaaagtggagaagcaggtttaccagaaattcgagaaagctctaattgataagcttaactatcttgtatttaaagagaaggaactcggagaagtaggccattatttgacagcataccaattgactgcgcccttcgaaagctttaagaagctcgggaaacaaagtggaattctgttctatgtccctgctgattacacatccaagattgatccaactacaggcttcgttaacttcctcgatttacgataccaatcagtggagaaggctaaacaactcctctctgactttaacgctattagatttaactccgtacagaactacttcgaattcgaaattgattacaagaagcttacacctaagcggaaagtaggcacccagtcaaagtgggtaatatgtacttatggcgatgtcagatatcagaatcgacggaatcagaagggtcattgggagactgaagaagtcaatgttaccgagaaattgaaagctttatttgcatcagattccaagaccacgacagttatcgactacgcaaatgatgataatctaattgatgttattctggaacaagataaggcatccttcttcaaagaacttctttggttgctcaagcttaccatgaccttgcgtcattccaagatcaaatctgaagatgacttcatcttgtcaccggtcaagaacgaacaaggtgagttctacgattctaggaaagcaggtgaggtttggcctaaggatgcagacgcaaatggcgcttaccacattgctctaaagggtctatggaatttgcaacaaattaatcaatgggagaaaggtaagaccctcaatttggctataaagaatcaagattggttctcgttcattcaggagaaaccatatcaagaatga

SEQ ID NO: 795 - DNA, 3897 bp, Artificial Sequence
  Description of Artificial Sequence: Synthetic polynucleotide
atgacaaagacgttcgactctgagttctttaacctgtacagcttgcagaagaccgttcggttcgagctcaagcctgtgggagaaactgcctcgttcgttgaggacttcaagaatgagggacttaaacgagttgttagtgaagatgaacgccgtgctgtcgattaccagaaagttaaagagatcatagacgactatcatagggacttcattgaagaatctcttaactactttcctgagcaagtctctaaggatgccctggaacaagcctttcatctctatcagaagcttaaggccgctaaagtagaggagagggagaaggcactcaaggagtgggaggctcttcagaaaaaactaagggagaaagtggttaaatgtttctctgatagtaacaaagctcgtttctctaggattgataagaaggagttgattaaggaggacctcataaattggttagttgcacagaatcgggaagacgatatcccaacagttgagacattcaataactttactacatactttactggtttccatgagaatcgaaagaacatttattctaaggatgaccatgctactgcgatttcattccggcttatccatgagaacctaccaaaattctttgacaacgttattagtttcaacaagctcaaagagggtttcccggagcttaagttcgataaggtcaaagaggacctagaggttgattatgacttgaagcacgcgttcgaaattgagtacttcgtgaacttcgttacgcaagcagggatcgaccagtacaattatttgttaggagggaagacgcttgaggatggcactaagaaacaaggaatgaatgaacagataaacctcttcaagcagcaacagactcgcgataaggcacgtcagatccctaaattaataccattgtttaagcagattcttagcgaacgtactgaaagccagtctttcatcccgaagcagtttgagtctgatcaagagttgtttgactcgctgcagaaattgcacaataattgccaggacaagtttaccgtacttcaacaagcgattctcggccttgctgaagccgatcttaagaaagtgtttatcaagacgagtgacctgaacgcactttctaacacaatcttcggtaattattctgtattctcagacgctctgaacttatacaaagaaagtttaaagaccaagaaagctcaagaggctttcgagaaattgccggcccattcgattcacgatctgatccaatatctagaacaattcaatagctctttggacgccgagaagcaacagtccaccgacacagttcttaactacttcattaagacggatgagctctactccaggttcattaagagtacctccgaagccttcacacaagttcagccactcttcgagttggaagcattgtcttctaagaggagacctccagagagtgaggatgaaggagcgaaaggacaagaaggcttcgagcagatcaaacgcattaaggcttatttagacacacttatggaagctgttcatttcgctaagcccttgtacttggtgaaaggacgaaagatgattgaagggctagataaggaccaatcgttctacgaggcattcgagatggcataccaagaattagaatccttaatcatacctatttacaacaaggcccgtagttaccttagccgtaaaccgtttaaggcagacaaatttaagattaacttcgacaacaacactctgctaagtggctgggatgcgaacaaagaaaccgcgaacgcgtctattttgttcaagaaggatggactctattatctgggaataatgcccaaggggaagactttcttgtttgattactttgtttcctctgaagactctgagaaattgaaacaaaggagacagaagacagctgaagaagcattagcgcaggatggtgagagttatttcgagaagattagatataagttgctcccgggtgcaagcaagatgttacctaaagtgttctttagtaataagaacattggcttctataacccgagtgatgatatcctgagaatccgtaacacagcgagccataccaagaatggtacacctcagaagggccactctaaggtcgaattcaatctaaatgattgccataagatgattgacttctttaaatctagtatccagaagcatccagaatggggtagcttcggattcactttctcagatacgtctgatttcgaggatatgtcagctttctatagggaagtagagaatcaaggatatgtcatttcattcgacaagatcaaggaaacgtacatccagtcccaagttgagcaaggtaatctgtatctctttcagatctacaataaggacttctcaccatattccaagggtaaacctaacttgcatactttgtattggaaggctttgtttgaagaggccaaccttaacaacgttgtagcaaagttgaatggagaggcagaaatcttcttcaggagacactcaattaaagcttcagataaggttgttcaccctgccaaccaagccattgacaacaagaaccctcataccgaaaagactcaatccactttcgaatatgatttagtgaaagacaagagatatacgcaggacaaattcttctttcacgttccgatttctttgaactttaaggcacagggcgtgtctaagttcaatgacaaagtcaacggtttcctcaaaggcaatcctgatgttaacattatcggaattgatagaggcgaaagacacttgctgtacttcacagtcgtgaatcagaagggagaaatcctcgttcaagaaagtctcaacacattgatgtctgataaaggtcatgttaatgattatcaacagaaactcgataagaaagaacaagaaagagatgctgctagaaagagttggactacagtagagaacatcaaggagttgaaggagggttatttaagtcacgtcgtccacaaacttgctcacctgatcatcaagtacaatgctatagtctgcttggaggacttaaacttcggtttcaagcgtggaaggttcaaagtggagaagcaagtgtatcagaagtttgagaaagctctgatcgacaagctcaactatttggtatttaaagagaaggaacttggtgaagttggacattatcttactgcgtatcagcttactgctcctttcgagtcattcaagaaactaggtaagcagtcgggtatcctattctatgtgccggctgactatactagcaagattgatcctaccacgggattcgttaatttccttgatcttagatatcagtctgtcgagaaagccaaacaactactgtcagacttcaatgcaattagattcaacagtgttcagaactacttcgagttcgaaatagactataagaaattgacacccaagaggaaggttggcacacaatcaaagtgggtgatctgcacctatggcgacgtgagatatcagaaccgtagaaatcagaagggtcattgggagacggaagaagtcaatgtcaccgagaagcttaaggctctgttcgcatcggatagtaagactaccaccgttatcgattacgcaaatgatgataatttgattgatgttatcctagagcaggacaaagcatctttcttcaaggagctgctttggttgctaaagttaacaatgaccctcagacacagcaagatcaagtccgaagatgacttcatcctgtcaccagttaagaacgaacaaggagagttctacgactctcgtaaggctggagaagtttggcctaaagacgcagatgcaaatggcgcttaccacattgcattgaagggcctctggaacttgcaacagattaaccaatgggagaaaggtaagacgttgaatttggctattaagaatcaggattggttcagtttcattcaagagaagccctaccaggagtaa

SEQ ID NO: 796 - DNA, 3897 bp, Artificial Sequence
  Description of Artificial Sequence: Synthetic polynucleotide
atgaccaagaccttcgactctgagttcttcaacctgtatagccttcagaagacagtacgattcgagctgaaacctgttggtgagactgcgtcatttgtcgaggacttcaagaacgaaggcttgaagcgagtagtatccgaagacgaacgaagagctgttgactatcagaaggtgaaagaaattatcgatgattatcatcgagacttcatcgaggaatcactcaactacttcccagagcaagtgtcaaaggatgctcttgaacaggccttccacctgtaccagaagttaaaggctgctaaagttgaagagagagagaaggcgctcaaagaatgggaagcccttcaaaagaagctacgagagaaggttgtcaagtgtttctcagactctaataaggcgcgtttcagccgtatagataagaaagagttgattaaagaggacctcatcaactggctggtcgctcagaatagagaggacgatatacccacagttgagacattcaataactttactacttactttacgggatttcacgagaatcgtaagaacatttactcaaaggatgatcatgctactgctatcagcttccgacttattcacgagaatttgccgaaattctttgataacgttatcagcttcaataagttgaaagagggtttcccagagttgaagttcgataaagttaaggaagacttagaggtagattacgatcttaagcacgcgtttgaaattgagtactttgtcaatttcgttactcaggctggtattgatcaatataattacctgttgggtggtaagacactagaggatgggacaaagaagcaaggtatgaatgagcaaatcaatctctttaagcagcagcaaactcgcgataaggcgaggcaaatacctaaattgattccattgtttaaacagatcctgagtgaacgtactgaaagtcaaagtttcattccaaagcaattcgagagcgatcaggaactattcgattctctccagaagcttcataacaattgtcaagataagttcacggtgttacagcaagcgatcttgggtctcgcagaggcagaccttaagaaagtgttcattaagacttcggatttaaacgccctttctaacacaatcttcggaaattattctgtcttctctgatgctctaaacctctacaaagagtcgctgaagaccaagaaggcccaggaagcgttcgagaaactaccagcacattcgattcatgacctcattcaatatttggaacagtttaactcctcattagacgcagagaagcaacaatctactgatacagtcctgaattacttcataaagacagatgagttgtattcaagatttataaagagtacttcagaggcgttcacacaggtgcaacctttatttgaactggaagctctttcgtctaaacgtcgtccgccggagtcagaagatgaaggagccaaagggcaggaaggtttcgagcaaataaagagaattaaggcttacttggatacattgatggaagccgttcactttgctaaacctttgtatttagtgaaaggacgaaagatgatcgaagggcttgataaggatcaatccttctacgaagctttcgagatggcgtaccaggagctggaatctctaatcattcctatctacaataaggcaagaagttatttgtcacgtaagccattcaaggcagacaagttcaagatcaactttgacaataatacattgctcagtggctgggacgctaacaaggaaactgctaatgcttcgattctattcaagaaagatggtttgtactatctcggaattatgccgaaggggaagactttcctatttgattatttcgtgtcatctgaagactctgagaagctcaaacaaaggcgacagaagacggcagaagaagctctagctcaggatggagagtcgtatttcgaaaagatacgctataagctgctccctggcgcgtctaagatgttaccaaaggtattcttcagtaacaagaatattggtttctacaatcctagtgatgacattctgcgtataagaaacacagctagccataccaagaacggaacgccgcagaaaggtcactctaaggtagaattcaacttgaacgattgtcacaagatgattgacttcttcaaatcttcaatacagaaacacccagaatggggctcatttggcttcacgttctctgataccagtgactttgaggatatgtctgctttctacagagaggttgagaaccaagggtacgtgatctcgttcgataagatcaaggaaacctacattcagtcacaggtggagcaagggaatctttatctattccaaatttacaataaggacttctcaccttatagtaagggtaagccgaacttgcatactctctattggaaggcattatttgaggaggccaatctcaataacgttgttgccaagcttaatggagaggccgagattttcttccgtagacactcgattaaggcttccgataaggtagtgcacccagcaaaccaggcaattgacaataagaatcctcatactgagaaaacacaaagtactttcgagtacgatttagtcaaagataaacgatatacgcaagataaattcttcttccatgttccaatctctcttaactttaaggctcagggagtgtctaagttcaacgataaggtgaatggctttcttaagggaaacccagacgtcaatattatcggaattgatagaggtgaaagacacttattgtacttcacagttgttaatcagaagggcgagatccttgttcaggagtcacttaatactttgatgtctgataaaggtcatgtgaatgactaccagcagaagcttgacaagaaggaacaggagagagacgctgcccgtaagtcatggacgactgttgagaacatcaaggagcttaaggaaggatacttgtcacatgtcgttcacaagttggcccatttgattattaaatacaatgctattgtatgcttggaggatttgaacttcggatttaagcgcggaagattcaaggtcgagaagcaagtttatcagaaatttgagaaggcgttaatcgataagttaaactacctggtgtttaaagagaaagagctcggcgaggttgggcattacttgacagcgtatcaactaaccgcaccatttgaatcctttaagaagctcggtaagcaatctggtatcctcttttatgtaccggcagattataccagcaagatcgatccgactactggattcgtcaacttcctagatttgagataccagtcagttgagaaagccaaacagttgctttcggatttcaacgcgatacgattcaattctgtacagaattacttcgaattcgagatcgattataagaagttgactccaaagagaaaggttggtacccagtccaaatgggtcatctgtacatatggtgacgttaggtaccagaacagacggaatcagaagggacattgggaaaccgaggaagtgaatgtgactgagaagcttaaggcattgttcgctagtgatagtaagacaactactgttatagactatgcaaatgatgacaatttgatcgatgttatcttggagcaagacaaggccagtttcttcaaggaactattgtggctactgaagttgactatgacacttcgtcattccaagatcaagtctgaggatgacttcatactctctccggttaagaatgaacaaggagaattctacgactctaggaaggcaggagaagtatggccaaaggatgcggacgctaatggcgcttatcacattgctcttaagggactttggaatttgcaacagattaatcaatgggagaaggggaagacacttaaccttgcaattaagaatcaagattggttctcatttatccaggagaaaccgtatcaggaataa

SEQ ID NO: 797 - DNA, 3897 bp, Artificial Sequence
  Description of Artificial Sequence: Synthetic polynucleotide
atgacgaagacgttcgatagcgagttctttaatctttattctctccagaaaaccgttagattcgagctcaagccggtaggcgaaactgcttcattcgttgaagattttaagaatgaaggactcaaacgagttgtaagcgaagatgaacgtcgtgctgttgattaccagaaagttaaggaaatcattgacgattaccatcgagatttcatagaagaatcccttaattactttcctgagcaagttagcaaagacgcactcgagcaggcgttccatctctaccagaaattgaaggctgcaaaggtcgaagaacgcgagaaggcgctgaaggagtgggaggctttacagaagaagctcagagagaaagtcgtgaaatgcttcagcgattctaacaaggctcgcttctcacgtatcgacaagaaagaacttattaaagaggatttgattaattggttagttgcccagaatagggaggatgatattcctacggttgaaacctttaataatttcactacctacttcacaggattccatgagaaccgaaagaatatctactcaaaggatgaccacgccacagctatcagtttccgtttgatccacgagaacttacctaaattcttcgacaatgttatctcattcaataagcttaaggaaggatttccagagctgaagttcgataaggttaaggaggatttggaagtggattatgatttgaagcatgccttcgaaatcgaatacttcgtaaacttcgttacacaagccggtattgatcagtataattatcttctaggtggcaagacactggaggacggaacaaagaaacaaggtatgaatgaacaaattaacctatttaagcaacagcagacccgagataaagcaagacagatccctaagttaattcctctctttaaacaaatcctttcggagagaacagaatcccaatcctttatcccgaagcagttcgagtcagatcaggaactctttgacagcttgcagaaattgcataataactgtcaggataagtttaccgtccttcagcaggcaatcttgggactggccgaggctgatcttaagaaggtatttattaagacgagtgatctgaatgccttgtccaacaccatattcggtaattatagtgtattcagtgatgcattaaatttatataaggagtccttgaagactaagaaggcgcaggaagcattcgagaaacttccggcacatagtatacatgatctcatccaatatttagaacagttcaattcctcgttagatgcagagaagcaacagtctactgatactgtactcaattacttcataaagacagatgaattatatagccggttcataaagtctacaagtgaggcctttactcaagtgcaacctctattcgaactggaagccctgtcatcaaagagaagaccacctgagtctgaggatgaaggtgcaaagggacaggaagggttcgagcaaataaagaggatcaaggcctacttggatactcttatggaagctgtgcacttcgctaagccattataccttgtcaaaggaagaaagatgattgagggtctcgacaaagaccaatccttctatgaggcattcgagatggcttaccaagaattggagtctctgattatccctatttataacaaagcaagatcctacctttcacgcaagcccttcaaggctgataagttcaagataaacttcgacaacaacaccttgctatctggttgggatgccaacaaggagactgctaacgctagtatcctgttcaagaaggacggattatactacctcggtataatgcctaagggaaagacatttctgttcgattatttcgtttctagcgaggactctgagaagttaaagcagaggagacagaaaacggcagaagaggctcttgctcaagatggagaatcttatttcgagaagattagatataaactcttacctggagcttctaagatgctccctaaagtctttttcagtaacaagaacataggattctataacccgtctgatgatatcctccgtatcagaaatactgcgagccatacaaagaacggaacaccacagaagggacatagtaaagttgaatttaaccttaatgattgtcacaagatgattgatttctttaagtcgtcaatacagaagcatccagaatggggcagctttggtttcaccttcagtgatacttcagacttcgaagatatgtctgcattctacagagaagttgagaatcaaggctacgtgatatcctttgacaagatcaaggagacatacattcaatctcaagtagaacagggtaatctatatctctttcaaatttacaataaggatttctcaccatattcaaagggaaagccaaaccttcatactctgtactggaaggcattgttcgaagaagcaaatcttaacaacgtggtcgccaaactgaacggagaagcagagatcttttttcgccgtcattccatcaaagcaagcgataaagtcgtacacccggccaaccaagcaattgataacaagaatccacacactgagaagacacaatctactttcgagtacgacttagtcaaagataagagatatacacaggataaattcttctttcatgttccgatatctttgaacttcaaagcacagggagtgagcaagtttaacgacaaagttaacggtttcctcaagggaaacccagacgtgaatatcatcggaattgaccggggggaacgacatctgctttacttcactgtggtgaatcagaaaggagagatactggtgcaggagtctcttaatacactgatgtctgacaaaggtcatgtaaatgattaccagcagaaactcgacaagaaggaacaagaacgcgatgctgctcgcaaatcgtggactacggttgagaacattaaagaattgaaagagggttatctatctcatgttgtgcataaactagcgcatctgattatcaaatataacgctatcgtttgtctggaagatttgaatttcggctttaagagaggtcggtttaaagttgagaaacaagtgtaccagaaatttgagaaggcgctcatcgataaattaaattatctggtcttcaaggagaaagagttaggagaagttggtcactaccttaccgcgtaccagcttactgctcctttcgagtctttcaagaagctaggtaagcagtccgggatcttgttctacgttccagcagactatacttcaaagatcgatcctacgactgggtttgttaacttccttgatcttcgatatcaatcagttgagaaagctaagcaattgttaagtgacttcaatgctattagattcaactctgtacagaattactttgagtttgagatagactacaagaagttgacgccaaaacgtaaggtgggtacacaaagtaagtgggtaatctgtacttatggagatgtgcgttaccagaataggcggaaccagaaaggtcactgggagactgaagaagtgaatgtaaccgagaaactcaaggccttgtttgcttcggatagtaagacaacaaccgttatcgattatgcaaatgatgacaatttgatagacgttattctggaacaggataaggctagcttctttaaagaactcctctggcttctcaagttaactatgactctgcgtcactcgaagattaagagtgaagatgatttcattcttagtcccgtcaagaatgaacagggcgagttctatgattcccgtaaggcaggtgaggtttggcctaaagacgctgatgcaaacggtgcttaccatatcgcacttaaaggcttgtggaacttgcagcaaatcaatcaatgggagaagggtaagacgcttaatcttgccattaagaatcaggattggttttctttcattcaggagaagccttatcaagagtaa

SEQ ID NO: 798 - DNA, 3897 bp, Artificial Sequence
  Description of Artificial Sequence: Synthetic polynucleotide
atgacaaagacatttgattcagaattctttaatctctactctttacagaagacagtgcgattcgaactcaaacccgtcggtgaaaccgcctctttcgtagaagactttaagaacgaaggactgaaacgagttgtgagcgaggatgaaagaagagcggtagattatcagaaggtcaaagaaatcatagacgattaccacagggacttcatcgaagaatcccttaattactttccagagcaagtttcgaaagatgccttggagcaagcattccacctctaccagaagttgaaagctgctaaggtagaagagagagagaaagctcttaaggaatgggaagctttgcagaagaagctccgagagaaggtggtcaaatgcttctcagattcaaataaagcccgcttctcgcgaatcgataagaaggagctcatcaaggaggatttgatcaattggttagtggctcagaatcgggaagatgacattcctaccgttgagaccttcaacaactttaccacgtacttcaccgggttccacgagaatcggaagaatatttattctaaagacgatcacgctaccgctatttcctttagattgattcatgagaacttgccaaagttctttgacaacgtgatctcattcaataagcttaaagaaggattcccagagttgaaattcgacaaggtaaaggaagatctagaggtggattatgacttgaaacatgcattcgaaatagagtacttcgtgaacttcgtgactcaagctgggatcgatcaatacaattacttgctgggtggaaagactctagaagatggtaccaagaaacagggtatgaatgagcagattaatttgtttaagcagcagcaaacaagagataaagctcgtcaaatccctaaacttattccactcttcaaacaaatactaagcgaacgaaccgagtctcagagctttatcccgaagcaattcgaatctgaccaagagttgttcgattctttacagaaactacataacaattgccaagacaaatttaccgttctgcaacaggctatcttgggactagctgaggctgacctcaagaaagtgttcataaagacctcagacttgaacgccttaagtaatactatcttcggtaactactcagtattctctgatgctctgaatctgtacaaggagagcttgaagacaaagaaggcgcaagaagcattcgagaaactgccagctcattccatccatgatttgatccagtatttagaacagtttaattcatcactagacgcggagaagcaacaaagtactgataccgtactaaattatttcataaagacagatgagttgtatagtagatttatcaagagtacatccgaagcgtttacacaggttcagccactattcgagctggaagcattgtcttccaagagacgtcctcctgagtccgaggatgaaggagctaaaggacaagaaggattcgaacaaatcaaacgaatcaaggcttacttggacaccttgatggaggctgttcatttcgcgaagcctttgtacttagtgaagggaagaaagatgattgaaggtctcgataaggaccaatctttctatgaagcgttcgaaatggcctatcaagagctcgaatcgcttatcataccaatttataataaggctcgctcttacctttcacggaagccatttaaagctgataaattcaagatcaacttcgacaacaacacattgctcagtggttgggatgctaataaggaaacagcgaacgctagcatactgtttaagaaggacggactatattacctcggcattatgccaaaggggaagacgtttctattcgactacttcgtaagttctgaggattccgagaagctcaagcagcgtagacagaagacggcagaagaggctctggctcaggatggcgaatcctatttcgaaaagatacggtacaaattactacctggcgcaagtaagatgttgcctaaagtattttttagtaacaagaacattggtttctataatccatcggatgatatcttgcgcattagaaataccgcttctcatacaaagaacggaactcctcagaagggtcattctaaggtagagttcaatttgaatgattgccataagatgatagatttctttaaatcttcaattcagaagcacccggagtggggctctttcggtttcacattctcagatacgagtgacttcgaggacatgtccgcgttctacagggaagtagagaatcaaggatacgtcatctcgttcgacaagattaaggaaacttacatccagagtcaggttgagcagggcaacttgtatttatttcagatctataataaggatttcagcccttacagcaagggaaagcctaaccttcatacgttgtactggaaagctttgttcgaagaggcaaatttgaacaatgtcgttgccaagctcaatggtgaagctgaaattttcttccggcggcactcaattaaggcctctgacaaggtcgttcatcctgcaaatcaagctatcgacaacaagaatccgcacactgaaaagacccagtcgacctttgaatatgatctagtaaaggacaagagatatacccaagataaatttttctttcatgtgcctatttcattgaacttcaaggcacagggagtgtctaaattcaacgacaaagttaacggcttcctcaaaggaaatcctgatgttaatattattggtatcgatcggggtgagaggcatctactttacttcacagtagtgaaccagaagggagaaatccttgtccaagaaagtcttaatacactgatgtcagacaaaggtcatgttaacgattaccagcagaaattagacaagaaagagcaggagagagacgcggctcgcaaatcttggacaactgtggagaatattaaggaattgaaggagggttacttgtcccacgttgttcataagcttgcacatttgatcatcaagtacaacgcgatagtatgcttagaggatctgaactttggattcaagcgtggtaggtttaaggtagagaagcaggtgtaccagaagtttgagaaggcgctcatcgataagttgaactacttggtgttcaaagagaaagaattgggcgaagttggacactacttaaccgcgtatcagctcacggcaccatttgagtcatttaagaaattgggtaagcaatcaggaatattgttctacgtccctgccgattatacgtctaagatagaccctaccaccggatttgttaatttcttggatctccggtaccagtcggttgagaaagcaaagcaattattatccgactttaacgctatcagattcaattcagttcagaattatttcgagttcgagattgattataagaagttaactcctaagcgtaaagttggaacccaaagtaaatgggtaatttgtacctacggcgatgtccgataccagaataggagaaatcagaaaggtcattgggagaccgaggaggtgaatgttacagagaaactcaaagccctattcgcctcggattcaaagaccacaacagttatcgattacgcgaacgatgataatctgattgatgtgatcctcgaacaagataaggcgagtttctttaaggaacttctctggcttcttaagttaacaatgactttgcggcattccaagattaaatccgaggacgactttatcttgagtcctgtgaagaatgaacaaggtgagttctatgattctcgtaaggcaggtgaagtgtggccgaaggacgctgatgctaatggagcttaccatatagcccttaaaggactttggaatcttcagcagattaaccaatgggagaagggtaagactttgaatttggctattaagaatcaggattggttctcgttcatccaagagaagccttaccaagagtaa

SEQ ID NO: 799 - DNA, 3897 bp, Artificial Sequence
  Description of Artificial Sequence: Synthetic polynucleotide
atgacgaagacgttcgattctgaattcttcaatctctactcacttcaaaagacagtgagatttgaactgaagccagtcggtgaaacagcgtcatttgttgaagatttcaagaatgaaggccttaagagggttgtttccgaggatgagagaagggctgttgattaccagaaggtcaaggaaatcatcgatgattaccatagggacttcatagaagaatctctcaactacttccctgaacaagttagcaaagatgccctagaacaagcctttcatctttaccagaagcttaaggcagccaaggtagaggaacgggagaaagctttgaaggagtgggaggctcttcagaagaaactgagagagaaagtggtgaaatgcttctctgattcaaataaggcaagatttagtaggatcgataagaaagaattgatcaaagaagacttgattaactggttggtagctcagaatagggaagacgatatccctacggtggaaactttcaacaacttcacaacgtacttcacagggtttcatgagaaccgtaagaacatatactctaaagatgatcatgctactgctatctcctttcgattaattcatgagaaccttcctaagttcttcgataacgtgatatcatttaacaaattgaaagaagggttcccagaacttaaattcgataaggtgaaggaagatcttgaggtagattatgacctaaagcacgcatttgagatcgaatactttgtgaactttgtgactcaggctggtatagatcagtataattatctgctgggaggtaagacgcttgaggatggtacaaagaaacaaggtatgaatgagcaaataaatctctttaaacaacagcagacgcgagataaagccaggcaaatccctaagttgatccctctcttcaaacagatccttagtgaaagaactgagagtcagtcctttattccgaaacagttcgaaagcgatcaggagttgttcgactctctacagaaactccataataactgtcaggataaatttactgtgctccaacaagctatcttagggctcgccgaagccgatctaaagaaagtgttcatcaagacttctgatcttaacgctctttctaatactatcttcggtaattacagcgtattctcggacgctctaaatctctataaagaatctttgaagaccaagaaggcgcaggaagcattcgagaagttaccggctcactccatccacgatttaattcagtaccttgaacaatttaactcgtccttagatgctgagaagcagcaatctaccgatacagtattaaattactttatcaagaccgatgagctgtatagtcgtttcattaagagtacatcggaggcgttcactcaggtacagccattattcgaactcgaagctctgtcaagcaagagacgccctccggagtctgaggatgaaggcgcaaagggtcaggagggatttgagcaaattaagcggattaaggcgtatctcgacaccttgatggaggctgtccatttcgccaaaccactttatctggttaagggtcgtaagatgattgagggcctggacaaagatcaatctttctacgaagcattcgagatggcttaccaagaactcgaatcactaataattccaatatataataaagcacgttcatatctttctcgcaagccatttaaagcggacaagttcaagattaatttcgacaacaacacattgctctcgggttgggatgctaacaaagagacggccaatgcctccattctatttaagaaggatggactttactacttgggaatcatgccgaaaggaaagacattcttattcgattactttgtatcctcggaagattccgagaagttgaagcagagaaggcagaagactgcagaggaggctcttgctcaagacggcgaaagttactttgagaagattcgctataaattactccctggtgcttctaagatgcttcctaaggtgttttttagtaataagaacatcggtttctacaacccttcggacgatatacttagaatcagaaatacagcctctcacacgaagaacggaacacctcagaaagggcactctaaagtggaattcaatcttaatgattgccacaagatgattgatttcttcaaatcgtctattcagaagcacccggagtggggctctttcggtttcaccttctcagatacctcagacttcgaggatatgtccgcattctaccgagaagtcgagaatcagggctatgtgatcagtttcgacaagatcaaggagacctatatacaaagtcaagttgagcagggaaacctttatttgtttcagatttataacaaagatttctctccgtacagcaagggtaagcctaatttacacactctttactggaaagctctctttgaggaagctaatctgaataatgttgttgcgaagttaaatggtgaagcagagatattcttcagaaggcattcaatcaaagcctccgataaagttgttcacccagctaatcaagcgattgataacaagaatccacatacagagaaaacgcaatcaacctttgaatatgacctggtcaaggacaagagatacacacaagacaaattcttctttcacgttccaatttcactgaacttcaaggcacagggagtctctaagtttaacgataaagtgaacggatttctgaagggaaaccctgatgtaaatattataggtattgatcgcggagaaaggcatcttctatatttcactgtcgtgaaccagaagggagaaatcttggtacaggagtcgcttaacactctgatgtcggataaaggtcatgtaaacgattaccaacagaaacttgacaagaaggaacaggagcgggatgcagctagaaagagttggactactgtggagaatattaaagaattgaaggagggatacttgagccatgttgtgcataaattggctcacttaatcattaagtataacgccattgtgtgccttgaagatttaaacttcggttttaagagaggaaggtttaaggtagagaagcaggtttaccagaagttcgagaaggcacttatcgacaagctgaattatttggtgttcaaagagaaagagctaggtgaagtaggtcattacttaactgcttaccagctgacagctccgtttgagagctttaagaaattaggaaagcaatccggaattctcttttatgtgcctgctgattacactagtaagattgatcctactacaggattcgtcaatttcttagatctccgctaccagtccgttgagaaagccaaacaattgctttcagacttcaacgctatcagatttaacagtgtccagaactatttcgaattcgagatcgactacaagaaattaactccaaagcgcaaagttgggacccaaagcaagtgggtgatatgtacatatggagatgtgaggtaccagaatcgaagaaaccagaaaggccattgggaaacggaagaagttaatgtaacggagaagctcaaggctctgttcgctagcgattcaaagacaactacggtcatcgattacgctaacgacgacaatctcatagatgttattctggagcaagataaggcgtccttcttcaaggaattactttggttgcttaaacttaccatgacattacggcacagtaagatcaagtccgaggacgatttcatcctaagcccggtgaagaatgaacaaggagagttctacgattccagaaaggcaggagaggtttggccgaaggatgcggatgcaaacggagcttaccatatcgctctcaaaggcctatggaatctccagcaaataaaccaatgggagaagggaaagacactaaatttggctatcaagaaccaggattggttctcatttatccaggagaagccataccaagaataa

SEQ ID NO: 800 - DNA, 3897 bp, Artificial Sequence
  Description of Artificial Sequence: Synthetic polynucleotide
atgacaaagacatttgattcagaattctttaacctttattctcttcagaagacggtcagatttgagcttaaacctgtaggcgagactgcatcctttgtcgaggatttcaagaatgagggcctgaagagggttgtttctgaggatgagcggagggcagtggattatcagaaagtcaaggaaatcatcgacgactatcatagggacttcatcgaggaatcgctcaattacttccctgagcaagtgtcaaaggatgcactagaacaagcattccacctttatcagaaattgaaggctgctaaagtggaggaaagagagaaggcccttaaagagtgggaggctctgcagaagaagttgagagagaaggtggtgaagtgcttcagtgattcgaataaggctaggttctccaggattgacaagaaagaacttatcaaggaggacttgataaactggctcgtggcccagaatagagaagacgatattcctacagtggagacattcaacaacttcactacgtactttactggcttccatgagaataggaagaacatctacagtaaagatgatcatgctactgctatatctttccgccttatacatgagaacttacccaagttctttgataacgtcatcagcttcaacaagttgaaagagggtttcccggagctaaagttcgacaaggttaaggaggacttggaagtcgattatgatctcaaacacgctttcgaaatcgaatacttcgttaactttgttactcaagcaggaatcgatcaatataattatttactcggtggtaagactctggaggatggtacaaagaaacagggtatgaacgagcaaatcaatttatttaaacagcaacaaacacgggataaggcacggcaaattccgaagttgattccactattcaagcagatactgtccgagagaactgagtcacaaagtttcatcccgaaacagttcgagtctgatcaggaattgtttgactctcttcagaaattgcataacaattgtcaggataagttcactgtactccagcaggcaattctcggtctcgcagaagcggatctcaagaaggtctttattaagacctcggatttgaacgcactgtctaataccatatttggtaattactcagtcttctctgacgcactcaacttgtataaggagtctctaaagacgaagaaggcccaggaagctttcgagaaattgccggcacattctatacatgatctcattcaataccttgagcaatttaatagctccttagatgcagagaagcagcaatccacagacacagtactcaactactttattaagactgatgagttatactccaggtttatcaagtcgacttctgaagccttcacacaggttcaaccgttatttgaacttgaggccctttctagcaaacgtcgtccgcctgaaagcgaagacgaaggagctaaaggtcaagaaggtttcgagcagatcaaacgtattaaggcgtacctggatactctcatggaagccgtgcactttgcgaaacctctctatttggtgaagggaaggaagatgattgagggactcgataaagaccaaagtttctatgaggctttcgaaatggcttaccaagaactagagagcctcataatacctatatataacaaggcaaggagttacctttcaaggaaacccttcaaggcagacaaattcaagatcaactttgataataatactctgctctctgggtgggacgctaacaaagaaaccgctaacgctagtattctcttcaagaaagatggattatactatctaggtattatgccgaaaggtaagacattcttatttgattacttcgtgagttctgaggatagtgagaaattaaagcaaagaagacagaaaaccgctgaggaagctctcgcacaagatggagagtcttactttgagaaaataaggtataaacttctacctggagccagcaagatgttgccgaaggtgttcttctcaaataagaatataggcttctataacccaagtgatgatatactcagaattcggaacaccgcatctcacactaagaacggtactccacagaaagggcattcgaaagtagaattcaacctcaatgattgtcataagatgatagacttctttaaatcaagcatacagaagcatccagaatgggggtcatttgggttcaccttctctgacacttcagactttgaggacatgtccgctttctatagagaggtagagaatcaagggtatgttataagtttcgataagattaaagaaacatatattcaatcacaggtagagcaaggaaatttatacttgtttcaaatatataacaaggacttctctccatattccaagggtaagccaaatcttcatacattgtattggaaagcactctttgaggaggcgaacctcaacaatgtcgtggcaaagttaaatggtgaagctgaaatattcttccgccgtcactctatcaaggcgagtgataaagttgttcaccctgctaatcaggcaattgataacaagaaccctcatacggagaagacgcaatctacatttgagtatgatcttgtgaaggataagagatacacgcaagacaaattcttctttcatgtccctataagtctgaacttcaaggcacaaggagtatctaagttcaatgataaggtcaacggtttccttaagggtaatcctgacgtgaatatcattggaattgatcgcggtgaacgtcatctgctgtacttcaccgtggttaaccagaaaggcgagatcctcgttcaagagagcctaaatactcttatgtctgataaaggacatgtgaacgattatcaacagaaattggacaagaaggagcaagagagagatgccgctcggaaatcatggactactgttgagaacattaaggaattgaaggaaggctatttgagtcacgtggttcataaactcgctcatctgataatcaaatacaatgctatcgtgtgcctcgaggacctgaatttcggattcaagcgaggtagatttaaagtggagaagcaagtttaccagaagttcgagaaagctctaattgataagctaaattaccttgtctttaaagagaaggagttaggtgaagtcggtcattacctcacagcatatcagctcacggcaccatttgaatcgttcaagaagttaggcaagcaatctggaatcctattctacgtgccagctgattatactagcaagattgatccaactacaggattcgtgaactttctagatttgagataccaatctgttgagaaggcaaagcagctactatctgacttcaatgctatcaggttcaactccgtgcagaactatttcgaatttgagatagattacaagaagcttactcccaagcgcaaggtgggtacgcaatctaagtgggtcatctgcacttatggtgacgtgagatatcagaatagacgtaatcagaaaggccactgggagaccgaggaagtgaacgttactgagaagcttaaggcactgtttgctagcgattcaaagacgaccaccgtgatcgactacgcgaacgacgataatttaatagatgttatactcgagcaagacaaggccagtttctttaaagagctcctctggctccttaagcttacaatgactctcagacattccaagatcaagagtgaagatgatttcatactctctcccgtgaagaacgagcagggtgaattctacgattctagaaaggctggtgaagtatggccgaaggatgcagacgccaatggagcttaccacattgcactcaaaggactttggaatttgcagcaaatcaaccaatgggagaaaggtaagactctcaacctcgcaataaagaatcaggattggttctcattcattcaagagaagccttatcaggaatga

SEQ ID NO: 801 - DNA, 3897 bp, Artificial Sequence
  Description of Artificial Sequence: Synthetic polynucleotide
atgacaaagacgtttgactcggaattctttaatctttattctctccagaaaaccgttcggttcgaacttaagccagttggagagactgcgtcatttgtggaagactttaagaacgaaggactgaagcgtgttgttagtgaggatgaaagaagagcggttgattatcagaaagtcaaggagataattgatgattaccaccgtgacttcattgaagaatcacttaactacttcccggagcaggtttctaaggatgcacttgagcaggcattccatctttaccagaaacttaaagcagcgaaggtggaggagcgagagaaggcgttaaaggaatgggaggctctacagaagaagttgcgagagaaggtcgtgaaatgcttctctgacagcaataaagctaggttctcacgtatcgataagaaagaacttattaaagaggacctgatcaactggctggtcgcacagaaccgtgaggatgatataccgactgttgagacattcaataacttcacaacatatttcacaggattccacgagaaccgcaagaacatctactctaaggatgatcacgcaaccgcaatctctttccgcctgatccatgagaacctcccgaagttcttcgataatgtgatttcgtttaacaagctaaaggaaggatttcccgagctgaagtttgacaaagttaaagaggatttagaagttgattacgatcttaagcatgctttcgagatagaatacttcgttaacttcgtcactcaggctggtatcgatcaatataattacctcttgggaggcaagacactggaggatggtacgaagaagcaagggatgaacgaacaaattaacttgtttaagcaacaacaaactagagataaagctagacagatccctaaactcataccgttattcaagcagattctttctgaacggacggaatctcaatcctttattcctaagcaatttgagagcgatcaagaattattcgactcccttcagaaactccataacaattgtcaagacaaattcaccgtgctacaacaagctatacttggattagcagaagccgacctaaagaaagtcttcatcaagacgagtgacttaaatgctctttctaacacaatctttggaaactacagtgttttctctgacgctcttaatctttacaaagagtctctcaagactaagaaggcccaagaagctttcgagaaactgccggcacacagcatacacgacttgatccaatacttagaacagttcaatagtagcttagacgctgagaagcaacagtctactgacacagttcttaattacttcatcaagaccgatgaactttattcgcgattcattaagtctacgtcagaagcgttcactcaagtgcagccgctcttcgagttagaagctctttcttcgaagagaagacctcctgagagcgaggatgagggagcgaagggccaagagggatttgagcaaataaagaggatcaaggcttatcttgacactctgatggaggccgtccatttcgcgaagcccttgtacctagttaagggccggaagatgatcgagggtcttgataaagatcaaagtttctacgaagccttcgaaatggcttatcaagaattggagagcctcattatcccaatctacaataaagctcgctcttacttatctagaaagcctttcaaagccgataaatttaagatcaacttcgacaacaacacactactttctggatgggatgctaataaggagacagctaacgcgtcaatcctctttaagaaggacggattatattacctgggaataatgcctaagggaaagacctttctattcgattacttcgttagttctgaagacagtgagaagctaaagcagaggagacagaaaacagcagaggaagccttagctcaggatggagagtcttatttcgaaaagatcaggtataagttgctaccgggcgcttccaagatgctgcctaaagtattcttctctaataagaatattggtttctacaaccctagcgacgacatcctgcgtataaggaacactgcatcacatactaagaacggaactcctcagaaagggcactctaaagtcgaatttaatttgaatgactgtcataagatgattgacttctttaaatcatctattcagaaacatccagaatggggctcgttcggatttacgttctcagatacctctgacttcgaggacatgtcggcattctatagggaagttgagaatcagggatacgtgatcagctttgacaagattaaagagacgtacatccaatcgcaagtagagcagggcaatttatacctgtttcagatctataacaaggacttctctccgtactctaagggtaaacctaatcttcatacgctctattggaaggctctatttgaggaagcaaatcttaacaatgtggtggctaagttaaatggagaagctgagattttctttagacgacattctattaaggcttctgataaagtggtccaccctgctaaccaggctatagataataagaatccacatactgagaagacacaatcaacatttgaatatgatcttgtgaaggataagagatacacacaggataaatttttcttccacgtacctatttccctcaatttcaaggcacagggagtatccaagtttaatgataaggttaatgggttcctcaagggcaatccggatgttaatattattggcattgacagaggtgaacgtcacctactatacttcacagtagtaaatcagaaaggtgagatactcgttcaggagtcccttaacaccttaatgagcgataagggacacgttaacgactaccagcagaagctagacaagaaggagcaagaaagagacgcagctagaaagagttggactacggtagagaatattaaagagttaaaggagggttacctttcacacgttgttcacaagcttgctcatctcatcattaagtacaacgctatagtgtgtttggaagacctcaacttcggcttcaagcgggggcggttcaaagttgagaaacaggtttaccagaagttcgagaaggccctcatcgataaacttaattatttggtgtttaaagagaaagagctcggagaggtaggacattacctaactgcctaccaacttactgctccgttcgaaagctttaagaaacttggtaagcagtctggtatcctgttctacgtaccagctgattatacaagtaagatcgatccaaccaccggattcgttaacttcttggatcttagataccaaagtgtcgagaaagccaagcagctactctccgatttcaacgccattagatttaattcggttcagaattactttgaattcgaaatcgattataagaagcttactcctaagcggaaggtaggtacacaaagtaagtgggtcatatgcacttacggagatgtcaggtaccagaaccgaagaaatcagaaaggtcattgggaaacagaggaggtaaatgtaactgagaagctcaaggctttgttcgcttctgattctaagacaactactgttattgattatgcgaatgatgataatcttattgacgttatactagaacaagacaaggcgtctttcttcaaagagttgctgtggcttctcaagttgaccatgaccctaaggcattctaagataaagtcggaagatgatttcatcctgagccctgtaaagaatgaacaaggtgaattctatgattctaggaaagcaggtgaagtgtggccgaaggatgcagacgcaaacggagcctatcatattgcattgaaggggctttggaacttgcaacaaattaatcagtgggagaagggtaagacattgaatctagctattaagaatcaggattggttctcgttcatccaagagaagccatatcaagagtga